European Patent Specification EP 3 579 852 B1, published November 20, 2024. Title: Verwendung von Lactobacillus buchneri zur Erhöhung der Fertilität eines weiblichen Säugetiers. Applicant: Freie Universität Berlin. The sequence listing filed with the application follows.

SEQUENCE LISTING (3 sequences)

SEQ ID NO: 1 - DNA, 2506301 bp, Lactobacillus buchneri
tatttaaaatttgtttcatgaacaattagtgtggataaccgcagaaataatcatagctgattttagagatttgcacaaggttatccacaagctcacaccgtgttccaaaagttatccacaggatgtggattctatcaacttttttgtgaataaagccgttgttgtcagctttagttatccacagttgcctgttcattacaccaaattccaacgaccttatccacttatccacaggggagttatccatttcatccacccctgtgaaacaattatgcacaggctgtttttgcctgtggaaaacttttctggggaatgctaaaattaatttgcatttcgttacacgactaaaaacagagggggaattcgtagtgttagataaggattcattatggcaaaagttaagcgaacaatttcgcagcaacaccactgatcttacatatgatacctggatcaaaccagtcaagccgatcagctttgatggatccacactcactttatctttaccttctgaattgcatcgggattattggaaagaacaattggcaccaaacttgatagagtatgcttttgtgatcactaaaggcaatatcgagccaaagtttattctggattcggacgttaataaagaagcccaagaaaagcctgtggataacaatgccagccaagatcaggacggcgatgagttttcatttagtaaggaaaatcatcttaatcccaattacacatttgataactttattatcggcaagggcaatcaaatggcccatgccgctgctttaattgtgtccgaagaacccggcaagctttataatccactgttcttttatggtggcgtcggtttgggtaagacccatttgatgcaggctatcggcaataagcgccttgaagatcatcccgagaccaacgttaagtatgtcaccagtgaagccttcaccaacgatttcatcaacgccattcagaccaaccgcaccgaagaatttcgtcgtgaataccgagacgtcgacattttaatggttgatgatattcaattctttgcccaaaaagaaggaacccaagaagagttcttccatacttttaacgatctctacaataacgataaacaaatcgtcctcacatccgatcgggttcctcaagagatccccaagctccaagaacgcttggtatcaaggttcgcttggggtctaccagtcgatatcaccccgccggatctggaaaccagaattgccattctcaaaaataaggccaagttggataacctggtcattccaaacgacaccttgtcctatattgccggccaaattgattccaacgtgcgtgaacttgaaggcgctttgtcgcgggttcaagcctattccaaattaaaagatgagccgattacgactgacctggtttatgaagcgcttcgtggcctcaaattgagccaagataaccgccagctttcaatagttgatatccaaaataaagtcgccagctacttccacatttccattaatgatttaaagggcaaaaagcgcatgaagtccattgtgatgcctagacaaatcgccatgtacctttccagggaaatgaccagtaactcgctgccaaaaatcggcaaggaatttggcggcaaggatcacacgaccgttattcacgcttgcgataaaattgccgaaatcatcaaacttgatgccgacttaagaaaagaaatcgcggatatcaaaagtgccctgaactaaaatggtataatcgattgtggataaatcatcgagaagtcaataagttgtgcacagtcttatccacaggttaatcgttagggacaggccacttgtgaaaagttatccacaatatccacatgccctactgttacttctcttttcttttattaattaatatataattacactttccgggaggtcgattaaagtatgaaattttccattggtcgaacagcattcacaaaagggttaaacaccgtttcaagagcaatctctaccaaaaccaccattcctattctgacaggactcaaaattgtagcaggtcctgacggtctggtactaaccggtagtgacgctgatatttccattgaaaccacgttaaaagccgatgatccagacaatatgttagttattgaatccgaaggtgccattgtgttgcctgccagattcttcactgaaattgtcaagaaattgcctaaagacaccataactctagaggttggcgaaaacttccagacgatgattacatcaggtcaatcatcatttactatcaatggtttggatgccaataactatccacaccttcctgaaattcaaacgaacgactcaattcctttggccgctgatcttttcaaacagattattagtcaaacggtcgtcgcagtttccaatcaggaaagtcggccgattttaacaggtgttcactttgtcatttccgataaccacgttatggccgtcgcaactgacagccaccgcttgagtcaacggaaagttactcttgaaaccccgatcaatggttcatatgatttcgtcattcctggaaagagtttgactgaattatccaagatgattgatgatggacaagacgaagtgtctttatcggttaccgaaaatcaagccctgtttgtcatcggcaacaccctgttttattcacgactgcttgaaggaaactatcctgacaccactcggttaattccagattcacatgacactcggatctcatttgaagcacctgaattactagctgcaattgaacgggcttctctgctttcacatgaatccagaaataacgtggttaaaatcacgattgatcctgacaaaaagacagttactatttacggtaattctcctgatgtcggaaatgttgaagaagaccttgagcccaagtcattagaaggtaatgaactggagatttcctttaatcctgattacatgaaagacgcattacggtcattcacccaggcgacaattaacattgatttcacgtctgctctgcgaccatttaccctcacaccaaccgaggacagtgacagttttgttcagctgattacgccaatcagaacgttttaattaaatatcgattcgccaacaacttccacaggctgggagttgtttttttctgaccaaaatgagttgcttgctatcgatttctttcaaaaatgctgcaatcacatttacataatgtttgaatcctaaaaaatgatcgtcatttcattagaagtccatataggcaccttttagcagtttttgccattttgatgcaaaaatatcaaaaatcttcaaaacggctcataatgcccaagaatcgtcattgacgtgtacttttagtaaacaaagaggtataatagaaggagtaaaaaggtgggtgaaattgtgaaaaaagatgttttcattgatagtccttatatcactcttggacaattactcaaagaagaatcgattattgccagtggcggccaagccaaatggtttttaagagagacaacagttaatgtcaatgacgagcctgacaatcgccgtggtcggaagctgtatgacggtgatcatgtcgaagttccggacgttggcttattttttattcgctcaaagcagggaaatgaatgaagctaaccgaaattgaactgcataattttcgtaattatgttgatcaaacgctcgaattttccgatgggatcaacgtctttcttggtgaaaacgcccagggtaaaactaatttattggaagccatctatgttttggcactcacccgcagtcaccgaaccaataacgaaaaagaattgattaactggaacagtcagacggcccaaattaaaggtcgcctgcaaaagcggcttggaacggttccgattgaactggatttaggttcaaaagggaagcgggcaaaggttaaccatttggaacaagctaagttgtccacctacatcggtcagttgaacgtcattttatttgctcccgaagacttatccatcgttaaaggagcaccacaagttcgccggcggttcatggacatggaatttgcccagatgagcaatcgctacttgtacaattccactcaatacaaaaagatactgaaacagcgaaatcggtatttgaaagatttgcattataaacgccaaaaggatcgggtatatctcgatgtgctatccgatcagttatctgcttatggtgcagaaattgtttatcaaagacttcagctacttaaacagctggaaaagtttgcccaaaacgttcattctgaaatttcacaaggtaaagaacagttggcctttgactatcacaccacggtagaggctgaccagttaggatcagtcgagtcgatttatcagagtctactgaagcattttgctgcgattaaagacaaagagattttgcgttccaccacgttgattggacctcagcgtgatgatctgcattttgtgattaacggcaaagaagttcagtcatttgggtcccaaggtcagcagcggacaaccgcgctttcggtcaaactagctgaaattgacctgatgaaggaacaaacggatgaatatccaattctattattggacgatgtcctttctgaacttgatgatttcaggcaaacgcacttattaaccgcaattcaagataaggttcaaacatttttaaccaccaccagtttaagtggcgttcagcaggagttactaaccaatccacgtatttttcggattagtgaaggtaatgttactttggcaaaatagtgaaggagaatcaaaatggccgacgaaaaagaaaccaaaaaagaattagcgcatgaatatgatgccagccaaattcaagttcttgaaggactggaagctgttcgaaaacgtcccgggatgtacattggaacgaccagttcacaaggacttcatcatttggtatgggaaatcgttgataacgggattgatgaagcgcttgctggatttgccaccaaaattaccgttaccgttgaaaaagacaacagcattaccgttactgatgacggtcgtggaattccggttgatattcaaaagaagacgggcaagcctgccctagaaaccgttttcacaattcttcatgccggtggtaaatttggcggcggcggatacaaagtttctggtggcctgcatggtgtgggtgcttcagttgttaacgccctgtcctctgaactggacgttgaagttacccgtgacggcaaagtttactacatggacttcagtcgtggtcacgtcaagaccaagatgaaagtcgtccgtgaagtttcggatgatctccatggtactaaggttcatttcctgccggatcctgatatcttccgggagaccactacttatgatattaaagtcttaacagcccgactacgcgagttggcatttttgaacaagggattacggattgttgttcttgacctgcgtccggaaaagccgactgaacaagactttatgtacgaaggcgggatcaaacattacgttgaatacctggataacagtaaagaaaccttgttggatgaaccaatttacgttgaaggtgtcatgaacggaattaccgttgaagtggcgattcaatataccaacgattatcacaatacattaatgaccttcactaataatattcatacctatgaaggtgggactcacgaagaaggctttaagcgagccttgactcgcgtcattaacgattatgcccgtaagaacaagctgttaaaagacaacgaaccaaacctttccggtgaagatgtccgtgaaggcacgacggctgttgtcagcatcaagcatccagacccacagtttgagggccagacgaagaccaagctggggaattcagatgctcgaacggtgactgaccgcattttcagtgatcatttcaccaagttcttgatggaaaatcctaagatggccagaaaaattgttgatcgtgggatgctggcctcaaaagctcgttcagcagctaaacgtgcccgtgaagttacccggaaaaagagtggcttggaaatcagcaacctgcctggtaagttagccgataacaccagtaaggatcctaaaatttctgaactgtttatcgtcgagggtgattcagccggcggatccgctaagcagggccgatcacggctgacccaggcaattctgccaattcgtggaaaaatattaaacgttgaaaaagcaagtatggaccgaattttagccaacgaagaaattcgttcattatttactgccatgggaaccgggtttggtgaggactttgatttatcaaagattaattaccataagctgatcatcatgaccgatgccgatgttgatggtgcccatattcaaacgctgttgttaacgttgatttaccgttacatgcggccattaattgatgccggttttgtctacgttgcccagccaccgttgtatcaagtccgtcaagggaagatgtcacgttacattgattccgatgatgatttgaatgcattcttaggaaccctgcagccatcaccaaaacccgtgattcaacgatacaaaggtttaggagaaatggatgctgaacaattgtgggacaccacaatgaatcccgaaaaccgtcatctgttgagagttgaatcctccgatgcggccgaagcagataaggtcttctcgatgttaatgggcgacaaggtggaaccacgacgcgagtttattgaagataacgcaacgtttgtggaaaatcttgatgtttaaagctgcttaataactaagcagaaaatgtttcacatgaaacatgccaccgaaacccatgaatggaggtaaataatttggcgaataaagataaccatgatgaaccaattgctggtcgagtgaccaacgttgatctatctaaaaaaatgcgaacgtcatttcttgactacgccatgagtgtcattgttgcccgtgcgctgcccgatgttcgtgatggtttaaagccggttcatcgtcgtattttgtatgatatgcatgaattgggtgtgacacccgataagccttataagaaatcagccagaattgtcggcgatgttttaggtaagtaccatccccatggcgataccgccgtgtatgagtcaatggttcgaatggctcaggactttagctaccgttacatgttagttgatggtcacggaaactttggttcagttgatggtgatggcgctgcagcgatgcgttataccgaagcccggttaagcaagattgcgatggaaatgctgcgtgatatcaacaaagataccatcgatttccagcccaactatgatgggactgaacgtgaaccaagcgttttgccgtcacgattcccgaacctgttagtcaacggtgcgtcaggaattgccgtagggatggcaaccaatattccacctcacaatttgtccgaagtcatcagtgccattcatgttttgatgaagaaccccgatgccacgacagcagatctgatggaggctttgccaggacctgattttccaaccggcggcgttgtcatgggtaaatccggtattcggaaagcctatgaaaccggtaagggaaccattattgtccgcgccaaagttgaaattgaaggggaagccggcggcaaacagcgaatcattgccaccgaattaccttacatggtcaacaaggccaagttaattgaacggattgctgaattagcccgcgataagcggattgaaggcatcacggatattaatgatgagtctgaccgtgaaggaatgcgggttgtgattgatgttcgtcgggatgcaagtgccgaagtcatcttgaacaatttgtacaaattaaccctgatgcagacttcatttagtttcaacatgttggcaattgtcaaaggcacgccaaagattttgagtttgaaagaaattttgaactattatctggagcaccaagttgaagttattcaacgacggaccaagtatgagctgaacaaggctcaggccagggctcacatcctcgaagggttaaggattgcccttgaccacattgatgaaattatcaaaattatccgtggttcacagaccggtgacgttgccaagaaccaattaatcgaaggctttggtctggatgacaagcaggctcaagcgatcttggacatgcgtctggttcggttaaccggtttggaacgcgaaaagattgataaagaatacaatcaattgatgaaggacattgaagaatacaaagcgattcttgccagtcgtgaacgggtcaatgaaatcatttatcaagaattattggagatccaaaacaaatttggcgatccacgacggactgaactcttggtgggtgaagttctgagtcttgaagatgaggacctgatcgaagaagaagacgtgatcatttctctaacgcataacggatacatcaaacggttaccaacttctgagtttaaagcccaaaatcgtggtggtcgtggtgttcaaggaatgggtgttcacaacgatgatttcgtagaacacttagtttcaacttcaacccacgatgtgctgttgttcttcaccgatgccggtaaagtttatcggatgaagggttatgaaattcccgaatacggccgttctgctaagggtattccagtgattaacctgttgaacattggcaataacgaaaaaattcaggctgtgattaacgtctccgataagaataacgatattgaaaaggatcttttctttgtcactttgatgggaaccgttaagcgcaccccagtgtctgactttgccaacatccgtagtaatggtctgaaagccattaacctcaaggatgatgatcaggttagcaacgttctgattgctagtgaggatcaaaatattatcattggaactcaccgtggctacgcagttagtttcaatgctgccgatgttcgttcaatgggacgatcagctactggtgtccggggtgttagactacgtgagaacgattatgtggtcggttctgatatcttgaaacctgacagtgaggtctttatcatttctgaaaatggctatggtaaacgcaccccagctgctgaatacccaattaagggtcggggcggtaaaggaattaagactgccaacatcactgaaaagaatgggccgcttgccggtttgacaacggttaacggtgaggaagacatcatgctgatcacagatcagggtgtcatgattcgattcagtgttgaggacgtttctcaaacggggcgggcaactctcggtgttcacttgatcagaatgaccgatggcgctaaagttgcaaccatggctaaggttgagaagcaggatgattcagaggatgacacaaaagatcagtcatctgattcagaacaagcaagtgatgattccggtaccaatgcggatcaaaactcagattcagataattaatattcagctaattacaaagtcgatgagatttaattctcaccgactttttgtttcacgtgaaacataagcatgaattctcctaagaaaatgggataaaaaagtcgagctaattctttgacttacttttagtaagtgatatgctttttgtaagaattaaaatacgactacctggaggtaatttattcatgactgttgttaatggttacaaacaaaacgataacgaagaaaaaattaatattttaaacttggaagagttggaagaacgagctaagcaaatcattccaactggcggttttggatacatcgtcggtggttcagaaaacaactggactttaaaagccaaccgtaaagcatttacccacaagcaaatcgttccgcgtgcgttgagtaatattgaaaatccatcactcgacactaacgtctttggaattccgctaaaaacgccaattatgatggcaccaactgccgctcagggattggcccactcacaaggtgaaaaggatactgcaaaaggtgtcgctgccgttggtggtttgatggcccaaagtacttactcgtcagtgtccatctcagatactgctgcagctgggaacggtgcaccccaattcttccaactttatatgagtaaagattgggacttcaactactcgttgcttgacgaagctaaaaaggctggcgtcaaaggcattatcttgactgttgatgccaccgttgatggttatcgtgaagacgacatcaagaataacttccaattcccaattccaatggcaaacttgactaaatttagtgaaggcgacggtaaaggcaagggaattgctgaaatttatgctgcggctgctcaaaagattgggcccgacgacgttaagaagatcgctgactacactgatttgccagtgattgttaaaggaattgaatcaccagaagatgccctttacgcaatcggtgccggggctgccggtgtttacgtatccaaccatggtggccgtcaattaaacggtggaccagcatcattcgatgttttggaagatgttgccaaagctgttaatggccgtgttccgatcatctttgattccggtgttcgccgtggatctgatgcattcaaggcacttgcttcaggtgcagacttggtagccatgggtcgaccggttatctatggtttggctttaggtggcgctgaaggtgttcaagcagtctttgaacatctcggtgatgaattgaagacaacgatgcaattggccggaaccaagaccattgccgatgttaagaagacccatcttctaagtatcaactattaatttgtgtgcaacgtcctatcatccgtatcctctaacagaaatttttaggcatttgcttctgttctcatgatgggaaataatattagaggatacccatgagtgctgcacagtattagaacattccccgtgttcttttccccaaaaatatgtaataaaacagcgttcctcattattgagggacgctgtttttgaatcagattttaggttaattaatatttttacgtggtcggccggttgtttggcctttatccagaatttctgggtgctcgctacgtgcataagcgtatgcatgaggatcctggccgttttgatatcgactcgagcgggtatttgtttgagaacttctgaagtagtaaaatgctgaaaccccaacgatgattaatagtaaaagtgtcattgaattcctcgtttctttatttttgttaaatcatgggacacgtgcgaaaaagcgtttccaaactccaaattgaatttggaattgatactagtttacttccaaaatcaaaagagtcaagtatctgcttgactgccgtaggtgatttactgggggaacccaagtgtagcaaggggttcctaattattaaggaattatttaattcctgatcgtgaattattttctccaaaagaataatccaggtggtttctatcgtatataataagtgtatcgtgaatcacaattaggcaattgatatttaggtccacacgtggtattattttatattgtgagtatctgggtaaaaacagaaactctccttgctctcgggaagagggccataagtccataaggaggtgcaaatcatggaagaaaagaaatacgaaattacttacatcatccgtcctgatattgaagaatctgcaaaatctgcattgatcgaacgattcgacaagatcttgactgacaatggtgctaaggtactaagttcaaaagactggtcaaagcgtcgttttgcttacgaaatcggtggcttcaacgaaggaacctatcacgttgtaactttaacaactgattcagacgcatcacttaacgaatttgatcgtctttcaaaaatcaatggcgatatcttacgtcatatgatcgttgttcgtgacgactaataattgattctaatatgagaggagcaaattcagcatgcttaatcgtgcagttcttacgggtcgcctaacccgcgatgttgatttacgatacactcaaagcggaaccgctgtcggttcgttctcacttgccgttgatcggcaatttaccaatcaacagggggaacgagaggctgatttcattaactgcgtaatctggcgtaaatccgctgaaaactttgccaacttcgttcataaggggtcgcttgttggaattgatggccgtattcagaccagaaattacgaaaacgcacagggacaacgtgtttatgtgaccgaagttgtagtagagaattttgcgctgcttgagccccgttctgcaaggaacaactcaaatggtcagcaaaatggcaatgctcctcaacaaaataacggtaatgccaatccatttgataatcattcaaatgccggtaccggaaatagtggcaattccaacaataacggcgggaataatccgactaacaatggtggaaataacggtaataacgggaacaataatcccaatgatccgttcgctaactctggggactcgattgacatttccgatgatgatttaccattctaatgaattggtaaagtaaattttcgaggaggaaaaactatggcatatcaaagacgtggcggcggtcgtcgtcgtcgtaaagttgattttattgctgcaaatcacattgaatacatcgactacaaagatatcgatttattgaagcgatttgtttcagaacgtggaaagattcttccacgtcgtgttactggaaccagcgcaaagaaccaacgtgctttaacaattgctattaaacgtgcacgtatcatgggcttgatgcctttcgttgcggccgactaataatgatttatcgaagtcatcctttcggggatggcttttttatttgctcataagacaagccttcccagaaactgaaccgggaaggcttgtatcgacatcaattagttttcgttagtaacgggcttggcgttgtcaacttgttgatcaggtcctaatttctttaaaccgaccccggtgaatccactcaatagtgagaagactgggcaaagcagactgaagaatacaaatggcaggtattggatagttgggacactcaatgtgttggcaatgaagacgccgccaacgccccatggaaccaagtagtttaaaacggtaccgccatcttcaagaacccgcccaagggctcggctggccaggccaccgttattgaacgtctttttgaaggctcgtccaggtaagataatcgaaagaaattgttcaccaacgaagatattcaccccaatgcaggctcccagtgccgctgtaactagtttggccggattattcaatctggtagccagtggtgacataatcgcgctgataaggccaaaatggactaatagaccaccaagcgataatgtcagaacaattagggcaactgtcggcatcatgctgacgatgccgccccgtgaaagtaataagttgacctcactgttagaagtctttgcgataaagccattggtgatgatcgtgctggctttggtgacgtttaatccagggttgttgacaaacatcatccccgctgaaacaaagatgttcagtagcatggttggaatagctgccattttaaagccggcgcagacaaacaccaagatgatcggaatcaaggcgacaattgaaatgtgaaaatcgttgttcaatgcggcaaccgttgtattgatcttgttcatatcggcatggttgtgacccattccaagaagagcaaaggcaatggtggaaatcgtggcagctggaatcgtcgaccaaaggatggttttcatgtgatcaaataagtcggtgtcgaccacggctgctgccaagttgttggtttcggaaagtggtgaacatttatcaccgaagaccccgccggaaataatcgcaccagcgaccagggccggattgaagttcatggtgacaccgatgccgaagaaagcaatcccgacagttgagacaaccgtgaaacaactaccaacggcggcaccaaccagtgaacagaccagaaagacggttggtaagaaccattgggcactgatggctttgaagccgatgaccatcaacgttggaattgttccagcggcgatccaggtactgatcatcgcaccgattaagataaagatgacaatggggatgatgcctttatcaatcccatccttaatcccggcattgatctcatcccaactaaacccagtcacttttgcccaaaagattgtgacggtaattgctaataatactggaacttgtggagacaatcccaaaccgattaccccggttcccataatggctaatgcaacaactaatactaaaatcgcttcacgcaaactcactctactatttctcatattgccaacctctttttattttcaaatttttggctactttaaattcagttgactcaaatatcgtggtaaaccgccattcgttgctcttctcatagaaaatcccccttaagtcaataaaaaatcgtccctactgcaaataaatgcaatagggacgattttaaccgtggtaccacccaacttgtgtatcaaaaatacaccgctcactagaagataatggattctagttattgaccattgtcgtgatattacggtatttcgccaccttaccctgattggttcgcagcaaccaccaacttcctgacacccagataaggcactacttcatgtaattcgactttaattattaaagagagtataaaacttgatgagaggaattgcaagaaatgtttccatgatcgattgctgagaatgacgaagctcataatcccccaaatgcacattgtcgttaaataatcttagcaattcttccccattcgcctaagattatcgaaaaaattcttattttcacctttttaaataacaaaatgtaaccaaacctaacatcaaatgcccatttgtgataatataaatgcattctcattagaactttttaatctaattcttatgttgctcttatttaggaggatgcctatgaagtcaaaaattcaagagaaccaagatggaaccatgcgtgcgttaagtaatcgtcacgttcagatgatcgcgattggtggaacgattggtaccgggttgttcctgggctctgggagcaccatcagtaagacgggtccctcagtcatgctgatctatttggtacttggcctgtttttctttttcatgatgcgtggaattggtgaaatgttctattccgatccgtcgcaacatacattcgtttcatttatttcccgttatctgggtccaacagttggtcattttaccggctggacatactggattgggttggtattcgtttgtatgggtgaaattagtgccacagcaacgtatgttaaattctggttcccccaggttccggcttggattattgaagttattttcttgggagttttagctggaattaatttaattgctgcacggttgtttggagaagctgaattctggtttgcaatgatcaaaatcgttgccattctggcattaatctttactggaatctttatgatgttcagccattcggtgacgccacttggccatgccacaattggcaatattttccacaattttcaactgttcccccatggcggtgtgagttttatcgctgcgttcccaatggtcttcttcgcattcatgggaattgaattcgttagtatcacaattggtgaagccaaaaatccgcaaacggttatcaaaaaggccgttaatgaaactttgattcggatcttaatcttctatattggggccttgactgtgattatggggatcatcccatggtcatccattacccctgacagcagtccctttgttcaagtattgaaactcgccggattaccagcagcggccgccgtgattaactttgttgttttaacttccgccgcatcatccttaaacagttgtatcttctcagccggccgacatttctatcagttggcaacagaagttccggaagacagctggatgcgaaaaacgtttgctaaaatttccaacaatggtgttcctgcccgggcaattatcttctcggcagcactggtcttgattacgccactgatcagtttgactaacagtttggcatccgtatttaccatcgtaactggaatttccagtgatatgtacatcattgtgtacaccttggcaatgctggctcacagaaagtaccgtcaatcagctgacttcctgccaaatggcttcttgatgccggcatacaagatcatgagtccgctgacaatcgcattttttgtggttatctttggttcactgttctttgttccagaagacattattggtgctgttggtgcaattgtctggacggttgttttcggtgccgcaacttatatccatcaaagacgattggttccagacaccgaccagtaattgtctaacaattcaatgaaatgaatttgcatgtctcttccaataaatatcatataatgactctgaaaaattcccgacagtgatgctgggaatttttctttgcttcatcattgagatgagaacccaccagaaataataaagcaggccgatttatggtaaaataagagcattaagctattatgaagaggaattaacatgaaaaattggttcacaaacaaccgtggtgaactgccaccatttgttcataaccgacgcctcagaaggatcatgatgttcatttcattaatcgtgatctacggcatcgttatttcatttttatataatatcgtggcttccctcattctcattgtgatcagtgttgtcggcttgatttttaccatcgtcatgatgaacgaaatcagttccgataccaaccgctatattaccgacctatcataccgaattcatcgtggggaacaggagtcgctgctcgaaatgccgatcggcgtcatgatcttaaatgacgacgaacaggtggagtgggcgaacccctatatggtgaagtattttaaggatgagaatttgttgggtcgaaagatcgacgacatcgatcatgacctccagcagttaatcaccaagtacgctgaatcagatgaattccacacgatcacttggcgggaccataagtttaccatgctgatccaaaaggaatataactcggtctatttgatggatattacccggtatgccaacctggaggaacgatacaacgaagagcagatctccgttggtcaaattttcttggataactacgacgaaattacccagtcaatgactgaccaggaaatctctaatttaagcaactatgtgaccaacgaattggcaacctggtcccaaaaatatgggatgtatctcaagcaaatcgatgatgaccacttcttcctgctggcctactcaaagtcgttgacggcgattgagaatgacaagttcaatatcttggacactgtccgagagacgacttccaagcaaaacttcccactgacgttgagtatcgggattgcttacggcgaagatgacctgaataatttggccgaccaagctcaaagcaaccttgatttagcgttaggtcgtggcggtgaccaggtcgttgttaagtcattggatggtaccgcgcggttctatggcggcaagaccaacccaatggagaagcggacccgggttcgggcacggatgatttctcaagctttgaacgaattgatgagtgcctcagatcaggtctttgtccaaggccacaccagaccggacatggactccttgggtgcttgtctggggatcagacgaattgcccaaatgaataataagaaatgctggatcgtccttgataaggagaaggtccactcagatattcaacgattattggaagcaaccaagaagtacccagaaattgccgattcaatcattaccccttcagaggcgattgccaaagcaactgacagcagcatgctgattatggttgatcattccaagccttcaatcagcatttcagaagacttatacaagcgaatgtcagcaaaagtggtcattattgaccaccatcgccggggtgaagagttccctgaaaacccaatgctggtatacatcgaaccttacgcatcatccacttgtgagctgatcacggaaatgtttgaatatcagccgcacgaagaagaaccaatcaaccggattgaagcaaccgcaatgctaaccgggatctttattgatactcagcgcttctcaatgcgaaccggtaccagaacctttgatgctgccagttacttgcgttctgcgggagccgattctgatgaaatgcagcaatttatgaaggaaaatattgatagttacctgcaacgcaaccatctaatttccaaagttgaattcttccacaagaatatggctttgattgttggcgaagaagaccaggtttatgatccggtcacggcggcacaagcctgtgactcgttactgacaatgtctggggttgacgcatcattcatcatcactaagcgctccgacggccaaattggcgtttctgctcgaagtaccggtgccgttaacgttcaagtcattatggagcaaatgggcggcggtggccacttatccagtggtgccacccaggtttccgacaagtcggttgccgatgtgaaaaaaatgttgcttgaaacgatcaagaatatcgatgataatgaataaaggtatttaaatttttgaggatagtaggagtgatctgttatgaaagttatttttctgcaagacgtccgtggtaaaggtaagcgcggggaagttaaagaagttcctgacggctatgctcaaaactttctgattaagaatgggaaggcaaaggcagccactaaagcggcaatgagccagttaaagggccaacaaaaggccgaagaaaagcgtgaggaagaagagttggaggaatccaagcagttaaaggccaagcttgaagacgacaagacagtcgttgaattaaaggccaaagctggaacggacggccgcctctttggttcaatcccaagcaagcaaattgccacagcactggaaaaacagtatggtgtcaagcttgataaacgcaagattgaattaccggaaccaattaaagttgccggctacaccaacgtcccggttaagttgcatgttgatgtgactgctaagatccgggtacatgtttctgaaaaatagagcgcgaacaacctttatccaggtaaatgtaacagagactcctcacaaaaggaccaccttgtgggcgagtctcttttcttctccaatctgaccagatttaaggggagtgtgctacaatttaactattgtatttaacgtgaacgaatttgaggaataaacatgagcaatgagtttgtaaacgaattaccaccacaaaatatcgacgcggaaaaggccgtcctcggatcgattttcttgagtaccgatgctttggttgagtccatggagttcttagagcctgatgacttttataagcatgctcaccaaattatctatcaggatatggtcactttaaacgaccgcgatgaagcaattgatgtggtgacaatcaccaacattttaactgaacaaaataacttggacgacgttggcggcatggaatacatcgccgatctggctggttctgtcccaacggctgccaacgtggcttactacgcaaaaatcgtcaaggataaggccattttgcgccggctgatccaaactgccaccaacatcgttactaacagctataataccgatgacgatgtcaccacggtcttggatgacgctgaacgagatattatgaatgtggctgaaaatcggactcagtctggttttaaaccgatcaaagaagtcttaaataacgcctttaacgaaattgaccgcttgtcccaagaaggggatgcggttaccggtctttcaaccggttatccggaactcgacaagatcacaacaggtttgcatagcgatgagctgatcattttagctgcccgaccggccgttggtaaaacggcctttgccttgaatctggcccaaaatgtcgggaccaaaacggataaaactgtcgctattttcagtttggaaatgagtgccgaatcgctggttaaccggatgctgtgtgccgaaggtagtattgatgccaaccatttgcgtaccggtcaactaactgaagatgagtggcagaatctggtagttgccatgggcagtttgtctcgggccaacatttatatggacgatacggcggggatcaagatgtctgaaatccgcgctaaatgtcgacggctggcgaaggaaaccggtaacttgggcttagtggttgtcgattatctgcagctgattgaaggcagtaacgccgaaaaccggcaacaggaagtttccggcatttcccgtcaattgaagaaattggccaaggaactccatgtccccgtgattgcgctatctcagctttctcgtggagttgagcaacgccaggataagcggcccgtcttatctgatatccgtgaatcaggttcaatcgagcaggatgccgatatcgtcgcctttctttaccgtgatgattattatcgtgatgaagacgatgatagtgatgattccggctccgagggtgaagacgacgaaaataatgtcggagaagttgaggtcattattgagaagaaccgatctggccctcgtggaacggttaaattactgttcgtgaagtcgtataataagttttcatcgatttcctatgctcagcagtaatagattttatccaaaatatcattctaagcggcctttgggaaattttccattggccgtattttaatatcgttatttgtaagattcttctatgtcagatatttggcaagaatttcgatgatcaagtataatcagacttgaggacaattgtgaatttgtttaaattggagggtctttaatgacaaaacggcttaagattggaattttggtagtgacttttctactcatccttggcatttcaaacaccagccaggcaaaaagtaaaattaaagtttattgggataatcatgatgatcgattggatacaacgcatatgtatacggccccaacaattcagaaggatcagcaaactggttacatgtggaactttaagcataccaagcgaattcataaactaaacaactataagtacaccgaatggaatttgtatagtgctgtttccgttacaactaagcatggaaagggcatctattataagattagtaacgctgatcaatcagttcgggggcttgtctatcataaatatgtaaccagggctttagctaagaacgttaattcatttactagcgatgcagaatacattaactatttaaagacggcaccatctcaaaaacttgctagacagattttgaagctattcccgaatagtcaggttagtttggatttgtcaaagcaagttgctaacaataatccaattgctaaaacaggattaatcccacttaatggatttaccaataaattggattttaatgccaattatctgacgtataagggtagtaaatatacaaattacaaaaaccattattttcttgggtctgatccttcatcgtttttgaattcgacatatttattacctgctacgggtcgagtaaatgcagttgccaaaatgcttgatgcggcgggatacactgctgagaagagagccaatatgggaaactatcaactaggaatttgtatttatgatgaggtgggggatcaagataatcacaaaagtgatacgcttatccatcctgggggatcaccatcattttatttgatttataatgttgttttaggggaaaaagaaaattaaaaatgtggtttatgtatactaaagggactcggaaaaatctgagtccctttagtattagtcagatattagtcaaaaaccgacttatcaaaactatagaccgtatgtggtgtgtcactcccgccatggaattctaagccaatcatcctcactacagacactaataatcaaattttgggaaaagcgattcgggtcataaatgagctgcaatgacgattcgttcctgcaaatgttaaatgcgtcaatagtgtttgtggtttgtaaatcgtttctccaatgcaaaaagacggctcctttgagggaagccgtctttgggatattcattattttttaaaacttggtcggaataacagctgccaaaccgcgtcgttctttgccgcgataaccaatccagactgccagtgacccgattaccaggccaccaagtgcaacccaccagagggtctgctggaaggcacctgtgttgccgaggttagccatgatgttataactgctgtagatgttttggtacattggcgtcgtttggcttaagaacttgtagaaactggtcatggccgcccgtgggagcgttccgccaccagccatgatttgaaggacgaacagtggtaattgaatcagcaaacttggtaggccgccaaatagaagtgccaagccgctggtaagttcgaaggctgcaaaatcgtacaagacattttgccaaagcaaagcgttgaaaaccccaccgtcaaagctgacgaggcatcgcagcgcaccaacggtcaataatgctaaaacaaccgcggtgataacgcccgtgacttgaaggccaaggaaggttttccacttgccggcgatgaaacgaaccgacatgaaggtcatcgtgatgatgattgaagcgatcatcaggcccagatattggcccatcgagataaacatcggtgccatctggtgctgcatattgacctgcttggtacccatggtatcggtcgatgatttagccgtaatgttaaatggtgctgccatcttagtggcccgggccatgacttgcttttggatcttgggttgtacttttgcttgaacctgtttttggatctgtttttgattaacagcttgaccttttgaggccgtcatagctttttgcatggcggtcttcattccagctgccattgcagttttcatcatcttaggcgcaagttgtttggcatacatgccgacaagcgactgctgggtcaactgggcgttaactgtactttggatccgggagatcagtccctgattaacgttggtttggaccatgctattagcgttattgacgacaaaattaacggttggtcgtttgccggcacgaacgtccttattaaatccatcgggaatcacaaccgccagcgaagctttacgaagttcgattcggtgtttggttcggcttaggctactcgaagtcgaaatatgcttgaagggcaggttgtccttcaaaccgtcggcaaccttatccgagatctgttggttatcttgattgacaatgacgattggtaagttttgagtattggttggcatgtgcttgaaagccggtagaatgcagaatacaaacgaaactgcaataaaactggcgactaacattcccagccaactaaatttatttgaaaaccattttgacattttagttgttcctccttaaaatgacgaatgaatgctcattcatttttgtaacttagcaacaataatctttttctaaacaaatgtcaaacacatttgaaaagtcattccaagtccgctaaactaaaaacgaaatgaggtgcgagctgtggctgatgcagagaatgattttcaacaattatataaagagacactcaaaaaaatggacggtctgacagataaacagaagcggatcctccaggcggccctcgaactgttttctactcaaggctttagtgaaacctcaagtgcccaaattgctgatcgggcaggcgtggctgtcggttcggtctatcagcgtttccacaataaacaggctttattggtggcggtgctggccccactattaaacgatgtattgcctaaagccgttgacgagtttggcaatacggctttcagcaagtcttacgatgaggtcgagccctttgtcagagcaatcgttcctgatcggctgagatttatcgaccagaactacgctgccttgaagttacttgccggacaggtgattgttgaagatgaggggattatttcacagcttacagaggcctttagcagtcacatatcatccaacgtgataccaaatatcaaacatctgcaaaagaccggcaaaatggcccggttcccggagcgttatgttattcaattcctgttttcgtctgtcattggctattttggcaaacgaattctcggcattccggtgaacattgaagatgaaattaagtatatgaccgtctttttgacgaatggactaacatatcataacgtcaaatagctgtccatcatcctatgaagggatgcagtggacagctatttttaggcaaaaaaataacaaccacggctatgagtagctgcgtgatcgttatttaatggtatgtaattgatgggcagtcagggtattgaacccaactttttagaaacccgctatcttacagtgttcatgcgacttttcgccaaaataattcttaaaatgcttaccgatttgcttaccattgactaaaaatcaaggtaatttgctaacttttcggctgcttgattatcttgttttttggtaacgtgggtgtaaatatttaaagtagtttgagcatcttcatgacctaatcgagtttgaacttccttaatggttgccccggctgcaaataacatacttgcagaagtgtgacggaaaccatgaacggttatcttttttaggttgtgagctttaataatcttattcaaccatttagcgggtgtgtttaatgatttaaacccattattactgttagcaaagatcaattgaccacgttgaatcgtattgaatcccagcattaaatattcgcgcctttgtcgggcacgccattgttttaggtaattaagcgtaattttgtctaaagcaatgacccgctgacctttcttggttttcggtggttgaatgatctgcttaccacgcattccttgagttaatgttttgttgatacttagtgttgatttgctaaaattaacatcattccaagttaaggctaaacattcaccacgacgaacccccgcaaaggctagaactcgaaacagcgtgtatttctctaattcctctttaggatcaatgtaactaaagaattgggcaagttgctgtttatcccagaagttttctggcttttcaccccaagtttctttacgtttagggatggtaatcatcttagcgggattatcaccgtgcatatagccgtgttttaaggcgtaatcaaaaatagccatcgtgtattcataccaccgcttatagttgtacgttgcctgtttgaaccacttattaactgctcgttgaacttgagcaatggtaattgtacgaatccttttatttcccagttctggtaaaatgtgattctcaaacatccctgctgttcgacaatatgtgctaactcggacagtgttaatatatccttgataccattgttcataaacttgtctaaacagaatattactttcctgatggaagtcacctcgactaattgataactccaattgattagctgctaaggtggcttctttttttgttttaaagcctcttttcatgattcgctttggtttacccgtttggggatctaaaccagcgtagacctgaaataaataacatttgttgccattctttaacgtgtaacccttgatacttgccataatactaccgttcctttcagcgccagctcgtgaacggtatgtaaactgaaagctatttacctttatgctgtttatctgataactttgttagatttggatgcgttatttgtcgaaaagtatcatcctcaattgtatgttcttgttcatattgctgttcgattccgtctgactcgtcatccatggaaataaccattccagagaacgccatgtattcaaagtggtatttttcaggattaagtgcgctttctgttccaaggttccaattaattattatttggtatcgtgctttactatcaatgtcaatattggaattactaataaaattctttattatttgatttccaatataggccattagactttttttgaggcttttaaacaggccaactgtttcgccaaaattcattaacatattgttaactcttatttcgtgcagtttcgattgattgattttgtttttcaataaatcaatatcctgtttattaacccattcgagcgagaaagataaattctttttaagcaggttgtttttagatgtatttaacccctctgttaatctttcagattcgattttattgaaactcacaataaatatggcaacttctaagtcagttttattgttaaaggttctttcgtattggataccaacaattctattttcgtccgtatttagtttttccccgcttaattcaataaattgaaatttctctgtaggtattgtccttgatattagttcagaaatcccgatgttaaaaaaagtacataaagcctcaagggtatcaaattgaattcccttgctttttccattgtacatattcgttaatgctggtcttgaaatccctgttatctttgacaatcggttgatgctaatttttgaagcgtcaacatatctctttaaattaacagttatcaaataattacctccaaattgtaaaatatatattcaccaaatatcatacaacttgttattcttattgacaatggaaaataatcaatataacatgtagttattaattacgataaaacgtaattatgtgaatatataatttacaaggaggggcgaaaatgccagcaaataaagaaattagagaggaaattcaaagaaacgatttactgaattgggcagttgctacccaaataggaattgcagatacaacactttcaagatggttaagaactccattaaatcaagaaagacgtaaacgtgttgaaaaggcaatcaaggaacttactaaggtaaaggagtgacagcatgcaggaaccgttaaaagtaaccttaaccagtgaagacagtgaacagctaagacgtgaagtgtttgcggtgatgtcagaagctgttcaacaggtcagaagcaatgcgattcaagcgccggaatggttgaaaggaaaatccggtgtggccaagtacctttcagttggaacagatacggttaacgggatggttaagttggggttgccggagcaccacacgaaagcatccccgaatatcgccttctttaagaagtcggaagttgatagttttctcttgaatgacggtttaatcaaataaaaacacaagtcgccagctcgtaaacaatcgtcaagaaagaatgtaacacataaaaaaagcccgctgaaattgatcaacgagcgatggtgaatcagtttgttggtatttagttttgaaaggaatgatgccattccctttgtggaacaagtctattatatcgcaatatcaatctactaacacgctgaaagaaggttaatcagatgaaaaaggaaattgtgtttctaagtagtgaagctgtttatgctgacacttttacaactagtgatgtgattgcaaaatatgccggttcatcgcacaagacggtgaatgaattaattcgtaggtataagaacgaccttgaagaattaggggtacttccattctcaatggagttacccctcaaaggaagtaaaggtggtcatcctcgtaaagtgtggcgtttaaatgaagaacaagcaacgctgttaattacctatatgggaaatacaaaactagttagacagtttaaaaaagtattggttcatcaattctttgcaatgaaacgggtactttataaaaaacaagtgcaattcgaattgggtaaacagttttccaaagatctacatcaagcgattgctgaaagcccccatttggatgaacatcatcacttgtatggaaatgttaacaaattaatctacaagcaggcgctcggcgtttcaacgaagacgttaaggcaacagcgggacatccctaaagatgaacccattacccattaccttaatagcaatgaagccggtgcggttaaacgagttaagcaacaagtccagatcttgttagggatgcatttagattatcagcaaattaaagacactttgcaggttcagggcattgtttatcaaataaccttaccggctaagcaacttatgaaagaaggtcattaggatgttaattgccgagattggcgcatggattttgtttttggtgaagtttttaactgcttttggtttaggagtcgtggccaagagtatgtacgatcatccccacgactggtttgattaagaaatgaggttacggaaatgaccaacgagggcacaaaaatagaccgttcaactttggcgagtaacggtctaacacattcccatatttttgtgcccttttattttaacaaagtaaagggagtaattaaagatgaaacaactagattttagaatggtagaagcccaaatgaatcaattaaacacggatacactcggttacatagcaaccgttaagcttattcaagatgctttggcgcgctacttagaagctgtctaaaatctcttaagtaatagtgctaaaaacgctaaaacgaccatttgcagactggtggttaattgacgctcacaatttttccaaagtcgccgacaattctctagccaactaaaagatcgttcgactacccaacgttggggcatgacttcgaatcgatgcaactcattgcgcttcgcaacctgcacggttgcgtttaaattactggctacatcgagctgaaaattaacgcctgaataaccaccatcaactaagacattttgaacctggcgtaaatgcatggcatgtaaagcgatcatggcactggccccgtctcgatcagagacgttcgctcgcgtcatgtgaatggcctgcggaaagccattgatatcaactgccagatggcgcttaatccccgagattttcttaccagcgtcgtaacctttgttttcagcagtagcggtgtttttgacgctctgagcgtcaacgataataaaggaagttaaagctgaacgtccttggtaagttcgccgagcaatgacaatttttttaaaacttgttccaataaagaatcagccgtaggctcagctttagttgaccaaattttgtaatagttgtaaactgaccgccattctgggaaatcaccggggacttgacgccattggcaaccggttttcaagacatataggaccgcacagaagacctcgtagaggtcatattttcgaggcttagttcgcttacgaaaattttctaaagctggtcgaattaattcaaattgttgccgagtaatattgctgggataatttttcatagcttaaactcgctttttacatagaagtatatcaaaaatcatagatcttggacagcttcttagaaacccataatatggattcaaagcattatgacaaaaccagctgggaactgattattaccacgaatgatattttaggtaatatgctacagcttatgattgaggatgaaggggttcaaaaccagctaagcttatcaattgaagaagtacagaaagtggggtaatggcatgcgtaaccgacaacaggaactattaaacgagtctttacaagaactcactaatttaaaagcagaacttaaattattaaccgcagaagtcaataccttaaaccagaccccgccttgtaagcgggctgatgtccgatatttacttaacagtctcgtgattaatgttgaacatgctgaacaggctgtccaaaccacccagcagttaactgtcgggattcccattttaggcactgtggattagagaggagttagcaagatgaaagatgatcgcattatttacccggagttagtggagcaatcccatgcttatatgttatcacggggcgtggatgtttctaaggatgtcgtttaccgccatatgatcaagagtcatttgatcgaccagaacggtcagccgaccaaaaaagcgattgatgaaggactggtatcagaagccaatgacccgaattcgttagccctcttcaaagcccagaatccattattcttaccctatgatgatcgtcactttatttgggtggccgaatcacaggaatgggcagccgatttatttgtcgccaaagatgtttctaaacggattatagatgggcgggcaattggaaataaacaccatgcacaagccgttttgaaatatcttgagaagcaagaaggtgataaccatgaatgagttaactagtatcgcccataagctagccaaacaaggcctaaaggtcttccctttacaagctaacagcaagcgcccagtgaccgcccacggttatttggacgctactgataacctaatccaacttggtgaatggtttgataatgaccggcagtataatcttggcttgcggttggctgatacaggcatagttgtggtggatattgaccatcacacccaaatagacggccgcaaggtgttaaagcagtggcaaaccaaggggatgactctcatccctcaatatgctgaacaaacgccccacgatggcttacattacttctttaagactaatcaaaagctaccggataaagtgattgtccctagtatcgaactcaagacgaagcaaattatgatagcgcctagtcagcttgacggcaagccctatcagacaattaagggcactgatttaacccatttaagcccgttgccggtatggtttgttaatctgttaacgagtcaacaaaccgctcacaagaccttacagcatcgtttatataagtcgtggacaggtaagctattagatcagctagtaaccggaactgatcaaggacaacgcaacatctatttaacatccctgttaggtaaattactgcataccggttgtgatggtgatactgcgtacagcttgttggtttttgctaacgaacatttaactccaccgttaccagatcgagaagttaatacaatttttaaatcccttttaaaacgggcattaaagtaagtgaggtgatcaattttggacagtgaggcgcaaatgttagcccagcaatatgatcagacagtcaatcatccgcatactctaaaagacaaattaatgatggatgtccagacatggcaacttgatcatcaaaccaaagcccaagcgaagaatgacaccttacctcgtttaacaacgttagctggttcgcaaattatgcaacgtcattttataacctgtttattttctgataatgaaagtgctcggttagccatttacttaccgcatgaaggtatttatacccagaattaccgatacattaaacggttgatcggtatgatgtacgccccatttaatgagcgagaggctgaagaagttatttatcatttgattaattgggcgaaggttaaagagccaaccgttgaccgctatttaattccggtggccaatggaatttggaatctccacagacatgagttaatcccctttagccctgattatgtgtttactactaagatagcaacaaagtatgtcaataatccagttccaccaaacattaacgggtggacagtagacggctggttaaatgagattgccaatcacgaccccgaaattgttaaattgctttgggaaattatcaacgacagcttaaacggtaatttcactcgcaagaaagccatctttttatatagcgaaaagggaaatactggtaaaggaacgtttcaacagttgatccaaaatttagttggcaaaagtaatgtggggtctttgaaagttaaccagtttgatgaacggtttaagttagcactattggttggtaaaacggtttgtattggggatgataccccaccggatatttatatcaaggacagcagtagttttaattctgtggtaaccggggatttagtcacaattgagtataagggccaagatggttttacaacaactttaaggtgtacggtcattcaatcttgcaacggattaccaaacttccataacaagggtggcacaatgcggcgcatgatcattgtcccgtttaataaccactttgaagggagtaatgacaactgggatattcgggacgattacatgagccgtcaagatgtcttacagtacgttttgtatcgggctttacagcttgattttaaaaagtttgatgtcccaacggtttctaagcaggcattaagtgagtttgagaaagacaatgacccattaattgggttccgagaattctttttgagtttagaggttgataagattccaacatactacgtgtacgaatactacaagaaatattgtcagatcaatgggctaaaagctttaggacagaataaatttattcggcgactattaccgctcattccggattataccaaaaagaaagccaaagctactcacgaggtttttcaacaagctaatcggtttaaaacacaagatgaaataacagtgtatgttaggatgcctgaaattggtaaagggtatcaatgcttaatcaaaaaagtaaaaaagtagaagtgagttagggtcaaatgtggaactctggaaccaatcatggccaatctctttggtatcaacggattcagcggttccacatttgaaataaaagtggaaccaaaagtggaactaatcacggctaatccttacagcctctaaggatgatctgcggttccagaaagttccagatatatatggaactttgaaaaaagtaccagaactgacttaaaatgtggaacctgaccagcaatcgaggaaaatgttgttgtatcaacgtttaaacgccttaaatcatcaaaagttccataattggttccattttgtttttaaaagtggaaccatgagatgccttggggaacaagcgatacagccgaaaagttccagagttccacatttacccctcctttacttttatatttatatgttttttagtcatttatttgccaaaaaggagtgatgattgatgaacgaattagaatttaaacaaaccaaattgcttaaaagaatccagaatcatgaaatgatgttatcaccgtcatgtgttagcggttattataatcggacgactgataataacccgctagattttaccaagttatcggataacgaaaaaataactttagtaaattggattgttaccgtttttaaaccaattaaaacggttaacaaatggcacagttcttacggattgaaacacttgtttgaacatgctccgttgggcttctatgttaaaaatggggcgtttaaaggagcaatgctgattgctggttttgaaccggttgaccctaatgaacttaattggcgctttaaaatttcagaggtcagcattgataattcagaaatagcgaaagcatgggattttaccagcaaaggggacaactaacatgcgtaaattaaccgaaaccgatattcaagtattgcggttgttgaaaaaaggcgctgataataaagtaaccaaacgccaattaatggataaagccaaaataaccgctcgtaacttgtatgatgccattgaagcgttacgttcgttaggtattcccatcatggctattcgtaacgtcaaggatcccggctactacattgcccagaccaaagatgaaaagattaacgggattgcccagtataagaaacaaattgctacggaacggcacaacttagctttacttgaaaaggctagcattgacgactatttgagtaatgccattaaaaaccctgatttttggcggttgtatggtcatgatttaatcaaggtaaccaatattacagatcattcagtaacgtttaaaattaaaagtacacggtaatgtccaaagttccatgaaaaagtagattctaatatagtttccattcaggtttgcagtctactacgtggtcgtaatcgtcaaatgcacctgacaagccggccaatgggttggcttagcggtgccgaggcgatggttagacgaaatcaaggccacttaaataagcctcgggtcatttaagtttaacccattggcttttcagctcgtcaagtgttcgctaccgccatttgacgataacgaaccaccgggctctaattaccaaaatcaagcggttggtagctgttcttgcgcgagtttgatgagtctcaaccacttgtctggcatgcgggtaagccccgttaattcaggaacttcaactggtggatggtatcccagactttgatggggccgtaaaaaattatggcagagtgaatacagcgtcacgtaagtgatggatccgctggctgacttaaagccacccattgggcggtagtttgcttttagcgagcgatttaaacgctcaatggtttgcttggctggtcgatattctcttgccacttcggtttcgttggttaagcctttaacgatattgaggccaaaattaatgccttcctgatgcgcataatacagtctggccactcgatagatgggattatcgtcgaccgtgaaccgcaggttctcaggaatcacttgatactttttgaggacttgatagatcgcgatgcacgctgattcagtggttcgcttgggggtcacgtaatctgccagaataatttttttgttcacgtcatagaagtagaacagatagtgccattttcctttcacgcgcagataagtttcgtcacccaccaattggctggaaagctgatacggataattatccaggaagggtcgaacattggccgccacggcttgtgcgtaattgagaatggtttgcttggaaatcttgatgccatggatgtcgtacattaacgcggcagtcttggcagcggagatgccatagttcacatagtagctgaggattaatcccagcacttgtggtgaggcctgaatgcgactgaggtcaacccgagattgcgcggatgattgcggggctatctggcgaattttaaaagcgtattcccgatagatgtaccgtaacttgaattgtgatggccgctttaagtattcctggtattgactggaatttagtttggccagctcacgtttgcgatgagggcagtgacgattattgcaccgccagaccttgaagttggcccgctgcttcgcaagttccagtttgttttggcagtcgggacagcgaagcacgacttctttccgataatgtttttccgggttgaaggtggtctgacaaatcttgcagaggagtaatgagcttttatcgccaccaccattggcgttcagaatagaattttgaaccgtctcaaccgaaccattgagattaaccggcaagccctttatcaattagatgctaatatcgatcagttattggccaaagattggcaaatgaccatgcgctaccaccggttgtatgaccatctaaaaagcaattgggtagagttgaacgatgaattagagcaagtcacccgtgacttatggtgcctcacacaagaccaagttccccttgattattcaaaggtgactcccaaacagcaccagttaattaagcaagagtttgccaaatatcatcgatagtcgcaagctaaaagtatccgtcagtaaacgggtgtttttttatgctgacatttctgacaccttaaaaagaaaaaatcttaatttctcggcgcttacaattccatcagtggtgttttacatctacttgtgatgtaacgatatctcttttactatcaaaatgaactcataaatggttttgatcatgcaataaaatcacaacttcgagaacttttatttggggatgcgtaacagttatagaccttgatgttataatatttgccaacctttcggcttaagcaattagcagttaaaaattgaatgatttaatttggtaaaaatgacaaggttttggcaaggtaaaaaccttataaaaccccatatttttttgagagtcatgcacctaaaacactgcaccctaaaatgcaacgtgttgcacccttttttattgtgttgcatatacttaaacccttggtaatactggtattaggttgctttatatgttgcttttttacatcaagaattggtagattgtaaaattaatccgaacgctgttcggacaaaaaagatcagcttcctttaaaatggtgtttaccacaaacccatcttttaggagctgatcttttgtctagtataacctattccgaacgaattaaaatcgaaaccttttgtgaactagggctgtccaatatccaaatgggcgttcggctgaaccgatcaccgtcaacaatttcttatgaattatctcgatgtcaaccttatcaggctgaattagcacaaacagatgccgaatacaagcgatcacgatgtggtcggaaaactaagctgagcgatgagctaaagcaaaaaattctcaaccatttacgcctaagctggtcaccaggaatgattgctcacgaatttaaactagctactaaatctatttataattggctaaatcaggggagaattggtttctccttgaatgatctacctgaacatggcgtacgccaacggcgtaacgttgaccaacgatccaaatataatcaatctttggggcgatcaattgaacagcgtcccatgatgattaatcaacgtaatcgcatcggcgattttgaactagatacagtcgttggtcctcgtgggcatagtaaggcagttttattaactttaatcgatcgaaaatcacggttcctttgggcataccggttaaaagatcggacgacagcgactgttaatgaagcactaactaagttcctaaccacttttaatggtccggtgcacagctttactgtggaccgtggcactgagtttagtgggctagtatcacttgaatcacaatatggtattaagacctattactgccatgcttatactccagctgaacgtggtagtaatgaacgctttaatcggaatttacgttatttttatcctaaagggactcgttttgagcacattagtgctcaagatttaacgacgacgttactccaaattaaccagcgaccgcttaaaatactcgactggccaacaccgtatcaggttatgctgacaaatttgtccaaaaattcggattaaatttgcaatctacctaataacgaatacaattattaatgagttagttcagtacacagaatatatttgtgatcgtttaagcatttatgttgattcatatcagaacataagggttttgattatactagtgggtcgtggaacgaaaagaacgtttctttacctttggataataatcttaaatcaatcatattggttcctgccggattgattgtgaataagtatccgtattcagttaatagttatatcagcaagtctattttgcctgcacgacaaactgaattgttgaagcatggcgaaaaaaagtctttgaaaaatatttttcaaatggacactcgtgatatttcccaaaataaattaaaaacttatgccttacaagaatcagttagggatcctaaaaggcttcacgagttccttgagctaattcatctagtagcatagtataaacagtgattaatttctttgcatggaggccttatatttgtaggtctcatgcatgtacatatagatgaatggtcttaaacgagtttaatagcatagtaaacttatgtatcacattaagctctttctaataggagtaagcaactatggaatacaaacaactaatcaaagaactaacggatttccgcgacaatcgcggatggaataaatatcataccctaccagccttagctagagcggtgggagttgaatctggtgaactgaacgaattgtttttatggcaaacagaaaataaagatcacttctctgaaaaagagcagcatgatatggagttagagcttgctgacattttaacttattgttactatatgtgcgataaacttggtgttgagccaaatgatattgttcaagaaaagttagatattaataaaaatcgtcactggaaattcgataaataggtaaagtgaggtgttagatcatggcagatgttgggtacccaatagttgaaaaaattccatataattctgacaccccagctactttggacgatgcaattcaaggggataagactaaacgcaaactgctgattgattatccaactatttatgtgatctattcacctgaaaaatccggtggctacaaggtttacgtcggtgaaaccaatgatattgaacgtcgaactgagcagcatcttaatgaagatccaaaggttcgaacggattggaaagaattgtctcgatcaaaaaatgctgagatatttgtgattgggcataatcactttaacaaatcgcttactttggatattgaaaatcaaatgatgttatatatgcttggagttccaagtgtcaaacgacttaataaccggcgggaaaacgaacaaaatgaatattatacttctaatgaaaaagaacaaatcttttctcgaatttgggggaagcttaggaagtataataatgacctgtttccagtggaaagtgtcattcgagattcggcaatttttaaggcatcaccgtttcataatttaactgctgagcagaagaatgcccgtgatgtcattattgataggataattgatgctcttctcgctaagaagaccggacaactcatcttggtagaaggtgaagctggttcgggtaagacggttctgttaagcacgatcttttatttgattggcaccctgactgatgatgggtctccgcttagacgaggatttgataatcttaataattacattttagtgaatcacgatgagcaactaaaagtatacgaagatattacccgtaagcttgaccttaaccacaaaaacaaggatatggtcagcaagccaacccggttcattaataatcacagcgaagacagtttagccgacgtagttttagttgacgaggctcacttgttatggacacagggaaagcaagcttatcgtgggcaaaaccagctggatgatattctgaaacgttcaagaataactgtagctatctttgataagaatcaaatgttgaaaactgaagaatatcttgaaactgaacagatcgccaaaatagaagacaaagctcggaaacaaaacaatttaattatgctgagtaatcagttaagaattcatgctaatgctaaaacaattgaatggattagaaacattacggataagaagatcattcagagaattccaaaagataagaactatgatttacgaatatttgatgatgctcaagagatgtatgaagcgattagggacaaagcaaaagatgagcagtatggtctatccagagtcttggcgacgtttgattggaaatataacagtaagcggaaaccggataatggtgattattggatggtaactgctggtgatttgtcgttaccttggaacttacagctaaagcccaagagcactcgttcaataaaacgattggcttgggctgaacaaccgcagacaattaacgaagttgggtcaacatatacgattcaaggatttgatctaaattatagtggtgtcattattggcccttctgtgaagtatcgcaatggtcacgttgtattcgaccctagcgagagtgaaaataccaacgcgattagaaatcgtaccttggaaaatggtaagaaagcgaaagtttctgacagattgttgccaaatgaattgaatgttttgctaactcgtggggttaatggactttatatttatgcggtggatgatgagttgagggatgttttactgaaatcacagtagaaggaaagtttactgtgagtgatcaataattcctttttgttatgatatgtataattgaatttgagattttattcatttgaagttatgctattataataagtaaccaaaagcttattgattggagatattcattatgggggaaaacgaagaaaaagaaattgaaattctggatattccagatacggtagattgtaaaattaattcgaacgctgttcgggcaaaaaagatcagcttcctttaaaatggtgtttaccacaaacccatcttttaggagctgatcttttgtctagtataacctattccgaacgaattaaaatcgaaaccttttgtgaactagggctgtccaatatccaaatgggcgttcggctgaaccgatcaccgtcaacaatttcttatgaattatctcgatgtcaaccttatcaggctgaattagcacaaacagatgccgaatacaagcgatcacgatgtggtcggaaaactaagctgagcgatgagttaaagcaaaaaattctcaaccatttacgtctaagctggtcaccaggaatgattgctcacgaatttaaactagctactaaatctatttataattggctaaatcaggggagaattggtttctccttgaatgatctacctgaacatggcgtacgccaacggcgtaacgttgaccaacgatccaaatataatcaatctttggggcgatcaattgaacagcgtcccatgatgattaatcaacgtaagcgcatcggcgattttgaactagatacagtcgttggtcctcgtgggcatagtaaggcagttttattaactttaatcgatcgaaaatcacggttcctttgggcataccggttaaaagatcggacgacagcgactgttaatgaagcactaactaagttcctaaccacttttaatggtccggtgcacagctttactgtggaccgtggcactgagtttagtgggctagtatcacttgaatcacaatatggtattaagacctattactgccatgcttatactccagctgaacgtggtagtaatgaacgctttaatcggaatttacgttatttttatcctaaagggactcgttttgagcacattagtgctcaagatttaacgacgacgttactccaaattaaccagcgaccgcttaaaatactcgactggccaacaccgtatcaggttatgctgacaaatttgtccaaaaattcggattaaatttgcaatctaccactaacagattaatttttcaccaagctaatgactttcactagctgatttttcagccacgagattagctagactatccaaaattggacacccccttatttaatcaaattccgaaaacctgaaatacaattcgtttaataattaatcaacagctatgatataatgaagttgtcaaataattaacatcaatctaagcaaccggaagcggtgcaaagaggtcactggaaacagtgatttttttgttgcctgtaatgaagcgctgcatccctttatggtataaagcacctcacaattagggatgattcatagattacaattaattatgaacgtgtcgaatattattaaatacatttatgatcaacgggtctcttttcgtagattgcccatctgcttgaacgaggtgaactatattcacctagtaatttattgaaggtttggttttactggaaaataagtagaactaagaccattagattaccgactgtagttaattaacgttgaaatgtagcacaacagttggttaatgcctccgcgaagccagtttaaatgctttgatggtgtactcactagtgtttagttcatggtgctggttattattagtgagattgttaccagttacataagcatagctgtatcgacagcggtaatgtacatatttgtacgaaacggataaagcaaaaattttcaatttaatcatcccggacgttttagacatttttgacaaaaacgccaaccaaacgcttggttatgcgaatcatagacttatttaaaaacaataaatggtggaaaaaggtggaatcttgcgttaataaagttaggtgccgaagttatgcaacgttttagactcagaataactaagatttcctaggcttttactcgtttgttgactagcatatacgatagcaaaagcttatttaacaagcgatttcaccttgcacctaattatgaggttgcgccccttttgtgtgcactctaaaatgaaaaagggtgcaccacgttgcaaggataaatgacgccacaagctaggcattgcaagcgtttatgatgacattaaccaatgaaaggatattgagagaattgttgagatttcttagggccttggtgcaacgaatgttggctaatgttgacgttggaatgagattagtaaaaggtggtcagtgcccgtactcatccattttaaaaattggatatttcccataatctaaacactagggatgctagtcattgctagtgtttgcgaagatacgttgtcgggagtgatccgcttttttgcttcaattcttggacatcgatagaggatgatacactgaacaacattatctgcttagaaaaagaaatatcccgacatttacgacaccctaaaaaagaaaaaaagccccgatttctcggcgctcacaattccattagtgatgttttacattctttctaagaataacagcttcccttctattatcaaggcaccttagccatacactaaaatgaccgctcgttaatgactgctaacttttcagcgtaaacaactaaaagttaagaattggcaaggttttggctaggtaaaagctttagtagaagtgctgaaccaagtcgaaatattcgacctacttagtgattgcatttgggctattgattatcagatcggtaactactaatgggatgattgccgatatttttgtgtgcaatattaaggattacttttatcgttgataaatgtgtacgaaaccccttgatgcataaagcatagagacgattaaaaactgataaaaataatggaaaatactggaattcgtttcgattaagttaggtaccaaaaaaggccaccgttgctggtgaccagatttgaacttaattataacaatcactaaggttttgttcttaatgttatttgaaggacaattccttcacgcttgtattatagcatgtcaaaacatgacatttaattaggttatgaaacatagcaaattaacttgctgaaaatgcaacaccttatcaattagtccaattttaaaagtaggttaatccgttggcacacaaatgattgcggcttttgctcgtttaattatcggacaccatataggagttaaggggcaatgatttacgcctaagagaaattccatagtatgctatgaaaagcgttactaaattagaatattgtttgtatggaaaagtcagttataagacaatccccttactagccaagttatctaaacattctttcaaatacgcatcgttatgttctgggtaaacgggactggttaaagggcactttttcaagtttgcatatggttcacattgcaaacctcgataaagaggattaaaccatttccgatcaggcttatagcctcttcgtaacatttcatgcattaccagcaaatgaaattgataaagtttatacggtgagtggttgaatacatagttcacggttgcgtgctttttaccccaaccatttcccctaagagcagcaatctctctatgttgacctaataactgctgacgggggagtttacagataagttgttcgtgccaaagtcgcataattacccccctaaatttctttaatgattcttgattcaagtaaataagttatttgatacttaatggctaattgctttaaaaataggccgagttgatcattatttggcgttaaggtaaccagcaatttaagataagtattcttttcgtcatcggtacaaatttttttaaaatatccccaaacgtgttgataggcggttactagtgttgctcttgtgggctttgtgttagcagcctcctcaaggattcttttaaagatgagatctttttctggtgtccactgattatcttttgccatttcacgcactttattataaagttgttgagatcgagccataatccaatatttattgtaagcccatacacgttgccactcttccattattaacctcctactttagattatctttccatatggataacttccactgacaccaatcaataaagtctttttcagtgatgtgtttgatattaggaatgtccaatttacgagtggttaatggttcattgatggtcttatgaatagcgccaactattaagtaatctgtttgtttgttaatctgtgcttttgggaacgcgccaaaagcactagcaacagcaaatgcttgcttacgtggcatactagctaatttacctgtaaaaacaatttccatatccgttagatcgatcattaaacatccctcaattaaaataaaaataataggataacattaggtggaaaaaattgacgttaatttatgattttggcatactaaccataattggcgcaaagaactaagtttatttgaaaaggttgaagtcatgataatttggtttacagtggttttactttttctcttttgggtatttatccataacagaaataaatgatatgtaatagaataaaaaataacatccctgatcaaagggatgtagaccaattcatggctggcgcattagatatattaaaatatgtttcgtgcttaccaaaatgcttaccattgattacgtctaaatcgaattgaatcgaagtggtaaaaagtaaaaaaacagcaaccacggcgttttaaggctgcatggctactgtttaaattgcgttagtgggcagtcaggggctcgaaccctggacccacggattaagagtccgttgctctaccaactgagctaactgcccattactaaccgacttaaatataatagcatatgctcaaaatatttgcaacacggaaaaggggatttatttgaccaatatcggtctgtgttataatagcaacatgttggcgtgtgcaaattttagaaaataacaatattaaaatccatgttaggagaaattgttaatggcaaaaaagatactggttgtcgatgacgaaaaaccaatcgtcgacattgaaaaatttaatttaactaaagaaggctacgaagtctcagtagcttatgatggtgaagaagcattgcagcaagtcaaagacgttgatccggatttaattatcttggatctgatgttacccaaagttgatggcctggaagttgccagggaagtccgtaagactaaggacaccccaatcattatggtgactgccaaagattccgagttggataaggttcttggcttggagcttggggctgatgattatgtgaccaagccattctcgaaccgagaattagtcgcccgtgtgaaggctaacctacgccgtcaggggaccaatagcagttccaataacgaagaagacgaaaataaagatatcaagatcggtgatttggtgattcatccggaagcttactcagtttccaaacggggtgaaaatattgaattgacccaccgtgaatttgaattgttgcattatttggcccaacacattggccaagtcatgacccgggagcatttactgcagaccgtttggggctatgattattttggtgacgtgagaaccgttgatgtcactgtccggcgtctccgtgaaaaagttgaggacagccccagtcatccaacctggctggtaacccgtcgtggggtaggttattacctgcgcaacccagaaagtgatcaagcataatctcaatgaaatcaatgcataaggggtattaactggttgtgaataatcgaattaaattttaccaatcaatcaaatttaagatcgcactggttttcgccctgatcctcctggtaacgctggaaatcgttggtgcggtctttgttaggcagctggagcatcaaaatttggcgacctttaagaaccaaattcaactgcagacttatgtcaccaattcattgacgacccaattgtcaagtgccgatgaaacaaaagccaacggccggatcaagaccatcttgaatgattccgacagcggcaataccgcgcaaattcaagtcattgataataaagggacaattcgcggtaccaatcagattaacaaccaggcgatcgttggccaaaagaccaccgatgataacgtcaagaacgcaatttacaacgggaaaaaatttgaaaagataacctatgattcttcaactggtgcgcgttattacaccatgatttcaccgttgattaagagctccaacaataatagtacggtcgtcggggtggtatacacccgggcgaacctcgacagcgtctatgacagtattaacagcattacgctgatttatctgttcgccgcgtcgattgccattattttggggttattaatctcgattgttatttcgcgagcaattacacgaccgattgaagaaatgaagaagcagaccatcagaattgcccgtggggactattccggccaagttcacgtttatggaaatgatgagctgggtcaacttgccagtgcggttaacaacctatctgtcagggttgaagagtcccatgagtcaactgagtctgaacggcgacgcttggattcggtcctggcaaatatgaccgatggtgttttggcgaccgatcggcgtggaaacgtgattatcattaatgaaacggccgccagtttcttggatcttgatgaaaaccaagccatgggcaagtcgattttggacgtgttggatattcgcaaagactacagtctgcgggacttgcttgaaaaaccggatgagttaatccttgatttttcaagtgaagatcacagtctggttttgcacgcccatttttcactgattcaacgggaatccggcttcattagcgggctggtctgcgtgcttcgtgatatcaccgagcagcagcgaatcgatcaagatcgtaaacagttcgtgtccaacgtttctcatgaattgcgaaccccattgaccagtgttcgttcatacattgaagcgctgtctgatggtgcctggaaggatccgaagctggcaccgaagttcttgaaagtcactcaagatgaaaccgatcgaatgattcgtatgattaacgacctgttaacattgtcacggatggattccgggacgcagaagatggaagtggaattggtcaatatcaatgaattgttcaattatgttttgaaccgatttgacatgattcttaaaaaagaagatcatccagaaaagacctatacgatcaaacgctactttaccaagcgggatctgtgggttgacctggacaccgaccgctttacccaagtattggataatttgatgaataacgccatcaaatattcaccggatggcggcgtgattacgtgccggctctatgaaaccagaaataaggtcatcttaagtgtcagcgatcaaggattgggaattccgcgaaaggatattccgcatatctttgaccggttctatagagttgataaggcccgttcccgtcagcaaggcggtagcggattgggcttggcgatttccaaggaaactgtcgaggccttgcatggccaaatttgggccgagagtgtggaaggcaagggatcaacattctatattgctttgccatacgaaccggtagaagaggaggacttgtgggatgaggtttagtaaatacttaataccccttgcactcaccattgcggtggttgccagtctaacgctctcggtggttctctggaccaatccggctaattatcggaccaataagcaaacggcgcaaagcccgcagacgcagcagatgattaagcccaaacggtacgtctactcaccggttcaggcaattcatacgaatgcggacgggacccaacagattatggtcaacaagttagtgaacaccgtgactgagattaagaaaacgatgcatcattatcaaaatccgcggatgaaaactttaagcaaaaattcgcaagttgactattttcgaatcgctaaccagactgattcgattatgctgaactattcagacacggtttcgatgcggacatttaacgcaattgtcagcaatcgattccggaagctgccgaacatcaaaattaaccgagttgtcttgccaaccaacaattcaactaaactgtatcttctctatgataaaaatttcactgtgtatgaagtcgatgttaaaaaacacagtttaaaatctttgaacaaggttctgcagatggacatgcggacgcaaccggccagcttcaagttattaaataatcggccgatcgtatacgttaccagctccgtgcagatgcagccttataagtatttgattgaccgtcaatctgacgattactatgttagccgactgctgaatactcaggattcaaccagcattaacgttaagcggcgaaagaatatgacgatctacggtgatcaaagttcgctgcaattaacgtttaactccagaaaccggatggcggaattttctgactttcggccaaatcataaccgccgcagtttgacgtcaacgattaacgattcctacaagaacatcactaagttagggctgccaatggataacgtccgtttcttcagctatgatccaaagagccggacggtgatgtatcggacctatgttgaaggttttccgatttttcgagccagtggctttgggaccgtctcgacgcggacactgaactccagtgctcagcggatccaattttcattggataatcctgaggtgccgctgccaagtaacaagggctacgtttcgctgccgtcaactgaaacaatgctgaagcggctggtcaatcgtgggtacaatttaaaggatcttcagaaagtccgtctgggttatacttggaagaaggattctacatctccattattgattgacctgaatccagattggtacatctattataaaaatcaatggcgctcttacactgcacttatgaaccaatattaggaaaggagggagcctggtgaactttcgaagaattgagatcatctttttagtgacctttatcgcaatcgacattttcttgtttgggatgttcaaaaagaacatggacatgcaggccgacaacgtgtcccaaggcgactcggattcagtgatcgtcagggaaatgcgtaacgaccagattaaagttggcaacttgtccaagaagaacgaaactgcctattacatttctggtgaacaaagcgacgttttgcgtaaccagatgggacaattggttaaccagactccccaatttgttggtcatgagctggaaagtgaacttaagcagccaatcacggttgataagaataatccacgcaaatcaattgataaattgttaaccgattccacgtttgtgttgtttggtgaccagtacgtttacagcaaaaacctttcaaccagtcggaatatcgtttacaatcaaaaggcgatgggaagttcgatttactcctctgaagcccagatcagatttacgctgaattccaattatcagattgtcagttacactcagtcttatctgcagggaatcaagagcctgcgcgaaagttcggaaaccatttcggaaacccgggcgttaatttggttgtatcagtataatgagattccgaataacaccacggttgcatgggcaagtctcgggtacaccaagttattgtcaatcgatggcgatcgagtctttattccaacttggattatcgcaattagacctcaaaattctacccaagttcagttgaaacggatcaacgcgtttacgggtggcattatcaaacaaactgatgagaatttaaagaatagtcaaacatcaatgaattaaagttaggaagaagaacggttatgaataatgatgatatgaaaatcagcgtcctcgccagcggtagtggcggtaacgtgacttacatcgaaacgccggaccacaaagttttgtgtgatgcgggattgagcggcaagaagattgaagcgctcatgaattcgattggtcgagacctcagtgacgtcgactcactttttgtgacccatgagcactccgatcaccgactgggtgccggtgtcttggcacgcaaatatgggattcaggtgtatgccaatgaaggcacctggaatgctatggcgccaaggattggtaaggtcgcagacgatcaaaagaacatcattgctcctgacagtgtgatggatatgggcgatcttgatgttgaaagcttttcggtgtcccacgacgctgctgagccacaattctatgtttttcatcataataacaagtcttttgttatcctaactgataccggttatgtttctgatcgcatggaaggcgtcatcaaagatgccgatggttatcttttggaatgtaaccatgatattgaaatgctggaaaatggcgattatccttggatgaccaaaaagcggattttgggtgatcaaggacatttgtccaatgaagatggcgccaacaccatgttggatgtcatcggtcatcggactaaaaaagtcttcttaggtcatcgcagcctgcataataacatgaagacgcttgcccacttgacggtggcttccatcttggaagaccacgatatgggtgtcggtgaggactttaagctgtacgatacctcacaggaccacgcttcgcctttaatgattatttaaaaatcctttagatatttctaaactttaaaacacactttcgtcatgaaaaaagtatattataggtaatataaaataataagggggcacactaattggcacaaaataacggatttggaaaattcattgcgaccgctgtgatcgctggcgcacttggcggcgggattacttacggcggagtttcttattttaacaacaataataatggaactggaacagagctggtttctggtacgaacaagaatggcaataccaaggtcagcaacgtaaaagttaatctcaatactcaggcagaaaaagcgtttaacgcaactaagagcactgttgtttccgttattaatttacagaaacaaagttcaagcgacgacaccttatctggaattttgggtcaaattcaaggcggttcttccagcaaaaagaagagcagcggcgaacttgaagcctcaagcgaaggatccggtgtgatctataagaagagcggcaatactgcttacatcgttaccaacaaccacgtggttgccggtgccaatgccctcgagattattctcagcgatggctcgaaggtttccgcttcggttgtcggtaaggatgccgtttctgatttggccgttatcaagattaactctgacaaggtcaagaaagtcgcaacttttggcgactctgataacatcaaggttgccgaaccggttctcgcaatcggttcaccactgggctcacagtacgcaacttcagtaactcagggaattatttccgctaagaaacgggaagtaccgcaaacttcagagagtggccaacaaattggtaacgcaacggttattcaaactgatgctgcgatcaaccccgggaactccggtgggccattgattaactttgccggccaagtggtcgggatcaattccatgaaattagcttctgatcagcagggtaccagtgttgaaggaatgggctttgcgatcccaagtaatgaagtggttatgattatcaaccagttgatcaagaacggccaagttatccgtccggcactgggaatcggctacaccgatctatccaacatttccgagcagcagcaacgctctattttgaagctgcctaagagtgttactcaaggggcggttgttcttaacgtgaacgctaattcacctgctaagcgggctggattggccaaatacgatgtgattaccgagctggatggcactaagattactcaacaaagtcaattgcgtgatattctgtataagcacaagattggcgataagatctcagttacctattatcataaaggtgacaagaagactggctcaattactttgaacgaaaaagcaaccagtaaagttttaagcgaagcaagtaaataatccttaattataagtattgataacctccgttttctcataagcggaggttattttttgccttaaaatgaattgtcggtcgttacttacttaacataagtgtaatacttaacattcatgtaatgttaataaattcacatttgagatacaataatgatgtagcacaaattgatcaaaggggatatcgacatgaaaattcatattaagggatcaatcctggtttccatggctgctctgggagtctttgctgtagttgggatatcgcagtcttcagctgtttcagcaaaatctcgggtccgggttacgtcgaacgtgaaattgaggggtaccggagcttcgcgcaacgtgacctttaccggtaaagcggcattgtggaccaaggcttcagcactaaaaggagccaagaaggtcgcaaccaccattacgttacgggatcttgccaaatcaacccgatcaagcaagaacgttcgcgcttatcgggttgccagaaccaaccggggaaaagtgtattataaggtggttacttttgacggtaaggatcgcggttggatttatggtggtaagagtcggtcaagctttgctggcggggtgaaatcctatctgacgttccaacagaactcgctcactgatgatatgagcaacgggacgttccaattcgcaaacccgggaaccgcaaacaataatcagacagttacatatgagcagccagcttggacgcaatacaaggttggccgtcaggtaactgattcaagaccttatgcaaatgtcagttaccaaattgaccaagctgggatgagaacccgtgaaggtgaccaatgggttcacatttctgccaccaataatggtaactccggcgcggatggctggattttgtattcaggattgaagaagacaaccaacatcaattcaccaattgctgataacgcgattcgaattaagttagttgattcggcgacaggttcgtcattgacctcggttgatttcacgaagactggggtaactaaaggcgcaacagtcggctccaatgtgaatggcacttggaagctggattccaatgattccagttcaattcagtcacagattgcctctgcactttcaccactcggttatccgggattcaccttgactcaaggccagatcgcggccattgcccagggaacctttggatccagcgtgacgatttcagttgtgaaaccaacgattaacaaggcagttcggattgttttgacagatccgagcggaaacgtgattaattatgttgattacacgactgctaacgctgccaatggtcaaccggtgggtgtgcaggatggctcaacttggaaattggcggcaaccgatacggctgctattcaagctaagttagttgatgcgttaaagggtaccggttttgcattaagcgccaacaacacattgaccactgaccaacaagctcaaattgctcaaacgacattcggtaaccaggtttccattaagaccgttgccgttgacccaatcaaagacaatgaagttcaattgtcgtttgttgatcaggccggtaaggctgttggttcaacaaccttgacgaaaggcacaaatgacaaaacggctttggacacgattaagactgttagtgttgctgacccaacgtcacctgatgctgctaccttgaagaaggcttatgctgctcttttggccaaggctggtattaagggctacaccactgatggtttgagcaaggatcaacttgctgcgaacttagctgccattaaagcggctgcatatggtcaggatgttaagttggttgtcgctaagctgccagcgaaggcattggtttccagtgcactgttctttgataaatctgataccaaggacgtaactcaggatcttgcatactttgaaaatgcaaacggtaaacgtgatagtgacgcaaactttagcaaagcattggctggagacgcgaatatcaatggttatgccggcgatgtggttacggttgcaaacctcaatgctgctgttaaggatcagggattgaatacaatttactacgcagcaaagaatgacggtttcctctggggagctggaactcatttagcggctagtgactacagtggaacgaatggaacgttatttgcagacggtatgagtggtaagacaatttatgtattcaaattaacctttaccgctaaacctgataatcctgatacgtcgattggtaacagactagattctaataagcctctattcgacaagcaggggaatgcaactattggtgatacaggcaatcaagtggtactgaagtatgatgaagtcaaggctggtaaacagattacccttgatagcaacaatatgaaagccaaaacactcgcagagttgtttggtgaataagcacaaaagttgatcagaggacttcaattctcaagttgggattgaagttcttttgtgtctgtagccacatggcttcttatttaagagccctaagtggaacacagaggataacaccctcctccgtctgaaacacgtgataagactcatatttagggctaatatccccagggatcggcaacgcccattccccatcgtgattaatcaagttgactgtcaatggtgattctccaatctttaaagtggatttgtttgggacaattcaggtatgatgattaaattgattcgatttgtccgcaaacattggaccgcttcactgtttacgaacggccttgccaaatatatggaacttgtaccgtacacatggtataaatacgaacgacgaaccaagttttatttaaaaaattcatcggatgtaaagatttgataaactatccacattttggctgtggataactctgtggacaatccacaagattctgttatccactgatagaataacgttgaatagttatcccccaaaaactaaaagttatccacagaaattgtggataactttttttgatataaaaaggggatttgttcgttgagataatgactgatataatagggcttgcggtgacagattgcgaacacacgttgtccacagttctgtggataacatttttgacccttgacaatttttaaaataatgcgggtcactgaaaagttgataaggtgcataaacctgtggataactctgtggacaacttgttaataagcccgcttttttacacaggataactataaatttggaggcaattacatagtgaacattaaattggtcgttgttggaaaattaaaagaaaagtattttaagcaggggattgcggaatacgcgaagcggttatcgcgcttttgcaagtttcagattgtggaagttcccgatgagaaggcgccagagtcactcagccaagcagaaatggatgaagtgatggacaaagagggtgcgcgaattctggacaaaataaaggaccgcgagtacgtgtacgcactcgcgatcctaggcaaggagcggacttcagaagcgtttgcgaaggaaattgccgacctgacaacctatggtcattcggacatcacctttgttattggcggatcacttgggttatcgaaacacgttctcgatcgtgccgacacccagatttcctttggccggttcacattgccccaccaattgatgaggttggtgttgactgagcagatttaccgggcttttatgattaatgagggcagcccttatcataagtgaccgcccattactgcgcaaatcaaaaccagctggtaaccctatttgggaataccagctggtttttttatcgttatgatgttatcagattcagagttgcagtaacttttccgcattcccatgcgcaaacaattccttctcctcatccgttagaggactgctctcaatgaaactgccagaattttccggtttgatataagggtaatcaatcgagtacagcaaatgctcaatccccacttcgtccttcacgaatttcaattgcggttcggtcaaaataccgcttggggtgacatacacgtgatcgcgataaatctttgaaatgggttcgctgaggttggtttccggatacatgacctgatccattcgctcaagggcaaacgaggcaaactcgccccagtgaccggagatcaatttcagattcgggtacttttcgaaaacgccacttaatagtagtctgacggtctggataccgacatcggtatgccaaccatagcctgcagttcccaaaataccggaaaccttgtcatcccacggaccgttagagtaatagtagtcgataatctgtgaatctgggaatgagggatgcagatagactggcacattgaggttggctgccgcctcaaaaatgggtaggtagaatggatcatcaaagaatggatgagcctgagaagttggtctcactagcatggcccccttgaagccgagctcttcgacaccgcgtttcagttctgccgcagcgtcagtgggatgggaaaccgggagcgatgcaaaggcacggaagcgatcgggggctttcgcaacagcttttgccagctcatcattcgccaactttgtcagttcaaccgcaaacttcggatctgaattttgcgggttctgattgccgtatgacaggatttgcattgaaatctggtgttgatccatccattgaatccgactgccggtgacgtcttccaattctgcctcgggtggtagtgagcgctgcatataatcctgcatcttcggactgacgtttccgattggtcgttttggtaagacctcggccattttctgacccaacttttgtgatgaaaaatgttcttctaatgtaatgactttcatgtgatgtctgcctccttagcttagcagcttacccttcttcaaaaagcggttgttcaagaaccagtaatgcttcgggtcccccagcaatgcagtataaggaaccggtgtgccgcctttttcaatgattttctcatccaggtacgctttgagaatccaaggttcctccaaccgggtggggttcaagtccaaaatgtcttgaacatgttccggcgtggtatccagatcttgagccacttgttcgatggggacttctgctagtttgaagttggcgttaatttgctgcttggtgtcgatttcttgttgtggtgtgagtgacatgtgattactcctttagttgttgataaatttgagtgagctggtcataaatcgcatccggtgcaagtaaagctgcatcgactttctcatcgaggacgtcgaacgcacccttgaccgccgtgacggtctctttgccgtttggagtcagggtcagctgtttttcgcggtcattatccggattgaattttttctcgatcaagtttctggtttccagtccttttaacaaattggaaacactggcagcgctgcgtcctaaaataattgtgattgcccgctgatttgtccccgggtgatcgccaatgtaccgcagcgtgtgggcttgatcgacatttaaattgagttcgcgcaactgctgattaatcaagccttcttccagcttggcaatttgatgaatgagcgatgatactgaatttcgatctttcaaaacatgacctcctcacttagatttatagtctaccaccaatagttgtaaatgcaactgttttaaccaaaactatgtattaaaaaatcccccctttgattgggaggaattcagattgtttgtttaattaaccgattgaattgatttcccagctaaaaagtccaaaatgttattggcacaaatctcagccattgaatcacgcgcctcaacggttgcgttgccgatatgcggcgtcaagatgacgttattcattgacttcagtccaggggtaacggttggttcgtgctcatagacatccaaagccgcaccggcgatctcatggttctctagtgccgatgccagagccgcttcgtcaacaattgggccacgggcggcgttgattaagaacgccgatgacttcatttgcttgaaggctttggcgtcaagttgatggtgattttcttcggtcagtggtgcatggaccgtgataaaatcactagtttgaagcagatcggtgaattcagcaaaccggatgtttaatcgattttcctcatctcgtggtaatctaaattgttctggctgccagtattgaacgttcattgaaaaggcttgcgctttcttggcaacatcccggccaatgtggcccattccaatcacacccaatgtttttcccgccagttcatggcctagaaaaaatagtggagaccatcccgaaaatccttggttgtgcatcaaacggtcgccctcgacaatccgatggctgatggctagaattaagccgagggtcacttctgccaccgaatttgttgaaacaaccggtgtgttggtcaccaagatgtggtgggtactagcggctttagtgtcgatattattgaaaccagcgccaaagttggcaattaattttaacttggttgctgcgctgatgattgattcgtcgaccttggtggataatgttgtaatcagaaaatcactatctttcacggcattctccaactcttcgtgagtgattaagccctgctcactgtcgtgaatggtaacggatagaccagcactttgtaatttcttaacagctttacttggaatttgatcagcgataaatacttttgtcatgattatcctcctcatatatttaatctaactacatcatgtggctaggttgaacaacctgcaataccgcacttttttgtaactgatggaaggagttggttcaaatgactgatagcgtaagagaagcagtccaagaaaaattagcgaacggcattttcaactgtcccaaggaattaactttgtcgatgattagcggcaagtggaaaattaacatcctgtatcatcttgggacagatggaccctattatttctatgagcttcaaaaattattgcctgcagcctcaagaaaagagattacggcaaagctcaaagaattagtcgaagatggcttggtcaatcgcaagccactgaagactgttccggtcaaggttcaatattcaattaccccgctgggaaaatcattgatgccgattattgacgccatgttgaaatggggccaacaaaggctcgacgacttgcagttggggcaggttgaatttggcttgggtaaagtcaaacatgaatgattgttcatttttcaaaatgcaaactccaaaatagacctaatcacgatcactcgttatactaatgattgcaattagtaaaacataatggtatacgcgaatattttggaggtgtcaattatgaacaataatagtcaaaagccagccaagccatggtataagaaatggtgggtttgggtattggtcgtttttggattggtgattgcagtcaatgcagtttccggtgaagaagacgattctgccagtaaccagtcaactactacagcgactcaggacagttcttccagtaatagcgatgggacgcttaaaagcaattacaatgtcggtgaagtggccaactataaagggtataaattcaagatcaataaagtgacgttctataatggcaacgaatttgatacgcccaaggatggtaatcggtatgtgatctgtaatgtaaccattaagaatgatactgatgagaagcagccatataattcatttgacttcaaattaaatgctaatgggaactccaccaacatgatggaagtcgtgacgaatgaaaaatatactaacaatacgttaaacagtggcgacctggatcccggcgcgagtgtaaccggtaacctgattggtcaggcaaaacgggatgccgacttgaagttggaatatcagccgtcaatctgggatgataagaccgtcaaagtcgatatcaacgaatcagcgtaagttatggggcatttctttcactccacttgctcaatcatatacaataatggtgtaagcgttttatgaataaaagggaggctttttcatgacagatcgtctaaagaataaggtcgcaattgtcaccggtgccggatcaggtatgggggctgcaatggccaagttgtttactgctgagggcgccagcgttgtcgccgctgatttgaataaagatcgggttgacaaagtggttgctgcgatcaccaaaaatggcggcaaagcagtctcaatcaagacagatgtttccaacgaagacgatattcaggcaatgtttaagttggcaaaaagtgaatttggtcaactcgatattgttgtcaataatgccggcatcatggacaatatggcgccggttggcaatttgactgatgacatgtggaagaaagtctttgccgttaacactgacagcgtcatgtactcgactcgtgaagcaatcaaggaattcctgccgaagaagcagggcgtcattttgaacattgcgtcagttggtggaacgaatggcggccgtgccggagttgcatacacggcctcaaaacacgcggttgttggtttaaccaagaatacggcttacatgtaccaaaatgacggcattcgagtcaatgcgattgcccccggtggcatcaagacaaatattgctgagtcaatgggcaagaatgttgataaatttggttatgagcgtcaatcccaagggatgggtgcatcacctgaacccggaactgcagccgaaatcgcaaacaccgctttgttcctggtttccgatgaggctcgttatgtaaatggtgctgtcttgccggtagatggcggttggactgcctactaaaattaaataagtttgaaccgtggaagtgattccgcggtttttgtttgccatgaagtgcactccagggtatagggtagaaacattatataaatagaaagaggctaccatgacaaaatcattgattatttatttttcactgtcaggcacaaccaaaaccgcagcggaaaccattcaaaaatatacccattcagacatcatcagactggaacccaagacaccatatccagctggttacgacaagtactccaaagttggtatgcagcaaatgcgagacaaagcagatgttgccatcaaaactgcaatacccgatctacaccaatacgattatatttttgttggctatccgacttgggatggacaggtgccgcggatcttcaacactttgtttatggaaaatgatttctccggcaatcgcgtggtgccattttcgactagcgtgtcgacgccgtttgaggatacccttggttcgttgaaggcggccgttggagacggggttgcgattgttggtgggtttaggtattccggggaggcacaagtaagggattatttaaaggataataattttaaataggcttattttttgatactatgaagacattggttagcacactaacactttggaggtatcaaaatggctaaatttgaatccagcattttgtcgattcctgattatgtacccgcagatatcattcgaattagaaaacttgtttcagctgataagaccaaaatggcattgttcatgaatgtctcattgcggacttacaaaaaatgggaaaccggtcaaagtcatccaagcaaacccgctcgccgtttactgcagatacttgagaagaatccccaattaattgataattggttttaaatcagcatttgatgaccatgtatagaagaataatagctgaaggagtcgcgaaaaaacgcggctctttttcatattctcacatcgccacgttgcatactgaatattcatgcataatatcaccatatattgacataaagtttaaaaggtttatgattgagtatattaaaattcaatgaggaaacggggaaacattatgagtatttctgttattaaacgatcgttattatcgcttggtattctagcaacaacagtcttgctggcggcatgtggctccaagagctccgatcaagggtcgactaagctggcatcaaatcaaaagatcagcttatccacgacagctgagattaccagcttggatttgtcaaaaatctatgataaaacgtcatttattcaaattgatgaaacttttgaaggcttgtatcgttatgatgcaaacggaaatgtggaacctgcgctggcaaccaagacaaaaatttctaaagatggaaaaacatacacgattaacattcgtcacaatgccaagtggagtaatggcgatcctgtgaccgcaaaagattttgtctattcttggcaacgggcggtcaatcctaaaacggccagtcaatacacttacctttttgataatgtgaaaaatgccgatgcaattgtgaacggtaaactttcaccgaataagttaggtgtgaaagcaaatggaaaatatcaactaaaagttcaactcgctcgtccaacgacctacttcaaaatggtaatggcgcgtgagacgctttacccgcttgatcaaaaagttgtcgaaaaatacggtaagaagtacggcacatccgctaaatacaccgtgtacaacggcccattcaaaaacgttggctggactggaaccaatgactcctggaagctggttaaaaataatcagtattgggataaaaaagcagtcaaactttctcagatcaattacacagttgccaaatcgccaagcacagcatataacctgtttcaatctggcaaacttgatttaatcagtcttgttggtgaacaagccaaacaacttgggaagagtaaagatgctgttaaacggccactagccgcaacagagtatctgcaatacaaccaacgtaaaggcgtcttcaagaatcgtaacttacggttggctttctctttagctttgaatcgaagtcaattaattaacaaagtgatgcaaaatggatcaattgtttcgaaaggatttgtgccggccgatttcgctaagaatcctaaaaccggtgaggattttgccaaagaagcgtatgttcctggaacagttgatcatgatgcggctaaggcaaagcaatactacaaaaaggccttatcacaattgggtaagaagaatttaactatcaagctcttgtcggccgatgatgatcaaaccaaagatgtcattgagtttattcaaagtgagcttcaagaaacgttaccaggtctcaaggttgaatcaagcagtattccatttgcctcgatgcttgcaagagcttcagctggaaactttgaagttaactttacgggttggtccgctgattttgctgacccaatttcatttctttcccaatttacatcaaacaacccagaaaataatggcaagtggagcagtcaagcatttgatcaagccattaaagattccaataacaaggatgcgaataatgccaccaagagatggcaagatttaatcaatgctgaaaagattttggccactgatcaaggaattacgccgatttatcaagccaatgggattgacctggttaaccctaagttgaagggggttgtctatgatcgaattaatggacattatgactacagaacagcttatttaaccaaataatttgaaaaaggggtaatattttggataagaagtcagcactaaatttaattgaacatttatccaatgcaaatggaccaagtggctttgaggacgaagtaaaggattatgtcgttcaaacagcctccagctttagctcggttcacgcggatcacatgaacaacgtctatttgaaaaataatcaaaattcaccttccaaaggcaaaactttgatgctggattcacacttggatgccgtcggtttgattgttcaagccgtcaagccaaatggaaccattaaatttgttccgctcggtggttgggtacccgctaatttaactgcagaaaaaatgcggattcgaaaccaagacggagaatggatcaccggtttggttgccaccaagccaccgcatttcatgacagaggcagaaaagaaaaaaccaattgatattgccaatctagtgattgacgttggaacaaacagcgctgaagagaccaaagaggtcttgaagattgatacgggttgtcccatcgcacctgacactgagtgggagtacttcaaaactcaagatgtcatgatgggcaaggcgtttgataatcggattggtactgcatgcttgatgacggcaatgtctgacctggctgaggaaaacttggatgttaacttggttggtgcgattgcttcccaggaagaagtcggctgtcggggtgcgaaagtgactgttaaaaaggttcatccagatatcgcaatctgtcttgagggatgcccagctgatgacacgtttacgccagaatggctgatccaaaccgggttaaagcgtgggccgatgctgcgtgatatggatacttcctttattgctaatccgcattttcagcagttggctgtagatcaagcccaccagaacggtattccatttacccgtgctgttcggactggtggtggaattgatggttctgaattgcttgagttccaaggggcacccaccatttgtattgggattcctgttcgttatgaacatactaactatggatttgtggcatattctgacttcgaaaataccgttaaattactcaaggcaattattttgagcctcaatgataaggtcattgacggtctataaatcaaggagctggtatatttggataaacaatatgtaattggatttcccgcagagactcgaatcattaataatcttgcaagaaataccgtcaacgatgacgaggtcgctggtgtcatcaaacacggtggggtcccagtgctcattcccacccgcaatccagaaatcatggagcactacgttgacctgattgacggtttgctgctgccgggtggaccggatgttgcgccgaagttctatggtgaagagccggttcaaaatctcggcgacacagatgccttcttggacgccagcgaaatcgccttagtcaaattggcggttgccaaacgcaaaccaatttttgggatctgccggggcgtccaagtgctaaacgttgcccttggtggcaccctttatcaagatctgtatagccaacggaatcatccaaccctccaacattaccaaaaggcgccgatgccacaaggaacgcacaccatctccaccactccggactcctatttggcaaaaattatcggccagggtgactcgactttggttaatagccaccaccacgaggccgttaaggcggtttctggccaactcaatatttccgcattggcaaaggatggcgtgattgagggcgttgaaagccaagatgacgacttgatcattggtgttcaatggcatccagaagcaatgtttcggaccgatgagaagcaagacgcgttgtttgcggatttcatggcacgagtggaaaaattcgcaaaccagaaagctgtacatgattcggtttccactgagaatgaataacaaactaaaggatctttgataggccagcgccaactggtttatcaaagatcctttgttattcatagtgttcagttgttgaattgtacgttagcgtgactggctgattattgaggttaaccgtgattttccggtaaggttgaaaaccatggtgaacaaattcaacgctgacctgaccgtggtcaacgttcacgagataatcgttgaattcgccgtgctgatacttgaagtctaggccgttatcctgatagtgatgatagctgcccgaatccccatagacgttgaatgtcattgtcggatcaggcgtttcagaaatatgatcgacttcggctccccaaggcaaaatggttcctttcttgataaacatcgggagcttatctaacggtgcatcaacgacaatgtcttgttggccctcatattcccggtggttccaaaaatcaatccattttccagccggtagataaaccagtcgtttggtctgcgatggttggacgatcggtgcgactaagattgcatcgccaaccatatattgatcgttgatgtttcggactcgtgggtcatcttcataattcaaaaccagtggccgcatgagtggcagaccatttttagattctttggcaaataggtcgtatagataagggatgaatcggtagcgcagctttagaaatttacggtaaattgataacgtgggttcaccgaaggcccatggttcctgggcacgggttcccatcgcactgtggtttcgcagcagcggactgaagatggctgcctcaatccagcgggtcaaaagttccggcgttgcgtctgaaccaaagccggcaatatcggtgccggcaaaagtgaacccactgattcccagattacacagttggggaatcaggagttgtaggtgaggccaaatgctatgattgtcgccggtccagacagttgaatatttttgcgtacccgaataagcggcccgggtaatgacaaatggtcgtctatcggttgcgcgtttcaccccgtcataggtcgccttggccatgttgtggccgtagacgttatgcattttcttatgagtcgacggctggtcgtgatcgctgaaaacaatgtcttggggaatttctccttgaaatgaagcgggttcgttcatgtcgttccaaatcccagcaacccccatatcagtcagaaattgatcatttttgccccaccatttttgaacagcttggcggccaaaatctgggaagacggcattccccggccaaacttggttgacgtagacattgcccgccggatccttgacgaaataatcattcttgatgccttgatcataaatgttgtagccgggatccttcttgacgccgggatcgataatggcgacaatttttgtgccggtggctttcaaatccgttacaaacttctttgggttgccttgataagcctcgtcattccaagtgaacacccggtagccgcgcatataatcaatgtccaagtgaatcacgtcaaatggtaaatcgtatttgtgcatcgaatccacgatatcttggaccatcttctggctggcagagtaaccccagcgtgattgttggtatcccaatgtccatttttgcggcaaaggggttcggccggttaagtaggtataattggtaacgatatctttgagagttttaccgccaattaggtagtaattgaggttgccggcttcagctgagtagaaataatagttgggattttctttgccaaaatcaaaatggctccggtagggattgtcgaagaagaggccatagggatgcccagctttgaggccgatcatcactggaatcgatttgtacaatctggtgaaattctccaagtggggcgctggattatcggtattccagtcatcatactcatagccccgtttgttcagataaccggtcttgtctccgagcccgtagatctgttcatcaggtgccaaatccttcacaacttgaaagtagtcgggattattttgatcgtcggcaccgggaacgttgtggccctcttcttggacgaactttttatgttcctcgtcaatcccccgatcaagcggagtccgactgccacggtagtcagtgaccagtgggttgccgtgggcatcataggcatcgatgtgcatggccgcgtccaccttgatggtcaaggcagcggtcgtgatttcataatggtcaggctgttgcttaactgtgtatgtcgttgtggtttccttgtcgccttcaatcgcgtatgaggcaccatgatcaccgcgattttcggagacccgaatgatctctggggtgataatagtcaattgaatttgacgatttgaattgttaaatgtaatggtttgatgatctgtttgataggtcggtaacttgggcaagtctgtcagtcctttcgtttagattatcgtagcatacgtcccctaagagatacaatactgttcgaaaagaccagcccgcctgatttggtgagctggtcttggttctcaatgatggtcgtcatcatgatcatggaggccaatataataaccgtccatataaccggagtcgtagttgtcttcgtcacttcggacatagccgccgccaagcggagtgttccaatgatcaatgatccagacgacaaatataatgaaacccgcgagcattaccagagcagattttacttcttcgaaggtggaatcacgcaagccatatggtgcataataatttttttggatagatttattgaggacgtcaaccgtattcatcacgttggcggcagagacatccatgtaatccagctgcaagcccataaacaaattttgaaagtcataaatgttgtccataaaactttgggatgcaatcggcatcacgtgatatggaaggttcggatcaacgagaatgatattgacatctgccctaatcactattttgtcttgatagggtgcttgagcctgaaaatttttagcatagtaatcgccaaacggattgttgcccattgagaatcgggaaacggttgggcccttttttctgatattgacgaggtatcgttcaaattttggatcctgcagatcggcgagggttttattcgttgaaataatccaaatttgctgaccctcgtattttttcatcaggtggcgattgatttgtttaatttggctgatctgcttctgatttaaaatgtgaagttcgtcagaaatgactggtcgagggttgccatccgctgagtttgcatctgctcggacggaggtgttgaacatcaaaatgattaatagtgcgataggcaaaaggatcgaacgggtaagatagtgcaaccgcgggttcatggtcattgtcctccttggattttatgctgagtatagcaccattatttttgtgggcggtcaaggtaactcttttcatttttttgtaataagtactagggttctttcatcttttgccataaaattgaaatgttgattcacgcgtttattcaaattggagggatccgtcatggaactgacaaccgcgaaaaattatttgttattaactgaaagaatcggtaagaagccaatgctgcgaacgcgatttactgcccaggcgtattttgttttggcggcgttatttgacttggtcgaccaaagaattttggacattggggagactatttcaatcaaagatgaccaagagtttgccaaattgccggattatctgagtgttttcaaatcagaactgactgatgaaattaaggagggacatgacctgcagacacaattggcaattatcaccagttgggatattgccaaccagctttatgacggccttggcgcaggtctgctggcggatcagttggttgagaagaagtcggtcaagaataatttggacacccacgtcatctatctgccaaaggacgctgctcgaaagcaggttcaggattatctgcgcaatcagattgacggcgcgaaaatcagtcaggacgccgttagtttggtgctgatcctgtcggagttggatgctttgaaatgggtgtttaccgacaaagaggagttggctaacttgactgccgcctttcagcagaaggtcgccggggatgcgttttacgccaaagaaaaagccctggccaaagtggctcaagacgtgattacgaagaagaagttttggtatgattcgtggttgagttgaggacgctctttgatttgaaaaaggcattctatgatataactaaagtaaatacatgggaggtttaatcatgaaagtccgagaacaaggaaactcacttgttgtaactgttcctaagaggtttggtattaagtcaggaacggaagtggtggccattaaaggaaaagatgggtcgttcatgtatattcctaaaatggaaaatccctttaaagatgatgcggttcacttccaacacgacgaagcgtttgatggtgattctacagggcgagaagaaatatgacagactcaatatattcatatcgcgggtatacaccagaacaggggggatattattcagtctgttctttttcatccgattcttcagttggtttcgtggatctggggatttatggttcatgggaaagcctatcactcaaaaatgctcaaagcccgatttgagagtcagtctcaaattagactttgggcatttcaagcttaaccgtcggccattgacgggatgtcccttgctcagcttgaattcccgaattaccaagcctatttcgttgcatttcacaagcaacctgccataattaaagtgtattcaatgtaaccgtttccattagcataagggggatattatcatggcaatcaagaaagttactgttgctggtagtggggtcttaggcagtcagattgcgtttcaaagtgcctttaaagggtttgacgtgactgtttatgatattagtcaagaagctgttgataaagctgaggaacgaatcaaaggtctgcgccatgcttatcgacatgatattgcggcgaccgatgaagaatttaatgccgggattagtcgattgaaatttacggatgatttagcggcggcagttaaagacgctgatctggtcatcgaagcaattccggaaaatcccgacatcaagcatgaattctatcaaaaattgagcaagttggcaccaagcaatgcgattttcactagtaactcatctacgctggtaccaagcatgtttgccgctgatactggtcggccaaagcagtttttgaacatgcatttttccaaccaggtttggttgaacaacaccgctgaaattatgggatcaccggaaactgatccggcaatctatcaagaaattgttcagtacgcccgggacatcgggatggtaccgattcagctgaaaaaagagcagcccggctacattctaaactcactgttaatgccgttgaacgcggcagcgggggcattgtggctgaaagggatcgctgatccaaagatgattgatcggacttggatggccgcaactggcgcaccatggggaccatttggcatcctggacgcggttgggattcgaactgcctacaacattactttggcagccgccaaaaaggatccggctgtgatgccgcttgctgatgctttcaagaagatgctggatgaaggcaagcttggcgttgagtcaggcgaaggcttctacaagtatcctgatcctgagtataagaccaaggcattccttgaaggttagcctattgttgaatgaacaacaggtctaaatcgttgattaaccagcgatctagacctgttttttgattgctgacaatttttgaaaaaataagtgcagttagttgtaaacgtttacaaacgtgctaaactttgggcgttgagataacttgttggttctactttagaaaggatcgattacaatgaccaaagtgttagcagttctgtatccagatccagtggatggtttcccaccaaaatatgtgcgggacgacattccaaagattacccactatccagatggctcgacggttccgacacctgaggggattgacttcaagccgggtgagttattgggcagtgtgtctggtggcttgggactgaagaaatatttggaatctaaaggtgttgaatttgtggtcacttcagacaaggaaggccccgattcagtatttgaaaaggaacttccaaccgctgacgttgtgatttcccaaccattctggccagcctatctgacagctgatttaattgataaagccaagaaattaaaattagcgatcactgccgggattggttcagatcacgttgatttgaacgctgccaatgagcacaatattaccgttgccgaagtcacttatagcaacagtgtcagtgtggctgaagctgaagtcatgcagttattggcattagttcgaaacttcattccggctcacgacattgttaaagctggcggctggaacatcgctgacgccgtttcacgggcctatgatttggaaggcatgaccgtcggcgtgatcggtgctggtcgaattggccgggccgtactggaacggttaaaaccatttggggttaaattagtttacaaccagcgtcatcaattacctgatgaagttgaaaatgagctgggactgacctatttccctgacgttcatgaaatggtcaaagtcgttgacgccgttgtcttagctgcaccactgcacgctcagacctaccacctgtttaacgacgaggtgctcgctactatgaaacgtggggcttacatcgttaacaacagtcgtggtgaagaagttgatcgagacgcgattgtgcgggccctgaattctggtcaaattggcggctactctggggatgtttggtacccacagccggcaccaaaggatcacccttggcggaccatgccgaatgaagctatgaccccacatatgtccggaacaactttatctgcccaggcacgatacgcagccggcgctcgggaaattctcgaagacttcttagaggacaaaccgatccgtcctgaatacctgattgcccaaggcggtagtttagctggaacgggtgctaagtcctacactgtcaagaaaggtgaggagacacccggaagtggggaagctgagaagtaggcttgctcatataatgctcaagtaaaataaaaaggttctgcaatatctgtcgttaatagatgtttatctattgctggtggcaggtgttgtagagccttttttattctggtgagcaattagagattgattgttaaccttctgcttcatggatatcatcttggatattatccactgaaaaatcatggtccatataatcacgattgtcgactggcaggtgttgttccaacgtatcgaacagttggtaagccacgtggcccttatccagatggaagtccagcagatgaccgccaaatgtcttgtcggcagaaaggaaatgattgtggaatccagcaactgcagcgccgtcaaataaggctggcgagtagtagctgatcagtgtcccttcaacttggtcgcgggtgaagatgctttgttttttggccgtttgagccaatgtttgaaatggcggcgttgatttcttgactgcccgggtcttgacggccgagaagcttccggtgatcttgatcgagaagaacgtgttgctggcctgggtaagtgagatgagctgttcttccacatcagcttgagaaagattttccagttctgccaaaggtgaatagttagccaagtggctgttcgcaaatggcatgttgaaggagttcgggaccacattcacgttgccgtcactatccacttggtagggcgtcccgtctaaaatgatcaattcaccgtcaaggccttcgccagtgccgatcccggtgtcgccgtgttgcagtaggtcacccattgtcagggtgccttctagtaggccggggaccagtaatgccaaagtgccgtgctgatacaaagttgttaattttgtcatcgttatcctcctctagtttaggatgtctggtaatagagcttatttgagttcaatgttgtcactgtagtcaactggaatgtcgatgatgaccggtccagctgcctgttgtgcctgatcaagggcattggctaattcctcggagttggttgcccgaaagcccttggcaccaaagctttcagcgtatttcacgtaatcaaccgggccgaacttcacgccggcattcttaccatacttggcttcttcttggaatttcaccatgtcatagtaaccgtcattccagatgagctgaacgatgtttagcttcaatcgcacggcagtctcaagttcctgacctgagaacaggaagccgccatcgccggagacggagatgactttttcatcgggtcgcaccaatttggcggcaatggcccatggcagtgacacacccagtgtctgcataccgttgctgaacagtaaatgacgcgggcgataaattcggaagtgacgcgccatccaaatataatgactgccgatatccaccgtcaccgtggtatcgtcgtcgactttttcctgcagcgtattgacgatatcaagtggatgcatggtaccgggcttggcagttgttgcagtggtgctttgaccgtcaaattctgatcgcagtttggtgagttgatcgactgctgttttcggaaggtggtagcttgctggcagagcatcggttaaggccgacagggttccggcaatgtctgattcaattaccatatccggttgataatcgacggtcaactccggggccaccgtatcgatattgataatttggtcattgtgttccacgttccagttgcgggcctcgtattccactggatcataaccgattgcgataaccaaatcactttgcttgagcagggtgtcgccgatttgatttctgaacaggccaacccggccaaagtaatccgcttcaaattcgtgagaaatggcgccggcaccttggtaggtttcaactactggcaacgatacttttgccagcagttggtgcaaggcctctgtgaccgctggagaagaagcccgcatgcctgccaggataactgggagcttggcgttcttcagtaaattaataatctggtcaagggttttggcggatgtttgagtctgctcgggtgcttgcagttgttgcatttccgggcgggtgacttcgccgcttaagacgtctgcgggtagggaaagaaaggaagcgccgggcttgcccgaaatggctgtgctgtaggcgttggtgaaggcttcggaaaggttgttggaatcttggacttcaacgctgcttttggaagcaacgctcatcaattctttgctggggatgctttggtgggtgtaacgggcaagatcgtcgcggggaacttgtccgcccaatgcaaccacgggatcaccttcagcggttgctgtcattagggccgtaaccaagttggaaaccccggggccggaggtggtggccactactcccggtttacctgtcaaacggccgatgccagctgcaatgaaggcggcattttgttcgtgccgagtgacgatcaattttggtgcattgggctggtcgctgtactggagatcttcgaataactgatcgactttggcaccagggatgccgaatacatattgaacctgttgattgatcatggattgaattaaagcttgtgaaccacgttttttatttgtcataaggaggacacctcttcatttttatgttgacaattcaacttacatttaaagataaagggcatgtgttgaattgtcaacaggaaaatgataatcttacggtaggatttgacgaatggaaaggaaaatgattttgaaagatattggctaccttgcacaggatatttcaattttgcaccggcagtattacaaggataccggtaagttttttaaggagcagcagctgaatccaacggctgcctgtattttattgacgattaatgataatgccgagattaatcagaaccaggtggccaagtcgttagtgatcgataagggactggcgactcgagaaattaaaaagatgcaggcactgggttatttgacgaaaacagccgggagcggcaaatcaatcatcttgagtctcacggctgccggccagcaggtgattccaaccatccaggcgattcggaaaaactggtgggaggaacggtttgcggacactgggattcagcccgatagcccgttagtgagtgcgattgagaaggttgttgactcgattgtggatgagagtttggagtgacggctctgctagttgggatgattttttaacgagaaaatagaaaaactgaacccccttgaattagatttctccaattcaagggggtttcttgtgcggtcaggtaaattcaaattgtcagagtaaggtcaatgataatcggtgatgtaaggagcatgctgactttggagattagttttcattaaattatcactaacacacgaaaaaatccgtcgtggctagttgtattttctgaaaattctgatgtaaatcagtcttaatactgtctccaagaaatctcaaaacgaattgtaaacgctttattagcagcgattccaactatctgctagtatttaacctcaaccggttgtaaaattgactttaatgaaacaaattcattttcataaattattctgaaaatgttgtgaaaggagtctttttatggacatcgtcaaaaatgacgtaaccacttatccggcatattttgctggtaactggcaagccagtgaatccaataagaccattgcaattcagtcgccatggcggcacgaaacgatcggtcgggttcaggctgttacccaatcagaggttgatcaagtgattgaggctgctcggaaggcgcaaaagccctgggcgaagttatcattaagtgagcgaggtgcctacttaaataagtgggccgacgaacttgataatcaaaaggacgacttggcaactgctgtgatggacgaagttggtaagaattacaaagccgctaaaggcgaagtcgttcgtacgattaacttgattcgctacactgttcaggaagccttacatatgcacggcgagagtgtccgtggtgatggctttccaggcggttcaaaagaaaaattagggattatcgaacgggtcccgcttggcgttgttctcgccatttcgccatttaactacccagttaatttgtcagcttccaagattgctccagcattgatggcaggtaatgcagtcatcttcaagccggccactcagggttcaattagtggcattaagatgattcaagcgctcgacaaagctgggcttccaaagggcttgttaagtctggttacgggtcatggttctgaaattggcgattatctcacggagcattccggcattaacatgatcagttttaccggaagtaccagaaccggtaaacgattatcccaaaaatcaattatgattccactcgttctggaacttggtggaaaggatccggcaattgtctgttcggacgccgatttagatgtcaccgtcaagaacattatcggtggggcattctcgtattcaggtcaacgttgtactgccgttaagcgggttttggttgacgacaagattgccgatcagttagttgccaaattaaaaacggccgttgaaaacttgagcgtgggctcgccagccgacaacagcaccatcgttcctttaattgacaacaaggcagccgactttgtttcaaacctaatcgatgatgcgttggacaagggcgctaccctggttaccggcaaccaccgcgatggtaatttattgacgccaactttattggataatgtcacccaagacatggacgttgcctggatcgagccatttgggccggtcttgccgatcatccgggttcattcattggatgaagccatcaagattgctaacaagtccaactttggtctgcaggccagtgtcttcacccaggatattgacaaggccttggaagctgctggcgccattgaagttggaacggttcaagtgaatggtcgcccatcaagaggacctgacaacttcccattcttgggggttaaggcatccggaatgggaactcaaggcgttcacaatagtattctttcgatgtcacgggagaagttgacggttgttaacttgcgaccttgatgacttgcagttaccggataaataatctttaaactaaataactcaactgattttcttgtttgaggagttatcctctgcagaatgattagttgagcttttttgtatattgatagattatttatgaaaagatgcgtgatgagtatttctaagcttatcgggtatgtaagtcatgtacacgcttctttatcttgtatgagataatatcattagttgataagaacgttgttgcacgacactttttacttagcagaacattggcaacagacggactgcgatgatgcatctagactagcttacgtagatgccaattcatacaaatctctttcaataaggtggtattaattaaatatggctcataaaaaaaccaacttgattacattgaaacagatcgacacttttattaacccaagtgcaaacgatttggggcaatcggatgataagcccctaaagaaattacctaaaaccctcaaacctttaaaaaagttgaataatcaagtagcttctcaggcgatcatccaaaatttattaaagagtaactatttctggagtgcccaaaccacaattttggggccagtgtctgcctatttggacagtttggttgatagtcaaaataaagatatcttgaaacagttaaccccacaaaatatcaaacttattaatatgtgccaaatcattaatcaactacagactaatggtgaaaatgggttgttatccggtgatcaattttttatgccagttacggagaagagtctgaccaaattgcattcaaccaccggggtatatgatttgctgacggatcccaaatcaagattgtatttttcaaccaaatactttcgcaaagacatcatcaataagcggccggtggtcacatcgaattatttaccacaaaagcatgctggtgaatatacagcaatggatgaagatttcagctttgcgcctcataacgaaaacgatccgcttcaaacgattactcaagacgagcaaaaaaagcttcacaaccaggatattgattcacaactggataatataaataatattcattcagtcaaggtgattggtaatccgttagaaactggacaattactgcatttgtcactttttgatgaacctgaattaaaggatcggtttaaaggtttgggttttggcaccgtcggcaaattgaagagagatattttctgggcgattcaaaatggttttgaggtcaaactggatggtgatgattatttggcaattagcaacctcaactggaatgacttgaagcgtaatttaatttctgaaaactattacagttgtttactcaatagtattttgagcattgggttgcttaaattactcagagttaaaattttgcatgaggatttagtcaaaattatcagtgctggtgccatgacgactgccaagtatttagatcatcaaggcatgacgatgatttcacccatgtgggctaagaaactgtacgggttaactgaagacttgcgctttcttgatgaaattgggtatcggactttaagcgcctatgacgctgatgatgacgttgaatttgggagtgatttggatgaagttatttgtgaactgcctaagtttttgagtgagttgtacgatatttgtgattagcgggtgagcgaggcatttaagggattattaataatattgtagaaccaataaatagcggcttgtggaaatagtttcccacaaaccgctattgttatggtgctaaatttgttaactgtaaaaatttaaattaaagcaatccaccgccgtcaacggcataagcttggccagtaataaaatcagcttccggactagctaagaattccacgatgtttgcaatatcgttgggttcaacagttcgacctagtgggatggtaccaatgaagtctttcttgttttgtccaagcggcttcccgttaatttctgacatcttccggtcgatttcgtcccacatgccagtcgtaccaacaactccgggcgcataggcgttaacagtgatgtgatcggcagcgaattcgttcgcagcagcttgagtgatgctaataacggctgctttagttgctgaataggttgcccaaacagggaaggcacgcattccggcaattgacgaggcgttgatgattttaccaggaacgccaagttctttaaattttttggctgcagcttggataccatagatgacaccaaagacgttgattttaaaactaaattcgaggtcttccggcttaatatcttcaaatttgtcaactcttgctaccccggcattgttgaccatgacatcaaagccaccaagttggctggctgcatcgtcaacagctttggcaacattcgcctgattggtaacatcgacggggataaagacagccttttggccagctgaagccacctcggtaataacagcttgagccttttccttttgttgtggtaaatcaccgattgcaatatcgtatcctttttttgatagatgacgcgcgatctctgcaccgatgccttgggcaccaccggtaatcattgctacttttgtcattgtaaaacctccatttgcattaattaaagcggttgcacagatgattttacgcttattatttggaagtgccaatgtacttttttatcattattgggggatttggcttactgattggtaatgggcaatattttgggaaaataatgagctatactctcttagtggtattacttaaccggagagtacagctcattatttcatatcaatatattaatttgtcgtttcagaatggactgcagctggttcttttactgacttttgaacgtcattggcagcaatctttttgcggttccaaaccatcagacctaaggtaattacagcgatgacgattggtccaactaaagtcaagttggcagtgaattcataaacgatccatgccagtggactagctgcaaaatcaatacttgcaactgatgatgtgccggctggaatcaagtttgattgcaccatccgaacagctgaagtgaagattgaggctagtgcagtggctgaaaggactccggcaaccaggctgaccaaaccaactaggaatgatcgtaaaacatttcctttggtgtatggaagaaccaatgggaaaatgtaaatcaatccagatagactggcaagtggtaggaattcgttacctgggacgattactgataagaagagaatagttggaaccaacagaagtgatacgaccaaagtggttgggtgaccaattaccaaagctggagtcataccaatgttgaaggctcggcctttgaacttcttgctgactagttcttgagaacgggtcgagatcgggtttaaaccttcaataaacatacctgtaatttttggaatcaataccataacggcactcaagataattcctaattgaagagtcttagccattggatatttggcaagcagaccaagaatgattccgatgatcacaccaagtaggattggatccccgaacagtccgaagcgcttttcaagtttcttggcatcgaagtcaactttgttgagaccaggaattctttcaacaatccagttaacagcgatagcaaatggaatgaagctgacacagaatgcctggggaagtgataccccctttaaatcttcaccatagaattcttcaacttttttctgtgaacggtcggcaccaaccaaggttacgatgatggtgatggtcgcggcaaacacgccccacaggaaacttctggttgcgatcgaaacgattgatccgatgaaggcaaaatgccagtagttccacaagtcgatattcaaggtttgggttgtcttggttaataacattaggatgttgattccaagacctagtgggatgatgatcgcaccaacctgggttccaaaggcaacagcagaagcagctggccaaccaatgtcaagggtatgtaggtgtaacccataaatcttgaccatttggttaaccgcaggtcctaagttatcagccaataattgggtaataacatttaatccaacaaaaccaacgccgacagacaaacctgatttcaatgattttgacggtcccatgccaagtaagacaccaaaaatgaagaaaatgattggcatcattacactggcaccgagggacataacataattaataactcccatagttatcctcctaatagtgtggatagtaacagctgaaattgatcaaatgattatgtgtagataaattattgcaaatacgaatcaatatcatcacctaacattcttatttggaaatgtttaattctatttaggaaaaccacaaacagagtatatgatattcatttttgaattgcaacaaaattcacaaaatattttacagaacaaagtttttatcataaattgctgcccctttgattcccagtatttgtatgcgttaacaattatttaagccccgttttattgattttgatcttctaaaaaaagaagaatgtttgttcagaattaattattcgttgacgtgacatagttcctatattgagttatactatttccaaataggaaacggtaaggagtaatatttatggaacgcaaattatatggaacagtgttaattaaagctgcggatattcttgacactttggccgacggtaagtcaaagtctattcaagaaattgcagttcaaactcaaattggcgcaccaactgtttccaaaatactgacgacactagagtatctacactatgtatctaaagcggaggcaaccaagcactattctttgggatctaagttggtacaatttggtttagttcatactcagacaacggatattgttgatatgacttttccgatgcttgaaaaattgcagtcaaagattgatgaaacaattcatttagcggtgccacaaggagataaagttgtttatgtcaataatctagagccaaagcaccaaggaatttatatgacatccaagattggtatgactcgcgaactctacagttctgggattggaaaagctgtactaagtacactttcggataaaaaaattgatcaatatttgaagagaaccgatcttaaaccttttaccaagcacacaattactaattcactggaattaaaggaagatattgaaaaaacacgcaaaagaggttacgccatcgataatgaagagcaagaagatggcggctactgtattgcaatgccaatcaggaaagccggcaaagcaattgcagcgatgagtatcagtattccaaagttccgtctcaccacgccatacaagacagaaatagtgaaagacctgaatgttgcaaaatcaaatatcgaagacgagcttaataaatagctcgtctttttttatttctttggtcaatgtgcttgtcctttggtgacacccaattggagccgctttttggacttgcatttagatctttttttaaaaagcggttgcaatttcagaaatgttgaatatactgtagtcacaaataggaaatagcaaattccaaataggaaatcacgttgttgcttgtcactcgcgaattataacggaggtttttcacatggctcaatcacaagaagaaatcaaacacaatgcagaatcattaaaccaatttaagatggactggtacagcctcaaaggtaaagttgccattatcactggtggtaatacaggactcggtcaaggttatgctgttgcaatggctgaggctggtgcagatgtatttattcctacatttggtcaagaaggttgggacaccacacgagaacttgttgaagctcgtggtcgcaaggttgaattcatggatgtggatttgaccgaaaaaggtatcgcaacccaagttgtcgccaaagccatgaaaatcttcggccacattgacatcctgattaacaacgcaggaatgatcaaacgtaacccactcttggaatctaaagatgaagactgggataaagtgatcgcaatcaatctttccgccgtttaccacttatctttagcggcatctaaagagttcgccaaacaaaagtcaggaaagattatcaatatcgggtcgatgctctcattccaaggtggcaaatttattccttcatatactgctgctaaacatggtgttgccggcttaaccaaggcatttgccagtgaaatggctgcctataacgttcaagtaaatgcgattgccccaggatatatcaagactgccaatactgctccaattagggctgataagtcacgaaatgatgaaattcttggtcggattgccgctggtcactggggcgaaccatacgagttgatgggaatctcagtgtatctggcaagtaacgctgctaattatatcaatggcgcaattattccagttgacggtggttacctggttcgttaatcagccctgtatattagaaaggggtctatagatgagtgaattaataacccttggggaaccgctagtcgtctttgcatcagatgaatgtgatgtttcaattgccaagtcttccaaattcactaagcggattggtggagcggaactcaatgtggcgattggaactaagcgattgggccattccgttcaatacattacccaagttggagaagagccactcggtgaatatattgcagaatccctttcgaaatatggtgtgggaactgattatgttttccaaagtgacgaatatctgacaggccatcaattcaaacaaagggtttcgcatggtgatcctgacgttgccaattatcgaaaggattccgctgccagccatttatcatttaacatgattgatcaaattgatttgacgggggtaaaaattgctcatttaaccgggatttttccagcaatttctcgcacggctcagaatactttgaaactatttattcaacagctgattgacaatcacatttttatttcgttcgacaccaatcttcgaccagcactgtggccaagtgagtcaacaatgattgattcaatcaatgaatttgcgaagctggcagacattgttttacctggtattcatgagggcgaaacgctgttgggcacacgtgatccggaatcgattgctgattactatcttaataatggccgtgccagtgcggtggtcgtcaaagttggtcctaaagggtcgtttgtaaagacaagatcgggtcatacgaatatgattagtggctttagagttgataaagtcgttgatactgttggtgctggtgatggatttgcattgggtgttatcaccgcgcttttggaaggcaagtcaattgattcagcagctcttcgcgggaatgcaattggcgcattacaggttcaaacgcctggtgacaatgatggttatccaacccaagaccagttaactaaattctatgattctcaaggagtttcagaagaaggagaagtgcaaaactatgctagagaagtctaaagtgctcacacaaattcaaaacgctgggattgttgccgttgttcgtggtaattccaaagaagaggcttatcaaacggccaaagcatgtattcaaggaggcgttggcagcattgagttagctttcaccgctcctcacgctgatgaagtgattggtaagttgaatgaggaatatgccggggatgcagatgtattgattggcgccggaacggtattggatcctcaaactgcccgtgttgcaattattgcaggtgccagctacatcgtcagcccatcattctccgaagaagtcgcaaaagtctgcaatttgtatacaatcccatacattcccggctgtatgactccaaccgacattcagcaggcactgaccttcggatcggaaatcgttaaattgttcccaggttcaatcatgggcagcagcatgatttccgagcttcacggtcccttcccacaggttaaggtgatggtgactggtggtgttaagctggataatcttgccgaatggtttgacaaaggtgccaagattgttggtgtcggtggccaaatggtcgggccggccgcattgcgtgactttgaaaaggttattgagaatgctcgcgtgtttaaggatcaggtgaatgaaattcgtcattctaatactgataaggtccttttgtaaaatacttaatgatctaacattgttagagattctgatgtgaaataaatcaaaaatcacgattcctgaagaatatcttttctcaggaatcgtgattttggttctacaatatctgttgttggtaatagatttttgtctattactgatgacagttttttgtttatcattagagtaaaaaagcggacatctcccgtccgttaacttgctcccaccacagaattaagtcaagaaaggaaatgccctatgtcaaatgatactacgaaaatgttgttaggaatagatgatgaacacttaataattgagaatggcaaaataggtgatgatggggtgatccgattaaatggatcgctgaactattcccccaaggcctgccacaactgtggggttattaatgaccatcagatcattggctatggttggcggaagaccaccattagattcgctaaaaccttgggcagcaccgttatcctctgcctcaatcggcgaaactttcactgtaaggcttgtcataccaacttcctggcgcagacgaatgcggtgccgaaacactgcacgatttcaaatacgacccgcaaacaatgcttagaaaaactgaccgaaccggtttcgctcaaacacattgccgatgagttatccacttcggattcattcgttggtcggcagctcttgcgcgctgaacgggactttgaaaccaactggcactatttacccaaagttctcctcatggacgaagttaaaagcactaagagcgccaccgacgcgatgagctttgaatttatggacgcggaaacccacgaattgatcgacctgttaccctttaggaccatctatcagcttcaaaagtatttccagcattacgaccaggctgcgcgagaaaatgtgaaaattattgtcaccgatatgaactatacctatcccaaattggtggggcagatctttccgaacgccatcgttgtcatcgatccgttccacttggttaacgctttaaatcgagcttttaataagacgcgggtgcgcctcatgaaaaccctggcgacctcatcacgcgagtatcacgccttgaaacgctattggaagctattattaacgccggaaaatcacctcaactacgaagctttccgtaagtggacaaacttcccttatccagcgactgccactgatgtggttgatgctttattggacattgatcccgagctcaagcaaacttacaacgtgatgaatcggttacgtgaaaccatcaaaaaccgtgattggcccaactataatcaagtattccatcacttagagggctgctcggaagagatgttggcaaccctccagaccctagcgactcatcatgatgaaattggcaatacctttactcaccattacaccaacgggcccttagaaggttcaaacaacaagattaaagtcattaaacgcactggatttggttaccgaaacttcttcagattccggctaagagtgctgttcgcttttcgagttcatacaaaaagagctctaatcaccaagtgattagaactccaatattttgttcaccaacaacagttgacgaagaaccttaattatttaattgtctacttaacctggagtattcccaccccgattaattggtttcattggcaaatttattgtaaagctgcgtgaagttaattgtccccaacccacttgcctggttgtaaatcttgccgggttggccggtgtagtacaaattgttgttgttatcagcgtcatcgaggacgttaaacggactgtctgactcttgagcaaatttgtaaatttgcggattccagaaaccgattggggtttggcggccactgttcatcacggcgttggcgccagccatctgtggtgaggtgtaactggtcccgccaccaatcagccatttggtgcttggaatgcgaagaacctttttaccctttagcactggattttttccggtgacgtaggtcgcatagccggtttgcaaatcagcgttgccggcaacgtcaggaatgttacgtgagttgccggttccaaagatgatgtggggatgcttggtgagagtgaacttgccgtttttatacgttagcaggttttccgctctaaatgtattcacaccggaaacaccttgttgataacgaggggtcggattcaaagctgagaagccgccgccactgccgccaaagatccccatctgcttttcgttggcagtctgggcgtatgtgtcgccccaagctcgttccttggaaacggtaatgactttattattcagaatcttctggtatggcaacgtggttccgcccactaagacctgataaggggaagttgacagaccatggttttccttggcactcggttgactaaccgggccatagtcaccactggcctgaaagacggtaatgccttgtgcggctgcctgttcatacattaagttaaacgcgtctgaggtttgtttgaccgttgcacttggatcgccccagtcggcggtcacttcaggagcagccgagaagcttgatgaaagctgcttgtcctggttgtcggaaatggccgacatcgtaccggtgtagatcgctgaagggtcagatgtatttggattggtgtcatcaccaatgtacagatcaatatctgcctttggggcaactgatgaggctgattccacgtcaaccgttgtttcggtctgcgggctgccgaggaggtagttgacgctcttttggacctcggcctttggattgacgaggtagtggtggtgaatttgactcacattagcgtcaatgccggattgcttccagtaggtcgccacgtcgccgtcatgaatgtcgctaacagtgataattccgatccgctgtccttgtccctgaaggcccttttgatacaggggatgcaattggtaggctttggcaaactttccggcaccatacttcagtgaaaaggtgtttgccgaaacattggtgtttggctgttgattagaaatcggcaaatcagccattaatgcatgggaggaagctgcttttttggttgttttcttagcagtcgcctttttagtcggcttttgcgcatagagcccgattacggcaaccaccttactcgacaaattgccaggcagcttatagctggtagtggcttcgtaacccttcttggccggtttaacatactttgcgttaaaagccttttgcatgtttttcggcgtggcggtcagcttcattgccaaattgccgggatacgcgtaactgcgaatatgatatttgttgagatagtctttaaatgactgaatgtagctggcggattggccaaatttgtcggcaaattcactcggcgtcaagtaatgatgatggttgggactggtcggatcgaccgtgtcgtaaacgtagttgctcaaatcagcctcgctggtactgggcttgaacgtcacgttgacgacggtccgtttaacggttgccgcctgactcgcagatccgatggccgcactggctcctaaaaccatcaggccgcttaaagcggtaatgacaaaactttttcccctcaatataatcactcttttcttgtgttatctggtttcaattataccaatcccattgtgagattacttgaatttaggctggtttccggggttagttgaccgcttttgccagccaatgcccaaaacgtgcgatgatggtaaaacatattaatatcataaacggcgcaaatcaaaaggcctggcaagtcagcacactcgccaggccggtaattgtcccttaagactcactaaatttaaacttcgcaggatcccacatccgcgaatggccaacccgatcatacccatagtgaaaattgatataagggtagggatcatccggctgaacgtccttgccgatcataagcagctgggattggatgaaactttgcacactgtggccaatgatcgtcttgtttgcattgctgagttgctggaaattgtcattgactttgacaataaagccgcgccgcttatcataaacaattccgccaacaaatagtgaccaagcataggcatcctcgccattttcggcctccttttggtcttgaatcaactcatcatccagactttggttaaattcatcttgttcttttgcggacaaagcggcataaggatcttcgtccgggtcatctgattctgattccgatgacgcgggttcctcggtttccgttgattcatccaacgactcctctgacgcactggattcgtttgctgtgtcagcttgctgactggtttgagtcgaactggaattatctgaaggggttccgccagtggccatcccaatcccaaataacacacagaaagcaatccctagatgtttccagccaaacggcgcaggctcttgcttctgccgattttggtataaataaattgctgcaatgatgaggccgatgtagcccaatcctaatagtacttgaagaaattccataaaatacctccgaataaagtgacgaataattgcaaattaaattgttgccagctaggccatactatatagatacggcacaaagctcgtttatcgtcattatctctaagaatttcttaaaattacaatttaaactctggatctgggcaaaaatccgacccccggcgacgacccgattcattaacagtgttacaatttctttggcgaaccaatcaatttgaatagggaagatgaaaacatgaatacgaaaaacaaattaaaggcaaccttactaatcgctgccggagcgctcttactgggcatctcgacgacccagccgactagcgccagtgccacagcatcatccactaccagtaccactaaatcaacgtccacccgttacgacgcccaaattgtcacaccaaagtcacttgcaagcggctaccaaatttattccaacgtccccggggtcaagaacaccaccggaacgccaacgactacaacagatagcagcgagtacaacaaccaatacgtccgcgtgatgcagacgcaaaaggccaagtcggttacatatgcgcaaatccgcctcaatgggaaaatcttgggttggatcaacgccaatgcacttaagcagacttcgttcaaggcaattgcccaagccaccatgcaaaaatataatgctgtcggcagtgtcttggtttctcacaacaagagcctgcaacccactttggttaacaacggctatgccaatatgcttcacagcaccaagaacaccagcgatgggtcggtcctctatccactggcctcgcttcaaaacaccatgactgcagccatgatccagcagctgattaacaccaagaagctgaccgccaccacgactttgagcaaatacttcccacaagtcgcccacagcaagacgatcactatccagcagctgctgacgatgacttccggcatcaaggggacgatcaaggcgcctgatgatcaggtcaccgaagatcaagcctacaccaacgccattaaggctttgaagtccaccaacaaacacagtttcagctacagtgacatcaactacgttctgttagctggcgtcatcgccaaagtcaccggcaagtcgtacaccaagaaccttcaatcacggattttgaacaaactgggcatgaagaatacctatgcgattaacgaaacccaaccggatttgactgcgattaaggcggtcagctatagcagttccaacggcaatgactaccagaactcccagtcggtttcctacccggccctttcagcgctgcccggcgccggcaacgttttgacgacgccaagtgactactacaaatttgtcattgggctgcaaaacggcaaagtgctgactgccaaggggtatcagcagctaaccagttacagcaccaagtattccggtgggatgtacgttgatcaaaaagggatgaagtccaataacggaacttatgacggcagcggatttaacaccggctacaccgcctcagacggcaaccagcacgtcgcagtggtcttcttgaaccagtcaccactgaagaacaacatgacggcttccgcatttcttaccaagatgaatattgtcgctacttattactaaaatgttaatcattaacgcccctgattgagagcatccaaatgcttggaactcccgatcaggggcgttttgttatccattcggttccggaatcgttatacggaggtgataacttaattattaagatttaagaagaaaaaccatgccaaaaccatcaccgaaaactaaagaaattctcaagaaactaaaacttagctaaagggcggccgaatttcctgcgaaatcgttgccatttatttcggtttgttcataatggacttaattaaatgttactggaatatcacaaacggtttacagccgtgtttccggtttttaaagggaggtgagcccatgaaacgggggcgcacgtacttatacataacactgattatcctggcggttgttggtactgtgggcggggccatgtactggcgggctaacaaccaggagtttcgaacgcaacaagcggccaaacgtgccaatcgccgcaggcaggagcagcagctcagctcaacggctaagaagcgggaggcaagcacaaaaaagtcggcgccaagacagattcagcacaaaacgacccagcagaccaagcagattaccagctacctgaagcgtaatcactttgtcggctcggcgattattgtcaaaaataaccacattctctaccagcagggcttcggttatgccaattacaaatcagacatcccaaataccccgagctcggaatttcaaattctatcgattcaaaaatcactgacagcggtaatggcaatgaagctgatcactcagggcaagttgtcattgaacaccaagctgtcaaagtactatccaaagattgccaattcccggaacatcaccatccgcaatctgatggatatggattccggtttgacgatgagtgaagccggttcggtccgcacactggatgaagcaaacgtcattaagtatgcggttaaccacatcgttacccgatcaccaaagtataaggactggtaccaaccggtcaacttcgtcgtattggcggggattatttccaaaattacccacaagtcatacggcaaatatttcgatcagctgcttaccaaacccctgaacctcaaggggaccggcttcgttcagcattggggcactcggccgaaccggacactcgggtaccactggttggcggctaaccaactgaagcaaaattacaccaggcagtatcacgaagctaaagcatcgatgcaaaatgaattgggaactggccaggttttcatgaccccgtttgacctcttcaaggttgagcaggcgatcctcaaaggcaagattattccgaaagccagtgtggccattttgcatcagccgggcctcaatgccccgtatggcggcggtatttataaccagcaaaacggaattcgctcccatggcattggctatggatatgaatcgtcattgttcatcactcgcaatggcaaatccggcgtcgttttactcagcaacgactaccggccggccaaccagattcaaaacttagctgcgaggttatttgacgacctggcaacgtaaaaattgaaaggtcactttgattgaaagcgctgtaaaacaagatattatatgggtgacgaaacgttacccatttaacaagggggatgatcatatgccagtacgacaatggttgcaaaagccgtgggtgcgctttacgatcacgacgctcatctacttttcgatcatgttggttcttttttacctctacgactatagcggcattaatcaagcgaaatttatctataacgacttctaagggggaacaaccagatgattgaaacgctcatttcaacaatcgattcacatgcacaaaaccagggggataaggttgcttacgcctacgatggcgagaaccacacgtatcaagaactcaaagattattcggatgctttagccgagcggatcgactcgatggcactaccgctgaaccagccaatcatcgtctttggcggcaagacttttacgatgatcgtgtcatttctggcggcggttaaatccggccacccatatattccggtggacattaattcacctaaagaacgtttggaaatgattaatcaaattgccaaaccggtggcggtcatcgcgactgagccactaccggagaaactgccggatattccagaaattgatcaggaacagctcgaccacatttgcctggaaaaagttgattatcgattgacccatcctgttcacggggatcaaacctactacatcattttcacttcaggaacgactggcgttccaaagggcgtcgaaatcagttacaacaacctggctggctttgtcgactggatggttagcgatgcttttgacttgccaaaggatttgcagatgcttcagcagccggcgtactcgtttgatttatcggtcatgagcctgtatccaacacttttccaaggcggcacgcttcacgtcttatccaagaagaccaccgataactttattgtcttattcacagctctgcggacgatgccgattaacacctgggtttcaaccccatcattcgtcgacatttgcctgctggaatcaacttttgatcaggcccattatccgaagttacatgattttctcttctgcggcgaggaattaacccacaagaccgcggctgcccttaacaaacggttcccggatgctcatatttttaatacatatgggccaaccgaatcaacggtggcaattaccgaaattgaaattaccaatgacattttgaatcactatgagcggctgccaatcggctacctcaaacccggcatgaatgcccaggtggtcgacgaaaatggcgcacaggtaaccgatggccagaaaggtgagttggtcatctacgggcagaacgtttccaagggctacatcaacaaccccgagaaaaatgctcaggccttctttaaaattggtgatcagcaggcttatcgaaccggcgatattgtcaccatggctgcagatggcctgctgcgatactttggccggaaagactttcagattaagctcaacggtttccgaatcgaattggaagatgtttccgcactggttagcaaagaagaacacgtcaagcaggcagtggtggtgcccaagtacaactcacagcacaccgtgtcgatgctgattgcctacgttgtcccgcaggaaaatgatttcaagaataacttggaacttaccgcggcgattaagaagaacttggggcaggatatgatggcctacatgattccacaaaagattgtttatcaaaaatcactgccgttgagctctaacgggaaggtcgacattaaagcagtgattgccgaggtcaacagtcaatgagatggtacattccatacggcaacccaacctacttcatctggctggcgctggcgattatcccgttaatgattggattgttgtatgggcaccggttccgcggctaccagacgattatctcgctgttcttcctgatcttgacctttggtggacccaactggaaaaccgggatctcgctgattggttacctgatttatcagctgatcctcgtgtggctgtactcagcgtaccggcagaaaaaggacacgcctaataaggggtggatctttgtcaccgcggtagtcctggcgattgtgcctttggttatcgtcaaactcacgccgctgtttacccctggtcgccaatcaatcgtcggcttcatggggatttcttacatcacctttaaagtcgtgcagaccatcatggaaacccgtgatgggatgattaaggaattccatccggtgttgttcggtcagttcctattgttcttcccgaccatttcgtcaggaccaattgaccgttaccggcgatttgaagctgattatgccaaggtgccggagcagagtgcctacctggatatgattcaaaagggtgtccgctacgttttccaaggctttgtctacaaattcgttctggcctactacttcggttcggtactgatgccccagattcaaatgcgggcgttgatggctcacggcttttcctggaacatcgtcgcttacatgtatgcttacagtatggatttattctttgatttcgctggttacagtttgttcgctgtcggcatcagttatctgatgggtatcaagacgccgatgaacttcaatcagccgtttaaatcaaagaacatcaaggacttctggaaccgttggcacatgactctgtcgttttggttccgtgattacattttcatgcggttggtcttcttctgcatgaagcatcacattttcaagagtcgaaccaccacagccaacgtgtgctacgtgattaacatgctgatcatgggattctggcacggcgagacctggtactacatcacttatggtctctaccatgggtttgcgatggtgattaacgacacctggctgcggttcaagaagaagcatcaggaccacattccgcataacaaattcacagaagcctttgcgatttttctgacatttaacgttgtttgtttcagtttcctgatcttctcaggattcttgaacacattgttctttgcaccgaaaccattttaattaagaggagttgttcataatggatgataaacaaacggtacttgatattttaaaagacttaactggtgaagatttttctgataatttggatgaagatttatactcaagtgcgttgctggactcaatggggacggtgcagttactgctggatctccaagataaattgggcgttcaagcccccgtttcagaattcgatcgaaacgagtggaacacgcctgccaaaattattgcgaaagttgaagcagccaaatgagtgttaaaaagcggctcttcatgatatttgggccgatttttgctgctgcgctgttgatgctggccgtgtttttatcgccgctttggtcggggttcagctatgtgaatcccacagtcgtcgacaacgctgccgcatcgctttcgccgcaggttttaaaaggccagctgattaaacgtaacgcacttgaacatggttatgtcccattttttggttcatcagagtggtcgcggtttgacccgtttcatccttctgttctggcggccaagtacaaacggagttaccggccgttcttgcttggtgcccggggcagtcagtcactgacgcatttctttgtcatgcagtcggtcaatcccgagttgaaaaataaaaaggccgtcgttttcgtatccccccagtggttcacacccaagggagaagaccccaatgccttttcgttctattattcaactttgcagacgactaattggattaagcagcagaacggatccaaaatggatcgttatgccgcttatcggctcttgcagatgccttccggtaattccgacaaggtgattgccggcgcattggcccggatcgctgccggtctaaaaccgacaacttctcaaatgttgtatgtcaatttgcgcaaccgcattttgttgaatgaagaccaaatcttctcgcgatatcggattcggctgaacaatgaggaaaccatcgataagaacgaggagctgcttccagctcaatacaactatcaaaagttggatcagctggccggcaaaattggtgccgaaaagacgtcttcaaatgatttccaaatttccaacagcttttggaatcgccgattgaaggcccacgtgaagaaactcaaggggttccagtccaatatgagcttcttaaagtcgcctgaatacggtgatttccaattgatgctcaaccaatttgccaacgaccataccaaggtgttattcatcattccgccgatcaacgcgaaatggcagaagtacaccggtttgtcggcaaaaatgctggatcagttcagcaataaaattacttatcagctgcggtcacaaggatttacccacattgacaatctcagtcatgacggcaacgttccttattttatgaccgacacaatccaccccggctggcggggctggctgaaaatggatcaggcaattcggccatttttgacgaagaaggtcaagacgccgcattaccgaattgataactactattactctaaagattggcaaaacgaaagtggaagtgacaacgattttgatgaataagtttaaaagcaggaccgtcatgttattcttggcgggcctgttgtctgttgggggcttgatggccggaaacaaggcctttgctgcctataatgcggtgatggcaaccagcaataagcattacgatgcccaaattgtgaatcaaacgaccgtcaaacgcggctataatttatacaccgacggtccttacaataccaacgccacgaccaagacggccgatggcaatggttataaatataacaatgcctatgtccgggtcttgcagaccaagactactaaaactggcacttatgtgttacttaggtactacaaccagaagctgggctggatgaatattcacggcatcaagtcggtgagtttcaatacgattgccagtaacatgatgaagcaatataacgtagtgggaacagctgtcttggcttctgccggcagcaacaataccgccgttgtcagcaatggctatgccaatgcgttgagaaacgtggttaacaccagcaacggaacagttgtctatccgctggcttcgctgcaaaaggcgatgactggtgccattatccagcagttgatcagtgccggccagttgacgccgacaacgccgttaagcaagtactatccgaccgtgccatatagcagtcagattacaattgccgaaatgctgtcgatgacgtccggcattgataacactgatgtgacgccaagcagccaattgacggaaaatcaggcgtataccagcatgattcagcggctgaagtcgaccggacaaaatacttataattacagtgatgccaatttcgtgctgttggccggtattatttccaaagtgaccggcaaaagctatgcccagaatctgcagagccggatttttaacgcggttgggatgaagaataccatcatcgtgggcagtaagcagcccagcaccaaatcaacggtggcggtcggctacaccaaccaaggcaaatacaattaccaggatgccgacgcggtttcctatgcccgactctcggcaattcccggtgccggcaacctgttaagcaccccgagtgacttctacaaatttgttcagggcctgcaaaatgggcagatattgtcagccagtcagtttcagcaattgaccggttacggcaactactattccggcggcctgtacgtcaacaaggacggcctgaaatataataatggttcctttggcggctcaagtttccataccagttactacgcccgagatgacaactaccatatggcactggtctttatgaaccagtatccgctggtggggggcattagtgcgaaggcgtttacgcagaagatgtatgatgtggcgacttattattaaacaatttcataataaaagaatcggtgattatttggtcaccgattctttttttaatgagtaattaaaatgttaagcgagccctgacgaatgacttgcaaaggatataatcaagaaaaaatggagatgtcaaaatgcctattgtagttctcaaagacttttatcaaccaaatgatttgactgaaattgtgactgccgcaattcatgccgacaacgctgactgccataccatcattgagccaaacatcatcgtttcgtcttcaaatgttgtcagtaatccaaggcgatatgaagatctcctgtactttaccgtcagaccctttaaccagaaattaaaagggatttatagtttttataaagagcggggtaatgtttttctagaaaaattacccgacaattctgtcatgggactatctccaatttatttaggagaaggtaagggtggcacagttcccaagcaattaatggtggctctcgaaaaaaagattgaatcattttgttatgagaacggcgtggccaatgtcgatcgttatcctttcgatcggttaaaatcggcagaagtgactttgcgaattgtaccggaagatacttatcaagttcccggttttactttcgatattcaagcattgcctgaggttgaggttgaataatctgactaccactcaatctcctcaaccggttccggcgaatcgttcaactcatcattcttaacctggccgtcaccaatttcgatgatgtggtcggccattggtttaatcatgccattgtgggtaacgatgatcacgttcttgtccgttttgtggctgaaatcttggagtaacttgaggatgcttttaccagttttataatccagtgccccagttggctcatcacagaggagtagctcggggttcttggcgatcgcccgggcgatggcgactcgctgctgctcgccgccggatagttgggccgggaaattgttggttcgtttggccaggccaacgtctttcatgacctcgggtacgtccagtgagtccggtgaaatttgggatgccaactcgacgttctccaaagcggtgaggttggggatcaggttgtagaactggaagacaaatccgactgacagccgtcgataggtcgttagctgttttggcgaataggtcgcgatattgcgatcgttgacgatcacgtctcctttagtaggagtatccatgccgcctaaaatgttgagcagcgtggatttccccgctcccgaggcgccgacgataattgtgagttcgccctttgtaatttcaaaattaatgtcgtcgttggcgcggacttcctgctcgccgctgccgtaaattttggatacgtgtttgacgtcgatgtatgccatgattgcctcccgaattgtttctttatcgattatgatacttgtggtttgcagggaaagcaaccgtcattgggttagaaaaaatcctctcgtgaaggaacattgcgagaggattttgcttacttcttcaatttatcaatgacttccttaagtgattcctcaaaagtcggcagtgggtgtcccaaagcctctggaaggtcgttggaggtttcttccaggtcgccatttcgaatcaagcgctgcatgccaacgattgaagcggcggctgctggactgtatcctgtggcaaccaggcgtttgcggtattcgtcatcggaaaccgacatcacttcaaaatcgttatcggtgactaattgtaatgcccgggccaaatcggcatagtcgtgttgcggtccggaaaattcatacaccgtttttggctcatcagtcattaaaactttggcagctgcttcggcgtactcccgctccagtgcccagccaacccggccgtttccggcagaataaacgaagggtcggttgttaatggctgcgggaatctgcaggcgctcattttccagataccagttgtttcgtaagaatgagtaaccaattcccgattgacggatagcctgttcagtattcttgtggtcaacggcaagtggtgatttggccgtgtctgcgtgtgggaagctggtgtaggcgatgaaccggacaccggcttttttggcggcgttaatcacgttttggtgttgttggattcggctgactgcctggcctggaattgaggaaattaacagcagtttatcgacaccggccagcgatttttccagcacctcctgcgaatcatacgaacctgggcgagcttcaatgcccggcagcagtttctcagccttctcagtgttccgtgccagtgcgatgatgtctcggttatcaacgttttcagctaacactttaatgacagtttgaccaaatttccccgtggcccctgtaacggcgtatttcatattggcgatcccctttcaaatcataatctgaacgactaaattatcctgtttaattgatgttaccaaggattggaggggcttacaagaatttgaacttggagaaattttcaataaaattcgattattcatgaaaattttcatgatgttcgatatactaaaatgaggtttttaactggaggacatgatgaaaaataatggctggtatcgattagggcaggttagtgcggtattctgcggtggcgcgctaggtgggattgcccgatatgaaattggagactggatccatagtgccaatgggttgcttggaaccagcgtcgtgaatttgctggggtgctttttactgacatttacaatctatggcctagatttgcggtttgatttaccggagtggcagattcttggccttggtacgggattcgttggggcgttcaccactttttcaacgtttactgtccagtgtgtgcagggaatttccagtaatcccttgggctcactggtcttcttactagtcaatctcatcggtggcatgctctgtgttctacttggctacttaaccgctaccacagttgggaggcgtcagcgatgacaacgatgatctgggtaggactcggtgccggattgggagctgcttgccgctatgggataaccgtcctgggcaaattggcatcaccgacggttccctacgcgacaattttaattaatgtgattggctcgtttctggccggatggttgactgggagtcagctaccggaaacttgggcgctatttttactgactggggtttgcggtggctttaccacgttttcaacgttttccgtcgatacgtttgtcttggttcgcaatcgtcagtatttggttgccggttggtattggcttgggacggttgccttaggtgttttggccgtggtttgcggtttgtggttgggtcgataagttaaattattgcttgtaactatacaaaatgcgatttttgtttagtgcaccatttgttgagatgttgcataatatgttttgtaaggaatgacatgacccgttggtcaagtggttaagacattgccctttcacggcagtatcatgggttcgaatcccgtacgggtcatttttcaacattgggttatagccaagtggtaaggcaacgggttttgatcccgtcatgcgttggttcgaatccagctaacccaatttcataatataacttctctctcaagtagccgactgtcattatcaactattgacagtcggctatttactgattgtaaagaggccttattttgttacacatagaattaaaaaacgctaatataattagaatttttaatgatttagtaaaataaacaaagtttttctatgctcgattaatcactaatagacaaagttatggatgtgtcgtatgccagtataacggacattttatgatgaaacatacggttcactagaaagttatagaaatatgggaaaaatgagcaaattcgctgaaatgaaaacgcttaattagaatgtcgtaaaccgctttaaaatctttattgaagtgttatgatgatgttgctgagtaatcatattattagcgttaagaattgaaaagagggatttagatggactcaatagccaagcatgaattaagcacatccttagaagaacttgtaactaagacatctttcgatgatgtatctgtaaaattaattgtttcaaatacttcttttaatagacaaactttctattatcattttcaagataaatttgactgccttcagtacacactgtctgagtttgctgacaaaattgcgtcagatatggattactcaaattggcaagaatgctacttgaggatattcagatatattgattatcataaagagtttatgcagcatatcgtggattctcaagcatactcactttttacggacttcgttcttcaatcaattgatttgatgctccatggggttctgaaatctctccaaaaggatgtttcacgtaatcgaatgcaagaacaaccttggaagctttttgagtatggactacagggtatcattatcaactggtttacagatgggttgagagagaatccagaattgttagtcaacgatttattgaatattgatatgcctcatcttaagatgcttcttggagttgatacagatcgtattgatcaaactggacactttgtccattccacgtctaccatataggcaattgcaattatatttttttaattatgatcacgtttcccaaaaagccaagcgatatgaaactttatcgcttggctttttagtcgcagaattttacatcctatacatatggggtcaggtgtatagaagatatacaaacggtagcttttgtatatttgcaacataatatttctgatttatgctcaatacgtaactaagagagatggcttagttaataaataaaaacgtggtctgttagcatttgaaagcggtaccacgtttgaaggagatgtatttggtttggaaagagacgacgttgaatctcatgctgaaagcattaaaaacgccaaccagatcaccgggtttcagttgttctcaatgacaacttccatggtgatgacagtttatggctttgcggcatttgctaagcaaggccccacagcattgttctttctcttcttggctgggatcttatggtttattccagttacgaaggcagctggagaaatggcttccattgacggctggagccgaggtggaatatttacctgggcaagaaatatgttgggtgaaaaaactggatgggcggcattgttctatcaatgggttcacattaccgttggaatgaacacgatgatgtactttattattggatgcctttcaataagtgtcggattaccaatcatgaatgataatccattcgtaaagtttggattaatgatggttatcttatggggattgattttggtccaacaaagaggaacgaaattaactggtaagatcgcgcaatggtgtttcacattaggtgttattattccggtatttttcttacttgcaatcttcattatctaccttgcacaaggcaacccaatgctgatcaatatcaatttccatagtattcttccaagcagttggagtggggatgtacttgttgggtttgttccatttatgttagcatttgccggtgctgaaggatccgctccgcatgttaaggatttggatcatccacgtgtctatcctaaggttatgttggctttagccatcgcggctatcgtttcagatattgtcggaagtatggctatcgctggaacaattcctaataaggatattcaattaagtactggaattgtatacgcatatggcgcactggtacaaaagtttggaattagtgttgttatcgtagaaaagcttagtggattcttgcttgctgtcggcgttcttggtgaaattagtagttgggtcgtgggcccgaatgccggaatgtttgaagcagctaagtcaggattcttaccaccacgattttctaaagcaaataaatatggtgttgaaacaaatgtcatgattttacaaggaattatcgtatcaatcatgggtgcattattaacatttggagcaggtggaagtaaagctaacctttccttccaaaccgcaatgagcttgaccgttgcactttatacactaatgtacatgttgctattcattagttacatggtacttcaaattaagcacagcgatttgaaccgaccttacgttgcatccaagagtaaggttatgagattagtatatggtggattaggattcatactttctgcgtttggattctttgtaacattcttcccgccaaaggatatgatcgcatcttcgcaaagaacatatcttacattgctattaactggatttgttgttgtattcttcattccgtttattttgtatcgttaccacaaacgttgggcaaacgagttgggacttcctgcagaagaaacagaaaaaccaactgttgttattaccccacaggcgcatggagaaactgctaaaaagtaggtacttgtgaacggctcaaaatttttaaaaaataaggaggaagctaccttacccaataagtaatctagctataacacgatgagtgaaaaaaatgatgaacagatgattgatgaaattggtcttgaacagaacttcttaggaagtgttgaagctggtaaatcattgccaactgaagagttgccagagcatccaatgccagctagcattgctgcccaacttgtccagcattatcggctgaatgaagctaaagctaatcaaaacctggcaacgttctgtacaacacagatggagccagaagccgataagcttatgacagatgctcttaatacgaatgcaattgataagtctgaatatcctaagacagctgcaatggaaaattactgtgtaagcatgttggctcacttatgggggatccctaagggcaagaagatgtacaaagatttcattggaacatcgactgtgggatcttcagaaggttgcatgcttgggggactgtcactgctgttgagctggaaacatcgtgcggaaaaggccggctttgatacgaaagatcttcatcatcatcttccaaatctagttattatgtcaggttatcaagttgtttgggaaaaattctgcacttactggaatgtcgaacttcgacaggttccaattgatcagaaccatatgtctatggacatggatcatgttatggattacgttgacgaaaatactattggtattgttggaattcagggaatcacttatacgggtgcggttgatgacattcaaaaattggatcgattagtgtctgaatacaacaagaccgctgtgcttcctatccgaattcacgttgatagtgcgtttggtggactgtttgcaccatttgtagatggattcaagccttgggatttccgcttgaagaacgttgtatctatcaatgtatccggtcataaatacggaatggtttatcctggtattggttggatcgtttggagaaacaattctgaggatctactgccaaaagaaatgagattctctgtaccatatcttggttcaagtgttgattcaattgctattaacttttctcatagtggtgcccacattgttggccaatactataactttgttcgatttggttacaagggctatgaagcgattatgaacaatgttcgtaaggtttcattgcggattacagaagaattaaagaaatttggtatttttgaaatcctgaacgacggaagtcagttgccgattaactgctggaagcttgctgatgatgcaaaagtggattggacattgtatgacttggaaggtgaacttgcaaagtatggatggcaagttcctgcatatccacttccaaagaatcgtgaagatacaactattagtcggattgttgtaagaccatcaatgactatgacaattttggatgacttcatggaggatctaaagatggccattcataatttgaacaaggaacatggaaacaacgaattggaatacaatattccttcagcagcagacgcaacaacggtcagcaataaataaagtaaataatcagatgggagaagtgtcagaaaatggacgataagaaggttagagtaaggtatgcaccaagtccaacaggattcctgcatataggtaatgcacaatcagcattgtttaactatttgtttgcaaaacattttggaggaacgatggtattaagaattgaggataccgatacaaagagaaatgttcctcatggtgaagacagtcagatagaaaacttacactggcttggaattgactgggatgaaggacctgataagcctaatcctaagtacgcaccttaccaccaaacccaaagagtgtcattgtatcacaagtatatccaacaattgctcgacaaggggtttgcctacaaagattacactactgaagacgaactcaaggttatgcgtgacgaacaacgaaaaaacggtgaagcccctcattatgacgggcgctggtatggaagaagcgaagaagatcaaaaggcagctgaaaagcagggattaaagcctgatgtgcgtcttcatttgccaagtaatcatatctatgcttgggatgacattgtaaaaggtaacgttcaatttaattctgacaatatgggtggggatttcattattgaaaagagtaatggaatgccaacatataacttcgcggttgttattgatgattatttgatggatattacacacgtgcttcgtggcgatgatcatattgcgaacactccaaagcaaattgcagtgtatgaggcgcttggtattactccacctagatttggccatatcactctaatttacaatccaaaaactggcaaaaagttaagtaaacgtgacaaagaaacgttacagtttattagtcagtataagaatcaaggttacttgagtgaagcgatttttaactttatcgcattccttggatggtctccagttggtgaaaaagaactttattccaaggacgaattaattaaggcttatgatcccgaccggatgtctaaatctcctgcattctttgatcaacacaaattagactggatgaactctcaatacatcaaaaatgctgatgttgcagatttaacggatcggataatggatctgattaaagaaggcgaatcagagattgctaagaagctccaggatgttaatttgccaaacttgcgtgaattcatcaagcatgtaactaaggtttatcaacgtgaggtttataaacttaccgacattatggaaaaagtatacttctttgcaaatgtggatagtgagacatttgattactcacaatttgatgatttctcgccggtggttgttcgactaattttgatgcaatttaggagagaattgttagatgccagtgaaaagggtgatatcgactttgacacgattatccgatcggtgggaaatgcaactggaattaaagggagagaactgtatttcccattaaacgtaacctttacagggaatactaatgctccacaggttggtagcattttaaaactgtattcgatcagtacaattattaatttggttgataaggcgcttacaggaactgaagtaaagagttaacaactaagttctactgtgcggattgggaaattatctccatcgatcaattatattattggtccggatgatgggcatcagaaaagggctggacaaattgatttgtccagcccttttcattgtataagcgttaatgattgataattttgtatgctgcagatggattgacaagtgcccaagtgtatgggaagtaattcatccaaatatcatcagtaaatgcaggttcgaatgattcaatctgtggtgaatcgattcgaactggtctgagaatatcagcaattaattccaaaccaaccgtagaaaatgcggtgacttgtatctcaccattttcgtccaaggagttgttgacagattgtccattcagcatggtaaaaacatcattttcaatttcgtttaatgccattctttgttgcatgagataaatatcccattccctggaattcggaatgtacattgaaaaataataatctaggagaaagtttacgtatgttccagcaaaatcctttgcaggggtgtacccaccgttttctggacgactataaactgatgcaccactaaatagatctcgtattgcttggaaaggattaggggcgctcgaatacattgatagaaagcccatttggcgtttataaagattaactgcgtccgatggtgttaatgatcgtactaccgagacgtccaacgaataatcaaccttatcaatgaatcggattttacgttgggttcccaaacctcgatcacgaagacggttaacgtttttcgcgaattcagcaaaacaatcttttcggcttttaagtgtaggtaaactattgttattcttttgccaagttacgaattgatttcccatatcttggttcttgggggaaaagttagttactggatcgatgcccagctgttcgagcatttttctcccatctagaccaagaatatggccattactacgatttctgtttctgaaaaataagctggtacaaaaatccatgtttaaatcaaaactattaaacattagcttttccctccttctttagattatggtagaacgactaagtcataaacttttatgtcattgtaattgtatcaaatacaaataaaaattcataatttgttgtctatcattaataactattatctccttttatttagaaaaagcaacctttcttatctatatattagtcagataatcattgtaaatggatgtaagcgctgataataaagcgtttatgcatgttagaaaacattacattgaatcttttacgttgtggaataaaattctagaaagtgtgaccattatgaatttggaacaagtaaaaactgatttaaaaaacgtcttaattgattattttgaaaatgttcagtttccgcggaacggaattttcgtcgttggatgcagcacaagtgaaattgttggcgattggaaaggtacaaattctagactagatattggccgagctgtcatcgatactgtgtatccatttctgaggatgcgacatattcacttggcagtccaagggtgtgaacatatcaatagagcattattagtcgaagaaagtgttgctgagcgaaataatcttgaaatagtctcggttgttcctgccattcatgcaggaggtggtacccaggtagcagcatatgaaagatttgaacgcccggtagaagttgaacacatttctgctttcggtggaatagatattggtggcacagatattggcatgcatgtgaagtttgttcaaatccctgttagaacagcccatcgtcaagtcggtcacgctggggtcgtaactctatcctcaagaccaaaacttgttggaggtcaaagggcacaatatagttttacagataacaatttacgtgaatttgtcctgaagagataagtagatgaaattagatcatgttccatctcgcctgcttgtacccttgagagctaaattgtgtcttcttgtcttaattaatgcggctgtcagtacatcatttgtcttaactgtccctgatacttcaattaatgtaactttttgtgattttggaatctttctgggagctttcatatatggctcatggggaggaggggttgttggtggaatcagcgggcttttgattgtgttttttcatgggaatctgagttttatgattccttccatgattattcatagtgttgagggaatattcgttggtaaaattgcctcaaactcaaatgatgaaggtggaaccctttatattgctgtggtaacgggggtcattataatggtattaggatattttgttgccgacagtttattgttaacacatactgtagcctatagaaatattacggacaatgttaccggagggataatcaatgcaataggtttgttgttaatttctccattgattcaagcatatcgccagactaattattaatagtggcttgcatgtattgaatcttgaagtgatatctgctgaatacagcatagaattgaaaaggacactgttctctgttcagatgaggattagtgttcttgtcatttataattaagtaaataagaaacacaattcaacctaattttaattaaccacaaatcgggaacttttttaatactcagtaaaatttaatttgaaaaatttgtgcaaacatgctgtgttgtcaaacgctttcatattcgttacactattatttgttgagctatattcgattaatccaataattttcgtggtgggggattattgattaataatcatattactaggcaggaccagtgaaaaatctgatctattttgtgttgtacttctcagaagggggaaaattatggacgcacaagtcgaaaaaccaaagaagcatttcaagctgaaaatgcccggtgcctttgtcattctgttcattttgacaatcgttgccgtggctgccacctggatggttcctgccggtagttattcaaaattatcgtacacgaattcatctttgcaggtaactgacccacacggtaaagtcaccacggttcccagcacccaaaaagaattagacaagctgggcgtcaaaattaacattaagcaatttacagatggcggcatcactgcgccggtatcaattccaaatacttaccagcgactcaaacagcggccggcaagcattgcggctgtcccgaccagcatggtcaaagggaccattgaagccgtcgatattatggtcttcatcctggttctgggaggcttgatcggagtcgtcaaagccagtggcgcttttgaatccggtctgctggccctgaccaagaagaccaaagggcatgagttcttgctgatcttcttcgttgccatcctgatggttctgggtggaaccctttgtgggatcgaagaagaagcggtcgccttttatccaattctggtaccgattttcattgctatggggtacgattcgatcgtgtctgttggcgcaatcttcctcgcgagttcgattggaacctgtttttcaaccatcaacccgttttccgtggtgattgcgtctaacgctgccggcatcgactttacccaaggtctgccggagcgggccattggtttggtgattgctgccagttttgtcgtgacttatctgcactggtacagcaagaaagttaaagctgatccaaagttttcttactcctatgacgaccgtgacgaatttaatgcaatgtgggaaattgccccaaccggggaagatgccaaatccaaatttacaatgcgtaaaaagctgattttgatattattcgttgtcaccttcccactgatggtttggggcgttatgtctcaaggttggtggttcccaaccatggcggcttcattcctgtcatttgcaattatcatcatgttcctaacggcaactggtaaaaatgggcttggagaaacgggtgtcgttgatgctttcgtgaaaggtgcttccagcttggttggcgtttcgctgatcattggcttggcacggggaattaatcttgtgctgaataacgggaagatttctgacaccatgctccagtattcatcaaccttggttgcccatatgaacggtccaatgtttattgttgtgatgctgatcatcttcttcctgttaggattcatcgtcccatcttcatcaggcttggcggtgctgtcgatgccgattttggcaccgttggccgatacggttcacattccacgttatgtcgtggtaactgcctatcagttcggtcagtatgcaatgctgttcctggccccaaccgggttggtgatggcaaccttgcaaatgctgaacatgaagtattcacactggctgcgtttcgtgtggccggtggttgtcttcgtcctcgtgttcggtggtgcattgctggtaactgaagttttgattaattaatatttaatacgtgaactcaaagtgcctccccgtcaggattgacggagaggcattttgctctaattattaaacaacttccaacaaatccagtgacaaaccagctataataattaataatctgcacgagacacattcatgaggaggttcatcatggggaaatatattatcaattcaaagcttagaaaagttggcgctcaagtcgacacaaaaacaggtattcatcaatttatcgtcgatgaaccgattgccggtcacggaacagacgctggtcctaatccggtgcaatacttgttgtcggccgtcggcagttgtttagccattacagccaacgacatcgcccgaaagcacccggaaattcaaattaagaagtttgaaaccaagacgactggcgagaccactcagtatcaagatgggcgatcggcggtgaccaaaattgttgttcagattcatgccgaaacgaatttggatgaggctgggcacaaggcgtttatgcattcagtcgtcaaggactgtacggttcatgaaacgttaaagcacgcggttccgattgagttgcaattcatctaggaggggtactatgggaaagatccgaaaggtgtcgttaagtattggaattgtcatggttgcggtatttttggcggcttgtggcaagcagtcttcccaaaataatgcgcagaacaagtcgattaccttaatgcagacatctgatttaacgtcgttggacaataccaatcaagccatgctgccggagtttaacaccctaaccaacatttctgaggggctctaccggcttaacagcaaggatcaaccagtcccagcaatggccaccaagattgttaagccaactgataacggtaaaaagtatgtctttcatatccgttcgaatgccaagtggagtaacggtgatcctgtaaaagcggaagattttgaatattcctggaaacgatccttgaacccggcgaacaacccggtttacacctacgtctttagtggaatcaagaatgccgatgcgattatcaatcacaagaagtcctacaaaacgcttggaattaaggcaaccggcgacaagacccttgagatcaatttggatcacccgatggcctatttcaacaagttagtcgcaatgccggtcttcatgccgcaggataaatcatttgtccaaaaggtgggtgtcaaaaagtacgggactaacgctaagaataccgtttccaacggcgccttcaagattaccaactggaccggtaccaacgatgcttaccggttggtaaagaacccatattactgggacaggtcggcgattaagttagaccaaatcaactataagaccgttaaggattccaatacggcccataatttattcgaggacggcaagttggacgatgccaccatttccggtgttaccgccaagtccctgcagaagaataaggacttgaagcggatacctaaggcctggacttattatctgcaggttaaccaacggaaagggcgaccacttgccaatcaaaagttgcggcaagtcatttcattagcgatcaaccgaaaagaactgaccaataaggtcttggcggatgggtcactgccagccagcagttttgtcagcccaggaacagccgttgacccaacgactggtaaggatttcagtcaagagactagttttagtgtcgcgcctaacatcaagcaagccagaagtttgctggcagccggtaagaaggaagccgggattactggtgatttgaagctttctattgttggtgatgatcaagatgtaaccaagaatgttgctcaatatattcagggacagttagattctaaactccccggcgtcaaggttagtatcgccaaccttcctgacaaagctcaacaggcccgccgaagcgaaggcaagtttgatcttgctcagtggtactggttagccgacttcggctatccaatcaattacttgggaatcttgacctccaacaatacaatgaatccgggcaagtttagcgatgccacgtatgattcactgattgaaaaagccaaaaccgccgctaatcagaccgattactggaaatatctcagacaagctgagaagcgattgatgaaccaaaacggcatcattccgctgtattacgtgagagaaagccatttggtcaacccgaaactcagtggcgttgagtatcatgtcgctgggttcccagattatacgcgggcaacgattacgaagtaagttgctgaaaaattgataatcgattttaaaagtaggagtgctagctcgattcagacacaatctgcattgagccaacatttctgaacagaaccccttgaattggatttttccagttcaaggggttctattgatcaaatatattttaaattcatgcgtaattccggtcagagaaccactaccagaaggctctctatgccgaatatatggtgattctagttaaatacatagaccttactttcataaggacgtaattccgtaccttgatcatcactgtaattgctgatgacgagtttgtcggctttaccctgaccataatctcgcgtcaccgtgtcggcagtgaagttactgattactagcaacgtcttgccttgatagtgacgccggtaagcaaagacctctgcgtcatcaggatcaatctcatcatagcttccgaacttaaccaagtcagaatcatgacggagctgaatcagcttttgatagtggtaaaagacggaatctttatcgtccaccacagctttagcattgatttctttataggttgggttcaaagcaaaccatggttttgcatctgagaagccggcatttttgccatcgtcccacggcattggtgtacgagcattatctctagaaatgttagctaaatatttcagcatggttggcccatcgactagcttcttttcttcaaccaactcgtgataggcattgattgattcgagatcttcgtactgatcgatgctggtgtagtgcacattggccataccgagttcttcaccttcaaagacaaatggcgttccttgcatcatgtgaagggtcgtgcccagcattttggcggcgcgaacccggtactttggatcatcgttggcgaagcgcgaaactgcccgcggttgatcatggttgttccagtagagactattccaaccctttccatctaaggctttttgccaacgggatagggcattcttcaactctggtagcttgaccggctgatcgttccatttgcccaagcgtttgtctggattgggttccaaggcaacgtgttggaattgaaagaccatgttcagttcatggctatcgaggccagtgtagttgatggcatcttcgggctttgaactcggcatttcaccaaccgtcatgacatcgtagtgggaaagtaccttttcgttcatttcgtggagatagtcgtttaacttaggaccatcggcaaccagaccttctgtgagcgggtaggtgcctggctcaggtgcgtccggcaggccttcaggtttggaaatcaggttgatgacgtccattctgaagccatcaattcctttatccaaccagaatcgcatgatgtcccaaacggattcccgaacggctgggttttcccaattcaaatcaggttggccaggggcaaacaagtgcaggtagtactgacctcgttctggaacgtatgtccaagcactgccaccaaaggctgcgtgccagttgtttggttcatgaccgttaactggatcgtgccacatatagtagtcagcgtactggttatccttggattgtttgctttcttggaaccagcggtgttgatcggaagtatggttaaccacgaggtccatcagtaacttcaatccgtgggcatgaacttctttcaacaattcatcgaaatcagccatcgtgccatattccggtaagattttttcgtaatcggcaatgtcgtagccgttatctttgagaggtgattgataaattgggttcaaccaaaggacgtcaacgccaagcttctttaaatagggcaggcgtttgatgatcccatgaagatcaccaatcccatcattgttgctgtcttgaaaactttgtggataaatctggtaaattacggcattttgccaccattttttggtcatattgaattctcctctttctcgtgattatagtttaaccggtttactcagttttgagtggataaagccaactgaaaatgcagcgattactaatgaaaccccgccaaccaagaacattgctggcattgagtgcccaaccattgggaagatgaagaatctgcaaagagatgctgcaatttgcggtaagcagattgaacaattgaagagtcccaggtaagctccttcattttcaccgttcaaagcctctgttaagagtgagaatggttgggtgttcatggtgatataagtgatcccaatcagacagaatggcaaaacgagcagccacttgatgtggatgaagaagatcatgatgaagccaagggcaccagcaagtaggccaaagacataccatgcttttcgatgttctggctttgtccgtgcttgaaccagcaaaccaaagataaccgaagcaacggcctggatgcaggtaaggacgccataccaattaccagcggcttgataaccggctgatgaagggttggatgtgtgccaaacattgagggaaatggcaccggcggcgtaggtccaagaatagagaatggcaaaccatgtaaaaaattggacaattgagatttcccagaagactcggggggcttttttagttaattcccagagactaggctgcttcttttgcttggttaagtcaatattgtgatataaagcatattcttcaggattgtattcgtgaactttggcaatcgtgtaaaacgaggtcagcaacagaacggctgcggccaggtagtaggctaatttaacggtaattggcacttcacctttttgagcgacgtttgaaaggccaatgaatgcaaggaagaatggaaccaggctggcaagaactccaccaaggttggagaaggactgctgccaagaccaagccatatctttttggtcctcgttgaccatgtcaccgatgatcatcttgaagggctgcatacaaacgttggatgaaaggtccataaatagtgtggcaatagcggcaaaccacagtgcggccgccgaaccgtaaccgaatccgaatgaaccggcgttaggaagtaataccaaaacaattgctgcgacgggtgcgccaataaataaatacggcatgcgtcttccaaaacgggtccaagtgcggtcagagtatttaccgattaaaggttgaataaccattccggctaacggtggcaagataaagaaaaatcctaagttattcgggttagcgccaatagtttgaaaaattcgccccatttgtgattgttgaagcgagaatgccatgttaaccccgaaaaaaccaaatgtcattgcaaaaatcgtacttactttcaaacttggcaaatgggatgcaaaacttttaggttcagttttaacgtcaccatttccagcttttacttttgcgtccatagtaattcctcctaaaaagtgagcggatccaggcggttagggatcggagtgtaagtctctttggcagaaagctcagttctggaattttttgtcgaaaacacttatatgtagatctctgcttggataagctatctccgtgaacgctttcgcaacttggccaatagatatatattgcaagaaaacgtttacagcgattataatagcacccaaagaaaacgtttgcaaaccctttatatcaacaacacaaacgattgcgttttactaaaaattaaagcgacgtttactgtgctaaaatggggtgaacaatgtaaaatgcttaacgttaatgatcccattaaagctttacaacgtacatagctttacaacgtacataatagagaggtggcgcaatcatggcagtcacaattaaagatattgccaaacaggcaggtgtctctactgccactgtttcaagggtgttgtctggccagacagcattttactcagaaaagacagcaaaaaaggtaaaaaaaacagccaaaaagcttggctatcaaaaaaatacggctgccgttgaactggttacccgtcgcagcaaggtgatcgcagtcattctcagctcaaccaaatcaaacttttctgatcagattatcaatggtattcagcaagaggcccgtcggcatgatttgaatgtgattatcgtatttgccggcgaaaatgattcccagatggagcggaaagcattggaaaccgtgatcgagcggtcggtaatggggattttgctggtcgccgttaaccttaatccggctaacgaggacttgttactgaatgctaatattccgtttctgttcctgtcaatcaccatcgaaaatcggggattgccgttcattacctccgacgattttcagatcggctatcaagccactaagtatttgattgataagggtcattccaagattggatttgccgctgcagatttagactctgtgaccggtcagttgaggttggatggttatcgtcatgccttggcagacaatgggttaccattgaattcaggttgggttttgggcggtgactttgcctatgaagatggcgttaatgccatgaaacaatatggccgtaagccggaagtgaccgcggtgatcgcgtccagtgacttggccgcaatcggcgtgatgaatcaggcgcgggattatggattaaaaataccggctgacctggctgtgatgagcattgatggtacgaaactttgtggcatcgtgcggccacaattaaccagtgtcactcaggagttcttggagatgggagttcgggggatgcagcagattatcagtccgccagcaaaagccgccaagtcatcctttaccccatttaaaattattcccagacaaagtgtctaggaccgtcgtacaaagcagcaacccgaaactcaacggggttgagtatcatgtcgctgggttcccagattatacgcgggcaacgattacgaagtaagttattttaaaagtttgtaacaaaataagaagcctcagttcaatgcggacgtgtgtctgaatcgaactggggcttcttattttggctataaaggcttgaatgctggatttcaattttatgcgaatagaaattcttagcattactgattaggcgatattctttgaacctcgccgtcgaatgaggatccagccacctgccaagatgatcagtgaaataacgacgaccacgacaaacaaatgttggtaagcttgctgggcaatttggtaaaaggtggctaatttgtcggagtgcgattcggctgcctttgctaataaattccgatagtattcctcaagaggtgtactcagcgacagacgactaaatccgctttggatgatggtcgcataaacggttggcgcaatcgtgaggccaacttgacgactgacagacaaagtcccaagcgcaatcccgttatcggcttggtcggcgaattgggccatcaaaacggaaagctgggcgcccatcagcatgccgaatccaaagccagccaacgttgaggtagctaagaaccaaccgtctgctggacttaagaaggcaatcatggcaaacccgactgctgctttcctgtcccccatatttccgatcctccacatgaatgttttacttcgtgagtgacgtcgtgtcacataaccaacatctgaattatagcgcgtcgatgacacggtgtcactatcgttgctcaataaaagcttttttgggatgtcagaacatttatcttgtgggcttaaattgaccccgattcaaataatcatgttagaatccttttgtaagctcttacattgaatatattgttgctaagaacaaagacacagtatcgatagtacagggaggttaccttatgaaaattacaacagcggttgcccagaaacagggtgcaaatttaacaattgaatctgcagagttggactcgcctaaagcaaatgaagttttagtggagataaaagcaacaggcatttgccacactgatgctgctggtagagactatgccacgacaccgtacccggttgcgcttggtcatgaaggtgcaggaattgtcaaagaagtcggtagcggtgtcagtactgtcaagccaggtgatcacgtggtcttatcgttttcgtattgtggtcattgtgaaaattgtttgactgggcatccagccagttgcattcactttaacgaactcaatgctggtggtcgtaattttgacggtactcatcgtattcatagtgaaggtggtaaagatatttccacattttttggacaatcatcattttccacttattcggttgttgatgaacatggtgttactaaagtgccaagcgatgtcgatattagtttgcttggtccattgggatgtggatttcaaactggagctggaacggttttgaatgccttgaaacctaaatttggtagttctattgctatttttgggactggcgctgttgggttggctgcaatgatggctgctaaaatgattggaatggatcatattattgcgatagatatccatgataatcgattggagcttgcaaaagaacttggcgcaaccgaaaccatcaatagtcagaagcggaatccagaggatgtagttaaggaattattgcaaactggagtggagtatagtattgataccactggtgtttctccagttatcaaacaagctgttcacgtcttaaaaccatctggtacttgtgcgttaattggtttggcaggcgatgtgactttcaatattcaaggagaagtgatcggtgaggcaaaacaaattattggtatcatcgaaggcgacgccatcccacaattatttattcccaaactggtcaactactacaaaaagggcttattcccatttgacagactggtaaaatattataagtttgccgatatcaatcaagcctttgaagactcagccgacggcagtgtcatcaaaccgatcgtaaaaattggcaactaaaaaatagaaacgctggctcaatctggattaaaatccacactgaaccagcgtttctatttttgcagaagattatctttcccaaccacacaaccgataaccatggctgcgggcccaatgcttggtcacgtggcgcttgtaaccggcgttactcaggcctcggcaagtctttgagtagtgatatcgtttgccgtggtttgacgcgatccagacataggtggttctggccgaaacttcttggggcggaattgacattaatccgccgcccatcgtgaatgctgcaacaactgtcaaagttgctttcttaagctttaacatgatgtttcccccgaaatataaaatatgtgaataatagcacaaaaatagtttaccataaattatcaggtattaatatcacaatattaatatttctataagggaaattgctaatcatcttgcatgatcttgcgaattcgtccctgcaagttcggcacgacgtccgtcaaaaaccagggatgctgcttcatccaaccatagttcaatggtgagggatggaccaaaggaaaatagtccggcaaatagtcttcgaagtggcgaactttttcagttaagtttctttggcgccgatttcctagataatatttttgggcatattggccaattaataatttcagtttgatattgggcatctgggctaataggggcggatgccatttttgagcgaagccttttcgcggtggcaaatccccgtgggcaccttttccgggataataaaagtccagtggcatgacggcaattttgcctgaatgataaaattctgtcttgtttaatcccatccagtcccgcagccggtcgccactcgggtcgtcccaaaagaccatcgatgcttgggccttgcgactgggtgcctggctgatgattaagatttctgcttggggatcaacgtggaacaacggctgaatgccttgtttggtgaacgactgattttgggggtcgtcttgaatctgcctaaataattccgcaactgtggccatgagatcacctcgttctgacttttaccttcattttccaccaaatgattatcctgtcaaagcaaattcaccattaacaaggagcaatggcgtaaaataaccttagttaacagaatccgaagggggaaggggcaaatgggccaaaagacaatctattttctctgcactggtaattcctgcagaagccaaatggcggaaggttttggcaaacaatatttgggtgaccactatcgggtgttctcggctggaattgaaaagcacggcgtcaacccaatggctgttcaagtcatggccgaagctggtgtggatatttctagccaaacctccaagctgattgacccgacaattttaaaccacgctgacttggtggttacgctgtgcagtgatgccgagaaacgttgtccgataacgccaccgcaagtcgcccgtcaacattggccttttcctgatccggccgctgcaaccggcagttccagtgaacaattacaggtttttcgagaagttcgcgacgccatcaaggcgcggataattgactttgccaatcttgaggccgaccaaaaaaatcattagtttaggcactgttatatcagccgttcacgccaccgaccccaaaaatgtccttgcaatctgcataatcgatgctaatattagtattaaattaaaacattaagcgatgatgagaagagtagcaagtatcctttggtaaagagagccgcgtttggtgagaggcggtcaaagtcaatcttgtgaagatgagctcagagcattaggcacgtgcaagcgatgcctacgttaagacacgttacgatctcagacttaattaaccaatttggttaacgagttgtgaaggtggccgattgtgaaattgaccataaaactgggtggcaccacgtgtttacgtccctgcagtatttgactgcaggggcgtttttttgttgggacaaatgaaatccagtcatttgtctccggagtgctcttacatcatccaaggaggttcaaacaatgttagcagcagaaaaaattgaggtcaataaagacggtacacggcgggggttatccaacctggccgtacaaatgattgcctttggcggttcgattggtaccggcctgtttctcggtgctggtagtacgattcatcgaaccggaccatcaatcatcttggtctacctggtcatcggcatcttcttctttttgatgatgagggcgattggcgagatgatgtattccgatcctgagcagcataccttcgtttcgtttattggcaaatacgtcaacgaacgcttgggcaaatttgcggcatggagctactggctggaacttatcctagccggaatggccgaacttacagcaatttcaacctatgtcaaatattggttccctgatgttccggcaccattaatacaagtcgcattcctggtgatcttgagtggggtcaatttggcgatggtcagttcctttggcaggtctgaaacctttctatcaggaatcaaagtcattgcgatcttagccctgattgtcatcggcgtctatctggtctttacccatcatcaaaatcccgccggcacccacgcctcttgggtcaacttgaccgatggtttcacaatgtttccaaatgggattcatcaattcatcatggcctttccaatggtcttcttcgcctttcagggaatggagtttgtcggcatcaccaccgcagaaaccaagaaccctcggcgggtattgcccaaagcagttaaccaaatcatcgctagaattttgctcttctacattggttcattaatcattatcatggcgatcaccccatggaagaacttgaatcccaatcaaagtccgttcgtccaaatctttaacctggctggaattcccggcgcctcagcggtgatcaacctggtggtaatcgctgccgccatgtcgactttaaacagcgccattttttccaccggccggcatttgtatcagctggctcaagagtctatgctaaagaaatgaaggcgttccaaaaggtttccaagagcggcatcccgattgtcagcgtcctcttttcggcagggatgatgcttttggcacccgtaattagttcctttaactcgcttggtgcggccttttcattcattgcctcagtttccagcgatatttacattctggtgtgcatgctgacaatggttgcccattggaagtatcgtcattccaaggactttcgaccggatggctttaagatgcccaaatatcgttggtccaatccattaacgattgcctttttcatcgccatttttgccagcctgttcttcagtcatgattcactgttgccggcagtcggtgcggtcatctgggccttggtattctacgcggtcttgcggcggcggaataccgagaatttgggcgttgaagacagcagtgactgattttgaatagaccggcgattcagcttcctgtatgatggacttaacagataaggaggatgaaatcgtgaaaaatgtttactttgaccatgacggtaacgtcgatgatttggtgtcgttattactcttgctgcaaatgcccgaagtcaatttgattggcgtgggggtgattgacgctgacggctacattgaaggatcggttccagcttcacgaaagattatcacccgattcggcaacggcgctcaggtgtcagttgcggcttccaactctcgcgctgttcatcaatttcctaaagaatggcggctcagctcgttttccttcgatgctttcccgctgctcaacgaacacggcggaccaaccacgccgttggctgagaaaccagctcacttggatatgattgacaagcttaagcaggctgacggcaaaactgacttggtgatgaccgggccattgactgatttggcaagggcgcttgaagtcgaccccacgattgttgataacatccagcggctatactggatgggtggcacgatgcggacagaaggcaatgttttggagcctaagcacgatgggaccgctgaatggaatgcttattgggatcctgaggccgttaaggcagtctttgatgccgatatcgatatccaaatggttggactggaaagcaccaatcaagtgccattaaatgccgacgtccagcagcactgggccagcttgcggcgttacccgatgatggacctgatcggtcaaggttacgcattggtatcatcttatgaagctaactcaacctactacctgtgggatgtgttgacgacggtggccagtcagtaccctgatttgattcagtcaaaggacattcatggtgatgttttgaccacaggtgccggagcaggtcgcacgtttgagactgataacggacggccaattaaccttgtgaccgaagttgacggccaggccttttatgataaatttgatgaattactgactcagggtcattaaaaattgcaaatgtgaatagatgaacaatcgcctccaatatggtagactcagcgtagagaacgttggcttatcaagttggaggcgattttatgtcggcacttaaaatgaaggagattaaggtaattgccaatattggcgcgggaaccatggggcatgccacggccctgcaatttgcgatgaatggttatccagttaatctcctggatatgaatcaagcggctttaaatcatgggatggatttgattgaacacgatctagccacttttgaagaaaacggactaattaaaggcaaccagaaggcggatattttggcacggattgtgccgaccaccgattattctgacgccttggcagatgcagatttcgtgattgaatcagttgtggaaaagttagccgtgaaaaagaccgtttggcagaaagttgaacactatgtttccgaagatgccattatggcgaccaacacttcgggacttagtccaactaccattcaagctgatctaaagcggccggagaacttggtggtgactcatttctggaacccagcacagttaatgccgttggtagaagttgttccaggtgagcagacgtcagaagtgacggtcaagaccgcaacggctttaatgaaccacattggtaaacacgcagtcgccctgaagaaggaatcgctgggatttgttggcaatcgaattcagatggcggttttgcgggaagccttcaagattgtcgatgatggcattgccagtccggaagcggttgatgacatcatcaaatacagtttgggccgtcgttggagcctggtcgggccaatcgccagtgcagatttgggtggtttagatgtttttgaaaatatcagcagttacctctacgatgatttggccaataataccggcactgatccagtcttgaagaaactggtggacgctgggaacctgggattgaagtctggccagggattctacaattgggaaggtgatatgggtaaggaagccattgccaatcgagatcaggccttatggcaattgttggcggaggatcaaaagaagcgctaagagatgttacacgtgaaacaaccaagtggcaggggaaatggttgaaccctgccatgcttgaagcttcaaaattcctcaagaaccaaaaatggcatctatttctatgatttagaaataggtgcctacttaatgctatctaacttgactttcattttcattgtcctttagtaactgagttccaaaagagtcggttgctttcactggtttgcagattgccggcatcttgaaccttcttggtaaatacacgttccaacatcttcttcaaagttttcttcatattacatgccctccctgtgttcaattctaagagtcattaatggtgtgatatcaaggattcaatttagttgattgagacacttttctttgactccacctttagtatagggcataaaatattacatttgaaatgttttgctcatgaatttgtaaattagttcatgaaagtgaaatgtatgcgtttacattagcccaagcgattcattgaaaaattttacgattcagggcagggtggggtccttttaacatcgttgtcagtttgtgggcagcctgggatcggcaaagaaaaagcacaacgccatctgcgctgtgccaagtgcccccacacttgtaatgaactaaatgctctaaacttgattcgatacatatctcttggatgatccccaataacgtttgagcgatactccccggctgatagctgttaagccatcgcttgtgatccgtgggacgagtgatgattgccccgttcacagagctattgtacgataatgtgaagaaatatacaagaagaatttgaatgaatagtccatggtcagcataagcgacgctctattactgtgggttgctaaatgcccagtttccaagaagtgataatttccataatcgccatcacgaccatggttgcgccgaagatctgtagtaataccagaattgtgccaaatggattaaatgccagcaggatgccaaccaggatcagtaacacaccatacaacacaaagggcattggtgaaacgttgacgtactgacgatgattgagcgcggtgaagacgttggaaatgcctgtgacgatcaggacgatccccaagataaatggcaaaaatgacaagagtggttctgccaataagaagacgatgacggcaacgattaactgagtaatgccgaccgccagactatagtcgaccacttcgttatttcgccgctgccgccaagcagaaattaaattgatcaccccaaagacaatgaagaaagccgcaattaaattaatggcgatattcaacgtgtcgtgtgggtcaaacaggaacagcaggccgaagactatgtaagcgatacttttcagccaaatataatttttaatctgattaatgaatgaatacatctgaattccccctcaagactcatattacctatataatactagtaataagtttaaaacgacagtctcgaggtgcgtgatgcaatatcctaacgttcatttagccaaattcatcgaccgacccaaccgattcatctctcattgtcgactgatcgaaactggtgaagtcgtgaccgttcacgtgaaaaataccggccggacaaccattctccaacctggggtgacgacagcgctggtgcataatgacaatcctaaccgcaagacagcctacgatctggtggccgccaagaagtacgatcgccaatggattaacattgactctcaggcgcccaataaagtggttaaatcagggttaatcagcaattacattcaactgccgggaatcgaatcgattgcgaccgttaacccggagacgacctatttggactcccggttggatttttccggaaccggcaatttgggccaacgattcttcctggaagtcaaaggggtgaccttggccaatcaggggatcgctgcattcccggatgcgcccaccacccgtgggttaaagcacgtgttgaccctggaaaaggcggctcaggctggatatttcgcctatttattatttgtcatccaaatgaaaaatattcataaaatgaccattgaccgtgatatttttaatgacctggcggtggcaattgcaaaggcgcaaaaaaatggcgttcacgtcctggcctatgactgtcaggtcgaaccgggatccttaacgttggaccagccaattccatttgatttggaccaaccatttgtcagtgatgggctgccgtcatcaattggtcatatttgaaagattggcggttcttagttcaaattcccttgaatgtctcgccagtcgtgttattatgataggcgcattggtgcgagtgcggcattgttgatcgcacatacttgatttatttggaaggaagcaattttacacacaatggtaagtaaaacattgatcttcggccaccgaggctatccccatatgttccccgagaattctttgaagggctttgcgtacgcgattgatcacggcatcgatggtttggaatttgatgtccatttaactaaggataacgttccggtgattatgcatgatgaaaagatcgatcgaaccacggatggaaccggcgagattcgctcatataccttaaagcagctccgtgagttccatttgagtgatggtgagacggttccaatgctcaaagagttattgacgctggcaaatggccaaccggttcatctgaacttggagttcaagaccaacgaaatccactatgacaatattgaacagatcgtcctggacatggtgaagcaatatgacctggtctatccggtcatctactcatcatttaacctcgactccctcaaaattgcttacaagcttgatccgactcagcagtattgctacctgtcggaagaagatattaaaaatccccgtgagttgatggcaaaggaacacttggtgggcttgcatttgagtcactacgtcccaatgcgccacgtgaaggaacggatctggaccgttgatgaccctaaggtgcaaaagcatctattcggactcaacgttgccggtattttcaccaataactttgaaggtgctgaaaaaattaaagcaaacgtcactgcttaatctgatcattttacctgcatttccatgacactgagtgttgtggggatgctttttttcttgtcttggatccgtgagccaactgttcagaaaatcactgttttcgtgctaaaatcgattcatagagcaccatgaggacactgagggggatggatgagatgagtaaatggattcgcagatttttagttggttttgtggccttattttcactggctttgtttaattcagcagccgcttcgaccgtcgatgccttcgggacgatttttgaaaatatgattatggcgaaccgaatgaaaccgacggccctgaaagccaattcgaccgcgagcttcgatattgtcatgaagccacaggactcgacggcttattatcaaaaggcgttggatgtcaatgatccaaccaaggctgattttaagaattatctgagcacttcggatattcgccagcagtttggccagcctgatgccgtcatcaatgggtgggttgccttgtttaaaaagaatcatctgaccactcacgtctaccaggatggattggtgttgaatgtgcaggggaagaccaaggatgtgaatcgcttgttcaaaacgaatttgagcgatgccacctatcactcggacccgctccaatttggtaaatccaaacccaacattcccgccaacctgcaagactccgttctggcagtgatgggaatggccgatcataacaagaaattctggttcccggattctgacgttacctttaagagtactcccaaagcgactaaggcactggctgataaaaatgccggctataccagtcattttacaaaaacctatggcgttgaccagctttacgatcacggcctgacaggcaagggccagacgattggcctggtttcttttggcaatgtccaaaccagtgacctcacgcacttttggcggcatgaacatgtaaatgcatccaagtcccggttccaaatggtgaaagttcttggtgataattatcggaaagatattaaatcgaccagcgacggagaagccacgatggatgctgaatatgccggatctgtggcgcctgaagccaacattaaaatgtttaacagcggttctgtgattccaacgttaatcaatcttattaatacttacttaacggcctacgacgatggcagtgtcaaccagatttccagcagttgggggatgggacccaacaactacttccagattttggagaaaatgaatttattgccatcccaatatgttgaggtgttgaacctggtgcttgcacaatcggcactccaggggatttccaattttgtggcttccggtgacagcggcgccttgaactacaccgtggtcggcattcatggaaatgatgttttgttggaccggaaaatcagtgacgccgatccgtataccactagtccttggatcacctcggccggcggaaccagcttaccgtttaagcagtccgttgctccaaacggcaaatcaattggcacaatctccaaccaaaagcaacgagcttggggcagcgattattggtggccgttccttcaggttaacgatgattacctgctgacaatgcctgaattcttcaacgacattagtgacggcggtggcggcgggttcagtcacgtctaccagacgccggcctatcaagaaggcgttcccggtgtgaatacctttaatgcccgcgagtatctgtcgcaattaagtggcccagtctataacgcaccactagtttccggaactgatgatggcagaaactacccggatatctcagcgaatgcagatgcgactaccggttacttcacgtatcaaaagacgagcacctctaatggctgggagataagcgggggaaccagcattgtttcaccacagtttgcgggggtggcagcgttgattaacagtcaagctgaccattcgcgaatgggtttctggaatccacagctgtatcaactggcaaccaaatcggattcaccactgcaaccactgaacgacactgagaataattcaaatctgtattatactggtcaacccaatactgtttataatcaagcgagcgggttggggaccgttgactttgcaaagttgatggatgtttacaagtgatgtaattgatagtgatataaaaagtgcaaaccgaaaacgcggtttgaacttttttgtgctctaagacggtgacggatgaagctctattcttcgtcagggctatatttcaaaatatctccaggttggcagtccaacgctttacagagtttctcaagggtactgaatcggattgctttacccttacccgtttttaagatggaaacattggtgggagtaatgcccactttcttggctagttcaccagtcgaaatatttctttcggccatgacaacattaagggtaattttgatcaattatattcccccttccttaaacagtgaggtcgttttcttgcttaatattcattgccattctaaacaacgtgtagattaatgcgataaataccagcataaccgcatcatccagcaaattttcccacgtattattaaatataccgttattgactcggcctaagaatgactgggtcatttgatttccgatcgcaagaaagacatctgagcagattgcgatcatttgggcatgaacgattctgcggagcattgctaaattatcagccacaaagtattgctttttccccaagttatgactgattcgaataaatgctgaaaaggcaaacagggcagagaggatggctaagaaaattccaatcgccattaagaccgagtatgggagaattgggaaatgggcaacagcgctgtgagttacttgggtgtgtccggaaacaattaagaaatcaccattgttggcaatcattttcataatattggcatgggtgaatccgttatacaagtaaataaacggcgtaatgaaactgaagcagacaacaacgaaggcgatctgcatcaggacggaaacgtcaccaatactgcgatctaataattttgacatggatatcagcctctctcttttaatctggattaattaactgtatcgaatatatcatatcgataaacgaatatcaatatctatttctcgataaaatatatttgaaattcattttaatttattcgacggtcaatatatgaatatcaaaaaatggctggcaggttggattttgagtggctaatatgtggttataccacaaccaatttgatcttatacaaagtcaaaatgaaatttttacattcattatcatttttttactttcaatttacattaacgaaactggcaatttacattgaaccctcacaataaatcttgtaacgaaataaatgattttgaggtgagataattgtcaattactttaagaaacgtccgcaaagattatgatgcgcagacagaagtcctaaaagatatttcggtgaaagtcgaaactggcgagttcttcgtcatcgttggcccatccggatgtggtaaaagtacgctacttagaatgatcgccggattaacaccgattaccgccggcgaagtcagtatcaatgacaaggtcgttaatgacttgccgccaaaggctcggaaattaacgatggtctttcaaaattatgcccttttcccatttatgaatgtccgagataacgttgcgtttggtttgaaggcccgcaaaatggaccaggcagacattaagcagcgggtcgatgaagctttaaagatggttaacttaactgaactcgcgaaccgcaaaccccgtgagttatccggtggtcaacgacagcgagtggcattagcccgggcggttgccagtgatgccaagatttgtctgatggatgaaccactatccaacttggacgcccaactgagaattaagatgcgccaagaaatttatgccctacaacgcaaactgggtctgacactgatttatgtcacccatgatcaagttgaagcaatgaccatggccgaccacatcatggtcctgaatgacaaacacgttcaacagattggaactcccagtgagatttatcaaaacccggcaaatgattttgttgccaagttcttcggtaccccacagattaacattctgaatgcccagcgttcgcaaaccgatagccatgttttgaatgtttcttctgatttggaaattgctttggatgaagaagttcccgctgaaaatgtgaagattggcattcgtcctgacgatatgaaagctgaggcagctgagagtgttgaagccaacgccaccgttaagaacaccgaattcttaggggacgaaactattatctacgccaccttgaatagtggcgaagacattcacgtcgttgtccctggccaagtcaattaccgaattttccagccaattaaagtttccgctgattccaacctgatgtttttttatacagaaggcaagcgaatgaacctttcaaaggaggcctatgttcatgcttaaatctccagcacaaagcacaccgacaagcccggtttcggttgagaaaaccaaaagtaagcttgctgaacaggaagctaagttcacattaaatgccaaggataagtactttgcctgggcatttctgggaccgtcacttttgatcttgggcgttttcattttctacccaatggttaagacactttatctgagtttgttcctcaccaacacggttggtaagccaacggtgttcgttgggatttccaattatatcaatttattgacttcggctgattatctatccagccttggggtcacgttattctacgttttcgcggtgaccattatcacgatcgctttgggattggttctcgcaaacctggctagcaaacggctgccgggaattggcctttttcgaacactattttcggcaactatgggagtttccgtttccgttgccgccatcttctggctatttatttttaacccatcaactggattcctttctctggtcagcacttggatgcatctaccacaaattccttggttgactgatccaactgctgcaatgtgggcggtcatcatcaccaccgtttggatgaacctgggctttaccttcttgattttgctaggtgccatgtcatctgtaccaacgactttgtacgaagccgccaacattgaaggcgcctcatcaagatttcagttcttccacatcacaatcccatccatttcgccaaccctgttctttgtttccatcattactttgatcgaatcatttaagagctttgggttgattgacctgatgactaaaggtgggccgaccaacgctactaacatgttggtttatcgaatttacaaggacgcgttttacagcggtaactatgcacaagccagtgccgaatcgatcatcttaacgatcatcattgcgctgtttacgctcctgcaatttaaagttttggaaaagcgggtgaattactaatggatcttgtgaccaagccaaaattgtcccggcgaatttgggactacgctttattaacgattctcgcggtgattgttctggcaccgtttctgattggtttgtggaccagtttcctgccaaccatgcagattgcgcagggaaacttcttaagcaccaaggtttccttccagaattacattgatgcctttactcaaacgccaattctcaggtacctgggaaatagtttggtaatttccacggcaaccatgattgcccaactgatcttttgttcgatgagtgcctacgcctttgtgttcctgaaattcaaagggcgcaaattcctctttggcctgttcttggcaaccatgatgctgccatttgaagccgaaattattcccaacttccagactgttaaagcaatggggctgctcaacagttactccgttatggtgattccatttctgacatcggcattcggggtcttcatgctccgtcaatcatttatgcagatgccgattgaacttaaagaagccgccgatattgaaggcttgggccacttccagttctattggaaaatggtcctgccttacaaccgaattccactgatgacattaggtgcctacagttttctgggtgcctggaaccaatatctgtggccaatgctgacgactttcagcaatgatttccgaccagtccagaacggattgcgccaacttcagtcagaagaaacctttaacgactggggcatgattcaagccacagctgcaatcgttgtgattcccacgctgattgtgctgttcatcggtcagcattacttcaaatctggtgtgaatgaaggtgcggttaaataatgaaaaaagtaacagcatttctcaaaacttacgcactgccaatctttgcgatctttgcaattgttctggggatcgcctttgtgaatggctccaagaacgcaagcagtgccaaagccggacgaattccagtcgtcttctggcacgaaatgggcggtccagctgagcaagctttggataagatggttgatgatttcaacaagtctcaggacaaatacgaagtcattccccaataccaaggtgcctacgatgaggccgttcaaaagattattcaaagccacggaaccagcgcctcgcctgccttgttccagtcgtttgatatttcaactgcccagatgatgcacagtaagtacaccaccccagttcagaaattcatcgatgaagacaactatgacgccagtgacatttcaccagttgcccgttcgttctattctaataagggtactcagctggcgatgccgtttaacacttctcaaccagtgttgtactataacgcttcgttgttcaagaagtatggtgtcaccccgccgtccaagtcgccaagctatagtgacgtgacccgggcagccaaggaactgtatgccaaatcccatcacaaggtgaagggcatgaccatggaaatttatggctggctaatggaagaagcccttgccaatgcccacacatcattgattaacaatggtgatggtcacactggcaatccaaccaagattgatttgaataacccgacaactaagaagttcctgacctggatcagagccaacattaaatccggtgacttcgtcaattatggatccggagccagtgccgaaaccaatgaaattgccgccttcctggcaaacaaattagggatcttcgttcaatcatctgcctatatcggccagttgaccaccggtaccaagaacaagctgggaatttcctacttcccacatccggatggtgtgaaggccaatggtgttggaattggtggggctgcgctttggatctcgaatgataaacccgctaagacccaacgcggtgcctgggaattcattaaattcgctgaaacagctaagaatcaagccaactggcaaaaggcaaccggctacttggcattaaacaagaattctcaaaagaccaagactttacaagatttgtacaaaaagattccggctgcccgagttcccggtgaacaactagccagtgccaaacccaacaatactaactctggtattttgatggaaggcatgcagttgacccgtgaattggaagaaactgcgatggaaggcgtctacaatggccagaatattaacagtgccctaaacactgccaacaaggccatgaatgccaacttgaagacgaccaacaaagcggatggcgggtagtttggatttactttttactaaggttcacgactgaatcttaaagggaaagtcgttaagagagttgaagaattgaaaggaagttacccattttgagtactaaaacgttaatttttgggcatcgcggttacccgttcaaattcccagagaattcactaaaaggatttcagtacgctattgatcatggcatcgacggcttagagtttgatgttcacctgacaaaggacaacgtgccggtcatcatgcatgacgaaaaaattaatcgaacaactgatggtaaaggtttaatcaactcatacaccctcaaggagctgcaacagttccacatgcgagatggtgaaaccattccaactttgaagaaccttttggctctggcagttcatcgtccggttcacctgaatttggaatttaagaccaacaagatccactacccaaagattgaacagattgtccttgatctggtcaagcaatacgacctgatgtatccggttatctactcctcatttaacctggattcgctcaaaattgcttaccaaatcgaccccaaccagcagtattgcctgttgtcggatcatgtgattaagaatcctaagtcattaatcgttaaggagcatttggctggactgcatctcagtcattaccaaccattagccaacgttgacgaacggatttggaccgtcgacgatccgcgaacgcaggaaaaattgttggcggatcatgtcgccggcattattactgataactttgaacaggcagtcagaattaagaatcgtgctgtagcaatctagcattaatgtcgacaaaaagagcattcggattaggtttccgaatgctcttttagtgttatttggtgacatacaaacctttgtatccattactcataccggctggattccacacaaatccgtggatgttggttcgccagagctgagttgtggctggctgatacagtggaatgacgccttggtctttcatcaagactttttcggcgtttaccaaatccgcatatcgcttggtgcggttatttgcatcagtggttttggatgcttcaatgtagcgatcatattgtgaattagcccagtgaccattattggttgggttattcttagtcattaagtccaagaaattgattggatcagtgaaatcggcaccccaagaggaaaccaccagatcaaaatcaccgctggttgaccgtgacagcttgctcttagttggcacattgtggatggtaatactcaatcccggtaacttgttgaactgactttgcagatactgggtggtcttcttggattgatcagtatcatcacttagcagtgagaggtgcagtttcttcaccccagtctgcttgaggccggctgcccagagtttcttggcttggctttggttgtaggcaacccctgatttttcataggcgtcactggcaaagtcggcaccagtcttaggattctggaagaagttggtggagacgaatccctttggtgcggttgacccatcacgcagaacttgggtagccagggattgtttattgataatttgggataaggcttggcgaattttgacgttctttaaggccttgacccgcttttgattcatttcaaggtagatggttgagccgccgacaaactttttgaactcaggccgattcttgtaggatggcacctcctcgccggaaagcgtcacaacatccaacttgttttgctggtaaagcgaaagtccggtgcttggcgttttgacaacttggaacttaagcttgttgagtttaacggcctgcttgtcccaataattaggattgcgcttcatcgtccaggtatcactggttccattccagtcggcgagttcaaacggtccgttgtatgcggttgtggcgctgctggtaccataactgctgccgtacttcttcaccgcggattcctgttgtgggaagaaggttggaaaggcgagcaataatttgaaatatggaactggatggctcaggtgaaccactaaagtcgatttgttgggggctgatacgcccaacttatttggcgatagcttgtttttttgaatggcactgtagttcttgaccccttcaaacaggtaagagtacccggaagcagtctttgggttgactacccgacgccagccatacacgaagtcgtgagcgaccactggttgaccgttattccatttatcattggtccgcagcttgaaagtatatttcaggccatcttttgaaaccttggtgctggtggccagggcattttcaactttggattttggaccaagtcgatagattccctcgccaatttggtaaagtggtgtcaaactgccgctatcagaagctttggcagtgtccagtgtcgagatttctgaatcggtgctgatattgacagtttggtccttggccatctggttgctggaatttttggtgctttggttgccgcatcctgccagcaccaagatgagtgccagcgcgcctgtaattgttagtaaatgttgattgattttcacgttttacccctcttttttgacatgaaaactgccagcacattgatacttgctggtcaggtgatgatacatgaattgagttacttggaatttgttagtgccaaggttgactatattaacatggaatgtggtggggtggcaaatgtggtgtaggaagtgcctgaaatgttacatagttgaaacgtgttttgagcaactgaggctaacttctaagggtactctgactaaagtcccaagaccagggactttaatcagagtacccttagaaaacgcctcacccgttgctcaaaacactctaatcaaattcctcatacacattcggatcctgcccatccactctgccatccggcttagtgagagcgttgatttttttcatttcatcctcagtcagttggaaatcaaagaggtcttgttcgtcctctggtgaattaagctgcttgaacggggcactgggatgatgcctctttgggtatgccactttaagatgatttggccggtattcttattgtactttttggctaactcttgaattaatggttctttcaatgcggcactccctcggcctaatgggctccaagcttcggttgcgatgccgcgctgctggtcctcttttaacatgcgttcattattccaatagggatggacttcaatctgattcaccgctggagtgacgccggtttcgttaatcaatctgtccaaatgttccggctcaaagttggaaacaccaattgaacggatcagactgcgttttttagcatcaatcattgcttgaaatgcttctacgtagtgattacgtttcggcagcggccagtggatcaaatataagtcgaggtaatccaatcccaaacggtagagagattcctggattgccttggttgcttcgtcatattgatgatactttcccggcagtttggaagtcacaaagaactccgaacgggggatcccggaacggcgaatcgcctcgccgaccatgccctcgttatcataattggtggcggtatctaaaccgcgataaccgtcctggatggcagcgagtgtctgctggagaccttcgccaccgcgaatttgaaaagttccaaactgaatcgtggccatcttgtagccgtcgtttaaagtgatttctggaattgcgttatttgtcaatatttgtacctccatgtttaatccttgcgcgacaatttatagttacgaaaaaaggagaactatttttttgtttgctgatcgttattttggggttgagtttttggatgcggcttggttggctgttggtcgacttttttgatcgtgatgtaccagccgacctgcatcgatttgttggggttaatgtattccacgctaaagtcataaaatttggcgtggagacttttttcgatgagcatattttttacctgcagggcatctgcccgactttcaaaccgcagattgctattggtgctgtacccactgtgcttattagggtcattataggtctggttaaaaaagtccaggtattctttggagtcgttcaaggtatcacgtccttccttcttccattgtacccaacatgccactcaatttcattgtccgtggctaattaagtggaaaacctaaaacttttcagatgatatggagaattttgatcaggattgaattgtgtttcacataggaaacctctaaaatatacatatatggcgaggaggggatcgtcttggcgaaaaatggtttgttattggtgaatttgggctcaccagtgtcgcccagtaatgcagatgtgaaagcttatttgaaagaatttttgagtgatcaaaatgtcgtaacgctgccgaagtggttttggcagcctattttgcgtggcatgattctaccgatgcgcacttggcgttcggcaaccttttatcagcacatgtggaccaaagcgggttcaccgctgacggcttacacagaaatcatgaagcaaaaggttcaacaggacttgcctgattgggacgttcaatacgccatgaattatgggcaacccaggattgtcgatgttttgcacgagatgaaagatcgcggtgatcgtgacatcgttgtcttgccgctgtttccggattacacacaaagcacccacgatactattattgaaaaagttcagtcgtcgggagtcgcgactcatattattaagaacttttatgatgagccggtgtaccaacagattttggcccggcaaattgacgaggcttacccaaagaaacagtatgatgcggtgattttcagctaccatggcattccaatgtcgatggtcaaaaaaggtgacccatacgaaggtgagtgtctcgccacgactcagggtgtgatgaaatacgttaaacaggttccgagtgacaaagtcaaaacggtttttcaatctaaatttggaccgatgccgtggctcaaaccttatttgaaaaattatttgatggagttggccgcaatgggtaaacgcaatgtgttactggtgacgccatcattcgttgaagattgtttggaaaccatcgaagaaaataatgttcaaaactatcagaccttcaaggcaagcggcggcaacgtctttgactcagtcaaaccaatgaatggcagcgatgatttttgccaattcttagccgacctcagtgttaaacaacttcggggaggcgaggccgatgagccaagagcaaacgcataaaagccttgatgaaattaatcaaagtgtcgaggttcccagcgtttatgaaacttcatttgtgcaaaagtttcttgcatatagtggccctggagcgttagtcgccgtcgggtacatggatcccggaaattggctgacgtcactttctgggggcagccaatatcggtattcacttttgtcggtgttattgatgtcgattttagtggccatgttcatgcagacattgtcgatcaaattgggcgtcgttgcccggctggatctcgcccaggcaattgcccagaaagtgcctaaagccggtcgctacacgttgtggatcatcaatgagttggcgatgatggcaactgacatgactggcgtcgtcggcacggccatcgcattaaaattattatttggtttaccattgttatatgggattttgttcacgatattcgatgtattgttagtgctattatttttaagatttggaatcagaagaatcgaatttattgtgttaacggccattttaattgttggtgtcatctttggagttgaggtatcacgggcaacgcccaatctggcccaaattgctggtggcctgctgccgacacccaagattttgactaatcatgaaatgctgattatgagtttggggattgttggggcgacgatcatgccgcataacgtttatctccattcttcactcgctcagagtcgccggtatgattaccataatcccgcccaggttaatgaagctttgagatttgccaaatgggattccaatgttcatttggtggccgcctttttgattaatgccttgttgttagtccttggcggaacgctatttttccacacgaacgggcagttgtcggcctttcaggatgtttacaacggcttgaagaattcggcaatcgttggcaaccttgccagcccgttgatgagcaccttgtttgcgtttgcgttattgatcactgggatgatttcttcaatcaccagtacgttatccgggcaaattgtgatggaaggctatcttcatattcgtctgccactttgggagcgtcggttactgacccggtttgttaccctgattccgattttagcaatcgggtttctggttggatttaacgatcacgattttgaacaaattatcgtctatgcccaaattgcgttatcgattgccttgccattcacactgttcccgatggtcgccttgaccagtaaccatgatttgatgggggttcacaccaaccagcggtatgtgacgatgattggctacctgctgacgacgatcattaccgttttgaatttgcagtttgtgattgctgatttttaatcaatgtatttagaatatttaagagataagggggagttggattgaaaatacttggcattttagggtctcatagaaatgacggcgcaacggacatgatgctggaaaccgtgctgtctgcggttaaagcgcctaataccactgacatgatctatttggaagactatccattcaagccggatcagggagatcacaaagatccggtgctggatgaacttgaagcaaagatgcttgaaagcgatgtttgggtgattgcagccccgacttattggggtggcctagcagggaagatgaaagacttctttgactgcatgcgccaacgcctggtccgctttgatcatgagggtggtacccatccggaccggttcaagaataagcactatttgagcatcacggattgttataccggaaccttcgagaactgggtaaccggcgtcaccgaccaaagttttcgaaccattgataaggtgatgtcggcggctggtgtgattaaaattcacgaactggtgttgaccaacacttggggaatgaaggcattgcccgagaacaaaaaacaggcctgcctcaaatggggtgcccgcctgaatactgaacaaaagagagatgatagtacattgaaacgatatattgaattattctttatggttgctgtgatggcgttattgacgatgggaattcaagttggtttgcgttttgtttccactgctgatttctggtggcgctacgcttcgtttgtcgtcatcttctatgtgttgttgggatgcatccttcatttctttacggttgtgaaacatcgccgacggtaatttaacttgatactaacatgagagtcagacgcacggcgttttgatctcataatttaatgtaaacaggccatcattcctagttttggaatgatggcctgattgtgttttagccgatcgtttcacgtttattctcgataacagtcggattcaacaagtctaagatgaggtctcagccttaccgattattgtaattttttcttcactttattcagttcctcagcaagtgcaggcctggatggatactcatcgattaagccatcgatccatttgatagcggtttgcacgctgccgaatgcggtatagtttttgattcttcggcccattcgtcgataggcttgtctgccgggatatttttcgttcagaacaacgttttggtaatacagcttgttgacgacatctgggtagttagggtacaggtccttgctataagtttcagtgagttcagggttctgcatgattagctgcatgagcttatcgaattcacgttccttgtctaagatgaaggcatagttttccggtgtcagtttcttcgccgctttagccaggaaagccggatattgggcatcccaactcttatcctgttgtcgcagtttcttgagtggttcgtatgcgtcggggtagtttgcgaacagacggttttcgagaaccgcttcttgtttttgctgctgatcggtagcgtcataaattttgatgagatatcgctcccaaattcgccgccacccctggtcctgttttgaagcctcgaggcacagttcttctgctcgaacatagtttttgttttgaatcgcattttggatttccacttcgcgaatttgcggaatggttttatgctcgtccataaacttctcggcatcggactgctctccaagttgaatcaggatccgagcatgaagcactttatcgtaaatttcagactgagtcgtttcaaatccttcgtcggctgctttgataactgcccgagatgcggattgagcaagcttggcagactttggcgtgatcagcgggagggcattatacaatacctgatagcgttgttcgggccagccggcaaatatttttcgcttaaaaacgcgaaccacgtccttaatgacgatttctttttgtgattccaaaatctcaggggcgatattggtgcttaagttcttcatcgaaccaaagacacgatcaaacgtgtcggttaaggcaccggaactgctgtcggcatcgctgagcattttcgcagccgtttccacgaccaacagcaagccattcattgcatgatgataatggccttgtctgaaccggagcatgtacttattgatcacatcatccaagacattgcaaacaacaatgcagccttggtaatcaataaagccgtaagatttgtttttacggactgtactttgaatcagtttcttggtttgcaccaactcagcatccgtgtcgagatcgccaaattgggcggtcacgtctctaaaaaatgtgggatcgaactgcgcctgattaattatgaattgccgaagcccctcaggagaggcttcgttgacggctttgattaaggattgtttttctccggaattcataattgtttcacgctcctctgacgatatcggaataattcaaatcgatagtaccatagattatgagtggttgctaccgctttcagtaactaagtgctaaatcttaatggacaaggtttgcaggctgaaagattacttcagtccacgggtgtttaaaaggtacccatgtgtggtattatttatatgggagctaaatcccaaattaatgaaaaacattttgcaatcactaggatctggtcggggagaaatctctggccttttttgtttggtttccggtttgcgtgttgcaataccttccattcaagatatataattaaaataatattagagctatctcattttcatataatattcacgagggagatattgccatgaaaaatgttaagaagtggttggtgatcgggacgattagtctgtcgacattggcattcgcagcctgttcgaacaacaaatcatccgagtcccaatccaagcccatttccatgccgacaacttatagtgcgactggaaaggcaagcaaagcagacgatgatagtacgctgaacgctgctgaagtcgttgacgcaccgtttaccgggattacacttgccgtactacaggataacgttgaggattctgatgtctattcaccaggtggtggcgatcagttgtttaaaagcaacaaagattttaagattgtcaagggcggcctggcgaacttgaagctggaccgatcgaataacacggctacgattaccatacggaaaaacgccaagtggtcaaacggcagcccagtaattgccaaggatgttgagtacgcttatgaaatcatcggcaatcaaaatacgggcgctgaacagtactcatctgacatggcaaccattaaaggcatggctgcttatcacactggcaaggcgaaacagattccagggattacctatcctgatggacaaaacggcaagcaagtggtgatccactacacccatttatcccctgcgatgcaatacgccggcaattcattcttatgggggacggtggttccttatcagcacattaagaatgtgaagatttccaagttatcgtcctcacctgcagtccgtaaacacccaattttcgttggaccttacaaactgcaaaaccaggttcaaggtgagtcgactgcttgggtacccaataaatattattggggaccgcagccaaagattaagcacgtcaatatccaagttgtttcctcaagcaatgctgcagcggcgtttaaggcgaaaaagttcgactttgctttgggcggcctgcctgccagtcaatataaatcagttaagaatatcaaaggctacaccctcgctggggcacctggtttaagttatggttactttggcttcaacgttggccactttgacaccaagcccaacaagaatgtcatggataagcacagcaaaatgggtaacaagaacctgcgaaaggccatgctgtacgcagttgacctggacaaggttaacaagaaattattgagtggggttcaatggcggccaaataccttgattccaccaattttcaagaaatatcatgataataaagcagccgggttcccatatgatatggcgaaagctaagaaactgctgaaagacgccggttacaagaagaagggcaagtggtacgtccaacccaacggcaagaaattgaccattcacttcggcgcgatgcaggggtccgctgccagcaacgaaatttctcgatatgaagttcagcagtggcggaaattaggtctgaacgttcaaatgaccaacggccgaccacttgagattaacagcttctattcaatcttgggcaagccaaagcaaaagcagattgacgtcttcgttggcggctggcagttaacttatgaaccaacgccaacccagttctatggtgaagatgccacttataacatgggacactttgtgaccaagaagaacaccaagttactcaacagcttgaatagtaataaagcttggaatcagcagtatcggatcaagcaatttaagaagtggcaggtttatatgaacaaagaagccgcttatgcgcctcaaagcaccttgctgagtttcacgccggttaaccaccgactaaagaactttaagcaggcggcctacaacaactacctcttcccaactttctgggatcaattggaactgacttcgaagactcctaaatagttctgtataaaagtagcgtcatgggatttaacttccatggcgctacttttatgtactggataaaccaaatgcaaaattcactcacaaaaagagaaaccggaaaccaataacgcaaacctaatgtgaaattagggggggcgcaacaaatgctttctggtaaagatagtaaagttttgtatattggatgtagaatcaaaatactttccaagcgaggtgccgcatgataacacaaaataaacctaattgggtcaacaatcccagaaagtggatttggatgctagtgggatttattattatcgagaaatttttggagaatggcatattagttccagtactcctaaaactgccctttggagatcttaccagcaatattttgtacaaagggatcgaagtgttgctagttttggggttaaatatctggctaatcaaacagaagttgtatttctccgttaatgttaccttaaagacaactctctttttcctttttggtattgtctacattagcctgtttatctcatcaggaccggtgaaacttttgcctccaattatactgtggacgttgttgacggtgatttctgaagaactgctctttaggggagtgatttttggggatttattcaaacgcctcactcagcgtcatctgacgaagcgtagcgttgcaattacgattggtttatcaagtctgttgttcagcctacagcatttgagcaatttggcaaatcagtcattgctggatacagtttgtcagatgattgaaacttttgggatggggattttgctggcagcgatttatgtgagaaccggatcattaatcacgacgatttttgcccattttctaattgactttccgattttgtatttaagtcagatcagcactggttctacctctactgcaaatatgtctgggaatgtttcagtggtcggatcgattattgtcgcaatcgtttatgccctggttggaatagttgtcatccgatcaaaattagccaataacaagttaccggcaattacacatactatggaaaatccagcaaattaaaagtcccgatcccgatagtcatcccaatccggcatctttgaatggttctccttggcggttcgaatgtcatgataaaatctgaccttgcgcttgatgtgacgttcgttttttttcaaaagcgccagttgttcaaggacgcgttgatagtggttatccaaaatgtcacaggttttgtccaagtccgcatcgtcgtcttgggcggcaaacagttcctgcaattccttgagtgtcatcccggtatctttgaagcagcaaatcgctcccaggcggttgaggtgctgctgagtataagcccgtcggcccttgatgcgggggatgtcgtaaagtaagcccaggtcttcgtaataacgcaaggtcgtggttggcaagtgatacattttagatacttcggtgatcgaataagttttcacggttgcggttttcaaacagttgacctcccaagtcgaaataagtttacttcaagtatactcgaagtgttacatttaagctaaacaatttaggagatggcgaaatgtatcaagcatccaaagatcgttacgataaaatggtttataaccgggttggcaaaagtggcctcaagattcctgccttgagccttggactctggcataactttggtagtgtcgattcctttgaaaatcaaaaggcgattatccatcaagcttttgatttggggattacctatttcgatttggccaacaactatggcccggaacctgggagtgccgaagagaacttcgggcggattatggcagaagatatgaagccttatcgagatgaaatgatcattgccagcaaagcgggctattacatgtggccgggtccatacggtgaatggggatcacggaagaatattattgccagtgccaatcagagtttgaagcggatgggattggattatgtggatatcttctattctcaccgatttgacccggacacgccactggaagaaacggcccttgccttggatgagttggttcatgaaggtaaagcgctctatatcgggatttccaattatgacggcaaacaaacagaagagattaccaagatcttcaaggatttgaacacgccgtttgtgattcatcaaccccgctacaacatgtttgaccggcacatcgaaaatgatctcttcccggtattgaagaaagaacataaggcagcggtcagctttagttcgctggctcaaggtttactcacggacaaatatttaaatgggattccagctgattcacgggctcacaaatctgccagtccatttcttcatgaagaacaggtcgaagagaccattaagacagttaagaaattgaatcaggtcgctgctgatcgtggccaaactttggctgagatggccttggcttggaatctgcgtgagccggaaattgccagcgttttgattggtgccagtcgaccggaacaactgcttgataacgtgaaggcactggacaatcttgaattttctagtgaagaacttaagaaaattgatgagattttggcgacccaaaagccgattaaataaataagagtggaacgcgaggcgttttgcttaaatggcggggatcagccgatcgttgcacgtttaaacttcataccattggaactcaagagaggccgagatataactgacaatcagttgtatcccggcctcattttgatatacaaattaacttcccattgatggttgacttgaagtgtaaactgctcgatacttcagaacaatattggctttcttttgggtgccaaccgatgaccacttacctttggtcttttggtagacgaactttggtgaagtgccattcaattgaacaaagaactgaccgtcacctgatttacgtacccggtaaacttttgttttgctggttggtgaaagggtcgtttctggatcggtcttgttataagcgacaatactctgtcgaatcatatctttatattggttggtttgatggcttttcatgataatcccgacgatgccggcaatcacaatcagcaccatcagtgacagcatgatccacatgatgttggctcgtttggcgttttgagctttttccttctcattcattctatatcaccccactatttccattggaatcgaaaaaccttacgtgttaaatgtatcacacaaatggccccttgagaaaaatgtggggggatttcttcaacagaacatcaaaaagtagtcccaattttgtgataaatacaaatcattttaaaatagtgttcagttggatgatggcagcacgatttcaaggtgtacaataatcacattattgcaattggaaggaatgacttgatgaacattctgttactgattatcgttggctttatcatcggcaccgttgtgattaccctcggcggtggcggggccgccttttaccttggaattctcacgacggtctttggcttggggccagcaagcgcggccgccacttcattggtgacctcgtttccatcattgttaatcggctcgtactcttattttcgactacacaaaattaaattacggattgcttggcggatgatcatttttgcagtcccagctgtggttgtgggatccttgatctcaccatatatcccggtcaaaatttatttgtatattatcggggggattttggcgattttagggctccagacgttgtttagcagacaaaaggatcaccaaaatcctaataaatggttggcaccagtctatggtgtcatcagtggtctaatggttggtgtcggcgggctcagtggtggtggaccggtggttgccggactgctcgtgatgggatccgacatggtcaccgcggccgccacttcttccttagtcctggtcgtaatgaccgcaaccgggttaatctttcacctttctgccggtaacgttgactggtcggtggggcttggcctcatgtttggggcgattctgggatcatttttggcgccggtcctgttgggcaaactcgatcctcagaagttcaccaaatatgtgaagccgattctgggagttctgttggttgtgatgggtgtctttacggcattaaagtaatggccataaaggtcttgaattaacccatggtgcatgataattgtggataaaaaagacgcaaacctggtttgcaattggtttgcgaacaaaaaccaattcaattacattcagatttcccttgctcatcaccttacgtcatcagctataacagaatcaggaggtgaaaccgatgtcgacatatacaacaggagagtttgccaagttgggtggtgtatcaatcagaaccatccaatactatgatcaaaaaggaatcttgaatccgacaaccatttcagatggcggccgtcgcttatacacggacaaagagttgaaaaccttgcgattgattttattgttgaaatcaatgggcctatctctgacgacgattaaagacctgttatcagaagataattcaactcaagtcctgtcgttgatgcttaaggaataggaaaagaaaattcagcatgagatgacaatgaccgcggatcagctggaaatgatttgcaaggttcaagacagcctggctgattatgcgctaatttcccaacctgaccttgacggcatcgaaaatatgatggaaagcaaaccaaaattaaccaagtttcgctggtggatgttaacttggggactgatgatggatgcactggaaatcttagcaattgccgtttggattatcaccggcaattgggtgccagccgcaatcatcttcccagttgtgattgtaatggccatttggattatccgggattattacaacaaagttgagtatatctgcccaaattgtcaccagcatttcaaaccgagctggcgtgactttacattttccaagcatactgccaagacgcggaaactaacgtgtcccaattgcggttaccgtggctattgcgttgaggtttacgatgtgaatccaaaacaatagttggcaattaatcatgaaaaacataccccttggactctttttgaagtttaaggggtgtgtttagtttgatagggtacttatgctaattaaaaactaggtttaatatacggaacacgtttgattgtcgccccaaccgaactttctgtgatccaattttggtttaccaagggcttaaagttttctgtttttccagtaatgatgatgccagaaaatcttgcttgatttaatgttggatatttcttggcaaatccgtgggcatagtcagtgattgaaaaactattatatgtgccgagatttttagcactttgcaatgattttctgaagcccttatagtcatttggaccaagtttgccattaaatgactgaattccaagaaaacaattatcttcaatcgttggatctgctttaccgttgacaccaagccagaaccaatttgcttggatgcctttcggcagcttttgtagtatttgtgaatatgtcattggatggcgaaaggtcaaagccacctcacctacataatttttcatttgcgaaattttcttaacttcgtaagccttcgacacatttggtgatttaactcgattattgtaaaataacggaatcttggtttgggttgttctcgtgtaagccgcctgattatctgtatccactaagttatcggtttgaatttcatgatataaccaattgtacttaccttcgacagtctgccatggtaaatgatagccatcaatgtctttatattggtggcttacgacagtgccgccgccaatgttactgttaccaataaccaagtcactgttttggatattggggctcatgaggtcttgttgaatttccatctctttcataagcccactagattgacgggcggaaaaagattgagtaattttatatccaactgccgtcattattggaaaaagaataataattaataaaactgtgattacccaacgcttgagtttaatacgaaaagctaatttttcaaattgtttatcttggttcattatgattcaccaaatcccttcttaatcttctttctcaaccgatacaaacgcattttcactcctggagaggttatctttagattggtggcaatttcatcaatagattgaccttcgatgtatttcatttttaagatttcttgatcaccaggagataacttttggataattcgctgtagtttttttgatttgtcttctgtgtgtggttccctcgtttgcttctgctgcggaataaggtattgttgtaaaattttctgaagacgggcttcacgacgatttaaatcaatgtatttcgttttggcaattttgtacatataagggcgaatcttatctggcgggagtattagatccatttccaaaacttttacaaagacatcttgaacaacgtcttctgcgatgtctttactagctccgcgtgaaaccaggaaatgatttaattcgattgagatgtttttcagtagtacctcatactcatcaagtttcatgacaaccccctttcactgtatataacgaacgggattcgaataagtaacgataattactcaattatgtaaaaagagccagacaagaatgtccagctcaacgactataatttattcatgttccaaaatctgattcatcgcgctgtcggcactactcttatacattgtgccgaatttattggtgtgaaccatcaagtaatacagccgataaaagttcagccgttcattggcgcccggatccaaagggtagactgcgttataagcggcgtagaagtccgcgtcaaagccaccaaagacggtggtaatccccaggtcgaattcccgatcaccatagaaagaagcgggatcaatcaatgccggacgaccgtccgccaagaacatgtagttgccgccccacaaatcgccgtgaagcagggatggctcgctctcatgcttcgacaactgatcgagaatcacttggcgaacccgtttgtatttttcatcgtcacttggattccataaatgctttttcatcaaagcatcgcggagccggtccagtcggtggttgacgaataattcactccaagagtcggtccaactgttatcgaagctttcatcgttgctgacatagggcaggtcaaagccaaattttccattcttgctgtaatgctgatgcaagttggcaaccagttcacctaagtcactctgactgccggaacctgattccaaaaagttcagcagcaaataagcatcgccgttaatttgaccattgcccaacactcggggagccaagacgttagcttcctcgaaagctttgagcccagcaatctcgccagcgtaaaagtcggcagtcgtctggggctgaaccagtaggaaatatgtgtcatcttttgtttctaatcgaaatgcctgattaacatcgccggcaccaacggggactgctttagtaatccctttgatgggcagttgtgatagccattgatcatccattgaatcatcacctctgggttcattgtaactgaaaattgaattttatgtaggctggaattgcgatgggggtcaaatcgggttaccattaaatcaaatcatatcgtcgattaagcaaatttgctggaaaggagctgcaaatgaattacttacaagttgccaagccgttggtgttacccaacggtcagcaggtcaaaaatcgattctttaaatcggccatgagtgaaacaatggctaaccaagatcatcagccagatgaacgatatgccaccttgtatcgagcatgggcaatgggtggttctggaattgtggtaactggtaacgtcatggtcgattcaaccgccttggcagaacccggcaacgtggtcgttgaggatgagcggagcttggcaacccttcaaaagtgggctcaagcgggaacgacaaaccacacccagttgtggatgcagctcaatcatcccggcaaacagtcaccaaaatatttgtccactcaaccagctgggcccagtgccattcctgtacatggccctaatcagaaatattttaatcccccacgtgaattgaagaattctgaaattcatgagattatcgctaaatacattcgaaccgcagagattgcccaagaagccggcttctccggtgtccaaattcacggtgcgtacggttatttggttaatcagttcttgtctcgcaaagacaaccagcggacagatgaatttggcgactcactggagaatcgaatgcgatttctcgtagatatctatgaagggattcgcgaatcatgtgggccccagttttcgattgggctaaagctcagcgtgcttgaccttgatttggaaggattcaccgaacacgattcgattgccgtgatccaaaagatggccgaccttggcatcgacttgattgaaatctctggtgatgattacgaaaactcaaccgttggcttttccggctatgcccatatgatccatcaacttacagatgtccccattgtgctcagtggcgggtttagacgaatttccacgatggaagaggcgctgggaacccacgacgccgacatgatcggaatgtgtacaccaatggcggtaatgccggacctgcctaatcaaattttagctggcagctaccaaccagttccactaccactaacgatggggagtcggaagttggatgagaagtattcgccaacattcattaccgcgtattgtgaacaacaggcgcgtcggctggcagaggggaaacgaccacagctatacacgagtgcctggcgcgccttggcggcaagcattcaaatgcacgggccaaatggacttacacctcgccgtgctcaataaataattgaagattggaagaaattcatgtcacaaccatttgaaccaaattcattagatgaactaaaagatcagtatgacgtcattgtcatcggctctggtagtgctggcctcaccagtgccattcgggcaaccgaactcggattgaaaccagtgatttttgaaaaaatgccgagtgttggcggtgatactaaacgggcctcgtcggggatgaacgccgcggcaacctttgttcagactgagcatggaatcgaagatagcgttggggccttttattacgagacgttgcgtggcggtcatggccaaaacgatccagcgttattgaagaattttaccgagcatggtgcgcgggcaatcgagtggctttataaacagggtgtccagctggatgatttgacaattaccggtggcatgagtgtgccccgggcgcatcgaccaagttcgactcaaccaattggtggttacttgattaatggtctgctaagccaagttcaggcaaaacagattccactgttcaccaacgtcaaagtgactgaaatcctgcacgatgatcgggtttccggcgttcaaattcaaacagaaaacggttcgcaaactgttcacgccaaagcagtgattattgccgctggcgggtttggtgccaacaagtcactcattgcaaagtatcgcccggatcttaccaaatacaagacaaccaaccagcctggaaataccggtgatggcatgttgctggcagagcatctgggtgcccagctggttgatatggatcgaattcaaattcaccccaccgttcaacaggatacggaccacgtctatttaatcggtgaaacggtccgtggcgagggcgctatcttagttgatcaaaacggaaagcggtttgtgaatgaaatggaaacccgcgacaaagttaccaacacaatcgagaagttgggtggtactggcgcatacctcatctttgatgccaaggttcgcaaacgtgccaaggcaattgacttctatgatcatgttggcttggttaagacaggcgatgatttagccaaacttggtaaactgattggtgttgatagtgatacactatcgcaaaccgtagccaagtggaatcaggccgtttccgatcgaatggacattaactttggcagaacgaccggccgccacatccttgaaactgccccatattatgcgattcacattgccccggcgattcattatacaatgggcggtttgaagactaacgatcaaactcaagtgcttaaggcggacggccaaccgattccaggattatatgcggccggagaggtggttggtggcctacatggtgataatcgaattggtggcaactccattgcggaaaccgtcgtatttggtttgcaggcagctcagcaggtacgcgattatatttttgaaatgtgaataaaacgaggggtcattggaatttacccaatggcccctcaactatttttatgttaaatccgttggatcaagaaacaaacttcatcgatctcaaaataatcgattaatctcatcaaattctgctggactcagttgtacatccaacgctttggcattactatcaacttgctctggcaatcttgcaccgggaatcaccacgctaatatcaggattggcaatgtaccaagccaaaatcgtttgagcaatcgttgcctgatgactttcggcgatggttttgacttgatctaaactatccatgatctgattgaattttgatgtagagaacctgctgaacttgtctgcatcgtttcgactgtatttgccagttagcaagcctgaagccagtgggaaataggggacaaaggaaatttggtgtgcctttagatacgggaagatttctgtttctgcatcccggtgaaccaggctgtaattgttctccacgacatcgacttgattgtcttgattggcttccttgatctggttcaaattaaaattagaaatcccgattgcccgaatcttaccggccttttttgcctgggccagcgcgtcaactgcttctgccttcggggtcttgtcatccggaaaatgaatgtaaaaaatgtcgatgtaatcggtttgcagccgttccaacgactcatcaatcgatttggtcaagaacttaggatcgttattaggcttcaagtcgttgttgggatcctgagctgctttcgatgcgatgacaaattttgaacgatcgaaatcttgaatgacgttgccaataatgtcttcagacttgcccaatccatacataaatgcggtatccagtaacgtaatgccgtcgttcaatgccgctttaacaactgcctcgccgtccgaatctttcaggccgtcaaataaattatggccgccgaccttgttggtccccagacccaaggggccgctgacaacctcgctcttaccaattttaactgagttattcaaagtcaattcctccttacatatcaataatgctctgccataaaaatagggctgaaattaaaatatttcaacccaagtgtctatttttcgataattgattattcgtcgtaaggccctttgccgaggtaggcgttaatcatccaaatattcttatcaatgtcttctttaaagccattcagcatatcttgagttggaaaatctttttcctcgtcagtgacctcgatgcccttttgatattgatcacgcaaatacctgaattgatcaaccagccgctgcatgaagtcacgcatggttaattgatcccaggtaaccttttcgtccggtaagccggtgttatcaatgaattcgtgagtggttgcgaacggcgaaccgttgattgcgatcagtcgctcggcaacgttatccaattgatcagctaattgatcactataatcatccatcagcgggtgcaggcgaaagaagttctcaccccgcatgtaccagtgggtttgttggatgttggtctgcagctggctgagatctgcgactaattgattcaattgtgcgcgtgtctttggaaaatcgtacttgtctgccatcagattacctcccagaataattttgaattcgcttacacagtcagtgtactcgattctgggagacggtcgcaaggaagttgccttttagttttcgaaaggcttagtggtcttttggtccactgacagtcggtgcctgtggttggtcaggctccgtcgtttccggagattcttccagtttggaatgcttggatgtctccagcatcctgacgtagacgaggaagctgacaaatgccgctgctgatacataatagaagaaccagtcttcatgaccgatgtgtttgagccacagggcaatgtattcaacacttccaccaaagatcgcaacggtcagcccataaggaaaaccaaccccgagtgcccgaatttcagtcggaaataattctgctttaacgatggcattaattgaagtgtagccactgacgatcagaaggccgcctagcatgagtagaaacgatgccacggggctatcgaaggatttgagtccgagaaagattggaacggtcaaaattgttccaccaatcccgaaccagtagagtaagggctttcggccaattttatctgaaaggtggccaaacaatggttgggcagccataaaaatcagcaaggcaccaaagttgatcattgtgaccagctttggtgccagccccaatgaattgatcatgtatttttgcatataggtcgtgtaggtgtagaaagcaattgtcccaccaaaggttaatccaacgacggtcaacacttgattgggatattttgccaactcacgcaaggatcctctggtggcctttgttttctcagtctgtttaaattgatttgtttcgtccattgaaagtcgcaggtataaaacgataacggcgccaactgccccaatggcgaaaggaatccgccagccaaatgcccgcagttgtccatccgaaagcattgattgtagaatgatttgaacgattaaggcgatcagttgaccgctgattaaagttacatactgaaacgatgcgtaataaccacgccgtccagaggttgccatttctgataaataagtggcagaaatgccgtactcgccgccaagtgataatccttggaccaaacgaatacagaccaacagcaacggcgcaaaaacgccgattgaactgtaggttgggataatggcaatcaacagcgatccggttgccatgatgctgacggagagcgttaaggcggcccggcggccttttttatcggcatatttacccatgataaagctgccgaacggtcgcatcaggaaaccgaccgcaaaaatagcggctgcactcagcagttcgacggtttgatcaccgtctggaaaaaatgattcggcaaaataaatggcaaaggatgcatatatataccaatcgaaccattcaatcatattgcctaaagaacctttaatgatattgcttgtaacccgtttttggctgtatcgttgcatgttgggacctcctttaattcagaaccgaattagaaattaattatagatattctaattaatcacctagtataggttaataattaatgggatgcaagatatcgtgttaggttatataacattttaccaaaacaaaaatgactgtcacctgtgaaccaattgtgggttcaactccatggggcagtcatttgagcttgattcaattagacaattgcttccagccgcaggagatgatcaatctcataagttggcttcaatcggatggtattgggctgatgggttgggttgaaccagactgaatcgaggccatataaattggcccctttaatatcggaggtcagcgaatcaccaatcaccagtgactggtcttttgaaaagccctgaatgttgtgtgcaacatagtcaaaaaagccaggatcaggtttttggacgccgacagtttcggacgcgaaaacatgagtaaagtagggtgccagaccagactcgttgagccgccgatgttgagttttggcgatcccattggtcacgacataaatatcgtgacttgcactgaggtcggccagcaattgcttggcttgcggcatcgggctgtgaccttcggctagaaaactgtgataccgttgttcataggcttttccgtcaacaacttggccgtaatggtcgaagaaacgacggaatcgagtatccagcagcgtttgtcgactgatttcgcctaattcatattgctgccaaagctgttcattaaattgatggtagtcggcatagacctcagaggtcagcggctggccgatggttttgaataattttttgagggcgtcatgctcagctgcctggaaattcaacagcgtgtcatcaacgtcaaagagtaatgtcgaatatttcatgaaaggagacctcacgtcatttttgttaaattctatcacaatccggtgggaattttgctgatattcacaaacttgtcagaattgttggcttacccttcctgcgaagtgctaccattaaaggaaaggtcttttacattacacacaggggagtcttaacatggcaaatcatatcacgctatatcagcacggaacgctggcattacttgttcccgggcttttaaagggaaccattacaatgggggaactgttaaaacatggcgataccggcattgggactggcgaaggattggatggtgaattgattattctagatggcaaaccatatcacgtccacgccaccggggatgtcacactagcccccaagttattcaccatgccgtttgccaatgcccattttgcccgctacacgccactggccgaactggaaaacgttgatcaggctgatttgaacaaacaattggtctcgttaagtcgagctgccaacacttttttctccattaaaataaccggcacttttgccaacatccaaaccagagcggcggttaaatctcagccgccgtataatactttggctgaaaccgctgaaaatcagagtgtcttcacccgggatcagattaatgggacgttgattggctattatgccccacaactgttcgagggtgcagctgtgggcggctttcatcaccacttcatttccgatgaccgcaagtttggtggccacgtcttgaatttccaccttgtaaagggtgatgtcagctaccagctgtttgatacctttgaacaacatttgccggtcagtgataaggactttatgcagcacgatttttcaaaggacgacatcgccggcagcattcaaaagtctgaataatgaaaccattaattacaattattccgattatcgttatcataatttaacgctttataaccttttagtaaacgtaatactaatattagtaaaacttttgcattcgccgtaaacactggggtgagtgcatttttgtttggtccaatttagaaatttgtatgataaccagttttagtacttgatttatacggatgaatccgttaacataacaaactatggacgctggttattttttgatagcggtccatatgtaatgctgtaaatgaatgtaagcgttacgactgtgcgtataagagagaatgtcacacaacaaagaatgtgttggatttgtctgatttgttatgtaaccccttccaatcttttggattggggaatcacgactaatcaagcgttggcttaaagtgtaaaggagaatgatgatggaaaaggctgttgcaacagaaaagaaaatctcaagcggatttatttatttctttggttcattcggtgggattctgtttggatatgatattggggttatgacgggggcactcccatttttacaaactgattggggactgcaaaataatgcgacgatcactggctggattacgtcagctgtaatgttgggtgccatctttggtggtgcgattgccgggcagctgtccgataagatgggtcgaagaaagatgatcctgctttcagctctgattttcatggccggatcattgctatctgccatctcaccgcatgacgggcaattctacctgattgctgttcgcgtcttcttaggccttgccgttggggcatcttcagctctggtgccggcctatatgtcagaaatggcgccggccaaaatgcgggggcgtttgaccgggattaaccagacgatgattgtgtctgggatgttgctatcttacgtgatggatttcgtattgaaagacctgcctgaatcaccacgtttcttagttaaaaacggtcgccctgacgatgctcgcagagtgttgagctacatccgggaaaacgacaccgaaattgatgacgaattagagcaaattcaagatactgcttcacaagaaaagaaaatttcaaaatcaaccagttgggcaactgtcttcagttcaaaataccgttacctggcaattgccggtatcggcgtcgcggctttccaacagttccaaggagccaatgcaatcttctattacattccattgattgttgaaaaggcgacaggaactgcagctaactcagctttgatgtggccaattattcaaggaattatcctggtaatcggatcactggtattcttgggaatcgctgacaaatttaagcgtcggaccttactaattcttggtggaacggtcatgggattatcattcctcctgccaactgccattaagttcctggtaccaaacgccagtccattactgattgtcttcttcctgagtatttacgttgccgcatactcatttacttgggcacccttaacttgggttctgattggtgaggtcttcccactggcaattcgtggccgggcatcaggagccgcttcatctgccaactgggttggttcattcgctgttggcctgctcttcccgatcatgaccgccagcatgccacaagacgccgtattcgctatttttggtgtcatctgtctgctgggtgtttggttcatccattcacgggtaccggaaaccaagggccgcagtttggaagatattgaagaagaaaacattaataaataatctgatgatcgattccggacaaattctgggatagcatcctataaaaattaaaagcgtctgacacaaatttttctatttgtgtcagacgtttttgattttgatagttacttctatatgatagggcaacaaaactctctacgaacccttattgcagcagctctttaataatcgcttcaccaacaccagtcgctgagttgggattttggccggtaatcagtcggtcgtcgacaacgacattcggctcaaaggcagtccccttcacgaagttggcaccggctttgtccaattcatcttccagcaggaactcaacgtcattcgtgagaccgtttaaggcttcttcatcattggtgaaggcagtcagcttgcgcccatgcacaaagcgtttgccatcttctgtccgcatgggcagcaggccacacacgccgacgcaattggctgagacaattccgccgttggcataaattgtttcggccagccccgccaattcggtgttctgtgggaaatcggtcatcgttccgtggccgccaacaaaataaattacctggtagtccttcggattgacgtcggccggggtgagtgactgggccaaatggtgatttcggaaggtgtcgtccagataatattcccaatccgtggcgtccatgtcatcggttcccaagctcagaggatcgagcgggacataaccgcccttaggactgacataatcgacatcgatgccgttatcggccatcactttgttgaaatgggtcgcttccttcagccagattccggtggcccgttgaatcttcttgaatttggggttgtttgtcacaaccattaaagctttcgtcataagcagcgttacctcgatttttcgttctgattagacttgtcgatttcatttcctcacccccatcataacagataattcatgaggatgatgagaaatggggtgttgtataagttttaacacatatgttatccttaaggccaaccattcatgaaaatgagtggccctttacttgtagaattgtgtttgagtataaatactaggaggaacacatggcagactcaatattaaatgtcgagcatcttaacaagaactttggccacaagcaggttctcaaagatgtgtcgttttcagtacaaaccggacatattgtgggcttggttggtcccaacggtgccggtaaatcaaccattatgaaagccgtcttaggactctttaattactcaagcggcaagatcaccattgatggcgatccagtttcacccaccagtcatcgggcgatggataaggttggcgccttaattgaataccccgggatttacccattcctgacaggttatcagcacctgcagttattttcaaaggaatcgacttcaaaagatcagattatggacatcgttgacaagatgaagatggattcatacataaaccgcaaggccaagacctactctttaggtatgaaacaaaagcttgggattgccttggctttagtcgaccgccccaaactggttattttggatgagccgatgaatggtctggatccccaagccaacaaagacttgcggaccattattttggatttggccaaacaaggcaccacattcctgatctccagtcatatcttaagtgagttggaaaaattggtcgatgacctggttgtcattgataagggacagatcgtttacactgagagcatggccaacctggaaaatggcggtaagaagttattggttcttaagacctcagacgacgcccatgctaaagatattttgagccaaaacggctaccagcttgatgacggtgataagctcagcattgtcgaaactgactcaaccaagatggctgacgtgatcaaattactgtccgataacgatatcgaaattgaagatgtccaacacgttcacagcgatttggaaacatcactcttaaatctgctcaaaaacgacaaagtaaaggagtcatagcatgataacgttagtcaaacaagaaatctttaaactgcttcataagaaaagcacctacgcagtctcagctacattattgattctgatgactgtttttggtgtattgaccagaaactatcccaagtactggggtgatcccaaaggattatttgtcgaaatgtttaccgggatcaactggatcgtcttgttcatgattgcggcctgcagctcaatcattgcgatggaattccagtacggcacgattaaagaattattgtatcgcaagtactatcggggtcaaatcctggtcagcaagtggattaccatgttgctgtactcgatttatttctatgttttgagctttgtctggtcgatgcttttgaaagttgttttgtttaacgataaattcaaactttcagatacctatcaatcaggtcattcagttatcgaagcacaatggctcggcattatcggctcctttctaacgatctggctggttctcagtctggtattattattggccaatatcttcaagagtaccgcagcagcgatttcaatcgggattatcggttactttgctttgagcatggtttccggggtcatgttcttattgatgcacaagtgggaatggctgaagtggaacccattgaacatgatgaacctgccacaacagttgctatccagttcggttcataaaatgactttgttatcgacaccggaaatggtggtcggcagtctggtatacacagcaattttcatggcaatcagctacgttgtcttcaagcgccggagtgtctaaattaaaattgaacgtttcaaagatggaatcggctaacagctggttccatttttttgtgcatagattcatgtttccaaaaaggtgtcattttaataacaatctcattatttgttaagagtgtctaacgtttgctcagaatgaaagcctgggaatagcaaaatctgtgatgtttggtactatgtatctgattaaatgttacagatatatttcaagattgcatgacggggggattgcatatggtacataagagttggctgctattgccactgacggtattgttgatgggatgcagcgcgcacaagacgaccaccgctcagacgacttcgagcacggcgagtgaacaggatggcaaatataacggagtgaccttagacgttgcccggcgccactaccaagtcggaacgttgcaaaagttcattcaattagtgggggatcataatggtcggtttattcagctgcacttaagcgatgaccggaattttgcgattgaaaatgactacgttggtcagtccttgaagaatgcccagaaggttgatggcgtttggcataacaaaaagacccaccagttcttttacagcaaggccgaaatcaagtatttggtcaacgatgccgaacagcaccacgtgacgctgatcccggaaatcgacaccccagcgcatgtgactgccttggtgaagctcatgaaggccaatggcaaggcacaactggctgatcaagtcagctggtactctaagagttaccgcgacgagattcacctcaatcaaaccggcattgatttcaccaaaaagctggacgacgaggttggcaccttgtttgccgggtaggccaatccccgctttcatttaggcggcgatgaattttccgataagctaaccagcaacgctgcttacgtcaaatatttaaacgccaccagcgccaatgtggaaaaaatggggttcacaccggaagcttggaacgacggctttttaaacagcagtttgagcaaactcaataaaaacatccaagtaacttactggaactggaccgcagatcaaactggcaagttagctgctgagcgccacaaatactgggcctcgatgccaaaattgatcaaccgtggttccaaagttttcaactataacgactactatctgtatttcaatttatccaaaaccaacatgtccaagaaaaacgtcgcttatatgattaaggatatgaagcaatactggaaaccgacgttatggcacaacgacgttgacaccaagttgaagtccaaacgggggattgtcggcagcagcgtatcactatgggcagactcggctggatcggtcaatgatcagcaggtgtacgccgccagtgagcagttcatcaaaacctttttggccttggccgaaagtagatagaatggggggatattatgagtaccttgagtgattttgtcattttatatccagtaattgtgtcgacaatttggatcgtggggtcaatctttttctccattcaagaacggcgggtaccgctgaataacgaccatcaaggacaaccagctgacctggtttcaattttgattccagcccacaatgaacaggacaccctggcccaagtggtcgagtcgatctcaaagatcacttaccaacggattgagctgattttaatgaacgacggcagtcaagacaataccttggcggtgatgactcagcttcaggaacggtatggccatcagtttccagttaaaattgttgatatcaaggtcaataaggggaaagccaacgccctcaatgaaggggccaaggtggctcaaggggaatttttgttgtgcctggatgcggattgctacgtcgatcaaaatgttctggaaccgatgctggccagattttacgatgatccgaaagtcggcgcagtcgccggcaaaccaattgtccgcaaccggaccagtattctaggtcggctgcagttgttggaatatgtgggcgtaatcgatattatcaaacgcggccaggctttcgttattggccacatcacaacggtttccggtgtggtggtggcttatcgaaaacaggcgattattgatgccggctggtggaatatcgatgccattactgaggatattgatattacttggcgcctttatcaccatggctggcaggtccgttactgcccggagtcggtcgcatggatcttggttccggaacgaataatcgatttgattcaccaacgaaggcgctgggcccgcggaggctttgaagtgctgtttcgcaaccgggggatgtttatcaccggtcgcttgagtgaacagtggctgctgatggacatggtgctcagtgatttgtgggctatcagctgctcatttgtgacgttgttttatctgttcacgattatgttcacaggtgacatcatcatggacggcgtgattttatttctactattgctcattagtttgattcaattcttgattggttatgccgattccagagagtccgattttatcaaatggcaggacctgtcactgttgccactgtatgtgattttttattggttcatcaacttggtcagttgcctaactgccctgggatcgttcttcctggatccgagtcatgttggcagttggcgtagtccggatcgggggctttaatcatgaaaaagaagactaacaacctgattattcggaaacgatcctcaattcttaaattgttggaacggttcatctttttggtggctttgtgggccatgacagcttacgtgatctacgtcaacgtttgcttcctattgaacgcatactcggacacgctggtttctgattacctctttttgaacctgtcctactttgcctatgcccgatttgccatcctggtcgtggtgatggtcatcttgatgacaatttttggttagctgcgaattaagaaacttgagcggagggcgaaaaatcatgagcaaaacaagtcgtaagtggattctaagcggttttattctggtctttttggcacttttggcagtcagtgttcgacacaatattgcctatcagctgggcaatcggcctgattttgcgatttccaaacgtgaccagcgaatcaaaaatggcatcatggtgttctcctaccaccggattttggcaccgaatgacattgtccggttcgatgaaaaagtgtcgccgaacacacagcttcacgattttaacgtcaacctgccttcctttaaaaagcagatgtattatttgaaatcccatcacatcaaagtgatttcaatcaaacaaatgattgctatggctcacagcaagcgccccattcgcggtaagtacgtggtaattacctttgatgatgttgaccggacgtcgatcgacaatgcgtttccgatcctcgaaaaattacattacccgtttacccagtcgattattaccggcaacaccggttggtataagcagggaactaaattggcaacttggccggcaatccaaaggctgcaaaaacaggccgatagtttagtgacctttggtgttcacaccaatcggatgcattatttggttgatcacgggatcccggtgttcaacattccggcgaactacactcgctttaagcgtgattatgcggtcagccaggatgtcttgaaggaaaaggtcggctataagtcaccaatttttacttatccatacggcagcggcgactaccagattcaaaagtttcttgccaaccgccccggcctaaaagtcatcttgaccttgaacgatggcttggtgaccaaccatagtaacttaaaactcaccccaagaattattgtgaataattacagttggccgagcatcaccaaatggattaacaattgaacgaaactttgagataaaatgaagataacgataaagggggatgcacaatgacgttttacacgtacgactatcttcaaggttctcaaagtagctggcagtacgccagaatcattattttaagcgtgctggcagtcatttttattggctttttggtccattaccttcgtaatcgaatggacagcaaatacaaagatttaaccattatcgtcgggacgctgctgctgcttattttagcgatccaatacgacgactttagtgcaattcagtccgcttctgcgcagactggtcagattacgcagacagttaagcagattgccaagcggcttcatgtgggaaccaaaagcgtcagtatcaattcgaccacccaaaatgccaacctgatggctaagacccccagcggttattaccgggtcgactataacgctgacgggagtcagtttgtgttggaaaaggtcgaattagatagttcgagccacatcaaagttcaggaggcaaattgatatgtttacatattcagacgttgcacttaaattaatcgtcggtttcttatttatcaccattttgattaacctgaccggaaaagggaatctggcaccgacatcagcaatggatcagctgcaaaactacgtccttggtggcattatcggcggtgtgatttataatccggccatcacgatggcgcaatttttagtgattctattgctttgggcactgttaatcatggtgaccagatatttgaaaacccatattcactggtttggcaaatttatcgagggtgagccaatcacactggtgcgtaatggtcagctcttggttgagaattgcattcgcgccaatctctccggtaaagatgttatttcaagctgcgaactgccggagtgtatgacattcaagacgtgaagcgggccattttggaacaaaacggtcagctgacggttttgaataaaggggagggtagtattcgctacccggtaatcgtggacggccaggtggatccggacgtcttagatctcatgggtcgagaccagcagtggcttgaagacgagctcgccaagcaaggcttcgacaatatccgcgatgtgtactgggcaacctatcgtgaaaatgtgttgaaagtcgcggctttccctgaaaaatgataatggtggaactaacacggccgtgtaagaataaacgcgattttaccatacgattattgaaatacacggcaatcaagaatcaaaggcataattatacaatcgattgatctttcattgacttctcagagaattgttatattattaacttgaatttacactttaagtgcaacactaattaaataaagaatggcccatggccaaatttctgtaaaatgatgtttgcgaaaacaatcatgaaaggaatttaaccatggatcactacaagcatattaccatagatgaacgggaaactatctttttaatgaggaatcatggaaactcacttcgtgagattgccagccatatcaagaaaagttactcaaccatttctcgagaattaagccgtaattctactggtaaatcctattcaccttcgaaggctcaggagaagtacaaacagcgcaaaggcaactgtggcagagtctctctcttgagtaatcctcaggtgtttgaagtggtgagagaacacttctgcgaagacctttggtctccggaggaaatatcgaatcgcttggcagtcgaaaagtatccggtgcagatcagtaccacgactatttaccgtgggattttcaatggcttatttgataatttgtttaaatctggcagctctagtgccgtgcgccatctaaggcatcacggcaagtctcgccacaataaagcttatcaagaaaagcgaggcaagattccaatcccaaacaagattcatgatcgtccgcgagaagctgacaaccgtgtagaaattggtcactgggaaggtgataccgtgttaggcaaaagcggaaaggcttgtgttgttacattggttgatcgaaaatctcgttacctgcttattggtaaagctgctaaaagaacttcagaagcagtcacggatactttgagcgacttaatgaagctatggcctggtagatcgttaacgattaccccggataggggtaaagagtttgccaaagttcaatgtttaactgataagtttggtacgcccttctactttcccgatcctcactctccttggcaacgaggaactaacgaaaatactaacggcttgcttcgcgaatatttgccaaaaggaactgaccttgattcaattactgaccgccggatacaagcatatgcagaacaaatgaataatcgtccccgtaaatgtctcggatggaaaacgccttatgaaatattctttaatgtcgtgttgcacttaatttgacaattcaagaacaataacttttaccgaatcattggcaggttttaaatctgagttttccggaggtcaccattatggaattagacagtatcaacccttatgtgttaaaagtcatgccgtccgcaatgcggaaatttgatcatgacattagttccgatccaaagattatcaaattaactttgggcgagcccaacttcaacgttcccgaccatattaagcaggccgcaatcgacgcgattaaccacaacgaatctcattatccttactattggggttaccaaccgcttcgtgaagctgcatcaacttattatcaagctaagttcggctatcactattccgctgatcaaattttggtgacggttggggcgactgaggccgttgcttctgcagtgaagaccttgtttaagcctggtgacgccgtgattattcctacgccggcctatccgctgtataacgctttgacgaccttaaacgagttgaatacgattctggtggacaccagcgatgatggctttattttgaccccggccaaagtcaatcaggcaattgccgaccaccctgactgggatgtcaagggtctgattttaaccgacccgaataatccgactggcgttgcttataccgaagaacaaattaacgcgttggcgcctgttttaaagaaaaatggcatctgggttatcagtgatgaaatctatggcgagctgacatacggccagaagcactattccatctcaaaagttctgccggatcaaacggtcgtgattaacgggttatccaagtctcatgccatgaccggttatcgattgggattggtatttggtcccagcggtttcatcgatgaaattgccaaagttcaccagtacaccgtgaccgcagctgcgtcaatcgttcaatacgcagcgattgaggcgttgacacacggtcaggacgattccaaaccaatgctgaaggaataccaaaaacgtcgagattttgtcgccaaggaaatggctgaagccggttttggcgtcgttcatcctggcggggcgttctatgtttttgccaagattccagcagatctacagatgaacagttgggactttgttaatacactggcaaaggaataccacattggcttgatgccaggagatccatttggcgataacgaatacgttcggatcagctacgcagccagtgatgaggccttggctgcagcgatgaaggctgttaagcagttggtggcggatcattcagcacaaacaactgaataaaatgtgctggctgacggtttcataataatttagatttaaatggtactcaaaaaaggtcgcaacgtaatttttgctaattatgttgcgacctttttgatttttattcaagattcaattatgcgcgcttacgatccttaatggtaaatgaaagcaggaaagccactgcagccacgatcaacgtaaaccacagaccaacgtggaccccattggtaaaagcaatttgatggctgacatgaccagcagccgagtttccaaatgccaacaaactggtagcgatggcggttgccatggccccgataatttgctggaaggtattcatgatagtgctgccgtctccggaagtttgttcatccaaagctcccaggccaaatgtttgggcgggcgacatggcgagcggcacacctaacataatgatgatgtgagccaagatgacgtaccacattggcgaagttgagctggccaaaagtaacaataccaggccgacgatggtcacaccaaagcccaacgttgtcagcagtttggggctaaccgtatctgagaagcgcccagcgatcgctgagacaatcgcgttgacgattccccctggcagcatcacaattccagtcatagcgacgggaattgccaaaccgttttgccagaacattggcagtaagtacattgatgaaagaataatggcgaaatccaacatcactaaaacggagccaaccgtaaattgatgcttttggaacacgcggaaattcagaattggggtttcagattttaattggcgacggatgtaccatgccaagataatgactgagacgatcaaggttccaatcacttggggtgagccccaaccggaatcactcgccaagctgacaccggcgacgaggccgccaaagccgatcgctgacaaaatgattgagaaccagtcgattttgggcttagtgatgtcacccacgtttggcaggtacttgaaggccaaaataaaggcgattaccagaaatggtacaaacaaccagaaaatccaatgccatgaaagcaggccgaggatcattccagctaaagttggaccgacagcgggcgcaaacatgatgacaagtccgatcatccccatggctgaacccagcttatagggtggaaagattaaagtcgctaccgtgaacatcaagggcagaattaaaccggtggcaatcccctgaatcattcggccgaccagtaaaatggcaaaattcggtgccagtgctgaaatgaccgcaccgacgataaaatcacatagggcgaataagattaatgagcgggtcgaaaaaatccgctgaagcaatgaagacatcggcaggacaatcccgattaccagcatgtagccggtcaccagccactgcatggtgccgatgctgacatgaagttcggcaatcaaacttggtaacgcgatgttgagggaagtttcactcaacatcccaacaaagccgccaatcagcatgcccaacattgctaagaatggacgagcaaccggtttggctgcttgtttttgttttggttcgacagacgcttggtctgcatttaacgatttttccataatgtttctcctaattcttaaaacttttatatcatgacaattgattacactaccataaataaaagctgctcgtaagttttattttcaaaaactttcataaaacatgaaaacttggtttaacagtggttactgggaacgcttacgaaaaaatgcaaatatgtagataacggtcacacatttatgccggttttctactacaatataggcagatgcgtagacggatttggcaaacgcatttcgctgaaattattaacggggagcgattgaatatgaaacatacagtgttaatactgaccggaatcggtgtcgtggttgccggtgcctgccttttgaagtcgatggggtggtttgaagatgactctcacctgtacgatgagtacgaagcgaaataatttgtttggaggaattcttaatgacaaaaaataaagcaattatgatcggtgccggcttggctaacatggcagctgcggtctatttgattcaagagggtaactggaagggcaaccagattactttttactcgattgacgaccatggttcaaatgacggttcacctgccagcgaggctgccggagaatattggaacaaagttcacccaatggaaaacaccaaaggcttcattgcccgtggtggacggatgctcaactatcgaacatacgttgatctgatggacttattaagccgagtgccttccgcaactgaaccggggatgaccgctgccgaagatacccgtgattttgatgccaagcatcgcacgtttgacaaagcccgcctgatggaaggcggcaagggcattatcaatggtggcaagatgggcttcaataataaggaccgactgaaattaaccgaattgatcatgatgccggattctaaagaagaacaacttgataacgtcacgatcgctgattacttcaaggatgatccgcacatgtttaccaccaacttctggtacatgtgggagacgacctttgcctttcgggtacaaagctcagcgcaggaactacggcgttacatgcaccaaatgatttacgagtttactcaaatcgagcacttggtcggtgtcaaccggactcgttacaatcaatatgagagtattatgctgccgctgatcaattacttgaaagatcaaggcgtcaacattattttgaatcgaaaagtaactaattttgaatttaaggatacgccgatgcaagacgagattacggtaactgccttgcggatgacgaatacggaaactggcgaggaagaagacgtgccggttgatgatgacacggccgtgatcttcaccaacggttcaattaccgattcagctactcttggtgatttcaatacgccggctgaagagaatatggattatggtgccgcggccagcctttggaagaaggccaccaaccggttctataatttggggaatccggacaaattctttaacgatcgtaatgccagtgagtgggtcagctttactttgacgacaaaagatcatattttgttgaatgaaattacccggattaccacccaagttccaggcaatgcattaaattcattcatttccacttcaccaattaccccaatgggcaataaggatgtcaacatgtcgattgtcgtgcaccaccagccgcatttcaccacccaaaaggccaatgaatcggtgatttggggctacttcctgtatccacgacggaaaggtgagtttgtgaacaaacagtacatcaagatgactggtaaggaaatggttgaagagctgctgggtcaattatccaaggttgatccgggaccgggcaacattatggataagaagcaggaaatcatggacagcgtgattaactgcatcccggcatacatgccgtatgcatccgctttgttcaacaaccgtgccaagacggatcgaccaaaggtgattccagagcattcaaccaatttagctttcaccggtgaatttgtggagcagccgtatcaaatggtcttcaccgagcagagtgccgtgcgatcaggagaaatcgcggcttaccactttgccggagtgccaatggctaagttggtgaagaatccgcggtatgatcgggatattaagactttggccaaggctacgcggaagatgttcgagtaatctggcctatacgtcggttgaatgagtcttaaaagcaacgtttaagccacatacttaaacgttgcttttttgtctttgaaaactatcccagtaaatgtggataaccaagatgagttgtacaccttcgacgcaccaaaaacggctgagaagagtcacctgacattgattccatattatgcttgggcaaatcgtgacgaaaaacaaatgaatgtctggatccaacaagcaagaatctaatcaaccaggattatataagtgaagttgaattaaccactttagatatttgaacaaaacaaagaatcctcctgtaaattgttctcattgatttacaggaggattcttcattacataaattgattaccggcgccgtcatccggtgtgtttggttttagactgatgtatttcttacggtattcggaaggcgacatgccataaccttttttgaaggccatcgagaagtaatagacgttttggtaaccaaccttcgtggcgatggtgctgatttggtcagaagtcaataacaggtacttggttgcttcttccaaacgatattttgtcaggagattattgggggtgatgccgaatgttttcttcatatataaagaaacagaattcggatggatatgaaattccttgcctagctcttcataagtaatcttttcgtcaaaatgatcttcaatgtagcgctggattttgttggcaatcatcgtggttggcgactcttgcgatgtttgaacctgaatctgctggagtaggtccaagaatagttgctgggccttccagaactcaattgaattttggatggtgtcagagtggttttcattggacttacggctgttggcaaagatctttttgatcattgagatcaccgtttcttcattaggaatcggctgttgcttctccaaaaataaagtaatggccgaggtgtagtaatgaattgccggcacgggaatgactggtcgcatctgctttggttcccgggcttggacgtaattgccggctgttgcaaagtgaatccagtagtattcagtggtttcatccattggtttccatgaatagtgatggtgctgtggttggagaatgaacatctcaccggcactcacggtgtattcggtattatcttctgcgataaataattttccgcgtttcatgaacatcatgacaaagaattggaaattcttccggttgggatgccgctcaccgggactaaaaaccacgtggccgctttgaatataggtcggtgtcgggatacatgaaatcgataggaattgcttaaccatagaataacctccagtgcaaaatcgaattgtttgctgatcacaattgggattttataaatctttctgttgttgttataaaaataattcagaaagcataaaaagtcaatttcaaatcagttttatatttcacaaagaaattggctaaagactatttttacgcgaattcttgcttgttcagcaaattataaaagcgcttttataaatatgttttattttataaacacttgatagatttttagattcaattgatgccgtttacacggtattctatatatcgtaagcggttacagaatcagatgatttgctgatcacattaaataaatttgtttccagaaagggcaattcaaaatgaaaccggtatcatattacgacattaaatatttgccagattcgactttgaaagaaacgttcgaaagaaacattaactggatgctttccctcacaccagatcaattgctatacaactacttgccgttgcaactttcttagccttcaccgcaccaaacttgcatggtaccgctaagctctggtatgccgggttcacttatatcttggccgctggtgttatttacactggtattcaaacaccaattactgctattcttcctagtttgaccactaatggccaggaacgtatcaatgccaacacattccgtatgtgtggtggtgccattggtattcgataaggtggtgatgcattcattcagaaaattgcagtatttcacaattcggacattatttctgacataatgctttcacgaacccattcgtgttccgagttacccactaataaatcaagaggctcaaatcgttgaataaacggtttgggcctcttttactgaatatatatttgataaatataataaaatgtgaagacttctaataaaatttctgctaagatattacctaatgatgtaaatgacggttgtgagtctacaatcggtttacaggatgtatttgtcacacaagctaatatagaaagtgggaataattttgaccaacgttaagtcatatattgaatcaatcaaagatcaaattgatcgtcgagatccgaaccaaaccgaatttcaggaagctgtatttactgtcctggatagcctggaaccaactttagaggcccatccagaatatgtgaagagcaatctgctcgcacaattagtcgagccggaacgggcaattcaattccgggttccttggcagtcagacgatggccaatttaatgtcaatcgtgggtttcgggttcaatttaactccgccattggtccttacaaaggcggtttgaggttacatcccagtgttaacttgagcgtggtcaaatttcttggcttcgaacaaattttgaaaaatagtttaactggtttgcccatcggtggtgccaagggtggcagtgattttgaccccaaaggcaaatctgattctgagatcatgcgcttctgtcaaagctttatgaccgaattacaacgccacattgggcctgacctggatgttcctgcaggcgatattggtgttggcggccgtgaaattggctacttatttggtgcttataaacggctgaatggttatcaaaatggcgtgttgactggtaaaggattgacatttggcggcagtctcgcccgtactgaagcgaccggttttggcttgctgtattacactaacgcgatgttaaaggcccagggcgacactttaaccggcaagaagatcaagatttcaggtgccggaaacgtcgccacttatgccattcaaaaggccacagaactcggggccaaagtcatcaccgtttcagattccaacggctacatttatgaccccaaaggaattgactacaaagttgttcagcagattaaagaagttgaacgcggccggatccgtgaatatgccgaccgggtggcatccgctgaataccatggtggatctgtctgggattttgacgttgactatgacattgctttaccatgcgcgactcaaaatgaaatcaacaaggatcaggcaaaattgatcgtcaaagacggtgtcaagtatgtctgtgagggtgccaacatgccgagttacccggatgcgattgcaatttatcgtgacggcgatattctgtatggcccggccaaagcagccaatgctggcggcgtggcggtatctgctttggaaatgagccaaaacagcgaacggttggcttggagttttgaaacggtcgataaccggcttcaagacatcatggaagatattttcaccaagtccgaagctgctgacaaaaaatatcatttggataaggactatcaagctggcgccaatattgctggatttgagaaggtcgctgaagccatgatggcacaaggattagtataagcacttaacaagttggaactgaatttttggtggaaatacctttgatgagcacttattgaaagcatcaaagatccatcaatctctcagttccaactttttgtataaaatatacaaaatatgaataattagataaatactcatcattcccttaaaatcaacccgcaagcggctttaagcttaatgatatgtgaggtattgcgacatctaaattgagccaacctcttcccatagtgctgataaaatgctatattttataaaagccatttttgaggagtgagtattttgaaaaaagattagaagattattaattatatttgtgtcggcgttctcgtttttattcctaatgaataatgttgcatccgcacaatcaaaagaacactacacaattggtgttggaccgacctttgtgccgtttgaaattcaggccaagaacggatcttataatacggctcaccctggtctcgatattgaaatccttcgggcggccgccaagaaggagaacttcacctacacgttgaaagtcatgaactttgcggcagccattcaagcgttggaaggcaaccaagttgacggcgtgattgccgctatgatggcgacgccggaacgagctgagaagattgatttttcaaagccatattataatgttggcctcgcattggcagtgccaaaggggagttcgattaaaggatataatgatttgaagggcaagaccgtcgccattaagaccggttcaacctctgagcagtatgccgaaagcattcaaaagaaatatggctttcatattacccggttcaacgatagtaacactgaactgagtaacgttttggttggaaactcggctgcggcgattgattccacggccacgttgttatactcaatcaaaaacaagatgaaactccagttagttgggaaggccgccaataaaaatccggtcgccttcggggttaagaaaggccacaatcaggaattgctgaaacgattcaatgccggtttggctgccatcaaaaaagatgggacctacgataaaatcgtcaaattctacactggtgaacacagtaagtcagcgatcccagttcaatcaaattccgatcggacatactttggcctgttgaagagtaacgccacttcgtttggcaacgggatcaagatgaccctggagatcacgattgttgccattttcttcgcgacgatcatcggaattattctcggtatcttgggcgccacgccaaacaagttcctgcgaggattatcttccacttacgcctttgtcttcaagagtatcccagtcatggtgttggcattcttcgtgtacattgggattcccaacctaacaggtgagaagatcccactgtttattgccggggtcatcaccatcgttatggaaaatagtgcttatacggcttcctttgtccgtggtgggattgaggcagtcgaaggtggtcaaatggaagcggctcgttccaacgggatgtcgtatttccaagccatgagatacattgtactgccgcaagccttgcgaattatggcaccctcatttatcaaccaatttatcatcgcattaaaagggacctcggttctgtcggcgatcggggtggctgaactgacccagcaaggaacaatcattatttccagaaacatggaaggtttcaaagtttggttgctggtatcgttgatgtacctggcaatgattgggttgttgagttacctgtccaatctcgtgaagaagcattatcaattggcaagttaaagcgaatctaacttaatagcagtaaaaaatgagcaggaccaccgtcaaatctggtgatcctgctcattttatttcttttaattcaaatattgttggccaatttctttgtaagtctcaatcatattgtagtaagtatccagatcaatatattcatcgtgctgatggctggtcgtgttccccggcccgaggaccaccacatccatcttttggttcactcgggtgtattcagaggcatctgttccaagcgacaccccgatcgttggcaggtccaaagattcatgcaggtggtgggcgccagctttttgggcgatgtcgataatcgctggtccgggatgattgatcaccggccgtttactggtaatatcgattgtcaggttgtaccctggctgttgatttaaatgatcaatcagctagtggagtttcttgatgatcgtttggttatcgaactcagggatcgtccgaactttgactttcaagctggcaatgtctggaatactgttgatttgtttaccaccggcaataattgtcggagcgtacacggtatcgcccagaattggatcagtggcttgaatgctttgatagaactgtttttccttgaggtagtaattcaccagcatatcgatggcgttgattcccatctttggcattgatgagtgggctgccttaccatgggcaacgacttcatacatcagccagcctttatgggcaaagaagataaaatgctgttcaggcgattttcggtcatgactgacctgatggagcttggctgccaattctggcgtgaatttagcgccgccactatcgacgtaagcatcgaggcgctcttttgagaccccactgggttcaccgatcaccacggcgtcgagatcatctacgtagcctttatcggccaataattttgacccgagctcaccgacttcctcacccatagtcacataaagcctcaaaatgccattgtggacgcttttggactccacaaggctgatgaacgcgattgttaggccagcgagtccacctttcatatcggcggctccacggccatataaacggttatcacggacattgggttcaaaaggtggcgtcgtccaagttgataaggcgccttcatggacaacgtcggcgtggccggagaagcccagaaccggcccaggattacccgtgtcatattcagcaatcaagtcatctcggttttcagcgtatttgatgaaagttgagcttatcccgtgtttggccagcaagtcgtgaatataggcggttaccagatgttcgttgccgttgacggtgcgaaaggaaatcagatcctttaaaatctgcagcttttcattattatccatattgtgctattccaccttatctttctgattaaaatgagctaacagtgccaatgcagcctgctcgtggaacttcgctgcgtatttgaggccttcggggttggcaataaagtccgggtgatgtaagttagcctggcccttgctgcccatgaatgcgtaacagccgggaattaattgctcatactcggcaaaatcatcatcggcgttggaagggatggcatcagtgactttcatgaattggcttgcctggtttgcgatgaggtttgtgattgcttcactgttgtccacaggagcgggtccctgatcccatgtaatggttgctgtttggtcataagcgctggcagtggcattcacaatctcgtaaaaccgctgtttggcaagtttgcggtcggcttcggaaaaagtccggatggttcctttaaagccggcactttccggaatgacattgttgacatggccgccgcgaatggcaccaactgttaggactagccgatcagaaggcgagatgtttcggctgacaatcgtctgcagggtcataatcgtatttgcaacggcaacgattgggtcacggccggtttgcggcattgcggcatgggagccaactccggtgatggtcacgtcaaaattgtcgttggaggccatcaacttgccgattttcatgccaacggtccccactggaatggttggcatgttgtggattccagagattgccaggacatctttaaggatccccgcatgaatcatttcccgtgcgccaacgtggcgttcttcgccgggttcaaagattaagcggacattgccggataactgcgattctcgttcttttagtaacttcgctgcccctaagagtgccgcaatatgaaaatcatgtccgcaagcatgcgctgcgccggagatttctgatttgtaaggtaaatcagtttcttcttggagcggtagtgcatcaatatctgcacgcaacgcaattgttggaccattacctgggccaatttgggcgacaaggccgctttgaatgggaaaattcaggattggaatggccatttgatgcagctcatcggcaatcttggccgttgtccatttctcttgatcacaaagttcggggtggcgatgaaattgtttaaattgctcgatcatatagcgatcgagttcgtctgtaacgggcgctgtttcaaccatcctaatcactcctaatcattctttaatatatatttaataatactttaagagtttaagaaaagatagtcaagcaaggcttaaaatgtttcgtgaaacgacttaggcagattaagcttattcaataaatgggcctgagaccttttgtattggcggctgatatgatacatttaagtgaaacaacgcaaggaggaacacacaatgggactattaattactggaattatcatcatcgttctaatcgtgatcgttgtcgccttatacaacggcctggttagccaacggaacctggttgacgaagctgccagccagattgacgttcagcttcagcgacggggagacttgctgcccaacttgctggaaaccgttaaaggttatgccaagcacgaacaggaaacctttgaaaaagtgaccgcgatgagatcacaaattcaagaccccaacgccagtctgggcgataaggttaaagccgataatgagttaaccggggcgttgaatcatttgtttgcggtttccgaaaactatcccgaattaaaggcaaaccaaaatttcttggcattgcaggaagaactgaccaataccgagaataagattgccttttcacggcagaattacaatagtaacgtcatggcatataataacaaactgcaaaccttcccaagtaatttggttgccaaattcggaaccttcccagctcgttcttatctggaagttcctgaacagtccaaagaagtaccacaaatgaaattttaaaggggcctgactgataatggataccataaatcagcaagttcagcagaatcgacgacgaacctggtcagtcatggctttctttgttgttttaattgccgttattggctttctaattgggttggtgtttgcggttgccacccaagatgaaagtattgattggctgattccgacttacacgatggttggctttctcattggggcggccatctattcgttctttgtctacatgagtgtgaccaacattttgatgaaatctgccaatgcgcatcaactccaagaatcagacgacccggaattgtttaacattgtcagtgacttggtgatggttgcccatatccctatgccggcaatctatttgacggatgatccttctccaaatgcctttgcaaccggaagagatccgcaacacgctgcggttgcggttactaaaggtttgcgggaaatgatgaaccgtgaagagttggaaggggttttggcgcacgaaatctcgcatatcaaaaactacgatatccgagtatcatcgattaccgttgccttaaccacgtttattgccggggccgggacagttctgattgtttccggaatcagcttaatcagaggtggccgttggttcagctggttcggcagtgacagcgacgatgacgccaaatccagttgggcaattgcggttggaattttagtttttggactcatcatgtggctcggcggctggatcatccgcgcagtcggagtgccagttgcccaaatcctccagttctctgtttcacgtgaacgggaatcattggccgatgtttccggggttaatttgacccgggatccgcaaggcttaattaatgcattaaccttgttaaaaaatgacaccacaccaaccaacaatccgactgccaagagtgccgcgctttatattaatgagccggtcacccggcaaggaaaaacaccttttttggccaagatgtttgatacccatccaccgttggatgagcggattgccaggcttaaacgactgctgggtgaacaataaccaattcaaattatgtatgcaaatgggcaaccgactcgtgttttgacacgtcccggttgcccattttatattttagattatgccacttgtgcactaggcgtaattttggttcgattgagcaatactgaactggtaacgactgacagggaactcaaggccattgccaaaccagccaattcgggactcaaggtcattccgataaagtagaatactccagcagcaactggaattcccaatacgttatagacaaatgcccagaataggttcaacttgatccggttaaatgtcttcttgctaagttccaatgccttgtaaacgtcgcggagatcatttttaactaagacaattccaccggactcaatagcgatatcggttccggatcccatggcaatgccgacgtcagcggtgctcaaggctggagcatcgttaataccgtcaccgacaaacgccactttgccggcgctttgaaattgcttgacctggtcggccttgtcggctggcagcacgtcggcaacgacttgatcaatgccaacttggctggcgattgcctgtgaaactgcctgattgtcaccagtcagcatgactgtctttagcccttgtgatttgagcgctgagatggcatcctttgaagtcggcttgggagcatcttgaatggcgattaggccaataatttggtgaccttggccaacaaagacgactgttttggcttgtgactgtaaagttgccatttgttgtttaaatgtgtcactcacttcaacgtcattcaacaacttggcattgccgacaaaggcactttttccatccaccacggctcgaacgcccttgccttcaatggctgaaaagttttcagcaggtgagtaatcaatgccgtgctccttggcattcttgataattgcggttgccaatggatgctcggatgaggcttccaaacttgcggcaatctttaagacttggctggcgtcgccaacaatatctgtgacttggggcttaccaaccgtaatcgttccggtcttatcaaaaatgactgttttaacatcgttgacagcctctaaaacttcaccatttttaatcaggattcccattcgggcactgcggccggttcccaccattaaggcggttggtgttgctaagccgagtgcacatgggcaggcaatgacgaccactgagactgcaaagatcagggcgttggcaacgctggcaccaatgaagacgtaccagattaagaaggttgaaatggcgattatcaataccagcgggacaaagatttccgagactttatcggttaatccttgaattggcgcatgactattctgagcttttttgaccaattcgacgatctgagccagcatggtgtttttgcccactttggctgctttgaaagtgaacgttccagtcccattgactgtagcgccaacaactgaatcaccggcctttttttcaaccggcatactttcgccagtaatcattgattcgtcaatcgttgatgacccactgacgatttggccgtcaacagcaatcttttcacctggccgaactttgatgaggtcaccgacgacaatctctgagattgggactctgacaatcttgccatcacggacaacttcggcatctttcgcctgtaaattgaccaatttttcaacggcattggaggcattgttgcgcatccgttcttcaaagacctgtccaagcagaacaaatgtggtcacgaatgctgcactttcaaagaacaccggctggtgagttgccatcgcataaatgctgtaaacatatgccgtggtcgttccgatcgccactagggtgtccatattggagtggtgttttttaaacgatgcccaggcactattgatgaatgggccggctgcgacgatcatcacgatcgtggtcagaataaacattgtccattccccgccaggcatcatccagccgaatggctttagaatcatctccgccaacattggcagcgaaaaaatcagtgcgatccaaaatcgttttgtgatagtcattagacaacctcaactttccctttgaacatgtccatgccacagctaaaaccaaattcgccagcctggtccgttggcacttgaaccgtcttggtgacgttgactgggagttcttcagaaaagccgagttcattggaatggacaacatccaagcacccctggtcattaatccgtttgaaattgatttcggctggcacaccctgcttcaatttgatgacagatggctgatagcccccggcgacggttacgttaactgtttgtttattttcattcatgattgattcctccatttatttaatcactaatttgccgtgaaacatatccattccgcaggcccattggaactctccggattggctggtatcgatttcaactgattctttttggttctgcggtaacgcttggttgattccaaagtccgaaaagacgactcgatccaaacaggatgatgaatctgttcgggtaaagttcagggtcgcgggaacgccttgcttcaacacaaccacttccggtgaatagccacctttgacctcaacatcgacgatttgctgatcatcgttaaccttggcgttggtttgagcaacttggtgcttgccgaagaaccaccagccgataaaaccaatcaaggctaatccagcaattaaaacaactattttcaaaaacccatctcccattcgtccaaaatctacatgtgtaaactttaattgtctatatcttatcgccaaaggttacacttgtcaacgtgaaaaacggaaattctttcaaaccatgactacaaatggattctccgaggctgcttcaggcattttaaaaaaagtttccaaattttggttgacaattaaaatcttgtgagttagattatagtcacattaaaatttgattgaaaaaatgcagcgatgaggagagtagattcgtctaaccatttcagggagtcccgttaagtgagaagggatgatggtgatcgaattgaaagtagcctctaagcagtagatgcgaagtgatgagtatcttcggtgtgcaccccttaaagtgccagtgtatcgtcagcaatggccgtacatgatgagacgatttgtgtgagcagatcgtgaatttaggtggtaacacgcgaaagcgcccttaatcttagagataagattaggggcgcttttttcagtcaaaaataaaatagaaaattggagtgtggtttttatgaagtttgcaatgattggtgcaggcgcaatgggattacgatatggtattttactgcaagaggctggcaacgatgtcacatttatcgatacatggcagccacatatcgacaagattcgtgaacagggtggtgtatatgtgatgcgtgatcataaggaccgccatttgactaagattaaattggaaaccccagaaacctttgatggccatccggacatgtttattttctttaccaaacaaatgcagctgcaagattatcttgatcgctgttcacatttcttccacgaagatcaatacgccttcactgcgatgaatgggatgggccacattgaaaaactacagaagtacttcgctgatgacaaaatcattggcggaaccgcgttaattgcgaccgtgcttcccggtcccggcgaggttgacttcatgggtaagcggggtgccggcaagatgaacatgtgcccactcaacgaaaagccggacgcaatgtgccaggcactcttcgatgaactgcaaaaagccaagatgaacccaaccttaacggatgacttcaccggaactttgatgaccaaggttatctttaactcagttattaacacgatttgtaccatgttcgagttaccaatgggtgaatttggcaacttcaaaggggcttatcaaatgggccggcaattgattgatgaagcctatgacatttgtgcccgagctgatatcaaattagtttccagccgtgacgaagaaatggctgcccttgaccacaacacccgaatcgatatgccgcttcattacccatcaatgtatcaggatatgattaaggaccggccaactgaagttgattacattaacggctacattgccgaacttggccgtaaataccattatgaagccagcacccatttgtttgttacccaagctgttcacctggcagaatttcatcgtcagaatttggccaagcaacgtgccatcaaggctaagcaggaggccccagcagctcagacagcatagtagccgaggggatgaacctgataattggcagccattcgctcaagcgtcttaaagagatcagcttgctgatcacgggttccagagacttcgagataaaatgaatagacccctaactgcgttttggtcggcaaggacattaatgccaccagatttaattggctggccgcaaagtagccgagaatgttgtagagggttcccgggtgatcgttgaaagccggcgtgacaaatagtggtgccttgaactggtcagtcactaatgtttgctgggcaagcctatccaggtgcgctcgtcttgatttgaacacaatgaaccgcgtgctgttatcgtcttggtctgcgacattatccatcattaacggtgcggataaatcgcccatctgcgattgggggatgatcgccgcgtcgcccggctggccggactggaacttctccagtgaaatcatgtttgatgatgtggtgatgatttgcacgttggggatggttgacaataacttctggcactgaccctcagtcttgaattgaacataaagtcgtttaatttgttgtaaatcagcaacgtttgccaccaggccaaaatcaactggaatggtgacttcgccgatttccgtgacgttggcggtctgcaggcgttgaagggttgcggacacataaccgtcaagctggttttctaatggcaataaaccaaggttgtcgccggaaacggcttggtagacttgatcgaaagtgggatgatagtcaaaagtcacgttggttaatggctgggttttaagataagctttcgcggctgcgtcggcaaaggtgccggctggcccgaggactgaaaatttcatgatataaccaccttgtcgttggaattgagataatgctgttattatctcacactggatttcgaaataatgataaaaatgaaagaaaactcttttaatatctgtggaagcggaaaattccctgatacttggaagagtttttgtttttgttaaacaaaagtaaagtcgtttgacttcattccaacgagtaactactattaatactaacgtttaagggggattaacaaaaatcaatgaaattagcaaacatcaaaccatcaaaattcaaaacactgattttaccgctgacggctattactgccggcagtttttgggttagtctcaaactctttgacatcgcgtttaagcgggtcgattatgtccctgaaacttcgaaagaaaagcagcagtacgccgatctctactatcaatatgtggattggttccatcaaatgccctctgaagaatggtatttgaaccgcaatgatcccgacaagcggatggtggcaacctacattccggccgagggcatttccaagaagacggtcatcattgcccatgggtataaggggaaccgggaaacaatggccaattacgccaaaatgtttcacgaaatgggctttaatgtcctgacacccgatgaccgtgggcatggtgagagtgccggcaaatacatcagttttggctggctggatcgtttggattacctgaagtggatcgatcaagtcattgaccacgttggcgaagacggtaaaatcttacttttcggcgtcagtatgggtggtgcgacggtggaaatgctgtcgggtgaacgcctgcctactcaggtcaaagccatcattgccgattgcggctattcaagcattaaggaagaactcacttatctgttgaagaaacagtatcatctcccggaatatccggttgaaccaatggtgagtgaaattaacaaacgggctgccggatttggcctcaacagtgcttcatcggtcaaacagctggccaagaacaaacggccaattctatttatccatggcggcaaagacacttatgtgccggcccacatggcttacgagaactaccaagccacccacgcacccaagcaaatctggattgtcccaaacgccacgcatgccgagagtttctggtatgatccggtggcttataagcggcgggttcaggaatttctgagaacttatttttaaccatgcaaatcaactgaaaaaagtgttggacatctgaaaatgcccaacactttttctatttataatgacgtcatttatcgttttcaagtttacattaaaccaactggttatacttacgaaaagtaagtctaaatgttggcattccattttcagcatgcctatacttaataattgaaccaaagatatattggtgtttcaccattacatgatatctaaatgaaggagattttgttgatgactaagatgattgcaggacaagctttagttaaagtacttgaagactggggcgtggaccacgtctatggaattcccggcggctcaattaatcatactgtcgaaggactctaccttgaaaaagataaaatgaagtatattcaggtccgtcatgaagaggttggcgccattgcagcttcacctgatgccaaattcaccggaaaaatcggtgtcgcatttggttcagccggccctggtgcaacacacttattcaacggattatatgatgccaaaatggaccatgttccagtgttggcgttagttggccaagtgccacagccaacaatgaataccaattacttccaggaaatggatgaaaccccgatgttcagcgacgtttcggtttataacaaacaagtcacaaccgctgatcagattccttacgttgttaactaagcaatcaaggaagcttatcgccaaaagggtgttgccgtggttatcttgccagaagacttaacctctcaagaaattgattacacaccaactcgcacgccattaacggttgctgacgatttcaaacagagcgtggatccgaaagctgtcgacgacactttgaagatgattaaagaagccaagcacccattgatttatgcaggccgtggcttgttgggcgctcgcgacaccttaaccaagttctctgagcagtttaacattcctgtgatgaacagtgtgccagccaccggtgtgatcagcaccgaccatcctaactttgtcggaacgactggccgtctgggcactaagtcaggatttgaggcgattcaaaacgccgatttgatcttattcttagcttcagagtatccatttgccaactattggccacaagataccaagatgatccaagtcaacaataacccttacgatattggtaaacgaatcgacgttgattacgccgttatcgctgacgccaagagttacttacaagcaatgattgatactggtgagagtcggccaaaagatgcttggctcgaagccaaccaagagaataagcagaactgggacaaatggctcgagcaattggctgatgatgacagcgatggtttgaacgccgaatcagttaccaagaagattgccgagttggctggtcctaacgatacctatgctgtcgatactggaaatgtttcagagtggggtgtccgtggcctgccaatgaacaagaaccaacgcttcgcaatttccggattgtttgcaaccatgggctttggccttcctggcggtcttgctggtgctttgagcgttccagatgcgcaagcttggtcactctctggtgatggtggttttgccatggtcgccccagacattttgactgaagttcgctacaagctgccagtgatcaacgtggtcttctcaaatgaccgcttcggctttatctggtacgaacaaatgcagaccaagcaacacttctacggtgttgacttgaacgatgctgactgggccaaagttgctgaaggcttgggtgcaattggcttcactgtcaagagcattaaggatctcgatgaggtctttgctaagatcaaggatctgcaggcctctggcaatcaaaagccaatcgttatcgatgccaagatcaagcaggacgatccggtcgcaactgcctttatgccgttggatgctcaaaagtacggtgaagagaccgctgaaggatttgcaaagcaatatcacattgatcgcaagcaacaaccatcattggaagaactgctgcgttcaaaggaaaagtagtcgatatatgagttcgtatgaaagtggtcaaatctttacaatgatttggccgcttttttacgtttgcttcgtggcgctcagaattaaaagaaactgaaacgctgccggacctgtgaatgagttgctaatgttacaaaacgattacgacaattaggcgaagattgatatacgagtttgtgaattttacattaatgaaacattgttatatcagtctattcatcactaataagattgtgcataatcaaatggtaaccgctaacttaatatttggtaaaggtgaaaatgttacaccaacatttcattgacatcatcctgtaacgtggcataatgagtttaatcttttagggaggtagcatgattatgaaaaaatttgcaacaatcattaccgtagcttcactggcattaccacttgcttttgcagccccattggccgtatcagccgcaacaacaccgaccacgactgcagccaagaccaaaggtaccacttacactattgctaagaacggtgttaagaacttcaaggcgcgtgcatatcacattaagaagaacattaccttatataagggcttcttctatgccgatgctggcaaggtaacctttacacctaaaggtaaattgaccaaaccaatgacatatagtgttacccgttcggtcacagtcgctgcaactaagacatccaaggctaagacattcttatatgttaagggctatggttacgttctttcatcacaaattaccaaaggacgttacatgtcagctgactaattgaatttgaataaatgattaagcttcatccttctataatctggtcaagagcaattgtgttcttggcctttttatatggggtataattgagaaaattgatattgaagaggcgattgcagtgactgcaactttaactttaattaccggtgctgataaggggatcggctttgaaacggcgatggcgttagctaaactcggccaacatgtcttattgggatcccgccatcaggatcaagggcagcaagccgttgataaaatccggcaggcaggttatgatgccgagctggtgattttggatgttaccaaacaaagtgatattgaccgagccaaggcaagaattgatgaaaaatacggttacctggatgttttgattaataacgctgggattgctttggataatcacgaaaacgccgaaactttgtccacgaatgtgatccgggctgagtttgatgttaatttcttcggcaccgtcagcatgatccaggcatttattccgctgctaaagaaatccaagtctgccaagattatcaacgtttccagcaatatgggctcgctggggctggcgtcagatccgaattcgcgcttctatcacgttagctccctgggctatcaatcctccaaagtggcggtgaacttcgccacgattacatttgccaaagagctcaaggatacccacatcacagtcaattctgttaacccgggatggaccgcaacttcctttggcggccgtgatgtcagccagccggtgccacaagggatgcagtcggtccaccagggggcccagcagattatcaagctcgccagtgatcctaccaatgaactgaatgggacgtttaccgagaatgaggggacgcttccctggtaagttgagtctattcaaaaaacaaaaacggcaccaactcgatttgctcgggttggtgccgttgtgcgatggtcattcattattcactttggctaataactttttaataaaggcaatgtagattaaaaacttgtcattggtcagccggtaatccagaccagttcgtttgtagatcatctccagccgataacgaacggtgttgggatgcgtaatcagagcttgactggtctttttgacggattcgttttgtctgaaaaattcccggatggtttcaaacatctcatgattctccaataactggtccatctcttccgggtacagacgactatcttgaactcttgagagctttttcaccaggtcccacaggctgacgtcccggtaaaagattggccgtcgtgaccagtccaaggttttagcgatgttgatgccgaagctggcctcaatataggagcgatgaatttttttggccgggtgggcattggagacaccctcgtagacggtaaaacgaggaatgcggacattactaatcagccgtttaaaaggaatgcggtcatcgggctgcaattccatttgttcgtggtcaaagaaggaaatcgcggtcgcaccatcagctgattcaacgataaagtaggttttgattcgtttttcctgttggactcggtcaaaaaacgcccggatttgattcatcaggttgaactggacagcaattcgttcacttggtttgggcatttccgataatgagattctggcgactctcactttgagactgtataggtcaacattcttcaaactggagatgaagtcgaagtctttatccgaagcggaattggtttttaataaatagtccagatccaaatcggccatcttattgatccggcggccctcaaacagaatggcgttaatgtcattcatgatttgaatgtaggtggtattttcccgaatttgaaatagcgggaaggctaagtgcgtacagtaatcgattaacgtctgggggatgtctgattcctcattgtctgcgtaaggcttaatcatcaagcagctggcttgtttttccactaattggtgaatcaacgttttggctgtctcaatcttttcgggcatcatccgggaactggtaatcacgatttgaccggcctgtgcccagccgtcagccgtgccgctgtccataatggtaatcgcgttgaccttgtgattggccaacggtacctggttgacttgaacaatgtacttttgctctttattggcgattttctgcaaatcaatcacaaatctcacctccaaaatccgacggtttcattaccattatggtaacgcttttttaaatcttagtacatatgaattgccaaaatgatagctgttttgttatcaaatgttttgtcgagagcgattttggacatttgtgctaaaaaaacgttaattttttggaggaagacacaaaacttttaggctgtcgggatgatacactcatccttgaaagatgacatccttcaacatccttcaaaacgaaagatcgagtgcttattagaaggtgtacgccatgtatttacttgacgtgattcaatattgtcgatgtcccccaattggggaatcacccttccattgccatcatgacgcttggagttaagatccccttcagagtgttactagacttacgagtggcagaagctgttagatgatgcagtaatatcaactgagagtgatatttaaccactaacatcggcagattagtggttcatcattgatggcaacatgcaccttgatggcagcaaaaagcacgttggtaaccagcattcagtgttggtcatcagcgtgcttttgtttattataaattaaagttcaacgccgttgacaatgtaatccggcttatcgcccttgtccattgccacagtattcttcgcaacaatctcagccatggcatcacgtgcttcaacagttgcgttaccaatatgtggtgttaagatgacgttcttcaatgctttaaagccatcgtcaacttttggttcggcttcataaacatccaggccggcaccggcaatttcaccgttttgcaaagcggttaataatgcggtttcgtcaattagcggtccacgggcagcattgatcagcattgcgctgttcttcatttctttgaactgctcagctcctagaagatgatgggtttctggagttgccggggcgtgaagggtaatgacgtcggcgttcttgacgatttcatcaacggtggtaaatttagcacctaatttttcttcggttgctgaatcaagttgatgacgttggttgtagagaatcttcatatcaaatgcgtgcattcgtttggcaaccgcctgaccaatttggcccataccgatgattcccaaagttttgcctgcgagttcgtgacccaagaagaacagtggtgcccagccagtgaagcccttggtccgcatgagttggtcaccttcaacgactcggtgggccaaactaatcatcaaagcacatgtgacttccgcggttgaagtggtcgaaacctttggtgtgttggtcactggaataccctttgatttggcataatcagtgtcgatgttattgaatccggcaccatagttggcaatcagcttgaggtttggggcggcgtcgattacatcagaatcaactttcgtggaaagtggtgtgatcaagaagtctttgtcagcaacccgcttgctgagttcatccttggtaatcagattttgactgtcatcaaatacatcaatgtctaatccggcatccttgagaatgttcaaggcatgctctggaattcgacctgcaattaaaactttagacataaactcactccctaacaaatatttcatacaactccattatagggcatatcagggttgtatgaaaccgcttttacgagtaatgctatcaactgattaactgaatgacagtgacaatttggtagggaaaacccatgttgttttaagctaaaatagatcttagaacgactatacgttaaaccattgttatatgcattaatcctttgatcggtttcgctgaaaaaaccaggtaacaattgaaccaattaggataacgacgcctataactaagaaaataaggttcataaccttatcaactatatcagcagtccccttataaagggtgtatccgctatctgcgacgatccaaatgccgattaatacgctaagtaatagcccaaccaccggaacaactccagctttcattttctttttcatacgtaactcctttcaagttgtttgggaagtggattatgtaatatggtgacactagagggttgtgcacttcatctagggtcaccatgccgaaattattgttgtaaaggttctgaatagcttacatatgaggcgcctttttttctggacgtatatttgattccttcacctataccataggtattccaaactggtgccaaagaaaattttgagcttccaccagaagtatttgctaacacactgttggaaagagttgatgtgttggtaaaggtcggaccaataagtttcattttaataacctccttaggctaaatgacttccttctttgaaacccttaccaaaagcatctctgtgcttccactcggagcgtgcaagccctatcatgacggttgtccatatattgccaccggataccattgctagtttctttgacgaaataggcaccacgtttaaagatgtgagtttatcaaaagtattttgactgtgattcatgtttgtcgacctccatttgttcgatttgccaaaaatctcgcgagaactttatgacatctttaggatctcatcaacatcgtggaagttcaagctgcaaattatagacatggcgataagtgaacgcgtttatttcaaaaattcaaagaataattgtcatatgaggtttgaaaatcatattggattgaaatagattaaaatgccgataatacatgcaagtaggaagattacccatgtgatcgtgatgtagataccaacatgtccatgggaataatatttggtgctgtcaagatttttattctgcattatctacttttcctttatcaagttatagtatttgtttctgttgcgtagtaattgggaatgagtaccactttcaacgatcgttccattatccatcacaatgatgcaatctgcagcctgtgcgacttccaatctatgtgcaatataaactattgttttgtttggaagtgatcgcaaattagtgagtattttcttttcggtcaatacatctaagttgctagttgattcatcaaatactaacacctttgcgtcgcttattattgcacgagcgattgcaagtctttgcatttgtcctcctgataaaccggtgtcttctgataagatagttagatatcccttaggaagccttttgatctcttcatcaatttcagctaattgtgcagccttttttacttgggcaagggttttatcattttttgtcccaagtaaaatgttatcgagtaccgaacctgaaaatatatacggcgtctgaggattatatgcaatatatttccgcaattctgatgttggggcagtagttgtactatagtcattgatcatgatagttccagtcgatggtaaataaaattttatcaataattttagtagagttgttttccctgatccgctagatccgataattgctgttgattcgttacgattaatagttaggtttatttgttttaagattggttggccgtacttgtattcaaaagaaacattagaatattgaataaagtttagagtagactggtccttattctcagaatttctaatactctgattggtttgttgatctatcggtatgtgcaatatttgatttagccgcgaactggcagttcctgcatgttgaagattgttctgcagattaattattgattcaaaaggaccaatgaaatatcccattaacgaattaaatgctactaactgtccaactgtaatttgaccattaattgccatctttgctccggaataaagtacaagtaaactcaaaattaacccagttgtagactttaatgactcttgcaatataacggcaacattatattggtgatcagctcgcaaggtatttacaaactttttgtcaagggtttcatacattttgtcctcagcattcagcgattttatcgactccattccccttagatcttcaataagttgagaattaaggtctgaatttttctccattcgattgtaattatatttgtggaagggtttataaaagataagcataattataatataagcgggaatgccaattgcggataatataaaaagcctcatattaatacaagataagacaattccagtgatgataattacaccactgtccaaaattgtgataactactgttcgagataaagtcgaaataatcgtttcggcatctgaaaaccgtgatgtgatttcgccgatctttctttctcttgaattgtcaaattaagtgcaacacgacattaaagaatatttcataaggcgttttccatccgagacatttacggggacgattattcatttgttctgcatatgcttgtatccggcggtcagtaattgaatcaaggtcagttccttttggcaaatattcgcgaagcaagccgttagtattttcgttagttcctcgttgccaaggagagtgaggatcgggaaagtagaagggcgtaccaaacttatcagttaaacattgaactttggcaaactctttacccctatccggggtaatcgttaacgatctaccaggccatagcttcattaagtcgctcaaagtatccgtgactgcttctgaagttcttttagcagctttaccaataagcaggtaacgagattttcgatcaaccaatgtaacaacacaagcctttccgcttttgcctaacacggtatcaccttcccagtgaccaatttctacacggttgtcagcttctcgcggacgatcatgaatcttgtttgggattggaatcttgcctcgcttttcttgataagctttattgtggcgagacttgccgtgatgccttagatggcgcacggcactagagctgccagatttaaacaaattatcaaataagccattgaaaatcccacggtaaatagtcgtggtactgatctgcaccggatacttttcgactgccaagcgattcgatatttcctccggagaccaaaggtcttcgcagaagtgttctctcaccacttcaaacacctgaggattactcaagagagagactctgccacagttgcctttgcgctgtttgtacttctcctgagccttcgaaggtgaataggatttaccagtagaattacggcttaattctcgagaaatggttgagtaacttttcttgatatggctggcaatctcacgaagtgagtttccatgattcctcattaaaaagatagtttcccgttcatctatggtaatatgcttgtagtgatccatggttaaattcctttcatgattgttttcgcaaacatcattttacagaaatttggccatgggccattctttatttaattagtgttgcacttaaagtgtaaattcaagcttcaaaaaatgccattggtagtttgaataggtggcgaatatatttcaacaaaatttctagagatactcgctgcccaagaaccattgataagtactcttgagtgtaagtgaagaagccatggaaaatgtaggctagtaataatgagagtgcagtggcacataatacatcggcctgcccttttttaaccattgaatcaataatctgctttaaaaaaaatgccccactaattgttatcaatgttgataacatagttgctaagagtacggaagcgatgattcctttttgcctaaaaagtaattttgaagtcgacctaagatcgttagtatcttctttgattacggtgtatttatcagttggagtcatgtgaagtgaaatgcctgtccaatccttaccaaatgaattgtatgacatacgaacagtttttatagatgggtcaggatctgcaatggtgactgtggactttgacaatttacatactacgacataatgctgtccatattttttattaacgtgggcaataaaagggatcggaatatctggtatatttccttttaaaaatgatatgttcgtttttattgcctttggggctaaattaaaatgtgttgctgcgtgaattagacccagtgcagtggtaccatttttgtctgtttgtgcatatttacgaattgttgatattgatactcgtgacccataatacttcaatatcatcgccagagctgcagccccacagtctgtttcatctaattgactgacataataatgattccacatcatatttttcctccatgaatgccatgctcaaatttttaatcgacaattaaaaattaagtaagatattttctaatagacatattgtaacattattttggtgattttatataaaatattgtacctaataaataatattatacctaaaaatattgatgtggtatataatgtttataattagacaatggactctggaggactagttatgaatgtttcacagaaaatacaatattgcagaacactaagaaatcttacacaagatgaagtcggaaatttgttgcacgtatcgagaaagacaatttcaggctgggaaacaggaaggagttctccagatattctcagcttagtcaaactttgcaatctttttgacatttctcttgatgatttgctacgtgacgaacatatgattgatcgtgattaccatggatagggttatagttaatggccaacaacaagaaagcttcaccaacgagatagaaatgtcattcttgctatgtattttaaaaatttgtagattgctcctaggttgcacagaaactcgttaaatatcatctttacaaattactattgacattgtactaatggatgtctacaatatttattaaacaattagaaaacgctgtgagaaagttgagtagcgtcatgacaacctgaagcgagcttcgtttggtgagaggaagcaggaggattgacgcgaaaatcccttttgagcgatgtaccgaagaatgacagtaacgtgcattggtgacacccattatcgtgttagcgtatcgcttttttggccgtacgtgaaaggcagttgtagcgatataactgcaaatataaggtggtacagtgcagtaggcgcccttaattcagcattagctggatgaggggcgcctttttagttactcaaaatttggatcgttttctagtgaatctagataggaaaagagttggtgaaaatgaaatctcagattgatattagtcagattaggaatcaaattcaggacttaaataatttattcattaaaggagatcttcatttatgcaggaattacatgacttaaatccaaacccgttacggaaacgcgattatttcgtcgtcagctcaatgttatttggcctctttttcggggctgggaatttgattttcccaattcatttgggtcaattggctggggctcactggctgcttgcggcggttggctttttagtgactgcggttttgctgccgctgttgtcggtactggcaatcagtgtcactcactctgaaggggtctatgacgttggtaagccgcttggtcccgtgtttgccttgacattcatggtattaattcacgcaaccatcggcccattatttggaaccccacggacagccacggtgccatttaccgtcggagtgcagccactgctgccgtcatcaatggcgcatgttggcctgttagtcttttccgccgtattctttggcttagcttttctggtttcttataaggaatctaacgtcatgacgtcagttggaaaagtgctcaatccagtctttttattgctattattcagtgtttttgcattaggatttgccaatccgatgggcgttgccggcaaacaagccgtcaccgctgcttacaagagtgattccttcttcaatggtttcctgcaagggtataacaccatggatgctctggctggcctggcatttggggttaccgtcgtcacggctgttcgccagttgggaaagaccaagcccagcagtaatgccaaggtgactgctaaagccggggtcttcgcaacgggggccattggcttgatctacctcgggttgatctggttgggtgccacgacactttcaacgtataaagcatctgccgacggtggtgtggccttcaaccaattggtaacttattacctgggtggtctgggtcatgctctgcttgccactttgttaaccgtcacttgtttaacgactgccgttggactggtggctgcctttgcacaagattttcataatcatttctctaaggtcagctatcgcggctggttaggctttatgtgtgtcgcatcgtttgcgactgcgaactttggcctcgatacgattatccagtggtcgacaccaatgctgatgttcttgtacccattcgcaatggttttgatcttgctgtccgtcttctcaccgttgttcaaccgtgatccactggtttatgcactggtcgttggcttcaccacggtcccagccttgctggacatggttgctgctttcccaccagtcgtgagtcaaagtgcctttggtcaggcgttgggtgctttccagcagcacgtattgccatttgctaatctggggatggattgggtggttcccgctgctgccggtgccgtcttgggacttggcctgcattttctccggccggttttgggcagagccaaagcaccttcatctgaagaaaataatgattaatacagtcacataatgttttaaccgataaaaaaatcgttgagccagccaccagtaatggccagctcaacgattttttgtgatttaacagctgattattgtaaattagtaaatgcgccgttttcttgaagcaatttcacaaatccaggaacggtatcttgacggttccaatcccgctgcagttcgcagactaattgtggaatcgtaatcaggtgagcgccggcttgttcaactcgacgcaaggcagtttcgtgcgcgatcgtggacgtgccgccgactgcgtcgacaactgggtagacatcaaagccttcagcgatggcatcgatggttgggaacgtgagacaagcttcggtccataaggctaaaataataatctttttccggccggttgccttgattgcatcattgtaatccttgtcttcccaagcattgatggaagaacggtcgtaggaaggggtgtcgcctatcaagtctttcagtggtttaacagtatctgaattgcgttgattatgggcattcactgtcgaaagcacaattggcagtttaaagagtttggctgcttccacaaccatttctgcattcttcagtaagtccgcatgccgcatcgaaccaattgaaccaatttgcactggttggtaatcaatgattgttaaaacggcattgtcaggtgatagtaagcggtcgtctgcgcctcgtttgtcaaaacttgtcatagtatcttcctcctcaaaattaaatccataagtcctctagaattcgctttcatgatacaacgatcagggagtcgatactactaattacaccttgacctcaaagccttgggaaaggattcaattgttgaaaaatttacattgaagactaacatggaaattggatgaaaaacgtagtaaataatttcaaagcggcgacaaatgaaatggttaaaaaattttttttagcaatggtgacaatcttagtttcagttctaatgcttgggtcggtcaattctcaggccagttccaaagtgaataactacatagcaagtcacaatatttctcacaatcaagtctcaagcaagatttggggcggttttccacattataaataccgtcacggtaaaaataagcctgagggcgtggtcgttcatgaaaccgggaactcccactccacgatttttggcgaaattgcgtacatgaagaagaattaccgaaacgcctttgtccacacttttgtcgatgacgaccacattattaacattgccagcaccaagtatctctgctggggcgtcggctatcccggcaatgcccgctttgttcaatttgaacaggtcgaaatgcacagtaagaaatcattcgccggtgaggtggaaaacgctgcttactatacggcctatattttgcacaaatatcaccttaagcccaatgacgcggtatacgacggccacggcaccgtctggtctcatggtgctgttgcccattatcttggcgggtctgaccataccgatccaaagggatattatgccaatcgcggcaaaaaatacttccaccaatcttataccatggcacaattttatcagctggtgttgaccaactatcacaacctttaatttggtgaaatatcaaaaaaacctttacaggtggaatcttttagattattatcaaaagagtaatcgttactatttgcaagggagaggatatctcatgttacataaattttcgggcttcaaggcctggctgttagtcgtagtggcagttgctttaggcattggcctaaccggttgtgcaagcaactcagccagcaatggcaaaatcaagattaccgctacgactgatttctatggcgaggtcgcaaaggcggttgtcggcagtaaaggggacgtgacttccatcattaccaaccccaacgtggatcctcacgattatcaggcatccacaaaggtggccaaggaaacggttggctcaaagattgtcattgccaacgggattggctacgatggctggatgaataatctggttaaggacagcagcaaggttgactatatcaaagtcggtgaagatttgatgggtaagcagaacggcgacaatccacatttgtggtataatccggcaaccatgcctaagttagccaatactattgcgacaaagcttggtaaactgcagcccaagaacaaggcctactttaagaagaacgctaagaagtacatcgcttcattgaagccggtcaatgataaaattgcccagctgaagcaactcgccgcaacaaagaagaacaaagaagtctacgtcagtgagccgatatttgactacgcccttgaagcaaccggctttaaggttggcgacacccagttcgaaaatgacactgaaaaaggcgtcgatccatcaccgcagacaattcgaacgatgcaaaacggcatcaagaaccacaagatcgccttcttcgttttcaacaagcaggttgacagcaagactgtcaataatctggtggccttagcaaagcagaacaaggtcccggtattaccagtaacggaaacattgccagctcataagacttacgtcagttggatggattcacaatatacccagttacttaatattttgaaatagttcgtatcaaaaaagccgagaagtcagaattgatttctcggcatttttgtatttaattttaaatttttcgatcagcgattagttcaaatagccacgccaaatccagccgccatgattgccgacggtactgcgaacgtgatagtaaattgcatagttaccggtgtttttcttgtacaacttttcatgcgcatcggttacccaagtcacgttggggagttctgagttgtagccataccgggtgccaaggtgcttggagtatctggcacccttggtggttgtgtagtagtgcttgcccatattggcgcgccaaactaatttgacggatgccgaacgagctgccgaatactgcttaccggatgggccaggaatcttgacgatttccccatcatttttagaactggaaccagagttgcttggttttgtcgcactgctggaacttgattcactggaagcactcgaggcactgcttgagttagcgttggtgttggtagaagctgccgctgaaccggagttcaagtagaagctgttatttaactggctaacatccaaattctggttgatatttgggaaccggtagtcggaagcccattgccaggcattggctgaagggtacttcgacccggttggggttgccggatagtcggcaatccagccctggttggaggcgttggtgtcaatctttacgcccaaccaacttgccatggtatataaatcggtcttgttatagccgccctgattcaaagctgaatcaaaagctgccaaattggcatcgttattcgctttggaaattccacctaattctgaagattcaaagtcagctaccatcacgacatctttcgaactggtaactgattgaacggcattcatgaagttttgggcttcctgagcggcttgatcagtcgtcgtaaagtgaacaaaatgatagaaattaatacttaaccctgcctgctgggcatactgcacctgttgagaaagatacggattgatatatccggttccctcagatgctttaatcgtgaccgctttaaccccattttgagctaatgtttgataatcagcggcagttaaatttccctgccaactggaaacatcaaccatgttggcgccaggttgggtactggacggcgtcaaagccgcgtgggcagtggcgttcgtcccaaataaaattcccccggcgaagagccctaagataacggcccctcttttgaaacttttcctcataatcactcaactcccatctatgtatatacacatcactgtgatactaacatgaatgagggcctttcggaagaatgtttacttattgtttccacttcgtcgatcaagtgaaaagctccagtaaattgcgagtaacaaaacggctgcgattgaaatagttgtaatattattggccatcgcatgggtgctgacctgccaggcaacgtaaattaacgcgagttggaaaacccacgataggatggactggccggcaaactttttggtaaaaaatttcattagataattcctcctattattctggaatgtcaccattctcagggatgtaatcaattgaatcggcaattcgcttgggaattggaatctgtggatcaacgtggggattgttaaggtgaatcaggttgtaggacttgcgatactcagtcggcgataacccggtggcactcttgaaacgccgcatgaagacctttggatcgttgaagtaagagttgtcggcgatttgcttgatcgacatatcggttcgaatcagcagcagtgtcgccacttcaattttgacgtgattcaagtactgcaaggttgtcatgccggtgcagtgtttgaacagcctggtcaaataatctggattcagatgactgcggtcggcaatctctgcgacggttaaatcactggacatgttagcccgaatccattctttgagactgttaatccgcgagctgtcttcattggcatcgggacgattgaagtatgacttgtacagctgaattaaaagtgcagaaaccagatagtcccgttcttcgataaatgataattcattgtggattgatagaatctgatgaatcagaatggttgcctcttcataatcggctaatttgaaatactgcggcagaaaaatttgccgcttcttgctggtactggctttaactttttcagtcatgtcgtcttcatcggcagtgagcgtatcttctttgtgctgggagaaaaagtgaacccagtagaagtcgacgtcacctggggaatcttgataaccataaaaagtggtaaacggcgggacaatcaagacttcgtgggtgttgagggtataccgccgatcgccaatctgtagataaatcggtcccttaatacataggattaattcataatcacccttatgatacatgcgtcgatggtgccagcctttatgagctaaaaattcaccacctttatagtagagtagcgttttttccattgtgaacgttgagaataacatttcaagccaacctcctaacggtgtcggaaatcgtcaccaaatgtacgcaaaaatagttttacggcaatgtcggaaacagtcaccaaatgtacaaaacagtgtcactattggcctcgtgacgctatcacggaacccaatattttctcaactggtcggatatcatcacttcttttgccattatagacctttttttattatttggaaacgcttactataagacttgtaaaaacaagttatgttttgaacattgatttttcagaaaggaagttgaggccaatggttcaaattgacgatcgactaagaagctcaccagtttcttaatcgggttagtttcagtgtttcagcaatcatttttatccgcccaacaatgagcgggttaccaaaattaatttatttggaggaattatcatgagctcaaatgcaaacgtagattcaaatacggcaagtgctcaagcattgcttaacgacacgttaccttggcacagaaagattacctatggttttactgatatgtctggtaacttactgtactgtattatcagttcttacatgctttacttcttcaccaacgtcttcggtctctctgttggaacggccggtgttttacttctgatcggccgtgtctttgatgccattggtgctcctgtcatgggtatcttggttgaccacacccacagtaaatatggtaagagtcgtccttggttcttgtggatgtcattgccatttgccatctttgtctggttactgtttaccaccccagcattgagcggcactttaaaagttgtttacgccggtgttatgtacatcttagccgacttatcatacaccgcaatgtccacaccaatcacttcggttttgcctaacttaacttcaagtaccgacggccggatgcaagccaactcaattcgtttggttcttggtaacgttggtaacttcttcgccgttactttcatcattccattcgctggtttactcggcggtgggaacgagcaaaaaggttggtcattgactgttggtgtttactcaatcgttgccttccttctcttaatcatcgccttctttgatatgcgtgaaaagaatatcgaaaacgaaaaagtgattaccattaaagaaagtttgaaagccactaaaggcaactggccttgggtcttgattgttgttgccaacttggcttactggactgcatttatcgttcgtaacgcttcaatgccttactacttccagtacaacatgggcagcaagggtctgatttcattcttcaacggtttcacaattatccaagttatcggaatggcttcagttccattctttgttaaatttatgcacaagtggggcaccacaatcttcttcctgctgatgaccatggttggtcaagcatgggttggtttagctggttcaaacgtcacttccgctctgatcggctggtgtgtcgcatgtatcggttcaggtagtgcctgcacaatgttcttcgccatggtcggtgataccgttgactttggtgaatggaagactggtatccgtgccaacggattcttaactgccatcggtgcttcattctgtatccaaatgggttcaggatttggttcattcattgcttcaatgcttctcaaaggtttcggtttcaacgctgccaatgcaactcaatcaagcgcaagtcttggtggaatcagctttaccttcgtctgggttccaattatcatttacgcaatcagtgttatcttgatgattatgtatcgtaaatgggaaaaccacgaaccagttgttaaggctgaccttgcaaagcggaacgccgaagctgaaaagaacgctgaagctgcacaagcttaattgtgagattgattttaaactttaggaggaacgcatagtatgcaagtttataccacaccaaaattaaataaggtcaaggttacttcagatttctggaaacgctaccgtgaactcgtcgtcaaagaagtcctgccatatcaatggaaggttatgaacgacgaagccgacatttctatttctgaagatccccaaaacaatggccaagacaagaacagtcatgcgattgccaacttgaagatcgctgccggtcaaatgaaaggccaccactatggctttccattccaagacaccgatgtctacaagtggttggaagcggccgcatactcattcgggtatcatccaaatccagacctcaagaagattaccgataatctgattgatttgatcgctgacgcccaagatgacgacggctatctgtcaacctacttccaaatcgacgccccagaacgtaaattcaagcgactccaacagtcacacgaactttacacgatgggtcactacatcgaagcaggagttgcctatcatcatgagactggcaatgaaaaagctttggacattgctaaacggatggctgactgcatcgaccgcaactttggccttgaagaaggcaagattcccggctacgatggtcaccctgaaatcgaattagcactgtcacgtttatatgaagaaaccggtgaaaaacgttaccttgacttggcccactacttcttgaaccaacggggccaagatccggcattctttgaaaagcagattcaagctgatggcgacagtcctgaccgcgacctcatcccagggatgcgtgatttcacccgtgagtactacttggccgcagaaccgatcaaggatcaaaaagttcctcatggccacgctgttcgagttgtctacctgtgcaccggaatggcttacgttgcccgctacactggcgacaaagatttgttagctgcctgtgatcgcttctggaacgacattgttaaacgtcagatgtatatcactggtaatattggtcaaaccacgactggtgaagcttttacctacgactatgacctgcccaatgatactgattacggcgagacttgtgcttcagttgggatgtccttctttgcccgtcaaatgctgaacatccacgccaaaggtgaatacgccgacgtgctggaaaaggaactgttcaacggtgccttaagcggcatggcacttgatggcaagcacttcttctatgtcaacccattggaagcagatccagttgcttcaaagggtaatccaggtaagtcccatgttttgactcaccgggctgattggttcggttgcgcctgctgtcctgccaatcttgcacgtttgatcgcctcagttgatgagtatctctacactgtgaatggtgatacgatcttgtcacatcagtttatctctaacgatgctgaatttgatgacggtctgaagatttcgcaaacgaaccacttcccatggagcggcgacattcattatgaaatcgccaacccagacgccaaatcattcaagctgggcattcggattcctagctggtccgctaacttcgacttgactgttgacggtaagtcaaccaccttgcctgttgaagatggcttcatctacatcgatgttgatgccaagtcgttaaccattgatttgaagctcgatatggacgtcaagatcatgcgcgccagcaacagagtcagtgctgactttggcaaggttgccgttcaacgtggaccaatcgtttatgcagctgaagaagccgacaaccaagcaccactggcttcatatgaagttgcaacagacgctaataccgactaccacttcgatgagaaattgttagatggtgtcggagttgtcaaagttgctgctcaacgacaaaagttggattccaaggatgcacctttgtatgttgacgccagtcagccggttgagtcagaatcagttgacctgaagatggtgccatactacgcatgggctaaccgtgagaatggtcaaatgagagtttggttaaataaataaatcatttaaagttagcgttttcaacctctttcataattggttaaaatgctgtatagtatgacgagatcctgatgttatttctgacataacatcacaacgaaccccattcgtataaggatcgagcccctccaagcaatcctgcttggaggggctttttgtgtattggcaggtaagacagctggcattttgaggttgaataatgaccttttttggctggaatccggggcattttcaaaagattttcattcttaacgcttacatcatgaaaatgtttcaaaaatctatatactgaattttcataatggcctataataaatccgaaagcagcaaggttggcttgctgtcgggggttcgagtgcttaggaggctattaaaatatgaacaaaaaatctggaatgatgtcgttttcgattctgatgctgtcattattaccaatgtcaacgggggcgacggcttccacaattcccggattaatgaaacaatttccagcggtttcatcggaaacggccgagctgactgtcaccatcccatcattcacgatggccgtagtgattatcctcagcagcttgattgtcaaacgaattggcaccaaaaaattagttctggcaggaactgcattaaccgcatttggagcaggactttcaatgttttcaccaagcgttgcagtcttgttgattgccagagcgattatgggagctggaattggagcttttaacaccctttgtatcagtttgattgatcgcctgtacagcggtcagcagcgtgaacggatgctgggttttcagaacacttttcaaggtttgggggctgccggcggtgcactgggagttggtctgatattgatgtacagtaactggcggatggcgtttggaatttatttgatcagcgtcgtcttgtttgtactgtatcttttctacgtacctgaagttcgttatgataacgatgatccccaaactgtcggtcaagctgacgagaaagtctcttggatgtccaagttgcagtttggttattattggatcgtcatgttcatcttgatggtgttctacatgactgttaatgtgaaaatgccaacctacattttgaataatcatttcggcgccttgtcagttggatccacggcggtcgttgtgatgtcgatcggcacgattattggcggcctgatttatggctttattgaatcgattgccaaaaacgccactttggtcatggcgattgccattgaagccgtgggtgtcttcatgatcagtacggccggctcggcgttggcctgcttcatcggggcttttaccgttggttttagctttggtctgtttattccgttcattttttccaaaggactgtcgtttgttcccaaaaaatatggcaatgacgcgacgaatattttgatgatcagtaccaatggcgccaacttcctttgcccatacgtcagcaagttcatcaacatcggcggtactgaccgcagtttgtttatgatgtccggcgtgattgcctcaattctgggaatcatcgagttggtcaaattattagccaatcggccgcgaagaactgttcccgaagcttaatgtttttgtgaattttactaatctaaatgtatttctgaacctctgtatgatattattcatacagaggttctttctatattatgagccatgctgagtgttacacttgagatggctttaatacaaggatcgagtgttaaaaaatcaattcggaatatgagtgtaatgggtgataagatgacaacaattaaagatgtcgctaacgaagcgggtgtttcgatatcgacagtttcacgaattttgaacttcgacgatacgctttctgtgggggaagacacgcgtagaagagtgttggaagttgctgaaaagctgcaatacaagaagcggaatcggcatgtaccaaaaggcggtaaaaagattggtattattcaatggcattctgataaagaagagctgactgatctttactacctgcaaattcaatacggcattgagaacaaggcggccagcttaggtgccggcgttgagaagttgacgtttgattcgatcgataagagtcgggtgaagggcctcagcggaatgattgccgttggtaagtttgataagaccgaagtcatgagtttgaaatcatatgatatcccactggtctttatcggtgagaactatttagcttacgattgtgatagtatccgtagtgatttcgagtcaccggttcgtaagattattgatcggtttattgagtacggtatcaaggatatcgggatgattgccggtaaggaaacgaccgtgactgaaaagcagggcgttcgcgatcctcgagtgtcaacatttgattcgtatttgtcagaaaagggtttgttcaatgatgccttcgttttccaaggaccatttggcccggattcagggtttgagctgatgaacactgcaatcaaacagttgggcgacaagctgccccatggattcttgattggcagtgattcaatggccgttggtgtcttgcgagccctccagcagcagaatatcagcgtcccggatcgggtcagcttaatcagctttaacgatgttgcaattgccaagtataccagcccggcattgacgacggtccacgttcacaccgaattgatgggtgagcgggcaattgaaatgctgacggaccggattaaagaaccgaagaaggtcccagagctgacggtgattgcgacggaattgatggagagggagagcagtttataaaatcagagtggagcaagaggcgctttgatcccagaatgtaaggtaattaagtgattattcccggttttggaatgattgcttaattgccttacatggcggggatcagccgattgttgcacgtttcggcaaagtaaaagtggtgctaatgcaagagtggagcaagaggcgttttgatcccagaatttaaggcgattaagcgattattccggggcttggaatgattggtttgccggcttacatggccgggatcagccgattgatgcatgtttcagcaaggtaaaagtggtgctcacgcaaaataacaggcagggtcaaaagcgaataacttttgcccagcctgttattttagtaaatttaaagattaacatctgttataacgtagaatccaagtcatcaaaggaaaaagcaagcctcattctctaggatgtttttctcaatagcgacggggattctcgtcccctttagaatagttttactaaaatctattgactatacccgataatatagtaaaattaaagcaacagcacaaaagaaagcgcttgcgaaagtgataaacaattaccacttttaaaccctaggaggatgaaacgatggaaaaaggtttactttatccagttaccaatcaatttagacaagatcaaaagttaggcggcttatgggattttaagtttgacccacaagctcaaggtgaggccaagggatggacaaccggttttgacgatccaattaagatgccggtcccagccagctttaatgatttctttaccgacaaagattcccgtgagtataccggggatttctggtacgccaagaagttcttcgtaccaacctacatggatggccagaccattcagttgcgttttggagcagcaacccaccgagcaaccgtttatgtaaatggccaagaaattcgctcacacgaaggcggctttctgcctttcactgcagatattaccgatgcagtgaaattaggtcaagaaaatattgtgactttgaagatgaacaatgaacttcatcgagatgcattgccagcaggtgatacagccactttgaagaacggcaagaagatggctaagcctttctttgatttctataactattcgggcttaaaccggagtgttcatttattagccgttccgaagaaccatatttatgattactcaacaacctatgatgtcagtgaggatcaggcaaccgttcattatagtgtccaagcaactgacggcagcaatttcaaagtcagcctgagcgatgaggatggcaaggtggtcgcaaccgctgaaggacagactggtgatttggtggttaagaatccgacattatggcaggttcgcgacgcctatttgtacaccatcaaatttgagttattggatgctggcaaggctggtgatgaatacagtgatgaaattggtttgcgaaccatcgaaatcaaaggtcacgaaatcttagtcaaccacaaatctgtctacctgcgcggctttggtcgtcacgaagacagcatttatgccggtcgggcatttgatttgaacgttgaacgacgtgatatgaatctgatgaaatggattggagccaactcatttagaagttcgcactatccatacgatgaacaggtctataaatttgccgatcgcgaaggcattctgattaccgatgaagtgcctgctgttgggttcaagatggctgcagccagtttcctcggcggtttaaaccaatcattctttgacggtgactggattgatgaattgtacaagaagcatattgatcaggttaaggacatgatcaagcgtgataagaaccatccaagtgtcctggcatggagcttatgcaacgaaccggatacttcaactgactcggcggtgccatactttaccaagttgtttaatgattcaaaggatttggatcctgaacaacgaccaagaacctttacccttaacgaggacgacacctttgaaaaatccaagtgtttgaaattccctgacttctacctcctgaaccgttatccaggctggtaccacaagtggggatacgaaatctctgatggtgaagctggtttgcgggctgaattggatgaatggaagaattctgacatcgataggccgattgtcttctcagaatatggtgccgatactgaaccaggactgcacaagttgccatcgattatgtggagcgaggagtatcaaatcgaattgctggatatgttcgatcgggtatttgactcctacgactttatccggggtgaacaaccttggaacctggccgacttccagaccgtggaaggcaacatgcgggttaacggtaacaagaaggggatctttacccgggatcgtcaaccaaaagccgcagccttttatttgaagaagcgttggacttcattaccactggattataaagcaggtaaatagcattgcaggagaggtcggaacaatacttaacgagtactggtgttccggcctcgttgtataaaagcaaatagggtgactgaaaaggagtgttaacatgaaccagacaagttttgtcattgacggggagcaactggatctaaatgccaaagatgccaatacatttaaaggctttggctacttgagctgtaacaattcttcccgactgctgctggattataaatgggaacatcgagacagttatgatcagattttgcagattctctttggtggtaagcatccattaatgcggatgttaaaagttgaaatgggcgatgatgccaacacgtcttctggaactgaaccggcaacgatgcgctctgcctcggaaaccgcaaacgttaaccgtggggctggtttccagttgatcgccgacgctaagaaaatccaaccgaacttaaaaacggccattctgcgctggggtgagcctggttggctgagaaaagattggttcaacgccaagtcggctgatccggatggtaaagtgccggcaactgcctatgagccgatgtatcagtggtataaacagacgatcatctcggcttatcagacatatggttttctgatcgattatattgatcctgaccggaacgaaaccaagcatccgatggttaaatggatcaaatggtttgcggatcgcttggaaaacgatcagtctgagtttccgaatgactttccgattagtcggtaccagcaaatcaaaattattgctgccgatcagaactatgaacgtgattttggcgatatgatgattgctgatccggacttgcgtgaacgagtcgaagcacttggctttcactacaacaccgatgatggcgaaaaacagccgtttacaaagttagcagacgattaccatcatgaagtttggtacagtgaaggaattgcgccgatgacgatgggtaagtaccgagttcgcgccagcaatggtgacggaatcggcggccgtcaaagcggcttggatgttgctaaccgactgattaagagctacgtgaaatctcgtcgaagtttgtatattttccaaccggcagtttccgcttattataccggggtcaattacagtcacaaagagctgatcaatgcctgccgaccgtggtcaggttactacgaagtcgataatgtcgggctgcagtgcatgaagcactttactgattttgccaaagccggttgggaagacgaaggtgcttggcggtacttaaccagtgcctgcgacagtcaagtcggcggaactgaaaacctggatcataatcggcaggccccaagttacatgactttgatggcaccagacaaggccaactactctgtgatttttgataatgacagtcctgaagcgcgcacctaccagattctgctgaaaaatcttccggcttgtgaagacaaaccggttgccgtttggcaaagcgttagtcccgagcatactggagatgcatatgacagtcggatgaagcagttacgagaaaccgtttcgccaacggacggtttgctcaaaattattgttgcaccccattcgattgcgaccgccaccacattggatttggctgacgatccggaagtggtctatcatcgcttggagagcccccatgaagaccacacccttggtatcaaatctgatgatggcgttttgtatgaagatgattttagttactcgggctacccagaaaattatttatcttctcgagggaatacgccacggttcactgctgatcaaggtggcgcctttgaagtggtccagaccgacgaaggcaacgtcatgcagcagatgattaccgataagcagcgggctcttgactgggaatattcatttgctcccaacttaacattcggcgacgaccactggacggattacgaggttgccgtgtcaatgaaatttgacgatcaaactcagcagaattcgccaaccggaaactactttgggatcggtttgcgggaaatgaccgacgtcaagggtcgccttgagagtgccccgtatgtctttaaagtagccattgatggtggatgtgagttgattaaggatgaccaaattattgccgtggaacacattgacggcttggatgtttcggcaacgcatcaagtcacgtttgcagcggaaggtaatcatttaactgcgacatttgatgggcagcgggttttcgattataccgacaccgacaatccacattacagtggccgcgtcaagcttgggagcgggtattaccatacccagattcagcagttaacagttacccagggcaaacagccacatttgattgaacacagggtagatgatctcgattcagctgttcaatatacaggcaaatgggatcatgtttgcggtttgggcaataccaaatggaatcgaacactgtcgatggcaagtgccgaccaagataatgtgccaggctttgaatttgacttcaacggatctggattctcactgattggggctcaagatgctggcagtcgtctgaaggtgacggtggatggagccgttcgcaattggaatctggcaccacaagttggtgctgatcggacagagaatatcgttgttcatgggttgtctgccggtaaacatcatgtcgccatccaagttgttggtggtcgttacacactagatgcggtggatttcttaaaataatcaagaaaaaagcgaactgaaatttcagttcgctttttgtatcccttaatattgacgaattttaggtggtgtgtagttcgtcatgaacgtataaatttcatccagtgaatcggagaacagcaccttcttgcggtcagctgccgataagaaaccttcgctggtcatcttatcaaacattttggccaacaggtcatagtaaccattcacgttataaaacacgcaggggttgggattatcccccagccgagcccacgagaaggcctgggtgatttcttcaagcgttccgatgccgccgggaagggcgatacagccattggagatgttcatcatctcagctttgcgggcagacatgttgtcggttaccgtcaaatctgataattctcttaaacgcggtgactcagctcctcgagccactaactgcttggtggtgacaccgtgaattttcccgccttcagccaatacttgatcggacaacacgcccatcaacccgacgccaccaccgccgtaaatcaattcaagatcgtggctgactaaccaagatgccagttttttagtggcggtgacgtatacgggattcgtgccggttgcggccccgcagtacacagctatccttttcatatccagtctcctttgaaaatagtctagtcttattctaccagtttttctgaaaacaatttttgaaaatcgacataggggactataattaaattaccatttcacgaaataatttaaggaggttaccatggaaacctatattttagatgattcagacgacatgtggcagcattttgccaaactgattggcaacgtttcttggccggcaggcaaatatttggccaatgaaatgctcggcggacgggtgtctgattgggaacgggttatcgttctaatggatgacgaccagttagtgggcttttgtgcggtcgttcgggaagatatcgttaaaggaaccggctattcaccattcattggctttgtctttgtcagcgaggattatcgcggcagacatctcagccaacagttggtcaaattggccgagaaccaaatcaaacaaattgggtttcataaggcatacattgtcaccaaacacgttggactgtacgaaaaattggggtacgaacaaatcgatacttccgtcgaccagttgggaagaaagatgaggattctagcaaagcaattataatttgattgaggagagaaagaactaatgaacgaagagaccacagtaccaagccgccagaaagtcattttgggtgctctgctgatatttttagtgggtgccaatatgcggacggcgattacgattgtgccaccaattttgaccaatattcaaaactcctttcagatgccggaatggtttctggggagcttaacgacaattcctttgatctgctttggattattatcaccgacggttacatattttattaagcgcttcgggattttgccggtaacgatggtggatctgggcttgctgacaatcggcaacttcatccgggtttattcctttaccagcttactgttcgggacaatcttgattggttgtgggattgcgatgttgaatgtcctcgcaccaactttggtttcctatttgtttccgatgcagatcgggacttataccgggatgtatgttttcgcgttgtcactatcgagttcgatttctgccggctttagcgccgtagtcagtcacttgatcacttggcaggtgatgattcaattcatttcgattattccagttatcacaattatcgtggcgatcatgttgagaacttcaggcaaacgcaagacctcagtcaaaaagacggcgacaccacttaatccagaggtcaaagtgagcgtttggaagcggccgcttgcctgggcattgggtggcttcatgggtttgcagtcacttcttttttactcaattctaacctggctgccaccaatcctgatggcatcagggattaatcagaatacggcaggatacttgttggggctgctccagttagtggcactgccgatttcctttgtcgttccaagaattatcagctcggttgccaaacagtcaacgatgatttggacgatctctggtttgtttatcgtcggattgggatcattaatgatggctgaaaccagtttctggtttgcggtccttgcttgtgtccttttgggattgtcaaccaatatggcgttcagcgaggcaatgaccttgttctcgctgaagacaagaacccccaacgaaacagcctcagtctctggaatgggtcaatcatttggttacctattggcagcgacaggcccgatgatttgcggctggatgcatggcctgaccacaaactggtttgcggttttgattttcctactggctgtgaccgttgtcatgacttttgtggggttgttggttgatcgtgaggagtatgtgttttaaaaatcagtgtgggcaaataagcgcctagcttccagagtataagagagttcgccaaatatccagggcttggatatttggcgaactctcttatacggccggaaactgcttatttgcccacgattccactaggtaatagttggagaccagggcttggatgtttggtgaacgcctttatacggccggaagctgcttatcgtcccactactccactaggcaatagtagggaccagaccgtggatgtttgacgactcccccttacacggccggaagctgctgatttgcccacgattccactaggtaatagtaaaaaggcacaaagtaaacaccaaaattacattccacaaacgcctcattaaaaataaattaaaaaatgagttgactctcagaaaaaatctgttacgataatcactaatatatttaacgaagatcgaatgagtaatcagtggagttagccaagagagctgtcacgtcggtgaaagacagcctaacgagattgatgaatatggttcgtgagttgcagtagccgagcacttgtaaggctacgatgttgggcacattatcgtctacagtttgaaaactgactgagaaagcatgcgtgagtgtgctttgaaatagggtggtacagcgatacgttcgcccctatggcagctttaacaattgaccggtttgttaacgcaaaccggttttatttttcgaaattttgaggaggcggatactgatgaagaagatagtcgtttcagtagtgggattggtgagtgttttggtgttaagcgcctgtggcaagtcaacgtccagtaaggatgcgaccagccggacctttcgaacgacagcccagacaaatgtcatcactgtcgatcctaatcgggcaactgatgttgggagttatttggcaatttcgcaagttgtcgagggcctgtataaacaaaataatcaaggaaagattgtaccgtcggtggcgaccaaaattgttcagccaactaatggcgggaaaacctacacctttaacttgcggcacgatgccaaatggaacgatggcagtcgggtcactgccggcgactttgtggcctcgttcagacgacaagttgaccccaagaccaagtctcaacgtgccggtcatttgagcgatattcagaattatgatgcggttaattctggcaaagcggcgccatccaaattaggtgttaaggccattagcaagtataaactgcagctcaagttgagccacccggttccgtattacaactagtgatcgctacccagttgtatccgattaatcagcgggcgctcgccaaatgggggagtaaatacggtcaggattcaaagcacgcggcttccgacggtgcttatgaaattaagaactggaattcttccaaagatacctggaacttggtcaagaacaaagactactacgatgcgaataaagtcgacttaaccagaattcatttccaagttgtgaaaacaccacaaaccagcatgcggttatttcaggaaaaagacatcgatgagacccaaatttcgggcagtttggttgctgatgccaagaaacaatttaagaatgaaacggtggtttcaaaatatggtcagttagcctttatcccttggaacaattaccgtaagacgacgcggaatctcaatttgcggcgggcactaagctacgctattaatcgacaatccttggcaaagaacgtcttaaaggacggatcactgccggcccaatcagtggttccggagggtgaagttaaagatgccagtggcaaagatttcaatgccggggttgccccaaagttgacgtataatctcactaaagcccgccactacttcaaattagcccaagaagagttgggaaaagaaaccatcaatgttcaattgttaaccgcggacaccgatgcctataaagccgtcgccgaatatattcaatcacaggccaaaaaagtatcgcccaactttaatttgaccgtgcgctcaattccattgcagcaagagatttccgacttcagtaatcacaagtttgacgccggcacgctcgggtggtcgacagacttcccagatccaattgattatctgaacttggctgccaaagccggggtcatcaactttaccaagtggacgaacgataagtatcaaaaactgattgatcagattaatgacacaacgcaccaaactgctgggcaacgagtgaaactgcagcagcaggccgcctcgttgttaaacgaacttcaaggcgtcacgccactgtaccagtacgcttcggttcatttgcgaaccaagaatattaaaggcttggattatccattaattggttatcagaagtatgagtatgcaagctggaagaagtagtagaggagatttgattttatgacgattaaaattggcattgccagtaatcatttgattcatccaactgaacgattcggaacaaattttgtcgattatattcaacgagactatgtcactgggctgagacatgctgggatgttgccgttagtcctgcccttgggcgatccgaaagacgctgaagattatattgctggagttgacgggctgctgttgtctggcggccagggggtgacgccaattttgtatggcgaagagcccttggcggaagttgctgaaacggatatttaccgggatcaatttgaaattgccttgattaaagctgctcagaaagctgacaaaccggtgctggggatctgccgtggcatgcaggtgattaacgtcgcgttaggcggcaatctgtaccaggacatctataaacaagccggggcaacggagaaacacaatcagtatccaacatcttgggagattcctactcaccatgtgacaaccaccgaggactcatggcttcaccaaatcttgggtgagcggtttgcggttaattcctttcaccatcaagggattcatgaaccgggtaatggcttgaaagtcgttgccaaaagtgatgatcaggtcgttgaagggatcgaatcaaacaatggtcgaattatcggcgttgaatttcatccggagatgatgcgggcagttcatccggaattccagcggatttttgattattttgctaaattggcaacagagaattaatataaatgtcaaaggctgaagcccagtgattgtactggtgcttcagcctttttttcgcctacttaacaatgatagagttgatgatgttacggcacctctgagcgccacttctatctagaccaaacgtgcagcaatcggctgatcccggccatgtaaggcacttaagcaatcattccaagcccgggaatcaatgcttaagtgccttacattctgggatcaaaacgcctctttctccactctatgcttaaatctccgctgccggattcgtcgtatacgttgcccacgcctgaacagcgactgtgcccaggattaggacggcgccgatggtttccggtacgccaaagctgacgccaagaaaaatgatcgaaagtgtggttgctgatagcggttcgaatgaccccaatacgctggcagtcgtcggttgaatgtatcgcaggctttgaaggtaaaataggtatgcaaacatcgtgccgaagatcaccacaaaggagacgctgccgtatgttgtccaagaaaaggccggcatgtcgtcccagatccggtaataaagactaaaggcggttccaccgattagcattgaccaaccaacgatgggaatcgagccgtattctttcaggaggtttcgtggtaataaggtatagagggtggaactaaccgctgcccccacaccccacacaaagccccctaacggcattgccaatgtggtcagttgaccatgagtcacgagaagaactgtccccgacaaagccataatgaccgagaagacgtcgattcgccggggaaagcgccgggtccacagagctaaataaataataatcattgctggtgccaagaactgaaggatggtggcggtggcggcattaccagcctcaatcgccatgaaatatgtatattgtgaagcagccattccaataaagctaaagaagattaagcttagtgagtcccttttgtggtgccaaacccgcatttcttgtcgatgattgccaatcaaaccatacaggaccaacagaatacccgaaatcagcattcggacagaaaccagccagtgtgagcttacatggatatcgtcaaataaaaattgggcaagtgttcccgagattccccatagtaaaggtcccagcattgccaacacaatgccgcggatacttccattcttcacctgattcacctcccatacataatgaaccaattatattacaaagataaccgatttagaataaccctttgtaaaataaagtgaattgcgttagagtatcattaatatttaatgatagaacaatacataagaggaggcctgcacatgtttgataaaattggccagattattttcaacaacgaaattgtcgcgaatgccagcgactttaatatgggcattgaggtcgaaacgattcggattgattcggctggaagattaaccaaggaaccgtaccccaaagcccttggcaatcaacgaaagaaccatttcatcaaaacagatgtttaccagattcaaagtgagattatcacaccgactgcccgcaagtccttggatgcgatgcattatttgatggcacttaatgatacgctgcgaaatgctttggagcctaacgaattattatggccgctgagcatgccgcccgtgttgccccaagacaaaagcacgattccaatcgctgatgttgaccccgaacagaaggcctactacgaaaaatggatcaaaacccgtagcgatacccaagggattcctgtcggggtccatttgaacgtcagcattaatgacgacgtgctcaaaacggtttggcaggcggttgacgatcagtatgattcatacgctgattttgtaaattatatttatatcaagatcgcccaaggctttgactactaccggtggttaatcacttatttgtttggtaatagtccaatcgctgaaaagaatttcttcaaacccgatgaggaccagccgcagcatgaagtgcgcagtattcgttcatcgaactatggattgacgtctgatgtgacccacagttatcgcagtgtgccggattacgtcaagaatatcgagtcaaatattgccagcggcgccttgttcagtgaagccgaataccattcaagcgttcgtctgaaaaccatgcatggcgacctaactgacatgatcaaaaacgggaccgaatacattgagttacgaatgctggatcttgacccgacgaccgccttgggtgtgcggacatccgccatccgctttttcagaatcctgctaagttatttcatgatgatgccgactcttgaaagcgatgagaagattaacctcaagttggaacaggggcgggcaatgaacgaagtggttgcccttgaaagcccatcccaacagacaatttatcatcatgaggcgcaaactttcttggatcaactccaattgtttggggcccagattcagtggggccctgaataccaggaagtcttggatacgatgcaggatcgactcgacaacccgaacctgacgccggctgcaacgctgtgcgatcatgaggttgacggctcactgatgtcatacggtctggcaatggccaaccgttatcaaaatcgcgcccatgagaatcctaatccatttaccggctttgaggaacagcccgatatgacggccaacgaactcaggcagcgtctgtttggtgtcatggggaaaccggaaaattataagaacggctgattcgttgacatgcggctgacgaatcactaaaatacttgataattaattgaagcctctaccaggtttagacgaagcgaagctgtgatgtcctacaagttttttcttgtaggatatttttgaaaataaaggatggtgggcaaatgaaacaagcaaaagaagtttctgatttcattaattcgacggttgggttggaggtggaaacccaccggataaataaaagcggtcagttgagtcacaaatcatatcctaaaggcctgctaaatgagcgtcagcaccattttatcaagaatgactttttggaaacgcagtctgaattgattaccccgccaaccaaaaccaccttgaaggggttgaaatacctgggcgtgtatcatcaggcactgcgaagtgagttggctggtaaagagtacctctggccatacagcatgccgccgaaattaaaagcggaccattctgatattgtgattgcccaaaccgaccccaagagctatgagtaccgccaacaggtggccaagatccgaaaaattgaacgaactgccgagaccggagttcacgtcaatatcgggttgacgaagaaggccatcaaggacttaactgctcaggaggccaatgtgagcaccgatgatctgtatctccaggcagcggttggctttatgcgctaccgctggctgttgacgtacctgtttggcgcaacaccggtggcctttactaattattttgctccaaataccgatgcgcccatcagtccggtcagatcactgcgtaattcgcactttggctttggaaatgggtttatttccagttatcaaagtgtccaacagtacgttgacggcatcttgaaggccgtggatgatcaaaagctgattgcccagcgtgagtattatgggacggtgcggttaaagcgtagcgataatgtttctgacctcctaaccaagggaattgcctacctggagctgagaatttacgatttagatccttttgaaccgttgggggtgtctgaagatgccgtcgacttggtccgtttgatgtttgcctattttgtcagtcatcgcccatttgatttgcggacggcggatgaagatattgctaaggcagaccagaaaaatgatgtcgttgctttggaaaatccattgaagattagtcaatatcatgatgaggcggcggaatttatcggtaaactggaaaagttcagcgctcaagctgttatcccattcaatgctcaacatctgtgtttcaaattaatggaaatgattgacgacccggtgttgacgccgagtgggcgaatggctaattggctcggtgaagactcgaaaaaggtgtttgaagaactgttaaaatttgccaagggctaccaggatgatttgattcataaaccggcaatcggcttcgaatcattgagtgccgcggaccagaaggaaatcttggcgaccttgaagcagggaattccggtgagaatcaaataagagtggagcaagaggcgttttgatcccagaatgtaaggcgattaagcgattattcccgggcctggaatgattgcttaattgccttacatggcggggatcagccgattgctgcacgtttcggcaaggtagaagtggtgctggtgcatggagcaagaggcgttttgatcccagaatgtaaggtgattaagcgattattccggggcttggaatgattgcttaatggccttacatggcggggatcagccgattgctgcacgtttcggcaaggtaaaagtggtgcggagtggtgtacaaaagttgcagactcatgtcaactaatgcttggaagccgccgcgaagagcccattatccaaacagaagttgcccacaaaaaaggtcggaacaataggctaaaccacctacgttccgacctttcaatatgaattggtaaattaataaaaactaggtttactccactcagtccccggctcacccaagcctaagctttcacgatggtaatccgcttttccggttaacaaatcagtgacaaactgagcaacggcttgtcgggtgacttgcgcttccttgaagggttcaccctttttagtaacgtgaacctgcgtattgccggcttgattatacagccaggtgatccgcaaaatcacatagtccaaatcactagcttcgacaatgtcggccgacttctttcgatccgatttccaaataattccggtgtgttctcgataccaggcttgaaacttgccggtaacttcctggtataaatcaggaatgttggcggcaatgaaccgggtgaccttggcttcatcgagaaccttcacaatgccgtcggtgatttccggtccggcaacaaagctcagatacaccgcatcggcgtcctttaagttggctttgattttatcaaactcggtgaaatcgccatcgacaaacgtcacgcggggactctttttggctgccaagcgagatgagacgttatgaccatacaagaccaaatcaaaatcggtttgagttaacaggtcatcagtcaccatttgaccaatctggccggctgctcctaaaatcattactttcaaaattttacctccattgggttacttatcgtcattgttccagcgaccgccgccacccagacgttcaaccatctttggatcacggtggtcaaagaatgccgattccttcatatccaggttttggatgagctgcatttcttcatcggtcaattcgaagtcaaagatgttgatgttttcaatcatccgctccttgtgaaccgacttggccagtgtgataacgtcccgttggtacagccagcgcagaacaacttggccaacccctttatgatgattttgggcaatttctgataagacatcgttggtaaataagccgtgcttgccttctgcgaacggtgcccaggcctctggctggatgcctaatttcttcatccagtcgagttcatcctgctgctggaaccagggatttaattcaatctggttgacttgtggggtgacctcgttatgctgcgctaagtcgacaaatcggtcggcgttaaaattggagatcccaatcgcccgaatcttgccttctttttgaagctcttccatggctcgccatgagccgtaaacgtctccgtatggctggtgaatcaagtaaaggtccaaataatccagcttcaatttggttaacgcctgctcaaactctttcttagtcgcgtcatagccggtatcactcacccaaactttggtggtcacaaacagctggtcacgagggatgttggattctttaatggcatcgccgacttcggtttcgttgccataagcctgagcagtatcaatgagtcgatacccagccgagagagcatcggcaacagcttgtttagttccaccgttttcgatttggaaaacgccgaaaccggctgctgggatttcaatgccgttatttaatttaaatgttggtgtattcatgatgattattctcctttatgattgtctttcaaatatggtttctgccagagtttctccgcgttgtcggcggtcatttcaccggcatcgaatttggctaaatgctcatcgaaggtgtcaattttatatttcagcagggcttgcgtgtcctgcatttctttgagtttttcgtttaaaatcgtcaactgttcatgcaaaatatccttttgagcttgccggacggccccacctttgcgggccagggtggcaaactcaatcaaagattcaattgacaggccggcgcttcttaaacttttcgccaggaaaatccaattcaagtcattggtttggtagacacgataaccgttgtgatcgcgtttaaccgggggaatgacgccaatccgctcgtagtagcgaagcgtatcggtagacaccccaagtagttccgagactttcttactgttcattatttcaatacctccgttcctcaactgacaaatacaatataaaccgtggagtggactccatagcaagtaaaaaaactttaaatatcaatttaatttatttcagatctggttatttgatttttgaaagactaaactgagtttcaaaggagtgataaatgaatgtgtacaagtgtgacttttctatctgaaacgggcgacaactttttagcccgaactatggattttgcttttgaattagatggccgaccaatcgtgatcccccgaaagcagcattttgacagtgatgccgcagaggctggatacgatacgacctatggttttgtcggtgccggcagaaacttgggccattatattttggttgacggtgtcaatgagaagggcttaagcgcagctgcactgtatttcagtggcgaagcaacctacgccaaaacggctaagacaaaccgggtcaacctggcaccccacgaagttttgaattggctgttgggcaatgccagtgactgtgaagacctgggccgcaaagtcgaccagctaaacatcatcgatgctccggtcaagattcttggcaaggccaccccgcttcactggatcatttctgatcgctcgggtgcctgctatgtcttggaaatgctggcagatggcattcattatcaaaagaaccccgttggcgtcatgaccaacagtccggactttggctggcatttgaaaaacctcagcaactacaccgagttgaaaccatcaccacatcctgcccgctcatataacgggtatgaaattacgtcatttgggcccggaagtggggcgctggggatgcctggtgactatacttctgtttcgagatttattcgcaccgtatttatgcgggaatatgccgatcaggtaccaactgatcaaactgtcaacgaactcagccacattttgaactcggttgaaattcccaagggcgttaagttgaagcaggatggcagcgaagattacacccagtaccgcggctatatggatatgaaaaattgtgcttactatatgcagccttacgataatcaaacgatctacaaggtgtccttgtcagaagaactgctgaataaaaaggcaccgagtgaatttccgattaaacaccaacaagtatacgaaacgcttcggtgaggtatcctcactgaatggcggttcgtgcacacatgagttgttaaaatctaagaaaaaacgctcgatcatccctttactggaatggtcgagcgttttttgaatagtgataaaacctattttctggtcttgtcagcgaccttttggctgcgattaatgaagtccttgaatagcttccgcgagtcctcataatgcttgtaaatgttttctggatgccactggactgctaatatctgatcattatctactgattcaatcgcttcaatcacttggtcatcggctctggcggtcaccttcaaatacggggcgacgtctttaacggcctggtgatgacgtgaattgacatatgggcgctggccaataatgtcattcaagcggctgtgtggatcaactgtgacgtgatgagatggcatgttgcctggggcttcctgggaatgtttcaaagtcgcgtgtaagtcctgggacaaatcttgatagagggttccgcccaggccaacgttaatcagctgcatccctcggcagattcccatgatggctttgccggcagtcacagactgtttcaataattcaatttcaaataagtcgcgtttgagataagtcatccccagcttctggaatggttcttcaccatagaaagtgggatcgacatcagcgccgccaaggaaacagacgccgtcaaacagtgtcatataatcgcgcacgtcttcgggattgacacttgggaaaatgacaggtacgccaccggatttaacgatggcttcgattgctggccgaggcgcgaacgcggcatttcgttcattaatgacgttggttgcctcggcgagcgtgtcagcaggtaatgcgattcttgggcgcaataaaatccctcctcaataattactttcagtctatttgtgttattgtactccaaactaataaatttacgtgatattttgattgttgtcaatgtaatttgagcttatttgtcgacttttgatttgtcgggttcccaactgcctttgaataattcctgctttaattcgttggctgacagcttggctttattttcaaatcctttaaatgggcgaatcgactggagtgccgattgttggtagcgcttggcccgtttaatcgcatattcttccaaagaaccatttttcaaatgggtgattaacttggcacttggcgtggtgagcggattttcgacgcggtcttggaggtcttcaagttcttcttggtattcaggtccaagctggattctatccgcgtacatttccaagctttggaggaaggctctggcattggcttgatatttggaaacatcattgggatgttcttcggagacttcttcgttcatcttatccgaacgggcgatgaccttctcaacttcctcaggattcattgccggcgacatgatgaaatagctggccagtaaacggataaaccgtaacgtattggtccgaatccccacagaactgctggggtcaaggtcgagcattctcaattcaaggtagctgaccccggtcttcggcagctctcgcaagtgggtgttgcccttaaagcggacggcaccatggaattcgtaatctgaaatcagcttgccgtcagcgacgcccttttcaattcggtcaacataacgctgaacgttcgtgtagtcgccgctaaatggattgccaaagccgtgtgaactctggcggatactgcgaatcggtgcttttggtcctttacccggatcaaaatagttggcttcagcgacggggctggcgccaaatagatatgtaatgacccaacgataccgcagaaagccttgggcaatcttggcgtataagtagttttgcagctcaactttggaattgaaacgatcgctcatgttggccagaactaaatcaaacacgtggggatcgatactcaagttgatatgcgcgccacaaggcgttccttgagaaaagccgtgacgtttcagccattcttttaagtaggcttccttcttgggtcccattttagcgaggggaatcttgctcttgtcttttggcagtcgcggcggcatcgataacggccacaacagctcacctggtgacagggctgaccgcaaggcgttgttaatgctgaacaagtagtgcatggcgtccagggcatgagcggccggtggggtcacaacctcagacatggtttccagaaaatcattggtaatccaggggttggtttgttcgtcaccggccccggctgggtagggttcttggcttaaattgccattttcatcaactcgctgcatctcaatttcaattcccatggtaaagtctgaggttttcgcaacggcttcgttatcaaatattaactgaccaatttcactgaacatggcatacctcctagttgaattaaaatttgatgataattgatgacaaaatactaacactatcgcgaactataagcaatgctaatggtgttatgtcacggagatttgtgctaaaattattttatttaattaatttctaatttagaggtggaatcatgagtatctttgtcaaactgggctggtatttcaaaagggaatggaaaatctacctggttggtttatttggcctgctgctgacggcgttggtcggaattattccgccacggatcatcggtaatctggtcgattcgattcataacggtaaattaacagctaaatatctcatgtttttgctgattgttttgacgattgtctcctttgcccaatacggagcccgttatatgtggcggaccgcgatttggggtgaagctgccaaattggaaaaagtgttgcggaatcggttgtttttccactacaccagtatggatcatgaattcttccaacgctatcgaaccggtgacctcatggcgcacgctaccaacgacctgtccgcgattcaacgagtggccggtggtggaattttgcagttcgccgattccatgattaccggcggcacgaccttgatcgcaatggtcacgttgattgattggcgattaaccctgatcgccattttgccgtttccgctattggcagtgatggcgcgatatttggggactaagattcacattgcttttcgagattctcaagctgccttttcacggctgaataataaagccgaggaaagtattaccggcatcaaggtcattaagggccttgggcagcaaaaagaagatatgcaggattttgacaaccaggttgccagaaccatcaacatcaaccggcgggtcaattttctggattctttgtttgacccgatgaccaccatgatcatcgcgctgtcctatgtgattacgattgtttacggtggctatttggtcaccaatgggacaattaccatcggttcgctggtttcgtttgtttcctatctggccatgatgatctggccgatgtttgccgtcggcatgctgtttaacacgttggaacgtgggaatgccagttatgatcgggtcatggacctgattaaccagcaaagcaaggtgattgacgatcctaatggtgtgacaattacaccgaagggcgaaatcgattatgacgttaagagtttctcatatcccggtgacaaacgactggccctgcaaaacattgactttaaagtgccggctggcaaaacggtcgggttggtcggcaaagtgggctccgggaagagtacgattttgcggctgattttacgtcaatttgataattataaagggtcaattaagtttggtggcattgatatcaagcaatataagatggacgctttaattcctgcaatcggctacgtgcctcaagatacgttcctgttctcacaaagtattcgggaaaacatccgctttgcccgtcctgacgctacccaagctgaagtggaacaagctgccaaaaaaagtgatttgtatgaccagattcaagcgatgccagatggttatgacacagctgttggtgaggaaggcatttcactttcgggtggtcaacgtcagcggctttcaattgcccgcgcgctgttaatcaacccggaactattaatcttggatgatgcgttatctgcggttgatgcggaaacggaaacccaaattctcgaaaatctgcacgctgaacgttccgataagacgacgatcatttctgcccatcggttgagttcagtgatgaatgccgacgaaattctggtgatcgatgacggcaaaattgttgagcgcggcactcacgatcaattaatgacccgcggtggttggtaccacgaaatgtttgagcgtcaggaactggaaaccaaagtgaagggaggcaacagctgatggctgattcatcaaagcatcaatctgcctggtcgaaatccattccggttaagcagcagatgcacattattgggcggctgttcaagtacgctgctccctataaatggtatttctacttttcagtcctgtttgcgattgcggttgccgttgtcaatattctcttgccaagaatcattcaaacctttatggacagccacttggtcgttggtcatcctgattttgcgatgatgtggttctttgccggtttgtacttctttggcatgttggcaaaggctgtgatgcaatttacccagacctatctgtatgaaatgggtgctgagtatatgctcgaaaataccagacggaaactgtttgcgaaactgcacaccttggggatgcggtactttgaccagacccccagcggctccattctttcaaggttaaccaacgataccatggcctttgcaaacttctgggccctgttcagtagtttggtggttaccatttcggccatggtttcctcatttgtcgcgatgtatttggcagacgccaaaattgccatgtggctgttggtgttcatgccgttcttgttcgtgacagtctggtactatcagcgatacagtacccgggtctaccgtcggatgcgtgaacggttgagccttttgaacgctaaattagctgaaggcattaccgggatcagtgtggttcagcaattccgccaggaaaagcggatcaatcacgaatttagtgataccaatgaccagtattataatacccgccgggcgatgattcgcatcaactcgttgttgttaaacccaatcattaacttgttctacgctttgggaacggtgctggtattagggatgtttggtatccgtgggctgcatggctatgtgcctgccggaattatttatgcgtttgtgacttatctttccaacttctataacccaatgtctgaaatgatggatcggctaagcgacttccaagatggggtcgttgccggctcaagagtgctgcggattatggatgatcagacctacgaaccgaagcagcacgcggatcccgatgccacgattacccgaggaaagatcgaattcaaacatgtcaccttttcttatgatggcgaaaatgatgtcctacatgatatttcctttgtcgccgaaccgggacaaaccattgctctagtgggtgaaaccggaagtgggaagacgtcaatgattaacatcttgatgcgcttctacgaatttggtgaaggggaaattctgattgatgaccgtgatattcgtgattacaccattcaagaactccgcaagaaaatggggttggtactccaggaacccttcatgttttacggaaccgttgcctctaacattcgaatgtttaaccaagaagtcaccgatgaagaagtccatgaagcggctcgatttgttcaagccgatcaatttattgaagacttgcctgatcaatacgactcgagagtgattgagcgtggtgccagttattccagtgggcaacggcagttgatttcctttgcccggactctggtgactgatccgaagattttgattctggatgaggcaaccgccaatatcgatactgagaccgaacagattattcaaaccgggttggccaagctccaagaagggcggacgaccattgcgattgcccatcgcctttcgaccatccaaaacgccgacttaatcttagttctggaggccggccggattgttgaacggggaacgaatgacgagctgttggagaaacatggtttctattacgatatgattcaacttcagaattccgcccatttggattagggtggtttgcgaattttgactgaaaaaatggttgatagcaaattttattttgctatcagccatttttatattacggtattaaattattgaatctcaatattgccgctgtcttcatgactgtcagcagcctttggcaatgtaatggtcaagacaccatcattgacttgagctgagatgttgtcacgatcgacaccaggcagttcgtaagttctggacatgacaccatgactacgttcactggcaacgacccggccttgttcgtccttcttctcagaatcacgttcttggtcgatgctcaatgccaagtcaccatgttgatatgccagatggatgttcttcttatcaatacctgggacatcaaccttcatgatgtagttcttatcattttcggtgatgtcagtctttagatcaccatttaccatgtagtcgttgtctgcatcagttggactgaagaaacgacgtgccaaagtatcaaagaaaggatccattgcgaaacggttcattaattcatttgccataataccaatctcctttgttgattattaataagattaattaataagcgtcaaaggtggtgaaacggggtcttggaatcacgttcccccaaaagaagctttactgaagtttcaaaagctgactacctgaatccctaaccaaccactccaaaatattcgtcaaaattactgaatatcaatgttgccggtttgatcttcgctttcagtgacttttggtaatgtcacatttaaaacaccattgtcaatgtgggctgaaatgttgtcgcggtcaacaccaggtaattgatagctgcgtgacataacgccgtgactgcgttcgctggcaattaccttaccgttttcatctttttgctcagatgaatgttcctggttaatattaattgagagaacgccatcttgatagttcaagtgaatgttgttcttatcgatgccgggaacatcaatctttaatgaatagtctttatcggtttcgttaatatcggtcttcaagttgccgaagttctcataatccttgtcgaaatcagaagggctgaagaagcggtgagccattcgatcaaagaacggatccaaatcgaaacgattcattaattcatttgccataatatctatctccttaatttcaaaatgattattcaagataacggggaacaacacgtcacttttttgttcctcctttacctttcaactactatgataatcagttttaaaatgaatgccagcatttagcactctaatgttgagagtgctaaaattttctcttgaattggtaatgtttgcacctaacaaagctcgcctatgcgcgttatcattgggatgtgctatgctgaagtgagaaatcaatgaggctgggtgaatgatcatgagcgatcgttttttcaacaaaaattttatttggaagataatttgggtaggcattgggaaaattctggtctgcctgttatttctgtcggtcggattttctacccaactctcaccagcattagtcgatcaaaatgacacccccacccagcaggtcgatacaacgactacgccggcgtacagtccgaaaacgaatttccactggtcaaccaagacagttgcctactttattactaagtagacgaacggccattaccgagatgtttggatgcgggcagtcaaagcctggaatgcggtcggggtcgttgatctgataccagcagacaatgcggatcgagctgacgtcattctcagtgtcaaacaatcctatcatgaaggcggcggtacggttgagaatatcgccggtggggtggttggctacaccagcgaggaatttggtcacgtggacgggatcccgctattcgtccatcaaaataaaagttatttgattactgattccctgaagcaagcccactacgattctgtcaatgaacaagcaagcgtggcgatgcatgagctggggcatgacttggggttggagcacagtgacagtccccattcgatcatgcagcaggcggcgccgacttatttggatagtattcccgaagttgatgccaagcatttggcgcagttgtatgctggggtgccgcgggggtgaaagtagccgtattacctattatggtaatgtttaccatgcaaaaaaaagagcggctcagaaagtcgctccaattaatagaactctaagtattgaactcaccacacttacactgccagcaataccccgacagagtagtgaatgatcatggtgatgatcccaacaataatatttcgaataatagctgttttaaccaaaccattccccaatcgggcacttagataacctgtcaggccaaccgagaggcagacggccagaatggttgccggccactggaaggcaactggtgtcagcgtcatggcacacaaggggaagataccaccggcagaggcggaaaagagtgatgagaacgctgcgtcccaaggattcatgtagtgtcccaacttgaggccgtatttgacattgacaatcgtttccaaaggatttttgctcattaagtctttggcgattttgtcagcagtttctttggtgacaccctgatcaacgtaataatcggacactacgttgagctggtcttgataattagtcatcagtaatgctttttctttcgtcaccacagattgttcagtatctttttgggtactaacagacgcatattcgcctgatgccatcgaaaaggcacaggccaacaggtcggataatccggcaatgaagatcgtaaactgattggttgtcgcaacggcaacactgaacagcaccccaacaacggttaagatgccgtcgttggatcccaacacgccggcccgcagggtattgagcttctcatccattgtctgaccatcttttttctttttggaacgaacacttaccatgttcttcgcctcatttctctaaaatatgatgttcaagatccaattaaagtcccaattgtgtaggtgactaacatggtcaaaatcccggaaataatgtttcgaatcataccccggcctttgttggcgttgcctaattgagcggcagtgtaaccagtgatcgccaatgcaactacgacggcaatgaaggttgccggaatgcgaatggtctttgggaacaaagtaatcgctaaaagtggtaaaattgaccccgtcggaaatgaaatcatcgaagcgattgctgctgataatggattggtatattcaccaacgttgaagccatatttttgacgaaccgttgtcttgaccggatcttttgccatcatttcagaagttgcttgggccgctaaatcggcagaaatgccgtcacccatcagtttgtgtttgacggtgttgaattcattatcgtaagcggaacttaaggccgccttttggagactgatggcgtgtcgttgagaatctttttgggtattaacagacacccactcgcccatggccattgagacggtcccggccagcatcccggaaataccggaaataaaaattgcaaaattatttgatgtcgccccggcaacaccgataacgattccggcaaccgaaacgatgccgtcattggcccccatcaccgaagcccgcagaacattaatcttttgtgaaagcgatcttttcttcgccatatgctcacctacttcatagtttataatcattattatctaacaaaaattattttagtcctttattgtttaaaagtaaattaaaagtattgtgttagctaaccacgttatcatgtcgcttgacacatatgctgtgaagaaccaatttagaatcactatcaaataattagctattaactttaagaaggagatgccactcgtgaccaacccgattcttgaacaattaactcagcaccgtagtattcgtgaatttgaagatcaaccgttgagcccgcaccaagtcactgaattagtgaatgcggcccaacatgcttcaaccagcaccttttctcaacagtattccatcgtcagtgtaactgatccagccaagctccacgcgattgccgaagtcactggccatcgttggatggtaaatggcggtcactatttcgtgatggttgcagatcagtatcgaaatctaaagattgccaaagcacatggtatcgatccatacatgttgcattcaacagataaatttctggcaagtgtctttgacacggcgattgccacggaaaacatcatggtggccgcagaaggtatgggactcggcggcaccattatgggcagtgtcttgaacaatcccagaaaaatgattgaattattaaatttgcctgagatgacatttcccttattagggattgcactggggtatccaaaagacaaaccagaattgaaacccaggttgccaaaagcatcaatgcatttcgaaaaccaatatgatctgggtgcaaactttgaccaggaactcaccgattatgatcagctaattcgcgagtattatcagtctcgcagcaccaatggtcgatcggaaaccttcagtcatcacattgtttctgaactcagcgggaatcggaatctgcggtcggatttgtttgcgatgatccaagcccaagggctgatgactcactaaacaattattagtaaaaatagttgacttttgagatgtttaacattacattattagttaattgattgacagtcatttgaatttcacaatgttgaagagaagagtacgttgttgggctgcacaaagcgaccgctgatagtgaaagagcgggcagacaatgaccgaaagtgcgctcggagttgtggcatttaattaaagatgcattcgaaatgaggcgttttgtttttgacaagacgcaaaaaagggtggaaccacggtaattcgtccctgatgatcagctgatgctggttatcagggacgtttttgtgttcaaatgactgcaaaataacttgtgaggagatgattgacaatgagcagctgggccgttatccaacagagcttaccgatgtttgagaaggggtttcaactcaccttgtggctttctttcgtcgggattattggatccattattgttggcataattgtgagcctgcttcaatatttcaaagtacccgttttgcaccaagtggcatcgatttacgttgaagtttcgagaaacacaccgttattgattcagctatttttcctgtattacgcgtttccagtgatcggcattaagtttggtgccgagttgtgtggcattatcggattgatatttctcggcggcagttacatggcagaagggtttaccggcggcttcaacggcgtttccaaaggtcagttggagtctggtaaggcaatcgggttgagtcgctggcagcttgccagatacattgttttcccacaaggattctcactgggcgttccggcaatggccgccaatgtcatctttttgatcaaggagacttcgatctttacggtgattgccattccggaattgactaacactgcgttggatttaattgggatgtattaccggtccaacgagtatctattggtcttggttgttggctatgcgattattttaattccactatcaatcattttgactttactagaaaagagggttcgctatggatcattcgggaattagtgttttattcgaaggaaccaattttgagcggttgctcggcggcctctgggtaacggttaaaattgcggcagtggctttgattgtcggcctcatcttgggaattatcctgggtgttttgaggacctttaagaatcggccattgcgagtggttttgagactgtatcttgaattcttcaggattgtcccaaccgtcgtgctgctatttttgttctattacatcttgccacgccaattgaattttaatctccctggcgatcaattggccaccttggtatttgccttgtgggtggctgctgaaatgagcgatattgttcgcggcgccctaatctcggtgccgcagcaccaacgcgaatccggtaaagcaattgggctcaatcgttatcagctctatcgttacgtattgattccccaagcgatcagtttggaaatcccggcgaccatcaatttggccacccgggtcatcaagacgacttctcttttgatgctgatttctgtgatggatgtgattaatattggccaacaaattattgaagccaataatcacacccatccaaccggcgttttctgggtttacggattgatatttctattctatttcctaatcgactatccactatcttggtgggccaagcgactagagaagaagagattggagcgggcaaatggctgagcagattttacaggttgaacatttagaaaagtattatcaaaagaaacacgtcttacacgatatcaattttcacgtcgataagggcgaggtcgtcacgttattaggaccgtccggatccgggaagagtaccttgattcgctgcctcaacggtctggaggaataccagcaggggacaatcacttttgaggggaagcggattaatccgaccgagaaaaattggcaacagatccgccaaaagatcgggatggtctttcagagttacgacctatttccaaatttgaccgttatggacaacattttgctcgggccgaccaaggtgcaaaagcaggataagttcgcagccaaaaaggaaggccttgaattgttggaacgagtcggtctcgaggattatgccaacgcatatccccggcaactgtccggcggccaaaagcagcgggtcgcgattgttcgcgccctggcgttgcatccggattttatgttatttgacgaagtgactgcttcactggatcccgagatggtccgaggaattctcaacatcatccaagacttggctgatgttgatcacatgaccatgatcgtggtgacccatgagatgaactttgcccagcagattgctgacagagtgattttcctggaagatggccatattttggaacaaacaccttcaaaacagtttttcaacgcaccacaaactaaacgcgcacaagcatttttggatagtatggatttctaatattgaggaggaacaatttcatgaagaaaagatcatttaccagaattatcgccgttgtgagtgtcttcgctgctttattactggtcttaaccggctgcggtaacagcaagaagtcaagttcgcaaagcaataacccaagttccgttcagcagatcaagaaaaacgggacgattagaattgcggttttcggtgacttacctccttatggctgggtcaacaaagacggtaagcgagttggttacgacgtaacattagcccaccaagttgccaaagacctcggagtcaaagttaagtttgtccaagtcaatgccaacaaccgagttgatgctttgaattccaacaaagttgatctggttctggccaacttcacggtcaccccagaacggaaacaggttatcgattttgccaaaccatacatgaaagtttccgttggtgtggtttcacctaagaataaggcgatcaccaaggccagccagctaaagggtaagaatgtgattgtaaccaagggaacaactgccgaaaattacttcacgtccaagcagcctgatgttaaactgttaaaatttgattctaagacgcagcagtttaacgccttgaagaacggccgtggggttgcccttgccgatgacaactcatatctgtacgcctggtccaaggataacccaaactacacggtgggcattaagagtattggacctaagtcctacattgccccagctgtgaagaagggcaacaaatcacttcttgattggaacaataaggaaattaataagttgaccaaggagagtttctttgtgaaagattacaatacccaattgaagccttacttcggtaaagaagtgaaaccttcagatattgttctgccagttaaataatcattgattaggcagccaaaaaagcttttggctgctttttctaacattaaaaaataattagagttgacgaatcaattctaatatgttttaataagttcaacatttcaagaaaggaattatatctatgaatactcaacttcaacaattgaatgcctattattacggctatgcatggtttaagtagcgctcgtcagatgcgggcgcaaaacgcgttcgcgtctaacctgggcaaagtcgtaactttgttgctgccagctagacgctagagtctagccggatgggtataatttcttaagcgagtgaataagaaatcagccagctggattctaatatccagctggctttttgtttacttacatacttgggagagtgatatcatgacaaaatctaataaacgcagattatcaatggccttatacctcaactacctggttcacggaattgggttgattattttaacccagaatatgcaggctctgggtggcttttggaacgtgccgattgcgacggtttcctacgtcatttcagggattggaatcgggaaattaattgcttacttcatcttcggttacctctcagaccgctttggccgggaaaagttggtcttaaccgggaccctcagctacatggtattctttatcgggattccgtttacccacaatatcgcgatggcctacctgtttgcaattattgccggagtagccaattcggcgctggattcaggaacttacccgacttttgtggaaatgggcggtaattcaagtgcctcgaatgttttcattaaagcatttatgagtgtgggtgagttcatcttaccgctgttcattgctactttggaagctcatcaattatggtttggttggtcattcatcggcgccttgctggtgttagtcgtcaacttattcattcttcgcggcgcagactttccagatcggaaccaggttgatgaagagtttagtgaagaacaccaatcactttccaaagttcggcgagtgattgcgacgattgcccttgcgttgtacggttacacaaccatggcaatcatgattttatttacccaatggattagtctattcgcaaccaacgaccttggttacagttcattgatttcccacggtctgttgtcgctgtacagtatcggttcaatcagtggtgtggtcgtgatgtttatcctgttaaaattgaatttcaccgaaacgaaactgttagtggtgaccaatacaatttctctcatcgcaattctcacggtgacccatgcctcaacggtcattgtcaccgccgttgcctgcttcatattcggcttcaccgcagccggtggggtgatgcaaattgccctgaacgttttgttgaaaatgtttccaaagcataagggtgtgattaccgggacttactttacgtttggcagtatcgcaacctttacgattccgattgtgaccggaatcttgtcgaaaaccagtcttcaatctgtgatgaattttgatgtgatgattggcttggttggaacggttttagtggtcgtgactgccttggccatcagtactgggaacgtcttcgcccatgccggccagtcgatgatgacccttcttcatatgggaccggcaccaattagtcagggccgctcaaaagatgaatagtttgtcagacaaaaaggaaaccgcaactttgcggtttccttttattgtgtttcaaatcgtttcatttctgttcgcagatcgtcaatcgcaatctgtccgggggctgatgcatcaccgaccgttgcaaaactcatcaccgacccaaacaatggcgcggtaactcgagagattcttcccagactgcccatggaaattgcgatgattggaatttccaacttgtctgattcggttgtagtggcccgcatcattgtgagaacgtccttgaatttgttgggcatggcagcgatcttggcaatatcagcgttttgattctgcatctgttgcagtaagttgataatctccagttccggcggggtaccttggaattcgtgggcactcaagatcaccttgatgttgtgttggtgtgctaagtaaatcaggttactgattgcctcttcgctgaaatgcagctcaacatccaatatgtccgtcaactcattggcaatcaaccgtttatatagggtcacataagctgcttcatcaaggtcggcttcaccgccttcaccagcggttcgaaaggtggttaagagaattgtgtcgcccaaaatacgccgtaacttggcgtaggtggcttgataagtggcgggatccaaaccagcttgatcatagtcgatgcgccattcaatgacgtccgggtgagcagttactgctgcttgggcctgcgccagaatatcattgacggtccgaccggtgatcggcaccgctattttggtggttccggttacaaatgacgttcgtcgaactgttagctttccactcatctcatcaacctctcttttctgtattaaaatcttgtcccaattctaacaagcggtgaccgcaacttcaatcaaaaaaagcctcccaaatatcgggaagctgctaatttcagttaaaatccgcggaaatctcctctgccaaagtactgcaggttagccaacaatggtttttgcatcagcgttggcaaggtcacaaatgtgtagccccgtttcttcagtgatcgaataatctggggaacggcggcaactgacgtcgggtgaatatcatgcattaaaataattgagccagggtgagtcgttgccagaacatgactgacggttttaggcgtattgagatatgcccagtctctggagtcaacattccagcggacgattggccggtcaaacaagttcccaatccgactgttaacggcgccgtatggtggccggatataggtgggaattgttcccgtggccttataaatcgctgcatcggtcaaggcaatctgatgaattgctttggcactggaaagggtggttaaatcaggatggttccaagagtggttgccgatttggttgccatatttgagaaccaatcgactgacgcttggatagcggataacactgctgccaacctcaaagaaggttgcgtggacgttatagtgctttaaagttttaagtaatttcggtgttaatgtcggatccggaccgtcatcaaaggttaaagcaacgactttcttgggtgttttcggtttgacaaagtcatattgcgacggcatgtagcgattgagaataatgccggttaacttactcaatggaatggcgacgtctttgacaccatatgaatttttaaccagatgaatggttaaagccgttttgctcaaagtaaagttatgggctgttaatcgcttgggtaacggcaggtaaatcaagttttgaacctgcttgccagacagcttgtgatcttcagccagttgggcgcgcgtcaattggcggatggtgcccagacggtggagactgttattggtgattttgccataggttaatgtagtcgctgcatgtgcttgtgggactgaatgattgctgatgctgaatgtcaataacgatgcagctgcgatactgaacgttaataatgcgcgtttgttgatcatgatgatcaccccaaattactttcaaattttatttcaatttcattttcacattgcctttgtgggaagtcaatcaaacttatttttgaaattttttcgatgcgattaagccttgatgacacggtgatgtgacattcaaaacgatcaattcaccagtgttgattttaagaataggtgttgacaatttttccagaattcgttattgtacatgacattagatatcgatgagaaagtgcttagagaaattgaaaagtcggtattaagaaattccaagagagcgtcgttatctgtgaaggcgtaatttcttaatcacttaaagtcaattttgagcacggtggttcgtcaagagtcactagggtgcgcccaatacagcgccaacgtataccgagtcgaccggtcgtacgtgagaggtggaatgaatttccgcaatgaaggtggtaccgcgcaaaagcgtccttttagaagtttaacttctgattggacgctttttgtgtttcatggacacaagcgcggctgtatggtcatcgatatcaatacaaaattattggaggaattgcgatgtttaaggatattagatttacagccattatcagtgttgtcattgggttcatggctgtcttattaagcggctgtgcgtcgacagcagtcggcggcggtgcaggaagtgccgaaaaagccttaaaaataacaatcccaggggagccattgacgattgacccaaccaagtcgattgaaactaatggcggtgtggtgatcgatcaggtcagcgaaggcatttatcgcagggatgcgaataacaaaattgctgccggagtggttgatgaggttgtcaaaccaactgataacggcacgaagtacacgtttaatatcaagaaggatgctaaatggcaggatggttcacctatcaagtcggaagattttgtcaattcgattgaccggcaggctgatccgaaaactaagtcccagcagacgacatccattcaatacatcgaaaactttgctgctgtgaacaacggtaaggccgatccaagtaagctggggattcatgcagttaacgaccgaacatttacggttaaattgaccaagccggtgccattcatgaattatgaatttacgaacttctatccgattcaaacggcggctattaaaaaatatggcagtcattatggcactaattcagagacgaccgtggccaatggtgcatacaccatcactggctggaacggcagtaatgattcttggaaatatgaaaagaataagaactattgggatgccaaaaacgtcaaaattcctgaagtggatgtgacggttgttaaagacaataacaccgcgcaaaacatgtttaacggcggacaaattgatttgaccagtttgactggacaatacgttaaacaaaataagaacaacaaaaatctggtggtaactgaaactggccgaaacaattacatttacttcaatgataagaagaaagccacttccaatgaaaacttgagaaaggccatcagcatggtcatcgatcaggatcaattggcaaaggatgtccttcaagatggctcgattggtgctaacaacatcgttccaaagaactatgctaaggatccgaaaaccggtaaggatttcacctcggaaatgggcgatcaagcaccaactgataccactaaggccaagcaatattgggcaaaggcacagaaggaaattggcaaagacaagatttcccttgatttcctggtggatgatactgataccgaaaagaaactcgctgaatatgttcaaggagcagtttcagacaatctgaagggcctgaccatcaatattgaatcggtcccgcatgccacccacgtaacgcgtgatttctcaactgatttcgatatttgtacggtcggctggggacctgactatccggatgcccagaacttcttggacggcatgcgcagcaataacaccattaatttctcgaaattcaaagatcaacagtatgatgacttgatgaataaagtggatgacacaactaagtacgatgccaaccagcgttgggactttgaaaagcaggcagataagcgcttgatgtcaatcgcagccgtagcgccaacctatcaagcctcgcaggcacatctgatcagcagcaaggtcggcggtttgaagtgggatgcaatgtcgggccagtccgggaagttgcagtatgcgtattggaaatagagcgcgacgagacccgggaagcgcggtttctaagggtactttgcttgaagtccctgtgtttgggactttaagcaaagtgcacttagaagttagcgcttgggtcgtcggagcgtattttcaaagccgaagggagcacgcaagaagctaacaaacgtgcttttgatctgaatcttgggtgacagaatactaagttccaagccagtgcacttgatcgcaaacttccatttgtgtaaccaaactacactgtcgaaaagtaaattcagttttgattcaaaaagaaaatcccacttaaggaggtggttgccatggcataccagttaacgaaatctaaagatgttccatctcagttagtctgcaaccaagcattttacatcgaaaggaagatttattatgacaaaaatcaattatacgaatgtcgcaatttacaaccatgagaagcagaactttatcgctaaccaacacatggtcgtcgatacggataccggcaagattgttgaagttggcaatggcagttccacaaaccaagttgtcgatgaagtttccgatatgcacggcaggtacgtgatgccgggaatcatgaacgctcatacccatatcaccagtattccaacctattggtggaacgatggcaaagaacagcgccattccgattcacgggaatttaatacgatgtttgccgtgagaaacatggccgatgcaatcgatcacgggattacttacattagaaatgttggtgcggcttttgacattgatatcgaagtcaagaaaatgcaggaaaaaggttggatcagagggccaaaggtgatgacatccggcaaggcattttcaattaccggcggccatggatccggtgggggttatgaagttgacggcgttgacgaggttcgtaaaggcgttcgccaggccatgaagaatggtgtcgacaacattaaaatgatggtgactggtggcgtccttaaaaatggggaaacgcctgatgatattcagttcacgcctgaagaggccagaacagcagtggtcgaagcccaccacaaggggaagactgctgcagctcatgcccaagggaacgcgggtgttaaagaggcagttgcagccgggtttgataccgtcgagcacgcatttgatatcgatgatgagacgatcgcaatgatgaaagaacacggcacggtggtggttccaaccatgaacgcgatgtacgccatctacaaatatgggaaagacacggttcctgattgggctcgcgaaaaggtgattgtcaacatcaagaagcattttgccagcatcaccaaagctgttcagtccgggattccaatcgcaatgggcactgatgccgggacaccatacaatggctttagaaatgaaagtgcctacgagatggaattatatgttgagaaggcgggcatgacccctgctcaagcaatcgattcggccaccatcaattgtgccagagccatgcacgttgacgatgagtacggccaaattgttgccggcaactacgccgattttatttctatggcagaaaatcccattaatgatattagtgtcattcaacacgacaaagacgtctatcaaaacggtacccgtgtccacgaacaggctgttgccactgctgctgagcgacaatctgctccaagtaaagtcagtgctgctatttaaaagtggcagcatcttctggaattaaaatcaaatgagtgaatgattagggttgacgaataatttctaatatgttttaattaatacaacttttacgagaggaattgataaccatgacaaagcaattcactgaaacttcagcctattattttgactatgcctactttaagtagtgtccgcttcggggcgggcgcaaatttgagcgttcgcgtccaagtggtgcagagtcaatgctttgttgagcccactagacgtaatagtctggctgggtgagttatcattctttacgaatttagtaaaccagctggataccatatctagctggtttttttaatggcaattaggggtgttaatgatgacaaataaaattgaaacagcaactgagagtgacaaccaggcaattcaagctgcccgcgagcaaatcaaccaattagatcaaggcattgttgacctgctgaagcagcgattccaaacgtcggcgttgattggacagatcaaggaaaattcccaactgccagtgctcgatggcgaccgtgaaagagaggtcctcaatcaggttgcacagctggattcggatcctggcacccgcaagtatctgcaaaagatattccaagaaattttgaaaaactcacgtgattaccaacatgaattaatgcaaaaggagactaaatgatgaattacttaacagctggagaatctcacggcccacaattgaccggtatcattgaaggcattccttcggggctgcatttggacgttggtgcgatcaacgaccaactcaagaaacgccaaggcggctacggtcgcggcaatcgccaaaaaattgaacatgatgaagtcaccattaccggcggggttcgccacgggattacccttggttcgccgattgcactagtagtcaacaatcgcgaccatgcccattggagtcaaatcatggatccaattagtcccgaaacgcccgagaacaccttaagaaaggttgaacgtcctcggccaggccacgctgatttggttggcgggatgaaatatcggcatgaggatctgcgaaacgtcttggagcgctcgtcagctcgggaaacggcaatccgggtggcaatcggtgctgtttgcaagcaacttttacaacagttgggcattaatattgttggttatgttgaacagattggccaaatttccaccgatgaaaatcctgaacttaatgtggctaaaattgaagcagaaattagtcaaaacgacttgcgaatcattgaccagtccaaggttagcccgattcatgatctgattgaccaaactaaacgtgacggtgacaccctgggtggcattatccgcgtggttgccaccaacgtgccggctggactgggcagttacatcagctgggataccaaattggatggcaagttggctgctgccgtgatgggcgtcaatgccatgaaaggcgttgaaatcggcgatggtttcaaagctgcaaccagcttcggcagtcaagtgatggatgaaattgattggaatcaggaccaaggattcttcaggaataccgatcatctcggtggctttgaaggcgggatgactaacggaatgccaattatcgttaaagcggcaatgaagccaatcccaactttgtacaaaccattgcaaagtgttgacatccagaccaaagaggttaagaaagccaatgtggagcgatcggacacaacggcaattgttccagcatcaatcgtcatcgaaagtgtggttgccattgagttggccaaggcactcaccgacaagtttgatggtgacaatttacaacgactacaagaacagcttgaccaatatcgcgatgaactgaaaaaattctaggaggtttctatggaaaaagttaaaacgcaatcaactaaacagctccaaggaagtctccaaaacggccttcacggtgaattggccgttcccggcgacaagagtatttcccatcgaggcatcatgtttggcgccattagtgaagggacaacgattttgcaccactttctaaccgcagaagactgcctctccacgcttaaggcgtttcaacaacttggtgtgccgatcacccgagatggggacacagtcacgattcaaggcgttggtctccacggactccaccaggtggaacaaccacttgatatgggcaattccggtaccaccactcggttgatcatggggctgcttgccggtcaaaactttccaagtgaattaaccggtgacgcttcgttatccaagcggccgatgcgacgggtgagtgaacctttggcagagatgggtgccaacatcgaagtgaccgatggccatcttcctgctgtgattaacggggaacaattacacggtgtcgactatcatctgaaagtggccagtgcccaggtcaaaagtgccctcattttggcggctttgcaagccgatggggtctcgattctggttgagaagcagccgaccagaaatcacacggaaaagatgctgcgggcatttggggctgagattgaaactgaatcggatgacgtgacgattaccgtccatcctgaaccccacatgaaagggattaccctgaatgttcctggtgacatgtcgtcggcagcgttcttcatggttgccgccagcttagtgccaggttccaaagtcaccttgagaaatgttggcatgaacgacaccagaaccggtctatattcgattttgaagcgaatgggcggcaggatcagcctatcaaacgaacaaagtacgggcgaaccgacagcggatttgacggtggaagctgccgagttaaaaccaatcgaaattggggcggatgaaattccagcagtcattgatgagttgccattagtcgcgttactggcagccaaggccaacgggatcagtaaaattactggtgccggggagctgcgggtcaaagaaaccgaccggatttcagccatcgtcactgaattccggaagctgggaattgatattcaagaactcgatgacggcttcatcattgacggcagaaaaccatggcaggttttggattcgaaattagacagtcatggggatcaccggattggcatggtgatggcagtggcagcgctgttggttgatcagccgttaactctcaccggtgcagacagcattaacatttcttatccggagttctttgacgatttggcaactttaattgcgaggtgagtgctgatgacaacagttttgattagtgggctggggctgattggcagctcaattgcccgaattatcaaggctggggatgcaactgttgagatcatcggcagtgacccggatgacaattccgcccagtttttgttggatcatcaaataatcgatcagcgggctgacttcgctcaggcagccccacaagcagacttgattattctagcgggtccggtatcggttattttgaggcagattgatgagttggcccaattaaaattaaaggagcaggtcttggtgacagatgtcggcagtaccaagcagtcgattatgacagaagccaagcgcctgacacataagggagttgcttttctcggtggccatcccatggctggttcacatttgaccggtagccggaatggctcaactgatttatttaacggttcaaaatacttcctggtaaccggttcacaaaccaaacagcaacttcgcgactttgaacagctgctggattcggcaaatgttgattggacggagataacagcggaaacccatgacaaactggttagcgaactgagccatctgcctcatgtggttgcggcaaccctggttaacagcgtcgcggacggcttggcccatgatccagtgggcttaaaagcggctgccggcggcttcaagagtacgacccgaattgctgcgtcggatccaaaaatgtggacggcgattatgatgagcaattcccaagtaattgcgcaggaattggccacttttcaaaccgcattaagtcattttgaacaagccattcaagaccaagacgaagctgcgatttatgccgctttcgccaaagcacaagaaattagaaagtccttggacgattaaggagaaagcctatgaaactcatattggttggatttatgggaagcggcaaaaccaccgtcggcaacttattggcacagaaactcggcttgccatatcacgatctggacgatgtcatcgtggaaacggccggcaagtcaattaaacagatttttgctgatgacggtgagccggcatttcggcagctggaacatgatgctttgaaagcgtctttggcagatgatgggatcttgggaactggtggcggcacgccgattcaagctgccaactttgagttgttaaaggccagtgatgtcccagtcgtgcttcttgatgtgatgccggaaacaatcattgaccgattgaagaatgataccgaccggccgttagctcaacagctcgggctggatggactggtggatttgaaaggtcaacgggacactttataccaacaggtgagtgattttcgaatcgccaccgatgatttggcgccccttgaagtcgttgacgtcattaaccaagagggcattttgaagatgtcgtttgggaggaattaaaatgatcgatggacacacaaaattatttggcttattagcccatccggctgctcacagcttgtcgccgttgattcacaataccagcttccaagtgacagggatcaacgggatctatttggcctttgacgtgacgtctgccgggctcgccgacagcttggcggcgatgcgggcgatgcacattggcggttttaatttatcaatgccgctgaagaccgacgttttgccattgcttgacgaaattaccccacgagctgagcgcctatctgccgttaatacggtcattaaccgcgatggtcgactgattggtgacagtaccgatgggcaaggctgggtagatgctctcaagcaggatgatatgaccatcgatgaaaaggtcgtgaccgttttaggtgccggtggtgccgggcgggcgattatttccgctgccgtcgacgcaggggcgaagcaagtttatgtatttaaacggaccaacgatctttttgaagccagaaaagaacagttggaagggtggtcggatgtcgtcactgtcctgccttatgaggatgaagggctgattgccgaagcgtttgatgaaagccaaattattgccaatgcgaccaacgttgggatggccggcgatcaatcgctgccagttagtcagtccgtgatgaaccatttgacaccgcaacacattgtgtccgacgccatttactttccactcgaaacgccgttcatccatgcagccaagcaacgcgggagtcgtacatataatgggattgggatgctggtgaatcaagccgccggttcctttttggagtggacaggacagcgaatgccgattaccccagtgatcgaagccgttcatcaggccggcttacaacggtcgaagaattaaggggctaaatgaccgacaagcattctgttttcggttatacttaatgaagtgtcgaaattaaatatcagataacattaggggagccaatcggctgagacggaacatcttcggacccttcgaacctgatctggtttgcgccagcgtagggaagtgttaaaagaagccaaaagcctccttttgttatctaacgaaaggaggctttttatgcacagaaatatgacttataaaatggtgctaacggcgattctatctgcgatcggcgtggtcggcggcagtatgtttgagttcactgtcggcgttgccaaagtggccccgatgcagcatttgatcaatttgatttccggtgtcctggttggcccatggtgggcagtcacccaggcatttatcacttcattaattcgtaatttattgggaaccggaactatcctggcatttccaggcagtatgatcggtgcgttctgtgtcggctggcttttccagaaaaccaatcgactgattattgcggcatttggtgaattgatcggcactggcatcattggtgcaatcgttgcttatccgattgccagttggatgatgggaaccaccggtgcgatttatctgttcattcccagtttcttcttgagtgccttggtcggtgttatcttcggctatatcattctcaagagtatttggaaacggatcattgtacctcaacaggacaaattggggatcggacgcaagactaatcgggattaaacgtttcccggtagtggaatttgccagggatgatatttctgacgtgccaatcccgtgggaacttgacgagggtctcggcgtgcaggactgctgcgtaccccaattcaactttgggcagccaaatgctggtgagcgatggtgtcaggtacgaagcgaattccaagtcatcaaaactgatgattttgacgttttttccaggaaccacgtggtgtttggctaagcccttcatcaccccaattgagagtgggtcggaagcgaccagcaggccgtcgagttgattgccatattcattcagcaggtcatcagtggcatccattgattgcttggtagtccagtccgtcaatttaacgattggctgatgatggttgatcgaacaccatgttttataggtgagggtccgtgcgtcatcaatgatacgaccctggctgccgtccaaattcacttcatgacgggaaccgccgataaaaccaattgtttgggcatgcggtgtcatttcgttcaaggctttatccgttagctgagctaaattcgtatcaaccgtatcgacaacgtcatcgacatcacttccgccatcaaccagaacgacgttgggattaaatgatttaatggcgttgatggcggatttggaaagactgccaacgacgatgacggcatcgtaagccgcaaaatcgtttggctcaacgccttcatccaacctgaccacccgcttgatactgatattctgagatttagcagcttcatagactcctctgcggacaaaccgccagtattcatcgcgcgtttcttctttcagactgagggtagtgatcagcgcaaagttcaactgatttttgtccggtttgggggctagggagtatttataacccagcttatcagcaacttctctcactttgtcgcgcgtttcttttgccacatattcgcttttatccggactcagcgcgcgcgagacggtcccgggtgagacctgcgccagtcgggaaatgtctttgattgtcgccatccatcttcactcctcaattgaattgtattacctctagttaaacacaattaaatgttttaataaatctttggtttattttaataaaatttattgacaatttaactgtaaacgtttacattctagatagcaattattttttaaaatttatttttatgggggattaatttatggcaagtaataccaacattactactggtcgtagaatcacatctcgattatcgtactcatttggtgcgttcggtcatgatatgttctacgcaacgctgtcgacctactttattatgtttgtcacctctcacttgttcgataaaagtgcgggcggacaaaatgatcgaatgatcttttggatcaccacgattatttcactgttacgttttgttgaattagccattgatccatttattggaaacaccattgataataccgaaaccaagtggggccattttaaaccttggatcctcgctggtgggacggttggttccattacattagctattttattcactaatatgggtggtttgaaccaatccaacccattgttgtacctgttaatctttggtgttttgtacatcaccatggatatcttctattcatttaaagacgttggtttctggtcaatgattccagcgatctcatttgattctgcagaacgtgaaaaaacggcaacgtttgcccgggtcggttccaacattggtgccaacattgttggggttatcgtaatgccgctggttgtgttcttctcaatcaatgccaaccatggtcaaggtgacctgcgaggctggttcatgtttggtgccatcattggcctgatttcctggctgtcagctgttgttgttgccatgggaactaaggaaaacgattcattactgcgtaaaaatgctgaaaagacccggatgcgtgatgtgttcaaagtgttagcccgtaacgaccagttaatgtggttatcattgacttatggtctgtacacctcaggaattgccattaccaactcacttgaactttactacttcacttatatcatgggtaaaccaggcgaattctctgtgttggcttcattgaacatggtaatcggaattatttcagtgttactgttcccaccgttggcacagaaatacagccgtcggaacgttttcttcctatctattagcattatgatcgtttcaatcatcttattcacatttgccggcacatcattaccactggttctgctcgccgcaattctcttctatattccacaaccactgattttcttggttgttttgatgatcttgagtgattcagttgaatatggtcagttaaaatttggacaccgtgatgaatcattaaccttagctgttcgtccactgcttgataaattaggtggggctctttccaactgggttgttgggattgctgccgttcttgcaggaatgactgctggtgcgactgccagcgacattacaactcatggacaaattattttcaagctgttcatgttcggtattcctgccttactgattttgagtggaaccttcatcttcttcaagaaagtcaccttggatgaaaaagaacatgccaagattgttgatgaacttgaaaagacttggaacgagcatttggaaactaacggagaggaatcaatggccgacatcgttaaagaagttgccaaagatacgacctataaagcgccgattagcggaacaatgattgccctttcagatgtgtccgatcaaaactttgcctctgggaacatgggtaaaggatttgctatcaaaccatctgatggtaaggtctttgcaccatttgacggaacggttgaagcaaccttcccaacccgtcatgccatcggacttcgttcagataacggtatcctgacactgattcatattggaatcggcaccgttgaaatgcgtggaaccggatttgttcaatacgttcaaaagggtcagcacgttactgaaggccaagaattgcttgaattctgggacccagcaattaagaaggccggctatgatgacacagttatggtggttatcaataactggaaagatatcaaagacttcaactacacagttgagtccggggatgttaaccacggtgatgatttactgacattgtccaaacctgaagaatcatcagacgatagtgatcagaagtaacgcttaacaaaaactgaaaagggattgataaacgtggcaattagaattgaagatcagaatctgctgtttcatttacagacggaccataccagctacatttttcacatgatggaaaatggtgaactcggccagatctattatggcaaacgggttcactcaaagccttcatacgataatttggtaaccagagagtggcataatgccgccgctgtttggcgacttgaccataaggacgtgcagccgcaggtccttaaacaagaatatgccagcttggggaagggtgatttccgttacccagcctaccaagttgcgcaagcaaatggcagccgcattactgaatttaagtatgagagttacgagttggtggacggtaaacaacgcttggccgggctgccatcggcatttgatgatacggatgacgacgcccagactttgacgattgcattacgggacaaattgttgggattagtgatgcatttgaactacacgatttttccccatcaagatgtcatcgtccgcagcgcagagttccagaaccagggtaatgaaaagctcaggttgaattcggcagccagcgcccagcttgatttaccagatgccgactacgatttcattcagttctctggtgcctgggcccgcgaacgtcatatgattcgaacgcacttacgctccggtgttcaaagtgttggcagcctccgcggtacttccagtcatcaacaaaatccctttgtgatgctggcacgtccgaatactgatgatgcacagggttcagtctttggttttaatctgatttattccgggaacttttccgaccaggttcaagttgatcagtatgatgccagccgggttcttgtggggattaacccagaagaattcgcttggaatctcaagccgggcgacaaattccagactcccgaagctgttctcagttacacggatgctggaatgaaccagttaagccagcaaatgggcgccttctaccaagatcacctggttaacccacgatttgcccacgagcagcggccaacgttgattaataattgggaagccacctttatggactttgatgaagacaagttgttaagcttcgcgaccaccgccaagaagctgggactggaaatgtttgtcttggatgacggctggtttggtcaccgaaacaatgacgacagctcattgggtaattggtttgtcaacgagccgaagttcccgagcgggtttgggacgtttacccaaaagattcatgacttgggattgaagtttggcctgtggttcgaaccagaaatgatttcaattgatagtgagttgtataagcaacatccagattggttaatcaacgcccccggacgccacgcttcacctgagcgtcagcagttcgtgctcgatatgacccggtccgaagttgtcgactatctcttcgatgccatgagcaagatcattgagatgaccaagctggattacatcaaatgggatatgaatcgcaacattaccgagacttacagcagtcagctcagtgctgacgaccaattagaagtgccgcaccgatacattctcggtgtttatcagctctatgaccgcttggtcaaagcttatccggatgtcctgttcgaatcctgctcgtctggtggcggtcgcttcgacttggggatgatgtactatgctcctcaagcttggaccagcgatgacaccgatgcagttgagcggatgctgattcaatttggcacatcttatggttacccgcaaacgatgatgggtgcccatgtctcagccgtgccaaatgatcaagtcggccggatcacttctttgaagacccgtgccaatgttgcttacttcggtgattttggctatgaactggatattaccaagatgtctccggaagaacaacaacaggtcaaagaacagactgccttctacaaggaacatcgccaactcttccagtttgggaaattctatcgaatcgataacccatttgccaatggcggtaacgtcatgagctgggaagtcgtcagcgatgatcaaaagcacgcaatcgctgcgcgttatcaaattttgaatcgaccaaacaccggttacatccgcttgtaccttaaagggctcgaccctgacaccaagtacaccgttaatggtggcagcgaacagttctacggcgatgagttgatgaacgctggattgtttgtaagtgacattctccatgaaacgcacggaactgatcagtcggctgactttaattcaaagctgtttgtcattgatgccgtcaaataatcaattaaaataaccaaaaatgccagttagaaaactgatgatcatcagtttctaactggcatttttatgtttttaaggctactcccagacatccaacttatgcgacttgaagtaatattccttatcatgatcgttaatcgatcgggccacccgacaaggattaccatatgcgacaacattatcgggaatatctttggtcaccacgctgccggcaccgatgacggtattgctgccaatggtgactcctggtaagatttggacaccggagccgatccagacgttatcttttatggtgattgggaaattatattggtaaccgtttttcctcagaatcggcaggaccggatgcccagcagtgctcattaccacgttggggccgatcatacagtgattgccaatggtgatgtcatcatcgtccaccaaggttaagttgaaattgatgtacacatcattgcctaaatgaagatggtgagcgccccagttagcgtgcatgggcggttcaatgtagcagttttcgccgacttccgcgcacatttcagtcagcaactgattgcgtttgtcggtttcttttggggatgtcatgttaaatgaatacaatttctccaggtattcctgttgtcgatccattaattccggaacgtccgggtgatacagcagatgtttggcttttcgctcgagattattcatggtggaaccctcctttgatgactcaagcttatcatttttggcgatccaacaggggagaagtgtcgaagatatttttgtacagttcggcggttttgaaattcttactttcttattctggtataaaagttgtagtatagaaagagtgacttttataagaaagaggagaatatcttgtctaaacgcgatatcatgattgtgacttgtgcactgttgctgtcaaacgcaatgagtggactggacaacacaaccatcaatactgctttaccagcaattatatccgatctccacggaattgaattaatggggtggatcgtcgccgttttcctgttgggaaccgcggtcagtacacctttatggagtaaattgggggaacacatcggcaacaagcgcagctaccagttagcagccaccttatttgtggttggctcatttctacaagggatggcgccaaatattgtcttcttgattctcgcccgaaccttgatgggaattggtaatgggggaacggtttcgctgccatacattatctatgccagaatgtacaagaatccccgcaaacgaatgcaggtgttgggatttgtttctgctagttatagcatggccacgattatcggcccactagtgggtggttatatcgttgatacatttagttggcactgggtcttttatctgaacgtgccgattggcctgatctcaattgccttggtccaaatctattacaaagtcagtcatgaaactcgccagacccaagcagttgactaccggggagccattatgatgactattggattggtgggtttgcttgccggaattgaaatgatcggcaatgccaacttgattttggtgctggccgtgattggattttccattattgtcctgattgtcatggggattttggaagagaatgtcgacgatccgattatcccaagtcgattattcaagaacctgccgttgatgattgactttgttctgttcacattaatctggggagcgtttattgccttcctgatttatagtccaatgtgggcgcaagggttgttggcaacccctgccctgattggtggtgccacgcaaattcccggtgcctttaccgattttatcgggtcagaggtcgttgcccccatccggaactttttgtcgccacaacgggtaattgccatggggatcgtcatgttaatgatttcctttatcatcatggtcatctctggcgttcaaacgccttattgggtgctattgattgccggcgcctttgaaggattcgggaacggagcctgctttaatgaactccaagttaaagtccagcaagatgccaacccgacggatatcccgattgcgacttcgtttagtttcttgattcggatgctcagtcagacattcacggcttcaatttttggaatcattatgaacaatgccttacgtgatggtgtcagtaaggctggcggttcgattaccatgaaaatgatgaacgaattaagcgatgcctccagtagcggttccttgccgcagcacttactgccgcaaatgagaatgattttgtataatggccttcacaatattatgtggctgtcgttgattttgatgattatttctctgcttattaacatttgggcacagaaattggaacatgataaagttgttaaacgggctgccaaagcatcataaaaagtctccatcaaaaaccaatttgaaaactggttttcgatgaagacttttttattgtgactatttcttagcagttaatgatgtatctttaaaggttgatagtgaaacatttgcggttgccaaactattgccggtaaccgtttcggccttgaagctgacccgatcgccttccgcaatgaactgcagcaatgggttgaagttcttggcgctggtatcaatcttataaacttgattgttgttcttcaaaatgaacagtaaactgttatccgttcgaacaactcggttgatggtcccgctcacggtcttaccggctggaaccgatgctgcaaccccggtctttgcctcgactcgttgttcgaagattgccaaggtgctttgggcatcgtcgccaattgcgtaagtgccactttggttgttaccatccgccaatagataaacgtatttcataaatgagttattatcccgatcaagcatggagacaacccaagtggggtccccattgattcggtacagtaacggtaatgtcccgcggtaattctgggggttgatatcctgttgggcataagagattgcccgttcaggcgtcataacattgccatgctcacgataatagtgcagggtgttggtccgtgcatcaacgaaagtatatccaagaattgaactctggtgttcgttgacactggtcataccggtgaagtaatagacacggcctttgtaagcgtaaggcgtcaacttgtcgccgccttcagttccggcagtggttggcttcataacgccactgtggcctccaaagctggttgcgttccagaagccgtgccgataacggccaaacattgagacttcctgactgacaaattcaggggtgaccgcaatatcaacgaacttcggcacctgcttaggtgagtagactttcactttaccggtaatcgtgttcagaacagcgactttatagtgtttaaagtcatagtttcggttcaagtatgaaattggtttggcaagtgttctgacatagtaaggcgtgccgttatcgtcaatttccaattgagccgttgcaccaaccattgagtagcccaaactgtgggcgctgatccgccggtcggcatcattgttgaagtaggcacttggcgtgtacttcatcggcttggcaacaaattttggatcggcattcttgtcggtggcgttggttctaaagtaaccaggcactttcaagtaatgaagataacgccagaagccaccggagaattcgacaggggcaacataaatcatcttgcccttatacatctgaacccgcatgtgattcaaatcataaacgttggagttcttaaaactattcaatgagttattcatatcggtcgaaatcgtttgtggtgcgttcactacaggcgtttcggcactgtttttgatcacgggcattggcgcgttcttggtgtcatcgttcatatccgtttggattgattgaacggctggtcgtggattcatcttggtgaccagggatgtaatactgcctaggatgatgaggacgatcacggcaagaacggcgaccatggcgattttacccaaccagccaaatgcgccggtgaatcgctgaacaatttggccaacgatcccatcgccggcttccgctgttcgagcaacagcagcgtgtggtgaatacagaaagcggcggagcgcagcgacaacaatcattccgaagatgaaccacatcaaccaaccatcgatcaaagacggatacgcaagatccggcaggttgaagtaggtgttaatgtaactgacgatgaacaatagcacaatggctagtgttccgtacgttcgaccccggcggtctgcgataaccagcagccagataaatggaattaacaaacctgacagcttaaccagggtgatgagtgcaaaataactaagcatgaaatttctcccttcaatactgttaacgagtttgagtattaagactattataccttactcaagaggcaacacctaaccgctttcaaacggttaattcaggtacccgcttgcaccataggatcacaaatgcgttcgagccgatgtgagttccaaccaccggtccgatctggccaacttgaaaactggctttgggatatttgggcttcagggatgcacaccatttttgaacggctggcaggttattggtgccggtgaccatcacgtgaagcggataagcgactttctgatattgggtgttgaattcttcatccaagtgcttcaaagccttcttcatcgtccgaatctttccgattgcttcgatttgatgctggtcgttcaaagttaataacggtttaactctcagtaagccacctgcaaatgcagcggcgttggtgagccgcccgccggtaactaagttcttgaggtcatcgacgacaaaatattcatcgatagttgcccggacatcatccagattttggagaattgtgctcattgattcgccttgattggccatcattgaagcgtatttcacaagatatcccaacggttcaatcgtgatgtgtgaatcatagacttcaacctgggcgttggtatagccccggactacagtgcgcagattgttgacaaagcccgtgataccagtagtcaaatgaatacttagaatctggtcgtagccttgattggccagctgatcatacacttttaacatttccatcggtgtcggcggtgcagttgtcggtaattttttggccttcgccagtgcggaatagaattcattattggtaatatcaattccctcacgataggtggtaccgttcatgttaacgacgatcggaacgatagtcacgttgccaagccgttggacttcttcatcagaaaggctggccgtgctgtcggttacgattgcgattttactcattgtttcatctcccgatcttagtgatgttaaattgattatagcatatactccagcatgccatgccgcatctgagggtacggtaagccagggatcgtaaaatttgatgaattatgaaagaattctcatcaaaatagcgaatcaatatgagaagattacccagtcaccaaagtttcgattgccgatcgttcatcattttgctgatcatattgtctatcgctcattaagcaatgcccttaaggattgcgaccgcttacttcaaaaacggtctatgtacacaaatggcccccagcgatttcttttctaaaatgggtgttgacatctccacgtaatgatgtttaaatgataacaatttaatttttatcattattttctcacgcaattataattatagaaaaaagcgaggtaatgccaatggatacagaagcaaataagccagttgataaactgacagtcaaagattacgtatacttagtttcagcaggggtttcaaacgccgtcctagtgatgttaggggtcggattattaacccagaccattgccaacttcgtgaattggccacagttacaccaagtcggggcaattgcccaatggttattggcacctgcatttggtgccgctgttgcatctcaattaaaaaccaacacactggtcctgtttagttccatgattgcctcaactgttggggccaacgccgtttatttcatttcatccggcgttcacgcagcaaccgccactggtaaccagatggcacaagcagccggaaccggtgtcttcacaactggtcaacctattagtgccgttgccgccgggttaatcgctgccttagttggtaagtatttaaccggtaaaacgccacttgatatgatgttagtaccacttgcctcaaccttagttggttcaatcgccggcttgggacttgcaagtgtcaccacgccagcccttaactggttgagtgcctttatcgctcaatcaatgcaggttaacccaatcctcggctcaatggccgttgccttggcatggtcactcttcttgatgacaccggcatcgtcagctgccctggcagttgccgttatgcttgatccactttcatcaggtgccgcattgattggaacgaccgctcaatttgttggcttcacggttatctcatggcgtcaaaacaaccttggtgccaacattgcccaaggcttcatcacaccaaaggttcagttcccgaacttgttggccaacccacggctcgcaattccttcaatgactgccgctgtggtggccgcaccgattgcgacaatgttctttggcttcaaggtgccttacacattaggcggcctgggattgaactcatttatcgccccacttaacctggcatcaaccaacatgaacatgttcgttgcttacctgacaatgggaatcgttgttccagccgttatctcaatcgtgctttacagagttcttctcggcatgcactgggttaaggatcaacaactgcatcttgaaattgtttaagctattactacctatattaataatataaaatcaataacaaatagaagtcccggagctggattgctctggggcttctattttgttgatcgtcattgtttatttagtgcacgatggctgttactttggaaattgcggtacctatgtaatgctggtaatgagcagcgggatactttggttccccatttatacctgtgattttataaccaatcttgacagtcttccaattcttttcaggtgtaatgaagacccaaacagcttttgacaggtcattgttttccgccccatttagtacatatgtcgtgtaatcatgcgtgtaaatcatccatttgcatctgagcgttcccgtagctgtatttttaatgacaaacccgtctttaacagcataaaagtacatatgttttggaatagaattagcccctcgattgaccgtggcacgccaatatcttccttgaattggggcggggaaacaatcatgtacccggctggcactggccgttgaactgaacataactgatagtactaagattcccacaaatgatatgatccacttgataatcttgttcatgatagttccccctgttggtaactttttagtacctaaagtgggattggttctaattatttaacttgtcaattatttttttggacaaaattgtgaataaaaatatttaaaatatttaattagtttggctgtcctgtcgcaaatatagaagaaaagatctaacaaaattcaacatcccgttacccattgaacaaagctattgtaatatattcgtaaagtgctataacgagaaatgggtacaataaatgttacccaggtaaaacaaattattttgggggtctcaagaatgaaagtcaataagattgaacaaacaatattgctagcgctttccgttatgggggtttgctagggggagcggttggtgcacatgcggccactgccggcacaaatagtcaaccgattgctcaaacctcagttgtgtcgcctgccggaaatgcgacatcagatacaaatacaagtaagagtgcttcggttcaatcaacaaatggtgttgaaagctcaaacactgcagggaatatggcgtcgaacaatgaccccaacaattcaaaagcggatacagttaatcaatcagcaacgccgaaagccaaaaagaccgtttctcgttcaaccgagtacagagaaacgaaaaccaacaccaaagttaagaagactaaacggggaactaagacggttaagcaacaagtgattcgcaagcaggttgttaataacaccaagaagggaaaatcagctgatcagaccactgataattcgaatggcagcaatcaggctgacagtaccaattcgacccaagccgatacatcgaccaatgcagctacaccagtgaataccaataatactgccgcgcaacaaaataccactcaggctcagccaacgatcacgccggcagaagcccaagcaaatcaggatgcacaaaatcaaaatatccagctgcagcctcagttaactcaatcgcaaatttccgccaataagggccaagcaatttacgatattacgggtgctttttctaatgttgttggtcagggaaccgcaattgttaattcaatctgtgagattatctcaaccattagaaacttgctttaacttgatctagagggggataatgatgatgaagcctatcaagtacaagtatttgtatagagctttaagtttagttggtatttcgataatgtcgctgttgttggttgggacaactggtgcgtccgctcatgagcagagccaattcaccaatgtcactaacagtcagaatcaaaataatgacgatgacaacaacgacaacgacaatgacaacggtaataacgataataataacaataatggcggtgggggctacattcctggtggaaattccggtgggggtagcgtcaataacaatggcggtggaggaatatctgccggtggtgcaacagctggtgccacagccaataatggttctgccactgttgtatccaatcctcaaggccagtccgttaatgggacgaataacagcactgctgagggcatgacaggtgtcaacgattctgttggttctgcaactacgaaaacaggtagtgctgtcaccggtagaagttctaaccagactcagtttcaaagtaacaactctaagaacaatggtgcttctacatctgttacttctcaaaaacagccacagaataaggaaactcgcaactcccattctgatcattattctcagaaatctatgcattcaaacggtcaatttcagccaagcaataagacaaaacacaagccttataagacgacttggagaaagggacaaaagctggatagaaaccagcaaagggaagtcaggtatgaaagaaggcattggaaaaatacaataaaagatatccaaactatagtcacttctggcagggtggtgactgtactaactgggcatcacaagatagattacatgctgggggacgaatgacttctagccagaaacatgctaaaaagcacttttggtctggaaacagaatttctacaaaacgatcaaaatggtattgtaaacggatgaaatcaacattctttggtgctcgcaaacactggaactattccacaagctggacaacggttaatggcttctaccgatattggacgaaaacgaagcatcgaccacactttacaacaactagttttcggagagtaatggctcatgtccatgttggtgatgtagttcagttacactcgaagaaagatggatggcaccatactgtaactatctcaaaagttacaaagcatatggtgtactatacgtctcacaacaaaaatagaatttttgcgccgttgacgaaaattaaatcattaactggtctttctaggacaaacaaaatgcgagttattgaaatggggatttaaaaatgaaaaggaaaataatgaaaattgtattcgtagtgatgggtgtacttttcctgacatgcttgttttttacgatttcagtaaaaaatgccgttcgagctaacttgatggtgcatggtgtatcgccggtttcagcttttaattgtaatccaaagttttctccaaaaacgagtaagtcgctacaaattccagtatattatgttcctgacaagtatgcttacaaagatgggagtacaggtgttcatacgtcaacctttgctatccggacgtatttaggaatttttcacgttgctgtcacggctgatcaatactttggatagaaggaaagctatgtaggagaccgatcagttgacctcactactggtgattggtattcacgggggaaagaggaaaagcagatgaaaaaagaatggtatcgagtatttcttctaatgatcatgacatttgccggagcactattgattggatgcaatcagatacatgctgctgcatggcagccatacagtcccaaaattatgggatacgcaaagaagcagcggattctcaaatacaatggaagtaactggggaaactatgaagagatttatgagaagaggtattttaaggataccaaatcaactaagtataaatataatcatcaatctcgggtgatggttattcgctatctgaacaaatcaaaatcccctgaagtaaatacaaagtacaattatcgaaaacttgttttccatggaaacaaacggcacccagttattcaatattattacaggctcggtagtcggaagtttcagttcctgtatacgatcaagtactggatgtttaagccaatcaaatattagtccttggaagtgggctatccggcgacgtatcgattctggttggtcaagccggttaatcactaactaggtcagtcgcatttaagattcgttggattgtggatgagtgttgttcacaaacacccattaaatgaaaggtcgatgatgaacttgttagttactaggcaacatcggattactttaaagtggttgttactgttagcgttcttttctgtattggttttagtccctacctcagcgtctgccagtgccaactggaaacaccttaatatgaattcattaggagctgccacaaagatgaaagttcttaaatacaattcacttaattggggtgagtattatgatgatcagagtgatttgtttaaagatactaagcatgtgcaatataagtacgccaaacgcacccgaacgctcatcatgcggtatcggaatccccagcagtttcttttaaaaactaagtataattatcggaagctgatttatcgacatggtcataaaaatccaattgtgacccattactttaaagtgggacacgaaaagtggaaatttgcaacgaccattcattattggctaaagaagccaatccgatattagttattaacggaacctcgaagctgatacttcggggctttcgttcctatggtttacctctcagtattattttaattatgtccccaaattgtttaattttaaacaatttggggacataattaaaatagcttgtctttaagaatcggtggcgtagttatttaaatctaatcttacgtgtgaatatccactgatttttaggaaattgggcgataatacaaaagcaccaactatattggaatagttggcgctcgcctgtgatttaatttaactcagtgaaatgcattggcttaagacgttaatcaaaaaagccaaaaatatctttaacggcagtcatagcttgtgctaattctgccgcattgacatgatcaacaatcttgccggatcgggcgatgtagtcataacccaaaagaccggttaaaataacatggccttctatcttatgagaagaaagtgtaatctgaaaaggtgccttaattttagttgcatgggtaattggaaagccgacaatcatacctgtccgttgattatatgctttatcactgacaaccagtaacggtctaaaagtattactggaatctggattatggccaccatattcatggcctgcatgcggttcactatcgatccagatgagatctccttgctgcgggatgtctttagtcattccaaatatcctctcgtccaaccggcgtgccattgtccccaatgttttcttcttccattgcttttcgaagatcgtagttcgagtctgcactataaatgttgtgtcgaactggtaacaaactgatcacgccgttttcatccttgattggttcaaactcaacgttttcccctatgttaaacgaagcaggaattgtcaccataatcgaattgccttgacgccgtgtttttacagtcattattaccaccctttctacacgtaattatatatgtaattacatttaaactcaagaaatttgtatcgattaaaattagaacgatctatttgttttgtacgttgaaaacatagactgggaggcttacacttataagcatgctaagtacatataataggaggaaaagatgaaagtaatcaagagcatcttcagctggatcctgccaattgccattggattggcactggcgttactactcaaagcctatattatttcaccagtcagagtggatggtgattcgatgatgcccaacctgcagaacaacgagcacgtggtcattttaaaaaccaagccaatcaaacgcttgtcagtggtagtgtttaatgcttacaaattggcaccggatacgcaaccgaacactgaatttgtcaaacgggtcattggcattccgggtgacaggattacctatactaagacggggcatttatatgtgaatggtaagtacatcaagcagccgttcatctcccgtcagcagcagaccactggtactttgagcaacgtcgacggtaatggttttaatttatcgattctttccaagaagtggcgcagaggtggacagactgctgtggttcccaagggtcagtattttgtgatgggtgataatcggaatatttcctatgacagccgttactggggatttgtgccaaagtcgcatatggaaggcgtcgtctacacattcccgtgggatgacaatcgaagtgaaattaataactatggataaagtaatgtccttcaccagttttagatctggcgaaggacatttttaggttctacaatatctgttcgcaattaaattctaaccgtaacgttttcggtcatttggcgaatagatagcgttctaaaaaaattctttgagaacgcctgaaatagtttggatgatcgttgtcgggacctgcccaactattttgccattagatcgtttctcgggatcaatggcccgaacatgttggagaagtgctgtcccatgaacttgctctaagtcaatcttttgaaaaaacggtgaacgaataaatctttcttgtgtccggtacttatcagatgaactgataggtatgactgggacggtgttgagatgccgattatactcatcgttactaacaaccatacatggccgctctttctttgtttcagtccccttggcaggattaagattgataaacagtatatctccttgatgtaactccattaatcaaaatcctccgaaccggcatcttctccccaatccacttctggggtgacaatactcccatattttttttcttgctcatcaaccattttccagaaatcatccttttcgggagctgtccgttttacagtaatttggccatcagcacctaattcccattcaatcttatctgatgattttacatttaaggcctcacgaatggttttgggaatggtgacttggtttttggcggtgattttagaaatgaccgcaatgttatgatcatgttttgccataacactccctccttacttatccttacatatattataattcaaagaagttggtaaggcaaatgtaaggtacaccatgtgttgtggtatcagattgtaatcagtttttgaaatatattttaagatgtttgaccaagaacccatttgaattacttgccatttaattcacgaacttgatcaattaagccaagaaaatcattagccgcctggcgataatcttcaatctgatcaccgtatttttcgttaaagccttccaagccaccggcaacaaaggcatattcataatcatataccttgtcataagcagcggtgaacttcgtcaacaggtcgtggtgcttgccatccagctgcagtgccatttggacaactcgcacatccgtgtagccaagctcgaattgaatcacccaagctcggatgaagtcgtgctgcgcctcgatgtgagcaaagtggtgctgggtattccaagttaatcgatctaatgatttgataacgtctaacatgtcattacctcccctaatcagtaatcatcatatttagttcatgttcattgaaccgcgtttggcgggggagggcaagtgattcgacttggaaatatcaaagagaaaaacgccttaaagtatgttataacagatatgtgataaaaatcacaaaattgtttctttggggagatcttatgatgcaatgcattcgtatttcggcagtctttcttagctttggactgctaacaactttcttattacagattatccaattggtatcgaatttttatacggtggacagtgcaaccgatgagccaatcaactattgggcaagcagcatgattcttgttccgttagcctttggagctctttttattatcacgttcgcattgggcttgtaccagatttatcaagagaaaaaacaaagtaaaaaaagtaaaaagtgaagaaacacaaataagcacccttagagcattgagcctccgagggtgcttgttattttttaagagattttatttaatcaattgtggctgaaacacacccataacggtatcctgggcagtgaacacaggaacctggtgactaagggctttggcaaccagctgcttttgatcagtggtttcatcctctgaactcagagcaaaggcgaggttgcttggccattgcattccttcgtggtaggtttgaatgccaaagccgctgccctttagttgctcgactaagctggcgttgttggcatcaaatgctgacaggagcacatcaccagttaggtgattggtatcaatgtggtagctgtcaaacagggcattgtgcaaggcttcctgcaggttgccgccggcgccgatgtcttcgccggttgacttcatttctggactcaatgcggttggggcacctggtaacttcgcgaaggagaagactggtgctttgacataaaccttggttggttctgggtgtaaccccggcttcaaaccaatttcagccagtgatttgcctaaaataagctgagttgccaattgtgccaaatgtagtttgacgatcttactcatgaacggcacggttctggatgcacgtgggttgacttcgatgacgtacacttcgtcagcgacgatgaattgaatgttcatcatgccaaccgcatgaacctgcttaccaatcttggtagcgatagcaacgatcttttctttctgatcgtcagtcaacgtctgtggtggatacatggcaatcgagtcgcctgaatgaataccggcaccttcaagatgctccatgatcccagggacaaagacgtcattgccgtcgcttaggatatcaacttcacactcagttccagggatgtactggtcgattaagattggttcaccatgactgttcttgagcgccgggatgagatattcgtttagttcgtcatcattatggacaacggccatccctttgccaccaagaacgaagcttggacgtaccaataccgggtaacccaggtggttggcaatttctaatgcttcaggggcatcggtagcggtagcaccctttggatgagcaatgttttggtcaattaagaggtcttcaaattgatgacgatcttcagtttgctcaatgccgtgaagggaagtgccaaggatggaaaccccatgcttggtcaagccttcggtcaagttgatggcagtttgaccaccaaattcaacgatgaccccaatcggctgttccaaattgatgatattcatgacgctgtcaatggttagcggttcaaagtagagcttatcagaaatggagaaatcagttgaaactgtttctggattattgttaataataatggcattgtaacccgctgcttgaatcgctttgacacagtggacagtggcgtagtcaaattcaaccccttgaccaattcggattgggccggcaccgataacgacgatactattccccagtggcttgctttcgttttcgttaccaactgtactatagtagtaaggcgttgtgctttcgaattctgcggcacaggtatcaaccatcttataaaccagatgttgatctgacattttgtctaatttggtcaactcatcgtcggttgcgtgatgaatggcttgaatcatggtgttgttgaagcttaatttacgggcttttaagacttcatcagcactcaagaggccatcggtcatctgttgctgcatcttgatgatgttttccagtttcgataagaagtacatatcgatttgagttgaacgattaatctgttgaatggtagcacccttaccaatggcggcaaagatttcaaataatcgataatcggttggcgtcttaatcttttccagcaagtcgcccattgacatgtttcgggtataagccggaatcaggtcagtttgcgcttgttggtcgagttccaatgattgaacggcctttaacagtgattcttcaatggtactgccgattgccatgacttctccggtggctttcatttgggttcccagtttgcggtctgcgtttgtgaatttgtcaaacgcaaagcgtggaatcttagcaacgacgtaatcgagcgccggttcgaacatcgcgaacgtggtttgcgttattgggttcatgatttcgtccaggttcaaaccaactgcgattttggccgcaattttggcgattgggtagccagttgcttttgaggccaaagctgaggaacggctgacccgtgggttgacttcgatgacgtagtaagcttcactgtttggatcttgggccaattgaacattgcagccgccttcgatcttgagggcgttcacgatggtcaatgatgcgtcacgcagacgttgatattctttgtcggtcaatgtctgagttggggcaaagacaattgaatcaccggtgtggatgccgactggatcgaagttttccattccagtcacgatgattgaactgccgtggtgatcgcgcattacttcaaattcgatttctttgaagccggcgatactcttttcaactaaacattcagttgagggtgacatggtgaggccacggttcaaaatggtggtcatttcatcgtcgttatgggcaattccgccgcctgttccacccaaagtataggcaggacgaataatgacggggtagtcgatcttgtgagcgaagtccaatccatcttggaggtcgtaaactgttttggaatcaggaattggctggtgaagctcttccatcaagtctttgaatttctcacgatcttcagcttcgttgatggtttgcaaactggttcctaataattcgattcccagttcatctaagataccgtccttgctgagttcaacggccaggttcagaccggtttggccgcccaaagtcggcaagatagcgtctggatgttctttgttgataatcttcttcaggcttggaacggttaatggttccaagtagaccttgtcagcaatttcatcatcagtcatgatcgtggcagggttggagttaaccaaaatcactgagtagccttcttcacggaggctgaggcaagcttggctgccggcatagtcaaattctgcggcttggccaatcacgattggacctgagccgataattaatacttttttaatatcttctctttttggcattaatgaacccctccgtttacgtgcattatttcgataaagtcgtcaaataatttggtggcatcgtgtggacctggtgcggcttctggatggtattgaactgagaataccgggcggccgggatagcgcaggccctcacacgttttgtcgttgacttcaagcgcagttacttccagtggggtgtctttaacggagtcgacgtccactgcgtaaccatggttttgtgaggtgatgtaaatgtcaccagtgatcaggttcttaaccggatgattaatcccacgatgaccaaacgtcattttgtaagtggtggcgccgttggccagtgccagaagttgatggccgagacagattccaaacagcgggaagttgtcctggagcttttgaatcaccggcacaaagtctgagtaatcggttggatctccaggaccattggataataggatgccggttggatgtaagttggcaatatcttcaaacgttgattcaggcgtaacgacggtcacatcaacgcctgggcgctggagtgacttgacgatgttatctttgacaccaaagtcaacaacgacaacatgttcaacatctttggcgtcgcctgcggacaatgtggctgatttgataatggatgccgagcggtcagcttttggttgatcaacgattgggtgattggtaaggctggccttcattgtgccatagcggcgaataatcttggttaactgtcgggtatcaatcccgctgattgctggaaccttcgactgctttaggaaagcatcgaggctgataacgctttggtaatgaaatacttgatcggtcatttctttgacaacgactgctgctgcttgaacggtgtccgattggttggtgcccagtgagatgccatagttaccaatcaacggataggtgaaactgatgatttgatgtttgtacgatggatcggtcaatgtttcctggtagccggtcatgctggtggtaaagacgagttcaccatcaatttcggcgcccaagtcaccacacgcttccccgacgaagacatcgccgttttctagagttagatactttttcatgtccgaacctcctcaatttgttcctaacaatgctgcggtatttacagttaacgcttttgaatatttaagatagaagtatttagggcaaatgtcaagtgaaaatatgcaatatttgccgatattcggataaatatgtacaaataaaaaacactatgtatatttattaaatatgccccaatgcctcgaaatcgcgtccttatagataagttagtcgtcactttttaatatattcgaattgttggataaataaacattttcaaaattaatttcacaaatagacttgttttttctctcaaaatagaatatgattctaagtaatcaaacagaacctttaacattaaccccgtgaggttaagaaggtatggcgaatcttgaggagactcagggctaactcaaacctctttaccgaacgcggtaaagaggttttttgttacatatctactaattcttattgacgatttaactgttcccgtgagagcaaaacgtcctggaatgtggttcccgacacataaggagcgctttgcgaacacggcaaggcgcttttaattttaggaggaaatcacaatgatgcagattactaaaccggtaagttttgaaaatgttgtaagtatggaagatctttcagccgaagatgttttatcatttatccatgaagcacaggatttcaaagccggcaagcagattgagctaaaacggccggtatacgccgctaaccttttctttgaaagcagcacaagaacccacaccagttttgaaatggcagaacgcaaattgggccttcaagttgtcaactttgatccttcaaacagttctttgagcaagggtgaatcaatgagtgacactgttaagactttccaagcaatcggcgtagacttggttgccatccgtgataagaagaatgaatactacaaagatttaatcgctgatccaaatgtccacgttggcattgccaacggtggtgacggttcaggtcaacatccatcacaatcattgcttgacatgatgactatatatgaagagtttggtcattttgaaggtttgaaagttgccattgttggtgacttaacccactcgcgagttgcccgctccaatatggaagtcttaaccatgcttggcgcccacgtctactttggcggaccaaagaagtggtacaccgaagaatttgccaagtacggcgaatggatgccaattgatgatttggttgaagaaatggacgttatgatgttcctccgtgttcaacacgaacgaatcgctgacgacgaaaatggcgccttctccgctgaaaagtaccatgcccaatatggtttgactgcagaacgtgaatcaagaatgccacaacattcaatcatcatgcatccagctcccgttaaccgcggagttgaaattgccgacgaattggttgaatgcgacaaatcccgcatctttgaacaaatgcacaatggtgtgtttgtcagaatggcaatcatgaccagcatgcttcgcaaccgtgacctcattaaggaagaatattaatagcgaggagaatttcgactgatgaaacgcatcattgcaaacggacaaatactggatcgtggccaattagttaaacgcgatattttaattgagaatggtagggtagctaagattgctgaagacatttcaactgatggagtggatgaagtgatcgatgccaaggggaactttgtctcggccggcttaatcgacgtccacgtccattatcgccagccgggtcaggaacaaaaagagaccattaaaactggtagtctggcagctgctcatggtgggttcaccactgtttgtgcgatgcccaatgtcaccccggcacctgactcagttagtaatatggaagctttaattaaattgaaccacactgacggtgccgttcacatcaagcaatatgcgacgattaccaccaaccgtggtggtgatgagttggttgatttcaaggcgttaaaggatgccggagcctttgcttttagcaacgacggcaatggcattcaaaagagcagtaccatgtatgaagcgatgcagcaggctgccaagctggacatggccattgttgaacacgttcaagatgatgccttgacatacggcggtgttttgaacggcggggccgctaaacgtctgggaatgaaagaaatgccttgggtcagtgagacggcccaagttgcccgagacgtcattcttgccgaagcaaccggcgttcattaccatgtctgccacgcatcatccaaacatactgtcaacgttatccgggctgccaaacaagccgggattaacgttaccgcggaagtttcaccgcaccatctgcttttgtcggacgccaacattaaagaagacaacgcgatgtacaaaatgaatccacctttgcgaggagaggatgatcgtcaggcattgatcgaaggcctgcttgatggcaccattgatatgattgctaccgaccacgcccctcacaccaaggcggataaggatcaatcaatcgccacagctgcctttggcattaccggcagtgaaacagcattcagtatgctatacaccagatttgtgaagaccggtcggttcacgttggcccaattggttaattggctgaccaagcatccggcatccgtcttcaaaatgagaggcgccggctcactggcagtcggccagcctgctgacattgccatctttgatttggaacacgaacacgaaatcaaagaaagcgactatttgtcaaaaggcaagaattcaccatttactggcgaaacggtctatggcgatacggtcatgaccttggttgatggtgacattgcctacaagagatcgtaaattaatcacataaaaacatattggtatcaataagaataaaggttcttcgtcaactgttgttggtgaacaaaatattggagttctaatcacttggtgattagagctctttttgtatgaactcgaaaagcgaacagcactcttagccggaatctgaagaagtttcggtaaccaaatccagtgcgtttaatgactttaatcttgttgtttgaaccttctaagggcccgttggtgtaatggtgagtaaaggtattgccaatttcatcatgatgagtcgctagggtctggagggttgccaacatctcttccgagcagccctctaagtgatggaatacttgattatagttgggccaatcacggtttttgatggtttcacgtaaccgattcatcacgttgtaagtttgcttgagctcgggatcaatgtccaataaagcatcaaccacatcagtggcagtcgctggataagggaagtttgtccacttacggaaagcttcgtagttgaggtgattttccggcgttaataatagcttccaatagcgtttcaaggcgtgatactcgcgtgatgaggtcgccagggttttcatgaggcgcacccgcgtcttattaaaagctcgatttaaagcgttaaccaagtggaacggatcgatgacaacgatggcgttcggaaagatctgccccaccaatttgggataggtatagttcatatcggtgacaataattttcacattttctcgcgcagcctggtcgtaatgctggaaatacttttgaagctgatagatggtcctaaagggtaacaggtcgatcaattcgtgggtttccgcgtccataaattcaaagctcatcgcgtcggtggcgctcttagtgcttttaacttcgtccatgaggagaactttgggtaaatagtgccagttggtttcaaagtcccgttcagcgcgcaagagctgccgaccaacgaatgaatccgaagtggataactcatcggcaatgtgtttgagcgaaaccggttcggtcagtttttctaagcattgtttgcgggtcgtatttgaaatcgtgcagtgtttcggcaccgcattcgtctgcgccaggaagttggtatgacaagccttacagtgaaagtttcgccgattgaggcagaggataacggtgctgcccaaggttttagcgaatctaatggtggtcttccgccaaccatagccaatgatctgatggtcattaataaccccacagttgtggcaggccttgggggaatagttcagcgatccatttaatcggatcaccccatcatcacctattttgccattctcaattattaagtgttcatcatctattcctaacaacattttcgtagtatcatttgacatagggcatttcctttcttgacttaattctgtggtgggagcaagttaacggacgggagatgtccgcttttttactctaatgataaacaaaaaactgtcatcagtaatagacaaaaatctattaccaacaacagatattgtagaaccagaataaaaagctgcagttcaccgagactcctaactcgatgaactgcagcttttgtattatttgagaaacatcgtgtaatagccgattgctgaaaccgcttgggcggtgttgactttaccttcgcggatccaatcgacgacttgttgaagtggcactaattgactgttgacgaactcatcttgatcaaagtggcgttccacgcgttcgctaggatcaaatttaatcaacattaggtcggcaaattggtccatgaagccttccgaagaagtgattcgagtcatcttagtgactgattgggcaacgtagccggtttcttcccgcaattcgcgggcagcagcctgttcactggtttcacctggattcactatgccagctggtaaggaaaccgaatcgctgttaacgccagcccggtattcgctgctcatcacaacttgatcagccggtgaaattgccaggatggtgatggtcgggtcggttttaatcagatcgcgctcaattttgagaccgtccggtgtctggatgtgtagttgatcgacggcaaagacgcgaccagtgtaaacgtttttctggtcgaggatcttgccggggtggtgccatgttttgaacaaacaattatctccttttgatgacttttctttcatatcggtcaggaaggctgatgtgaaaagccgattcattacagcaattattttatcatcatttagacgcccatcaaggctgaaggagcactcaacttgtcatcttaatcccaacaatgcttaccagcagcagaatcacaaaaccccaagtaatcggagaaatcttgtcgccaaacagaataatgccggcgatcactgttccaacggctccaatccctgtccatactggataggcaatgctcagcggtaatgttttcgtggcatgtgctaacaggaagaaactgatcagcatgccgacaatggtgacaatcgatggcatcaagttggtaaacccgtggctatatttcatcgccgttgcccaaaccacctcaaagatgcctgctataatcaaaaatacccaattcataaaaatcctcctaaagaaaaagggtacccctcacaattccttctatgacctaacggaattgtaaaaagtacctaaagttgctgcccggtggcagtcgaatatcaagttgttattagtgtagcacatttgaaatcgaaagggaatttacttctttatgccaaacttctcttccaatgctttcgttagtaactgggaaaagtttaggtttgattcaattcctttttcattcaaataatttggaatgttgacggttttcttgacaggatgggaatcatgttggcgacgataagcactgatattcacatctaccaaagtggccaattcatttggcttagtgtctggaagactataaactgattttggcacagaacctccgtcttcaatcagatctaatacttttagaccaataaaatctcggcccatttcaatggagttttcaatggatgtaccttgtgtatatccgcctaaatttggaatactaacaatatacggaaccgatttatcattgggatcttttataataatgattggatagactactttgacatctttcataatgacctccaaatattgatttaacgtaattgatgtttccttattagatctcgagcaagccattcattaatatttggatgccgtggaataacttccttttctttaccgtttgtccaaatatcatgatttccaccatggcgatataaataccaaccatgccgttcgaagagctgcaacaaacgcttccgcttcatcgaagataatcctcaactttctgtatattttatacgtgcattgtacgtagatcaagtaatttgtatttcctcaaagcacttttttgaaggtgacaaattcgatgacttacataattaattacgtataaatacaagaaaggattttaaaacaaaaaatggatgacatccgccatccacaaaattcaacaattcaactacttttgcagcacccggaccctaaacaccgcgtcaatcttcgaaagacggtcaaccaattggtgttcttcctcgttgttcaagttatccaggtcaacaatcgtgtaggcgacgtcttttctggccgcgttgctcatactttcaatgttgatgcccgcatctgccaacagggtggcgatttggccgaccatgttggggatgtttttatggatcaacgttaagcggtaaggggtgttaaacggcacttggaggttggggagattcacggaattttcaatgtttccagtctccaaatatgtcatgatcgtattagctccctgagtggcgccgttggcttcagcttcgagtgtcgatccgccgatatgtggagtgaccaccacatcgtctcggttcaacaggatattttcaccaaagtcggtatagtatgtccgaattttgcgcgcgtccagatagtccacggccgcctcgttgtcgacgatcccgtcgcgagaatagttaaatagtttgacgccatccttcataatggccatttgttcagggccgatcagtccggtcgtctcttcattcttcgggacatggacggtgacataatcggcttgctgaagggcttctcccagcgtggttgcccgagtgatggttgtcgaaatgtgccaagcggcatcggctgacagatatggatcgtaaccaatcactttcatccccaaagcgctggcggcattggcaaccagggagccgacgtggccaaccccgatcactgccaaggttcggccggtcaattcggttcctttgaacttggtcttgtctttttcagttcgcagcgaaatgtccgcgccactattgtgggcagcgtaatcggctgcagcaaacaagtttcgagatgaggccaccagtaacgcgatgatcagttctttaacggcgttggcgttgctgccgggggtgttgaagactgcggttccgttggcagttgccttgtccaatggaatgttgttaaacccagcgccggctctggcgatcacctttaatttcttgggaaagtcctgatcatgaaggttaaccgatcgaatcagataggcatccgcatcatcagttttgttaatttggtagttgtcggagaagcggtctaatccagcttgtgcaattgcattgtaagtttttacttgatacatatgagttccccctaatgttgtttttcaaagttgtgtaagaaatcaaccagtgcctggacgcctgccagcggcatcgcgttatacagacttgctcgcagaccaccaacacttcggtgacccttgagattcatcaaaccggcttccgtggctgctgtaatcgcctgggtatctagatcggcatcaccagtggtaaatggaatgttggtcaacgaacggtcagagaccttgatgtggttggcaaataattttgagtcgtctaagaagtcgtagagcagggatgccttttgccggtttaccttctcaatttcagcaattccaccttgatccttcagccatttcaataccaatccggtggcataaatgttgaaaaccggtggggtattatacatcgagttctttttgacgaataaattgtaattgagaatgcttggaatatggtcgactgtctgaaccagatcatctcggacgatgaccaaggtcaccccggctgggccgagattcttttggacgccgccgaagattaagccaaagtcattgacgttgtattgttctgccatgaaattggaagataaatcaccaaccaaggtcacatcgccgtgttcgggcagctgatgataagcggtgccttcaatggtgttattcgtcgtgatgtgtaaataatcataatcattggcggagattcgctggttcagttgtggcagtgcttgataatgctgatctttggttgaagccaacacattaacttggtagccgaggttagctgcttcatcaccagcccgggtagcccaatgaccactgtccagtaaggcaatcttcttgtgcttggttgccaggttcatcggaacggcggcaaattgacccgtgccacctccttgaaagaagaggatgtgatagttatcgggaacgtccatcaagtctctgacatcctgttctgctgcattgataatgtcgtcaaacattttggaacgatgggaaatttccataatactcattccactgccgttgattgatggcagttcagcttgaatctgtttgataaccggatcaggaagcgttgccggacccgccgcaaaattgtataccgtcatgaccaaaaactcctttatataaaattaaaaagctcccacaggtttgctgtgagagcttctaactgacgtttttagcggtctcacagtgatgaaaaagatttcatctatgcaaggccttttgttgaatcgcacgtatcaaaagatggcctacatagatgtgactgtagaccaggaggatgatgtagttgtcgttaaatcagctaattgcatgttcatgtgaacaacctccatttcttataactaaaatctaacagaactcacagataaaagcaacacccattttgaagaaagtgtcacggaactgtttgcatgtgcttgaagatcatggtaaattcaatggataattaatttattgggaggaacgcgcatgactgatttttactttgttcgccatggccagacggctgccaacgccgccggattaaagcagggcaccattaactctgaaattacctacctatcagaaaccggaaagcaacaggtggaaagtttgcggaaaggtttcgatatttcgtttgcggatagaatcattgtcagcccactgcagcggacaaaagacacggcggccattttaaatcagagcgcgaacttaccggtaacctatgacaaacgactcctcgaaatttcatatggcgactgggatggtgagaagaacgctgatttgatgagcaaatatcccaaactttttgacttcactctaaatgacgttcttcctgcctacgcagatgtggcacatggtgaaactttcgatcacgtcatcgatcgcgtcgctgaattgatgcaggaaactgcaactaattatcctaatgacaagattatcctggtcactcacgggtttacgatcaaagcggctgtgttggcagccatcggtcgtcccaaggacatgatggtgattgaggagccggataacaccagtgtgacccggatcactttacagaccacaacccactcgtattatctgcggtattacaaccgggttgtcaattctcagttttaaagtgattgacaaatgaaagtcaattggttatattaaatggcatcaagtaacgaaagaggaggaagccattcatgcaaatgtcagctgctaatatgatgtgttgttcaatgtgtcaagctcaacttagcgctgatcgtggcttctttggtaaacgattggatttttgggacaagctgtgagctgatagttgacggcccattttctcaagaattaccaatgccaagagtgtctcatttcagcgtcaaagctggagtggggcactctttttgtataccagaggatctcttttgttgaataaataatcttaaaggtggcggttgcagtgtgtagtcagatgttgattgaagtgaaaaggacaaactaaattctttggaggaatcattcatgcgaaaactcagatcacttttattattagccttgagtgccattctggtagtgactttggcggcttgtggcaaaaccgcaaccaaatccaacagtcaaaaacagacattgaatctcagcacgacggccccgttggatacgatcgacatttcaaaatccaccgggtatggccagaccgggaacgtgtttgaaagcttttatcgcttggggaaagacggcaaaccaactgctggcttggctaagagcggtaaggtttccaaagatggtaagacgtggacctttaccttgcgcaacgctaaatggagcaatggcgacccaatcactgcccaggattttgtctactcgtggcgccgaaccctgaaaccaagcaccaaatcgacttacgcctatttattcagcggaattaaaaacgccgatcaggttaacgccggcaagctctcaccaaacaaaatcggtatcaaagcactgaataacaagacggttcaaatccaacttgagaaaccgattgcttacttcaaggtcctgatggcctatccattatttggaccgcaaaaccagaaaattgttgataaatacggcaaaaaatatggtaccaactccaagtacatggtgtactccggaccattcaaaattcaaaactggaacggcaccggcaataagtggcagttcgttaagaataaccgttactgggataaacaggccgttaagctccacaagattaactataccgtggtcagcagcccgacgactggccttgagttgtatcagcaaaacaagctggatttgacgccgctttctaatgaacaagtgaaacattacaaaggcaacaaggaatttcagcagtatccatattcattcatcggttacttgaagtacaacttcaaagacgccaaccaaaccaaacgcaaagccatgagcaacaaggacattcgtctcgcaatttcactagccattgatcgccaacagctgaccaaaaaggttcttggtgatgggtcagacacaccaactggctttgtggcctccggattggctaagaatccgaagactggcgaagactttgccaaagaacagactgttccaaatacggtggattacaacgtcaagttagccaagcagcattggcagaaaggtttgaaagcccttggtaccaagaaggttaacctgacaatcactgcttccaacgatgatccaaccagcaacccgattacacagtacatgaagtctgaattgcagcgggacttgcctggatttaagctcgatattcgaaatgtgccgagccaagttgccaatcaagaagtcttaaagggtgactttgacctgtcattatcgggttggggtgcagatttcaacgatccaatttccttcctgcagatcccggaaaccggcaccgcatacaacagcggcaagtacagcaacccggcatatgataagctgattaaacaagctcaaaatcaggatgccaataacgctgacaaacgctgggatgatttggttaaggcagctaaattgtttaatgctgatcaggggatgacgccactgtaccagcaagtcacctcgtatctgcaaaagcccgacttaaagggtgttattcataacactgccggtactcagtggagttacaagtacgcctatatgaagtaaacagccaaggtctaatgcctgcggccactcgttgtcatctcattaacttaaattaaaatgagaatccattgaccattgagagcgatatcatggtacacttttctcaactaaaacttttgaggtgattaaggatgacaagaaaaattggtgttatcggaatgggacatgttggctcaacagcagcgcattacattgtcgcaaacggcttcgcggatgatttggtattgatcgatatcaatgaagataaagtgaaggctgacgcaattgattttgaagatgcaatgtccaacctgcccgtccacaccaacattactgtaaatgattattctgcactgaaggatgccgatgtcattatttctgcattgggaaatatcaaactttaggacaatccgaatgacgatcggtttgccgagctgccattcaccagcaaggcagtcaaatcggtggcacaaaagattaaagactccggcttcaatgggatcattgtcgccattaccaatccggtggatgtcatcacttcgatttaccagcaaattaccggtctaccgaagaaacacgtgattggcactgggactttgctggattcctcacgaatgaagcgggcggtggctgacgaacttaatttggatccacggtcagttaccggatttaatttgggtgaacatgggaactcccaattcactgcctggtcaaccgttcgggtactgagtcatccaattaccgagattgctaaagaacgcggcttggaccttgatgcgctggacaaagctgccagagaaggcgggttcaacgtcttccacggtaaaaagtacaccaactatggtgtcgccaccgcggctgttcgtttagccaacacggtgatgagcgatgcccacactgaactggcagtttccaactaccgtgaagaactcggcacctacttgtcatacccagcggttgtcggtcgtgatggcatcattgaacaggttcaactgaagttgactgacgacgaaaagaagaagctgcagatttcagctgattatattaagacgaagtttaaggaatcaatggaaaactagaacagattgggactaaaggcgctttgatcccggccatataacgcaatcgggccgtcattccggaatttggaatgacggcccgattgcgttatatggccgggatcagccgtttgtaccaagttttatcattataaaattggtgattgtagttgcaatgaaaatcaccgtaacgattagtggtccaacctctgttttgggacaaaaaaataacctccagcaattaagaactgaaggctttaagcaatttatctaactcgaattgttaatatacttgtattataacgcgacgaattcgatttgtcaacgttgcctgcaaaagatattcgagtttaactggctggcagattcagcctaaaattaagccaataaatcacgattggagcaatcaattttggcaaactacgaagcagtgtttcatccagacggttacaattctcctgagtaccgcagcttaaattattcctatcagaataaaatggccgaattattctcccaccgacggattgattatccggccaaagaacttcaatttgaaattgaaaccgtcaaaatctccagtaccatgactcagcggcaatacctcaaacttcagagcttggtggaatcatttcctgaaactcaacgcagtggagctgcccccgtcattggcaaggacgattaccagagtattattttgtatcatgactaccgattatttgattcgacccagtatgttgtccgcagtccggtgggatttggctataccgtcagcaagttgatcacgattacgagtgagccagcgggaggtcctcatcaccaggtgaaggtgacgttggcaattaacccgaatcgtttcgttgacgttcccgaagaacctttgcttcgcctggtcatcgaagaggtgttgccgctgatggtaaccccacagatttctgaaatggatttaacgttagatatgccgctaatcatgaacaactttcatgttcagatgggtggccaagctgggacaaaacagcagattacccaacggcttaatgatcatcaagaatatgaattgagccgaattgcctatgtggatcctcagcagacccgaaaactgatcttggcagacaagtttcaatccctgttggacaatcaattgctggtggcggatactgactacatttctgcgcgggaggccgaatactatcgggaccaagttggagaacggcagtttttaacccggattgaattggcggtcaccacccctaatgccgtcatgcggtacatgaagaatcacgagtggctgatgcgggacatttccatcgagtatcgtgataatagcggcatctcaagatttgcgggtaccgattacgcgaccaacgggaaggacttccgccgctcatttaaccggatgctgacgtatcggctgaaggaagttcagcgacgagcacgcaaactgccatatctgactgatgcgatttggcggaataccctgaaatagaatttgaataaatctcattaaatgaaaattcgctgttgaactgacatctcaaagtggtatgctgttaccattaaaaatttttgaggtgattgaatgacaagaaaaattggtgttattggaatgggaagtgtgggctctacggtcgctcactatatcgtgtccggcggctttgcagacgacttggtactgatcgatataaatgagaaaaaggttaaagccgacgccttagacttcggagatgccatggccaacttaccgaatcatacgaacatcgccgtgaacgattatgatgaattggccgacgccgatatcgtgatttctgcgattggcaaactccagctgcaacgcgacaatcccagcaatgatcgcttcattgagtatccatatactcaaaaagcagccgcatcagttgccggtaagatcaaggattcaggctttaatgggattttaattgtgattaccaacccggttgacgcgatcacgtcaatttatcaggcggtcactggtttgcccaagaagcatgtcattggaaccgggacgttgttggattcgtcatggatgaaacgggctgttgccaagaaattacatatcgatccgcgttccgttgccggttataatttgggggaacacgggaattctcagttcaccgcttggtcaaccgtgcgggtcttaggcaaaccaattactgaattggctgacaaagaaggccttgaccttgataaaattgatgaagatgcccgaatgggtggcttcgtcgttttccgtggtaaaggatacaccaactacgcgattgccagtgctgccgttcgcctggccaacgttgtgttaaatgatgcgcgaactgaactgccggtatccaattatcgtgaagaactcggttcatatttgtcatacccagccattgttggtcgggatggcattatccaacaactccaacttgacttaacagatgaagaattagcgaaactgcaaaattgtgccaatatcattaaagagaagttcgaagaatcaagagccaaggactttgcggctgaatagggacttttcacatagaacaattttcatccacattcatatttgaggatcgtcacgcctcatagtaatggccaggtcaaaatcagcaacttttgacctggctttttgtatcccaggaggtcactggattaccaattcatgatttttagcgctcttttacatgtttctcccacttttggtatatattaagattaatcgagggggaaaaatgacgaaaaaagaacgggtggaagcttttacggatgccgttttggcaattattttgacgattatgattttggagttcaagaccccggaatcgtttgcgattagtgacattttagatcaagtgccatacctgatttcctacgcaattgggtatttgttcatcggcgttgcctggtacaatcaccattacatgttcgccaagaccaattggatcacgcaaaatgtgtattgggcgaacaacttgtggatgtttaccacgtcctttgtccctgtggcgacggcttgggtcgggcgcgggttaaatgaacaggggccggaaatcttttacttcgttgtctttttagcatggtcgagtgcttattattatctgtccaaccgattaatcaaggccaacgaaaaagaccaccgaccgaaggcggcggaggcgattcgatcgatggtgatttatcgatatatgagtaattggaaactggtgggcgggcaactcattttgtcagttattgttttaaaattcatgccggcgcttcaaatggtcattgtcacgttaatgattatttttatcggtgcccggtttaacgcggacagcgatcggctctttcgctagtgggcaatcagggtgtagatgaagtagccgagaaagccgacgcacaagctgagtgagccaaaaatcatgatctgaacagaacagacaaaagtcttggttttaatttgttcatggttgaaaatcagggactgcttgatgatcagtggaactgccagtagaatcgagaacagtgccaatgggaagacgccaacgtacatggcgtaaaacaccagcggaaccgctaaaacgttggcggtattgaacattagcagggaattcttcttgccgatgtagtggacgatggtccaacggtggttgacctcgtcttcttgatcatcgcaaatgttattggctaacataatgttggcaatccagaagaacaacggtgacgaagccagcagaatctggccaagcagcgaggcattccaagtgaagagctgataggaattaacgtagaccgagatcagggtaatcatgatccccatagcgaagccggatgccacttcaccatacggcgtgctggagatgggatgtggaccggatgaatacataattccgatggcaaaacagatcaatcccatccacaacagcggcaggccgactttgaataccaggaaaataccaatcaaagctgatggcacaaccataatgacgatcataaaacgaatgaggtttaaagagatgtggtcccgaccgatgatgttggtaccggttttccattcctcagcggttgaatgcatgtagtcgttatagttgtccaaggtgtccacggtcatattgaacagaatcatggcaatgaaaaaaagcgtagcgtaaagcccattcaccgagtcgagcaggtaccagctgaaaaacagtccggtaaaaaacggaaagatgctggcagctttggctcgcaactcgacgagctgggaaaaagttgataaactcatgatgacctccaagataaatttaaaataatttcaaaaacatagtctaattataccaaaggagcgggaaaatgacgctgacgaacaagacgccggaaacaaaagttgaatcattatttgatcaaattgcggacaactatgatgggatgaactcgctgattagtttggggaatcataagcactggcgaaagttggtcatgcagcagctcaacgttgaaccggggagctttgcgattgatgtttgctgcgggaccggggattggacaattgctttggccaaggcagtcgggccctccggacaagttgttggcctcgactttagtgaagagatgctgaaacttgctgacaagaaggttcgtgcagccggcctgcaggatcgggtaaccttggttaaaggggatgcgatgcagctgccatatgatgacaaccactttgacatcgccacgattggcttcggtctcagaaatgttccggatgctgaccaggtgctccatgaaatgagccgggtggtgcacgcccgggggcaggttgcctgcctggaaacgtccaagccaaccaatccggttatcaaattcggctggcgggtttactttgatttggtcccattaatggcaaaagtggccgtcaataaatatcaggagtacgcctatttacaaaaaaccactgccgaatttgtctcggcgcaacagttggtggaaatgtttcaaaacgccggcctggttgacgttcactatcgtccattcacttttggggccgctgcttttcactggggaatgaagccctgacaaaatttcccttgattcacaagattaaaaacgttatcatgtgtttaacatattctaaggagtttttaattatgacagataatttaaacatccaaatgaatagttgccgatattacttttggtttttccgagtgtgatctgtggataagccaaaagcatttcgtaatgcatactaaaggccgcacagatcactgagttgactgtgcgggattataccattggtgggtcctcacagtcagttcgttgactttgaggacccactttttaggaggagaacacaatgagtaaattatcagataagatgaacaaacgagtagctgcgttaacgcctgccgcaattttgactttcaaccagaagatttcagcgattccagacatcgtcaaattaaccttgggtgagcctgatttcaacactccggaacacgttaagcaggccgctattaaggcaattgacgataacgaaagtcactacaccaactcccgggggacagaaggactccgtcaggcagctgcgaacttcttgaacacgaaatacggtctgaattacgatcctgacaaacaagttatcatgactgaaggggcaactggcgccatctactcggcattgactgccatgatcaaccctggcgacaccgtgatcgtcccaacaccaattttcccactctacgtgccgatcttaatgctggccggtgccaaaccaatttttgtggacacctcggataatggctttgtgctgtcaccggaaaaattgtctgcagcgattgaggctaataaagatactgttaaagcggtgatcctcaatttccctaacaacccgaccggggttacctaccacaaagacgatttacagaagttggcggacgtcatttccaagcacgacattatttgtttaagtgatgaaatttacagtgagttgacctatgacggcacccacgtttcgatggggtcgatcctgccggaacaaacccttgtcatgaacggtgtttccaagtctcacgccatgactggctggagagtcgggatgatctgtgggcccgaagatatcatcaatgaaatcgccaaggtcagtgaatttacgatcacgtcactgaccaccaacgcccaggctgccgccgaagaagcattcaagaacggtatggacgatgccctgccaatgaagaaggagtacatgaagcgccgcgacttgctagttgctggtttggaaaaagccggcttcagctgtcctaatccaaatggcgccttctatgttttcgccaaaattccagctggtttaaaccagaatagtgaagcattctgttatgacttggccaaggaagccaaagttgccttaattccaggttcgtacttcctgccaggcggcgaaggctacgtccgaatcagttacgcagtcagcgaggaaaatattcaagaggccgttagccgcattcaaaaatacgttgaaaaacagtcagtcaaataaagggagcttgagttattttgaaaattttaatgtacaatgttcgaccagacgaacaaaaaccactggatggctgggttaagcaaaacggtgtccaggtagataccaactcggtaccgttaaacgctgaaacagttgaccttgccaaaggttacgacggcattgtgattcagcagcacggaccagtctcagatccgacaatttacgagaaactccatttatttgggatcaagcagattaccttgcggatcaccgggtatgaaatcattgatttggaccaggctaagcaaaacgacttggtcgttaccaacgtgccggcctactcaccacggtctgtcagcgaactggtcttggccgatgtcatgagcctgcttcgacacatcggtgaagtgggtgaacgcgaaaagcacggcgacttcagctggaagggtgtcgaagcacgtgaaattcatactttaacggttggcattattggtgccggcaaaatcggcagcgcggttgcccgaatttttagagcgctgggtgccacggtgattgccgctgatccgattcatcgaccagaactcaacgacacgttgacatacgttgatcacgaaacggtcttcaaaacagctgatatcgtgaccatgcataccccattgactgacgagaccaaccagatgattaacgccgacgtcttcaagaagatgaagccctccgcaatttttatcaatgcttcccggggccaagtggtggataccggcgcttgggtgaacgccttggaggaccaggaaatttccgccgccgcaattgatacctttgaaggcgagaatacgattgtcggccaagacttaaccggcaaaccaattgataacgataatttaaagaagttactggcaatgcccaacgtcaacgtgacgccacacattggtttctataccgaagtggccgtccaaaatatggttgagattgctttgaatgacgttatgatgattttgaatgggcaaaagagccctcatgaggtaggcgaatagatgaatttaacagcagaaccatcagcacggctgaacggtcgtgagctcattatgaatacgttaaacgggctgtcggttgggatcattgttgcactggtccccggcgccttgcttaatcaattgttgaaggctttgctgccagtatttccacaagctgctttcttcttgactttgactggaatggcggccgttttaatggcaccgattagtgcggtctgtgtcgggatgatggcgggctttggctttgccggcttgatcgggccaatcgctgcagttaatggttatggcaatgccaatctgatgaatattgtcttggttagcttacttttcttggtgattccggttacgcttggatatgttagcaattacttattcaactccaagctgagttattttgacgcccaagattttgagttggattattcataaggagtcgagaatttgggaactgaatttgccgtgctagtcctattaatctttgttggcggtgcgatttactactattacttcagtaaacaagagccttcaatgattgtggggtatcggacaaaacaaagtcgcagcacaacggcaaagtggcgggcctcacagaagtggttctaccaaggggcaatcacttgtgccgcggttgttgtggtggttaatctggtaacgccattttcgattggtgtgaatttggttgttttgtggtagattgcaaatttaatccgaatttttggacaaatttgtcagcataacttgatacggtgtttgccagtcgagtattttaagcggtcgctggttaatttggagtaacgtcgtcgttaaatcttgagcactaatgtgctcaaaacgagtccctttaggataaaaataacgtaaattccgattaaagcgttcattactaccacgttcagctggagtataagcatggcagtaataggtcttaataccatattgtgattcaagtgatactagcccactaaactcagtgccacggtccacagtaaagctgtgcaccggaccattaaaagtggttaggaacttagttagtgcttcattaacagtcgctgtcgtccgatcttttaaccggtatgcccaaaggaaccgtgattttcgatcgattaaagttaataaaactgccttactatgcccacgaggaccaacgactgtatctagttcaaaatcgccgatgcgcttacgttgattaatcatcatgggacgctgttcaattgatcgccccaaagattgattatatttggatcgttggtcaacgttacgccgttggcgtacgccatgttcaggtagatcattcaaggagaaaccaattctcccctgatttagccaattataaatagatttagtagctagtttaaattcgtgagcaatcattcctggtgaccagcttagacgtaaatggttgagaattttttgctttaactcatcgctcagcttagttttccgaccacatcgtgatcgcttgtattcggcatctgtttgtgctaattcagcccgataaggttgacatcgagataattcataagaaattgttgacggtgatcggttcagccgaacgcccatttggatattggacagccctagttcacaaaaggtttcgattttaattcgttcggaataggttatactagacaaaagatcagctcctaaaagatgggtttgtggtaaacaccattttaaaggaagctgatcttttttgtccgaacagcgttcggattaattttacaatctaccttgttagtttatttatttgtgattagttatttcatcgagcgtcgcttgcgtgagatgggagattagaatgaaaaaggcccgctgagttggcgggcttttttgtgttttagttatttgtttgttggggttagtggttttagttggggggatttgttgttttggtgattcccttttatctagcggaaacgtgctccgatgaccctgacccctaaaatgtaaaacaaggattgtatcgatgaacaaatgcgttcatcaatacaatccttgttttacataccggggtcaacccgggtctcgtcgcactctaaatttggccccaagcatccgccgcaatcgttgggaacaatgtgaccaaacgttccagctgtgccggttcgaacttgaacacaattgctggcaataatgcgttaatagcatcttctgcttggtcgctgatttcagtggcaccaaccaaatggttctgcttgtcataaaccagtgtgttatcgccaatttcttccttggtcacttgacggtaccagtcgtctggtaaatggttctcctttgttgtgaagccttcttttttggcatcctcaactgatacgccgactttagcaattcttggtgaggtaaagacgactgatggaattgccgggtaattgatgggatccgtcgtgtcgccagcgaaagtatgcatcaagtaggtcgactcaaagatcgccgttggggtgagctttggttgatccttgtcgatgacatcgcctgaagcgtagatgttatcaacgttggtctggagatggtcgttgaccttaatacctttttcgctatagtcaacaccaactttatccagtccaatgtcgtccacattaggcatccggccagtcgcgtccaagatccagttggtctttatttgaccgcccttatagttgacgatgaagttatggtcgtcctgctcgaagttggcaacttcagtattattgacaaaatcgacgccacgagatttcaaatcggcaacaatttgcttaacgtatggttgatagaatttccgcaaaactttgtcgccgtgggtaatcacagttaccttggcaccagccgcgttggcaatcgttgcgaattccagactgatgtagccggcaccgataattgtgatgttggctggcaggtgagtgaggttcatgaagtcagcactatcgtgagccaattccgttccgggaatgtccaaacgatgtggatgttggccggttgagatgacgatgttttcagcggttttggcttcaccgtcgaccattaccgtatgagcatcttggaatgtgccgtggcccttgataatgtcgatgttaacggatttcatcaagccgccgatcatgtccggcaagccttcgatgacttcttgcttatgtttttcattggcggtccagttaattgccaaactgccattgagaatcccctggagtctctcagtttgacgtgtcaaagctactggtgcatccaacgtaatcttggcgttacagccacgattgggacaggtgccgccaattaagccggattcgatgacgccgactttcttgccgcgggcggccagcggaatcgcaccgtcaaaggttccatgtccactaccgatgtataagacgtcataatcataatttgccataaaaaatgcctcccatatagtctgctcggaaacgattacatcttgaactactaaaagcgtaacctgtaaacaaattgcgtgcaacgaattggtttaaaaatttacggacagtcaaaaatgtctatatacgacgttgcccaaaatggctatacttgaagcaaataaagggagctgatggtatgcgcagaaaagatcgggaagttacagatattgacgaaattaagcaaattttgcaggattcccatgtgattcacagcggttttcggacggctgattatccgtatgtggtccccactaattttggctacgaatttgacgatgatgaccatttgacgttatatattcacggcgcaccggtaggccgcaaacgtgagttgattaaggaagatggccggatgggctttgagattgatgatggcggccaattaatggtgcccaaagatcccaagcaaaacaccccgagcttcgcttatcgcagcgtgatgggctatggggatgccgaattggttgatgatccagcagtcaaaaggcacgccctgcaagttgtcttggcgcatgagactgggcagcagttgagtgaatttacggttccagataagacgatcgcctacgttggtattatcaagatcactgttaaagaattcaccgccaaagcccacggtggcgatgatccggattttgaataggcgtgcgacgaggctggtagcagcggaaataaaataatagcagaacactaaaaagccggagcacaactaacaagtagtggctctacaatatctgttgttggtaatagatttttatctattactgatgacagattttttgtttttcattagaataaaaaaagcggacatttcctgtccgttcatcaaaaccaacaaccacgaagattttagagaaagaaggaaatgccctatgtcaaatgatactacgaaaatgttgttaggaatagatgatgaacacttaaaaattgagaatggcaaaataggtgatgatggggtaatcagattaaatggatcactgaactattctcccaaggcctgccgcaattgtggggttattaatgatcaccagatcattggctatggttggcggaagaccaccattagattcgctaaaatattgggcagcacggttatcctatgcctcaatcggcgaaactttcactgtaaggcttgtcataccaacttcctggcgcagacgagtgcagtgccgaagcactgcacgatttcaaatacaacccggaaacaatgtttagagaagttaacggaaccagtgagcctcaaacacattgccaatgaattgtccacttcggattcattcgttggtcggcagctcttgcgcgctgaacacgactttcaaaccaactggcactacttacccaaagttctcctcatggacgaagttaaaagtactaagagcgccaccgacgcgatgagctttgaatttatggacgcggaaacccacgaattgattgacctgttgccctttagaaccatctatcagcttcaaaagtacttccaacattatgaccaagccgcgcgagaaaatgtgaaaattatcgtcaccgatatgaactatacctatcccaaattggttgggcagatcttcccgaacgccatcgttgtcatcgatcccttccacctggttaacgctttaaaccgggcttttaataagacgcgagtgcgtctcatgaaaaccctggccacttcctcacgccagtatcacgccttgaaacgctattggaaactattattaacgccggccaatcaccttaactacgaggctttccgtaagtggacaaacttcccttatccggcaactgccacggatgtggttgatgctttactggacattgatcccgagctcaagcaaacttacgacgtgatgaatcggttacgtgaaaccatcaaaaaccgcgactggcccaactataatcaagcctttcaccacctgcaggggtgctcggaagagatgttggcagccctccaaaccttggcggctcatcatgatgaaattggcaacactttcacccaccactacaccaacgggccattagaaggttcaaacaacaagattaaagtcattaagcgcactggatttggttaccgaaacttcttcagattccggctaagagtgctgttcgcttttcgagttcatacaaaaagagccctaatcaccaagtgattagaactccaatattttgttcaccaacaacagttgacgaagaacccaagtagttgtgttccggtcatttatttttcacggtgatcgtgtttttgagcctcatgtttccaaaaccatccgggaatcgaaatcaatattcccatcccaaatggaatcaagctgtaaatcaatgccccagtagaatgatcgccactccaccacatgaagtagcatatcccaaggatagagacgatcaaacccgccaatggcactgtgactatgaggtattgaatcattcggtcgcgaagctgctgcatactcatttggattacctccttttaattttagattaacactaaccagtcacaaaacgggttacgaagtccgagtcaaataatgattccgggtgacgatgtaatcaattacgcctgcgatcaaaagcgtgaccagacaacagccaacaaatcccatcagtgtaaaatcgccgttaatttgaattggtgtaaaggggctgttttcatgaaacagtttggaatagagcagcaccgcgttttgtttgaagtcaaatgatcctaatacagggatgccggaaaagtacccaaacatcaaaatacctgccagccaaggtcgcttgagcaataaggtgaggtagtagctgacgatcacggcgatcaatgataagccaaataccgataagaactgcaacggggcttgtgccaaataagattggccgtccgcgagatacctgatcaacgccagtttatttgggatgtggataaaattgttaaagcctaattgaaagatgaaagaggtcagacaaatgaagatcaggctcaaaaaagtgagcatgctcaaactaatcagtttggagaggacgacattttgaatgctgttcatgctggccttgattctgacctgattatttttgagttcccgataggcaaaagaaattgtgtagatcaccatggtaattggaaagacaatgaacattgacgatcccagaatatgatcaaagctgtttctgggggccatctcgaccagatcctgcttgaccttttctccagcatcctggagactagtgaccacttcggctttttccccgttgctaaacgtgattgggccaccggctaatatttgatcaacgtcaaccccagcgcgtttatcacgctgctggatccgaatcagactactggcgtcatttttgtaagcagtgtattgcgcccaagatatggagaaacagagaattgtcaaaacaaataacactaaatagatcgcatcagaatggagctgttgatccagttctttttgggttagggatctgagctttttcaattgcgcacgtcaattcccttcggtgaatgatgaatgtggtaaacaataacttcagcataggcattttggctagtgaagacaacggcaaaccgggaatgttcagacttatttcacacaaaattcaataatttaccaatggcatatacattcagcaactttcgttctatcataatggtaacggttccagaactagcaattatgaaagaaggatcttgtatgttctttattgatacgtctagaaatggcaaacctgtctatgatccgattgtgaaccaatctttggataactacttagtaaatgatttgaagttgccgggccacggcctgattatgtacgttaaccaacccgctgtgattgtcggggttaaccaaaatgcctatgccgaagtcaacatgccctatttgaaagaaaagggcattaagttggttcgccggacatccggtggtggcgccgtgtatcacgattacggcaacattatttttgaaaatattgtgattaatgatgaccaacattttggtgattttaaatacttcgcccaaccaatcatcgatgccctgcacgacatgggcgctaccgatgctgaaatgcgtgggagaaatgatatggtgatcggaaatcaaaagttctccgggatgacgatgttcaaagttggcaagtcctacgctgccggcggcaccctgatgtttgatttggatatggatgtggccactgaagttttgaccccggaaaaggataaattggaatccaagggcgttaagtcggttgaaagccgggtaaccaacgttaagccattcttgaagccggaatttcaaaagttggatattgaaggcttcaagaaggccctgctgctgagattgtttaatgccaagtcattggacgatattgaaacctatcatttgaacgatcacgattggtcaattattgatgagcgtttgaaagggaaataagataccgacgagtggaactacgggaagaatcccggctttgattactatgtttccaaacattatgatatcggcacggtcagcttcaactattcattgaacggcaaccaaatttccgatatcaagatctatggtgactttattaccggcggcgatatttccgtgattgaaaaggcactgaaaggcgttgatctcaacaaggatgcgttagtcgatgctttgggtcaagtggatattaaggctaatttgggtgacatttctgccgcggagttggcggacttgctgctggagaagacgcggattaattagatatctgctttgttttggagttctagttttgagctagggctcttttttattgatttgatcgttgtcggaacgacttgttaccggcatatgtcagcttgcaagctaatccgttgaccttacccgaccattcgtggaataatataacgtcataagtaatgcgacaagttaccggggggtgaacacatgaatcaagcaccaaatcagcatgacgacagcggggaacagaacggtgtgagcatgatggggatgttcagatttgtttttggtacggttctcaaacggccatggattttgattgtcaacgttgtcgttttgaccattctgtcattgatggactttttattgccacaattcaatcagtacatcattgaccacgtcattccaaataagagcacggcacagctggccgtggtcgtcggtctgctactgttgaccgttacgatttcagggatttttacctacgtttctacctattacatgggcgtcatgagccaaggggccatcaccaacctgcgaaatcagctgtatcaatatttgatcaggttggatacccacttttttgaatccagtaaaacaggtgatttgatggtgcgattaacgtccgatattaacaacctgcaaaacctgatttcaccaaacatgctgtccctgattggcagcctgttcacgtttgttggggtgctaggcttcattttcttcgttaactgggaaatggctttggcagtcagcttgacatttccaatgatttttatggtggtccgcattttcagaacccgaattcgaaattcatatcaaaaggctcgtcaatctcaagccttgatgaccaatcaattgcagaacacactgactcaaatccagttgattaagagctacaccactgaagatctggaatccagtcgtttcgacaaattagccaacatgaacaaaaataacatcattgaggctactcggaatcaggcgatcttttcgccgttggtgaccttcattgagtatctggggaccgcgattgtcttattcttgggaacattgtttgtttttaaaaatcagttaaccgttgggcaattggtcgcttatctcagctatgttggtatcctgcaaagcccaatcagtgccttttccagattgttgaaccaattccagcagtcactggtttcttatggccgaattgtcagtatcatgggcttgaagccggcgatcgttgacgaggacgatgctgttggattcccacagattaagtctggagttcaatttaagcatgtcactttttcatacgcatctgatgagccccagtcaccgcacaaagccgcgattcagaatgtgaccttcgatattccgtttggtaaacaaaccgccttggttggtcactcgggagccggcaaatcaacgattaccgatttgctcgatcgattgtacgatgtcgatagcggtgacattttgttcgatggcattccaatcaaacatatcaagctcaagtcactgcggcaaaacatcgcgattgtgtcacaggatatcttcatcattgacggcacgattgccgataatatccgttatgggacgcctggtgcgactgaggatcaactgtggaacgtcgccaaattagccgatattgatgccttcattaaaggattgcctgagcaaatgaagacccaagtcggtgagcgaggaatccgattatccggtggtcagaagcagcggacatcactggtgatcgcccatagattgtcgaccatccataacgccgatcagattttggtggtggataatggcaagattgtcgagcggggaacccatgatcagttgatgaatgaaaataagtattataagcagttgtatgaggcgcaatttgaataagagtgcgacgagggctgggtggcccggtttacaagaggactttgcttgaagcccccggttttggggctttaagcaaagtcctcttggaagttagggtcaagcccgtcggagcgtgttttaaaggccgaagggagcacagaataagctaataaacgtgctttgggttcagacctgggagtcgcggtttctaagggcactttgattgaagtccctggttttgggactttaatcaaagtgcccttagaagttagtgcttgggtcgtcggagcatattttaaaggctgaagggagcacataagaagctaacaaacgtgcttttggttccagacccgggagtcgcagtttctaaagaagcccccgacccagcatagacgctgagtcggggacttcttgaatacaatagcgaaagtattggaccagtcaaagctttagcgtgtggttgaacccttctttccgattttaacgatatcctgaaaaggatacgatgtcgagaacatgctcatttatgctagacagttgtgagcataaaaagagaaaaccccgcttcagttttaaaactgactcgggtttttcgtgactccaataacaaaagcaatagacgagctaaagccttagcgaacggtcgaaccgtcctttccttgctaataatatataagaatttcagcctcttgtcaaacattcatcaactattaattagtttggaaaatagttgataaaacttaattagtacaggctcatgagtataataatttgcatgcttgctagcccttttcagtaatttttgcccttcttttctggttaattcctgtgaccctacacttgaaaatcgtctatgtaagaagctgtctaaaatctcttaagtaatagtgctaaaaacgctaaaacgaccatttgcagactggtggttaattgacgctcacaatttttccaaagtcgccgacaattctctagccaactaaaagatcgttcgactacccaacgttggggcatgacttcgaatcgatgcaactcattgcgcttcgcaacctgcacggttgcgtttaaattactggctacatcgagctgaaaattaacgcctgaataaccaccatcaactaagacattttgaacctggcgtaaatgtatggcatgtaaagcgatcattgcactggccccgtctcgatcagagacgttcgctcgcgtcatgtgaatggcctgcggaaagccattgatatcaactgccagatggcgcttaatccccgagattttcttaccagcgtcgtaacctttgttttcagcagtagcggtgtttttgacgctctgagcgtcaacgataataaaggaagttaaagctgaacgtccttggtaagttcgccgagcaatgacaatttttttaaaacttgttccaataaagaatcagccgtaggctcagctttagttgaccaaattttgtaatagttgtaaactgaccgccattctgggaaatcaccggggacttgacgccattggcaaccggttttcaagacatataggaccgcacagaagacctcgtagaggtcatattttcgaggcttagttcgcttacgaaaattttctaaagctggtcgaattaattcaaattgttgccgagtaatattgctgggataatttttcatagcttaaactcgctttttacatagaagtatatcaaaaatcatagatcttggacagcttctaaggaatacaagctaacgaggtcatttactttcatatcggttactaaagatgcatcaattcccatcttcgttgcaaacatgacaaccgttgtatttcgatgttttactttttcttcagcggaaaacagattaaccataatggcattattatgtgctgatgcatttcgaatatgctttgcatacttcaacaatatatgtgcaagcttaacatctttgtttctggagcggtgatagtaaaagtctacaaacctggaaaggacaccaaatgttgcgacttccaaaaacatccagatggagaggtgatttcggtgctttacatacatatcgtgcaagtaatcatttcgctttaagtatttcatagtttgatcataacctcgctgattaaatgtactgaagtccttcaccactgaatagccatcttcttctggatccttggttataagatcaattatccgagttttaattccatgttcaatgtccaatgagattccaagtaagtatcgccgaagttgcatatcgatcgacgccaagtcggttaaatatgcaaaatctaaattttcatatttaccatcaatctgatgaaaattctttcgataggatgtcaacttgaaataataatttttagtcgccagcatttggattgcgtcaggctctgatactaattcgaatctaattcccttgtccttcatgtgtttgatcatttgtggatatgtgtactttggttttatttagttcacctcccagtttattgaaattgtctgatcagcctgtcctactatgtatatacgataaattgagcgaggatatctatatagtttgtgaagtattggggcgatttagtgatcaaatccaaaaccagttttgttttcggacattttagtttacactaatcataaatacagaaaacgggtgacaatcaatgaagacaatttatgattacaaagaaaccgaaatgagcggtaagacgattgacttgagcgaattcaaaaataaagtcgttgtgattgtgaatactgccagcaaatgtggtctggcacctcagttggagggcctggaagaattatataagaaatataagaatgagggcttggtcgtgttaggactgccttccaatcaattccaccaagagttgggaagtgatcaagaggccgatgattattgccggattcattatggtgtcaccttcccgatgactcgacgggttgccgttaatggggatggtgaggatccactgtttacccatctcaaagaagagtccggtcatggcaagattaaatggaactacactaaattcctggttggcaaagacggcaccctgattcatcgatatgcgccaattaccaagccggagtccatggaagaggctatttatacggccctcaatcaaaaaaatgtcttgtaagaaggtggaaagttgaatacgacctatttcaaagccaccattcgagagattacttatgcgtgggggaagtttatttcgatcgtcctaatcattttgttgggatcactgctgtatgtcgggattcgggcgactggtccggatttggacaattctgcggatcagtatttcgctcatcagaatctcggtgacatgagggtgacgtcaaccttgggattaaacaaccgagatctcagcttgatacgcaccgaccccaaggttcagattgccgaacccagccatatggtgacggtgaagaaatcgccgaatcaagtggtccaggtgtattcctatgccaaatcggcaaaattaaatcaactcaaattggtatctgggcatttaccccagaaagccgatcagattgtcttggaccaaaaagctaaggactacaagatcggcgaccgttaccgtttgccggcaaccgatgggctcaccactaaaacttttaaagtggtcggattcgtcaactcaccgttatttgtcagttcaaccgaccgtggcaccaccaacgttggcagcggccaggtgaattattttgcctatgcgccggccgcggcctttaaccagaaagcgtacgcggccattgccgtgcgctttaacaacacggctcatttaacggctgggaccagcaagtacaaccagcaggtggatcacgataaagcccggctggaaagcaaactcaagcaacggccagcccaacggcgctcagagatgatcgacccgcagctaaagaaggttgaccagcaacttggccaacttcagaaatagcgccggaagctgtcggctgtgccaagtgcctatcaaacagcaaccaccaaagcagccactgccaaagtcgctgccggagtcaaacaactgacccgtgccaagcagcaattacagaaggcgccccaagcgacttacctgtacaacgaccgaaccgccaacgtcggctaccaggattattttgatgagtccaaaagtatcgcagccatcgccgtcatttttcccggcttcttcttattcattgccgttttgatcacctttacgaccatttcaagaatgattgaaaagaaccgccgagaaatcggtctcatgcgggcgctgggctacaccaagggcttcatttccatgaaatacgtcatttattcaattcttgcgggaattctgggatcaattgccggcggcgttttgggaaccttgaccctgcccaaatttattttcagcatgctcagcaataacaacctgactcactacgtcggcgtgattccctgggcatttatcgtcgaagcgctcgtggccgggttgatcgccacccttggcagcgcggcagttgttctaatcattaatttacgtgaaaagccgaccgagctgatgcgtgaacgagctccgaaagccggtaaacggattttgctcgagcgaatcaaaccgctgtggaaccggatgaatttcaaccaaaaggtcagttatcggaatctgttcagatataagacccggatgatcatgactatcgttgggattgccggttgtactggcctgatgctggctggatttggcattcgggacagcgtcaacgatctgattcccgatcagttcaatcaagttcagcactaccaggggattgtcacgctatccgatgccgataaacgggtgcatgatccaaacattaaagcacagactgcggcgatggttcaatcgattaccgtctcaccaaccaaaggcaccaagcgaaatgcgacggtcaccatggtggcccccaagacaccgacgaaattgaacgattatgtctcactgaccagcactcaaaccggtcagtctgaaaaattaactaatcagggtgtcatcatcaccgaaaaattggctactgatatgcacgccaaaaaaggcagcctgctttcagccaagctgggcaataagctgctgaaagtcaaggttgccggggttaccaagaattacgcgggccattatctctacatgacccccaagtatttcaatcaagtttcaacgacgacctattcaccgacttcacacctgttgaagctcaagagtgagagtgccagccaacgacagaagacctcacggaacctgctgaaacaaagcggcgttatgaatgtgacttatccaagatacgccagcagctcgctgggaaccgttggtttaagctcagtcgtgctgatctttatcgctttgtcggccgcattaggtctggtggtgttatacaacctgaccaatgtcaacatctccgagcggatgcgtgaattgtcgacgatcaaggcgttgggcttctacgataatgaggtcacagcctacgttgccagagaaaatgttgtgctgaccctggccgggatcgtctttggctggggcatcgggttaatcctccatcattttattatgatcaaggctcagaccggagcgattttgttcccgctgaccgttcattatccagggtacatctggtcagcggtcttaacggcctgcttcagcttagcagtcggcgtgattacccattacaaactcaaacatattgatatgttggattccctggcagcttcggaatgatggatgccagtgtctaaataatgtccacactcaaactgccacaaaggtttttgcttttgtggcagtttttggtgttccagtaccaacctcagtttcaaatggatgttcagcagttcacccggttatgacgcacgtccccacaaaaacttgaccaacagcttatcaacctgcggattatcgtggagcttgctgtgctgcgcctgtgggccgacgattcgcttttcctggtaggatttgacttgcggcaccagatatctcaaggatttcgaggaggcattgctgacgtcgccgtccgagtgggtgccgtcgtttttatcgccataaatattgagaatttcaagtgttttcaattgcttgtcgtggcgcaatcccagcaactcacggtaatggctgttaattttagtcggctcgccatctgccttcaatttcatccggttgggggcatcgtccattcccaggatgccgttgaaatgccccgcgatgtcgacttgcttctcgagcttgggcagcttggtgttgccagcgttgtccagtaaataaaagacgatcgccatgttgccgacagaatggccgaccatgttcatcttcttaatgccgtagcgttgttgcagcttgacgaccacatttttcgcccatttcccctgggtatgatagttggggtttcgtgaattcaaatagttcacttcaacgatcgggtggaagtcgtccggcttgaaagtcccgacaaaggtgactttcccgctatttgaaacgtctgcgcgaatgaccgacttggtgacgccggctttgaccgctgtgttagccatgtgcgtttcagcgtggtaactgctgccgaagccgtggaaaaatagggtcggggttgcctgattggcaccctgaattttgggtgtgcctgtggctgatgtggtgcaggcgctgagcaagccaattagcaggaataagccgctcagtaaggccaaacgtcgtttcttcattgtttgcctccattattgggaaagattctttttgccaatcattataagcggattgctgctaatgagaagcaactagcagtttgtctttccgcatttttgcgagattttgacaaaaaatccagaattcattccgaagaatgtgagcgatccccgttatcattacaaatgaagcatgaaagccatttacttttgttaaacggaaggctaatataggttgtgaactaattttacgaaatcttaatattcattcatttctgagggggaattgcatgaagttgactaggaccctggcttgctgtgggctttttttggcgttgacgatgattttctttgccgccccaagcactgcacaagccaagtttcatatttatcaccagcgctcgtccgccctgcacaagggatcgctgcgcaatctgaataacaaaaaggttcattatgtcaaagtgccaaagaagtattaccacgttgccaacactgatgttgagcacacaatcaaatccgaacgcggcaagaaggtcagctttcatacgcggtacattttgccgctgcctggtaagaacggccagcattggggaaatccacaatcgattgcgatgaatggcaagggggatatgtacattgtctactgcccgactgatctacataacaagggtcgaattgttcgatttaacatcaagaagctggatgcgatgggcattcggttgcatccaaaagaactgcgggatgcttatcacaagcggcatggcaaatactccaagacccaacagaaaattcacaagtatattaaggcagggccgatatttaccactggtcatggtcaatccttggcatataactggaagaaccacggcttatatatgtggcgggatgtcgaaaaggcgcctcgggttccaatcaataattggggctatatccaacacatcaaggcttcgacgttgcggccggacttcgcgatccgctttcgtctgcacagccacggaacatcggtgcccggcggccacgatctaacctttgatcgctccggtaacgcctacttctggtcattcccaggctggggcgcctacattttcaagggtaaaattcaccacaaatcggtgcactttcgattgacccatcaagtgctgaaacatttaccggggacccggattcaaagtatgggttataacccggttagaaagcgcctgttgatgctgtccgatgcgtcgattgccagtttcccagcgaaacggctggacggccacggtcatttaactaacggcagctttgagtggacccagtttggccccaagcgtgaatttgagggaatcgcctatgatggcagttcccgaggcaatctattagtgaaccattgtccggaagttctacaggccgatcgatcgtactagtttttatctgaaattgaaaaaattgactagtattttcacgattgagcggtacacttatgttatatcaatataaccaaatatctggaggggtatgtatgaaattgggaaagttatcggtggggatcgccacagcgattctattgagtacgtcatttgtgggtactgttgatgcggcgacgtatgtgcaaaaaagcaacgccatcagccaatattcaggcgccagtttacgcattttgaataacagtaaagtccagtttgtcaaagccaatggcaactatggctggtcaaagaatcccagcggtagtgagaccatcaagagtgtccatggtacgaagtggacgctgaagaccaaatatctcctcccaagtacgcatatggcattggggaaatccagtcgtgatttgaccaatcctcaagctgccgcatttggcgggaaatatctgttcgtgctgtatgcgccgcaccaatttcatgggaagggctttgtggtcagatataaccgcagtaccctggatcatatgagtttggccaaggctcaagattctctgcttaaaaagactgccggtatgaaagttggtccaatgtttgatgtcggtcacggtcaatcgctggcttacaataagaagcagcattcaatttggatgtggcgggatcgggctgacatgaagccgactgcctggtcaaccattcaacgaatcagcatgtcgtcgctgaagccaaatcgtgccattaagtttcacatgaacaaccgtggtgcaatggtgccggccggccatgacctaacgtttgacaactccggtaacgcttattggtgggggatttccggcggccacgttaaaatttacaaaggcaagttgggcagccgctcgatccatgttcgtttagccaagcagctgttgagaaagcagaccggaactcaccagcagtctatggggtataacccgcacaacggccgactgtacctggtttccgatgactcaattcaaaccctgccggctcgtaaattaaacggcagtggcagtttgcgtccaagtgacattaaatacactcgttctaattctcaccgtgagtttgaaagtatgatttttgactcaaccgggcacgccatgctgctgtcgaaccgtaatccagaactattacgttcaacaaccagatattaataccattaaaatccgtcagatcaaggctgctgccttggtgacggattttttgagactttatgttgacacggtgtcaccgatggggtatactcagttcataaattgatgacacggtgtcatacgcaaaggagaacaattatggtatcaacaacctttaccaatctaagtgatgagaagcagaccaaaattcgaaaagccttactcaaggaatttacagatcaaccactggcaaccgctcaagttgccccgatcgtcaagactgccgggattgcccggggggccttttataagtattttgatgatctaaccgacgcttacaaatatttatacggcgtggcgatgcgcgatattcacagtgatgtgaacaacgaggtgggaactgaatttgacccgcagttttatttggatcaagttgaggcgttcatcaaaggtgctcgcgatagtcagtatctgggattgatcaagatgcacctaatgaaaaatgaatcactgatttcgcaaggatcaattgaccccaacacggttagttcgcgggaatgggcgacgatgatcctcagtcatgaggccattaagcaaatcatgattgagccgcaaaatgaatcagtagtcatgaaaaagttttctgaaacattgaacttgttagccgggaaggggaatgcataatgtatttggcactaaaagaaattcgacacgaaaagttgaggtatggcctaattattgccatggtggccttgattgcatacttaatttttatcctgacgggtttggcattcggattggctggggaaaacacccaggcgatcaattcctgggatgccaagagcgtggtcttgaataaggattccaatattaatctgtctcagtcgacgattaccaatgcccaagccaaggacgacaaactgtcggctaaggaatcagtgattgggtcgacgccggtggttgccaaacacaaaggtcaagaaaagatttctgcccaatttgtcggcatcaagaagagtgagttcatctataagggattaaaaatctcttcgggtcataaagctcgcaacaaccatcaagtggtggttgacgaaaagttcaagaccgatggctacaaactcggtgacaaggtgacgttgaactctgtgagtgacaaatatgaaattgtcgggttcactaagaacgctaagttaaacattgctccagtgatttatggtagtctgccaacgtggaaacatttgcgggggatggaccgggttccgattgccggcagtgcgattgtgtcaaagaatgctaagtacagtgctcacaatagccagttaaagacgtattcgatgaatgaattcattaataagttgcccggttattctgcgcaaaacaccacgtttggcttcatgatcggctttttgatgattatttcattggtgatcattgccgtgttcctgtacattttgaccatgcaggctctgccaacctacgcagtattgcgggcccagggaattccagcgagagctttggtgacgacgattaccagccaatctttgatcttgatggcttcgggaattatcattggtggtctcttggcggctctgacgggatcgttaattccggtcggtgtgccgatggcctttgatattccggtgctcacctggatttccattggcttgatgattatgggcgtcattggtgcggcaattccagcgcaaaagatcgcaaccgttgaccctgtcagtgttattggaggttagttatgtcagtgattgaattaaaaaacattaataagtactttggatccggtattagcaaggttcacgttttgaaggatgtcaattttgcggctgatcggggacagttgatcctagtggttggtccctctggatcagggaaaagtaccttcttgaccattgcgggtggcctgcagacgccatcctccggttcagtggaagttgaaggtcaagcagttgagtcactcacaaaagcgcaacgagatcagctgcggttaaatcaaatcggctttgtccttcaatcatataatctggtgccgtacttgaaagtcaaagaacaatttgagtttgtggataaaatcaagcatgacggtaatttagatcagaaagaattagcggatttgcttgatcagctgggcatttctcagctggtcaaccagttccccggcgaactatctggcggccaaactcaaagagtggcgattgccagagcactgtatgccaatccggatattgtgttggccgatgaaccaacagctgcccttgatagtgaaaaggttgccgaggtcggccaactgttcaaaaatctcgcagaaaccaggaataaggcggtagtcgtggtcacccatgatcttcggctgctggattttgcggataagacttatgagattttggatgggaagattagtcttaaggacaagggacatgtcaccgatcggtaaactatatgttatagctcaaataattcctgctttatagctatcattttcgttgactaccagccggaaaatgtggcaaaaaggacgctacagtaaaagcaaataatcataaaaaagtgaacccctgcctgggttcacttttttatatttggtgattgacaactaccgggtttgtccaatgaccttttggtaggagaacaattgacaacaaaatagcatggtagttaccaaagaagttaagacttttgagcgacgttggtcaaagtaaccgtactaaaactagtgagtcgattgccattatgaatcgcaactcgccacgtttgcaagtgcccgccggcatgcaacggggtggcggttgccaccagcttgccatcaaaaaccggcagcaaatgctgagtggtgatgtcgacgcccactgcgtaatggctgttatccaatcgttcgttggcaccgattgaagccgccgtttcggccaacaccgagttgatgccgccgtgaagaatgccgtatggctgtttgaccgaatcggtaacttctagtgatataataacctcagcttggctgacagagacagttttgataccaagcaattcaattaagttagacaaagtattcacactccaattttgaaaggatcgagattatgacttcagttaaatgggaatcggtaaaagattaccaggaaattatttttgaacgggccgataaaatcgcaaagattacgatgaaccggccggaaaaaatgaatgcttttacaccactgaccatccaagagatgattgatgcattcaatatctgtcgtgatgatagcacaatcggcgtgattatcctaaccggcgctggcgacaaagccttttcttctggcggtgatcagggggttcgggggaatggcggctatgttggttcagaccacattgcccggctaaatgtgctggatcttcagcatttaattcgaatcatccccaaacccgtgattgccatggttaaaggttggtcagttggcggcggcaacattcttcagctggtatgtgatttgacgattgcagctgacaacgctcaatttgggcagacaggcccgaaagtcggcagctttgatgctggctacggatccggttatttggcccgggtgattggccataaacgagccaaagaagtctggttcttaaaccatttctacagtgcacaagaggcttatgaaatgaactggatcaataaagtggtcccactttcagaggttgagtcggccacattggattggtgtaacgaaattctccagaaatcgccaaccgcgcttcgattcatcaaggcagccatgaatgctgataccgatggtttggctggccttcagcagttgggtggggatgccacgatgctcttttacaccactgatgagggcaaagagggccgggacgcctttaatcaaaaacgacagcctgattttgatcaatttcctaagttcccataggaaggttgatgaaagtggataattggattttaaagcaggcggaaactgcccctggtcggctcgcggtcgatgacggcaacacccagctaacgtttctggaactcaagcagcaggtttctcaactggctggacaattgaaggctgcctccgtgttggatggcgatcgagttgggattatgaccaagaattctttactaggctatctgatggccatggcggtcttaggatccggtaagacaatcgtttggattaattggcgtttgtctgatgatgaaatccatcgccaattatcagatagtgaaccagcggcctgtctggtggcggatgatctttttcgagaaagttttgaccaacggtttattacctttagcacgataactgatcaagcggcggttcagatcacattagttcccgaatttcgctctcaagaggtggccagcattatgtatacgtctgggacgactggtagacccaaaggtgtgatgcagacctttggcaatcacctcgcctcagcaaccgcctcagcttttaaccttggggtcatgccgggtgacgagtggctttgctccgtcccaatttttcatatcagtggtttttcgattatgatgcgtggcttgatatatggaatggcagtccgcttggtcggccacttcaatgctgaattgattgactacgtattgaaacatgaacccatttcgacgatttcggttgtcccgtacatgttaaagcaattattaaaatatcgaacggctgataacacaccttatcaggccaattttcagcgcatgctgctgggcggtgggccaattgatcgccaaacccttcagcaatgtcgtcaactccaagtcccggtggttcagtcatatgggatgacggaaacctgttcacaaatcattgccttgaactcagcggatgctgacaagcgaattggctcggttggcaagccactgtttctgactcagttaacgttaagtcaagttaatcaggaagtgctgatcaaaacgccggcattgactccgggttacttgaaccgacaggctgcttttcaagataagctaaatgacaccggctggtatcgaaccggtgatgttggtcattttgatgatgatggctttttatacattgatggcagactggatgatatgattatttctggtggcgaaaatatctttccggatgaggttgaagccgtttatgtcaatcggtcagacatcggcgagattgccgtggttggccaagatgatgccaaatggggtcaagtgcccgttgcgtttgtggtcagcgatgcgcccttagatcaggtagacctgatcacttatggcagacagaagttagcccactacaaggtaccaacgagatttattagaattgacaaacttcccaccaatgtcagcggtaaggtgcagcgattcaagctgaaacagttgttataaaatgaaacgttaacaagcccgcaatcatgagtaaatcattttactcaggttgcgggcttgttttggcttaaaagtgagttaaaccggtttacatcagcctcgtgtaacatgttaacaaaggtggaacaaactccatcgttgttctggcggcgtctagaaggcctcaaactatatattttagcgcttacatccgttatattaagagcgtaaagaaatcctcgagaatttctgagatccaaacgacaaacaaaattataggagatgccaattatgaaacgagactttatcgataccaacacatacacccgagaagaaatccaatacctgatcaacttaggtttacaaattaaacgcgacattaagaatggaaactatcccgacttattatcacatcggacactgggaatgatttttgaagaatcatccacacgaacccgagtatcatttgaaactgcaatgactcaacttggcggtcacgctcagtacctcgcaccaggtcaaattcatttaggttcagctgaaagtgaatcactaggcgatactgccattgttctttcccgcttggttgatatcctgatggccagagttgctaagcactcaacagttgaaaaattggctgaaactgccacggttccagttctcaacggaatgagtgattacaaccatccaactcaagaaattggcgacatcatcaccatggcagagcatttaccagcaggtaagaaactcagcgactgcaaggttgtcttcgtcggtgacgccactcaggtttgtgtatcattaatgttcatcgcttctaagatgggcatgaagttcgttcaattcggaccaaagggttatcaaatcaagccggaaaccttggaaatcggcaagaagaatgctgaagtatcaggtggtagtgttgaaatcaccgaagataccgacgcagcgatgaaagatgccgactttgtctacaccgatgtttggtatggcctgtacgaagccccactttcatacgatgaaagaatgaagatcttttatcctaagtaccaagttaatgacgatttaatggctaaaggcaccagccacacaatgttcatgcattgcttaccagccaaccgcggcgaagaagttactgacagagtgatcgactcaccacactcaattgcctgggatgaagccgaaaaccgtttgactgcaatgcgcgctttgctggtttacttgatggcaccacggatgaactacaccgaaaaacaattggatgatttgaacgatcctaaattgaagtcgatgatcttaaacttagttgacgacacgactcattaatgagctgacgcaacggatgtgcaggtgaaagaaatgcaaaaagagaaaaaatttagactatttgatgccgtgctgatgtcggtggtcgttgtcctggtggttgaatcagttgctccggctgccgcaatcggcccgtcgcaattcttctggtggggaatcctgttggtattcttcttcctgccatacgggttgatttctgccgaactagggacgacctatgacgaagacggcgggatttatgactgggtgagaaaagcctttggccgccgttggggtggtcgggcagcttggctgtactggatcaacttcccaatttggatggccagcctggccgttctgtttaccggtgtgattggccaagtcttcccgactcatttcgggacgtggaccaacgtcttaatccagctggtcttcatcgggattgtcactttgatttcctcatatccagttgccgacagtaaatggattttgaatctggctgcgattgccaaagtgattatcatggtcagcctgggtgctttgggcatttacgttgccatgaccaaaggcgttgccagcaacttcaccgttaagacgatgttgccgcagatggacgttaaaagtcttggctacatctcagtgatcctatttaacttccttggctttgaagtggttacttccatggccagtgaaatgcctaatccaaagaaacaaattccccaggccattatctggggcggtatcttaatcgctgtcttctatgtctttgccgcatttggcatgggcgtggcaattccaagcagcgaactgtcaacttccagtggtttgatggaaagtatcctacttttgatcggtgggaataattggttcgtcatcctgattgcgttactgtttatgtatacgttagcggccaacctgatttcctggtctgccggggtgaactacgttgcctcatacgctgccaagaaccacgacttgccaaaggtatttggtattgaaagcaagaagaccgggatgccaaccggtgccaatctgttgaacggtgggattgcggccgttctggtggtcatttcaccactgattcccaatcaaaacattttctgggcattcttctcactgaatgtcgttgccttgttgggctcatacctactgatgtttccatcattctggaaactccgcaaaattgatcctgatactgagcggccattcaaagttcccggcaatcatttgatgattaacttgatgacttggattccggtggcattgcttgccatcacgacaattctgtcagcattcccactcaacggcagtgccgaagagcttaacaccaagattccaattttaattggaacgattattacaatcttacttggtgaggtctgcatcagagccgctgaaaagaatcatccgttgaagaaaaaagtcaaggcgagcagtcaccacacagaagaagccttaagtaaaaactaatttctgaatctaatgcaagaggagcaaatacgatgaaaactttacaatcatcacctaaaaaagatggatacagaatgcccggcgagtttgaacatcataagggtgtctacattctttggccagagcggccggataactggcgcaatggtgccaagccagctcagcatacctttgtgaacgtggctaaagcgatttcccagttcgagcacgtaacggttggggtatcagatgcccaatacgccaatgcccgccacatgctgccagacgaggttgaagtggttgaaatttccagtgacgattcctggatccgagactgcggcccaacgtttgtcgtcaatgacgatggcgaccttcgcggtgttgactggacatttaacgcttggggcggcttggttgacggtttgtacttcccatgggacaaagacgaccgggttgcacaaaaagtgactgaaatggagcacgccgaccgttaccgtttagacgacttcattttggaaggcggctcaattcatgtggatggtgagggaacactgatcactactgaagaatgcctgctttcaaagggacgcaactctcagttatccaaagaacaaattgaaaatgtcttgaaggaatatctcaatttggacaaagtcatttggctcaaacgtgggatctacctggatgaaaccaatggtcacgtggacaacattgccaacttcgttaaacctggtgtcgttgcccttgcctggacggatgaccaaaacgatccgcaatacgagatttccaaagaaaactacgacattttaagcaacgcaactgatgccaaaggccgcaagattcaagttgaaaagctttatgtgccaaagccggtaacaattaccaaagaagaaagcgaaggcgttgatgccgttgacggcagtttgccacgtcgtgaaggcgaccgcttggctgccagttatgtcaactattacacagccaatggcggaattgtcttcccaacctttgacgatccaaacgatgctaaagcacaagaaactctgcagcgcttgtacccagaccgcaagattgttggtgttcctgcccgagaaatcttacttggtggcggtaacattcattgcatcactcaacaagtgccagctggcagataggaggaatcgcaatggccaaaattgtcgtcgcattaggtggaaatgccatcctctcaaaggatgcttccgctcaagcgcaaatgaaggcagttaaaaagactgccaaagagttggttaaatttatcaagaacggtgatcagttgatcatcactcacggaaatggtccccaagtcggcaacttattgcttcagcaaaatgccgccgacagtgaagtcaatccggcaatgccgctggatacctgtggtgccatgacccagggcggcattggctactggttccaaaatgccatgaaggaagagctcctgaataacggcatcgataaagatgtgatggcaattgtcacccagacgatcgttgatgaggacgatccagcctttgaaaatccttccaagccgattggtcctttctataaggaaacggatttgcctgagatcaagtcactgcaccctgactgggaaatcattgaagattccggtcgcggctaccgacgggtggttccatcaccgaaaccgttggaaattaacgagtacgcagcgatcaagaaggtcgttgacgcaggtatcgtgccaatcgtttccggtggcggcggcattcccgttgtcaaaaaaggcaaccgcttaattgggaaggaagccgtgatcgacaaagatttcagtgcttcaaagatcgcccaattaattgatgctgacaaattgatcatcctgacgtctgccggaggggtttactacaattacggcaagcctgatcaagttgagctcaaagaagtcggcattgacgacattcaaaaacacattgatgccaatgaattcgccaagggcagtatgatgccaaaggttcaagcagcagtcgcctttgtccgcagtaccggcaatcccgctgtgatcggtgatttggaagatgttgaacaaatcatcgaaggcaacgaaggtacaactatcgttaaggatgctgttcccgcagcagttaaatagtttaaaatgaacgaggcatggacgaaacgacggttttgttgatgcctcgttttgcgtcgattgatggggtattagcagaatgatagtgctttcacagcaaaaatgttatgattgagcgagaaaatatcgaggtaaataatgaagatcaaaaagacaactccacaagaggataaatacaatgtggcccctgaatggcatcaacaccagcaggcctacatgatgtggccggaacgcacggataactggcgggatggagccaaacccgctcaaaaagttttcagtgaagtcgctgcgaagattagtcggtatgagccgctgacaatgctggtttcgcgtcaacaatacgagcacgccctgcatgccttgccggaatcggttcgggtggtggaaatgagttacaacgatgcttggatgcgggatgtcggcccaacttacttggtcaacgcccaaaataacgtccgagccgtcagttggcagttcaatgcctggggcggcctggtcgacggcctttacttcccgtgggatcaggacaacctggtatccgggaaagtcagtgacttggaccggatcgactactatgaagccgattttgtcttggaaggatccgcgtaccagaccgatggcgaaggaacgctgattgccactgaagaatcggtcttatccgaggggcgcaacggccaagttaatcaggcagatgttgaagcggtttttaaacgctatttgaacgtcaccaagattatttggttggcccggggctatttcatggacgaaaccaatggcgatgtggacaacatggtcaactttgtccgccctggtgaagtggccttaacctggaccgaagatcagactgatccaatgtatgaaatctgccatgaagccttggcaactctagaggcggcgaccgatgcgtccggcaggcatttcaagattcaccgggtccagatgcccaaaccattattaatcaccaaagccgagagtgaaggcgttgacccggtcaacggtcggctgccgcgttacgaaggtgatcgtttgatggccacttacattaactgttacttggtgaacggcgccgtgattctgcccatttttggcgatgagcacgaccaggcggccatcgaccaatacaccaaaatctttccagatcgaaaaattgaacccgtgtacgcccgtgaactgctgcttggcggcggcgacatccactcgatcgtcctcggggttccagattagaggttttatatgaacttttttgagatcattaaaccatatgtcgaaaaattgaataaaaatgaatacggcttactcgactatgtgatcaagaatatggataaaatccaaaacaagagtatccgagaaattgcggcggcctgttatgtttcgaccaccacttttttgcgttttgtcagaaaaatcggcttctccggttatagtgaatttagcaccgtgattaagtacacggtcctgaacagcgataagcaggaagacaaggctgaaccgtttgttgaagaacagtccaaatatcgtaacgaatatctgaaaaatattgaagaaactgtccgggtgcttgacgagcgcaaactgttaaaaatctgtcaggtgttggaccatcagcccaagctgtacttttttgccaagggcttcagtaagtactctgccgaatacattgaatacttatatactttgaacgggttcattgtaattttcccaaagaatcacgagcagcgccggctggcctaccgtaacgtacagctcaacgacgttgtctttgtttttgattatgaaggtgaggatgatgaactgattcaaattattcaaaatctgcaaagccaaaaggaatacgccttgctggtttcaattaccggcgcgaataacaatacgattcaaaacatgagtgacgaaaacctctatctgttcacggacgaactcaaagtcagcggagttgatatgacgtcgcacgtttcgttaattgtgattatggaattgctgctgtatcaatttatggagtatgagaagtcaaaacaatagtgtattggaagctaacagcttactttccgtacccgattttgtttgtcttcaagcccacatatggtaaaattcaagaaacaaattgattcgaaaggaatttgagatggcaaacaactcgcaacaagagctcttaaaaacaatcaatcaggctaaacctgaaaagttaaaaaatgtgctgctaaaaatgggatcccttgaccccgacatggctgcattaattttggcgatttttaacgatattcctgttgatttagatatcgacgccggctttgaagttgatcatgatactgtcgaggcagatccactaccatcaaccaatccggataccgacccgcaagcgattgaagaagaaattcgccatgttcgcggcgttatttccaaccagcttcagattgcccgtgagtctgattgggactggaacggtatgaacaatttggtcaacttcttttctgatctgctaggggaagtcattgacgataccggtgaactcaaagtcccgtttgcattaggcttcccagttgccctaatggtggtccaaaatcaaatgaaggtcttttcagaggatagcctttcgccgatgactctggaggattcagttaacaatgtgttgggcgttatcatcgatttgatcaatgaatccggcagtcatttaccagtgaatgaacgtgaaaaatatctggaccaagcgctgaaactgttcggcagtccagtgttcaaagatttggaagcttttcgatatgagtttatcgatgacgttctcggtttggtcactcagcagactgccaataaagtcattaaggcctctgaaagaattatgaagcaaagtactttgtgggatgaagatcaacgcaagaaacatcacctgatgttgcggttacatctttacctggcactgggagatttgggggtcgcccaagagatagccatcgcaaatatggacgatgacgatgtccgcaaacaatggttttttgtcttgaaaagccgccatcgttatgatgaagccaaagaattggcacttgacgttccccgatatctaagaaaagaatgggacgaattgttgtccaatatgtatcaggaattgggtgagaccgacgaattaattgcgctgttgagaaagcggttgttaaaccatcaaaccgccgtctaccaacaatataagcagctgttagtcgagcgtcatgagtggcagagggtttaccctgatttgttgaaacaactggaaacaaaactgtcgcgctatgaatatggtgatattttagctttggaacgggaatattcaaagttgtttgaacaactgaagaagtatcaaagcgcaccaatgatccggaattatctgcgacagatttatccggcggttaaaaataaaatgattccactgtatcatgacgttgtcctgattcctcagtcgcagaagacagccgccaatgcgccaaagcagcttgagaaggatttaagcaacttcttggaaattagccacgatgccaccacggttcaaaaatgggtggatgaacttaaacagcgcttgagcggccaaaccagctttttagagggattggaaatcgttcagactcaaattaatacagttgtatagtcaaaaagttccactccaagagcctgacagcttggagtggaattcttattaaacgccacatcaaaaaggcggccgcagcacaagtctttcaacttgtactgtggccgcctttcagctttaaaaactagctcttcttttcttcaaacaaaacgcgcttacgcagctttggtgaatacttcattaactttaaccgatctgggttgttacgacggttcttggtggttaggtattcttcaccagtttctttgttatgcattacaacatgaattctcattatcttacctcctcacgaatggtaattgttatcattacaaatataaagcactgaccgaatttgtcaagtcatcctcactggttgaactggtttgagcttcgattggccaacaaaaatcatttagttattgtactggtaccagattgctttcccgtttgtcacctgcccgggctcttaatgcccacaggatggtcacagtatcaacgacttcctggaagagggcgccaatgatcgcagggatgacgccaaaactggcgattaacatcaaaatcgtacagatagcgattccaatcaaaacggattgacgagcaacgttcatggtgtcgtctgagattttgaccgctttactgaccaagctcaaatcgtctttgaggacgacggcatccgcggattcactggcagcggttgccccgtgagctcccatggcaatgccgacgtcagccattgccaatgatgggacatcgttgacaccatcgccgaccatcacgactgggcggaacttcttttcgaccttttcaatgacggaaattttttcttccggcagccgctcggcgtagaccttatcaatcccaactcgatcggcgatttcttcagcgatcggttttcggtctcctgagatcatcatgatttctgtggctcccatctgatggagactatccatcacagccttggcttccggtcgtaattcatctgagaaggccacgtacccgacatatttgccattgacggatacgtagactgccgtttgatcaagcgggtcaattgggtcatcggaaacataagccggtttaccaacccgaatcgtttgctgatcaatggttgcctggactccttgggcagtggtttcaataacgttggtggcagtcggaatttgatccggaatcgccgccaccagtgaacgggcgagaatgtggctggattgctgttcggctccggcagctagcgccaagacctgatctttggtgtaaccagctatcgcgaagacccggctgacggtcaaatgccccttggtaatcgtcccggttttgtcgaaggcaaacgttttggcattggccagcttttcgataatcgtcccactcttgacaatgatcccatttcgactggcacggctcatgccggatactaaggcaattggcgcagctaaaatcagtgggcacggtgaggcaaccaccaggacttcagcaaaccggaccggatctttggacaggtaccaagctactccggcgatgacgtaagccagtaaggtgaatggtacggcgtagcggtccgccatccgcacgaagtgggcaggggtgctctcagcctgtttaactaagcggatgatgttttggtactggctgtcatcggccgttttgtcagcaatcatgtcaaaggatgcatcgccgttaatcgctccggacatgacggttgaaccaacgaccttatcgatggggcgggattcaccggttagagaggattcatcaaccgaagtcaccccgtcagtaatggtgccatcaaccgggatgacttctccaggcttaacgacaattcgatcgccaacagtgacctggtcaattttgacgtcgaccattttgtcgtctttcagcaaatgagcggattggggcgaattctccagcagtgactgcagttcggagttagctttgttggccgcataatcttccaaagtgtcgccgccggttaacattagcaaaacgatgagagcggcccagtattcacccacggcaatcgttgcgatgacagccgtaattgccagcaggtcgacaccaaatttcccggagcgtaaagttttcaccatgtcgataaacatcaaaagggcaattagtgaccccagcgttgagataacaatctgagcgtaaagcggcaagtgcagcccaaattgtagaaccaaggcgatcaccgcgacaattaagacgccgattagacgcatgtagttggttagtttgttcataataagccctccaatccggtttaatcttctatctagattataacaattctaacgtagaaaggcgagctataactccatgggttaccattttcaggcaaaatatgtacaaaaatggcccgccatcatcgggcaggccagtgagacattattgggattatttggaaagttgactcaaagcttcaaagtcttcatcactcaatttaacattagcagcagcgacgttatcctccaagtgttgaatcgagctggttccaggaatcggtaaaatgtttggtgaacgtttgagtaaccaagccaaagcgatctgggcttctgagacaccatactttttagcgatggtgctgagtggactatcggcgccaattaaacgaccagtgtccagtgggaaccatggtaaaaaggccatcccttgggattgtgcgtagtccaccacatcgtcatccttgtggttggaaacgttatagaggttttccacagcgtcaatcttggcgtacttttgggcttctttgagttgatcaacactgacttggctcaagccgatatgcctaattttaccttcatcctgcatcttcttgagttcaccaacctgctcagcgactgggaagtgactgtcaattcggtgaaggaagaccaagtcttcgtgatcaatccccaaagtcatcatagaaacttcgacttgctggcgcaggtagttgggctcaccatgaggtgtccagatacccgggccttggcgagtttgtccaaccttatcagaaatgaaaatctgatcacggttggcggcgccctttaagccttcagccagatagcgatcggcgaaccacggaccgtaagaatcggcagtgtcaaaaaagttgattccaagttcagtcgcgtgggtaacaacatcggctgcacgggcagggtcagcgtatggaccccaagtgccgttaccagtcagctgcatggtcccgtatcccaggcggttgacgacaaattgatcatcaaatttgtaagtgccagcgtttgctgcatttagttcagtcatcaaatacacttctttctgacaataatttggtacaggtctattttcaaaccgttgctgcctgatgtcaatcaaacaaacgcgcaatcgtttgtggttaatcaattttacgaaaaatgacaaaaagttgttatccaagctatacggatgggtcagcaccctgtaaaatattgtatacttacgttgataagagagatttatgaatagctgtgtttgattggggaatccatacagaaggtgaaaacgatggcagtaaagtattatggcgtgatgatggtgaatgttcagggctctgaattgttgatcgtgaatttaaagaacctgaagccactcgagcacgtcaaaaaagatattaacctgggagacgatgtctatcaggaccaacccgtgaagtacgaatccgttaaccgggtgtccgaagctttgaccggattcattcaaagtttgaatgattacggtgtgaccaactacaaactatttggcagcaatgcccttcaccaagcgctcaactcggattttattgccgatcagctctttttacataccggcatgaatattgagtggctttcaacaagtgaagaaacttatttcagaaatcaaaacatttcagttgagttgacgaaggataagcaaaacgataagcgcaccacttttttggtgggcatcacttctggaaatactgccattacggagttcaaggaaggtaaatttgtcgactccaccagttttgccttggggccaatcaaaattgccgaggacttgcagagcctgcggcaaacggcacccaattcaattgggctgttgaacgattacattgattccaaattgaacgacttttacatcgggaatcctgccagcgtcgtgtccagcaaagttcccaccaagatcattttgctggggtcgctgcctttgcaacggctggtggaaaattacgagcacactaaggccagcgacacgattactgccagcaatttcactggattagtggacgacttggtggatgcttccgatcaatttttgattgaacggctccaagttgatccggactacattcctttggtgctgccggaactgctgttgaccagacggattttgagattaaccaatgcttctgaaatcgggttttccgattctggggtcgttgatggtctggtcaatcaggaagccttggaacagggctactcaaaacgggatttcacacccgagattattcgtttggctttaaacctttccaaacactatgatgttgagccggtccaccgggatttggtaactaaatttgcccttcatctatttgatcagttaaagccgctgcaccaactgggccgccgtgagcgaatcctgcttcaggttgcctcaattctccacgatgttgggaactacgttggcatccatgaacactacctgcattccgagtatattattctccattcagaaatcattgggttgtcccgggatgatattcgggtgatcgccgcaattgccagatatcacagttcgacgacgcctaatgaagatctgattcactttcagcatatctcagctgaaagccggcgattaattgccaagttagcggcaattctgcgtttggcagatgccttggacgacgaccgccagcagaagattaaaaaaatctcggtttcaatcaaggaatctaaagttgtcatcacaacgttcagcaatgccaatctggcctacgaaaactggatcttcaacaccaagagtcagttctttactgaagcatatggttataaagccgttctcaaacaaaggggtgtaaaggcaaaatgacagacaaaattgattttaaaaatcccaaatactataacaaccgcgaactgagttggctggattttaacgaacgcgtcctagaagaagcccgggataaaaacaatccattattagaacgggtcaaattcttagggatcacccaaagtaacctcgatgagtgggtcatggttcgggtggcgtcactggcaaaattggttgaagttaagtgggatggcaaagattcatctggccgttctgcagaagagcagctccgagacgtcaacgtgaaagcccatgagatgctggttcgacagtacagcaccttaaaccggtcgttgttgccggcgctcaaccaggtcgacattcatttactaaaagtgggtgacttaacacccgagcaataccagttcattaaaggatacttccacgatgagctttatccagtgctcaccccaatggcggatgacagttcgcgcccgtttccatttattaacaatgactcattgaatttgtcactgcggcttaacaagaaagatgatgaggagggcaagacactgtatgcgacgcttcaagtccccagcatcttctcacgggtcatcaaactgcccggtggcgataacgattttattttaattgaagatattattaagcaattcgtcgatcaattattcattaactacacgatcaaagaagtcagtgtcttccgggtgattcgggacatggacctggatgttgctgaagaagatacctctgacctgttgaaaaaggttcaacagcagctgaagttgcgtgaacacggccaagtgattcgtttggaagtggattcaaccatcagtagcaaacttcgaaagcggctggtcaaggaactccagacggccgaagattcggtctatgaagttaacggcccacttgacttgaccttcatgagcaaattagctggtaaagtaatcggtcatgatgatttgaaatatcgaccgttcaagccttatcaaccggcagctttagactccgatcacaacatttttgatgccattcaaaaacatgattggctgatgcagcatccatacgacaaatttgattccgttgttgaatttatccgtcaggcatccatcgatagtgaagtcttagcgattaagatgaccctctaccgtgtatccggtgattcgccaatcatcaaatatctgggacgagctgctcaaaatggcaagcaggtgacggttttagttgaagttaaagcgcggtttgatgaagaaaacaacgtccattgggcccgtcagctggaaaagatgggctgccatgtgatttatggcctggttgggttaaagacccactccaagctgtcattagtcgttcgtcgagaagaaaatgggatccgtcgctacgtacacatgggaactgggaactataacgacgtcactgcccacttctacaccgatttgggtctgttgacctgcaatactgatattggcattgacgtcacgaatatttttaacatgttatccggttattcacggccgccatacttccaccaactgcatatttcaccaaatgggattcgtgaatttatcaccgagcgactggatgaagcgattaaatatgccaagcagggcaaaccggttcatgttcaaatgaagatgaattcgctgtctgatcaggatatgattgccaaattgtatgaagcatcccacgctggtgtgactgttgatttgattatccggggaatctgctgcttaaagaccggcatcaaagatgtcagtgatcatatcacggtccattcgatcgttggtcgattcttggaacacagtcggatttacatgtttaattttgacggtgaacaacaagtttatcttgccagtgccgatctgatgactcggaatttgaaccgacgagttgaacagatgtttccagtccttcaaccggatttggcccagcgagtggtcagcatctacaccaccatgtggaatgataacgtcaagacaagaaccttggataagaacggtgtctacaaacgagtggacagaagaggccgtgagccattggattctcaagaattctttgcagctcaggcaactcggttgaccgaggctcagcaaggagagaatcggcccaagagtggggcccagtttcagccaatgatgagcccgcaaaatcagcctgatccattcaatgatgaagatgggggcgacaaccagtaatgaaaaatttggcggtgattgatttaggatccaactcagtgcggatgaccattagccgaatcagtgacgatggcacctacgagacagttgctcaagaaaaggaatatgttcgactgtctgagaatatgggggttgagaaaattcttcagcccgaagccattgaacgaaccatcggcgctttgaagaactttaaaacgatttattccaagcttgaccatctcaatattgttgcggtggccacagcggcggttcgacaagcgaccaatcaaaagcaatttttaaaacgggtcaaaaatgacattggcattaacctcaacgtgatttccgggacccgggaagcttactatgattacgttggtgtcagtgagacactgccggcaaccaatgcggtgattatcgataccggcggtgccagtgccgagatcgtcctggttcaaaacggcaaggtcagtaacctgatcagtattccaattgggtcagtcaccttatcatcaaaattcgatttggctgacgacattgctgctactgaagtctttaaagcaatgattttcgttaacaaaattttccaaagtgtctggtggctgcgaaacggtttgaacttgccaattattggcttaggcggtagtaatcgaaccttggctaagattaaccggcgtttcaataatctgttggataccaatgacatccacggctatcaattaagggatgacgccattaatgaaacctttgaacgcattattgggatgaatcttgacgaacgcaaaaaggttcccgggattaacaaggaacgggctgacattattgtcggcggtctgatccccgtcattttactgatgaactatttggattcagacagaattatgttttcaaccagcggcctgcgagaggggatcttgttcgaacggctgcatgatattattcaagagaatattaaaaccaaggaataattaaattctttcattcactcacaaacgggcctgagcaaaactaactgttttgctcaggcccgtttgtattctaattttcaatatggtttcatcgaatagtgtgaatctaaccgcttattttcccacactcgcggtatctgtcccactcaaccgttcaaagaacagcaggtgtttttgtgagaaccagtcaatcagtaagtcgacaaagactagcagcagaccaaacgatagaatcagcacaacgtggagaatgctggttaactgggctttgggggcggttgccgtcatgtctaacagccggccgacaatctcgtataggctaccgatcaccccgtagccaaacaaattccggattaagattttcgaccagctggctgtttggccattacggttaatcactttgatgccaaccaggcgcatgccaatcgtctgctggcggctgagttccagtaccagaataaagatgacaaagccaatcgcgatgccaatccagtgtggaatcaggaaaatgcccaaaatattggtcagcagaccaatgatgatccaatccaccgccaaagcgactccacgccgcagcggcgaaacgtttttactgagcgccattgtccgggctctgacctgttccttggttggtagaaaacggccaagcagggaagctccccaagcaccgatgatcccaccagtggtatttaacagcaggtcgtcgacatcgaatagtcgataaggacggggatagatgccgtaaagaccggagagttgggttaactcgaagaatagggataagcagaatgtgaataagattgtctgtttccatgaccgctggaaataatagtgcaggtaaaagccaaatggtaccgttaagaagatattaaacaccggttggataaccgtgggggcttttaaggccgcaacccacgttccgggatgcgtcagtgaaaacggattgtatttaatgaactcccgaacgaatgtgaacggcacgaaattgtgagtcggggtcgtcaaatgggccacaaacgattggcttggcaatgggagaatggtgagaaagtaggcgcacatcatgtagaagacaaatgtgtagagcataaaaatactccacttgggaattgcgccatacttgtggtagttcactaacagaatcggtaaggtaataaaaattgctagaattggaaaaataattgcagccgtataaataacgtgaatgtactgtgacatggaaatctcctaaactttattttattgaatgggctcaccggggacaaaatagagtaacagcccggttccaagggcaattaaggcaatcaaaacgataattgcgatattggcgcgtttgttcattaccagaaaggcgaggtgttcgcggatgactgcgttgggcaaaaagtaaaatggtgttggcgcgccaacaccgaatgcggcaaatttcaacttccgggcaagcacgccggcccgcaaaatgtgatagttgttggagacaaaaatcactttattgtcgtctcggccgctgtctttttcgatgattttccgggagaaggctaagttctgttcggtgttgatggacttatcttcaaccaaggtatcaactttcgggatgccatgttccaaagcgtatttctgcatggcctcaccttcgggcaataattcgtcaccgccttgaccgccagaaaagatcagctttgggtgtttgccggtggctttgatctcacttcggtaaaaagaaagagctgtttcaatccggttgcccaacagtcgaccaactttgtagccgtcgatcaaaccacttcctaagacgataatgtaatctttatcttttcgtggaaagtacagtcggtataagatcatcgacgaaatcgtattccaaaccgttaataggacgtagccaattagcaaggtcaaaaacatcgtgatggccccttgaagcggtttgggcccaactgatggattgaagaagaataacaggtcaacggcgatgacggcaatcccggtaatcaaggtcagcgaactactgaggctataaccttcacgtttccacacaataaaggcgttaatgaaaaagaagatgaagcttaacgtcaaccccaagaaaaccagtaagccaaccaaagcaaccgccagccctaaaatgatgccccagaactggctgttgaggaccgagataatttcaaccagcaagaccagcagaaccagcagcgataagtttgccagggtgccgatatataaggaatttctcagtttaattaagtatgtaaagaataatccgaccaggacgatgaagataatcgcggtcggtatcagtaaagtcatagaaaacacccctttgaaacattatatttcaaaggggtagtggaaaacaagcacggtcgcttcccgtaggcaaactttaactttttagctcattccgacagcctcggcatgtgccagcatatcattgagcatttctcttctggtttggtgtggcaggaagctgcggatgttttcctcactaaagccaacctggagctgttcatcattgaagatcagcggccttctgagtaaatctggatattttaccatcaggtcaattaactgtgatacagtaagattatcgaaattgacttttaatttgcgataactgtgacaacgagttgaaatcaggtcctcagtgccattttccgacagtctgagcagttgcttgatgtcatctgcgttcaaagtttgtttggagatatctcgttccacaaaatcaatgtggtggtcggtgagccactttcttgcccgtcgacacgatgaactgccaggcgacaaatataaactaagcatggttgccatctcctttactgactgtgacgacaatgcggattgatgcaccggctcatcaacctatccccactttcatcttatcataattataactaaagtcaaatgttcgctataagaaacaggttaataaggccttgctacatcaagggtcccgacccttgtgaaaggttaagcaattcttaatatttaatctgaatcattcaaattttgaaggagtgaagatcaatgaaaattgctggatttggcgttgaagaatggttaaataaatgggagaaatccgcaacttatgacatttctcaaagcacgatttcatcaatgacgatgcaagaagccctggcacttgatggccagcagggcgcatcattttatcaacaactggatcaagaaaagatgaactatggctggattgaaggctcacctgaattcaaacaggaagttgctaaactgtacgcccatattgacgcggacaacattttgcaaaccaatggtgccaccggagccaatcatttggcattgtacgcattgattgagccgggcgaccacgtgatttcagagtacccttcctatcaacagctgtatgacatccctaagtctttgggtgccaacgtcgatttttggcatatccatgaggatcagaattggtatccagacattaacgaattaaaatcattgatcagacccaacacgaagatgatttgcttgaacaacgccaacaatccgacgggaaccctactggataaggcatttttgcaacaagttgtcgaattggcccggcaggtggacgcctacgtcttggtagatgaggtttatttgccattggatgatcccgatcaatttacttccattgtcgacttgtacgacaaggggattgcgaccaattctttgtcaaagacctattcaatgccgggaattcgaatcggctggacggcttcaaatgcgactgtggccgatctctttcgcaagtatcgcgattacacgatgatttgtgccggcgtctttaatgatttgatggcgacctacattttgaagcatcgtgaccaagttctggcgagaaatcgacagctggtgatgaataatctggcaatttatcgtgactggattgactcggaacctcgagccagtgtcgtgatgccccaagcggtttcaacttcgtttcccaagttggatgtgccggaagatattgaagccttctgtattcgcctgctcaaagagaccggcgtcttactggtaccaggcaatcgatttgatatgcctggccatgttcgcttaggatattgtgccgatgaagcaacactcagggaaggtctgaaacggctatccacatttttgcgccagtacgattaagctgatttgattatgaatgtttaaagttgtttgcgtttgtttaaaggtgatcgcttgaaaagccacattggcccaactttaagtttgggttaagctggcccttgtaatctatggacaatcaaataagaaagaagggatcagtaactgattgtcaccatgataagtgcagccaatgacttaaagtgccaacaatgagattgaagattgtctcctccaagatatgattcttctacaaggcattgtcatttgggctacaggaaaggaagtcatctatgaagcgaaaacgtctttactttacctctggaattgcggcgacagccattgccttagtggttgccggacgcgttttccaacggtcacgcatgattgcccatgcgaactaaaccagaaccactcctccaaaaaaatcgctgtgccacttaatcgttcaagccggttaagctgacacagcgattttttaattttgatttgctttttgcttggctaagttggaagcagcaaagactgattcagtttcctcccagattcgcttggcaattttcgacttgttcatcgtgtagaggtgaataccatcgactccctgagagaccagatcaatgatttgatcaaccgcaaaggcaatcccggcatccagcatggcttctttgctgtcttggtaacggtccataattgcggcaaatttctttggaatcggcaccccggagatttgggtgatccgctcaatttgatttttgttggtacagggcatgatcccagcttcaatcgggacgttaatgccggcaatctcagttttttccttgaaatcgtaaaacgcttgattgtcaaagaaaagctggctgattaagtgatcggctccggcagccactttttccttgaggtggctaatgtcatcgacaaagtcggctgcctctgtgtggcagttgggataacaagcgctggcaatgctgaaatcggggcgctgctcgtggacaaatttgaccaattcattggcatgattgaagtcgccaaccggttctttgccggggatgcggtcaccgcgaagagcgaggatatttttgacgtggatctgatcaagtcgatccagaagtgccaaaacctggtccttgctctgataaagcccgggaacgtgcgaaaccgccgggatattgagctgattttgaatcaaatcagccactgccacagtcccatcacagtgattggttccgccggcacccaaagtgaccgagataaaatccggctgcagtgactgaagtcgtttgagagttggcaggatcgcatcagttggggagtcctttttaggtggaaatacttccagcgaaaagacggttttttgtttaaacaacgctgttaggctcattgatctcactcctaaccttcttggtggcatcaacgatattcttcaggctttcaaatgactcgtcttcagagcgggtcttcaaaccacaatcaggattgatccagactttatccactggcagcttggcaactaattgcttgattaagccttcgatttcttgctcggaaggaattcgtggtgaatgaatatcgtaaacgcctggtccaacttctgtttggaacttggcggccaccagctgatcgatcaaagtgaaatcggcacgggaggcttcaaaggaaatcacatcggcatccaaagcgtcgatggctttaatgatgtcaccgaattcgctgtagcacatatgggtatgaatttgggtgctgggttgaaccttgctgtggacgaggcggaaggccggcactgcccagtccaagtattcagagtaccagttggactttcgcaagggtagattttcacggagtgccggctcatcgatttggataatcttgatgtcgtgcttttccaaatccaagacctcatcttgcaaggctaaagcaatctgggtcaccgattcttttggcgtcacgtcttcacgtgggaacgaccagttaaaaattgtgaccgggcctgttagcatgcccttcattggtttatcggttaaatttttggcaaagactgaggccgcaaccgtgattggtgcggttcgactaatatcaccccagatgattggcggcttaacaccccgggtgccgtatgattgaacccagccgttttgggtaaagacaaagccggctaatttttcaccaaagtattccaccatgtcgttacgctcatattcaccgtgcaccaggacgtcgagcccaatcttttcctgaattttgacgatgcggcgaattttatcttcattaaatttatcatattctgctttggtgatttcaccgtggcggagttttgcccggttctggcggacatctttggtttgtgggaaggagccaattgtcgtggtcggcaaaattggcaaattgaattcctttttttgaatcttttcgcgttcacttcgggcgggtaaacgggtgtagtcatcatcggttaaattgttaatccgttcatggacggatttattgtagggatgtttgacgttgcggaaaagggcgtcatttttttcgagcgctgatttaccgtcggcttcatcgtggtaaatggtgtccagttctttaatttcggcaagcttttcaatcgcaaatgccaagtgctgtttgacgtctgatgggaccttggtttcatctgcggcactgtatggcacgtgtaatagagaagcagaggaactcaaaacaactttggcgtccgtattcaggttgtttagcaggtcgatggttgttgcgtaatggttgcgccaaatattcttgccgttaacaactccggcgaataataccttgtcagcggggaagtcgttttgtttgacgagctctagattgtatttgccttcaacaaagtcaagaccgattccgtcaaaatccaggctggtgacgtcatgatagatgtcgcggatatcaccaaagtaattttgcagcagaatcttgctggatcctttggcagccagaatgccgtgatacaatttgtcaaaaagggctttttcagctgaattgacgtcgaagcttagggcaggttcgtcaatttgaatccagttaaccccttgttgatttagatgctcaatgacttgtgagtaggcagcaatcaaggcatcaacaaagtcattgggtgtcgtcccatcaaggaaacgactgagtttgagtagtgtgtaagggccggtgatgacggccttggcattgatccctaatttgagtgcttcgtcgacttcattaaataatttatcaccgactaatttaatgtccgtcgtcttagtgaattcaggaacgatgtagtgataattggtgttgaaccacttcttcattggcagcgccttgacggtttcagaaccgttctggtacccacgggcttgagcaaagtattcgtcaagcggtgataagttgagggccttgtagcggtcagaaacgatgtttaagaggttggcggtgtctaagaccccatcaaaaaacgagaagtccccaacaggaatcaggtcaatgccggcgtcttgttgcgcctgccagtgattcttggggatttgataagcggtttttagtaattcattttgatcaatcttgtgcttccaataatgttcggtagcaaattttaattcacgatggtgaccgatgcgcggaaagccgataatggtggttgtcatgtgtttgtatcctcctagagtgcgatttggggcggttagcaaccggagcctaaggcaacttgggggaaaatcgattttgattttgtcccaagttgccttaggtgcaggttgctgccccaaagagcacgtttcatcaaagtaaaagtcagtgtagatagcggcaggctcagcatttatttaacaatgagttttgacgcgtttttggcgtcaagactcgttgttagataaagcggagggagctgccccaaagagcacgtttcatcaaagtaaaagtgagtgtgccagcagcaggtctcagcatttatttaacaatgccttttgatgaagactcgttgccaactaaaattaagcgaaacaaatacgtttcacaaacccctaaatcacgtgccgctcatatgggtcattggaaatcccctcagccaaaatcttcttgctccattctttggccgaaaacagtgagtggtcgcggtaattgccgcaactgtatttatcaacgccgggaacgtctttccattcaacttggttggcaatttcatccaatgaaccttttaaggcctcggcgacttcggtagtactgtgttccccccaggtaatcaaatgaaatcccgtccggcagccgaatggtgaacagtcaatgacgccatccaagcgatcccgcagtaaactggccagtaagtgttcaattgtgtgtaagccggcagttggaacggcggtttcatttggctgggtcaatcgcaggtcaaaatttgagaccacgtctcctttggggccggtctctgtggtaattaaacgaacgtacggtgctttaacctttgtgtgatccaatgtaaaactttcaacttttgccataaatgatcaatctcccataacatttaatttgtttttaatgctaatatcaccatccgaagttgaggacacaaaaaaacatccgtccctcgcatcagaattaatctgacggaggggcgaatgtttcgctttaccaccctgaatttgttttggcctcacaaccaacacctctgaaagtaccagacttcgatactcggcgatgtaacggtcgcacccggggttcaagcgttaactcgaaaccgctattcagagttcatgttcgttagcttatgaaccatcctttttcaccgaccggattctctaagggttcgttcactaattactcttctcttcagagctttaatttactagcattaaaatttagtgataatactagtcgtagttctaatgattgtcaacctgatatgctaaattatttattatccggcgaaaggcccttgaccaaaaactcgacagcttggtcaatatcccggtccaaatcgactttccgatcaagtaatataatttgggcaccaaagccggcaccaattgaaagaacgtactccaaaattcgggaggtctcccagtccaccaagaggtggcgttctttgagctgatcaatcaccttaggaatagtggtggtcagcacagccttaactggaacgaccaattctgacaataattggggatcgttgacggcctgcataaataaaattttgaggatttgcttgttttcgctggcaaaggtcaatcgattttttaaagtcggctttaagaattctgccaagctatcgtacttgaaacgcttgaggtcttctgagaactcttgggcagctctgggaacggtttgcgaaaataatggctgaacaacggcttggagcagctgttctttggttttgaatcgtttgtaaaccgtgccttgactaacgcctgctctttcggcaatgtccgccgtcgttgtggcttcaaatcctttggccgcaaacaagtccaagcaggctttcagcacctgtttttgtttttggggtaaatcttttgtggaatcaatatcttccgaataaaatgactgaatcgaagttgatgccatgttaatcacctacactttccgatacttgcgcattccaatcatatttaaagcaatgaaggcgaccaagaatgctaggatagctgtaaattgtgggacaattgccgaaaagttggcctgcttttgaatgacgtcggttaacgcactggccccgtaatacagcggcatgatatgggcgataacctgcagccagcctgccatgttggcaactgggatcaaacctgagaagaaaatttgtggaataacgacaatgggaatgaactggaccatttgaaattctgaagcggcaaaggtcgaaacaaacagccccatcgacagcgcaaccattgctaaagcaaaacagatcaataagacgacccagatgctgccaagaatggagatccctaagacatagatacagaataacacgatcaccgctgtttgaatgatcgccacagcgccataaccggttaggtagccgtaaatgatttcacttcgtttaaccggtgttgccagcagtcggtccaaagttctggagtttcgctcatttaacagtgaaattccagaaattaggaagacaaagaagaagaccatgaagcccaagaacacaggcagcatcgttgtgaagaaggtggaattactcttgccgtaaagatagtgctgggttaatttcaggttggttggcttttggacgttttttggagcggacgctgccggaatccgactgctgagggtcgctggcagctgctttttaatttgctggagctgagcttgcatcttcattaagccggctttggactgtttcgtggtagaaaccagctgcttaatttgaacttttatcagagccatctgaactgatttcttgatgatcgcggtcttactctgatcggcattttgatacgtgacgactaagtggccatcagtttttttgatgaaaccggcgtagtctttgttacgaatggtcttttttgctgaaacattcgaatccatccgatgaattttgatgtgcttgttgtcgattgttttgaccaatgaactagacacattataggtgccgatgtctgcgaccgtgttggtatttgactgaaataagaaatacatcaatgacaggatgaacagcggcgcaataaacattaacgcaagcgttcgtttatcgcggaacatttccacaaagatacgtttagtgattgttagaattctcatttgatttccccgctttcaaaaagacctgttccaaattatccacgtcgtattctttttccaaactggtgggtgacccgtgggtgatgatgtgaccttcgcgaatcatcaatagttcgtcacattcagccgcatcttccatgacgtgagtggtgatgataattgacttgccggcttgggcatattttctgagttcatcccaaatctggcggcgaagttccgggtcgatgccgactgttggttcatccaaaattaacaaatccggatcttgaattaaactgatggcaagtgataatcggcgcttcataccaccggaataattactgacccgtttgtccaaatcctggtttaaattgacaacgcctgccgtgtagtcaatccgttgcttcagctgctcttttttgacaccgaacagttgagcaaaaaatttgagattttccttgccggtcaaactttcatatagggcatcatcctgagccataaagccgattcgctgcaggacggggcgattgggcattcgtttaccaaaaatagtcacttcgccaccgtcgggctgttccatgcccatgatatttttgataatcgttgtcttgccagctcctgatggcccaattaaacccaaaatctcatggcttgaggcagttaggttaacatcatgtaaaatccgttttttattgaagcttttatcgacgtgagtcactgttacaacagcatccatagttgattcctccttttgtgagtgagtgctaactcatttacggcttcagtataccccattcaaagtgagtgtcaactcacaaattgcttttcttgccggtctcacgtataatgacattaaaatttagtcctttaaatagtccagcgagtctgtcaaggaagccattagtgaacgttgtttttaccagcaatagtctgggaatgagcacttcgactcgttgtgggttgaagtgcttttttatttgctaatgagcattttagtttgcttggaatgatttaaaggacaacaaggagatctatcatggaagacaaaagtttcggtcgcgttgagtccatcccaaaggctcatcggcatcaatcctattgggatatgtttgctacttgggtgggggcgaatgcgaataatggtacttggtatgttggcggggttatcgctgcttgtgggtttgcgacggcttcgacgactctgattatcgtaggtgtgattacatattttttactggcattatccggctatatggggtacgaaaccggtttgcccgcaatggccttaacccgagcttcgtttggcctcaaaggcagtttcctgccatcggtgattaatgtcgtccaatttatcggctgggccgccgtgaatacgtttatcgcggccacatcgatcagttatattctccacgatgtcttgggttggccggtatacggcaagccgggcggcctgaaagggttgatctcaggaattgtggtgatgagtattctgcatttattgagtatctcgatgggtgaaaaatcagtccggatcatcgagcgaattgggattgtcttagttttcatcttggtaatctgggaatctatcgttgttttccaaaatgtgtcgttatctgaaattgtctcttggcatgcacccagtgccttgaagatgtcaccaggtcaagccgttgatgtcctagctgcctttaatttagcctgggtaacagctgccagtgatttcacccgcttttctaagaagcgttccagctccacttgggcaccgttctttggcgccaatctgggattgatctggtttgcgatgatcggaatcatttcaacgatcgcgactgccattaccctgaatcattttgatgccaataattcagacccatcaacgattgccagcaaacttggcttgggtgtcttggcgatgcttgtcatcatcattaccagtaccaccgcaaatgccgttaacctgatgtctgccggatctgcgttgaccaatatgactaaacgattatccttgactgtcagtattgtgctggtgaccttggtggccgtctttgtgaccttcattcccattttctactcaacattcctgaacgttttcactgcctttttggacggcatcgggatgttcttaggacccgaaatcgccatttttctgaccgacttttatctggttgccaaacggaaatatcgagttgaccattttgcctcccggaccggtcaatattggtatactggtggtattaactggattgcgattgcttcatggctgatcgctgtccttgcatacggatacattaaaacggtggccgtgttggcggactcagtcggcgcaaccttcatttcgatgttgattgctgccgtcatttattgggtcggcagtcgattgaccagtcgcagtcaacttcaggaggattagagtggcaacttttaccaaacaaaccttgtctttggatgacgttgaaccggacaatgaatacgtgaactgtacgttgacggtttctaacgagctgattcggattaatgacgttgtgtttgaccactgccagttcgagcagagcaactttgacggcagtgattggggctacgtggaatttaaaggctgcaatttcctaaacgcgactttccacaagagttatttctccaactgcaaattcacgaatgtgcagctgatgggggctgatttttcgatggaaacgctgcttaagaaatgtcaatttcatgattctaacctgcactatgccaactttagtgaaactaaaatggaagccagcttctttatggactgtaatctggtcgaaagtagttttcaggcagtgagtgtcaagaaagaattatcctttaacgcctgtgaaattaaccaaatcgacttcttggacacgcgaatgaaggggatcgatttgtctcaagcccgctttgacgacttaattgtgaatcccgagttgatcaagggcttaaaaatcaatccttggcaggcagggcagattgtcgctatgctgggtgtgattgttgtcgattagctttaattaaatattttctgggattccttcaatttcgagtggcagctgatgatataataatcactcagggtcaacatcgatttgaaaggggacgtccagccgtgaataaattgccgacacgaatgacatttttttatcaacttcatccagtcgtttcggcagtttatttttttgaggcgattttgagtctgctcttgtttaaccatttggcgacggcattgaccggttatgtaggattactgttggtgggcattttttataccggacaatcagcggtatggcggcaattcaagtggaatttgagcttattattgatgatcgtcttttttaatgtgttgttaaatcagcggtttgggccgatcctctgtcagttttccgtgggtgatgtgtcattcaaactcaccttgccggcactgctatacggtgtcgttatggggttgatgttagttgagatgctcatggcttttgctgttctgaacgtcattttaccggcgcctaaattggtatatgtcttgtcaccagtgacgccgaaactgggcttattagtggttatgtcaatgaatttagtgaaaacttttagccacaccctggctagtttggcgatgctccagcagacgcgaaacgttcaggataacggtggcggggtacttagtcgcatccggaatgctggtcgcctgttgcggattttattggaggacgcactcgcatcggggatggaaactgcccgattaatggacgccaggggattcggggttggtaagcggactcactaccgggcctaccattggaaggtcagtgactgggcatttatgattgcgtcgaccttgatttttgtctgggccgtggtttcccgaattcagtcagccggttggtcgacatcagtcggcgaattcacccgtggctggatgagccaggatctggttgccttatccgggctgggaggattactattattaccgctggcggccgaaggagtgtatcgcgcatggacaaattaattgaaactagacagctcacatttacatatcccgatgcttctatcccagtcttgcaaggggttaatttgaccatcaaccgaggggagtttatcgtcatcgccggggcgactggcagcggtaaaaccacgttaattaatcatttcaaaaaagaactgctccccaatggccaccgaagcggcaaggtattggttaagcagcaagccattacggatctttccaaattagccagcgctaaaacaattgggtacgttgggcaagatcccactactcagccgattatgacaacggtgattgacgagctggcgttcggccttgaaaatatcggtatcaagagcgctgaaattgaacggcggatcgccgaattggctaattatttgggcctggacgaactactgcaccaagatatgcatgaactgtccggtggtcaattgcaactggttaatttggcctcggtgttaattttgcggccggaagtgcttttgttcgatgaaccgactgcccaactggatccgctttccagccggcatttttttgatgttttggaacggattcatcaagagctgggaatgacgattgtaatgaccgagcataacttgggaaccgcattgggattggctgaccggatgatcctcttacaaaatcagcgggttacttttcaagggcagccggcagtcggcattccgaagatgatgacagatcccgatctggcggcttttgtgccagctgtgtcgcggctatttttggataatcatcttgagacaaccgggctgccaatttccgttgccgccggtcaggcagctatcagcaagcaccacctggagttcaccgctcacacggaccagccgatggtcgtcgagtcgtcaacgaccatcttagcagccaaagagatctcgttttcattcgacaaacaggtaaatgtggttgatcatttgaacttgcaattacctgctggcgactggctttcgattgtcggcaagaacggctctggcaagtcaacgctgttaacgatgctggctggcttgcgagttccacagcatggaaaaattacttttaacaatcaaaaggtctggcggattccaacagcagccagaatccagcagctttcttttctctctcaaaccccggccctgcagtttggggctgaaacggtccaagaggagttgcaccagcaagctgccgaacttcagctagaatttcccgacaaacaggttaaaatgatagttgaccgattgcaacttaacgatctgcttgaccaaagtccatttgatttgagcagcggccaacaacagctgttggggattgccattgcgttactggctaacccgaaattgttaatcttggatgaaccgactaaggggcttgatccgatggccaaacaagctttgggacagttattgacgaccatcaaccaggctggaacgaccatcctgatggccagtcacgatatggaattttgcgcggcatactcactgcactgcgccttcatgtttgacggccatttgaacacagtcttaccaaccagatcgtttttttctgggaatttcttttttaccaccgcgattaatcggctgctgagaaggcaggtgcccgatgcaatgctggtgagtgacgttagattatctgaagggacgagtgaacatgtcgaataagcggcgagccaaagtgatcggtcaaatattgctcgtctcggtgttgatcgccgggtttttggtattgacgacgttactgaaaaataagcattttttgttgtttagcttcatgcttttgttatgtagtattttgccggcctattggcggtttgagcgcgagccgttaaagacccaaacgctaatgtttttggcgattctgattgccttggcggtcgccggcagagtgccgttcgcctcgcttcccagtgttcaggctgccagctttgtcattatcctcggcgggatttcgctgggaccggagctggggtttgtgaccggctcgaccaccgccttagtttcaaatatgttcttgggacagggaccttggacgccgtggcagatgtttgcctggggattgatgggcttgactgccgggctgattggccggactcagcttcgccacaaggtaatgccaatgattatctttggcggtgtctggggatttgtctacggctggatcatggatctgtggtttgccttggcatatgtcaatccgctgaccatgaagtcctttattttggcctttaccgccagcgccggtttcgatcttgtgcactgtctttccaacgttgtcttaattgcattgttgtatcgttcctgggaaaaattaattgaccgactgaatcggaaatataattttttaccaaccaaaactcattaaagggatggaatctatcatgaaatcaatcaagaaattaatcaccttatcgatgactggcctcttattggctggtgctgctgcaccactcacaaatgtccatgctgccggcgccaagactgcttctagttcttatcaggcttcaaaggccaaggccagttacagctatgccaagaagatgctggctaagaatcgaactggcttttctggtaagacaagttacatatttagtaaaaaggcatatccaacaaccggtgccgtctatggctactcggactttctcttgggattgaaagggttgggctacaaatttaccaaggctcaacggaccaaggttgccgacagtttggtattgaaccgtaagagtacggctgccgatttggcgaccgcaattattgccacccgtgccgttggtttgaacccgcaaaagctgcatcaaaccggcgctaaaacgaacttgaacctggtcagcgcgctttatcaccgttcgatgaccaagcaaactgtcaacgttcaaagccaggcgctgattgctttatcaactggttcgtatcaacgaccaagcaatgccaaattttccaagaccagcttgagcaacgccatcgttaagaatcagttgagcaataatggctgggcgtataataatcaagctgccagtgctgacagcgacaccaccgcgatggcagtaacggcccttgctcggagtaaatcgaccagttccgccgtcacgtctgcaatcacgaagggccagagttatctcaaagatgctgtctatccaaacggggcgtttggttatgcttataagggcaagactttcccgaacgctaattcaactgcagaagcgatcattgccttctcaaccaaacaaaagacggtcaaattggtgaatagcgtcttcaaatcaggccagactacctctccaatgcgggcaatgatgagctacgttcggtcaaccggctcgattaagggggctgctactcaaacgttaggagtcggccaggtcaatttggcaaacgccgcttatcggcaagccttggcacaccgatcggtttattcaattaagtaagattaaaggatgagtttatgaaaaaagcaattggaattgtcattggtgtgattttggtgttggggatggcatttggcgtcagggaggtcatcgcaaatcaggccgcccagcatcctcgaaccgagaaagccgctaagatggattcgggcagtcagccaaaggccacctcaagttctcaagtgagccatccagttaaggcgagaaaagccaaagacaaaggttcccaggcaaagcatcaatcacaagccaaaaaggccagtcaatcaagcactgctgactcgtcgtcaagtagtcaagttaccagtaacaagcccagcagttcgagctcgaaatcacagacaaaacaggcagtaaccaataagcctaaatcgacttctaagcagtctcggccaaagcaaaaagcctcaccagcgtcaactggtaaggcttatctaaaggtttccggatacaaaaagctgttttattctggcaatttgcacattattaagaagacgaccgcgtttacattgctccagcaaaccaagctgaagatcacctacaccagtagcccggcaatctacgtcagtgccatcaatgggctgaaagaaaacgacattaaggtcggcagcggctggatgtactcggtgaacggcaagtacgttgataagtcagctggtgataagttgattaaaccgggagataaggttcactggtactttacgacggagggattcaagtagagcgcgacaagcaacgggtgatgcggtgtgtaaggctgaaaagattaaaatcctggtcttggatttaaatcttttcagccttacacaccgcatcagttgcgtcggagcgtgttttcaaagcagaagggagcaccaaagagaataacaaccgtgctccagcgcgccagaatccatttcaaagcaaaataaccctaactacaccactacaaagccggcagcgatgaacaaatttcgttcatcactgccggttttgtgttatcaattattatcggacttgagcagttaaagcagtcaaaaaatcggtgacatcaccgacataggcaaagtctgactcatcgaaaatcggggcgtctttgtcaatgttgacagagacaattttcttggcatttttgataccaaccgtgtattgaacagcacctgagattcccaaattaatcaacaggtcggctgagaggctggcgccaccaatcccaatttgatcatcatgggtgaactcgtcttcgtcagtgagagggcgagaaacgccaaccattccgccaagcttggcagctaaatcctgtgccagttgaatattttttgcgctgtaagcgcctcggccaagggcgatcacgactttagcatcgtcgagtttggaggagctgttgatgatcgggtcagtggcgatgatttggctgtttccttctttgtggaaggtaaagctggccttaaccaccttggtctgggaatcagtcactctttcagcacggaaagtatttggccgaaccgttaccatttgaggccgcttttccgggcagacaatgtcacacatcacgttgtcgccataggtcggtttgacctgaaccagtaggtcattttcgtaaaaaatatccaaacagtcaccggttaagccagtctggagtttggcctgcagccgcggcgcaattgatcggcctaaaatggttgccggaaacaagaggctgttggggcgattttgatcaagtacttggaatagagcatcagcgatttcttcatcggttgcgttagtaaagtgatcatcgaccaaagtttcaactcggtcgggtccataagcttgtaggctattttcagccttgattgtcgaggcttcaggaagcacggcaaccacttttctgccgtcagcaatggctttggccttggtgatcaattgcaggctggttggttcgattctgagccgacggtttcaacatatacccaaatttcgttattatccatttttgtgctcctctcagtccaattgactcaagagttcagaaactgcttgagcggggtctggtgacaatgtgactgtttgtttaacatccttggttggtgcataaactttggtcactttcgttggtgatccagcctggccaatttttgccaggtcaaggttcaaatcggcttcagtccaagtggtaattggcttttcaaaactttctttgatattgactggcgtttcataacgcggcgtattgagttctttgcggacagtcaccacagcaggcagggtcagcttgatatcttggacggcggagtcaagttggcgtttggccaccagtgtcttctctgagtccaaatccaaggtttctgcaaaagtcacttgggggaactgcaagaattccgccacaatcgggccaacctgaccagtgtcagcgtcgacagactgtctgccgaataggattaagtcgacatcgccaattgcttcgattgctttggccagcgtgtagccggtagccaaagtgtcagccccaccgaatgcccgggaactcaccaaaacagcccggtcggcgcccatagccattccatctcgaagtgaggttgtgtaactatccggccccatactgagaaggataacttcgccaccggcttgatcacgaagctgaagggcagcttcaattgcatttttatcaaatggattaataatgccctggattcctgaacgaaccaggttatttgtgtttggatcaattttaactgaatcggtttctggaacttgtttaatcccgacaacgattttcatagtgcggactcctttacttggcaatctctgcgttggtaatttctaaattcatcttttcaatggtaccttcagccaattccattgctcgggcatctctgatgaggtgttcgactggatattcatggctgtatccatacccgccaagaatctgcagggctttatcaccggatgcaacagctgatcggctgccgtacgattttgccatggcggcaacttccgcatatggcttgttggcgaccttgttatcggcacctttctgatacagcgcggtggtgttttctttggcaattgcgatatcagcgatcttttcctgagtgacttggagttggtagagcggtgtgtccatagcctttcgctctttggagtagttcacggcggtttgtagctcgtgttccataattccggctagaacggcgcccatcaaaactcgtgcgtcagcgtgggcattgtcgccaatttccaatccttgtccgattcttcccaataaatgactatcaggaacaaccacgtggttaaggacaacttcgccgacaggcacgcccttgaggccaataaaatcttcccgcttgccgaatttgaatcccggcatgtccttgtcaacgacgaagacggccatttggtcatcctcagtcttagcgaggacgcagtagacttctgctaggccaccattggtaatcatgattttgtcaccggtgatcacccagttgtcaccctgtttgattgcccgagtggcgatgcccttaggattcgagccgccggatggttcggtcatcgagaaggcaaaaattcgtttggctgcacttggaaggtattcgtcattcaatgatttattcccatatttgataaactgttcgatcgttttgaaatggccttcaagagttacggccatgctggcgttacctgtggccattttctcaagggattcggcagctgcttggtaatcaaaggctgcaccgccatattctcttggcagggtgatgccaagcaagcccgtgttaacgaccttttgaaataagccgtccggatagttaccggcacgatcaatctccatatcgagcggtgccaattcgttggccgtaaactccttaatcatttgaatcagcattttagtttgatcatttgttatcgacatattgagtcctcctgtgcatactttcacaatactttatattccaaaattatatatcctaatattcctaatgtcaatatataaatggaatatttagcaatcttatttggcgtcacattatataatatggtaatattaagttattattttatccgaatcggccaggaggcttgataatagtgaacatccaaagatttattgatcgcagaaaagaactcggttattcccaaagcgagttggctaaggggatttgtacccaggccacgatcagcaaatttgagaacaacggcaaaatgatctccactaagatcctgacgcagttatgccagcggttgggactttccttgaacgatattttccccagcgaggccgacagtgattcagcggttcgagcggaattgcggcgggccgaatttgatttaattaccactgaatatgatgatgcgttgggaattttacgatcgcttgaaattgatcaaattgatgataaacaaatccaaatggaatatttatttatccgcggatatgcactggctttaagcaaacgagatgttgatgaggcgattttttgcttcgaccagattttgaatggctatgacgaggcccacacgacggtttattcaccgctggcatacgtggggatggggatttcctaccaacaggctggcaattttgacaaagctgagttttatttttccaagatgccggaacggttgaagaccaatgcaaataaagacgttgattcggtgtggaaatcattgacgatgctgttttacaccggcaatttttatgcggccagaaatgaaatcgagatcagtaatatgctgctacagtctttgattaatctcagttcggatcggcacgtaactttttatgtggctcgggctcagtatcaattggcggataacgaatattcggtcaatggcaaaacccagcgcttctccgaacttattagtgacgcctttgcgttcgcccgatttaatcggaatcggaatttaattaagcagattgatttgtatgctaaaaaaagagtgtagagtgtgaaagaggacgtttagcaattgaaatttaagcgccgctggacggaaaccgagtcaggttttcggctggcggcgcttaaatttcaattgctgtcctctttcacacgtttaatccaaatcacagtaaaacaccaggaaaccgagtcaggttttcggctgaagcggcttaaatttcgactgctgtcctctttcacacgtttaaactaaataacagtggagctaaagagaggcccagacataacttacaattagttgtgtccgggcctctcatttcgtcaaatattggtttcgcaattgccgaatatcatgattcgacaaccgcatttgctgatgtaaataatgcttcattgtgccatcacagtggtaaatcgctgaataggcggcattcaaataggctgatcgagcggtttttgaacgtttcaggttcctgagcacggttgggttatgcgtataacgggccatctgtcgatattctttggccgtcgttttcttcagataatggttcgatgccaaatagtttttcataatggtcgttttgggaacgccaagacttgaaagaatcagcatggtcgctacaccggtgcgatctttgccatatgtgcagtgatagagaatcgcaccggatctttgcttgagcagataatgaaacatcgtgcgataagccttaacacagtgggactcaagaaccattttctgataaaattgttccataaaatttggctgtttggcagctaactgaccggcatactgagaagtcgtgtggacgccgaaatttgggcttctcatgacggataggtggagatgacgaaccccagaaattttggcatctggtgttcgtttgatttcaccacttgagcggaaatccaagatgaccttaacgtgctgcttataaagtagccatttatcgtgatgatttaatcgggttagcgcagccgatcggatgagtcgattttggcgaatgtgctgaccatttttcgtccgaatcccaccgagatcgtgggcattgggcgtggtcgtgagatgaatgggggagcctaatgaaggagtgttgttggcagaacaaatcgcaaaattagcagtgagtatcactgtcactagtaatgtccgactcatgatttgactcaatgacttcatccactcacccccaacattcattataggactgggcagtcatcatgacagaaatttttggatgtgggccaaatccgcctggcgcttttgtggtgattcatcttcagcgttgaagttgtgccacttgattttcttgagaccgatctttttgaatgtgcccgtggccaaggccttcataatgggattaccatatttgagtttatagagaaacgttggtgtgccggcaattgtgaagatccggatgattggattcttttccaggaccactctgggatgcatggataccgcccggttcttgctaaaaactttatcaatgaaacccttggtcatcgccggcatcagctcccaccaaattgggaaaataaaaataatttcatcggcggtttttaggcgttcgaaataacggtcaacttggtcgttaatcggtgtccgtgttcgccaggcactcaggtcttttgcgtgcatcaccgggtcgaagtgatcttgattcaagtcgatgacatcaacctcgtggccttgggcagttaaataattgatcgtttgtttgcaaccgctgcactatagctgcgatggtggggctcgttatttgcagccgacagggtgtaagggtggtcaaatataatgacatatttcatattagaaacctcttttttaaaattgacagtttgactttccaaaatacattccaaggaatataattagtataagctccgatgatgaaaagtcaatatatattccgaggaatttaaaatgaaaaagaaaaatgcaattgaacaaatcaagaaccaactagaaatatttagaagtcatgatgttgatcgtgagatcctgacggccatcaggcaaaacgatcggttaaacgctgctctggccaatggcattaccattaacgatctgcatattattcgcgctgctgctgccaaggatggtgtgaagatttccgcgattgtcgaccaggtacccatgacgcaaggcgccgtttccaaagccgtcaacaagctagctgaaaggggcctgcttcaaaaatcgcaccaccctgataaccgcaaggacacgtttgtagaactcacggcgcctggggaaactattaatcaaattcatagcgactaccatggtcaagaagaggccaaactggctgagttagccgacagttattcaaaaaatgaactggagatgattgcagaatttgtcaccagcctcaatcaaatccggcaaaataattctgaattgaagtaaccggtttcttctttactatatcaaaaactcctgtctactgcttataaaaagaaagttaggtttccctaattaaagatttacaagtctagaaactatgctaccattagatttgtacagaagataaggaggtaatgggatgtcaaaagaaaaaaagtcccaaaaggaacatttgattcattacgccaatgggccttcactggaagaaattaacggaaccgtggttgtgcccaaaggcaagggattctggcgtacgctatttggttattccggtcccggcgcgttagttgcagtcggttacatggatcctggtaactggtcgacttcaatcaccggtggtcagaattttgaatacctgttaatgtccgtcatcttaatgtcgagtttaattgccatgttgcttcagtatatggcggctaaactgggcattgtgactcagatggacttggcccaggcgattagagcccggacaagcaaatcgctggggtatgttttgtggattctaaccgaactggcaattatggcgactgatattgccgaagtcatcggtgccgcgattgcgttgtatctgttattccacattccgttggtcatttcagtatttattaccgtatttgatgttctgctattattattgttgaccaaaattggcttccgtaaaattgaggccattgttgtttgtttaatttgtgtgatctttgtggtgtttgcctatgaagtgatcctgtctgatcctgattggctcggggtctttaagggcttggttccaaatggcgagaccttctcttcgtctcctcaaattggcggtcaaacgccactgactggtgcacttgggatcattggagcgacagttatgccccataatctgtatctccactcagctgtttcacagactcgtaaggtggatcacagtgatgaagaagatgttgcccgaaccgtttgtttctcaacttgggattctaacattcaattatcaatggcattcttggtgaactcactgctattgattatgggagttgccgtcttcaagagtggggcagttaaagatccgtcattcttcggactgttccaggcactttcggatccttcgaccttaagtaatggtgttctgattacggttgccaagtcagggattttatcgattttgtttgcggtcgctttactagcgtcaggtcagaattccactatcactggtaccttaaccggacaagttatcatggaagggttcatccacatgaaaatgccgctttggatgcgccggttggtgactcgtttgatttcggtggttccagttttgatttgtgtgggtatgacgagtcgtgaaaccccgattcagcagcacgaagcgttgaacaccctgatgaataattctcaggtcttcttggcgtttgccctgccattctcgatgctgccgttattgatgtttaccaataactcgttagaaatgcatgaccgtttcaaaaactcgtggattgttaagattcttggctggttctctgttatcgccctgacgactttgaatatgaaaggtcttcctggccaattcgaagcatttctaggtgatcatccaacccagagccaaatttcaatggctgataatgcctcgtacgtcgttattgtcttggtcgttgctttattggtatggatgatttgggatatccacaagagcaacaagcgttttgaagcagcagctgccgaagctgaaagcaaagcagccgaggcggagaaataatagtataataatcaattgaaagagatttcttttgtacccaaataattcatcatcaagaagggatgttacaaaatggcaaatactgaaggcggtcaaaaattcgatcgaattcttgtgggtgttgatgattcggaagatgcccaattagcatttagatatgcaattcgtgaagctcgtcaatccaatgcacgtttgatcattacttcaattttggaagacgataacgttaacgttttccaagcattaagcaaagattttgttcatggggagcgttcagcgcttgccaagcatattgaagactatcggcaattagctttacgtgccggtgttaagcaagtggatacggtcatcgaggaaggcgatcccggcgagacaatcgtcaaacgggttattccggctaccaaggccgacctgctgattgtcggttcactttctaagaccggtgtgcgtaagtactttggttcgcaagcagcctatatggctaagtactcaccaatctcagtgatgattgtccgttaatcggatttaaaaatgattttaaaacaggatcgggaagaatatttccggtcctattttgttagacactagggggaataatcttggagttaacagaaaaaagccgcaggtggttcattgccacattactgttgggaacatttacgatgtcaatcagtcagtcgtcactatcgactgcctatccgacatttatgaggtattttgatctgccggccagcacgattgcttggctgacgacggggtttatgctgattatgtcagtggttatgccattatcaccatggctgatgaagaactttcgatttaagccattatatctttcattattggtaaacttcgtcgttggaaccttgattattatctgggcaccgaatttcctggtgatgatggtgggtcgattaatggaaggattcagtgttggggtcttatttccatcttatcaatcgatcatacttgaaatcacaccaaccgatcatcgtggcagtgtgatgggcactgtggggttggtcatgggatccgcactggctgttggacccatcatctcgggggtcttattgcaatttttcccgtgggaagccatctttgcgttcttcttgattattctgacggtggtctttttgttggcactcaagaccgtcattagtccgttgaaaattgaatcaactcagtttgattttgcttcagtcttcatgtcgctgggaattattggcttattgtactttatcaacgaaatttctcatatgactgtcactagctactggaactgggggattttattggtttccttggttctgctggtcttatttgttcgccgacaattgcgcatgccacagccattattgcgactggatattttgtcgatcactaactttgatttgggagttttattaacttcattgtcctatatgtccttgatcacggtcaccattatcatgccgctatactaccagcagatactgggattgacgccgttatggtcaggcctggcactggttcctgccgcagctatcttgtcttggttaaatcgacggagtggccggctagcggatcgcattgggtttaagccagtcattatgattggttttggattattcatcgttggctgggcaggtttattgttgctatcagggttgaaaaatatttggattgccattctatgttcaattgtaattgaatctgggaatgcctttgccatgatgccggccaccacgctgggagccaattctttaaccaacgatttgattccccacggctcttcgattattgcgacgattaggcaaattttggggtcgaccgcgattgtcattgcgacagttgtattaggagaccggaatttcaacggcgtgttcctcacctttctcattctggaaatcattgccattttcttggtcctcaaaattaaggatacgcaacagcaggcgggcaaagcttaatttggctttgtgaaatgaaaactattttcacaagtaatatacgttaaccattgcgttcgtcaaccactttaaaaatcacaatgcattttgttgtatctgttttcatggcatgctatcctatatctggatgtaaaaatgtctaggatagctgaagacgttacggatttatccaaattttaggaggtcatataatggcatatcggactgtaaacccttacaacaatgaagttgtgaaggagtacccatttgcgactgaggacgaattacaatcagccttggcaacgggtcatgatttatacgaaacgatgaagaagcaagatatttctgagcgagccaaaattctgcataacgttgcttccaagctgcgtgagcactcagatgaattagctcgtgcatgtacgattgacatgggtaaattaatcggtgaatcaaagggtgaagttgaactggttgcgatcattgctgactggttcgcagatcatggtgaggacttactgaagcctgaaaagatcgataccattgcaaccggtgatgctgaaattcaacatcacgcaaccggagttgttatgatggttgagccttggaacttcccttactaccaaatcatgcgtgtgtttgcacctaactttatggttggaaatccaatgatcttaaagcacgctgccaacacgccaacatcagctaaaatgtttgctgacgttgtcgccgaagccggtgcgcctaaaggttcgttgactaacttgttcctttcatacgaccaagtgactgaagcaattgatgaccctcgtgttcaaggggttgccttaactggttctgagcgtggtggtacagctgttgccggcgccgctggtaaagcgcttaagaagaacaccatggagcttggtggaatggatccatttgttgttttaggtgatgccaacatggatgatgtcaatgacattgcatggcgtgcccgaatttacaacactggtcaagtatgtacttcatccaagcgattcatcgtgatggacaatgtttacgatgaatttgtggagaatttgaagaagaagtttgctggtttgaagcctggcgatccaatggatcctaagacgaccttagcaccaatgaacaccgaaaaatcaaagaacaagttacagaaacaattggacgatgctatcgcagctggtgccaaagttgtttatggtaatgaaccaattgacttacctggtcaattctttatgccaacgatcttaacggatattgacaaagataacccagcatacagtgaagaaatgtttggtccaatcgctgctgtttacaaggttcacagtgagcaggaagcaatcgacttggccaacgacaacccttacggacttggtggcattgtctttgccggcgatgctgatcacggtgcagaagttgcctcacaaatcgaaactggaatggtctttgttaacaacttcatgtccaccttacctgaattgccatttggtggggttaaactttcaggttacggccgtgaaatgagccacattggtcagatggcctttgttaacgagcagttgatcgtcaagactgacaagcctaacatgggtaaccttgccggtggcttggttgcacttgatcctcaagaataatgaacgtaaaataaattgactgaaaagtaaagaagtcgggagataacgttttgttcgttacctcccggcttcttttgcgtgccattgttattttgtttaaatcctaggatcaagattcttcgtgcgatgctcttggcacaattacctgtaaaaagtcactcttggttgtgacggtaattggcagagacatcgctggatccccatcgattctggcctgaatgtcgcgttttgacaggttatctattttaacggttgtggttttaaaatagcgaaccccctgggcatttttgagattgccggtgatgaaataactcaagtaggtgagtagtttcatgggagtgaagctcttcagcaagaagacatggagataatcatcgtcgtaggacgcatccggattaaaggcgatgaaaccaccaaccgaattggtcgtcgtgatcagtagaatctgggctcgcaagacttcggagcgatcattggctgtgatttttaatttgtaagaacgattggtgaacagctccttgaagcctttgaccaaataaatcattttgccaaagcgcttcttttcgtcgtccttgacgtttcgagcgatatctgccaatcttcccagggtgaggctgctgaccattggtgttttccccacagccccgaggtcgacctctgctggtgagccatccaacagattgttaatggcttgatcggtgttcagagggatgtgaagggctctggcaaaattattgatcgtgccgccaggaatgattcccagcggaattgattggccagccttcaagaagccctcacaggcggtattgatcgatccatcaccgccaatcgtaatcaggcagtcatagttttcgggtgatttttgggcctgtttgaccgcatcatcacgtgacttggtttgactaagggtcaccgacttgccattgctttccaataaggattgagcctttttggcaatcgcttcgttgtcgcttttaccggcactgccattataaataattaaatattttttcatgttgcacctcctcaaaggaatgattcggatgacaactttattatattacgcttttggggaatggtcgtctttggggattatggttaacgatccgttcatgaccggcgacgttgcatcaacgatgtgggggtcggtgaagatctgcaggaatttcataaaactttcagctgtattagcttcgttgaggtcctttaacggcagccaataatttttgccttcctcagactgcttgagggtgcctgagaaatgactggtgcggaagagaaatccgagccggcggtaggcagggctttcgttgaaccattcaacagttccacaggattcgagctgactgaccgtcaggccggtttcctcaaatacttctcgaaccatgccgtcgtaaagactctcacctttttcaacgtggccgccgggaaaagtgtggccaaatttccaggcgacgtcggttttatcttccaccaagacttcttgagtggctggattgtaaatcatgcacatatttaccaattcaattgattcggttctggaataggtcatttggctgcctcccgctcaacttcttcgttgacactgaattgtggagtcactttaagggctttgatccgattctcgccccattcatacatctgattggcaatgggcatcagtgattgaccgagctcggtgatttcataggttacctttgtttgagatcccgagttgacatgccgggtaatgaggccgtcttcagccatttcccgcagctgattggtgagcactttgtgggtgactttgggtaacagccgcattaattcgttaaagcggtaggcgccgtcagttcccaagtgaaataagatgaccaatttccatttgccgctgaacatcgataaagtgagctccttggaacagttgtagtcaccgtttttcagacggtctttgacatcttttctgatgacatcagtcatttgtatccctccaagattttaggcacctgaaagtgcgttattgtatcattttgatacctagtataaagtagatagtatcttggaacaagaaaggatgaatttgatgagtaaagtagctgtcatcgtgaccaacgatgttgaagatattgaatacacatcaccggttgaagcactcaagaatgccggccatgaggtggtaaccattgaaaatgaagctggcaatcaaatcgtcggcaaacacggcactaagttgactgccgataagggaatcggggacgtgaagccggatgagtttgacggcttattgatccctggcggcttttcaccagatcaactgagagctgatgatcgatttgttaatttcgtcaaagcctttttgatggacgacaaaccaacttttgcgatttgccacggtccgcaactgttcatccaaaccggcttgacgactggtcggacaatgaccgcctacctgactgttcgaccggatttgtattatgccggcgcccgtgtgaaagatcagccggtggtggttgaccgtaatttggttaccagccgcactcctgatgatttagacgattttaatggtgctatgctggctattttgaagaagtaattgaatttaaagtaacttgactgcaaaaagaccggaacaaggcgcttttcaacgcctgttccggtctttttgctttttatgttatgaatgtctaactcaatgcaaatgagggtccttattaggatccagtccacctaactggcctctgaattccttggaatacaggttcaaatctgaacggtaggcgtcaaggttgtcgctcatgtcaacggtataatcaacttcttcaccgtgctcacctttatccaaaccaagcttttcttctttacggtcaactcgcattggcatcactaaactcagtaatttgataatcactgaagccgcgatggtaacaaagataatcgttgccaaagttgcgacgatctggacggtaatttgatgccaaccgccgccataaaaggcgccattgtgggcaacaatcgggttgacgctcttggtagcgaataaaccggtggcaatactgccgacgatcccgctgacaccatggcagccaaaggcatccaaagcatcgtcaacaccaattcgatctttcaaatagttaacgaagaagtagctggcgaaagttgagaacatgccaatccaaaatgatccggcgattgttacaaagccacaggcaggggtgataccaactagtccacaaagcgttccggtacaaacaccaaccagggttggcttaccgctgataaccatatccaagatcatccaggtaaccattgcagtaccggttgacatggtcgtcgtaatggttgcctgagccgcaatgttgtcaacaccgagtgctgaaccggcattaaatccgtaccagccaatccacaagatggtggcaccaagcaatacccatggtaaattgtagtgggtgtgagggatgtcgccgaatttaacccgtttccctaagaaagcggaaaggacaaaggcagtgacaccggcattaatatggacaacggttccgccggcaaagtccaatacgcctaatccataaaggataccgtgtgggctccaaaccaaatggaccattgggtagtaaatgataatcgaccaaagaatcaagaaaaccaacaaaaagttgaatttgatccggccaacaacggcacctacgaataaggcaggggtaataatagcaaacatcatttcaaatactgaaaaaatcccagtcggaatcttggttgccgtcaatgaagtcagatcaacgccattcatgaaaaagttcttcacggttccaatgactccgccaatgtctccggaaaatgataacgagtaaccaatcacgatccaaagaacaatggcaacaccggtcataatgaaaaccgacagcatcgtgttaaccacgtttcgttttgaaaccaggcccccatagaaaaacgccaatccgggagtcatgaataagaccaaaatactggataaaatcatgaacgaagtatttgcagcattcataacatcgcttccttctcttttaatgtcataaattctaacatcatatttttggaacgtccagcactttttgaaattggttagaaaattagaatgtatctaatcatgatggaaacggtgccaatggcgctgggtaaggcgtctttaagatatcaaattttattaaaaaggtgaagcccgctaattggtatatgtaattaaaactaacattaagggccggaacacaagtgctgcttcaatgtgttccggcccttattacatactctgtatcacgatattctttgttaatttaactcattaatggcttcaggaatcggttcattcccggtactcatctcaatgacttctttgatgccggcatggttttcgactaaaccaattaatacgtcggcgacattatcgatgctattttcattggtgctataggctcccaaagtcactttgcctgacccggttttttcaaccaacgcggttggctggaggattgtatagtccagattggtgttgtgaatcaaccattcgtcagcatagtatttggcgatcaagtaattctcaagcggagagtcggcgaattcgtctggtgacaatgatcccttggaactcagcatgacaaaacggctgatttctttttcttcggctgcctgcatgactttgacggcaccatgtaagtcaattttaagcaggtctcgaccacccgatccggcagtgaagataattgcatcggcttctggtaaggcctctttaatctcatccatcccgtcattgagatccaatttaaacggcgtcacgttctcagacgttggcactttttccggcttgcgggcaccggcatagatttcgtctgcagaatttttggcgagtttggcgacaacgtttgaaccaacccggccagttgcaccaatcacgataattttcattgttggaatcctcccttatccttattagctcaattatggtagatataagaccggaatgcaaaagaaagattgacattggcctaatctttcttttgcaaatctaacgtactaagcaggcagtgggtgatttttaaagcaacgattagtgcgacaaccagaatcacgatgaccaggggaaggtcgatcgctgaaagtttaacgatcgacatgctctctgaaacgtcaccatcgcgaatcaccgaaaaaccaaaaaatattcgccatcaattaccaaacaaaatttcaaacttgatccacgtcaattctttatcggccgaaccaccatatactaaagacatcaattgagaaatggagcgggagattatgaaattccaaagatatattaatcaacatacaaatcaaattacactgataacggcagtattaattggcgtaggcctcttggggaaagttgttgacagcgatatggtctacacggtttcatttatcgccgcttcaattatctcggctgtgccaatcgttcttcgggcagtttccgcactccgatttaaaacgatcagcatcgaattacttgtcagtattgctgtgattggcgctttcatcattggcgagtacaatgaatcagcaatcgtcactttcttgttcttatttgggacgtttttggaagacaaaacgttggccaaaacccgccactcaattaaagatttgacggaaatggcaccgactacggcaatggttgtagacgatgacggcaacactgaggagactgatgttgactttgtcgacgttgacgacgtcgtcttggtcaaagccggcggtcagattccagttgacggtgaaattgtggatggatccggtcacatcaacgaagccagtattaccggcgaatcaaaattagtcactaagggcactggcaatcaggtattctctggcaccatcttagacaacggaacacttaaagttcgggcaaccaaggttggcgacgacaccacgtttggcaaaattgttgaactggttgaggatgctcaagacaccaagtctccagcggaaaagtttattgacaaatttgcgacttattacactccggcagttttgatcattgcactgattgtgggcttggttaccaaagatttccgattagcgattaccgttttggtcttgggatgccctggggccttggttatcggcgccccggtttcaaacgtggctggaattggtaatggtgcgaaaaacggtgttttgatcaagggcggtgaagtgatgaacacctttgccaatgtcgacacgttggtattcgataagaccgggaccctgactgaagggaaaacggcggttactcagttcaaagactactcaaaagaccagttggccttgcaaattgctgcagccgttgaaaagcagtcggatcatccgttggcacaagcggttgttaaattctcagctgatcatcatattccgtttgatgacgttcaagttgccgatgctgacacagtcaaaggccgtggcgttaaggcaactgccaacggtaagaatgttttaattggtaacttgagaatgatgaacgatgaaaacgttgatttgacgtctgagcaacgtctagacttggaaaacatccaaggcgaaggcagctcaacggttatcgttgccttcgacgggcaaattcaagccattcttgggatctcggatgtgattcgtcaaggcgttaagcaaagcctggcaaccctcaagtcactcggcatcaagaagacggttatgctgaccggtgataacctgcagaccgccaatgccgttgcagaacaaatcggcatcgacgaagtgcacgcagaacttttgccggaacaaaaagtcgaatacgttaaacaattccagcaggaaggccacaaggttgcctttgtcggcgacggcatcaacgacagtccgtcattggtaaccgctgacatcggaattgccatgggaagtggaaccgacgtggcagttgaaacctctgatgtcgtcttgatgtcatcaggattcgatgaattgatccatgcatatggactttccaaaaaaacggtcatcaacaccaaggagaacatttttattgccattgcgacggttgtcgccctgctgattggcttgattctcggctttatttacatggccagcggaatgtttgtccatgaagccagtatcctggttgtcatcttcaacgcaatgcgattaattaattatcaaccaaaagccgccaaacttgatccagatcaattatcagttggcgaatatgatttatcattaaaacagtaaatgagatggaggttatcaatatgagtaaagcaattttacaattagacgcgctgtcatgcccgtcatgcatgcagaaaatcaagggcgcacttgaaaagcaggatggtgtggaaaacgtcaaagtgttgttcaatgcagccaaagtcaaaactgattttgacggcgataaaatttccgcagacaaactgtcagacacggtaactgatttaggctatgaagttcaatcaatgaaagtgaaataggtgaagaatatgacaacagcaaccccagaaaaattatttgaagcagaagttaagcaagcagatatcgaccaccataccccaacggctggtgcgatgactggccacattgttgccaatttggaagttttatccaacaaactccagatggcaaaatggtatgtgaagggaatgtcggcccaacagctgaaagtcctattcggcgacttacttaagcaggcgtatgaccaaaaggatgccttgggcacggtcttaatcgatgaagcgttaatcacgccaagtacccaaaaggaattcacggagtacaccatgctggaagaaaatggccagaataaatatgaatctgcagagtggctggtcaacgacttcgtccatgactatgacactgagaacatgtttgtcacccgggcaattaagttggctgaaaaagaagaccgtccagtcttggcacaacatttggttggcgtactgcgggataacaaccacaacatcgctaccttgcaggccttacttgggaagacaccgcgagagggcttggacgaggaagacgacgaagattaatcattaacctagatacgaaaaaagttccgaagcaaaatttgccccggaacttttttaatatcattttttcgaattcaaagattcaaacaaatcagcacgataacacaggcaatcgtacttgccaggatccaccagccaacccgataagctgtccgctgataggttgaaatttgttcctgacttaatttatcaaaatccggcatcctaagtgaggcattttgaaacatgctagtctgcagcagcgtatagtcttttttgatcagaagctgatagcttgtccatgacaataccagaatgaggccaatgagtgcaacattgattgagacaaatattaacaggacgcagatactgattgcactagtcagtataatccgccgagttctcattttcaccactccttaagggcacactacttcactggacgagtgatggcagattgccatcaagaacaaattaccagagatattcaactggatttttgatgtgttgatcgtaaacgtcacggacaatttgcatctgagcatcagtcagcgcgggtagatccgctgcagtggtgttgcgctcgatttgagtgggattacttgcaccagggatgaccgcagaaacggcgtcatacattaggatgaaacgcaaagccattgctgcaagattatcggttcccaaacgttgcttcagttcggcagcagctttaacgccggtcaggtagtcaacgccggaaaaggtctcacctttatcgaactgttcaccatgccgattagttgttcgatgatcttcgggtgcaaacttggtgtccgcggtaaattttccggtcaaaagaccacttgccagtggaacccgggccaaaatgccgacgttatttttcttcgctaagccaaagaagagatcggcaggacgaaggcgaaacatgttgaagatgatctcgacagccgagatgtcataactgagggctttgatgccttcttcgacccgctcgacactgacaccgtagttctgaatttttccagcttgcttgagcttgtccagttcaaaaaggtttcaggcatgtagtaattcatcattggcgggcagtgcagcagcaccatgtccaatgagtcgacacccatgttttgcaatgactcatcaacgtaccggtccaagtgagtcgggtcaaagtgcttaatatccaagggcatttcttttcggccaattttagtcgtgtagtgaacatcaggatgattcctgacaaattcacccacggctttttcactttggccatcttggtagccatcagctgtatcaaagaagttgacaccacgatcataagcttcctcgagtgtgtcccgagcatctttagggtcaaacggggtgccccattttccacctaactgccaggtaccaagggaaacctcgctgacactataaccagttttaccaagtgttctgaatttcattagtgttacctccaaatagcaatctacttgcttcaatcataacatctcggttgatactttaactaagcgtatttggtggtggacaggtccacggtcgttaaaaattgaccatcttttgaaacttggacggctccaaacacgtaaattaatcaaatatttttggtaaaagttgcaatatatcgttttaaacacgaacaatgacgttgacttccatgatgatggcaagtatcctatagacaccaaataaatttgaaaaggtgagtggttggaatggcaaacgttgtcggtgtggcaatgggatcaatttctgattggccaacgatgaaactggcttgtgaacaacttgaaagtcttggaatcccttatgagaagcacgttatctcagctcatcgaatgcccgatgaacttcaagaatttggcaagacagctagggacaagggcatgaaagttatcattgcgggtgctggtggcgcagctcatttgccgggaatgattgcagccaacacgacacttcctgtcattggagttccgatgaaaacacgaacattaaatggtgttgactcattgctttcaattgtccagatgccatttggggctccggtcgccaccgtcagtattggtgaggctggtgccaagaacgccgccttattggcagctcaaattttaggaacaactgactcagctatcgcgaagaagttggctgatttaaaagaaacccagagagtggaggccaaaaacagtgagcagcagtttgattaaaactatcttaccgccagctacgattggcattgtcggtggcggccaactcggacagatgatggcactgattgccaagtcgatggggtatcacgtgggcatcttagatccaacacctcacgctccggctgggcaagttgctgatttccaaattgttgccgaatatgacgacgttgactcattgatgaagttggctgaacaaagcgatgtgttaacctacgagtttgagaatgtcgacgaagattcactgctcaaggcaaagaaggtggctgagctgcctcaaggcgtcaacttacttcatatcactgggcagcgcttgaacgagaaaaatttcatcaaggattgtggcattccggtaaccaagtttgctgcggtgtccgatgaagcgtcacttaaagttgctgttgacgaagttggctatccggcaattctcaaaaccgtttccggtggctatgatggtcacggtcagatggatattaattctgccgacgatcttgctgaagcctcgtcactgtactccaaagcggaatgtattttggaagcccgccaagacttcattgctgaagcctccgttatggttacgcgagacttgaatggcaaagtgattaccttcccactggttgaaaatcgtcataagaatcacattcttcatacgacgattgccccaggcagattttccaagacggtccatgctaaagcaaaacagtatgccgaaactatcgctaatcagcttgatttatatggggttctaggcattgaactgtttgtaattgatgaccaagacgtcatggttaatgaactggcaccgcgtccacataactccggtcactacacgatcgaagcctgcaacatctctcaatttgaagcacatattcgaagcatctgcggcttgccgattcctgaaattgttcaggaaaaacccgcagtgatgagaaacctgttaggaaccgatttaacccttgcccgcaatctactcaaggaacatccggaatggcacttccacgattacggcaaggcagagattcgaccacaacgcaaaatgggccacgttaccgtcgttggtgacaacatcgaccagttactgaaatcaaccgacatgttaaagggagaagactaaaatgactgaaattgtgaaaaaagatttgttgtataaaggtaaggctaaggaaatgtacacgaccaacgatcctgacatcatgtgggttcactacatggatcaagtaacggcttttaacggcaagaaaaaagttcaaatggcaggcaagggtcaaacaaactgtgaaatttcagccttgatcttcaaggacctcgccaatcatggtattaagaaccactttatcaagcaaattgattccaacaatcagttggttaaacgggtaaagattattccattggaaacagttgtcagaaactttgcttccggcagttttgaaaagaaatttgccgttaagcatttaatgaaattcgacaagccggttcaagaatttttctataagagcgatgaattggatgatccattcattaacgatttccaagctgaggctttgaaggtggcaaccgaagatcaaatgaatcagatgagggcgattgcactgaaagttaatgaccgccttaaagaaattttttcagaaatgaacattgatctggtggacttcaaagttgaatttggcattgattccgacaaccaattgattttggccgatgaaatttctcctgacagctgccgattaattgaccgcgatacgcaaaagtcacttgataaagatgtcttcagaaaaggcctcggtgccttagtaccagtatataaagaaattcttggccgccttgaaaaagtggaggatgttaaataatggctcttgcaaaagtttatgttaactacaagaaatcaatcttaaatcccgaagcagaagccgtgcataaagcattgaaacggttgggatacagcgatgttcaggacgttaagctgggtaaatactttgaattaaccattgctgacggcaaatccaaagcagagattgataaagaaattaacgaaatttgtgacaaattgctcgctaattacaacatggaaaattaccactatgagattgttgaaacggaggttgcccaatgaaatttgctgtccttgcttttccaggatccaactgtgaaatggacctctacaatgcaattaaagatatcatcaaagaagatgttgaactggtttcttacaagaacgattcacttgccggctttgacgctgttctgattcctggtggtttctcatatggtgactacttacgaagtggtgccattgcccgcttttcaccgattattcctgcattacaggattttgccaaaagtggtcgaccagttctgggaatttgcaacggatttcaaattttaaccgaagccggattactgccaggaagcttgcagaagaacgtttctgccaagtttatctgcaagactgaacctctggtcgttaataatgaccactcgatgtttagctcagcttatcaagctgggcagttgatcagcttaccgattgcgcatggtgacggcaattattactgtgaccaagatactttgcgggaactggttgccaatgatcaaatcgttttcaagtatgccaataatccaaatgggagcgttgataatatcgccggcatcaccaataaagccggcaacgttcttggcatgatgccccacccggaacgggccgttgaagcaatgcttgggtctgatgacgggaagggcgtcttccagtcgatcgttaatcacattaaaagtcgaggggtaatctatgaatagtgtaatggatcaaacaactgaagcgacaccagaacaaattcgtgataacaagttgtaccaatcgatgggattgacagaccacgaatatggtttgattaaagatgatgtcttgcatcggctgcctaactacaccgaagtcggtttgttctcaggaatgtggagtgaacattgttcttacaaaaactccaagccggttcttaaaaagttctttaccaaaggcaaacacgttgtcaaaggaccaggtgaaggtgccggtattattgatattggcgataatcaaggagttgttttcaaagctgaaagccataaccacccttcagcagttgaacctttccaaggcgccacgaccggcgttggtggtattttacgagacatcttctcaatgggtgcccgaccaattgccagcatggacagcttgcgatttgccgaaccgaaaaccgatgcggacaagtattttattcaacaaattgttgccggcattagtgcttatgggaactgtattgggatcccaacggttggcggagatacggcatttgacgatgcctacgcccacaacccactgattaacgtgatgtctgtcggcttgatggatctcgataagattgaagttggtgcagctgccggcgttggtaacagtattatctacgttggccataaaaccggtcgtgatgggattaacggggcctcgtttgcttctttccaatttgattctgaacatgaaagtcaacgttcagccgttcaagttggtgatccatttgaagaaaagctggtgatggaaggttgccttgacgtcatcaacaatcattcggacgccttagtcggaattcaagatatgggtgctgctggactggtttcatcttcggcagaaatgggctccaaggctggcggcaacggaatggaattgaatttggatttggtcccacaacgtgaagccgggatgtccgcctttgaattaatgctttcagagtcgcaggaacggatgctgttgtgtgtcaaagccggtcatgaagatgaagttttgaatgtctttaaggaccatggcgttaacgccgtcgttattggccacgtgactgaaggccataattacaaacttcttcaccacggcaaagtcgttgctgatgtgccggttgactccctggcttctcaagcaccggtttatcaccgtgaatcagctgtaccagcacacttgaaaaatgccgatgagaatcagtatcaacctcaaattagcaacccaactgaaaccttgaaagaaatgcttggccaattaaccattgcttctaaggaaagtatctatgaaacctatgatacccaggttcaaaccaacacggttgtggctcctggatccgatgccgccgttgtccgggtgcgacaccacgacaaggccttggcaatcacaactgatgttaatggtcgctacctctacttgaatcctcgagtcgggggtgccatggcggttgctgaagctgcccgcaacattgttgcatctggtgccgtaccgttgggaattaccgattgcctgaactttggtaatcctgaaaagcccgatcagttctatgaattggatcaagcagtgatgggaatgagtgaggcttgtgaaaagtttgaagctcctgtcatttccggtaacgtttcccttaacaatgaatacgataatattccagtctatcctacgccaatggtggggatggttggcctgatcaagggcctggaccacatcacgactcaagactttaagcaagccggcgacctggtttatgtagttggtcgaactgaaccgggatttaacggttctcaaattcaaaaaatgcaaaccggaaaaattgccggcaagctcttcaattttgatttagattatgaagtgaaaattcaaaaattaattacagctgccattcaacaacatttgttgaattcagctcatgacatctctgagggcggtctgattactgctattgctgaaagtacttttggcaatcagcttggcgttgacctgtcaggtaacttaaccgttgctgacttcttctccgaaagccaatcaagatttgtcgtttcagttccacaagaaaagcaggccgaatttgagcaattagttggcaatgacgcagaaaagcttggaaaggtagtcgatgacaatcacctatttgtccaagccaatgatggttactttgatcttgatgttgataaagcatttggtatttggaaaggggcattgccatgccgtctgaagtaaaaagtttaaatgaagaatgtgggatcttcggtgtttggggaacgcctgacgctgccaaattgacctacattggcttatttgccctccagcatcgtggccaagaaggtgccgggattacggttaataatgaaggccatttgaccaccaagcgggggtttggcttgttgaccgacgtctttgattcacccaacgcggttgatgaaatgaccggtcaagctgctatcggtcacgttcgctactcgactgccggcagtaacttattggaaaatattcaaccgctgccctttaactttagcgatacccaatttgcgcttgctcataatggtaatttaaccaacgccatttcaattcgaaagaacttggaagaccgtggtgcgatctatcattccagttccgatactgaaaacctgatgcatttgatccggttgagccaagaagacaacttggacgaccagatgaaagaagccctcaacatcattaagggtgggtttgcctacttggtcatgactaaggatcgcttgtatgctgcccttgatcccaatggctttcggccgctcgttgtcggtcagctgccaaatggtgcttacgtcgtctgcagcgaaacttgcgccttggatgctgttggcgctgagttcaaatttgacgttcaaccaggtcagttaattaaaattgatgcttccggcatcaccgttgataaatataccgacgatactcagttggcgatttgctcgatggaatttatttatttcgctcgccccgactctgacatttacggtgttaatgtccattctgccagaaaacggatgggggctcgcttggctcaggaacagccggttgaaaatgccgatatggtgattggagttcccaactcgtccttgtcggcggcaatgggatacgctgaagaatcaggcttgccttatgaaatgggtctggtgaagaatcaatattctgccagaacattcattgaacccactcaagcactccgtgaacagggtgtgaatatgaaactctctgctgttaaaggggtcgttcggggtaagaatctggtgttggttgatgattcgatcgttcgcggaaccaccagtcgccgaattgtcaaattactcaaggatgctggggcggcctccgttcacctgcggattgcatcaccgccgctgcgttatccatgtttttacggcatcgatatccagcacgttcgcgaactgattgccgctaacaagacgattgaacaaatgcgcgaaatcttcggggctgattctttgggattcctgagtgttcaaggggtgattgattcagttaatttgaagaccgacgcacctaataagggtctctgtgttgcatattttgacggcaaatatccaaccccgctttacgattacgaggaagaatacgaccgtgatcaagcccaactacaatcaatgagatgaggtaattcgaatggacgcctataaaaaggccggtgtcgatattaacgccggttacaagttagtcgatgatattaagaatttatcaaacaataaagaccttggctcattcggtgggttgtttcccttgtcgctgggtgtctatcaaaacccggttctggtttctggaacggatggggtgggaaccaaattgttgatcgctatcaaagccaatcaacaccaaaccattgggatcgacctggttgcgatgtgtgtcaacgatgtgttggcccaaggcgcaaagccgttgttcttcttggattatctcggagttggtcacctggataacgaaaaagccaaagcaattttagccggcgtggtcgaaggggtttctcaggctcaggcaaaattggttggtggcgaaactgccgaaatgcccgatatgtatactcatgggcattatgatttagctggatttgcggttggtattgctgattccgataagctcttaagccctgacaatttgcgtgaaggggatgtcttgttgggacttgcctccaatggtcttcattccaacggtttcagtttggttagagacatcttgttcaaacagaatgcctattcattaaatgatcagctgtccggctgtgagcatgatttgaagcgtgaactgttgcgcccaaccaagatctatgtaaaatcagtgttaccggtgatcgagcagggcaaaatcgcatcaatcgctcatatcacaggtggcgggttaccagaaaatgttgccaggattttaccggataacctttcggcagaatttgagtatggcagttggcaggtgccggcgatcatgacagacttgcaagaaattggtcatttatcatttgatgatctcttgcacaccttcaacttgggacttggcatggtaattgccgttcatccagctgatgccgatgccgttgaatcacaattaaaagcagctggcgaaaccgtttcacgggttggtaagctcatttctggcgacaaacaagtaatcattcgaaaggatcagcaatgaaatctgacgtaaaaaacatagcgatatttgcatccggtgagggaaccaatttcacagcattgacggaatctttcaaaaaagaacacttaccgctcaatgtgaggttgttggtttgtgatcattccaacgttcacgtcctcgaccgggcacataaggaatccgttccaacatttgtgattaacttcaaagattatcccaataaagctgccgctgaaacggtgattgcccagaagcttgaggaagcccaaatcgacttcatcattttggccggttatatgcggatcatcggccccaccttgttagccaagtatgaaggcaaaattattaatattcatccggccctgctgccgaagttccctggccgccatgggattgaagatgcctatcaagctggtgtcgatacgaccggtgtcacggttcactgggtggattccgggattgattccggaaaaatcattgctcaacgcgaggtgccagtccacaaggatgaccagttgagtgaccttgaacagcggattcatgcgacggaacacgtgttatatccaagcgttgtcaaacaattattagaaagaggagaaatttaatgtcgaaaagagcccttttaagtgtttctgataaaagtaatttggttgattttgctaaacagttaaaggatttggattttgaaatcgtttcgaccggcggcaccaaaaaagccttggaagacgctggcgttgaagtgaccggcgttgaagaagtcaccggttttccagaaatgctcgatggacgggttaaaacccttcatccaaagattcatgccggaattcttgccaagcgtgacgatcccgaccatatgaaacaattaaaagatgccggcattacacccattgacttggttgccgttaatctgtatccattcaaacagacgattgaaaagcctgagaccactcaagtagaagcaatcgaacaaatcgatatcggtggaccatcaatgctgcgggcagccgcaaagaactttgccggcgtgctgacagtcgttgacccagctgactatcaaccagtgattgatgctctgaaggcacacactgatgacgccgatttcagaaaacatttggcagctaaagtgttcagacacactgccgcatatgacgccctcatttcgaattatttgacggaagaagaatttccagaaaaactgactttaacttacgaaaagcaacagtcattgcgttatggagaaaacagtcaccaaaaggcagccttctaccgcaaggcgttaccgtcaaaactgtcgattattcccaaccagcttcatggtaaagagttatcatacaacaacatcaaagatgctaacgctgcattgaatatggtggctgaatttgatcaaccaacggttattgcgatgaagcacatgaatccatgtggggttggtgtggctgataccatcgaaaaggcttgggatgaagcttatgaatcagatccgatgtcgatctttggtggaattattgctgtcaaccgagaaattgatgctgcgacggccgaaaagatgcacaaaattttcttggaaattgtgattgcgccatcatacactgatgaagcatttgaaattttagctaaaaagaagaatattcgtctgctgaaagctgatttgagtcaccgaaacgaacctgatcgcttcgaagaaatcacggtgagtggggggatgttaattcaagaaagcgaccatgaaattgatcagattcctgacttcaaagtggttaccaaagtccaaccaactgaacagcaattgaaggctttgcaatttggccaacacgtggttaagcacgttaagagtaacgcggtggttgtaacaaccgataccaagactttgggtgtcggcatgggtcagcctaaccggattgactcagctaagattgctatccaaaaggcaatgccgaaggacggttacgaaaatgccattatggcatcggacgccttcttcccaatggatgactgtgtggaatacgcagccaagcatgatatcaaggccattatccaacccggtggcagtatcaaggataaggattcaattgcaatggctgataagtttggaattgccatggtgatgaccggggtaagacattttagacattagaagcagagcgcgacaagggctggttgacccggtttccaagggtactttgattgaagtccctgggtttgggactgtaatcaaagtacccttggaagttagggtcaggcccgtcggagcgtattttagaagcagagcgcgacgagccccgggtgtccccggtgtgtaaggcggaaatttaaatgatgaacgggtttcgttcatcgtttgaatttttggcttacacgttagggggcaggggcattggagcgcatttcgagcagagtgcggatcggggcggttaacaaccggagcctaagttggctttgggggaaattggttttgatttcgcccaaagccggcttaggtgcaggttgttgccccgaggagcacgtttcggcttggctgcctaaccgtttccaacaagtaaaaccacaaatcaaataagcacaacaaggctgtccatcagccttcatacataaaccaaccatcaacaatcaaaaaggagatcaaattatgacaaatgttctggttatcggatccggtgcacgtgaacacgcaattgcagcaacaatgttaaaaagtccccaggttaccaatgtctattgtgctcccggtaatcctggaatgaagaaggataacattcaaattgtggatatcgatgaaatggactttcccaacttggtggagtttgccaaagagcatctggttgatttgacgttcgttgggccggaagtgccgttgtccaaagggattgttgatgcctttatcgccgctcgtttgcgggtattcggcccagatgagtctgccgcccgcctcgaaagtgacaagacgtttgcgaaaggattcatggcccgaaacaacattccaactgcccagttcaaaacatttacgacctttgatgatgccgaaaagtacgctgagagtttgtcattgccactggtagtgaaggaaaatggtctggccgccggtaaaggagtcacaattgtgaaagactcagccgacctggcagcaaccatccaacacgcacttgataaagccggtgaaattttaattgaagaatttctggaaggtgaagaattttcactgatgctgtttgttggcggtgacaagaaggtaatctttccaatttcacaagatcacaaaaagatttatgaaggtgaaacgggtccgaatactggtggaatgggtgcttattcaccggttccacacatcacccaagatgttttggatgccacagttcaaaagattgttaacccaacgatggctggactggcgaaagaggatttagagttcgccgggattatttacatcggctgcatgctgaccaaacaggggccaaaagtgatcgaatacaacttgcggctgggtgatccggagacccaagttctattaccccagttgaagagtgatttttaccaaatgacctctgatttgatcgaccatcaaatgccaaaagttgagtggcaggagggtgagttctatcttggcgtcgtggtttctgctccaggatacccaacttcgcccaagcaacatattgcgctgcccgatgatttaccacggaatattttttatgccggggtaacagaggaagatgggaaactttacagttcaggcgggcgaatctttacgttatacaatcatgcttcgactctggaatgtgcccaggcaaaagtatacgctgagttaagccggcttgatttgtcaggattctattaccgaaaagatattggctttcgagatttataaaactatttgaacaacacaaaacgggtatccagagtttggatacccgtttttgatttttataatttgagtgtggctggccaatcttactagctttgtcacagtcagtgagcggacttatcaaagtgatttcaagcaataatgatggcaaaaaagacaccgaagccactgggagtcggtgcctcaatctggatcaatgattatttgcgcagaaaaaccaaattgtccgctgttgagtcagtttcactaaaccgatagttgggtgaatcgaaatctttcaggtcagaaatttgttcaacctgatgtttggccatgaaccggaccatttcaccacgcgccattttcgcaaaggttgccctggttttaatgttgccgtcaaccaagtgaccaaaggtgatattgatgaaacgatcggttggttttaagaattgggtgacggtcttggcgtattcttgggaggctaaattgataattggttgatcgtctgccaaagactggtaaatgcgatctccccagtattggtacatatttttggcaggactgatcgttaactttgaatccatatcaaaacgatagggagccacgccgtcaaagggtttcagaatgccataaaatcccgagagaatgcgtaaatgttcttgcagataagtcagcgccgctgcactcaagaggtctggcgccatgtactggtattgaatgccggagaaacttagaatggctggggttaatcgatgatgcaggtcaatagtctgtaattgctggtaactagcttgggtcagcttgtcactcgcatgccacaactttttgagctggtcgtaactcagctgacgcaatgcatctaaaatttcagtcgtctgtttcaaatacaccggcattccctgcacatcaaaatcatcttgattgacgaccattttcttggctggtgaaataatgactttcatcgctaatcattctcattaagccagctgtcaagaacgttgatgaattcatcatgctgatccagcaaagcaaggtggcggctgttggcaaatagatgccacttggcaccaggaatatgatcataaaccgtcttggcgattaacggggtgcagaggtcgtctgtgccgttggtaaccaatactgggacatgaatattctttaagtcatcagtgacgtcaaaatcgctgatggtgccgttctcggtaaactcattggggccttcggcgatcaaactggcttttttaccgttggttggccggcggagtggttcaggcgaattttcgtctggatcatcccagcagtacatttccatgtaacggtcattggctgcggcatatttggggccagagaagtttccagtccgctctgcctcagcgattgcctggcgatcttcgtagctgagatatttcaagagccggtgctgttcttgaatccataacttgatagaagatggggagccatcgatcatgacgcttttaacaccttcttggctataatgagtcaaataaagcatttccagcatgccaccccatgattggcccagcatatgtacttcatccaaatgaagatattttctcagggcaattaattcttctgcccaagtctctttaacgtagagggattcgtcgtctggaatcgacgatttgccgcagccaatttggtcatacatgatcagttggcggccagtctcggcataatcatcgagtaattcgaaatagttatgtgatgaacccgggccaccgtgaatcagcagcagtggggcttttccaggtgttttctcgccaacgatccggtaatatgttttgtagcctttaaatggcatgtaaccttcttcaattttcattcaattatccagtcctttccagtaaaaatctttgattggcatccattatacgccagttggcagtcgattattagaggatttatcataattaagacagtgtggaaaaataaacgcttagttgccagaatatcagggcgtgattcaaatatccagattttggatgtttgaatcacgccctgatatggccggaaactgtttatttttccactatttggctgggtaacataaaagccggggcaaagcattcacttttgtcccggcccctttgtaagtcgatttaatcattgattaatttatctcgtaattgatccactgaagtataaacctcaccgggattaattttctccagctctttgtgtttggcattaattgaccaagcagccgagtagcatttaatcccagcttgcttgcaggcgacgacgtcggttggagcatcacctatgtatgccatatcgtctttggtggcgttaaattgtttgatcacgtcactaaattgttctgctttgatcgagccgtcaggagatcctgataagacaggggagaatgcatccgccaatccaagtgagtccagactgacttggaggctttgctcacccttgccggtaatcattggcgtgatcacatcgcggtcgtggagttccttaatgagcttttcaattccctcaaacggatgccgtaattgcaaatgcgcccgccggtagttttcgtgaaagctttccaagacctcatcggaataatcagggatcaactcctttaacatcccaacttcgtttgctccaaaggtggcgaggatgacctggttgctgatccatttgccagtataatcgtgaacggttcttctaaacgaatcaaagattaccgggaaagtctcggcaaccgttccatccatatcaaacgcaataattttttccattactatttttgacctacctttcgaagtgcatgaccaggattccctgccggatgtgcacttcatgacagggttcctaaatgagcctatacaactattatctgctactaggcacaattattcaaatgaataaaaaaatcgccggcttgatgtcgacgatttttgaaaattttcattgaattatgcccgttttaaactcatctttttcaatcctggtaatgtaatcattgtgatgaaactgatgacgtagaggattgagagaaagcccatgacaaccgtcaatgagtagttgtccattaaaatgccaatgacaactgatgagaagccccccacggcacggccgatgttgacgatcacattgttggctgtcgaacgaatttcagttgggtagaggcggctgataactgcaccgtacccaccaaacatgccgtttgagaagaagccgacgatggcaccgataatgaggagcgaaatggtattgtgggccagggtaattgtgaagaccatggcagccgaagcaatcaagaagatgccaaatgctcgacgtgggccaaagtaatcaaggattgagccgaaggtaatcattcccaagctcatgccgatgatagtggaaatcatccacagtgatgaaccggaaacgtttaagccaagttgtttttgcacgatgattggcagccagttcatcaagccgaagtaaccggcgatttgaacggtggtcataatcattaaggcaaaactttgataggctaatttgggtgaactgaacatgtacttgaagacggcgctggtcgtggattctttcttcttggcttcaaccttcttggctgcgacaaactcttcagtctcggtcaagtgacgacggacaaaataagttaagacgaccggaacgattccaaccaggaacaatgcgtgccatcccagatgtgggatgacgattgcggcggtgatcgctgccaggatggcaccgatttggccgccaattgcggcaaccgatgtcatcttgccgatttgattcttgtggaaggattcggcaatcattgagatcccgacgccatattcaccaccggcaccgattcctgccaagaaccttaatatgtaaatcaatgtgatgttattggcgaaggccatcattgcggtcgcaaatgcgaagatgaagattgtgtaggtgaaagtcttaacccggccaaagcggtcaccgatcagaccaaacatgatcccgccaaataacattcccaagttggtaattgagccaatcaatccagcagcgccaccgctaagatgaagttggccaatcattgaactcattgcaaaagataaaaatagcacatccatattttccagcgcgaatccagaactggtagaagcaataacccatttctgattcttcgtaaaagtatggctgtgcgtaagtgctcgtttgtattttccatgttcgttcctccaaatgaatgctcgctgacattctttatttttgctgttcacattattacatggatgttttggaaatgcaagttggtcaattaaggatatctgtgattgtttgcttagctcggacaaaagatggtgtatcaagtacgctcacaaattctgcatgatgactttgaaagtcataagtaaaaaattgaagtggattcacaaaaccatcaattttgtcattattaactctgattaaaaagccactttctcgtaaggagttattcattgcatgggttatgggagcaaccgccaccaagtgagtcattcgactgtacccttgattgcttaaaactagagcagggcgtcgctttctgatttcatgaccgacggatggattgaaatcaatgtagatgatgtcttgttgatttgggacgtatgggctaatctttggggatttctctgccaactaatttacccccaaattcttctggttgttttaaatcgtgtgattctatgaacgcctcattgtggaatggattatcatgctttgggacataaacaattaccccatctctaccctgaaaaacatcaaactcgtgtgcgattggcttgatactatttggtacagttaaggtattcgagttgccaactttgcgaattttaactgacatggatatcacttccttctttcgtatacacgaagtatacacataatgcatctgatgttcagcaaatatgatcactaagtttcacttgaacaacctggtccatcgtgataaagttataaacaaataaaagagctttaatttggttcagagaggccaaaagcggacgacaattaatctaagagtccgtgattttgtggaatttagtacagggatgtactgaatacacagtctcgggctctttttctgtcattaaccaggagggtaattatgcgaggaccacttattgtatcacttgatgtttggaatcgagaaggcttgttcaagatcattgaccagtttccaaccgacgaagggatgaccgtcaagatcggcatggagctgttttacggcgaagggcccacaattgtcaaagaactgctgaacaagggcttcaaaatcttcctcgacctcaagcttcaagatattcccaataccgttaagatggggatgatgcaaattggtcggatgggcgtcacttatacgacggttcacgcattgggcggctcggaaatgatagcggctgccaaagagggccttgagcttggcagtgaagaagctggggtgccgactcccaagttattggcagtgaccgagctgacctcaattactgaagatgctttggaaaatgagcagaactgtaaattagacatggttgatcaagttgtctccctggccaaattggccaagcgatcgggtgccgatggcgttatcacttccccgttggaagtcagttcactgaaagaacaggttggcaatgacttcctatatgtgaccccaggaattcgtccggcgaacttccctaaggatgaccaatcaagaaccgcaacgcctaaacaggccgcagaatacggcagctcagctttagttgtcggccggccaatcattcgagctgaagatccggttgctgcttatcacaaaatgttggaggaatggaattatgcaaactaatcaaattattcaatcactgattgaccaccaaattgtcagtatcaatcttgaaaaacccttcagatacgccagcggaatcttatcaccaatttacaccgactttagactaaccatttcgattccttcccttcgagatatgattgccgacggtttggcagaaaatatcaaagagaattatcctgatgccaccgtcatcggcggggttgcgactgccgggattccccatgctgcttgggtagccgaaagattgaacctgccgctgatttatgttcgggccaagcccaaggatcacggtgccggtaagcaaattgaaggtcgaattaccaaggacgacaaagtggttttgattgatgatttgatctccaccggcggcagtgttttgggtgctgttaaagcggttcgcaacgaaggcgtcaacgtgattggggttgcttcagtcttcacttacgggttgccggacgccgacaagaatattgccgacgctgacaccaaattggttccgttactgagttacgctgatttaattgcccaaggccacaaagaaaataaattctcagatgaagagtattcacgcttatcaacttggcacaaagccccttgggactggacaaaacgggaggaagcaaatgcaaaataatatctcactcgccgctcacattggcgactatcaattcgataatttattgttaaacgcagctggcgttcgctgctcaaccacagacgagctgaataagaccctggattcaatggcaggtggctgtgtcactaagagtgccacaccagaagaacgggccggtaacgaaagtccccgcatgaaggcattaccgcttggcagtatcaactcgatgggtctgcccaatcacgggatcgattattatttgaaatttgctgaagaaaatcaaggcaagaacggtaaacaagtgatcttatcgattgccggcttgtcaattgaccaaaatattgagatgctcaaaaaagtccaagaaagttcattctctggattgactgaattgaatctttcctgcccaaacgttaaaggtaagtcacaagttggttacgacttcgatgccgttcgggacgtcttaacttcaaccttcaagttcttcaagaagccacttggcttgaagctgccaccatactttgactttaaccagtttaatgggattgctgaagttttgaatgatttcccaattacttatatcaacgttatcaactcaatcggtaatgggttagtcgttgatccggaaaccgaatcagtggtgatcaaacctaagggtggctttggcggcctcggtggcgattacgtcaagccaactgcattggccaacgtgcgggcccttcgtcaacgcttgaacccggaaatttcgatcatcgggactggtgggatcaagtcaggcatggatgttttcgaacacgtcctctgtggcgctaatttggtgcaaattggtaccgcatttggttacgaaggcacaccgatttttgaacgaatttcaaaagaactcaaagatatcatggacaaaaagggttacaagacgctcgatgatttcagaggaaaactcaaaacaatttaagtatgattcaaggtcaagccagcaatggtttgacctttttatattcactaaagccaatggtgcggtaaaattgaaacaacaccatttttgaaaggagtcatcctatgccagcaagtaagcttcccgatcatattgaagtgattggtggaaaagtgaataatttgaagaacattaacgtcaatattccgttacataaattcgtggcagtctccgggttgtccggttcaggtaagtcatccttagccatgggcattctgtattcagaaggtgcccgccgctatttggattctctggccacctacacccggcgacggattagccaagttggccgggccaatgttgactcggttaagcatattccatcggccttggcattgcggcagcggccaactgttcccggtgcccgctcgaccgttggcacaatgaccgaaattttcaacgtgctgcggttgatgtattcccggttgggttcgccaaaatgtcccaacggccaccaagtcccgccaaccattaagattgcggaagccatggacgtcatgggcgaccaaatgggtgtgattacctgtccaacctgtggcgtcaagttccacgcgtttggtgccgaagactttgcctttaattccgacggtgcctgcccagagtgtgaaggattggggatcaccaaacagcttgatctggacagattgattggcgatgaaaccaaaaccatccgtgagggggcagttgccgcttggcggacaccaggcagaaacttcatgccgattgttgcccaggcggcaggtgtcagaattgatgtaccctataaccaattaatggacaaagaaaaagatatggtcctgcatggtcaacagaaacattacaccatcgatattcccagcaagaacggccgggtctttcatatggacaacgccttgtacgaaaatgcctacaacgccattgaggacagcatgaaaacgacgaagagtgagattgccttgaaacggctaaatcgtttttaccgtttcttcacctgcccaatgtgtcacggaacccggatgaatcccaatcgtctgggacagctgattgacggcatgaacattgccgaagccagccatatgccacttgggaagctgccggcctttgttgaccgaatcaaacaatggttgccggacaatatgcagaaattggcccaaaacttgacgactgaattgctcaatcaaacgcaaccattgctcgacctggggttggattatttaaccatggatcgggctggcgcatctctttcgaccggtgagcttcaacgaatccaactcggccggacgttgcgaactcagactaccggggttctgtatgtcttggatgagccctcggtcggcctgcaccccgacaatgttgccggtctcatcaagatttttcaccaactggttgaccagggaaattcgttggtggtcgttgaccatgaaacggcgattattaacgcggcggattacatcattgaaattggcccggggtcgggggtcaatggcggccaagtgattgatcaaggaaccccggctcaaattcgccagagtcagcattcattaattggaccgtttttgactgggaaagcgcagttggtgacccgaaagattgccaatgacgatgtttttgccaaaggggctgtgatgctgacaatcaaccagcggtttaatttaaacgatgttaccgcagaatttccggttaaccggttgattgcggtcaccggattctcaggtgccggtaagacgacgctcgttttggatggtttacttgatgccttcaccgccaagtttcacaaccattcattaccgagttatattagcaagtttgaacccggcaaaatgaagcatatcgtcagtgtggacgcgactccggtcgggaaaaacgcccggtcaaccctggcaacctacaccaacattatggacaatctgcgcaagaagtttgcccagctgcctgatgccaagaagcatcactataccccaagttatttttcctacaataataagcagggggcttgccccgcttgtgggggaactggtgaaatatcgctggatattcaatatctgcctgacatggttgaaacctgtccaacctgcaaaggtcgccggtttaaccaggatattttgaatatcaaatggaatggcaaatcaattgccgacgtccttgactacgacgttgatcacgcgattgatttgtttaaagacgatgaatccattttgaagaccttggaagttctccagcagatgggcctgggttatcttcacttgggggaggccaccccgagtctatccggtggtgaagcccagcgattgaagctgacttctcatatgaagagccgccaaaatgatacgttatttatcttcgacgaacccacagtcgggctgcacccactggatgtgcatgtgttgttaaaagtcttttcacagttgattgaccagggggccaccgttttgatgattacccatgatcttgacctaatggccaatgccgattatctgattgacatgggaccccgtggtggtgatcagggtggtcggattgtcgccaagggtcggccggcggatttggttaaggatccgcggagcttgacgacaaaatatttggcggaacattttcaaaaatttcaaaagtaggtaaactcccgcctactaatcaatcttgcggattggttctgagttgattgaaattgtatgtaagccttcacaaaatgctattgacaccgttagatgaaaattgtaaattgatttagatagttggttttttagaacaactttgatgctacaaccaaaatatcgtatttaatctgaaggtgtcatcatcgtaatcactgccttcgtgaaaatatagcggtatctcgtggctcagttaggttgattgttgaatttagtgataaaaaatggagggaataatttaatgactaatgcaacggggagggagcagcttcataagcgaaacttgaatctagttctgcaacaaatttttaacaatggtattatttcgcgaattgatatttcacacacgttaaatttaaataaatcaacggtatctgctttgtataatgaactagacgaaaagggtctgctgcaggaagtcggttcagggcaatcaaccaatgttggtggtaggaaaccggtcttagtcaagattaatgagcaatatggatatacgatcagttttgatcttggtttccgtcaccttcatgtgatgggcaattatcttagtggtaaggtcttttactatcaaagaattgagcttggcagtagagatattcaaaaaattctgggaatgattgatcatcagatcaaagtttcaatgcaaaacgatcagaccaagcgtggactactcggaattggtttttccattcatggaattgttcaagataaccaggtgatcaattcgccttttattgatatggagggtgtggatctggtcgaattgtactccacaaagtatcgagtacccgtccttcttgaaaatgaggcaaatctttcaggtgtttatgagcgcgatttcaatgacggcaaggataagaataatattattgccattagtattcataaggggattggcgcaggcattattttgaacaggcagttatacagaggcgttaatggcgaagcgggagaaatcggccgctcgttgatgtttaccgaaaattttactggcagtaaaaatgataaggtcgaagacttttgctcagaagatgcaattattgagcaagtagaagttcagactcatcaggaaaatttaacacgtgaggatatcgtacagagaaatcgtgctggtgataaagttgttcaaagtgaacttaaacattttacttatgcaatttcgcgggttatttataatgttgcaattagttttgccccccaagaactctacttgaactcaccattgattgaagatattccaacgttgtttgacgatatcgttgataatgctcagaagcttgggatgaagatacccattcggctaatcccccattcaggctatgcaacgcttttggggtgttgctcactgttgacacatcgggttttggacatggatgagtatgatttgacatttacaagtcagaaataacaatatattatggccagtgattttcttgggcaagtagtaggtcagtatatttaaaaagttgaccaatattgaaagaatactcttccaaaaaggtcaacttttgatttatccagagatgtaattctcttggatcgccttatcatatttagtcactttggatgacttgcgatactgtgctggtgtattcccggtgacgtctttgaaattacggttaaaggtccttagattttcatagcccacgttaaaggcaatgtcggtaactggtaatgaagtgttctttagtagttcacgtgctttggaaatacgaaaactgttgaggtatttagtatacgaaaggttgattgttttctgaaagagtttggataagtatacatagtcatagccgattgagtcagcaatttgcttgagtgtgcatgattctgtgtaatggtcattaatgtagttaataatttggtagattgtcgtcaattgagaagaagtcttttttagcgttagctgggtctgttccaccaccttattgcaaagcccgtataaaaagctcttgatcccaaaaatattgtccaaatgctcaaattctggcggaacattatcgaaaatgactgggttgtctgcaatatgatccttatattgttcactgaatgcgctaacaatttctggcgaaaacaaaataattgttgctgtggtatttggtgacatgtcgaagccgtggagctgatcgggaaaaacaatgataaattgatggggattaacgtgatagatgcggttgtcgacttgctcttgaacttggcctttacgaacatataagatttcgaaggcacggtgaagatgaatggggtagtttaagtcggatatgtcaaagtgtttaaagattggtgaggattcaagtccaaaatgttgaaataaaaccaaaagatcgccttctttgctatgacagttattgtttcatttatagcagataatcaggttttttgcaattttacaatgaaggtaggcatcccgtttgcagttgatactggacgagagaaggagttgcagatgacaatatttcatgttgctaaaaatgggtctgatcaaaacgatgggcaaaaaagttcaccgttactaacgattaatcatgccgcccaattggcaggcccaggagattcagttatcgtccatgaagggacttatcgtgaacgggtgaatcctgctcgagggggtcgacttggtgagatggtggcatatcaggcggctacaggtgatcatgttacaatcaagggatcagaagttgttgatcacattgataaaatggaaaacggtatctggagaatggtaattgataaccatgtatttggaaacttcaacccgtttgccttttctttaaaaggtgattggctggaacaaagtaatgggcgtcacgctggggcagtctacgtcaacgggaaagcgttatttgaggcggcggattataatgagctggtgatggggactgggcccacaaaaacgcgagaatatattacgcaaaagcttgtacacaggactaccaccagggaagaagaggataagtggtatgcaaaagtcaatgacaatcagacgattatttatctgatttccatgggcttaacgttgacgaccaactagttgaaatcagcgttcgaagatattgcttttatcctgaccggcctggccgaaattatattaaagtaaccgggtttgagatggcacagggtgccactaattgggcgccaccgactgcggagcaggaaggcctaattggtgtgaactggtcaaaaggttggattattaaagacaacgatattcatgattctaagtgttgtggaattagtcttggatcttacccgttgtcgaaaggacaacagaaccaatttgcaaggtaccatgatcgaccaggatatcagtatcaaattgaaacgatgtttaaagcatatgataacaactgggatcaagatcatattggttcccatttaatttgtaataatcaaattcatgattgtggacaggctgggattattggttttctgggcggtattttctcaacgatttctaacaatcatatttataacattggtacacgatatgaatttggtggttgggaaattgccggaatcaagctgcatgcaccaattgatgttagagttgagcacaacttgatagatcactgcacattgggaacatggttggattggcaggctcaagggacgcggctgtctcggaatatatactttgataacctacgtgatttattgctggaagtcaatcatggcccatttttggtagatgataatgtgttgctctctgaagtggctattaatgaatattcgcaaggtggtgcatatgttaacaatctcattgcgggtgaggtcgcaattcagtcggtcctcaaccggacgactccttaccatcagccacattctactataataaagggttatgcctgtgtttatggcggagatgatcgttattttaacaatttgttcgtcgccgagactgacgtttcagaagacgacaatcacattggaactgcagagtacgatggtagtccaacatcaatgaaggaatatattgcggcggttgagcaaagactaccgggtgatgttgagttgtttgaaaccatccgacaaccagtctatatcaacgacaatgcgtatcttggcgatgctgatgcattttcagaagaacagaacaatatccgattacgtaattgggatgcaaagttgaagctaaccagcgtagacacgcatatcgtgttacaactcaacgttcccgaggaattgttcaacacttgtgttccagttcagaaaacgcgttcgctcgggaaagtgcggctggctgatgcagtttttgataacccagatgggtccgctttaactattaataatggcattgataaaaagaccggattaagtcagcgaattatcggtcctttttctcagctacatcaaggagtcaatcaaatcgtattatttgacgatttggagcctgattgataatagatatacaagataagtgaaagtaagtgggatgtgtgaactgaaacccacttacttttttgtttatcgatagtattccaaactaattgtggcgattttgcgcaaactaaaatccagttttaaatattagatgacaaataatgtccaataaatgtcaaatacaagcatatcggtaagtttgtttaaaagataaactaaccatgtacttaattaaggatcaacttttctgaaagcgtttcaagtaactgataatgaatgcgctttttaaggtgatagcgttctggcctaattgcatatgtgatgattcgtgtaccaaagataagtggcggtgacgaccgttagtgattgttgcaatcagctaatttttttgatgataattgtaagcggcttcaattatttgttttaagacgacaaacgattattgaagatattctaatgaacggaaaaggtgaataaaatggcacaaaatgaaaatgttccagaatggcatggcactgttttagatagtgaacaacctaagaaaccaattaaaattgggattgccactgggattggcgcactgctgtggttaggaccctatttgggtgttaatggggttttgcttccagcaaaagttcagcagattattcctaatgaaaaagctcaggtagttgctttacttgcttctgctgccatgatcgcagcaacgttagcgaatattattattggcggattctcggatattacgcgatcaaagtttggtcgcagaacaccgtggataattgctggatcagttggaagtttattaacactgctgtggttcaatatggtaacgacagtgccaatgatggtggttgcttggtgctcgtatcaagtttgtttgaatgcgattgttgcgccattgcttgcttttttacaagaccaagtggcccctaagaaccgcggaacgatttcttccatttatgcttttggatatgtgattggacaatatggtggtcaagttgttggggctcaatttctgagccacgttggtactggtattgttgtgatggcttttctaacattactttcaggaccaattgctgcaattatcgttcgtgagccttcaagcttgggaatgcctaagaagcattttacagcaggaatggttgttcaaaactttattttcccattacatcaggcaaaagatttttacttagctctatttggaaaattgttgattaacactgcaactacagcaattatgggttaccaattgtacattttgagtgattacattcagttaaatacgggtggccaacagaagtacatttccatcatcaacatgatgctgatggtaactgcgattatcatgtcaattactgctggacctgtatccgattggatgaagagccgaaagatcccggtatttattgccgcattcttggttgctgttggggtggccttcccgatgttaagtaataatccttggactatggtggtttatggattgcttgccggattaggaatgggaattttcttcgcggtcgaccaggcacttaacctagaagtattaccaaacccacaaacagctgctaaggatttaggaatcctgaacttggccaatactggttcacaaattattggaccgattgtggctgctgcaattgtcacagcttcacacggtagctattttggaatcttcccggtatgtgcaggtcttgccctcgttggtggtattatgattctcttcgttaatgaacatcgtgatgttaaggttcaagaagagaatgccaaataaggacagttttaacaatccttggcccttagtccttatgaaccaaggattactctaattaatgtaaggacaaatatacgatagaggtgaaaacgttcatgactgctacacaaatcgaaagtactcaagattcaaaactggttgagagtcagttgagcaccacgagtgagaagctccataataatctcgaagttggcaccgagaaacgtcaagaaatttggggctttggtcaaacatttaacgagttgggctggcaagcactacaaagcctatctgaagaaaagcgtaacgagattttggacgatttgttcaaacccggagagggtgaaaattatcgaatttgccggatccccgttggtgccagtgactatgctttgaattggtattcattagatgaaacaccaggcgattatgagttaaaagatttctccatcgagcgtgataagaaatacttaattccatatatcaaagctgcccaaaaacggaatccagacatcgtcttttccgcttcaccatggagcccgcctacatggatgaagacaaaacccgtgtacaattatggaatcttgaaacatgataagaagactcaacaagcatatgcaaattactttgtaaagttcattcaggcatatgagactgaaggaattcacattagccaactgttcccacaaaatgagcctcaacgagatcagaaatttccttcatgctactggactggtgaggagttacgtgacttcatcaagaattaccttgggccaacttttgaaaaagcagggttgaataccgacatctggttaggaactatcaactcgccgctcgaagatactgaaatgaccaaggatgaaaccaccgactatccagtcattactgaaacggttctttcagagcccgatgcttatcggtatattaaaggggttacctatcaatgggcaggcaagtctgttcttcaacggactgtacaagcattcccggaattgaactatttccagtcagaatctgaatgtggcaatggtaacaatacttggacttatggggaatacgtctttaacttattccgtcactatatcagtaatggtgtgaacgcatatatgtactggaattctgtcttacaagatggtgaaagcacttggggttggttacagaacagcatgatttcggttgattcaaagactggtcagacgacctataaccctgaatattacgttatgaagcattacgcacattacgttcgaccaggtgctcacttgctttcgtatggcggccacgctgctggggaagcaactgcttatgagaataccgatggtagtgtcattgtggtgatgtctaatagtatgaaccatgatcgagacatctcgattgatgttaagggcaaaacatacgaggctcacttaaaagaacattcattcaacacattcgttttctcttaacgaggcgcgggctgaaaaaacggctggatagatttaaatattttaaaagagcttgaaaaagtatttgcgacatgataaatttaaaatgtaagttggtttatataaccaactaactaactaacaaaacctggaggcttgcttattatgagttattggaatgtcgataaaattaagtatgttggtaccggagagaaaaagtcaggattaggatttcaatattataatccggatgaagtcgttggtggtaagaaaatgcgtgattggttacgctttgcggtcgcttattggcacacatttgaccaacggttagtcgatccgtttggtgatggaacggctattcgcccatatgacaagtacactgacccaatggatcaagcgttggctaaagtggatgccgcatttgaattttatgataaattaggcgttgactttctttgtttccacgatcgggatttagctcccgaaggcgatacgcttcgcgaaaccaatagaaacctggacaaggttgttgacaaaatcgttgaaaaccaaaaaacttctggaatgaaagtgctttggaacacatccaacttatttaccaatccccgttttgttgagggtgccggtacttcaccatatgctgacatttttgcttactcagcagcgcaattaaagcacagtttggaaattggtaagcgtgtcggatcggaaaactacgtattctggggcggccgtgaaggttatgaatcactttggaacactgatatgaaacgtgaacaagaacatgctgccaaattattccatatggctaaagactacgccaacgaaattggttttgatgcacaaatgctgcttgaaccaaagccaaaggaaccaaccactcatcaatatgattttgatgctgccactacgattgcctttatgaaagaatatggccttgataaagacttcaagcttaatttggaaggtaaccacgcgaacttggccggccatacctatcaacacgaaatccgagttgctcgagaagccggtttgttgggctcattggatgccaaccaaggtgataagctgattggctgggatattgacgaatacccttcaaacttatacgagacgactgcggcaatgactgaagttgttgaaaatggtagtattggacctcgcggcggattgaactttgatgccaagccacgacgttcttcatttgaaccaaatgacttgttctatggccacattgtcggaatggatagctttgcagccggcttgagagttgctgttgcaatgaaaaacgacggcgtccttgatgacatcgttaaaaaccgctatagttcatttgactcaggaattggtgcagatattgaatctggaaaagcaagtatggcagatcttgaaaattattcactggataaaactcaaaaagatcttcgcgatgcaactcattcagatcatcttgaagagattaaagatacaattaaccattacatcattcagactttaaagtaacatcctgatcaaatacaataattaatgggaatgggattaatttttcattctcatttttttcgaggaggagaagatatgactgaatgcgtactgggtgtcgatctaggcaccagctctgttaaagtaactgcggtaagtcggactggtgaaatcattgcccaggaaggaatggatttcccactacaacagccacaaccgggttacgcggaacaagaccccgaagactgggtcagtgccacgactgtttcaattgttcgactcattttaaaagataagctcacccccgaccaaattgtcggtatcagttattccggtcagatgcatgggctcgtcttgctcgatagcaataatgaagtcctgcgtccagccatgctttggaatgacactcgttctacccaacagcgccaagagatcatggctaaaatgggtagtcggttcatagaaattacccataacaagccgttggaaggctttacgctgcccaaactgttgtgggtgaaggaaaatcagccccagatctttcagcaggctaaaacgatgttattgccaaaggattacctaaggttcagaatgactggtcaattggcaattgattactcggacgcaactggaactgtgatgtttgatgtcgacaaacagcaatggagcaaagagattttagatgcatttgatattcccgagaagatttgtccgccattagtcagatccattgatgagacggggaatattaatgagtggtacgcagaatattctggattatccacccacaccaaaacctttggcggcggtgctgataatgcttgtggcgcagtgggtgccggcattgacggacccacaaaggtgctctccagcattggaacttccggagtgattttaaaatatgaaccccaaaaggaaaccaattatgatggcgtgattcaatacgaggaccatgccattcccaatgcctattactcaatgggcgttaccttggccgcaggattttcactgagttggttcaaaaagacctttgccgaaaacgaggactttactgcagtcgtggatagtgccgccaaatcaacagtcggcgctaatgggttgctctttgccccgtacattgttggtgagcgggcgccatacgccgatgcggacatccgcggcagctttatcggcattgacggaatccatcagcgccacgattttgttcgcgccgtattggagggaattatcttttccttcagagatattttggatttgtatgaggcgaaaggaaaccaatttgagacagtcatctcgattggcggcggagccaagagtcccctctggcagcagatccaggccaatattttcaatgtcaaagtggtctccctgcaaaatgaacaggggccgggactgggagctgccatgctggctgcggttggcctgggatggtatcatgacatctccgagtgtgccaagacctttatccagttcaaagatgtctttttacctgagccggataacgtggaaaagtatcgtcaattgcatcaaatttatcgaaaaatttatccaagtaccaaagaaatcacgcatgagctggttgatttccgacgagataatcagcgttagcaaccatccgatggaacttcgaaactgcaggttccattttttatttaaaaaaggtgacgagatgtcacttccaaaaaaacaactcaactttatggaggaattcatcatggatttcaaattaattgtcgcaatcatcgccatcacctcgggggctgccacgcctgtcctgcatttggtaactggtttagccgcaattgtcttgatggcttttcattttctgtgggccggttacgttttatggctggggagtgaaaagtccaaacgcaatttccacaagttcagcttgcttgtatggctgttctggctgatcccgtacgttgccgggttggtaatgggaatgagcaactaagcaatcggacacgaaagggtcaaaacaccagtttgatgatgttttgacccttttgacaattagtttggttgaaaagattattttaacgacatatctgaaattaaaacgaatgccatttttcaattaatcattctgagcttcggcaaccgccaaactgcgttgatgcaggtaggttacaccgccgaagacaactgtccagatgatggcaccgaccgcaccgataatatcttgtgggatgaagaacaaggtcacaaagataatggcgaagaaggcaatggtgagggggctggtgaaattgtaccaaggcattttgaaaccatttggcagaaagtcactggattcacggtatttccgatgagccatcattgccaaggcgtataccaggatatacatgtcatttgaagaaccagcaacgatcgtaaagactgaggccgtggcgttggtcagactcatcaacggggtaatcaagaggcacaatgcggaaaagccaatcgcagcggctggaaccccatttttagaaatcttagcaaaatggcggttcataaagctatccttaggcgtctcagtagccagctggtagaagtgacggccagccgagaagataaagctgttcaaagacgatgaagcggatgtcaaaacaacaaagttaatgacagctgctgctgccgggaagccggctaatttgaagacctggacaaatgggctgctggcaggcgtcaaatgggtccatgggatgatgcccatgatcacgattaaagcgccaaagtagaagatcaaaattttcagtagcgtttcgttaacggcttttttgatgattcgatgcggtgtttcggcttcaccgatggtaatgctgacaaattcaattccttgaaaggcaaagaagaccattgggaaggctgagatgaaactcaagccaccgtgagggaacattgagaagttatggaaaatattttgaacggatgcgtggccaagtggggtggtcgagtgggtaaacatcatgaagaccccggtggcgattaaggcgacaatcgcgatgattttgattaaagcgaaccagaattcagcctcaccaaagaccttggcggcgattaagttaacagctgccagcgttcctaagaacacaatttgaatcagccacgacgggatatttgggaaccaaaactgaacatatgtagagatggcggtaatttctgccatggcacaaaatgaaagtcccagccagtaagtccagccggtaaagtggccgacggtgggtcctaaatatcgggtaatgaatgagacaaatgtgtgttgtgatggatctgaataaagcatttcaccgatggcacgcatcattaagaagaaaaagatacctaacactaaatagactaataaaattgatgggccggttttactgatggtggtcccggaacctaagaataagccggttccaatcgtgcctccgatagcgatcatctgaacgttgcggttgctcaaggagcggcgggtgccgtctgcgttttcagttacttctgttttttgcatgaataaacttcctctctgttggtaatgatgaatcaaattagaggcctctaattaatttgtcattatactaacaccacggtgtctaaatcgggcattttagagaggaagttttcagatgattttgtgattttgattattttttcatgaaaaaaaggcaggattgccggtttgcctatgaaaataaaaaactttttgcagctcttgactattcgtcgttttccggcagttttagtgggcgagggccaatattcgttgtgaaggcaacgtttgtgtgactgtagccgaactccttaagagacgcgttgaattcattcagttcggtcatggttttatagaaaaccttcagctgaaccgaggcgtctccggtgatgtagttgcattccaccacattgggaatttttgaaatgaagtcaacaaacttaggcatttcaacgtaactaacgtcaattcggacaaatgctttgatcaaatagcccaacttttcgtaattgacattggcggtatagccgttgatgaacccatgattttcaagattttgcaggcgaacggacgcggatggcgcggagatgaaacatttttcagcgatgctcttgatggatgcccggccgtcttcttgaatgatatttaaaattttgcgatctaatttgtccattcgttttctccttaaaaatagtttgcgtacattataccattcaccattttgaatggttttgagaaagctcgttggtaaatgcgtcatggtattaatgataattgccacatacaatgagaatggctataatgaattttgtatctaaaattcgaatttagtaaggtcttgaaaaatgatgaaatcgaaaacaccacaatggaagaaaaacatgtgggcgctttggttcggcaactttgccaccggtgccggcgcgagtatgtcaatgccgtttctgccgctctttatctccgagatgggcaacttccccaagtggcaattaacgttatatgccgggctggcattctcaggcgtgttcttgagtcaggcgattgtctcgccaatgtggggaaatctggctgataaaaccggtcgaaaaccaatgctgctgagagcggcgatcgggatgacgattagtgccacactgacagggttgtcgccgaatgtctggttcctgatcattattcgttttatccagggaactttctcgggatatatcaataatgcctacgcgctgattgccagtgaagttccaactgaagacagcggtaagacgatgggaactttgacgaccggaaatgtcggtgggcaactgattggaccgattatcggcggatatctttctggtatttttggctaccggctgccattttatatgtttgggttcatgatgtttctggcatcactgtcgacttggttctttgttaaagaagacttcaccccaattaaaaagggtgccaagacgggaatgaaggatgcttttcgagggatcgctcacaagcgcgtggtctgggcaatgatcatttcatcaatgctggtcatggctgccacgacctccatcaacccaattattagtttgtttgtcaaagaattaatgcatagtcatggaaacgtagcctttaccagtggggtgatcgcggcactgcccgggattgcgacgatttttgcagcaccttatttaggtagattgggcgatcatatcggacctgagcgaatcctgttggctgggctgatcttctcggcggtcgtcttctttccaatgttctttgtgactacggttgtgatgttgggtgtgctgcgattcttgattgggatcgccaatgcggcactgctgccgattactcaaaccgtcatgacactggaggcgccggcccgttcggtgagtcgaatttttagttacaaccagtccttccaggcaatgggggcggttgttggccccatgctggcatcaggggttgccgggattttggactatcgatacgttttcttgatgaccacgctgttggtattaatcaacattgtggtggttgtcgttgcttataagaaggaccatgttaaggttgttccaaatcaatagtttttgtgcgcaactttttactgattattttgttgactttacgttcctaaaaccgtatctttatgttagaggcagatgatggcagatagggctgtgaagagggatagtatggccacaaaaagtttccaaactgattttaagtttaccagcaaatctggtcatgcgctcgcagaagcattcgtgcattctcggcgagtagatattaagattacccaaccagtaaacaggtacactgacaataactctgagcaattccataaaaagttcgataagttatttgctcagaaagtgagaaaatagaatatggcatttgaagtagtttcattaggaaagctgctagagagctacccagaagatagcattcgccagcagctttcttcttttttgcctataaatgatgatgtggctcactttattcacgatactgcgattcaatttgaaaagattggtttatcacgaacgacactagtttatacgtcaataaaggggcaattagttatagctgggtatttttccatatcttcgaaaccactctcgatctccaagaaaaactggcaccatttgagtaaaagtgttcaaaaaaaggttaatgcccattggttacaaaactgctcaagacagctatgaagtttcctccatacttcttggccagttggggaaaaattttttgtataaagatcaaaatgttatcacaggtgaagaactgcttggccttgcttatgaggaaattaaacatgcttggaaagcaatcgtcggtaccatgttgtatcttgaagcaaaaaatgaaccacatttgagagacttttataccgctaatggatttagccagttattattaaagaagagtgatatcgacaaacaacccacgattccatatgtttctgtcaatgggcttcacttatatattaagaaactaagcgatatttgatcagacattgtccaatccattgtgtactgcaatcaaaccaaataagaccatcaaaaaagttggagtttatctccaactttttgtgtcccttgagttacaaccgcgagtcgatttggttaattcccccgagaacagtaccatattaaattgcaaaatggtaatattaacttaatacaaattgtgcgacaaaaggatattgaggagtgaatttcatgattttgagtttcaaaaaatcattgtatcttggcctggcagcagttgcgatagtggccgcagttgaattaacaaccactgatgccagtgccaaatcatatgctagaatcacatccaaccaggtgatgcagacagccccgcagaaccgtaacgtgacgaccaacgggaccaatgcgctttacaccaaagccggtaccctgcgcggtgcccgaatgattgcgtctaagtatacgttgcagcgatatggcagctccaagctttccagccagtatttccgggcttaccgggtcgccacgactaatcggggtgcggtttactataaggttgtttcattcaatggtgtttaccgtggttggatctatggcgggcgagtaaacgggacctttgccggtggtttgaatccggccaacacaatggtaaatgcgaatttgcctttgcaaaagaccggctacacgttgaccaatccacagaaatacacactgtgggtcgatcccaaatggtcacagtataaggccaaacaatttgacatgagcagctatagcgccaatgacacctttacaattaccgatgcggctgttaagacccgcgaacaatatttatactataaagtcattgatgataaaaattccgcgattgttggctgggtctattcaggtggcgtggcagctcctaattcccaacaggcaactaaagataacagcgtcaagattaactatgtaaatccagccggccagtccgttggggcttacacatggattattcaaaagacagatctaaaagccggggctaccatgaccgatggtgacaagctgggggatattctccaaaacagcactcaactaagtgatgtggccactaagaacgtgccaaccgggtataagatcagtgccacccaaagcccaaccaatcaaccggctaacttcaccgttggatcagaggactatctggtctatgtcgatccgatcaaggccaacttcctatcaccggttgcctattatctgaccaataccggtcaacaaattagcccatctcagctagtgggcaatacctatccgattttgatagacgcccagatgacgattttctcatgtcaaacccagggaatcgtgccagctaaagtctttgataacgctttgtttgcagaccctaacaaactggcttccttgaccggcgtttcggtgaagaatgctgacggtacgatgactacaccaatttattacttcaacaagcaggcgacaattgccgccaacacaacagctaggtatggcgatactttgaagctttattatacgctgccgcagagataatctaagatggcattcaaattcattgatgaatttgaatgtcatttttgtttataaactatcaaaataccagttctgaaagctttttgcttactttttccaccggattagcccataatataaatactctaaaaagtaaagggaggcatttggatgtcgattttaactgatacctatgaattaaataatggcattaaaattcccaaagtgggctttggtacctggcagattccgggcggccaggatacttacgacgctgtcagcatggcccttcaggctggctatcgtcacattgataccgcaaaagcctatcgaaatgaaaagagcgttggcgaggcaattcttgattcgaatgtggaccgggaaaacgtcttcgtaacatcaaaattaccagccgcaaccaagtcctatgacggggcgattgcggattttcgttccacaatgaaggccttgaacctatcttatttggatttgtacctaattcatgctccgtggccatggggcgaacggggatcgaccaactatgatgaagccaatgtggaagtctggaaagccatccaggatatttatgccagtggtgaagtgaaggcaattggggtttctaattttaatgtccatgatcttcaaaacattttggctcatgctgatgttcaaccgatggtggatcagattcgctacttcgtcggctacaccgagcctgaaacaacccaatttgcccaagataatgatatcttggtggaggcatattctccacttgccaccggcggcattctggagaacttagacattaaaaagattgctgacagatacggcgtgagcgtcgcgcaattagccattaagttcgtcctgcaaaatgacttgctgccattacctaaggcaactcacaagaaccatattgaaaataatacccaattagactttacgattagtgcagaagatatgaaacttttgaatgggctgacagcaactgatatgtaatatagagaaatcttgaacggatcgcacatttgcgacccgtttttgtttgaaatttgttacagtggagttgaatcctaattgaaaaggggaaaatcatttatggcaaatgtattgattttaggtgctaatgggcaaattgcgaagttggttgaaaaacaattgctcgatgaaacggatcaccagttaacgttgtttctgcggcaggcgaaccggatcacggtcgctgatcccaaacgtgaaaccgtcattgaaggggatgccaccaatcgacaggcaatcatcaaagccctcgacggcattgatattgtttatgcaaatttgagtggcaaaaacattgaagaccaggccaaggcagttgtcggtgccatcgatcggaccaacgttcaacgattgatttggatttcgactttgggaatctatgacgaagttcccggtgcgtttggcaaatggaaccatcagcagctcgacggtggctatcttgagccgtataccgcagctgccaaggtagtcgaaagctccgatttggactacacgattatcaggccagcctggttatcgaataaagacattgtgagttacgaaaccaccgaaaaaggtgaacctttcaaggggaccgaagtctcgcgcaagagtattgccgacctggttgttaagttgattaaccatccaagccaagcaattcgccactctttgggtgtcaaccaaccgaatacggatggggacaaacccagttggtactgattgtctcgatttgcgtctgaatgttatctagtagaactgtgcgccaataagcagcttccagtgtataaggaaggctaaccgcttattggcgcacactttttttgttcaaaacttacaactctctaaaaaggtttgcgattttgttaaggaaagtgcaactttatcacttggtttgcgtttttaagttgcgtttaagctgccaacgataatctagtgacaatcaataacgaagggagcaatgccaatgccacatcagccattcaaacaaaggtaaatcatcaagcagcacttcaacaaacatttcaacttaacaaaatcgattcactaaaaaatgaaaccaaaaaggagatcatcaatatgaacttaaaaacaatcttatacgcaaccggtgccgcaatgggaatcttcacaacgagtgcagtgactggcgcaactgccaacgctgccgttaccccaaccccacaatctcaacaagctaataaaacaaataccaacagccaaacagctaatggcaataagacccaatcgaacaaccagtccaagagtaacactgatcaagctgctaagaagacggatcagagcaagacggatcagaataaagctgcaacgacaacgccaaccaaaacgcaaaccacaccagccaaaaccggaaaccaaaccactacgccagccaagtcaaattcgagcagcaatcagcaggcgaataattcaactcctgccaaaactacgaccccagctaagacaacgaatagtacagccgctacgaccacatttgatcaacgagccccaaggctaaccggttcagcttataagagtgaaaatgccgggtttaaaccaactgttcaaaataagcgcgctaataaaaatgtgactgtcaaatactcaattaacacctacgaatctgacggttcagccagctccaagccgttccaaattaagatttacaaagacggcagcctttacaagacgattaacgcatcttctggtaccgcaaccgggtcattcagcgctcctaaaggtacttacaccctgcgtgtctacaccagccaatcaactcattacactggcggtttatcagttgaataaaaaaatcaaataaattttagccatttaagcttcgtttaagttggctgaggtaatctatagacaatcaaataagagaggagggaaacaccaagcaagcacatcaaaccaaacccctaatatgatttctaatcagctcccagatgactgtctatgcgaaaggaaggatgaactgtacatgtcaaaaaagacccttttaaaacccaagtttaaatacgcatacggttccaaccagcatcaaagatttgtggtctggagctgctactaaaaccaagtaccgagttaattcaagaccgagcgctggaactcactaacccattgaaaggactgatgccatggagaataatcggatttactagcgtatcacaatataatattcacccctcaaataattactaagaaatacccaacaagattgacaagattcttaacttcatgaaatacccctcaatatgaattgaataagaattacccctcaatatgaaatataaaattcccttagaaagtcctgtatgcgagcagggctttctttttgtcttcattcaaatttttaacgtgcatttgattgttggtaaaagcgaagttgcgtacaattagtttagatgttttaattcctaacaaaaggtggtggcaatcttgaagtcgagtgctgaatggtcaaccaggtggactgaacggatcagctatggattaagtgatgcggctgacaatctgatttttcaaatgatgacgacttatttgctgtttttttacaccgatgtctatggtttgacacccagtgcggtcgccatcttgtttgtggtcgcccgagtagctgatgtcgtcgaaagttttatcatcggtatcatgattgaccacacccattcaagatttggtaagagtcggccgttctttctgtggtattcggtgccttacgtggcctttgcgattctgacgtttgtcacaccgaatttctcctatggcggcaaactgatttgggcttacgtgacctatcttggtctgggattcttatacaccgccgttaatctgccaattacatcaattctgccaacgatgtcacagaatactcgtgagctgacactgcttggggttatccgccagttctttggcagttcagtacaaatcatcgtggcagttttcacactgcctttggtttggctattcggccacggcaaccagcagaaggggtttctgggaacgattatcgtgtttggaatcatttcactttttttgattctcaacaccttcgtgcacgtgcgtgaacgcttctccaatccacacattgcccaccaaccggtcaaggttgttttgaacatgttagctcacaaccagccgtggattatcatgtcgattgtgatctttatgtattggctggtcacggcgattaagaatcagacgaccatttattacttcaagtacacccttggcaatgaaggactggttccttgggcaaatggctttaccttggccgctttaattggcgtgttaatgattattagactgaccgatcaccaaagtaagaagaaaacaatgttacatgggatcttgattgcgttaaccgcgcaggcgattattgctgccggcgtgtatggtaaatggctgctggttttgtttgccggtgtctttattaactcaattggaaacggcattatcatcggtctggtctcaattatgattgccgacactatccgatacggtgccagcatggggattcaggcagaaggtattttagcttcaacggatgattttggcgttaactttggtctgggaattggcggcttgattacggccggcttgtttcacgtgtcgggttacgttgccaatcagtcacagaatgcggcgactttgtcgatgattaattggaactatgtttggattccactggtgatttatatcgggatgtatctggtgttgaatttatatgatgaacagcgaattattgatgccattgaaaaataaaattgtggtgaaagtcgatttgataccgcaatctaactaaacaaggcacccatttctgaccttgaaatgggtgccttgtttagttgaatgaccggttccggaaacatttacgagtgcggcgtcctcaactgcatattggtattaaaaaattgtggatacgccaaataacacgatatcgtactgccaatactagtggccgccatgagcataaaggtgaccatgatctggtacataatcgccttcgtagggtcaacaccagcaaagatcagaccagacatcataccggggaggctgacaatccccacggtttttgccgaatcaatcgtgggactcatcccagtccgaattgcttctcgtacgaccgtaatggcggtttggtaacgcgtcgctcccaaagccaacctttccaacaacccttggcgctgatcatggaactggctgttcaagcttcggtaggccaaaccaatcgcaaccatcgcattgctggcaatcataccggaaaccggcacgatttgactgggaacaaaggcaatcgctttcgccaaaaccagcaagccaattgtaacccccgtggcaacggcaatggcaagcagactgatcacaaaagcatggggaatgcctttggcacggcctcttgcattccaagctgcgttgaagacaatgatcgctaccatgagaagtgtcagccaagctcggttaactgagatgatataggtcaggacgtaaccgacaattgtcagttgaataacggcacggatgacgccgattaccaagtctttttcaagaccaattttttctttgaggctgataaaaaatgcgacagccactaaggcaactgcaaaaaataaagcggtcggggtaacaatcaggtgattcatgctgtcacctccattctgccgtcaacaatggtgataagccgatcggctgccgccaattcagactcatcgtgcgtgacagtgataatcgtgacgccttgtttggtaaagttggccatcacttgatggacagtgtcctttgttgccgcatccagcccagttgtaatttcatctaataacagcacctttggcgtgaagatgagattgcgaatcaacgcgacacgctgcttttcaccaccagaaagttccgtaatgttctttgtcagcatatcggcagggagattcacatctgccaaagcttttaccatccgatcgtgattgaccggcttttggcgaatttggaaaggaaaggccagattgtcttcaactgtctcaccaaaaagactgggttgctgatagcaataagataccatgcgacggtacgccgtcgtttcatattcttgttgtggctgacccgaaaatataatttggccttctgtgggtgtgagcaaggtggctaataataacagtaaggtgctcttacctgacccggaaggaccggtaatggtcacaaattctcccggtgccaccttaaaagaaatattagccaatagcgttcgttgtgagactgttaagccaacgttttgtatgtcaaaaattgcctctgccatttttgattcccccattttcgttttctattattgattgtagaggattgcaaatacaatgtcactgataatgattattaatttataatcatactaaattagcttgtgagtcggcgtgacagtcgagtgcttgccgtcatgacataagttgaacgctaagaaaaagtgccccaaatatcatctatcatcgtaaaatggtatttggggcactttgatttggacattattatttattctttcgcaccagctaattcaaacagctgagccattttggtggacccatcagcgtggaagctgaaggcaacttcactgtaagttgcccaattatttaactcggtgtctcggtgttcggcgtcgcaggtcagcagttcatggctggctgtttgggcagtctttttatacgatacataaccattggagttgtacaccagaattgccccttggccggaattgtaagtcgtgatgccatatggcgtgaaataagtcggcaaaacggccatacactctgcgtagccactccccgaggcattataggactggccatttggacgaacgtgacttagcttggtccacagttctttggaacggacaacagttttagctttcagtgaagatcgatgcttaaaagccttgagtcctttcgtcaatcgataagcattaatttgtttcatgtactgtgtgtcaaccttgcgagccaatgttgattcctttatgtacttcacggttagcgagcttggcatgctggcataggtgtaattctgctgaatcttgtggggtaaatagcccttgattgttttgacatagccggacttagtggccggataaccgctggtcgtatacgtgtaggtggtaccaaacgcattaataccatttgaaatgcgggtatacgtaatgggtgcccgcaaagtttgccccgatgttgaaacgtaattaaccgtcatagttttggcggctttagcgttgctgccaaatacggcagccgaaaccagtcccaacgtcaaagcgatgattgataacaattgactgcttgatttcatctatatccccccaatacggatcgaaattattaagaatttcttaagtgtttgcaaattcattatagcaaattatgccggagggcgttcaagaaaaaatgaattatttcgtgattcttcgagtccggatgaaattaatgattcgggcactcgtggtaaccgttgtccgcagcgcaatcccgatgatcaccacaattaggaagtactgcggtgcaaagtaagaaatcagcaggtatagcagactgaatccgagcatgatctgagccgatctgtattcttcgcggtcatgagccgacattttgatcccatctgattcaccgatttcaataacttcgtggaacatgattgcctgggtcaggttcaccaaaataatgatgactgaataagccattgtcggcagctggtggccaaaatcgtcatttaaccaagaggtcgcaaacggcgtcaaactgatgaagcaaaggtaataaatgttggtgattgtaatcaaagacgttgtatgttcgatgcgactaaatagttcctggtgatagacccaatactgagaaacaatcccaaaactaacaaaataaatcaccaaatgtttgatcagatccagcattggtccctgcgctgtactgattggtgttttgatgtccaacaccataatggttagaaccacagcaaagatcccgtccgaaataccaattaagcgtgattttgaatagtgaaacaccccgaccatccccctagattagtgtatgagcttattttacagctctttagtcggagagggtagtttagttatgaaataaatggttggttattgttctttttaatttgtaggtatattcaattattgacctgcaatgtcattaacatattgttatcaatatcaaatcaaattagttatgttttttaggatagtgtgataatattattttgtaaattaaacgggaatggaattcatataggagtgatacttatgcgtgttttagggaagagttcatttattacacggtttcaacaggcgtgtgtggccgtggtagcattctttgcagttttaacaggccttggattttcaacaacgtccacggccagtgctgcaacaccttcaaaggatattttgcgaccgacacttgcgataactggtgatgacgctaatgggaagcagcagacgattgcttcaatccaaagtgttgccgatccaacaactactcatgccttgctgaatgtcgataaatattcaaacatatatgcgcggtattcagttacaaatgacttgggatattcgttgccggtttggaattttgtccatcttccgtggttgtttgatcacaccgccaataacccaaaatccttagtttttgacccaagccgagggaacccggaaatgaagtcaattgggtttgccagcgatctcaaagaaccaatgatggaatcatggtcatattctcaagacagcagatacgttttacaatatacaccatcagaagacttaacaagtattttttatggtggaatgactgacacaagtagtgtttggccaattcagatggctgcaaatgcaagagttgagatgacagttccattgaaactggcaccggattttgattttaatccatcacgtatcgctcgatttagaagtgaaatgcaattctatacggacaataccagcgtggataaggtggtaaaaaatgaaattacactccaaattactcggactctcgacgttgccgacttcgaatccgaaacctacgcaacgttaaccaacgcggataaattcgaagggatcaatcatatgtttgatgctgatggtaaggaacagccggacaagaccaaagccgacgccaagatcaccccaactgatcaaaaaggcatttacgatgttgcctacacttacgatggggttaccaagaaagtgaaggccactgtcaaagatcaatcaaccatcgaggctggcgactttaccatctctcatggcagcaactgggacactcagaagtttaatggaattaagagtttgaccgacgctaacggcaataaggttaaatcgccaggtaacgtgaagattaccaatatcaaagacgcagccggcaaggatgtcgacaaggttgacaccaacgctgcagagaaaacctataccatcacttacaccaatggtggcgcttctcaaactgtcaaagtaaccattggcaaacgggccagtgtggtgacaccacctgccagaaatacaggttcgacaagcagcacagtgaaggttccgggacgaccagttacggataactccaaagctagcggtggcaatacccagacatcaacaaaccagcagcctgccaacaattcgcaaccagaaattcaggtttcaccaggggtcgctaagaaaggcgctgctgtgtacgccaagaagacaatttatctgcacaagggcgttaatttcaagaaagcggaccgcttggttaaatatcacaaagcacaacgtgttgatcgaccgatgtttgtggtcacaggatatgattgctcaagcaaaggtgccttaagatataaggttcgggatgttaaccataccaagaaatctgatggtaagatcggctacattacggctaacaccaagtacgttgtcaacgtatactaccagaccatgccaaagaaaaatcagctcacggtgatctcgaagaaaggcgttcatgcctataagaacgtcaacctgaccgggaagacaaagacttataagaacggtagccatctgcgggtcaagaagattgtcaaatatcatttaacgactcgttatcaacttaccaatggtgactacatcaccgccaacaagaaattaattattcaaggaaatcactaaattattttccagaaaaagtcctggcatccgctgctcaggacttttttgatgggtaaaattctcattacaaccgatttgcacacaattgtaagcgctttgtacttaactgatcgacttcccctaacatgatcgttatgtaataatatattaaacaaattagtactaaaagtaggaacaaagtggtactatgtgggtggagtggggaaagtatgaatatcaaattatgagggagtgtttatgatggatagccgaattagcaactcatcaaatttgaagtttcgaacaaaacacagacggatatggaagatcctaacggggatggttaccacaatcgcagtcgcgtgcggattgggattcatgcacgcttctgccgatgatgtgaccaacgttatcccgcggaccgatgaattcaatattagtaaagtgaatccactgcaatacacatacgtccatgagagtctcagtcacttgggagggtggcagggggcagcttatgccgccgcaattcctaacgacgccaagggaactgatccgaagaccggcaactcgtacgtcagtgaatggatgccggatcctggacttgagtatttcatttggcaggcagcctttgcggacaagtacaaaacggcggaaagcttttttgccaacttttcaaaaaatgatttgaaggatcttgagtcactttatagcgaaatgggcccacaaaatgccgggaccgactcaaatccaaaaccatcccagtattatatggctttaatgggaatgaattctcttgagggactgcaatatgcaacgaatctcaaacagattaatctggatcccaacgcggctgtcagtgcggcagcgtttgggacaggtaccaaaaatggaaatttgtgggatatcagcgcgctgaaaaatttgaatcaattacagtcggtgatgatccaaatgttttcaattaacgacgtctccgctctggccaataaacctaatttaaccaacctttcgttgacttacaatcaaattgccgacttgtcacctctggcaactaacaaaggcaataaaggactgaatttgaagacagggttcaatcaccagcacattcttttggaaccggttactttgcggggcagtgccgctacggctgctcaaacgtcgtttacgactccgtcctttatcatcaaggatctggaatccgccaatttaccggtcaaggcgtttgacatcaaaagtgaaaagtctgattacccaagtttgtacccaagcacctctgatggcggcaacatcaatccaaccactttgacgtggacaaacttcttaccagacaaaaccaacttgtatggttcgttgtccagtcactggaccgatcccaactctgattttgaaggctggattatggtaccttatcagtttaaccaaacggtcgggaatgtctttgtgaactatcagctgctgcagtccaatggaaatcaactccagttggccccaaccagcacaatggccggaaatgtgggggatgcctataatattggcaataatcctaacacggcttacaccctgaataaattaatgggagaagacaaacgggtggcaattggcgtgtttgatggcaccggcttatatgccgatttcaaagccaataacggtaaagccaacgcggttggccagtccggaacgtacaccgatcttcctcagacccggacgattgtgtttgcatcggattcatcaaccgtcacaatcaactacgaggaccaagacggcaacaagctccaagattcaacggcggttaccggcaagaccaatactgattttaccttaccgacaattccttcaacaatcaccaaagatgatcaggtatacactttgaaggggctcaaggaaggccaaacagtaccagcgaaatttgattttatggacatgtcactgacctacgtgtatgaagtcaagccaaccgaagccaaaccagtcaccgttcggtacgttgacaaggacaatatgcctcatgagatcgggccacaaaaggttttgaccggcaaacgggatgacacctttaatgtgaacagtgatgattacaagttgaccattccaggctatacattcgcaggtattttgggcgatgcgacaggaaaatttggtgacgatgcgcaaacgatttacatgcagtacaccaagaatcctgtccagccaaaatcagtgaccattcggtacgtcgatattgacaacctgcctcacgagattggtcctgaaaaagtgattaccggaaaaatcggtgacaactacaacaccactgaagctcagtacaaacttgcaatcgatgggtatacctttgtggatatccaaggaaatgcgacgggtcaaatcagtgaacaggggcagacggtctactatcgttataaacgggatcaagcgaaaaatgaggctaaaccgattatgattcgttacgttgatgcggacaacatgcctcatgaaattgcgccaaccagaactgtagccggcatcattggtgacaaatatgatgtccgtgacaatatgtataaactcagcattaatggttatacctttaaagatatccaaggggatgctaccgggacctttgatgccactggccacacggtctattatcgttacaccaaagataaggccaccccagtgacgccgccggttaacccaccagtaacgccggtaaccccaacaccgacaccacagccgacgccacaaccaactcctcagccgaagtcagaaccgacttcacaggagacggtgacggcaccaaatgaagccggcaagattgccaagaaaggtgaagcggtctattcactgaagaagatttacctgtatcggcacgctgatttcaagaaaggcgaacgaattgccagctatgccaaaaagccgcgggtaaatcggccgatgtttgtcgtgagcgattatgccaaatcaaagaacggcgccctgcggtacgtggtgaaagatgtgaatcaccacgccaaatctgatgggatgaaggggtatattaccgctcggtatgcatacgtccgcccagtgtattaccacagcaagcaccaagttctgacagtcattaacccaaccggcgtcaatgaatataccaaccgaaatttgactggtaagattaagaacttcaagcagggcactcaactcaaagtgaagggatttgtcaaacataacctgactacccgatacctgctgagtaatggacactatattaccggtaaccggaagctggtatttgccggcaaactggttcaaccaaccaagattaaggttaaacggtcgatttacttgtacaacaacgtgaacttgaataaacgattgaaacacatcaaggcaggaactgttttgaaagtgaagaagtgggattactcccatcaatattcaacaacgacctttggtgccaaacgatatcttgtcagtggtggatatgtcaccgctaatggacattttgtgaagattgtgaaataaggccgtattaaaagcttcggtgtcagtagttggcatcgaagctttttgatttggacggagtcgttattttacaaattcattgatctaatcacgattttaaaactggcacttccagcgttgaatcgtttaagttcaatgtgtaagtgatggcttgattaccgtggacggtgtagaccaggtcactggcatagattaccaaccccaattgatggcctttgagtaagtgccaaaaggttggctggaaggcaaagcgcaacttataaccggtttgtggctgcacatcatcgacgcgataagaattttggcggttctgcatgttgatgtgagcttcggtgattcgtttaaagtcggttgggttcgtctgaggaagaaattcttttaagtcatcctttcgccaatggtaaccttgcaaaatcttttgggaaaccagcgtttgagggacttcagttaatcgctgatcctcaccgtagtcgacaagggcaacgctgatttggccgacaatggaactggtttgggcaactaacgagatcgttggttggccatcaattgtgatatcgtgtgtcagtgggtcggacaagagccgaatgcagtggttgtccatggcggtgccttggcgtgaatataaatcattgcgccagtcattgaggtgctgggtgtaatgcttgaaaacctggtttggcagctgatctgagaaactgaaattgcctttgatgttattcaaactggcgagcgagaaagtgcgcttagttgattcagatccgccccagtcaggatagttatgccacgtttctgcgtgggcgttgtcctgaacgattacatctggcatcacgtcgtcgacccgattttgaatcccaaatagtttgttggacagccacaggttcaccagatcggtgtaatcaaaggagcgaaaattgttgagatactcgtgctggccttggtgaaggatcaatttttgcgtgatatctcgggtctttaacttattccgggaattccagacttgaccggtcttgacgttccaatcattcaaaccgtgaaccagtagcatatccgccttggtatggttatatttggtaatgtttcgggcgtcccaaaactgattgaagctgccggtatcgtgttcttggtcgtgagtcatctgtttaaaatgcttcagccaagcatccttgatttggacataatccccagcggtctgttggcggctgaaagtccattcggctaaaacgtcggcatcatcgccatctggggcaaccaccaggccgttttcccgataataagggtagtaatcggataagccggcctccacgatgctggtttttaagccgtcaacgccagtaaacgcggcttcggtggcaagtgttcctaaataagagcggccagtcatcccaacactgccgctgctccaccaagcatcaatcgcaatttgatcggagcgattggtaaaggcagtccggttgccgttgagccattcaatgaccgccgttgcgcttagggtctcagccttggtaccagtggtccggaacccgtcagagtccttggttccgatccctgatgagtaaacgatcgtgaaacctcgcgccaaaaaataatcattgagagaatacgaccaaaacttggtaaaggtttcaccagttttagtcgttcggccgttaatttttcgcggcttgggtggggtgacgttgctgggttgtgcttcaacatcttgataggttaggtgattcggttgttttcgcttgagtggacgcttgttgtcgtgggagaacttctctgaccatttttcgttcatgccttgggcgtatgggtcggcagtgaagataaccggcgcttggtagccctcgttggtttcagcaggccggatgatattggtttttagcagatcccgtttaccgtcgtggtccgagtccagggatgattcgacgtagacgacttcgcgaattaatttatctgtattgaaaacggcttgggctttgccgttgaagaatagtggtattttgaaatcggaatcgttgagcaactgctggtaataccctttgccagctatgtagtcgatcaggagttgaccgtatttgttccgggtattcaacaaccgataccaagcatcgatcagctgatcacggttcatcgttgactggttcaacggtttcggcaggcccagttgcgtgatgcccttgaacggagcttcgagggaaaaatccaatccgtctaagaatcccagtaattgcaggccaatattatagaaggctttagcggacacggaaccagttgccttggtaaatgttgctgcatcaatcgtttctgttgccattaagttatgaatcttttccagtcgagtggttagggaagcgtgctgggagtagtattccagcaaaaaatcgcgatagagttccatcggatcgcttatcttaagattggccggattcaaaaaatgaatttctgtcagttcattgattatttgttgatggttggtgggggcatacccgaattggttaattttcattaagtgacctcctgaatgtaattaatgccattatacatttgcggcttggcactgcaaaattaatttaaaaagcagcgattccgcttggtggttaaggaatcgctgcttggttattcacaagtttttgaggaggttaatctcaaatcaaattggctggtggggaatcttttagcctggggatgctgtgctactcttcatgcttttcctgatcggactgttcagtgtcatggtcagtgggtttggaattttgatccggctcataggcttgagccttagcctgcagcttcttttgcttgacttcgtgcttggcatcccggcgttctgctcgccgttgggtgcgtttttgatgctcaagaattttatcttcttcgtgagcagcccggcgcttggcctttgcttggcgttcaatatctttggcagcctgcttggctgattccttatcagcttcctgttggcgttcggtctccttagcggcttgttttgaggctttttcacgggcttcacgctgaatttcggcttccttggcagcagcttcggcgtcatgcttgcgttgatcttgctgctgttcggcttgtcgtgctgcttgcttgacggcttctcgattggtatcacgctgttctttacgaatttgttcagctgcgtcacgatatttcttggaaccatcacggatttgcttggcaaattcttcccactgtgcctggcgctcttttctgacttcgacgctgtctggattattgctgggagcgtgtgggttgaccgaatggccggcactgtcggtggcgaccgggtgatcaagccaaccgctaaacccgtgttgaggatgactcgcgtttgacgttgttctgtcagttccggttgctgcctggtcctggaccatttctctaaattgattaatggcgttctgcggcagcttcaagtattcctgtcgctgctcggtggtcaattgcgaagcatcgtacatttgttgacgatcgcggctgcttaggatcatatagacgattggatagggaaggtagaaccacaagacaacctgtgggaaaaaataggccaggacaatcaagacggcgttgaaaattaaatagtattgattgtgacgcccatagattttccgatacagctggcgcatttttgatttgtcagtgtactcaaagtgcatgactgatcgtgccagcaggcgaaatgatgctgaaaccaaaaataacaggagaccgtatgccatgaccggaatccgggtggtgttgctggccatcatgttagtggccagtggtgtcagtgatagtgggattaagaagataaaatcatacaacatgattcgataactcatatcatcaatgtcattgaacaaggtggcatgctgataccacatgttggccacaaaagcgaagctgataatatagatgccaatttgtttgcttaaaaacaagtaatcattcaagttgtcccgcaagactggtgttagatccaaaaccataattgtcaaaataatggcgatcaccgcgtcgctaaaagcgtccagccgactcttcaactttttcatttgttttgcccccagaatcgatttagtagtatgtattatgctttaaatgtagcacagtggtcgtcaataaggtgataaattgtttaagaaattttatcagtctcacaaaataattgggtggcgatataataaaactaattaaatgattgtgaaagaggtggcagtatgtttccttacttgggtctcaaagccagtaccaaccaagcccaaattgatgaacgattaaaatatcatcctgaagtatttgaattcttcaccaccgatcaggatgtgacgccaagtggcctgaaccatttgaaggcgatgattgaacacgtgaaggccgctggggtcgacagaattgtcatgcaccacccgatgaagtttaacggccaacacaatgaagtggcagttgaccgattgagtaatccggacgcttaccactttttaatgcagagttctgaaaatttgattcagctggccattcagactaacacgcaagttttgattcacggggcctacaactcaccggtttcagatattctcagcaactacccttcgattgattccgcccgcaaggtggtgttcaatcgcttggaccattttaaatcactgggcggggaccatgtgatgtttgaaaattccatttcaccgctgtttgattacggcgatccagaaattgaaaacctgatcattgagcatcaataccggctgtgctacgataccagtcatgggttcattgtgctgcacggcaataattcgaaactcaaggccagtatggcgcatttgcgagatcaggttgtccattatcattttgtggattcaatgggccagttccacgacagcttggaactgggaaagggcgcgattgattggcagcctttaaaatcggtcgtcaatccggacgccaccgatatttttgaaatcaatctcaaagaccaaatgaacagtcaagaaatgcgtgccagctatcagtacctacgagcatgctggcaaacatctggttgattttgttgtaagatgggagtagttggtttgggggagttacatagtgaaatttaaaaatgtctttgcatttatcattgtttcagtattcatcgtcatggccttggccgctgctcaacattcatttgcagttcggaaggcaacaacgccaagtgatagtcagaccaccattcaaagtgtctattggaaagcgccgtctgaaaacaaagcttatccagaatggtccaaaatgagcaagccttggatttatgtgagtgtcaaacaacagaaagtcttcatccatggtaatggcaaggttcaatacattatgaactgttcaactggcatccccagcagcccaacgccacggggaacgttccatatccaaaaggaacgcggctattcattttataacaagcgctcacacgaaggcgcccactactgggtttcctggttggatcacggcgtctacttattccacagtgtgccgaccaacgcccacggtcagtacgtggtttctgaagctgagaagttaggcactcccgcatcccatggctgcgttcggctatcaatcgctgatgctaaatggatgtatcaaacggtgccgtttggaactaaggttgttgttcactaatgaagtcatatagtcattattcgatgaatgaggctgagacaaagagctaatctgtttgcctcggcctcattttattaattaaacaggctgggatttccacgccgacaaagaatgatcaggcgttctaaataattaactgaaagaaggttctaacatgacattgcataccattttaaccccagagtggattcatgaagccaaattgattgccgccgagaatccccggctggagggctttgttcccagcgagggcggccttcatccacgaattctcttgttgggtgaagcccctggtgacaaagaggtcaagattggtcgcccatttatgggaccatccggcaaagaactggatcgttggctggcatcgctggggttaacccgtgaggatatctacattaccggagtggtcaattcccgtccattttcaattgggaaaacgggtcgaaaaagtgaccggcgccccaatcagaaggaagttaagcgctcggctgcgatgtttgactgggaactatcccattttcctgatgtcctgttggtgccaatggggaatgccagccttcagcggttattaggtaccaaggccaaaatcggtgatttacatggccagttgttggaacgctcaattcaaaaatataaccagcagacggattcctttgaactctctaaggaaaaacatcaaatctttcctttgtatcatccatcgtattcgaagcggttcaagaatatgaagcccgtggtcgatgcggattcgcaaaagctcaaacaattactcgaacagcaatcaaaccgtcattgaacgccgaatatgggctggatggtgttagtctataatcaaatagtgttttgaggaaggtgaggatgatggcaaaaccgttaaatggcgttgatctctatcattcattatttggcactgagattcacgatccacgcgtgttgtttgaaatgctgacagtgaacgtttttcagccaggattaaattggcgggtggctgccagcaagattccggtatttgataaagtcttcaagcattttgacgttcacgaaatcgccaagttcgatgaaatggatctcgaagctttggaagccgatccagaaatgattcgaaacccccggaagattcgggccgttgttcagaatgctcaagcaaccttaaaactgcagcctgaatttaaagatttggcagactatttgtggtcgttcgagccaaaagatgatgtggttcgcggatcattgcagcaagattcccatggcttgggagttgagctggccaaggatatgaagaaacggggcttcacgttcgtcggtccgaccacgatggagttgctgctgattggcagtggcattttgaaacatgaacatgattaggaaaccttcaagcagactaaaagagagtggaacgcgaggcgttttgatcccagaatttaagccaagaatcgagttattcctgttcttggaatgactcgattcttggcttaaatggccgggatcagccgatcgttgcacgtttaaactagataccagtggaactgaagaaaggttgaaacataacttacgattagttgtgtctcagcctttttttgcgatctaatgctcagcgtcaggattaatatagttccacaatccagtttttgtcttggtcgctgtcatccaaatactccggatgatcgatcaaagcagtgttaattttggccactttaccggcctttggtgaatggacttccgtgactgctttagccccttcaaatgagaggatgacgtcaccttctgcaactgcactgaggttctttgggaatgcagcgaaggaaatttcaccaatttcaccccgcgccaggtcatttaacccaattcgagtatgtgaatcatcaactgttgcctgccagagatattttgaatcatcaattttttgtgccatattaatcttcctttcgatttttaacgttagagtgacgagctttatagaatttgagaatctgttctgtttttgaaatggcattgccaaggtggccgtccgacctcattagtcggtcaaggtcatcggaacttaaatacttggcaatggtggggtcagcgtaaaacaagtcccttaaagtgacgtgttcacgatcagcttggtcacgcagtttcaccagtagtccgtgggcgttttctctgcccatgtgcttggcgagggccatcatcaatgatccggagtacattgtgccatcgtcagcggataagttttgccgcatgcgttgaggcttaaattggccaaatttaagaatattaatggcgtagttcaactggcctgaaaggtacattgtcatttcagggagggcaacatataaatcacgccacacggtggtgtccttctcaccatcaactgacattgtgtcgtacatcagacccatctcgtttcgaatgaccgttgccaaattgacgaccgcttcgaccatatatgggtttcgtacggtgggcacaacagttgatccttggcggccgggcgcataggtttcctgaaattcaccaacaattatctgactcatatagagtaaattcttgcctaatcggcccagtgcctgggcaatcatcgtttcgacatggcagtattcagtgaatcgttcccgctgcgtgtgccaatacatttccggttttgataatcccaagcgatcacaaaaatcctgttcgatctgatcatagtcatcacccagcattgaagacgtcccgtcggcacccgctaagctgccagcgaaggtaaatggtgccagtgaatcaagcttgcgcatgaggtagtccaattcattcaaaacaatcccgagcttgaatcccagcgtggtgggggaggcgtatgttttgtgggcgacggcggcagtgacagtgctcttgtatcgttcacacaagtcataaaggaccgaaccaagttgatcaagataatccttcagcacccggtcagactccttaagttgaaggacaaacgcggtgtcttcgacatcctcactggcagctccatagtgaatgtattgcccgctgtcgtcatcaaaaagtgactgacaaactgtgacaaatcccgccagaaagtgtccagctctggctgactcaatttttaactgcaccctatcaatattttctggaaccaatttggcttggatttcttggtaggctttatcagggatcttgccgtttttggccattgcgtaagccaccgccgtttcaacttggcaaatgactttcactcgattttggtcagaccagatatttcgcattcgagccgttgaataaccattttgattgtacagcgaacctagcatttcaccactcatgttagttcacctcctgaaaatgaggattaagcattaggtcggccatttcagctgctgaaatggggccaatgttagctgataaatttgtcgttctgaaggcttcttccaggttgtctttcttaaaaggcgttccgatcagcttatcctcgattactttcaagtgaccattggcctgattaaagtcgccaaagatgcgtgcatgggtcacgatgccatcatctactgaaaaactgatttcgaccgtgccgagaccatcaaagtgattcccatggaagaaatcatcatcgcgtttggttcccataatgaaatccggatcagtgaacttgttctgagcaattagttcaacctgctgccaatccgcttcagacattgtataggtgggaatagttgccaagtcagtcgtttgaaagacttcttcgagaagcagccggcgaatttcagcaaaagtgatttggcgatattgtggtaggaaatactgacgaatgttggtaacccggctgtgaaccgacttgattcctttggaggccaacttggttttgggtggggttagtgcttttgcagcctgatccagatcgacgtctatcatcagtgttccgccacacgagaatcggttgccgattttaagcgatgacatccccgaaaactttttgccgtcgactgtgaggtcatttcgaccggtcatttccgcgtccaccccgagcttgtgcagtacatgaatggctggtgtcgcatattttttgaagttgaggtaattcgtgccatcatcgttatcgataaaggcatatgtcaaattacccggatcaacgtaaaccgcaccgccaccggcaccacgacgtgccaaacgaatatcgtgggtcttaatataatctaaattaacttcggagtatgcgtcctgattgacgcccagaacaactgatgcggccgccggttgcgaaaaatgaaaaatcgtgtcggtaaatttaggcgaagtgataaaaaacgtcgagagactgccgctgactcccgggtcgcgcaaatgcagttgtgaatttggatcagataagtcgacaaaaataatgattctcagtcccttcaaaaaaattcccctgttaacgattacatagaaaagtatagcacgtccgggttaaaataaaaaagagcggaataccccatcacaatggctatttccaactccctattaaactaaaacgataaaccgattatttttaaaaaagctccacaatccaagttttgtcccgattatcctcgttcaaaagttcgggatgctcaattaaatctgagttcactttggcaactttgccactcattggtgaatggatttcagtcacggctttggcaccttcaaatgacagcattggatcgccggcacttaattcagtcattttttccggaaattcggcgaaggtaacctggccgatttcaccgcgggccaagtcgtttaagccgattcgagtgtgtccttcactggttttttcttcccataagtatttggaatcatctgctttatctgccatgataatcatcctttcattatttaagatcgtacttctcttttaacattaaatctgccatgtcaggtggcgttactttgccgatgttagcttcaagattgctgattctaaaggcctcttccaagctgtccttggcaaatggcacgttggtaatgtgattttcaatggctgccaaatcaccattgggattgttgaaatcaccatagatttttgcgtgagtcacgacatcgtttttgactgagaaactgatttcaacagttcccacgccgtcaaaatgacgaccgcggaagtaatcatcattgggtttggtgcccatgacgaagtcgtcaccggtataggcttgatcagcgatttttaagacatccttccaatcatcatcagtcatcgtataggttggtacatcacgaatatcggtgactctaaagacggtcagcaggatacgtttttccagttcttcaaaggtgatatttttgtatttcggatcaaaatactgccgaatgttggtgacccgactatggacagatttgatgcctttggattgcagttttactttcggcgggtaagggctttggccgctttggccaggtcaacatctaccattagagtaccgccgcataaaaagcgatccccgatttttaatgccgacattcctgagatttttttgccgtccacggttaaatcatttcggccggtcattttggcgtcgacacccaatttcttcagggttgaaatcactggttgggcatagcgtttgaaatcaccataatttgagccgtcatcgttgtcaataaagacgtacgtcaaatttcccggatcaacaaacactgcaccgccaccggcgaaccgtctggagagttgaattttttgatcacggataaagtttaaattaacctcggaataaacatcttgattcaacccaatgaccaccgatgcctgtgggggcctggaaaagtagaaaatcggttcagtaaattttggactggtgatgaagaattttgagagactgtcggtgatgatcggccggttcaaataatctttaccactggaaatatcaacataacggataataatcagctcctctgattgaagtaagcggttacaaaagaattcaaaaaacaatgcaaccgaaccttgactctgtctaattgcattgtaacccattattgggggagttgctcgaaagttaactgaaacgtgcgggtcacccagcccacgtggcactgtggttgaaatgtgctgcgagcaactgacactgcgatctaagccactttgattcaaatccaaacccgggatttcaatcaaagcgatcttagctctctgtgtcaaaacgttgctctccgcactctaatcaaaatgtgctccgccaagcagcaacctgcacctaagccaactttggacaacaccaaaagcgattttgtccaaagtcagcttaggctccggttactaaccgctcggctccgcactctatctcatgtccaacggttgcttactcgttggctttggaaattcaacatccaattgagccaactcattatcagttaacgtaatatctgcagctttaacattatcgaccgcatgcttggggtcacccgattgagggatggccaaggtattgccatcgcggattgcccaagccaaaataatttgccaggcagttgccgaatggttgtcggcaatttgtttgacgaccgggtcattagtcaaacgacctcgggcatcaccagctgcaacaggtgtgtaggcaatcagtggaatatgccgttgtctcatccaaggcagtagggtgtattcaatgccccggctgccgagattgtacagatcttcattggcggcaacctgatcggcattcggcaaatccatcagttcttccatatcagaaatgtcgaagtttgaaactccccaatgcttaatttttcctttttgctgcaattgctggagcgtctcgatggtttcactcaaaggaacggcaccacgccaatgatacaggtataaatcaaaatagccggtcccaactaatttcaggctggtatccaggctgtgttccattctggaagctgaggcatttgacggcaggactttgtcgatgataaacaaatcatcatgctgcatgtccttgatggcctcgccaactaagcgttcgctgcggccgtttccgtacatttcagcggtgtcgattactctggcaccggcagcaataccatcttgaattgctttaatttcatcagcccgggtgctggcactgtctcccatgtgccaggttcccaaaccaattgcgggtactgttgaaccacctatgttcaattctctcatagactgtcatacctcctaattttcattagttaatagtataaccctgataatggcattcatcatctaatttttaaccactcaaaaatttgttggccgactgcttcgggtaaatagcgaatttcaaacagttggttgccattgccatggcggacgttgaccctgatatgcgctaatttggtatgggtcatccaaattgattggacaaataaaaatgactggatattcttgtgaggaatcacgtattgcgaccgggtgaagaaatggccgtcttggagaatcagctggtcgttgacaatcttccagccggtattggcagctgaataccagcccatcaaagccgcgatgacaaccaccggcaggctcagtaatccccacaatttaaagagatatagacaaggcaggacgatcaccaggctgatcaaagtggcattgcggatgaaataccagtaagttcgtttggctaaatgatccaattggctgaagtgagtgggcgcccagctgacgaagggatgcagggtgtcaaatacacgatcggttttcaccacgggtaagatcattaaatcattgcttttctcatcatccccagccgatgacgctgccagtgcttggacggttgaaatgtgacaccactggcgaatcacgttttgtttaattcggagtgcttggatccgggcaatcggaatagtaactgaattacgttggaatagaccctgctcagttttaagctggtcgtttgtggaattcaggcgaaaccgatagtatttttggacgatggttaaataggaaccggcaatactgataatcacaattaacaagccaatggcgcacagaatgattgcagactgatgaattaatttcgcggtcaaggaatcaattaacttttgcggaatggcttcttgaattttgccgtagaccgcaaagccggccccgataatcggaaagacccccagtgaggtcagtgcgaagatgtttagttcatgcgggttgatttcgtagtcggcatgttcagggcttggttttaactgttcggttaagtgttcagctgcaggcgctggttcggcgtttccggtgcgctgacgttcaatttctgctctgacccgttcgttaactaatggcaaaaccgcttccggtccgtgctcatcgtgaccagccgtttcaatttgaagcttttccagatgaaatgggaccaaaaagaaccactgggtgtgctgaattgtttgaatccgggtgtatggaatgtgtgtgtgtcgtttgacgaagatgccgctgttaatcgtcagcatgtccgagtcgatttcaaatgtaaagcacaggtaacgaacggtatgccaaagaatgatgagtaggataagaacgctgaatcctaggagtggcgcgatcccaatggctgttgaccagcgggtaatcggcccggatccaatgatcagcagaagcagtgtatcccaagaatgctggaagataaagtagatgattgacaatgggttgagatgctgtcgattagacgtcattgttccgcacctccaccgccaaattcataatttgtttccggagttgttcgccaacttccggttcgacaccatcaattttgtgggacgttgaggccgtggtgatgcggacttcttgaagcttttgcgactgtaaaatcggcccggcagaaagggtcacgtcctggactcgggcgatgggaatcgagactaacttgcgaaagataaatccggaccgcagttcgacggcatcatcggacagggtgtacagccaaaaagaataacgatacggaaccaggctcatttcgacaacgaaattaatgacggcaacgataaaaaagaatccggcagcgtacagtagccattgatagttgaaaaaatagtgaatgatgaccccagcgaccccgacgccggctgacaacagtgtgttgaagatggccgagattcgccaaacggttttgatttgggcgggtaaatgatttgattcattcatgtgattcgcctccttaacgggaaatacgatatgtcgtgtgttaagtttacaaaagaatgacgacaattaccatccgatgacttttgaataagggaatcaatccggtagacgtaacgcggtttatagcgttatacttacttttatgcttttcacgaaaatcgaaagggggctatcaattgtcgaaaaaagttagaaacgcgataattgtcctgatatttggaaactttctggtctgtattgggatgagtctgatcttcccggtcatgccatttattaagaacgaactgcatttatccgccaccgatatggggatcatgaactcgctgtttgcaatcgcacagttggttgcctccccaatcgttggtcaaatctcggataaaattggtcgcaaaccaattctggttgccggcctgctattatatatggtttcagaaattctctttgccatgaccaactggttgtggatgtttgatatttcccggacgatcgggggcctgtctgccgccatggtggtaccgaccaccaacgcattggctgccgacttgaccacgccacggcagcgagcccgagtgattggcttgttgtccgcggccttcagtggcggcttgattctgggacccgggattggtggtattctggccaagtttgattataaaacaccattctggttcgcagccggattaggtttcttgagtatgctgtcattgtggttaatgctgccgaacgaaaaagaaattgagaagattgctgccaaccatcaagttccggcgcaaagcaggccacccaagcgggcgtcttggacgcaggcaaagaagctgtttgcagggccgatgggactactgtttcttctgattttaatttcttcatttggattagttggcttcgaaagtatttatagtctgtatgtcaacgaagtttttggcttcacaatgggcaatatcgctttggtattgacgttaaacggactgacctcgctgacatttcaagcgttgctgttcgacaggctggttgtttggctgactgaaaaacgcctgattcgttactgcttcttactctcgtttctgggcaccggctggattattctggcgcactccaaattagaagtgatcattgcaactttaatcgtgttcacagcgtatgacttgattcgcccggcaattacgactctgctgaccaaagcaagtgccactaagcaaggtttaatcaatggggttaacatgtctttgaccagtgtcggcaacatcgttgggccgattgtttccggcgcgttgttggatgcaagttatcacctgccgtatctggtcgtgatcgtcttcctgtttatttcatggatcatgacgtattggattcgggatcatttctcagttgatttgactgagactaactaggcttttcctgctgtgagtgggagaagccttttttgctgaatggaatcggcagccaattttttgaaatttagacgacattttcctatcatcgcctttcataatcagttacaatgaaagcgcatactggatatgcacaaatgattttcacaaatggaggtaacaattatggcaaagcaagttgcattagttactggagcaggtcagggaattggtgaagccatcgcgactcgtcttcacgatgatggattcaatgttgccgttgttgatttgaacatcgacaatgccaacaaggtagccaagaagctttcaccagatggttctgaatcgattggcatcaaggccgacgtttccgaccgtgattcagtcatcgctgctgtaaacaaagccgtagatgaattcggcgacttcaacgtaatcgtcaataacgctggtctggggccaacgacaccaatcgatacgattacccccgatcaatttaaactcgtgtatggtgtcaacgtaggtggtgttctgtggggcatccaagctgcacatcaagcatttaagaaattaggccatggcggcaagattatcaacgctacttcacaagctggcgttgtcggtaatccaaacttggcattgtactcaggcaccaagtttgcggttcgaggcatcacccaggtggctgcccgtgacttggcagaagaaggcatcaccgcaaatgcttatgcaccaggaatcgtaaaaacaccaatgatgtttgatatcgcgcatcaagtcggtaagaacgccggcaaggacgatgagtggggcatgcagacattcgcaaaggatattgccctcaaacgtttgtcggagccggaagatgtggcagcagctgtatcattcttggcaggtaaggattcaaattatgttaccggacaaacgctgatcgtggatggcggaatgcaatttcaatagaagtgtgcgacgagacccggttaggacccggcgtacaaggagaaacggtcaatgatgaacgggctttgttcatcgttggccgttttttcttgtacattagggccctgggtcgtcggagcatagctcaaaagcagaagggagcagaaaataaaataagtgccacaaaccctgtagcctctttgaaaaggtattagtggagtcaaaaaaaggaccagtgatgaacggtttttgttcattactggtccttttgacttgtgtagcaggggtcaggggtgtcgcccacggggctaggcaggctttcagccggccgtcggagcatgtgtataaggcagaagggaggcgtaactccaataagttcattcaaagctgtagcctctcttaagcaccactgctatcgagcctaaacgtgcagcaaccggctgatcccggccatttaagcgacgaaacgagtcattccagaaacaggaataactcgtttcgtcgcttaaattctgggatgaaaacgcctcgtcccctactcagggcataatcatcttaataaaaatcggcgtaatataagtttccacgatcgcagctacaaacagcagcggcatcaccaggaccagtgtatccgtcagcgtctgcttcagcaactcaatatatttaatatcctcgcgtttacgttttaagaatttattcatcccataccatgccaaccgtgcactgatcgcagcggcaatcacctgggcagaaatttcaaaaattccgtgtggcaggacaccaccgacaaacatcaggaaaggactaccaacgatcgaaatcaccaaaccgacactataggcattttgcaaaacataataccaataaatcggtagtgcaatcacacccaaggcgatgacaaccgcggcaccagcgaagttccagaaaaataatggcaaaaaattagtttcgctgggtgctgttttatcaattccattcgtaaagtgatggactagactgccggtgtccatgaaattcttggcatagatcaacacgatgatccagacgattgccatgacgatcagatattcaacggctttcttaaaatagatgcttttaaaacgatcaatacttcctctaatcataacctgtcccccttgttttctataatgaaagtatacagttgaattgtccacaagccaattaatgtgtcgtcgtgttttcccttcaacaaatcattttcattggccgcgggcggtatggtatgctaaaggagtaccaacattaaagattggagatgtttgttcttggacggattacaatcaacaattaaattaaataatggtgtcgagatgccacgcttaggtctcggcgtttggaaaaccagtaacaacgattcacgagacgcagtcattacagctatcaagcatgggtatcgggcaattgataccgcacgtgaatatgggaatgaacccggtaccggtgaaggtattcgtgaagggatgcaacaggctggattaaagcgtgaggacatgttcgtcaccaccaagctgtataacggtgaacagggcgactatgacaaggtttccaaggtattggacaaacaactgtctgacttgggcctcgattatgttgatttatatctgattcactggccggttgatgccacttatttggaaagttatcatgcacttgaacgcctctataaagaaggaaaagttcgggccattggggtatccaacttcgataatgaccgtatgagcaaattgctggaagaatctgaaattgtcccagcaatcaaccaaatggaatttaatccgacccaacaagaaaaagacattttgaactttgacagcagccatggcatccaacttgaagcctggtcaccacttggtgctggtaaagcattgaagaacccgattatcgacgaattagccaaaaagtacagtcgttccgctgcccaaattattctccggtgggaatggcagcgagacattgtcacggttgtgaagtcagtccatgaaaagcgaatcgttgaaaatagtgatatttttgactttaagctgagcgatgaagatgttcaacgaattaatcagttggatgaaaataagcgtgatctttggtatgacgattttacctggcataatccaaacggccgttatggcaatgaaattgaaaaggttccggatattcaaaagtagcccgaaaccagatttatcaggagttttcgactcctgattttttattgtctaataatgactgcatggttattgactacccagtcatttatgatagacttaaggcgaatttgaaatatcaaggctttggctgctcgaaaggagtgggcatcatggaaaatcaattaatcttagatgtacaggggcttaaaaaatcatttggcaaggtgcaggcattaacagacgtgaatcttcaacttcatcgtggtgaagtattggggtttattggacccaacggtgctggtaagtcgacaacaattcgggtgattttggggctcatcaaggaatcgggcggatctgcgacggtctttggtgaagatgcttggaaagattcggtcaaaattcacaagaacctggcatatgtaccaggggatgtttatctgtggccgaacctgaccggcggccaaacgattgatatgctgctgcatatgtctgggcaaacccatactgccaaaacggacgaattaatcaaagaattcaagctggataccagcaagaagaatcgaacctactcaaaaggaaaccgccagaaggtcgccttaatcgcggcattttcaaccgatgttgacctctatattttcgatgaaccgacctctgggctggatccgttgaacgagctcattttccagcagcgggtagccgaactcaaagatcatggtaagagtgtcttattgtcgagtcatatcttatctgaagtcgaaaagatgtgcgatacgattgccatcattcgagaaggcaaagtgatcgaaaccggttcactggagtcgatgcagcacttaacccgaaacgtggtggcgatcacaactgcttcaccaatggacgggctggacaaagctaaaggtgttcatcaattgaactttaaaaatgatcagcataccattgccgagtttacggttgattccgatgaaatcggcgctgtgatggatctgctgaccaagagctcaatcgttcagttgaagacgacaccgccaactttggaagatctattcctacgttactatcattcagatgccggtcaaaaagtaggtgagtaagatggcacaatacacacaaactttgacgttattaaaggccaatttgaaacgggactggcttaaaatcacgatttggctggccgcgctggtcggcgttttcgtggcagtggctgctaagtttgaaggcatctatggcaccagcaaacaaattgccgccattggatccactttgcggtccaaggcgatggtcgctttgatcggcagcgttccagacggtcagctgaccacagccttgattttcgcatctgaaatggcggtattctggggactgtttatcattatcttcaactattcattagctgtcagcgccagtcgaggtcaagaggaatccggcttgacggaaatggtcctcgggggtcatccggttggtcgtttggcgccattactggctgcggctttggaattactgattgccaatggcttgtttgccctgattaccgggatcggcacaatgattgccgacatgccggggagtgatactaacggcacttggctgtccgcagttgccattgccgctgttggttgggcgtttggcatgattgccttgatattcgctcagctggttgctgacagccacaacgtttcgatgtacaattacgccttcttgggaattgcttatctcattagaatgatggctgacgtctccaatcctgattacacctggatttcaccactaggctggctcgaaaagactgaaatttacaccaacaataattgttggccggtcgtgatgcttttggccttgggaatcctggcgtttgctgctgcagttgccttaaacagcaaccgggacatcgatgccggggtcatccacgtcaatccgggcagtgaaaagagccatttcctccgtggaccggcaaccttactggtttggaatcaaaaatcgtcgacgatattctggattgttggcatggccgttttgggcgctagctatggatcggtcttcaatagtatcagtaaaattttcaacacctcaccgaccattcaaaaagtcttgggtcaaagtggcatccgccatattgagcagacccaagtattgtcgtttgtcggtttgctgggaatcatctttagcttgctggcagtgattgctggtgtgatggttgttaatcacctgataaccgaagaacgtcggggttatctccagatggtcatgaccaagccgcaaagcagaccttatctgctgggagtttatgtggccttcggcttgattttggcagcactcctgcttttcgtagccttaataagtgccatggcagccggaaatgttgtgatgactcatccaattgcttttaaatacttctggcaaacgttcgtcgctaatttgccgtcaatcgcattgtttatggccttgatggtgggcttgattggtgtttacccacgactgcggacactggtttgggcttatttgggcctttcatttctcattacctactttggtaacctgatggatctgccaaaatggacgctcaaaatttcaccgttttattggacgaaaaaagtcccgatcgacgcgattaataccacgcctttgatttggatgctggtaatcgctgccattttgataatggttggctttgttggttacaagaaccgtgatttggaaagttaaggaggactaatatggcgaaaagactgccacgtgatccgaaaaaagaacacgcaattttgaacgccgctgtggtccagtttggcaaggacggttttaatgccagtaccgataagattgctgaagcggccggtgtttccaaaggatctgtttttagatattttgataataaaaagaaactttatgtagctgccgttaagcaggcgatggcgacgttggttgagacggtcgatttgagtgtgtggaccgattcggacgatttggtgaccatgattattaatgcgaccaaatataagacggagctctctcatcagtttccaaacgaatttgccttgttgacccgcgtgtatgcgcaggataatttgattccccaaaaggtgcgtcaggaagtattcgcgattttcaccaaatggcaggcagaagtagaagataccgtcgtgacccgtgtagttgataagatgacaattcgcaaagatctggataaaggccaagtaaaaaaatatttgacgctggttctggggacgatttcagcggatgtccaaaaagaacttgaggagcatcctgaaatgaagcggattgaggatatggacgacctgattgccaccgttaagaattatctggaaatggcggaatttggcgtcgtcgaatctagacgggattaaatcggttaaaggaatattttaaacacgtcacacacgatcttttccggcaaacaacgtgcgtgacgtgactagttactttggtgatgttaatgttgtctgccaaacacttaccaggacccagcaagcaaatggcatggcactgaggaacagtccaataaagattaatccaggggcgtcgccggacttggcccagatgtaggcaaacgtcagactggtggtggcgatgcttacagtgataatgccaagcagccaccgcaaacgatgaacagcaagcaccacttgttggggccgttgaatgagccgccagagaatgacgatgccgaagatagtacagccaagaaccacccagccgccacctaggaccaggattaacgccaagttgatcttggtggttaagaccaggaggactgttgcccagatgcccactgttaagagtgcgaggcacagcaatgccaagctggcgtgcagaagttgatggctttggttagggttagatttcattttgaagacctcctatgttttgagtttaggcgatttttggtgggggaggttggttgttgggtgatctttggaaaaacgtaaataggtatgtggatgaaaaaataccagctgggccttctttttggaggctttgctggtacttttggttgttgtttgatgatgtttttctgttatctagtggaaacgtgctccgagggcctgaccctaacttctaagtaagctttggtcaaaacccaagttcagggttttaaccaaagctcacttagaaaacgggtcacccagccctcgtcgcactctgattgaaatgtgctccgatgaccctgacccctaacatgtaaaacaaggattgtatcgatgaacaaaatgcgttcatcaatacaatctttgctttacataccggggtcaacccgggtctcgtcgcactctatggcattaccaagtcataatgatttcccacgatcgctgtcccgcggtcatggaccacgccttcaccaagtggtgtttggacatgggtgccgaatgggacgtctgatggggctgccacgattaagtagccgtctgcatcgtagccgccatgattggtggtgccatccgcgaatgctgcgcctgtgtagtacgtccactttttaccatcttggtaaatcacaccttgtgattggaaagctgccggtgttgtggttgcactgctggttgcgtcattggttgagttgtccgaccctgattgggaagtgacgacagctgcatgagcggaaccctttttgattgaagttgatgtcttgaaatgttttttgttaactttcttaacggtcgttttcttagcagatttgccaatttcaagtttttgaccgaccatgatcaagttcttgtcagcaattttgttttgcttaacaagcgtgtcaacgctggagttgtgcttagcagcaatttcagccaaagtgtcgccggatttaacggtgtaagtacttgcgctggcagccactccggtgaaacctaagaaaccagcaacgacggataatgttaatagactctttttgattgtaataaccaccttttagattactgtgtctagaattacgttcacgattgaaatgaaagcccgacttccaaaattgataaaatgattgcttgaatgttaatgtgtgtgttccggaacacaacttggaaatggtgagtgaattttggaagatgattgattagtaatgtgaacgtggaacaatcaatcacgcaagtataatatcagatctgaactaaccgtcaaccgcgattacaaataagacaaaagtatgacaatgaacgtccgtggtaattcagtaaatgaggcagcatgttacaaacacgttaaagttaaaagagactgtttcccattaaatgaatgtaatgattgtgtaaatggcgaatgaatacctgtatatgccaattaatttgagtggagtggtgaatggcggaacttttatataatcattaggcgaatttgaggttcgccggtataatgaaattaacaagaaaagtgagtggtgaacaaaatggttaaacaaggcagatttgccagatccagtaaaatgaagcaaattaaagcgattcgcaaacgaatgcatcaaccggcgggacggataattcacccggaccaatttcaagattttgttttggtccgttatgggctgacgctgaagaaacgattgacgggggttgataaagaaacggttcaacgatttattcaggagttgttggtggtgacgccgattgatcagacttggcaattgaaccagattttgcgggacacgcttcgaagtattggcaacaaagtcccatatcaattttatcgaattgtgaccaacaactggccggagattcagcacttcctccagcgagaaattccggcggttccattggctaatcggatcttggtgaccaatccggtttccgatagtcaactgcaggaaattgtctcagccgaactggcgggaaataccatgattgaaatggttcatgagaatccggcaatggagaaaatgattaccgacgaaccgtatacgacactgcagacaaatttactgagtgatgggaaaattgattggcaaaaagttactgctattttcacgcccattcattttgatcccaatattgctgaagatgcgggtacgaaacaatggctggaacagttaatcaaggaatagtgaggtcatgacgatggatttacagcaagcattagaatgcgttaatttagtaccgatgtttcactcgctaccggaagagcaaaagactgaggttgccaaactggtggtccagcataattatcccaagggaaccattatctatctggccggcgacaaagtcggtcacttcatgatcctcgaagcaggccaggttaaaatttctcaagtggccgccaacggtaaggaacaattgttgaaagtccttcaaccgggtgactttgatggggaggcggctttgtttaacggcgatcagagaaacgtgacggcgaccgccttggtggactccaacgtctgtcaaattgagcagggggcctttcaaaaattactccagaagagtccccaactctcggtgagtctgctggcaactatgagtcagcagattaatagcctccaggaagaaaagacgctttcgtctacggcggatatggccggcaaactggctaagtacctggttgaaaccggtgcagccctggatgaaaatccatttaaacttccattaaagaagaaagatattgcgacctatttagggacgaccccggaaacgatcagtcgaaccttcaagcagctcacgagcaaagggttgattgaagctaaaggatcccaggttaaaattatcgatgaagacggcttggacatgttagtctaagctttttctttttagtaaatatttattgcataaatttagaaaagaattgatttatacgtacgaatattttacaatgagagagtaaacgaaaactaaacgtagctacgttggaggaaaaaacgatggacgaaagtcgagtacgaaatgaaattgtaagcggaaacatttcgttgggaattgaactgggatcaactcgaatcaaagctgttctggtttctgacgatttccaaacaattgcttcaggcgattatctttgggagaacgaattagataacggcatctggacttacccacttgaaaaagtttgggatggcattcagaccagttatgcaaacctggcattagaagtgcatgacaaattcggggttgatatcaagaaaattggttcgattggtgtcagtgccatgatgcatggttacatggcatttgataagaatgatgaaatcctggtaccgtttagaacttggcggaacaacattaccggcgacgctgccgaagcattgaccaagctgttcaacttcaacattccagaacggtggagtatcgctcatttataccaagctattttaaatgacgaaaagcacgttaaagatgttgacttcatcaccactcttgcaggatacgttacctggaagttatctggcgaaaaggtcattggagttggggatgcttcagggatattcccaattgacgaatcaaccgtcaactacaataaggaaatggctgacaagtttagttcattacctgacgttaagaaatatccgtggaatctactcgacattttgccaactgttttacctgccggcaagaaagccggtgagctgactgatgaaggtgccaaattgcttgaccaaagcggcacccttcaaggcggctcattgattgcgccaccagaaggtgatgcgggtactggaatggttgctaccaacagtgtcaagaagcggactggtaacatttctgccggtacgtcagccttctcaatggttgtccttgattcaccaatgaaggctgttcatcgtgatatcgatatggtaacgacaccagatggtgcaccggttgccatggttcataccaacaacagttcttcagacatcaacgcctgggttggcttgtttggtgaatttgccaaagcattgggtctccaattgaagccggatgacctctacggcacgttgtttgccgaatctgtcaagggtgatcaagatgctggtggattagtcaactttgcatatctttcaggcgaaaacattaccagaatgcctgaaggccgaccattgtttgttcgcaagcctgacagcaagctcaacttggccaactttatcaaagagcagatttattcagcctttgccccacttaaaattgggatggatattttgcttcgagaagaacacattaagaccaatgttttggttgcacagggtgggatcttcaagaccccggttgttgcccaacaagtcttggccgatgccctgaataccccaattgccgttatggaaaatgccggtgagggtggcccttggggaatggctgtcttggcactcttctgtgttaaccgtaagaatggcgaagctttggaagattaccttgccaaccgggtcttcaaagactctacgacggcaacgttgtatcctgaagaggccagtgttcaaggttatgacaagtttatcgacaactacaaggcagccttgcctgtagaagccgaagctgttaaatcaatgaaaatgaaaaactagaggtgcgagagaatgttagaagatcttaaaaaagaagtttatgacgctaatatgcgtttaccccaacttggtttggtaacgttcacttggggaaatgtttccgcaatcgaccgtgacaagggcttattcgttatcaagccttccggtgttgaatacgacaagatgaagccatccgacatggtggttgttgatttggacggtaaagttgttgaaggggacatgaacccatcaagtgatacaccgacccatacttacttgtacaatcatttcccaaatattggcggcattgtgcatacccattccccttgggctgtgtcatttgctgcagctaagatggacatcccagctgtcagcaccactcatgccgacactttctatggcgacatcccatgtgcccctgctttgactaagaagcagattgaagaagcatacgagttaaacactggtaaagtgatcgttgatgaattcgaacgtcgcggtgttgatcctgacgccgttccagctgttttggtcagccaacacggaccatttgcctggggcccaacagctgataaagcggtctacaatgccaaggtattggaagtttcagctgaaatcagttatcacgccttacaattaacccgtgatgaaacccatgtcccacaatacttgttggacaagcattactaccgtaagcacggtaagaatgcttactatggtcaaaataatgctaagtcaaagtcacatgctgaacatgaataatctgctttaacgaatagggcagtttattaagaagagaaaagtcgagacaaaaccatccgttttgtcccgacttttttgtagtcttaatatcacttggcggaatagtgggaaaatcagcagctcccagaatagaaacgctgattttcccacactcatttttcagcatgagcaaactatttgcgtcggcctaacttcagccttatactcaccaaaaagcaatcttggaggcgattacattggctgagaatccattaattacgatttccattccggcgtacaacttgggatcatacttgtccaagactttggatagtattttgaaccaaacttatcaaaattttgaggtcattttggtagatgatgcttcaactgaccacaccccagacacaatggccaaatatgcagataaagaccaacgcatccacacccactattttcagtcgcatgaaggggtctcaaaagcccgcaattacgcgattgataacgctaaaggcgacatcattgtctttgtcgatggcgatgatttattggagccgaaatatctggaagtcatggcccgcgggttggctgatccgtcggttgatttagtggccgttggctacaactggggctggcgtgggggcagcggcactggtgatcagttccgcgaagtttccaagaccaacgcatatgcctcaatcaatcgccgaggcggcgattttggcggctatacctggaataaaggattcaagatgtcgattattcgtgatcatcaaattcaatttgacgaatcgttggacttggcagaagatctgctgttcaccgcggattatattttcgtgtcccatcgtttcctattctacccaggggcactctacacaaaagtcagtcgttccaatagcatcattcactctgcgacttgggagatgcggagtaaagagcaggttgttcgcagacacatcgatgaaatggcaagaaagatgcagccgtaaaatttatgtaaagattgtggataagcttccatttagcagtcagtttgaggtaatatagcttcatctgaggaaatctatttttgggggtactctggtttgccaagttttaccaaatctcgccagcaaaaattaaataaactcattttgttcatgatgacgcttgtttcgatcctgacaatgagcgccattagtgtgtccgcaaagtcagccaatcaacaaaagtttcaggccaaagaggcctatgtgatggatgcagaaaccgggcaggttctctaccaaaagaatgggagcaccaaacggccaattgccagtctgtccaagctgatgaccctttatctgaccaaaaaagcaattgataatcaccaaatcacttggaaccaaaaagtgccggtggacgaccaacttcgtcgaatgagtaaaagttatgaagttggcggctttcggatcaagcgttccaaggaatataccgtccgcgatttgtacaaagccgcattgattgcgtcgtccaacccttcagcgatcgccttggggaaattagtcggtggcggcaataacactgaatttatcaaaatgatgaacgaacaggcgcacgcctggggcatagatgccacttttgtcagcagttccggcttggacaataccgatttgagcaagtatcattaccaggttccccacacgacatcaaaagctcagaacatggtgagcgccaaagccatttcgacggtggctgccaaggtgctggagatcttccccaccattacccaatggagtaagcagccctcgatgaaggttggtaaccaagtgttggttaattctaatcgcctgctgccaggctcggcattttatcacaagagtactcatgtcgatgggctcaagactggttttaccgtgaacgccggcctctgtattacggtgacgtactggcatgacggtcgccacttgattgccacaattattgacagtaacacactgtatacttcgatgaataagctgatctcgacggtcaaccagcaatatcagcccaccaaggtcgccttaaagtcgcatgctttctcaattgacggccatcagttgaccgccacccctaaagaccctgaagcagtcatttggcagcgcaaagggaccgatggctcgcatgtgaccaattattcagcaaccaaaacgacgttgccgattaccaaaggccaactggttggcaacgcgatcgtcaaactggcagataactccagtacggcggtggtgccaatgctggcagcgactagcattaagcagccaactaaaaaagtgaaacatgcgactcacaaaacctcgttgctcaaacggatttttggttttgtcggcagtatttttggcggcatttatcggctgtttgtggatttcgtgaagtttatgacgccatagttttttctggcatctccttaataaagggggtgctttttgttttccatgccaaagttgacgtatgataggggcaaatccttggaggcagccatcgtgaaaaattatcgaatcgttcaaatatcagacacccatttaacaccacagaatgcgcaacctgcgaataaccagcagattgatccgatgctcaagctgatgcaggtctttcatgacatcgaggcaactcaagttcaccctgacatgattgtaatcagcggtgacctgattcatgaaggaaaagccgtagattatcgtcaattcaagaagctggtcgacagggaacaagcccaatttggcgtgccgatccaagtcctactgggtaatcatgatcgcacgtccgccttttataccggctatctggataaaccagttcagccccgatattattacagtttgtcagataacggctgggatttttactttttggataccaaatgcggagacttggaacccggctacctggatgagcagcagttgcgctggctgaaggagaagctgggtgaatccaatcgaccagccgtgatctttatgcatcacccactcctgggagcacccttggaaaatatgaagtacagtattttgcaaaatggcgatcaattgcaatctatcctaaagggcagccaagtcaaagcgattttcaccggtcacgtgtattttgccaatatgttcatcaaaaatggcatcttaaatgtgtcagctgattccaccgcttatcatattaattgttccaattctaaacgtcatctaatttcagaaggcaccggctataacgtgatcactttgtctgaccaacaaacgagtgtcgaacaacgaccgttattgctgggaaatacgaccatcaaggcctttaacattccgtcaaccgacttcgttaacccccagattgttgcccaggaaatgaaacgggttttccggtaaactttcaagtgtttttaatagtctgatcggccatcctggcgtacactaatacagaatttaccttacaaaaaggggtgagctgtatggataagcaaccagttgaaccaattggcccatacgaaagactgctaagcgggtcactattggttatggccgcaggggtgctggactcgtacacctatctgcaggatggcggcgtcttcgccggcttgcagacgggaaacttaattttaactggattgagaattggccgcggcgattacgccagcatcggccaagccttggtgtcattggtgatgtttgcggttggcgttgccatcatccgggtgattcagtaccattatcccagtgagcgggcagtgacacgcaagcgggtgacgttagcgtttgaaattttaattttggtcgtcgtgagtttgattgccggccgtgtatccattttggtcacaactggactgttggcgttggctgcagcctcccagctgcaggaattccgccggatgaagaacgccccgtttacgccactgatgatgaccggcaacgtccgcaccttatctgaaagtgtcttggactttgttgcccagggggatatgaaggcactcaaaaaagccggtgacattgtgacaatcatcggctccttcttcattggggcgctgttaaacggctatttgattcagtttttccatgggcagaccattttaatcgctgccgttattttgctggcaaccatcttgtttgccaagtaagttattctgatttgagttttgaatacatggccacgtcatggaattggccgttgtataagagatattcctttaaaatgccatcttcatgaaagcctcgtcgtgttgctacggcgcggcttttgttgtttttaacatcggcgattaactccaggcgatttaacccgagttcagtgaaggcaatttgttccacatgggccaagcagagcgtcatcacgcccattccctggtattgattagccagccagtagccgatttgggcccgctgattttcatggctgaattcatggaggtcaatcatgccggccggctcattgtcgaccagaataatggtgaaccaaaaatcaccatgagccattttttcgattccgtattgcagaaatttttgctcgtcactgactgctaccatccctttggcccatggcagccactccgccagctgcatgcgattgctgttgatgagatccaaaatgccgttggcatcagtcgctgccggtaattttaaggaaatatggtcgttcacttgatcaataaacatagagtccctcctcgtcaaactgttacaattaagtataacctttttgagggaggaagacttgttgaatgaaagacgtacgttggaattgcctgacgcgctaaaagcacagttgggcgttaaatctggtgagcacgtggaggtccgtattggtgctgatgaattgaaaatttccactcctaaaccagtggaagtcaaaaaacggcgctgggggatgatcattttaaccttcgtaatgagctgcgtctttttgggctacttcatggtccgaaaaatctatcaggtttccctggtcggtagtgaatcagtggcgacaatggtgttactattgacgacactcagcggcctgatgagttttatggtcgtcttcgtccggttgaaacggcagtctggctcggcagtcgaatccgtttcgtggcgaaacctgccaacggtcgccctggcgtttgcgttgatcagcttcatgctgatggcgggattgttttggattgccggtcgactgtttaagggcgccagctttgatttggtgacctcaacggcattatttgcgctgatgaccagtgttgaaattcaagccatcaatagtcttgttcctcagctatcttcacgccttttgaccaacatctttattgccgtgattgtcagcggggtcattttggcgatgatcagtaatcagaacttgtattggtggaaacacaacctcagctttttgggtaccaacaaagcggttgattcttgggagtttaacctggcactatttttttcggggttaattctgttggccctggtggattatttatttgcttctttgaaacgaatcttccctaaaagccggcagttgctggtgttaagaatcttattgactttgctggcgattgatttggggatggttggggcttttcccaacaacttggaaatccattcgctgcatactcggctggccggctatttgattttcctgatattaggactgatttttggtattcgctggctgctgcctgatatttccaccgattttcagcacatctcctggatgattgctgcagcattgctggctggcgagatattatttcaggtggttggctatttgtcgctgacagcgtttgaaatcatggcgtttttactggcctttagttggctggtgatgctgtttgaacgtttgaacgactatctggagccaattcagaatcaacggtatgtcattaaataattgtgaggttattttgatgtttgaaatgaaagcaaacaaggcaaatcaggcacccatggcaagatatatgcggaatcagtttcaatttcttggcctcaaaacaccacagagaaaagcggcctcgaaagcttttatccaagcttccaaaaccgttcctgttgctaaaatgatggaagaaattgctgaactctatgaccgtgacgagcgtgagtaccagtacgtggcgattgatgttgctgatgccaatgtgaaacgattatcttttaaagacgtcaagacgttaactaagtatattcaggtgaaatcctggtgggatacagttgacacttggcgaaaagtgtttggggatttcgtggtattgcatccggacgaaaagcgggcggtctttgatttgttctatcagcacgacaacttttggatgcggcgagtcgccattcttttgcagttgctggaaaaggagacgttggataccgagctgctggccaaagccatcgaatatgatattgacaccgatgagttttttattcaaaaggccattggttgggcattgaggaattatagtaaattcaatcctgcttgggtgcgtcgatttgtggctgagcatcatttgtcgaagttggcggttagggaagggacgaagtatttgtgacgggtgtgggtgtttttgagatcattcattgtcgagcgccacttttacttggaataaacgtgctgcttacggctgatccctgccatttaaacaaattgggcaattattccaaaaggaataattgcccaatccgcttaaattctgggatcaaaacgcctaaagcaccactctcaatgcttagaagccaaatgatgatccgtcaatctgaaaccagtgacgacaataatagctgcgacaaggaatgaggacaagccgaggatcatgttcgtaaagccgatgcttgccaagattgatgcaaaaattgtaccaaacactaaagttaacaaaccgatcaaagtgatttttaaattctcatccatgagatcgcgcccccatactattaattgttgtaaaaatcgcaagcaattctttgtcaaatcagtggttatagttagtagtcattagcaaattgtttgcgctttctttacaacttcattgtaacgtactcaggtttaaaatacagcttttttctcatatttaaatcgttttatttcgagggaataattaggggcatgaatgttcaaaatgaccggtgctggacaagttatgaattgtgtgtaaaaatattggtaacagaaattcgaaatgaaaaggaagtgaagcccattgaagattgcaaatcgttaagacagaatttgataatgaatcactgttcagaacaggggttcttctgcgcgattttgcaattttagtgggttttaagttcgatacttttagtgtgtcagaacacccaattagtctatcaaaatcgcctgcgtgccgatgtgcacagcaggcttttatattgcacagaaacccatctgaacctttaatgaggtgagattatgggaaccattcagattaaaaatttatcgtttaggtatgccgggatgctgaccaatcttttcgatcagttgaacttaaacattgatgaaagttggaagctgggattgattggccgcaacggccgggggaagactacttttctcaaactattgttgggaaagtatacctaccagggagaactaaacagcagcgtcgactttaactattttccacaaagaattccggatcctactcagctgacaaagcaggtcttattgaagattgccggacttgatgacagcgagttatggcgaattcaagttgaaatggataaactgcagttgactgacagcgtcttggagcggccatttgagaccctgagtcccggcgaacgaaccaaggcgttacttgctgtcatgtttaccgatgatcagacctttcaactcattgatgaaccgaccaaccatctggatattgaaggtcgagaagtggtcgctgactatttaaagcacaaacgcggctttatcgtggtgagccacgaccggcactttatcgatcaggtcatcgatcatgtgctgtcgattgatcgcgcaaaaatccaattatttgctggtaattacgaaacttgggcggccgagtatcaaagggaaaatcaatcggagcttgccgaaaagcagcaccttcaaaaggaaattggccgactgaaggccactgcgaacacaatggaacgttgggcaggtcatgcagaaggccagaaacagaaaagccgacagagtgaccagcacgctaatatcgataagggattcgttagccataaagctgccaaggtcatgaaacgctccaaaaatacgctgcggcgcactgagaaagatattgaggtcaaacagtctttgctgaaaaatgtcgatgaagtcgcacccttgaagttgaataatattcaaccaccacaaaaatatctcctacaagtggaaggcttgcaggtccaacaagccggcacaattttgaatcaacccctgagcttcgatttaaagcgcggccaacgcttgatcctgtttggtcctaatggaatgggcaaaacgaccatcgttaaagtgattatgggcgacaaagagttgctcgctggcggaacagtcaataagcccgccagcctcagaatctcatacctgagtcaaaactttgaagatctcaatggatcgattcagaactacgctgatcagtttggaattgagttaaacgacttactgaataccttgagaaaattgggctttgagcgagcggcatttaatgaagacttgaaggatttgagtatggggcaaaaacgtaaggtctcgttggccaggtcgctgtgtgagccagccaatctttatatttgggatgaacctctgaactatctcgatgtgatcactcgaaagcaaatccaagacctgatcttgcgcaagcagccgtcaatgcttatcatagatcacgatgaggcctttattgaagcagttaaaacggcgcctttgttaaaaattgcgccgattgattcacaataaggtgtacttattgatgactttgttataagatgtgctagatattgttgtgaatttttagaggggttaagatgccaaaacattcattgaagaaacattcggtcaatcgatcgttattattgagcctcggggcaattatcgttgtgggtttgctgatggttaccgtcggcaaagtgtcccagggcaacaacagccattcgacggctacccgcagcgctaagcagatcaagaaagccaagattgccaagttgaatgctaagattcatttgacgaaacgcgagaagaagattgccagtcattacaagctgaccaagctggagacacgaacagcctccaagacctatatcaccgcgattggtgattcggtgatgattgacgttaaaccggatgtcaaacgggtctttcaccacagtgctgtgagtgggtctgtcggccgccagttttattcgctgccggggattgtccgccacttgaaggcgactggtcatttgtccaaatacatcgtcattaacttggggattaacggaccgccaactcagcacgatattaattcagtattgaagaccctgggtaagaaacggcaggttttctggattaataccagggtgccacgtcattggcagaacacgactaatcggatgatcgccaagacagccaagaagcattcaaacgtgcatttggtgaactggtatcaagccagccgtggccataaaggttggtatgccagtgatcgggttcatttggatttgaccggtgaaaaatactatactcggacgctggccaaacgtgtttcggaaattttaaattagtcagaaaaaacactttgaatcaagttaatagctcaaaaaaatcagcagtcgcatttttgcgattgctgattttttagtatgctgtgtatttgcatgccaataggacacgtatttatttgatgagttgcttgagttcctcaaaaacgatcggcagctgcttgtccttaccggtatctgtgaaatggtgaccggatggcatcaaaacaaacttggcgtgtaggtgccgtgctagcgttaatgtgtacgggtacggtacactatcgtcattaatagctgaaataaccgctaccttacggatctttggcagaattccggaataatccaccggatgttccgtgaaggaatcaagttccggcagtgtccaaatgggttcgtcaaagcctgatactaataagacattgacgttgtggatgtcgtgctggtcaaggtagtggaggacttgaatgcagccgaggctgtgaccaacaagggtcatgccgtccgctgggtcaatatttgcgtcacaatactgatcccaagcctgttccaccggatggtcggaatccggaaagttcagttttttaaatggtcggtggagttctgtttccactcgattttccaaccaaggaaaccaatgatcgttggcattggacgtatagccgtggaacatgtagatggtcatttatgctaccttctttcccagtattaaagcgcggttaccattgctcatgcttgtaagccatttcccaaaagtgcagttcgaaatagctgcttcgcaaaaacgccgtctgcatctgttcctgttcttcagcatcggcagcctcaccaagttggtcgacaatggttttcattttgtcagttgccgtggtaaatgcggggctgtcataagtctcaataaattgctgataaattttaattggcgaacctgcttttatcaatcgctgaccgatctcattatataaccagtagcagggcagcaatgccgcggcggcgcgagaaggggtgccttcattgagttcatggtacatatgggtcacataactgtaggcattgggggcaatctcagtttgatcaatctctttttgggtgatgttcaactcttggaaaaattcagtccggacttccttttcgctgtcattaaagcctttggctccagcatagagaaattctttgatatccggatcgtccatttgatcggcaattgtgccatggaggacggcaaaattctgcaaataataacggtcttgtttgaggtaataacgaaatgtttgttggggaagtgatccgcctgaaagctgcttgatgaagggatggttaaaactggcttcccaaagtggttctgattgttcacgcattgtgtcggtgatttttgccattacgcttaactccttaggttagttagggacatgtttgagataattttaccatgattattaagcgataacgacttgaattaatatgtgaattagcgagcaaattgattgctattgggaatttgctcaggtacacttatgacgattcaaaactgaagggagaggttgtaatggatcgtttaaaagataaagtcgcaattattaccggtggcgtggccggaattggattgggaatcgcagagtgttatgttcgcgaaggtgccaaagtggtactgactgccaaccataacgttgaaggcggcaagcaggctgtcgacagatttggagatgatcaatctctattcgtccagcaggacgttgcggatgaaaaatcctggcaggacaccgttcaaaaagcaatcgctaaatttggcaaggtcgacattgtcgtgaataatgccggtgttggcggaaaaaacggcccactcgatgaattgactatggaagagtggcagcaagttattgacgtgaatttgaccgggacctttcttggagagaaatatgggatcaaggcgatgaagaaatactctggtggaaaaggttcaatcatcaatatttcctcagtcgccgggttagttggattgccgctaagcccagcctattccgcaagtaaaggtggcagccgtttgctgactcatgcgacggcgttatccctggcccaacaaaagctcaacattcgggttaataatgtccatcctggttggattgatactgatatcgttcctaaaggctttgaagaagctctcacgaagacgatcccggtcggtcacatgggcgaaccaatcgatattggtgaggtgtgtgtttacctcggcagtgatgaatcaaaattcgccaacggcgctgattttgtgattgatggtgcgcaacgggcataaaacgattaacaaaaaagtcctgccttgtaaagtgaacccttaaaattggacaactttattaagctgctttctggacggtaagttcccggtattttaccggggacttgccgtccagttttgttttgatgcgccgatgattgtagaagtctatccattcgttcatagcttcgataagcgctgttttggtctcaaaatgttcatccataacctcgactttcataatgtgaaaaaacgactccatggcggcgttgtcgagacaagtggctttacgcgacatactctgaaatacatggtgctctttaagcgtgtcttgccagtggcgatgctgatactgaaacccttggtcagtatggacggttgtccgataatctaacaccggtattcgatttagggcttctttcaaaggttttaaagcaaattcaacggtcgggtggtcactgatattgaaagccagaacctctccattgaagaggtcgaggactggttctaaataaacccgttcattttgactttggttcccatatcggaattcactgacgtcggtgactaacttctggtaaggccgatctgttttgaatcgtcgcttaagtcgatttggggcgatgacgccaacagttcccttgtaagaattatactttcgtttctgccgattaaaggcgccacatagccagtcttgttcccgcataatccgtaagacccgcttatgattgattttaaagccataagcgtcatgtaaagcaccggttattcgtcggtacccgtatttccgagtatattttggatcttgttgacgaatctcatcaattgcctgaataatttgtgaatcatctaagttacgaccacgatgctccttagcataataatacgtgctacggggaatacgaacagccttaagaactagtttgatggaaacttgaaaattctgccttaactcgtctactagttcgatgagttcgtgtgttttgacttctttcgtgctaaggcatcgagtttttttaagaattcattttctatttttaacatttgattctcttgttttagctgcttcaattctgcggctggagtctgtggtttttcaggtttggggttgttctgcttgtgtttgaccatggtcttaggattccctcgtttgcgctcaagtcccgctattccagattcctggaagtgtttttcccactgccaaatcgtacttggcgacgacaagtcaaagtgtaaggcagtcactggaagcgaagcttgatttcgtttcttccagtttaatacatcgactttgaactgactagaatattcttgggacattgaccggtcttttagaccttcaatacctcgccgctcaaatcgatgaacccagtccagaatgattgaatgattgctaatgcgatacttcttagctagagacggtgaacctttaccagataagtattcagtaacgacctttattcgaagttctaaattaaattttgacatagtaaaacccccaaggttagatttggtgtccaaccttaggggttcactttacttgacagggctttttgtatttcctaaggttctggaactttcatggtctgatcaacgtgtgagcgaccagtggcataatcaaactggatgccgggctgaacattgaacaaatagacgttgaagttcagtgtccgatctgttgaaatcgcttcaagatggatgccgcgggccattaattcatttccccgaaaaataggcttggaaaagaagatcactttgtttccacgtcgcagggattctctgattttaccttcaaaaatcgtctgaacccgctgattggcgaagctggtctgggtgaataggttcttgggattgttttggtcgcctgacgtgtcggttggattatactggccggatgcactgataccaccggagatcgaataggcaattaaatggccgcgattgataatcggctggccatcgaggaattcttggtgccaagcggttggctccacatactgacggacccggttattgtcagaaaccacatttctaggttccaagtaagccaaattgccggtgctggtccgattaaagttgtccagatcggaataaatcaccttattggttttccaagaacttggatccaactgtgctttgttgtggttcacaaagatgtagctgggatcactggaatgataatccagcttcgccagttgatctgatttgacacttttgttcgaatggaacaaagaactggtcagattgttgaccattgaagcgaggttactaggctgttggccgacccccagccacatgccgacaaggatgattgccaaggcaaagattgtctttaggccggtgttgcgtctttttcctctggactttctgggatattttttatgttgactcatgatcatgcctcaattctatatgtaagctctgccttcaaacataccagaagggcatggatgaaggcaagagtataaggagagtatgcacacctgtgtgcaatttgctggggaaagcaaagatggctttgcggccatcactttatatatacggtgaaatggttggggaatatttttattttttgaaattttttggaaaaggtttttattttacacttttatctagcgaaaacgtgctcaaagacccaggacccggccacacaagcaataaaagccaacgatgaacaaaaggcgttcatcattggcttttattgcttgtgctctgggtcctaaccgggtcttttcgcactctgattattaaataaatgctcaaaagctacccggtttggtccgcactctgatctttatggcaaatcatttcccgccgcgaagaacaggtcgtaccactcctgctttgtgagttcgacatctgctccggctgcgctgtccttaatgtgttccggattcattgttcccagcagtacttggacctttgccggatgtcttaagatccacgctgtggcaatcgcgttctttgagacaccgtactttttgcccagttcttccaacttatcatttaactttttgaactttggatcgttgatgtacatgccggcaaacaagccataattgaatggtgaccaagcttggatcgtcatgttctttcgacgtgagtattccataatgccgccgtctctcacgatgctggcatcgtcgatcatgttgacgtgcatgccttctttgaccattccggaatgaaccacgttgaattgcaattggttaatcaataagcgttggctgatccaggattggaccatttcaacttgttgaggattaaaattcgatacaccgaagtgacgaacttttccttcccgctgcagggtgtcaaatgcatcggcgatgtcgtctgcttccattaacggatctggacggtgcagcaagaatgaatccaaatagtcgatgcccattcgttgtaaaatcccgtcgaccgagtcaatcaggtgttgcttggagaagtcgtaccgttggccaaataccaggccatcatgactcctggcaggatctaaaataatcccgcctttggattgaataaataatttatcccgagaaattccagaagctttcaaggcttctttgaatttggtttccgattgtccgtcaccgtagatgtcagccgagtcaataaaattaatgccagcatcaacagcggcttccaatgtcttggcagcgtcagcggtttccataccagccatgcgcataattcccaaggcaactgcggaagcttcaaaatttgtattaccaatctttacagttttcatgatcgtcctccttcattgattaccttaattatacggcattctgagggcggttccaaaggtcttgtaaaaaagaatatgttataattcgaatacttacaaaacgaaatgaggaaccaatttgagtgaaaatacaattactgaattaattaatcagtatggctacctcggcattgcttttctaattgcaatcgaaaatatctttccaccaattccttctgaactggtgctggtcttcactgggtatttaaccgttaccagcaagatgaccatttgggggtcgattctggctgccacggctggcgcactgattggggcaatcgctttatatggtgttggccgtttattgagcgtccaacaaattgaaaaactggtgtctgggcgatttggcaaaatcatgcggttgaaaccggcagatattgaaaaagcggccaggtactttaacaaccatgggggtaaggcgatcctgattggtcgctgcatcccggttgtccgcagtttgatttccgttccggcggggatgaccggctatccctttaatcgattttgcttcctgacgattaccggaacgctgatttggaacaccattttgattctgatcggccattttgccggtcgggcttgggatcagattctggggatgatcgatcagtggctgatggtgattttggtagtgattgttgtgatcgtgggatgttatttgtattatcgattttctcggaaggcggattaggatcgggcagctgtttgttgagtattgatgtttttgcctaataggattactcttccttggttgtcattttacctagcggaaacgtgcaaatgaaggctgatcccggccatataaaggacttactcatttattcctgatcttggaataaatgagtaagtcctttatattctgggatcaaagcgccttcatttgcactctcttttacttttccttaaaattccccaaactttccaataaactcctcacaaacttcacaaattactcggcaaaatttgttatgatatttataagtaatgcaccacgacagctgaacccccacaaggaggcccactatgcaatggtacagtcatgaagcagaaacaatattacaagaacttgatacaagtcggatccatggtctgagtgaggcgcaagctcaacgacagcttgccgaagttggacccaacgagttagccaaagaagaacgcgaacccgcttggaaaatgttaatcaagagctttaaagaacccatgatcattatcctgctcatcgccattggtctggcattggctagtgccgcctacgatttcttcatcagcggtgattccgggcatgcgatggcttctgtgtacgaagcgattgccattgtcttaattgtgattatcaacagcggtttgacctttcatcagacccggaccgcgcaaaaatcactggacgcgctttctgatatgcgtcagcaccacatgaaaatacttcgggataacaactggacgtcagtggcagccaatcatttagtcccgggagacatcgttagtgtcaaatccggcgactttatcgaaggtgatttgcgctggctaaagacgtcagaactgtagattaacgaatctcatttgaccggggagtctgatgccatccaaaaaagtaccgtctctctccctgaggataccgagttggcagatcgtaccaacatgggatactctggttcgatggtcgtcaatggaaatggaattggtgtggttgtggcaactgggatggcaaccgaactgggtaagatttctggactgatgcagcaggttgacgaccaaaagacaccgattgaaaaatcagtccacgggttgagtaagaaattgatgatcatcgctgcagttatcatcgccgtgacgattggctatgacttagtaaaataattaattcaggtcggcagtatttcaatggacagctttggcgggatttcagccacggccatcgccattgctgttgcctcaattcccgatgcaatgccggtggtgctgtcgattgtgttaacgatcggtgccaagatgatggccagccaaaagggattggttaagtcgttgagcagcgtagaaacgctgggctcaatcacctatattgcctcggataagacggggactttaactaaaaatgagatggccgtgacccgctttttggcaaatggccaagtctacaatgttgaaggaaatggttacacaccaattggcgatttcatcagggatgatggcactccaagcgatcctaaagattaccagcggttcttagaagtcgctgtcttaaataatgaagctgaaattaaaccggataccaagcaaaattggcggccgtttggtaacccaaccgatgtttccttagtcgtgctgggagctaaagataacgtcaaacgcgacgtgctgttggaagataagggtgatcgggacatcgatattgtccgaatcctcccatttgacagtacgcggaagatgatgaccgttgtgattaaagaaaatggccggtactacagtttgaccaagggcgcgccggatgtgatcaagccattgaccaaatcgaccatgattgatgggcagccggttccaattgcttcagtggccgcaaatattgaaaaaaccatgctggcatttgccaaggatgccttacggacgatctcaattactcagcgggagatttccaaagaagatgccttgaacgcatccagtgccgaattggaacgtgaactgacctttcttgggctggtggggatcattgatccgccgcgtgaggaagtcaaagcgtctgttcgcaaattaactcaagcatcggtcaacgttgtcatgatcacaggtgaccacgcgatgaccgccaaggcaattgccaaacagctgggaattatcgagtccgatgacgcccgggtgattaccggccgtgacttggaagacatggatgaccaacagctggcagacgtggtgttggacacgcgggtatacgccagggtaacgccagaacacaagcagcggattattaaacaactgcaggcccatgagcaggttgttgggatgaccggtgacggcattaacgatgctccggcactgaaagccgctgatattggtatcgcgatgggaatcaatgggacggaagtgaccaaagatgccgccgatttgatcttgctggatgataaatttaccaccattgagaagtcggttgagtcgggcagaacgatttttgccaacattttaaattttatgagacatgaactgacgaccaatgttgctgaagtgctgtcattattgctgggagtcttcttgattacttcttccattggaaatatcaccgaagtgacaccaactctgacagcgttgatggttctgtgggtcaatatgatcagtgattcactgccatcgtttgcactgggctatgatgaagccgaatcagatgtgatgcagcagcgtccccgtgataccaaacaatctattttggcaaatgggatgctgcggcgggttctgttccgtggtggcgtgatgggcgcaatggtctttctggctttcatttgggcagcatcacagggctatacggtcgctcaaagtcagacgattgcctttctgacattggtattcgggcagttatggcacgtttatgatgccagaagtgtgaatacgttgttcgatcgaaatccgttttccaattcaagattaacgttggcggtcgggtttgcggcgacatcctcaatcttggtgacgttgatgccatttttcaataatgtgatgggaaccgcgccattaacgatgacgatgtacgtgttgattatcctgatttctgcggtaccaacttttgtgatttctggaattaagaaattcatgggtcgaaatcgtaccgaatcagtggctgttactcaagcaaattaatatagaacaaaaacaatctaagattaagtggttcttcgtcaactgttgttggtgaacaaaatattggagttctaatcacttggtgattagggctctttttgtatgaactcgaaaagcgaacagcactcttagccggaatctgaagaagtttcggtaaccaaatccagtgcgcttaatgactttaatcttgttgtttgaaccttctaatggcccgttggtgtagtggtgggtgaaagtgttgccaatttcatcatgatgagccgccaaggtttggagggctgccaacatctcttccgagcacccctgcaggtggtgaaaggcttgattatagttgggccagtcgcggtttttgatggtttcacgtaaccgattcatcacgtcgtaagtttgcttgagctcgggatcaatgtccagtaaagcatcaaccacatccgtggcagttgccggataagggaagtttgtccacttacggaaagcctcgtagttaaggtgattggccggcgttaataatagtttccaatagcgtttcaaggcgtgatactggcgtgaggaagtggccagggttttcatgagacgcactcgcgtcttattaaaagcccggtttaaagcgttaaccaggtggaagggatcgatgacaacgatggcgttcgggaagatctgcccaaccaatttgggataggtatagttcatatcggtgacgataattttcacattttctcgcgcggcttggtcataatgttggaagtacttttgaagctgatagatggttctaaagggcaacaggtcaatcaattcgtgggtttccgcgtccataaattcaaagctcatcgcgtcggtggcgctcttagtacttttaacttcgtccatgaggagaactttgggtaagtagtgccagttggtttgaaagtcgtgttcagcgcgcaagagctgccgaccaacgaatgaatccgaagtggacaattcattggcaatgtgtttgaggctcactggttccgttaacttctctaaacattgtttccgggttgtatttgaaatcgtgcagtgcttcggcactgcactcgtctgcgccaggaagttggtatgacaagccttacagtgaaagtttcgccgattgaggcataggataaccgtgctgcccaatgttttagcgaatctaatggtggtcttccgccaaccatagccaatgatctggtgatcattaataaccccacaattgcggcaggccttgggagaatagttcagtgatccatttaatctgattaccccatcatcacctattttgccattctcaatttttaagtgttcatcatctattcctaacaacattttcgtagtatcatttgacatagggcatttccttctttctctaaaatcttcgtggttgttggttttgatgaacggacaggaaatgtccgctttttttattctaatgaaaaacaaaaaatctgtcatcagtaatagataaaaatctattaccaacaacagatattgtagagccgattaagtctggtaagaaagctgacagccgtcaatttctcactggaactaatcttagattgtttagattgagatggaaatgattttaattttgtaagtgacttgcggcgcggagacagtgacaatgtcgccggaatggtggttcagtagtgccgaaccgatgggagaggcgattgaaattttaccgtggtcaatatcaacttccggcgtgccgacaatttcatacgtttcagttgagtggtcatccagaaattcaaatttgaccgtcttaccaacttccacggtatcattgttcgatggggtataaacctgggcgtactggagctgttttcgtaagaatcgcaatcggctctccaggtggcgaagatctcgcttagcggcactgtactcggcgttttcggaaagatcaccaagcgctcttgcatccgccaaacttttgatcttagcgggccgggaattttcaagctcacgaatttcagattcaatttgttcgtagccaaacttggtaattttgttgaaatgaggttccatgaatgtatccctcctgacatttttaagtatacaacatgtctaaattatagccaattaaactaattacttataaaaatcggcgaaatttccaacatttttattgaaaataacggcgatttagtcgcaaaattaccagactgaaaccttgttttataagcgtttgttgatgatatgttatgggaatattaccaaatccctatttggtttaacaaggttgtaattttctggacacgtctctgtaaataggttggagtatatttttcactgttgattaaacacgaaaggaaaaatatatttcatgagacttaaaaagatcattatcgcattaatgactgcattaactttctacggcacaatgaacgttgccgcatccactgaaatcgctgaagctaaggctactaaagtatacaaatcaaacttatcaaaggctaatcaaaaagccaagaactggatcgcctaccacgaatcacgcggttcataccatgccagaaatggccgctacatcggtcgttaccaattaagcgcttcatatcttcacggtaactactcaaagagcaaccaggaaaaagttgctgaccattacgttagtcagcggtacggcagctgggtcaatgctaagaagcattggaaggcttatggctggtactaagctataatacgaatatgttaagagatcaaatgatgaacaacacttgttcattgtttggtctttctttttgcttattgattgaatttgagcctccttcaaaattgtaaccgctgtaatgaaccattattcggaatctccgttgtgattcctcaaaattcatgttaatataaaattattgttttaaacacgaataaaaaggagaacataatggaaaatgtttctgttccaggcaagaaatcacctgttcgtaatgcaattttaggttttcaacacttactcgccatgtattctggcgatattttggtaccgttattaattggtggggcactgggattcaatgccgctcagatgacctatttggtatcgatggatattttcatgtgtggcgtggcgacattgcttcagatccgcagaacgccgattaccgggattgggttgccggttgttctagggtgtgcggtcgagtacgttgcaccgctacagtcgattgggaagaattttggcttgggttatatgtatggcgggattatcgtcgctgggttatttattatcctcattgccaagccatttgcgcacatgcgtaagtacttcccattggttgtgaccggctctttgatcacactgattggttttaccttgatgccggtggcttttcaaaacatcgggggtggggatgccactgccaaagcatttggtaatccgacgcacctattccttggcttcttcacagcgcttgtcattattgtcttaaacatttgggctaagggatttttgaagcaaatttcaattttaattggtatcttggtgggttcaattgttgccatcttgatggggacggttgatttcgccgccgttggccaagctcactgggctcagttgccacagttcttctactttggtgtgccgaagtttgaatggtcgtcgattgccaccctgattttggccgctttcacctgtatgatcgaatcaaccggcgtttactttgccttaagcgacattaccggccggaagttggaagaccgcgatcttgaacacggttatcgttcagaaggaattgctgccattttgggtggggtctttaataccttcccatactccactttctctcagaacgtcggaattgttcaactttcaggaatcaaaaagttaacgccaatttattactcagcattcatgctgatgattttgggattgatccccaagtttggcgccatcgcaacattaattcccgcttccgtattgggcggcgcaatgctggtcatgtttggaatggtgggtgctcaaggaatcaagatgctctcacaagtgaagctcaataacaagaatctgctgatcattgccgtttcgatcgggcttggcttgggagttaccacgcaacccaatttgttccagtacttaccagcaaccgttcaagtaatcatgagtaacggaatggtggtcggaagctttaccgctgtgattttaaacatcttattgaaccacacagctttgagcaaaaaagttgaagaataatttaattaaatcaataataaaaggccagcgagttaatcgctggtctttttttggttaacgactgtctcagaaattatcgttttggaacgtattcttcgacatattcagaaatgatattaagcaaatcagtcactggttctgacgtctgtttgttcttgatgaatgaaataccaaagttggctgtcaggacatccgttggaatctcgatgacgttgatgtgtttcttctgttcatcagtcaaacgacgtgggttggcaaatggttccggcgtgatgattgctccgacatgttccaatgcgagatcggaagccaagtgcaggtcgggaacttcgacgctgatttcagctgaaacgccaatgtcgttcaggaagctggtgaccaatcgttggtagttatcttcttgcggtgtaccgatgaattcttcacctgaaagcttggtaaggtcaagatcttcataattcaagaagactttatcaggatcatacagcttggaagtttcaggaataattaaaaccaatggtaattgggcgattggtttgtattcgaccttgtggctttgaagcgcatggccaatgaaaaagtcgagggttcctgacaagagccgtttttcggcgtctcgactggtcattctggtgatttgcgcatgaatattagggtacttgttatagaaccggaccagaaccggtttgtataagtcgttggtcacaacctcattggaagcaatggttaaatggccgtatttgaactgtgacaggtgcgtcatttcgcgatccaagttggctcgcagtcggttttcttcctgtaaaaaagccagaagtcgttcgccggcgtacgtcagctggattggatgagatgatcgatcaatcaatttaacaccaaagttcacttcggcatttttgataacccgactgatataaggctgggtaacaaataatgcctgggcagctttggacatatttccttgtgccttgatttcttcaagaaacgaaagtaatttgctgttcataatgtaattctcctttgaagacctctcgcctttagtttatcttctaaccagattatatgatattctagtaatatatgcatgaatagtgacttctaatgttggtattccacaaaaaagctacaatcaagtatagcaattccccgtgcgccagtaaaggacatgaaccttttagcccgggtattatagtaatcttaagatttcattatttatattaccattaggtactagtacctaatcgttatcagtgaagaaacaaatcatgcttttttctcgttgaatggtaaaatagtgtcataacttttatcccttaaatggatacatagcctactagaagggagttatcacattgagaattgaacaatcacctgaatttcaaattcatttacaaaccttaagaagcaaggaagaattatttctcgaaactatttataatgtcggcaacggtcactttggcgtccgcgactccaatccgctccagggaaacaaccatgattatattggctccccgggcttatttattaatggcttctttgattacgaagaagtcgcctatgttgagaagtatcgtgggtacccggacaataaccaggtaattaaccggttatttgatccacgctttattcgtatcaaggtcggtaacgaagattcgttgaccgatcatttcaaagttgaaaatattgataagaacttggacatgcagactggactgctgcacgagcttttcagcgtcacgactcctggcaaccggaattttaatctggtggttgaaagctttgccagcctgagcaagctgaatgtatacggagtccgatattctgtgattccaaccaacttttccgatgaaatcgaagtgatcaaagttcacgattacgtcaaccaaactgttcaccagcaggatgaagacgtccgcgtcagcattgatctggggcaaatgcagctggactttattcctgataacggccaacccagttacttggtaaccacttttcgaagccagcagggagcgattatcacctaccaagccagtgagaattttgccccgaacccgccaattgaatatttcagagacgatgatcatcactacggttatcggagtaaatattacgccaaaccgggcagcgccaaagactttgaatttttgtttgcgattggcgatatccatccactggtcaatgccaatatgtattccgatcagtacctgtcatcgctgaataattacattaatgacaccacgttcaaatcagaattgatggcttcggcacaagtttggcagactttttggctccacagcgacgttgaaatcgatggcgatcctgctttgcagctgtgcgtgcgtttcaatttgtttgagcttaaccagtcagctgggcgagatgccttaaccagtattccagccaaaggactgactggtaatggctatggcggtcatttcttctgggacaccgagatcttcatgctgccgtttttcacttacacccaaccggaagttgccaaggatctattgatgtttcgctatcacacacttcaaattgccaaggagcaggccagcgactttggtcttggcaaaggcgccatgtatccctggcggacaatcaacggttatgaatccagtgcttactggctggcaggccaggcgcagttccacattaacgctgatattgcctttgccgtcgaacaatattatgagattaccagtgacgatgactttatccgtgattatggatttgaaattattttggaaactgcccgattttggatggagtacggcaactatgccgaacttgacggcaagcgccaatttgtcctcaaccgggtcaccggtccggatgaatatagtgccttagttgacaataactactacaccaacgtattggcccagagtaacctccgtttggcagtcaaatatgttcgcaagttcaagggcgacgacggcattttgagtcgacttcacgttactgacgacgagatcgacgctatggaaaaggccgccaatgccatgtatctgccttatgacaaggagaagaacgttaagctgcagttccaaaactttgaacagcttccgaaaatggatatttctgccattgatcaaagcatgttcccattgctcttacactatcatccattaatgttgtaccgtcaccaagttaataagcaggctgatacgatcatggttgattttatgttccctgaaggcaacaccttggatcagctaaaagccgactatgaattctatgaaccaatcactacccacgattccagcctctctaaggcgatctacgcgattattgcggctcggatcggtaaggatcagcaagcctacaacttcttctctcaggccgttcagacggatctgatggatgttcatcataatactaaaaatggcattcacgccgggagtttgggcgctgcatgggaagggatcatgtacggcttcgcaggaatcgtcaataatgcgacgagttttagcctcgagccccatttaccatctacttggaactgcctgaagttcaaggttcatctctatgggaatgaatttaaatttacgatttatcaagactcggttgaagtcgagctgctgagcggtgaggggacagatatcaccgtttatagccatcgtaaacacctcactccggacaataaccgcgaaacttggcaatactaaatttttttgaagaaagtctgaaatattaacgtcttttttggaaaacaggcgaactttggtttatgatttgttatgatagtgttatgcaaattcatcgttgattgctgaatatttaaacaagcccttgatcgttttgggcgagtcaatttatctgatgtgaaagggatgcactttataatgaagaaggaagctcgtcaatccaaaattgagcagattattaatcaatataccattacaacacaggacgaactgatggagaaactgaaggtggctggtattagcgtcactcaggccactttgtcccgggatatccgcgagatgcagattgttaaacagccggatagttcaggcaactcacgctacatgatttttaagtcgggtaaccaaaatgaaatcgagcggatgtatcggatgattaacggcacggtaaccgacattcgccagattcagtttgtgaacgtgattcacactcagcccagttatgccaacccattggctgcggtaatcgatgatctccacatggaaaatgtttccggaacgttggccggctacgataccattgtgactttcagcccgtccgtagactctgctcgtgagattaatgatttgtttaccaagcacgccaatccagacttgctggtttcttccattcaggatggggaataggcattcataatataaaaaataaggctttctcagctttgaggaagtcttattttttgtgctggtaattattttgcgaatcgtcgataaatgcgtcgaccaatcgccccaatcagaaatgccagccaccaaatgatgccgactgcggtgaccagtttgccaagcgcgagtcccggcgtttgatatttcagtgaaacaaagtggcggccaaccggaattctggcacccacaaagccgtgattgaccttgaagatgtccccggcctggccatcgatctttagatgccaaccggtggagtagggaattgacgtggtcaatatgcgggtgcgctccgttgcatccgtatagccactcacagaattattggtgactttttgactggtcaaaccagctttttgaagttgttgaatgcgggtgttgtactgccggttaaatggtacggccatcaacttgacactcctgaacttcagttgcttaacgccattaaagtgaatcgtcatcgacttttgcagattgtcggcgtaacccagattcaaaacaatgtgttgtctatcctcgtaatcggagaggttgttttccggtaattgacggacgtaagtgaagttgttgggggtttgaaccgacaatgtgtaagcaccgagatccggatgctgcagagcagttctgatacgatcaattttttgcagtttggaaaccggggtgccatcaataatcgaatcggcagtcaggctgttcagtcggtctgcagtggaatgagtggtgtgggagatgccatcgatcaccagatacaactctgaatgacgatatttttctggctggttaatgtttaattgatatgaaagatggcgtccctgcgcatcattatccatcagatgaaggccgttggcatttgcagcctgattttcggcaacgatccggtgattcttagccagcacactttgtagcggcttggcattgggattgatgccagtggctttctcccagatccggatcttgttggccggtaaagtggtcttgtatttcttcgcggtatcacggtagcgggcgtttggtgaaatccgcagccgatccaagacagccttgactgggttattggcgatgtgttcgtcaaataatcgtgtcgtatacggcacattttgaatgttgttctgcggttcggtcatcgaaacgccatcaaccggcttttcaaccacagcccccgataacatagcctgttcacgttgaagcggtgacatgttgcggtagttggcagctgaaatgacatatttttgtgtatagactaacggcaaagccaaattggattttagcaaaatcgtcccggaatggttgcttaacccgctcaccggttgttccgggaagtcgacaattttgccgtttttcccgcgaacataatggaacccatagggaatggcttggggctttttgacaatatccgttttggcaaacatgtatttaacacccagcaggttcagcagggtggttctaccatctgcttcaccaagcacggagttgaccaccgcctgtgaattatccagtgatctgctgaattgaaacaggctgccgttttggatggagtaataagcccccaagtcatgggttcccaagaccatcgggatattgttgccggcggttcggtggggatagtagttgtgaatggtggttgttcgatagaagccaccgttttttgccaacccattttgagcaccatcataatacttgtgaagccactgttcagccgacccggatgccaggttggaattgatattcttactattattggggctgaaccagccttgcccggcactaatgacgttaatgaagacgagtccgaccaaaatggtgccaacgtgcctgggagatattttaagcgacgtttgacaggcaaacaatagtagaaagctcagcaataatccgtaagataccaaatcgttttgcggtaatttgagggtaaagcctttggtgatccacacgagtacaatcaagccggcactggcgccaatcaaccagcgcaaatcgttttgagtcaggttcttgagttgatcaaccagaatcatcgttgccaagctcattggtaacacgatcaggaacaaccagcgattggacggtgttgacatggcgttggccactgcactaaactgcggcagcatcaacgcaatgatcgttaacgtgataatggttgccagtgatcggtagcgtttgaaatgtctgaggacgtacactgctccgagaaatgtcaatccgcagaaatttagcaccagccagtaatccttggtggtggtactggtgatcagttgattgggcatcgccagatagtatttaagtggataaagaatcagtccgttggcaaacttggcatgataagcaattcgagttgattgaaaaacggccaataaagttggaatcaagatgaccccagcagtcagcaggccagtcacgacaccctgcaccaaaccgtagataattctgccgttcttgagctgctcagggtggttgtgacggatgttgaagtatctggtcaatagatagacaaacgtcccgattgccagcatataagcgaagtaaaagttactgatgagggccaaggcaacggcaaccgccaacggcagccagttctgcttgtggagaaccttttcaatccccattgccaacagcggaaacagaatcatgggaattaagaaaaatgggtgatgcatcgagacatagaagttgtagccggaaaatgtataaatcaacgtcccgattaatttactgtgggtgctgaaatcgcgctcgttggcccaagccagaaatgacaggccgacacagtaaagacgaagcaagattaagacttgaaagccgagctccagcttggcagccgggaaaagggcaatcaggtagctgaatggatcaccaattatgtaaaaggcaaaggtggtgagttgatcggccccagctccaaggttccacgaccagccgctcattgcctgatgggcggttccttgaagcattcgctgaaattgcgccataattggaaaatgttgggcaatgccatcgacgttccagatcaaagttttgccggccagccagggaatcgtgtaggtggcgaggcagacaagtagaaaagcgatggaatagatcaaataagttcgaaactgaaaagactttctgcgagtatcaattctcggttccatgaaattacctccaatacatatcccattttgcctgcattgaggccgatagacaaggctattgacagatttttaatgtttgtaacattgacgccctcaagttgaaacaatgtgcatgaacattcatcgatgaattttagtaagctgagtaaaacgcttacatagccactgatttgttcaaatccggtcccagcaaaagtgaattttcttttaccaaactgtgaatattttatgaagtcgaaacatatttataccaaacagatgagaacaaagtatgaatgttgtgaagaaagtgttatagttagagcattcttaaatctaatcaaattcttatgttctaatttaaacattttgttttgcataattaaccgctaaaagccttttgtgaaaggaataattagcaggataatttataaaatgaaaccgcaatcattttcggccttaattgtgtgagttttttcacgttcacaatgtccaaaaatgtacggtaacctttttcaaaggggttatgatgtacttgtattaatggaagaggaggtaacaaaatgacaagtccaattcatgtaacatcggaaatcggtaagttgaaaacagttttactgaaacgtccgggtagagaaattgaaaactttacacctgacatgatgccccggttattattcgatgacattccatatttaccaattgcccaaaaggaacatgactactttgccgatactttacgcgacaacggtgtcgaagtattgtacctcgaaaaattagctgctgaagctttagacgcagctggtgacaaagttcgtaatgatttcttagagcaaatgctgactgaatccggatatgcaacaggaaccatccatgatgcattgaaagaatatctcagcagcatgaacaaccaagacatggtcaacaagatcatggagggtatccgtaagaatgaagtagatttcgtgccaacagacttagtaagtgctgctgaaaccgagaactacgaattctacatggatccaatgcctaacttatacttcacccgtgacccttcggcatgtatcggtaaaggtttgagtatcaaccacatgacattccctgcaagacaacgtgagtcactctttaacgagattgtcatcaagtatcatccacgttttgctgacaaaggggttcatgtatggcgtgaccgtaaccacgatacccgtatcgaaggtggagacgaattagtcttgaacgatcacgtaatggcaatcggtgtttctcaacgaacttccgctgacgccattcaagatattgctaagagcttatttaaagaaggtcactttgacacagttattgcgattaagattccgcataaccatgcaatgatgcatttggatactgtgtttacaatgattaactacgatcaatttacggttcatccaggaatccttggtgagggcggccatatcgacacttggacaattactccaggtaagaacggcgacttgaacttggaccacagaactgacctcaagcaagtcttgaaggatgcgcttaagctggatgatttggacttgatcccaaccggtaatggcgacccaattatcgccggccgtgaacaatggaacgatggttcaaacactttggcaattgctccaggcgttgtggtaacttataaccggaactacgtttcaaatgacttactcagaaagcatggcttaaaagtgctggaggttatctcaagtgagttgtcaagaggacgtgggggtccacgttgcatgagctgcccaattgttagagaggacatctgagagcgcgactaggcccgggttgaccccggagtgtaagccgggaattttaatgatgaacgcctttagttcatcattggaatttttggcttacacagttaggggtcagggccgtcgccaagtaggctaggcaggctttcagccggccgtcggagcgtgtttacatcagagcgcgacgagcaacgggtgaggcggtttctaagggtactttgcttgaagtccctgggtttgggactttaagcaaagtgcacttagaagttagcctcagttgcgtcgaagcgtgattacgaggcttcctcatccaggcagctgacaaaaaaccaccaactcaactctactctacaaacaattaaagcaagtgtaccgtacccaaaaacaatcatcatcaaggagaattcgattatgacaaaagatttcaagcaaaacgtatttcaaggacgcagcgtattagccgaaaaagacttcacagcagccgaactcgaatatttgatcgattttggtctccatttgaaggcacttaaaaaggctggcgttccgcaccactatttggaaggtaaaaacattgccttactcttcgaaaagtcatcaactcgtactcgttcagcatttaccactgctgcgattgaccttggtgcccacccagaatacttgggatcaggcgacattcaattaggtaagaaggaatcaacttcagacactgccaaagttcttggcagcatgttcgatggcattgaattccgtggcttcaaacaaagcgatgctgaaattcttgccagagacagtggcgttccagtatggaatggtttgaccgatgaatggcacccaactcaaatgttggctgacttcatgactgtgaaggaaaactttggcaaacttcaaggtttaactttgacatttatgggtgacggccgtaacaacgttgccaactcattgttggtaaccggtgccatcttgggggttaacatccacatcgtttcacctaaagagttattcccaactgacgaaattcaaagcatcgctaagggctttgctgaaaaatctggtgccaaactgttgattaccgacgaccttgatgaaggtatgaagggctcaaacattgtttataccgacgtttgggtatcaatgggcgaaagcaactgggaagaacgcgttaagttgttaacaccatatcaagttaacatggaagccctgaagaagaccggcacacctgacgatcaattaatcttcatgcactgcctgccagcattccacaatactgaaaccgaatacggcaaggatattgaaaagaaatatggcattactgaaatggaagttactgatgaagtgttcaccagcaagtatgctcgtcaatttgaagaagcagaaaacagaatgcactcaatcaaggctatgatggccgcaacacttgggaatttgtttattccacgtgtataggacaaagtaaaatttcagcctagtacccaccttgaaaaatagctcaacaatacaagggactggcaacaaaacatttgttttgtcccagtcccttattattttctaagacggaggagaattattatgggacgtaaaattgtggttgccctcggaggcaacgccatcctatcaaaagatgcttcagctgccgcgcaacaacaagcgttgcgcgataccgctgagcacctggttaaattcattgaaaatggtgaccaactgatcatttctcacggaaatggtcctcaagttggtaacctgttattacaacaagctggtggcagcaccagtgataacccggaaatgccgctcgattcttgtgttgccatgacccaaggcagcattggctattggatgcaaaacgccatggaccaagtgattaaagaaaaaggcttggacaagactgttgcgacagttgttacccaagttgaggtcagtgctgacgatccggcatttgccaacccaaccaagccaattgggccattcatgagcgaagaagatgctgatctcgctaagaaacagaacccggacttcagcttcgtggaagacgccggccgtggctatcggcgggttgttccttcaccaaagccaattggggttgttgagacgaaagcggtcaacgccttggttgatgccggcatcgtgccgatttcagttggtggcggcggtgttcctgttgtcagtgatggtagtcgactggctggtaaggaagcagttatcgataaggatttcgccagtgaaaaacttgccgagttggttggtgctgacgcattgattatcttgaccgcggttccaaatatctttgtcaacttcaacaagcctgatcaaaagaaattggagcatgtatcagtcgctgatttgcatcaatacatcggtgaaaagcaatttgctccgggaagtatgctgcctaaggttcaagcagcgattgactttgttgaagcaactggcaacgaggcggttgtaaccgctttggataacatcgaaggatttattaatgatgggtcggggacaattatttcggcaaaataacacataattccgattttgtccttaaaatcatcttagactttgtttaatgtacaatctggttatttgaggtacacttctaatgagaacacaattatgtaaccgtttttgggagtgtatttatgattttaaagaataagagtgattatgagtattatgctaaaaaactgcgccgccatcctgaatttagtccgctgagtgataagtatatcaatcagttgattgatgagatgactgttaaaacctatcatcgcggtcaaatcttgtttgaccagggagatacccgtgatcggttctattatttgatcgatggggtttgtaaatcttttcactgggacaaagacggcggcgaacagctgtatctgtatattcgacccgaaaaggcattcccatatattggtttgtttgaagacgatcgctatgcatacacggtccagacaatgtccgaggtcaaattagccgagttcccgatgccgatttatgaggaaattttgcgtgagaaccctgagttgatggtcaatgctgtcaaagaaatgagtcaaattatcaacacctctgagactcagcttcaacgcatggtgaccaccagtgcaaaatgccgggtttggaacgcaattctcttcattggtcaacaaattggtgattatcaagaagatgagacaatccttgttccgtatccaattacattggttgaactgtccaaggtgagtggaacaacgagggaaacgaccagccagatggttcagcagttggttgccgagaacaaggttcaatataatcgcaaatatttcaaaattttagagattgacgatgattcatattaattgaatattattcaagggagtgagctaaatgaaagagcatgatggtaaattagggctgctcgaactgatcggattggttgttggatcaatcatcggtggtggtgtgttcaacctgatgcacgacatggccgtaggagccggagccggtgcgatcatcattggttgggttattaccgccattggaatggtgatgttagccttgacgttccagaatttgaccatgaagcgtccagatctggatgccggtgtctatagctacgctgaagctggctttggtaagtacatgggatttaattctgcatggggctactggttgtccgcttggcttggaaacgttggttatgcgacactgttaatgagtgccgttgcctacttcctaccggtatttggggatggccaaaacatctggtcaatcattgcagcatcgtttattttatgggcctgccattttatgattttacgcggggttgaatctgcatcgtttgttaacacaattattaccattgccaaattgattccaatcttcctattcatcattatcgtattgtttgcgtttaagatgaatatgtttaccagtgatttctggtttacaccaagtgggaaatttgaatttggtagtgttatggcacaagccaagagtacgatgttagtaactgtttgggtcttcatcggaatcgaaggggcggtcgtcttctctggccgtgcccggaaacgttctgacgttggtaaggcaacagttcttggaattatcaccgttattttgatttatatgttaatcacattactatcatttggtgttatgagtcgtgcagggttggcacacttaactcaacctgcgatggccgaactgcttcaaagcctggttggtaaatggggcgccatggttgttaacggcgggttaatcatttccgttgtgggtgcctggctgtcatggaccatgttcgccggtcaattgccatacgaagctgccaaagaaggatccttcccgaagatgtttgccaaggaaaataagaatggggcaccaattacctcattgaccgttaccaacatctgtgtggaaatcttcatgttctcgtacctgattacggcttctgcttataacttcttctattcaattgccagtgccgcaattttgattccttacgcattttcagcattctatcaattgaagtattcattcctggaagatcatggcaaaggacgaaccggcaacatcattgttggaattatttccagtctgtatgcctgctggctgttgtttgccgctggagccaacttccttctcttgatgtcactgctctttgctgccggaattccagtgttctggatcttacagaagaaggataaccacgccgagaaggtctttggaccgattgaaatgttgctggcaatcttcattgtgctggccgcaatctatgcgatttatggattgattgttggacaaattactttctaattgtaattcgtgacggagaatgaatttgaacagccgtatatttgtaactaagggagcagctcaaatgagccgctcccttagttattgattcttttaaaaataagcagtcacaaacaaatacccagccaaaccaaatgcagctaatgaaatcaaaatccgcagcaaatggatatttgagtgacggacaatgatcggtccggtgtagccgccaattagcaagccaaatccaagcgggatcaccaatagccagtcaatttttgacttgaaaataaaaataacggttgcaatcaagttgccaccaaaggcaatcacattcttcatggcgttgaccacggtaaaacgatcatcagtgatgattgataaaattgcgaggaagataacgccgcccgcagcaccaaagtacccagtgtaagctccgactaggacaattccggtcaggctgatcagtgacacccagaagcgcttggttggcgtttggtgtgcctgcttcaatttggcagtggaaacgtccttttttcgaccggacatgaataacagaatgccggcgaagaggatgaagaaaggaaccactttttcaaacgacgaagccggtgcaatcagcaacagcacactaccaccgatgcttccgataagtgaaagtatgacgtacagggtcaattttttccaatgccctcggagttcctttagcgaagaagccgtcgcaccgattcctgagaagatcagggcagtggtattggtaacattggcaataactggcggaagccccaccgctaacaaggctggataggagacaagtgaagccagcccggcgactgaggcgagcaatcccgctgcgaggccggcaatgattaggaaaataaatgtaagcaccatgagttgggctgacctcttttcaattttttgatacttctaatatactacattttacaaagtagtcgaattcatcttgtgaggggcttgatttctgatgcccaacccttgataatatttaactatcaacacaagatgaaagcaggttacccatgacacaattattttttgactttgacgggacgatcgccgactcggaagccggcattctcaaatcgctgaagtacgcagtcgacaaaatgaaattgccggaactgacacatgatcaatacttgaaatttattggcccggcactcaagaccagcctccaaaaattttatccccagctatctgaagcggatcagatgcaggcgttaaaatactatgccgattattaccgtagcgaggggatgttccaactcgatctgtatcccggcattgtccaggagttgcaggccttgaacgaacagggctacgacgtcaatatcgcctctgccaagccggaagatttgattcatgaattgacggatcaactagatttgacgcaatactttaccggtcgatttggtgcggggactgacgagaaaacccggatgaccaagacagcggttctcaaatatgccttggaacaaactcatgccaacgccaacgacagcatcatgatcggcgaccgtgacaccgatatgcttggcggctatcacaatcaggttaagacgctgggagttacttatggatttggcgacgttgccgaactgttgggcgcccatgcgaatacgttggtggataagcccgagcagattcagggcggggtagagaaattaatcagctaaagacgccaagagcgtgggccaataagcggttagctttcagagtataaggggattacccgaatatccagaacttggatatttgggtaattcccttatacggccggaagctgcttattggcccacagttctgctagataatatttaggcgcaaaacgaggctggaacaaaatttttagttttgtcccagcctcttgttagtgactaaaatttctattaaaaaagcgtgctcccagataacgactatgatcgtttggttcactttaaggcttgatataggcaaaaccctgttcctgcagtgaaaccaaatcagcgacaccggcagcgacgatttcaacgtttgccggtaactgattttccttaatcgaatggctattcatcgaattattgcaggcgtggaatctaaccccttctcggctgaattgctcaacggcatttcgcagatgctcgtccaaatagcctttgatggcatcgccgttgactaagacgacaatgtggtattcttccttattcacccgtccataatccagcaggttactaatattgctcagtgtgtgatcccacttatccaattcatcaatgtgaaagacaactttatgcatcattattccctcgtttcatccgcgtccaacgaatccaaaaattcctggtaatcctcgtggacctgttttgaatattcatttgcccagttaattaaagcggagactagttttttcttggtgccgacatatccgtgaacaatcgcggcggtcggactttgggcgtggccccgtgccagcaggagcccacagattttagcgtaggtggcaaaatcatcggcgtctaatttgtccaagttaatcgattctttcatgtcccagaactgacggacatagaagctgcggccggtatcatcgttgtgatagaagcccagcagtggatcagacgcccgctgtaaaatttgctggcaggtgacgattcgctcaccattatccggcttgctctggctaaatggggtcgtcacatcaaaacctctaaaacgccgagtctgcaaggcctccttgatttggagaaccaggtggctgccgtcaatcgcggttaacaagaccaggtagcaccgggtgccaaaactaccaacaccgacgctatggcggacaatatcactgatatgaaattgtgaaaggaggacggtgacgtccgggctgaccgagcgggtgtaactccgcaagtgctcgcgaatttcgttgaagcggcgatcactgacatggacggttcgtggagcgttttctttaaagacaagatgtccccgggaatccaatgtcgtgaattttttgaccactttatccgagttccgttgttcggcactatctcgaattttgcgccaaacttttggtagtttgtgatcggagtcctccgactacaggaaggattcaacttctgtggagaagtagtagcgttccattgccgagtggtcatcaaaacattggctgagaatctgctggtaggtttcaaccgctccctgcataatctcgttaatttggtcgctggctagtcccagctgctctccttggaggacaatgctgacaagcaggcgccggaggtcccagtcccatgagccaatggtggattcatcgaagtcgttgaggtcgaacagaagttttcgctcaggagacgcataaaaaccaaagttccccaaatgagcgtcaccggaaatgaccaccggaatattggtggaggtctgtttcgacaggtcgaaagccatcaattcatccgtgccgcggaaaaatgcgaaggccgaggctgccagacgcttgtggcgcagcggcattaaatctccgatcatcttttcttcaacgtgagaaattccttcaaccacgttacgcttaaccgggacaaattttcccagctggtcaaatgagatccggtcacgaatcttttttccgtcatcaatcagttcgtgaatcgatttattaatattaattttacttaagtcgtagtgcaagcccgtggttgttcgggtaaaagtcttgctggtgtctgccatttaagtcggctcctttattttgacaatctataatatcattgtggcaattcccggtccgtgagtcaagcgaagccaactcatccgccggcttgatatgttacaataatggaaatagacgatttgtaggtaatggagaattacatttatgaaaaaattgtattgggaaagcatcgaagtgaataatcaaaaattcttcttcacagtcactgaaaaagggttgaactttgtttccagccccggtaagtacttgtctgaactttttgatttttaccccgatcgttatgatgaccaatttatgtacgacgattcggtgaccgctgattatttatctgaatttaccgattactttgatcaaaagcgtcaagactttgatttgccgctggatttggagaatatcggcaccgatttgcagcaccaggtctgggcagaaattcaaaagatcccatatgggcagacagtcacatacaagcagttggctgaaaatattggtaaacccaaggcaatccggccggtggctcacgccgtggctatgaatccggatttgatcgtgattccgtgtcatcgggtggtacgcagcagcggcgacatcggcgagtaccgtggcggtaaagaaactaaaaaagcccttctcgagttggagaagaagccgattgaaaagcatgctttgattagcaagttaccgttgcctaagcttagtcaactaggtaaatctgatctttaattaaatcaaatggttggtgatgtcggttcagctgtttggcagtctcgggcttgatgaaatgggcttgttgccagaaagctttggagtcggtagcaccatttttttcgccgacaacgattaattccaaatcgttgtcggcttttctaatggcattgaggacgtcgacatcaatcgtttgtttgtccggtgaccagctcatgataacgtatttcacctggctctgatatttggcgattgcagccagcgcatccagtttttcaacgggaatcagctgatgcttacccgtttgattttcgtcaacccattcaagactgtcggttgggaagacttttacgccaagatcattcagtcctttggaaatatatccgttgccggccatcacttccagcaccggtgagtcaccaatggagtcggcgagatccttgataaacggggcagagatataggcccacatcccgtattgactctctaagtaatcccggaatgaacgcaattgtttatcaagtttgggcagcgcatccgacagctcgttccaaagctggtcgcctttgggatcaccgggtttgaatcgaccgttgatatctttgaaaatttgatcttggatatcatcggggagaattaattccggcaagtcttgcggtaggagtccttgtttgattaaatggtcactttcaatgacattattgatgagaaatttaacctgtggataggcagcaaattgatcgcggtattttagcatctgggcgatatagttggattcagccggttgggtagtggggtgctttttcttgagcaactttttcttttgtttattggttagcatactggactccttttgagataagcgtttgagtttcttttttggttagcactgaatgtgacggtacgtaaatacgctcaccaagccaacttcgaccgcattatccaataacgaggctcgatgcgcgaaaacgcatcaaacctcgttattgaataaatgctcagaagttaaacagcttgcttgagacattaaagatctaattctccttgttccgtccgcggtccttgatcgtgcggggcattgcttcttccgtggacgtaacctgagattaactgatagatttcatatcggtccttggaactcaaatcttgaccattaaattgcaaggttttatctgaaataaatagtcgcgccaagtcataggtattattttcagataaccctgtcaaataatccatggtgacgtcgaagaacttggcgaggcgctggatttcgatgtagttgggcgttctgatgccacgttcccagttaccgatttgagagccggtactttcatgctccttatcagtcggggaatctttgttgatcgcgcgggctagttcttccaaagttaattgttggccttttcttaatgctcgtaatctttctggaaacatgtgatcaccgtcctgttcgttacttatattatacgacttttttgctaatcaccaaatttcggcgttaaaattcagaatgtggtatatttatcacgagaaaaattgaattggtgggatggatgaatgaaacgaaaaacaaaagtttttattggattggcttctgcagttgtgatcatctgtggtggtctatttggtgccgggatgtatttttacaatgttgccgtggtaccggctcccaaatcatttttaagcaagactgagccaatcaagcccggcaactcgcgctatccggcctacaaatggtatcagggtgctgacaagcagcattggtttgaaatgtctgctactcggcaccttaaattagatgccaattacatatcagctgacaaggccaccaagaagaccatcattattgctcatggcttcatgtccaacaagaaccgcatgttcgactatgcctacctgttccacaacctgggctacaacgtcttattaccggacgcccgcggtcacggcgacagtcaaggaaactatatcggctatggctggccggatcgcttggactacgttaaatgggtcaaaaaggtcatccaccacaccggtcaaaagtctgaaattgcgatttttggaaccagcatgggtggtgcgacgacgatgatggtcagtggagtcaaaggcctgcccactcaagttaaagcgtttattgaagactgtggctacacggatgtctattccgagattgcctaccaggccaaggaaatgtatcatctacccaaattcccgttggtcgacattgtgagcgggattaatcacatgaaaaatggttattcgttcaaaaaagccagcgctttgaatcaagttgcgaagaacaaacggccgatgttgtttattcatggtgccaaagaccaatttgtcccgaccaaaatggtttacccactgtatcgggctgacaaggggccaaagcagctgctgatcgttccgggagccgctcattcacgttcatttagtacccacccgaaactctatacggataccgtcaaaaagtttttgaatcgctatttgaactaactataaactttggcgacttcaatcagtgagtatgttaaactactattaggactgtttttagaaaggaggtccgcacttgttactaatcataattctaggaattttggcggccatcgtgggtgttgcatgcggcatgcagctgcaaaagcgtcacttccagcaggagattcaaaatgctaaagccactgctgaaaagctgttgaacaacgccaatgaagacgccaagaaacaatctgccaagattattgccgatggcaagcaacaaaccattgactaccaggattcaattgaagaagaacttgacagctaccaagccgataacgtcacccgacagaccagaatccaacaacgggaaaccggtttgaagcaaaccgaatctcgtctggatcagctgcattcaaagctggctgacgaaagtcatgaaattaatcagcaaaaagctgaaattgaacagcttcaccacaccgcaaatgatttgtcccaggaacgattaaaaacgttgcaggagcgcggttcaatcagtttagccgaggctaaacaacaaattctcgatgaattgaagacggcgttgaagcgtgaaaaagatattgaattgaaatatcaagatgacgaagcacaggtcaacgcgccaaagatggccaaaattttggctgacgacgccatccaacgcggacccgtcgacatgccgcgtgaacacattgagcattcagtgcaaattaacgacaacaatactaagcagaagttaattggtcgcgaggcctctaatattcgctacatcgaaagtttgacgggtaccgatttggtgtttgatccagatgatccgcatttgttacacgtggtcacccaggatccactgagaagagaagttgccaagacggtgattaccaacttggcggtcactaagcagattaatccgcaatcaattgagcaccaggttgagagcgctcaattggatttgatgaacgagctccggcgcaccggtgaaaaagtggttggttcgcttcacatcggctggatgcacccggatctgttaaagattgttggtcgactgaagtatcggaccagttatggtcaaaacgttttgaatcactcgattgaagtcgctgatatttcagggatgctggctgccgaattgggcttgaacgtcaagattgccaagcgggccggcttactccatgatattggtaaggcaattgatagagaagtggacggcactcacgttgagttgggtgttaagattgccgaaacctatggtgaggacccacaagtcatcaattccatcgcctctcaccatggggatgttgaagtaacaacgccaatcgctcatctggttgcggctggagattcaatttccggtgggcgcccaggtgctcgaagcgagtctgttgaagagtatgtcaaccgactcaaaaatctggaacgcattgccagctccaagcagggtgtcaaagaaagttatgccatccaagcgggccgggaaatccggattgtggttgatccaaagaaactggacgatcaacagaaccaacagttggctaatgaagttaaggatgagattgaaaatgagttaacttatccaggtaagatcaaagttacctcgatccgtgactttaaagcggtggcttatgttggcgctgagaagaaaaaagtgcataaacgattgaagaaagcataattaaaaaaagacggggacaagggaccttttgattcctaccatttaacacaaaagtgcaatcattctaaaaccaagaatgattgcacttttatgttaaatggcaggaattggcctattgttccagtttcttttagggtgcgatggaacagtttctaatttcatttaataaagtttgtcgctaaggcataaaccaagaaaagcagaacaccgacaatactgatattcctgaccaaacgcgggattttgtatgccggaacattcctgtacggtggcattatttcgcttgcccatagataaaggccaatgatagcaagaaagcaaaatgagagttgatatgaaaaacttaggccaatccggacgagcggcatgaggacgaatatcaaaccgcaaaacaccagatataatctaatttggattttaaatgatcgattgataattacagaccctttcttcatttagttggggttataagagcattttaaaaataacaggagccttttgatcttgccgaataaattaattgcgcttctcagaatcagaaataatttcaaaattatgattgacggtggcttcaatcaccggatgcttctgtaagtattccataatcacgtggctgattgtcatatcacttgatttgacgatcttatcgctggtatacatgggatagtggccgccgccgcttgctcgataacggttaagggcgatggtcaggacttgatcgtcttggacatccttgccatgatacttcaatcgggtgactcgatgaccaaccggtttggaaatattcagggtataatcaatcccttcatacatatcgtagttataaaaacgttcctttggaaaaacaaatttctcgttcaccacgacgtcaccgtgccggaccgtgaagtattgagcggtcacttccaaagcgccgcgcaaatcggcgccggtaatctttgaggcgaccagggtgtttggatacacgtagttggtaatgatgttgcgcatggtaatgggatcttcaaatccgtgggcctcattgttgtaaagggcggttgccgaaaggtcagttcccatcttatccatttgaattttttggattaattcgataaatgctgattcgtgaattcgggctttgaatgggtcatcgaaagttaagctgcccttgattcttgaaagcggcttgtccagccacgcttccaaatgtttggataaatcggtaaccgttgatttgattgtctggtcgggttcactgtctttaacgttcagcaattcggcctcacttcttgtgaccgtgtggttcttggtctcaatcgaaatcttggccacgtattgtccgcgagaacctggctgaacaattggcacgttaaataactggctggcaattttgcggtgttggtgaccagagatgagcgcatcgatccccgggatattcttcaagatgtcgtagccgcggttttcgcctgggttgatatcgttccagttaccggtatgatcacgttcaaaaccgccgtgatacacgacgacgaccacatcggccttcttgcgcatttccgggacgtagcgtctgcacgcgtccaactccgaaatgagattaaaatcgttgagatcattgacgttcttccattttttagtagaagtggtggtcaggcccaagaaaccgactttgacgccggcgacatccataattgtgtatgggtcggccaacagcggttcgttattgttatcaacgatattggcgcacacaaaatggcggtctgaattcttcatcatgtagttgagataatccagtccgtaatcaaattcatggttgccgatggtgccgagttggtagccgacttggttataagcagtaaaaaatgcctcttggtcctgcttatctgctcgcttggccacgtaataagccatcggtgatccctcaaggaaatcgccgttatctaacacgatgatcttttcatcgggatgggtcttttgataatttttaatcgtcgaacacgccttctcaataccgaagggtttatcaagacctgaatcaacgtagttggtaggttcaataaacccgtgcgtgtcgctggtcgctagtagcgtaattttcatattttcacccacacaaaatcaagtatatcgtcaagtatagtcaattatgccatgattgtaaattagggttggccaaagtagttaagccaacaggaaatcggttccggatccctgctccatgtaagccatctgatcagtggaaatactttggctgagctggtctgacaggcttttggaaatcttaccggctttgaaggcatctgccacgtaggcgtattcatattggaatgatttaattaacaagctatttctgtcactgtcagtttgggtgtcacctgcagaacggctctggcggaagctgtatgagctgcggacaaaattaactgcattgctgttttgatcgtcttcaatttggtctaaatagctgttggcactggtaaacatggcgtctttgatcaatagattagtctgttggcgctggtcatgaatctgctggcgggtttgcttgggaatggctgcttggattcgttgtttgatttgtttggttttcttccgcgatttaaatcggcgcagctggtatttaaaaatatacttaatccttgtccaaaagcccaagtggttgctgggcgctgtgatcatccgtcgtgaaaacaaattggcaatcttttggtcgattttgccctcggcggctaaatcgaccaccgcttggacgctgacttgctgggcgccggccataatttcctggacctgtttgcggtcgacttccggattatttttctggctgttcaacatgtcaatgacatagttgcggtccaaaagtgcgatcgtcgagtcttgtttgacctgggaaatagcgtagttgaccatttcaccacggtattgattgaactgaccctgatcctcaacttgctttttcggacataacaggggcagggtgattgttgggacaatcaggcttaataagatgacaattgtggcaatgtagatcaactggtcgcggaatggaaacggctggccaagggacgtcagcggaattgacagtgccatggccaaagtaatcgttccatgaaccccaccgacagcgctgaccagggcttcgcgcgtcgttgggactttatcttggacgccaaacaggttggtccgcatccaaatataccgaatgagtaacataaccagataaattgccagtgcatcaaagaccaatttgataattaaggtatttgaatagggaatcattcgtttgatgactttcggcagggtaacgcctaagaggacgaacaccaccccatttaagaggctggtgatcacacctcaggtcgcattggtgaccagccgcacactggtcgaagtgagctttaaacggctttgattgatgccgtagatgatgccggcagccacgactgccaaaatcccggaacatcccagttcctcggaaaataagtaaatggcaatcggggtcatgatactaaatggcacgatcacactggcagtatccattgatttattgaccaatagcgtttgaatttttacgaagatcaaaccggcgactgcgccaaccaccaggccgccgaagaagctgatcaaaaaccgcgtcagcccctgagcaaatgagaaatccccggagataaaggatgccagggctaaattgaagataacgattccggaagcatcgttgaataaggattcattttccagtgcaccggaaacgcttgtcggcagttcaatatctttagtgattgatttgaaggccacagagtccgttggagtaacgattgcggccactgcaaagcaaagtgccagcgggatcagcggcagcagcaagtgggcgactaagccgatgatgacggcggtcaccaccgccaggatgactgccagattcagaatttgtctgattgaatgtcgaaaatagctcgcgctcgtgttttggccgtcattgaacatcaacggcgcaatcaccatcagcatgaaaatttccggctccaaagaataattctggaagaatggcagtaatgataataagaagccgcaaccaatttgatagaaggttaacgggaggctgggaaagattgtgtacaagatgttagcaatgatcgcagccacgattaacagggtgagtgaatagaagactagcatttttttctcctttaaatgattttaataccaatattatagttgattgagcagataaatggtgtataattaatttcacaagtaagttactataagtaagtaaccgtattgacaaatattgtcagtatgataatatagtaatcgaaggatgttgtttctcgtttgtattttttgttactgagcaggggggaattgtaatgctgaatttatatgtagcacaaagcagcgcttcaagtcggaaggcacgtgcatggttgaagagccatcacattgattttaaggaaagaaatatcaattccaaccctcttaacgctgatgaggtaaaacaaattttacgtttaaccgaaaacggcagtgaagacattatttctacacggtctaacatctacaagaagttgaatttggacctggacaacttaactgtttcacagttggttgatcttgtcgttaagtaccccgatttgattaaacgtccgattatatttgacgatcatcgtcttgaggttggatttaacgaagaagaaatcagaagattcttgccacgaagtgttcgtgaagcagaacttcgtgaactggaatcacaaattagttaattcataaaaataactaatcagttatacggatcaattgaggaacttgggtaatatcttactcaagttccttttttagtttgtgaaatcggcccaaatcattactctcccacgcggataaaattatcgataactttggggcaattttaatttgtacggaacaacattaaaagcaattaaggaactgtttatgattctcacataatgtaaggacgacggaaaattcctagtgttgtgtttcacgtgattgttgcttaaaatcaaatcagataaataaaggagacggacaagttgattaaaatggtcgcacttgatttagatggtaccttgttaaccagtgacaaaacaatttccaaaggcaatgagcaggctttaaaagccattcatgacgccggcgtgaaggtggtgctctgcaccggccggccgattaatgccatttggcggttcattgaacagttaggattaactgaagacaccgattatacaataactttcaacggtgcactagtggttcataacaatgataaggccgagttggcaaaaagtgggattgagaaggccgatttggtgccgctgcacaattttgtcaaagccgagaatgcaccattagacatcttggacttccagcaggtctatccaatgaccgatttaaagccgtcgatgtaccagcagcagttcaagggaaatattgactttgttccccgggccttttctgatttgagcacgactgatgaatactccaaagccattgtcagtgacaagcctgagttactggatcagtatcagagcgccattgatgacaccttacgcagccaatatcacattgtccggtcacaaccgcagatcatggaatttttggccgccggtatggataaagttgtcggcttgaaggcattgttggcccactttgacatggacttcagcaatttaatggcctttggtgatgctgaaaatgatctgggaatgatcaaaaatgccgagatcggcgtggtcatggaaaacggccaagacccagtcaaacaagcgggggatgtcattaccggcaacaacgacgctgacggggtggctcagtacgttaatcactattttaaataacccgaaccccagctcccggtaaaatgtttaagattgatctgacagtcttttttcgatttttcatttgtattatgataaatgtaattcaaatcaacaatcatgaacgggggaatcgttatgaaacaaagacaaggcatcatgacattaatttttgctgcggtcctttcaatcgggctgctcggcggttttacttcgacagctgacgtgagtgccaagcagaccgtcaaagtggtcaaagttcagaaggttgcgaccaaagcttatcgggcaaccaagggttacatgtataattcacccaagctcaccaagaaaattcataaccttgaatttacactttaagtgcaacactaattaaataaagaatggcccatggccaaatttctgtaaaatgatgtttgcgaaaacaatcatgaaaggaatttaaccatggatcactacaagcatattaccatagatgaacgggaaactatctttttaatgaggaatcatggaaactcacttcgtgagattgccagccatatcaagaaaagttactcaaccatttctcgagaattaagccgtaattctactggtaaatcctattcaccttcgaaggctcaggagaagtacaaacagcgcaaaggcaactgtggcagagtctctctcttgagtaatcctcaggtgtttgaagtggtgagagaacacttctgcgaagacctttggtctccggaggaaatatcgaatcgcttggcagtcgaaaagtatccggtgcagatcagtaccacgactatttaccgtgggattttcaatggcttatttgataatttgtttaaatctggcagctctagtgccgtgcgccatctaaggcatcacggcaagtctcgccacaataaagcttatcaagaaaagcgaggcaagattccaatcccaaacaagattcatgatcgtccgcgagaagctgacaaccgtgtagaaattggtcactgggaaggtgataccgtgttaggcaaaagcggaaaggcttgtgttgttacattggttgatcgaaaatctcgttacctgcttattggtaaagctgctaaaagaacttcagaagcagtcacggatactttgagcgacttaatgaagctatggcctggtagatcgttaacgattaccccggataggggtaaagagtttgccaaagttcaatgtttaactaataagtttggtacgcccttctactttcccgatcctcactctccttggcaacgaggaactaacgaaaatactaacggcttgcttcgcgaatatttgccaaaaggaactgaccttgattcaattactgaccgccggatacaagcatatgcagaacaaatgaataatcgtccccgtaaatgtctcggatggaaaacgccttatgaaatattctttaatgtcgtgttgcacttaatttgacaattcaagacaaaaaattatccgaagacgactttttattctaaaaagcgggtcaccattaagaccaccaacaacaagacggcatactacacttacgttgccaataagagcggcaaaatcaaaggctatgtctactcgaaatacttaaaactgtatcagccaaccaagacgacatcgaccagttcatcgaattctcaatcagataactcgatttccactccccaagtcatttccaaatcgtcattgtcgtccttaattgcggcttctccggacttggatccgactggagagttactgagtctgacctcagctgattataagacctatcaatcggttttcaataagaatttcaatgttggaaactatgccgatgagggtgtctttacagatgatcaggcctcaatttatgtcaaatcaccaaccctgcagccttacgtgcaaaaggcaatcgataaatggaacactgctttaggcaccactgtctttacgcttgggacggcacaaaaccacagcttgacattgggatttggtaacggccaatcagaaggctgggatggtgtctttgacggcgacagtgtccaggtcgattattacgacttccacgatcggacttatccatatggtccgatgccattgccctcatcgcaaaccatccagattaaattgtcgactgatgatacagatgttgacggggccgctgaggggatggcagcaacccgtgtcaaacagtcagctgccactcatcgtgatactagcgctcattatttgaccaccaccgtcagcggtacgccaactgaactgctggaaaattactgggtcggcgtgattacccatgaattgggccatgctctcggtctggatcataccccatacttccaagacatcatggcagctccggccagcaccgaagatggccagagccaagaaaatgccaagtatgattggacgacttacaaagattccgacaacgtccaaggcggcgctttaaccgcgacattgagtcagcgagacattgatcgtgccaagctgactaaactcttgggttactggtaagacgaagttaaacgcatcatcgattagattcatagacacaaacaaaccgcttattcctgtctggggaataggcggtttgtttgtgtaacttataaggcaacttctatttcgaattaatgtttactgaacagtccagtcaagtgtgtcatgaatgcattcaggtaggctggaacatctgcgttgacagccactttaacgttggtgtttggatcatccagtcttgccgggtctccggtcgttcggccgtaatacttctcatcggtggtgacatacatgttcaaatcgatggtttgaacgaaacctgggttaattgccacgccaaccgcaaacggatcgtgaagggcacagccgtgaaggtctgggctggtgacttcataagccttgatgtagtaatcaacgatgtcggcgaaggcttcacctgatttggtgtgaagatcacgccattgctgggtttctttgtaagttaatagggttctgagggtcacgtccaagccaacttgagtcagtggggcctttctaaagacgtgatcagcggcggttgcatcctgttgaatgttagcctcggcgacgttggttacatttccaggaaccgtaacagcgccacccatgatggtaatattgccgatttccttggtaatttccggagccttcttaatggcagcgtcaaggttggtcaatggaccagttggaaccaagatgagatccttaccgtattgcttaacggcgtcaataaagaagtcaatggcatcgcctttttccggttgacgtttggggtcgggcaattgaacatcgccgatgccgttttcaccatgaatctgggcactaaccggcattctgtcgaagtgatcggattcggatgagtgtgacagtccttgataaaccggaacgtccgttgcgcccaagagttccaaaatcttcagtgaattttgaagcccgtcttcaacgtacacattaccgtaggaaccgataataccaattaaatcaacatcgggatcggcgaccgcataggcaattgccattgcgtcatcaataccggtgtccaggtcgagaatcatttttttctgagccattaagaactacctccgtttgtgtattatcaaggatgaaaaccctttacctaatcataaccgaattttattggaaactcaattccgcttcgaacttgaaaccgattaatttgtaagttacgcttaatggtatcaaccttaggagtaaattatgaaaaaaagtgttaaaacaattggtagtcattttttctctttggtgtggaccggtgttcgtcgaaattatgataatttggatgataacatcgccaaacatctgggagagtccgagcccaacagtccggttgagattcatttatcacggatgttttcggaagtctttaaacggcattccagagacgaagccgaccgtttattcatcgtcggcactaaaacaacgactcccagcctgcggaaagtatccagccggccggtcacgccgtggttttttacccgcgtctttttagttctggcagtcagcttcgtcatgctaatggccttactgtttgtcttcaaaagtaacaaggtcattcccggaattatttttatcgggtctttggcagtgccattctcccttttgatgatgttctttgagatcaacgtctatcaaaacatttctgtgcgacaaaccatggtgatctttttagtcggcgggattctgtcgttaattgtgacgatgaccttttatctcatcctgccgattcgaaccgaggttagtattgaatctgctttgattgttgggattgttgaagaactggccaaatgtgtcgtgattattttgttcattaatacctataaagccaactacattttcaatggcgtcctaatcggcgcggccattggtgcagggttctcggttttcgaaagttccggttatgtcagtgaatacggtctggccacaatttttacccggagttttcaagccatcggcacccatgcgatttgggcagcgattatcggtggggccgtgattctcggcaagacgcggaaaaagcaatttaccgtgcgggacttctttacgaaacccaaattttttatattctttctcgtggtcatctgcctgcacacattttgggattgggatatccccaacaccggaattggcgtatcattactgcaggaattaattgatattgcgatcggctggttcctaatctttgtcatgatcgatgccgggttaagagaagtcaagacactgcaggggcaacagattatcattcatcgaagtaaacagaagaagttcgttaataaacgctaggaggatcctgatgacagaagttgattcattttatgacattaccattattggcggcggtccggcggggatgtttgccggtttttacgccggtttgcggaatgccaagacccaaattatcgaaagcttggcagaaatgggtggtcaggtgacggcattgtaccctgaaaagacgatattagacgttggcggctatccaaacatcaaagccagaacattagtcgatgagttggaaaaacagctcagcggctctgatacggccgttaaattaaatcagacggtgatcgatgtccaacagattgacggcggctatcaggtcaccactaatcaagaagtcaccaagacgaaatcaattattattgccaccggggtcggggcctttaatccccgtaagctggcagttgataacagtgaagattttgaaggcaagagcctattttatagtgtcaaacatctggatcagttccgcgaccaaaccgtcttagttgccggcggtggtgactctgccattgatgaggcactgctcctgcacggcgtggccaaaaaagtgtacctgctgcatcgccgtgataagttccgtgccttggagcataacgttgaacgattgatccagtcgaccattgaaccggtgaccccttatctgattaaaggcttaactcaattagataatggtcaagtggaagtcgaagcaaagaaaatgaagaccgaagagatcaagaagctggccgttgacaagattgtcgtcaattacggctttattgctcaagatgatgccttgaacaaatgggaggctcatccggaaatcaaccggggcaccattgaagttcaacccagtggcaaaaccaatttacagaacgtttttgcgattggggatgtttccaagtacgaaggcaaacagccactgatcgccacagcttttggcgaagcgcccattgccgttaattcgattatgaaaagcttgtatccggatcgcagaggtccgattcacagtacatccattagaaaataagacacaaaaagacggttatcctcaattttgcggataaccgtctttttgtgtcttattttctatctaaattatattgtttcaaagcctgaccagtccgagattgtgattcttgttgggaatcttttggcaacccggagaacaaaatccgaccaccataaatcccggcatccggaccgacgtcaatcagccaatcagccttactgatgacttccaggttgtgctcgacgatgatcagggtgttgccggctgccaccagctcatcaaacagtttgatgagcttggcgacatctttcatgtgcaggccggcagttggttcatccagtaagtaaatggttccggtttggttcaattgaactgccagctttaatcgctgcagttcaccaccggacaatgttgtgagcggctggccgagggtgaggtagtccaagccgactttttgcatgttgattagtttgtcataaattttggtcatatctttgaagaagtcaatcgccgattcaattggcatattgaggacttcactgatgttcttgccttgatacaggtagctgagagcctcgttattgtaacgtttgccgtcacacatctcacatttttggacgactgggtccatgaatgccatattggtgatcgtaacgccttttcctttacagcgggggcaggcacctttgccgttataactgaacagactggtggaagccccggaaactttggcaaaaatttttcgaatatcatccaaaatatcgaggtaggtgacaggcgtcgagcggatattcgttccaattgctccctgcgccaagtcgatatacggttcgtggagctttggccgtaaggcatccactaacgaactttttcctgaaccggcaactcccgaaatgaccgtttcaacccccagcgggatgtcgacgctgacgtctttgagattatgggtggtgacatccttaagtgaaatggctgatttaaatggtcttggcttccgatatgtcagcggttgtttcaggtattcaccggtcatcgtgtgcccattgagcagttggtcataagtaccggtaaaggtcacctgaccgccaccacggccagctttggggccaatttccaccacataatccgcaattggcatcagctcggggttgtgctcaacgaccatgattgtgttgcctttgttcttcaaattgatcaaagcattcttaatcagctgaatatcatggggatgcaagccgacgctgggctcatccaaaatgtagaccatatccaccagtgaactggtcaaaaatttggcgattttaatccgttgcgtctcgccaccggaaagcgtttcggtgctgcggtccaaagtcaggtagcccaagccaatatcgatcaacgactgaattttggttgcgacttcacgaatgacgtccgtaaccaatggcacctcgatttcgtgcagaaactttaaggcatgaaccaggtccattgacaaaacgttggcaatatttttgccgttgattttgcaagtgagcacctcaggacgaaggcgagtcccatgacattcaggacaaggccttctggtgacaattttagccaaggcttccttgtgatgctgagcttcctttttgccgataattgatcgacgaattctgggaatcaagccttcgtaaagggcagttcggtgccatgcggccggcgcatccttcagcgtttgttgaggtgcatataacaaagtatccatttcttttttagtgtagtctttcaaaggcttatcattgtcaaataggccgctgtccgtgtaccgccgccagcgccaagtgttgggaccaaagctgacaaaagtgattgccccttggttcagtgacttttccgggtcaattaacgcgttggcatcaatatcatcgacgtagcccaatccctgacatttttggcacattccttggggcaggttaaatgaaaaagtgtctgaatagccgacaaagggttgaccagcccttgaaaacagtaatctcaacaacgagtaaatccccgtgtaggttgaaagagtcgagcgggcatttttaccgatgcgtttttgttcaatcacaatggcaaccggcaggtgctcgatatttttaacgtgcggctgcccgtattttggcagatactgctgggtaaaactgggaaaagtttcgttcaattcccgccttgaggctgcggcaattgtgtcaaacaccaacgaggatttccctgatccagacagaccagcgaagactgtaatggcgtacttgggaatctttaggtcaacgtgctttaagttgttttgataagcatcgtgaacttcaattgcaccatgttcgaacatataaatttaggacctcctatttttttgatgatttttagcagttgggagctttttgggaacggcttctttcttaagttctttttgcagctgattgacctgtctggacagccgggtgacttgtttggttaaatctttcagcgcatcggtttcgtcattgtgtttatcctgagaagtgaaaaagtcggtgatggtggaagttagtaaaccaataaaaccgattccacccagcatcaggacggccgaaatgattttgccgccgtcggtcttgggggtaatgtcaccgtaaccaacggtggtcgcggtcgaaatggcccaccagagtgaattctgcagggaatcatgctcaaaagacgcaaagatcagcgagctgaagatgaggattaccagactgattgataacaggtagataaagccggtgtcatagagaaatttgtgaagggcgttggttaatttgccagagagaccaaatcgccacagcaggttgtaataacggacaatcgaataaatcctggcaatccggaagaagataaagattgggtgcgaggggatcagcgcaatcaagtcaaatagattggagattaggaaatctttttttgacttggcccgtttgaaacgaattaaataatcgatcaggaaaaagagccatatgagtccaaagatcactcggtatggcccttcattgagggtaattttagtcacgagggcaagaactgccaagacaaaggaaaccagtgccaatgaaacgacaaggatattgtaaagcaagattggcatgttcttggtggcttgtttcatctcagatttcccccttagcgactgctgtcgttgttattcgcatctggattggtaatcttgattcggttgctgtcggttgtcttatggtgaatttccggcgcgtcggtgaagtattctttccaagtcgacttgtcaccgttcttggaatagatactggtggacttcttacccaaacgtttctcaatccgcttttctttttgataaaggtcggcgtaattgtaattccgtgggtcaattgccttaaagccctttggatgatagaagcgcaacagattcttttcgttcaacgaatctgacagtgaaagctcagtttgaacccgctccttatccttcttgacttgagcctgttggcgtttggttaatttcaacagttggccggtcttattggagtaaatgccgccactcagtgaagtgaacgccgggctgacccagtcctgatttcgaaaggcaacgacttgatcgtgctgcttggataaaatgtcggtcccaaattggacgtagcgcttgctgctgatgcctaggagatgcatcaaagtcggcaggacgtcaatttctccggcatattttttagaaacaaacccgttcttttggccgggtacatcaataattaacgggacccgctgcagctgggcgttatcaaaatcgtcccagtcgtcaggattcttgcctaatgccttggccaaattggtgttttccgaattggaaatgccgtagtggtcaccataaagcagaatcaacgagtgtttgagcaggccggttttgcgcaggtagttgtagaactcatggacggcttggtccagatagtgggcggtcaagaagtagttgtccaccacgtcatcgccggtattggtggtcttgaaattggtatcttctttatccaaatcgtatgggaaatggttggtgaccgtaatgtatttaacgtagaacggctgttggagattctggaggtatttgaccgaatccctgaataacaatttatcctttaaaccatagcccaacgagcggtcaccggtggtgttgtagtaactggcatcaaagaagtattgataacccatgttcttgtaaacgttgttgcggttccagaaactggcaatgtttccatggaagactgcagaagtgtagccacggcgctgatttaagatggctggagcggcttggaaggtgttgtcgctgccaagttgggcgaacagagatccctgcggcaaaccgtaagtgctggtctccagcatgttttcggcgtcagaagttttcccttggccaacctggtggaagaaattcttgaaagcgtaagaggatttactcttatagagtttgtttaaaaatggggtcacttcttggccgttgattttcttgccaatcaggaattgttggaaactttccaagtgaatcacgatgacgtttttacccttggcaatcccatagaactttttattcggtttggcataatgcttgcgggtgaacttcaagacgtcgtttaattccgatttggtagcggtggcccgtaaatcattgttgtgctgggattttaagccatcgtagactgtaaaggcatccaggccgaggtacttcactatgtaagcccggtcaaaggtccgcgtcagcagctgcggccgatccatttcggccagtgacaggttaacaacgaaaaaaaggaccgaaaacgaggtcactgccagaccaattcggcgattcagcggccgggggtcgattttgattttgcgaagaaccaacagcaaaatgatgaccaccagatcaatccagtaaaagatatcgtggaaattggtcagggcaagtgaactgccgctgagcccttggttgaccttggagtagccggtcattgtgctgacggtcataaaatcggtgaactcacggaagtaaatcacgttaaggtacagcaaaacggtgtttaaaattgaaattaagatcgccagcggataaaagaaccggctttttttgaaataaagggcgatactgagtaacaaagtcgtcgttgccaacgggttaattaagacaatcaggaactgaaagggattggtaattcccagcccgaggtcgacaaaataggccaacatggttttggcccaaaagcaaacaattaataaaatgatgaagcccttgcgagtgctgcatttttccaggacccaattaatatatttcaaaacagtgtgctccttacaataattacttgctttatcttatcaaaaaaacgcgcagaaataaccattgtcaagagattttgcagaaatcttaagttgattggtgtgcgcggattctcaaaaaattgttatactttagatattaagggtaaaggatgtgtcatcatgagtaaatttaatttgtacatggttcgtcacggtcaaacctactttaacatttataacaaacttcaggggtggagcaattcgccactgacggaaaagggcattcaaaacgcggtcgataccggtgagaaattgaaggacaccaagtttgcggctgcatattgcagtgataccaccagggcggagcaaactgctcaaaaaattttagatgaaaatgacgcctcggatattgatgcgccaattacgtcaatgtttttccgtgaggagttttacggctactttgaaggaaatgatatgagccaagcttggtatttggctggcgccccacacggattgccgaccttccgggatattgttgagaaatattccattggcaaagcgaaagattatctaaaagaagccgatccgttccatcaagctgaaaacaatcaggaatactggaaacgtttggatcaggggtttgacctgattaaacagaacccagaaatcaaagacggcgacaacgtcttattaatcagtcatggtaacacattgctaagcgttgtggaacgctatggcaatggtcaatttgatgtgactgagcggccagccaacggcagtttgaccaaattgaccgttgacggcgatgacatccatgtggtggcctttaaccaacaataataacaagttaggcgggtatgaatttggagattaaattaactgatcaattggatcaaatttatcaagacgcaagaaccattcgccatcatgtcttcgttgaggagcagggaattgctgaaaccgacgaatttgacggtactgattccgacgccattcattttgttggctatgtgaatggggaaccggtggtaactgctagaacgaccgtcaccaaaaagggcgttcatattcaacgagtggcaactgaaaaagccgcccggcatcacggttatgcccagcagctcctggaatacctgctgggccaaccaatgtttgaagatgccccaatgttttatttgggggcccagaaaacggcgatcggcttttatcaaacactgggatttgaggagtatggggagccatttgaagaagtcggcatcccgcacgtcaatatgcggcgaacgcactcagccgccgatcaccacgatcgataaaatgatagttggttgtatgtaaatattaacagagagatccaagcggaattcaggtaccgcttgggtctctttttgctttgcggtccgtgatcactcaaggccatgacattaaagtgacattttacttgacaaaattggcagataaaacagaataagagtgattaaatgaacgattccaggggggattggcatggatcaattaatggcccgttcaatgaaagcttatcagagcaagtttgcccgtgtgattcaggatactttggcgctgctgtttccaattatgttactgggaagttttgccgaggtcttgaaatattcttttttgacgcccagtgggtttgttgccaccgtattcggggtgaccaagtggctgcccgctgcgaggcagatttcacagctattggggctgattgtccactgtacggttgacatgattgccttatacggcgcttacgggattgcctactgtacggtaaaagcatacgggcgccaaacatcggcgttgtcaggtgctatcggcctgctggcgttcttgatggctgcctatcagccccatagccacgggcgattgctgtttaacagcactttgatggggcagggactgttaattgccttgataattggctatatcgttgggcggatcattgttgcctttgagaaacgccgggcgttacgatcctaccaaatcatttggcccttgctgctggtggttgtgttttcaattgtggtcaatgttgttgtcagcctcaccagaagtccggaggttcaatcgttcatctcgtcaactgccttgcatgcggttcaggccagcgcgctttcctatgtcatcggcatgggattgttgacggatctgctgtcttggatggcggttggcggaccgttttctgcaagtccgacctttaccgatccagcagcgttgaccaatttgaatcacgctctcaaaacagggtcagccttcaatgtgccattcaaatataccgatgtgaccctctttcacagctttgccaattttggcggcaatggcgcggtactggcgatgattattgcaattttagtcttctccaaacgacagcgttttttgactgtctcgaagtggtcaatttttccggcgctgtttaataataattatgcgatgatgttggggatcccaatcgtttacaacccgatttttctgattccgtttctgctggcaccactggttaacatgctggttgctgcttcttttctggcgctcaaatggattccggcagccgtttatccggtaccttcagggacgccggggcctttgattggtttcttgggcaccaatggcaattggttggcgctcattctcggagcggttctgattttcgtggatgtgctgatctatatgccatttgtcaaactgtatgatcggcttgatcgaaaccggggtgagcaatgatgaaacggacagttaaaatctggttatggagtcttcttgcggtgttgctgtcagttggcttgattgtcgcttcactctagtggtcacaccaaaatgtcagtgagttaacccggtaccataactctcagttatcgccagtcatcatgattccggggagttcggccaccgaaaaccgttttgatggtttagtcagtgagatcaaccacaaccgcacgaatccgcatagtttattgaaggtcaaaattaccaacgatgacaaactccacttcaccggccggctgagaccgggggacaacgagccattcattgtggttggctttcaaaataacaaggacggttatagtaacatcaagcaacaggcccgccaatttaacgtcattttccataccttggtcagtcgattgaattttaataattttaaagcgttaggacattctaatggtggcttaatttacaccgtatttttggaaaattattttgatcaatattctaatgacgtttggatgactaagttgatgacgattgggtcgccgtttaatttcaatgagcggtcaattgataacaagacgcaaatgttatcggatttcatcaagaatcgcaacaagctgcccaataatttgagcgtctactcagttgccggcactaagaactacacgtctgatggattagtgccgctggtaagtgttgctgccggccggtatgtctttcaaggcgccgttcgtcattttacaacgatcacagtgtctggttccaacgcccagcactctgatttaccggaaaacaagcagattgttgatttgattaaccgatacattctccactcgacccgggttccaagagcaaggcaaaatgaaccgcgactacattaaccgtcgtcgaaaatgtctgttaagccacgaccagctttggtgaatcgtaatcgctgaggcaaatgacagtagccaagttccaatgtagacggagaaaatgcctaaaactggttggcgactcatcaacccttggccaaatgttcgccaaagcagttgattccaaaagacgttggacaaaaaggctggataggcaaagttggccaagcggtgaatcagatgagtgacctggagtttccgtctaagctgggagtcgcctaaagcagcaatcaaactaatgatgctgaggtcataaatggtcatcgatggtttgtagtatggggcgttagtcagttgaacggggaacttgaaggcaaataattcacagttaatccaaacgaacgatcccagagcaaaaacggttatcaacccgtgtttttggagccagcgatgggccacttggcgatactgccaagccagagtcccgacaactgcatataataagaaactgacaaatagtctgtccagcaggtaccaatccttggcgtgcgggccgtgaaagacttgggtgtcatagaagattaaccagaccaactggaccaccgaagtcagcagcagaaccagccggccacgctgttgattatggccacaccagctggccagccaccagaaaggcggcatcagaatgatgaattgcaacatcatcgaattgtaccaaaggtggggtgcagcattcccgttgatgaattgccaggcaaagtcgccaatcgtgtgataatgctcgacttgctggacatttggcatgattaataagtagatcagggtccaagcaatggtggggatgaatgacgcatgccacatttgctggagatagcccgggtagcttaaatcggtgtcgtgagtgactcgcatggtcgtatacaggattccggtaatgaacgctggtgccgtgaatttgatgaggttgtaacaaatgccaatgccgatctggatattgacagtcggatgagtttgcagggcttgacctagaatgatttgcagcatgacggccgcgcaggcaaataccttgaggtaatcgcccatgtctggggtactgggagatttgattttgcgatccatatctgtagctcctttgaagaattgtctactaccaatataccaagtgaagccgaaattacaaaaagaggctggaaacaaatgaatgtttggttcttcgtcaactgttgttggtgaacaaaatattggagttctaatcacttggtgattagggctctttttgtatgaactcgaaaagcgaacagcactcttagccggaatctgaagaagtttcggtaaccaaatccagtgcgcttaatgactttaatcttgttgtttgaaccttctaatggcccgttggtgtagtggtgggtgaaagtgttgccaatttcatcatgatgagccgccaaggtttggagggctgccaacatctcttccgagcacccctgcaggtggtgaaaggcttgattatagttgggccagtcgcggtttttgatggtttcacgtaaccgattcatcacgtcgtaagtttgcttgagctcgggatcaatgtccagtaaagcatcaaccacatccgtggcagttgccggataagggaagtttgtccacttacggaaagcctcgtagttaaggtgattggccggcgttaataatagtttccaatagcgtttcaaggcgtgatactggcgtgaggaagtggccagggttttcatgagacgcactcgcgtcttattaaaagcccggtttaaagcgttaaccaggtggaagggatcgatgacaacgatggcgttcgggaagatctgcccaaccaatttgggataggtatagttcatatcggtgacgataattttcacattttctcgcgcggcttggtcataatgttggaagtacttttgaagctgatagatggttctaaagggcaacaggtcaatcaattcgtgggtttccgcgtccataaattcaaagctcatcgcgtcggtggcgctcttagtacttttaacttcgtccatgaggagaactttgggtaagtagtgccagttggtttgaaagtcgtgttcagcgcgcaagagctgccgaccaacgaatgaatccgaagtggacaattcattggcaatgtgtttgaggctcactggttccgttaacttctctaaacattgtttccgggttgtatttgaaatcgtgcagtgcttcggcactgcactcgtctgcgccaggaagttggtatgacaagccttacagtgaaagtttcgccgattgaggcataggataaccgtgctgcccaatgttttagcgaatctaatggtggtcttccgccaaccatagccaatgatctggtgatcattaataaccccacaattgcggcaggccttgggagaatagttcagtgatccatttaatctgattaccccatcatcacctattttgccattctcaatttttaagtgttcatcatctattcctaacaacattttcgtagtatcatttgacatagggcatttccttctttctctaaaatcttcgtggttgttggttttgatgaacggacaggaaatgtccgctttttttattctaatgaaaaacaaaaaatctgtcatcagtaatagataaaaatctattaccaacaacagatattgtagagccgaatgtttccagcctcttcaggtgatagttgattgaattgttgttatgttgctatgtgttaaaaagattaatcgtcggtagcgtcatctgagtcaaagttaacgacgtgagcggaaccaacgtaattccaccatggtgctttaacagtttcggtgatgacaccgcggttttgagcatcgatcatcttaccgttgccgatgtataaaccaacgtgagaaattgatgctgcgctccaaccgaagaataccaaatcacctttttgcaggttcttgtatgataccttctggccggcgttgtattgtgcttgggcagtacgaggaagggtgacactcgcagcctttttgtaaacgtaactggtaaagcctgagcaatcaaatgctgaaggaccagtggcaccataaacatatggcttgccgaggttttgcttagcaactttataaacggctgaatatgaaacatcagtgtcggcagctttggatgcttgagcatcttggaaaccggcaaatgataatgtgaagaatgctactagcgtaagtaatatttttgtatgtaatttcattttttatcaacaactccctatcaaatctacagtgataacaataccaatgaattgttgcaaaagtgtaacaaacaatttgcaatgcagttaaatgtcatatggcagttgaaacattggtaacctggcttgtgaataaccgtttccacaagctgatttgagggtgtttataactgagcaattaaaaaagccgcctaatgtgaattgagtgacttttttgaaaaatgtcgccatgatttggattaaatttgtctgaagatgacgtggcaaaaatagaaatcttaataaattatttatttattcttcaaaagattgtctttattgggcaaggttacggccaatttccccatcgaagtgacaatcattggcaagatcaggtagtagacgcagaccgtgtaaatgacgatcaatgccgtttcaatcattgcaaacgatgcaccaaatgtgaggccaattgccaaggcaatcacgactagcagaatgtagcggacaatcttgccgtaactggccatggttggccgaatccattccagcagtgacaattccgtgtatctgaatgacaagcccaacgcaatgatctgccaggcggcaatcgcggtcaggatgctgattgcaagaattggcacctgccagtcaaattgattggtgcccgtgacataatgcatggtcagataggttaattgaaagccggtgatcgcagacattacgaatgcaacggtccaatacagcggttggagaatcgaacgactgacaacgaagacagtcaccaaaatcccgataatcactattgccaataaagtaatgaaatgatgattgagtttggactggttaatggattgtgtaatcggctcgccagtgaaggcaacctcatctgacgacagcggagttccccgcagctgcaagccaacttgagcttcgagcatcttaacctgcttaaggttggttttgctggatggggcgttgttcatgacaacttgaatggtggtaatcttcttgtcctggctggtgtagttaagcatcgtctgcaagaagtcggtgtccgccagctgcgctttggtaatgtaatagacattggccgcaccggacttttggagaccattcaaataatcatagatgttgtttaactgatcagtcgaggaattaacctgggaactgacctgttttagttgcttctggacttggctaatttgttgactgtaactctcaagattattggcgctgttttgaccgtaattttgaatgaccgatccctccgcgttcagttggctgatgcctgacgaaacactttgtaaggactgattcaattcgttaatcttctgctgatacatgtggactctgcgtgaggcgccccgctggacggcgacactggagttggcagcaacactgttaacctgtgaggctaagctggagctgtcttccacaatttgattactctttttaaccaggctctgcatgtccttgacctgttgcttgaggccggacaaattcaggttgctgccgctggtttcgatgccattggaggcctgtgaaagttgtccggttgcctgcttggcgtttaacccgatggactcaagttgattggaaacgtaatacttttcgatcggcatcccacttggctgcgttaatgaataagcggcactaacccctttggtatgctgaagtttagtggttagttggtccaaatgctgcaggtatttttcgttatccaagggctgatcgtttttaaggtaaatcgtgatcggcgtggctttaccctgtgaaaaatgtgcctggagaacgtgggcccctttaacggcttgattagtctgcgttaagttggtcattggagaaaagttcaggctggtatggtagaagtaaatgaacggtagggtcagatatagaacgaccagaaaggcggcaatcggctgccagagtgaaaaatcggttgcccggttccagaagtgggacttcatcgcactcaatggggcactggacggccagaaaatactttcccctaaagcggccaggaaaacagcgttcagggtcaagacggccagcattaagacaacgtaggtgatgccaagaacccacagtgattgtaattggtcatagttaatgaagccacagcaggcgaagatgatggccaacgcactgccgacaatggtgattggaaagcgtaggtcggcaattgtctgctgggtggcgtaacgcgcttctcgttggagtgccagcacgcttctgagtttgcggtagatgtagatgttccaaatggtgccgatcaccacggtggcaattccgatttcaagtggcgtgtattgagtgaaggcaaagtgaaaatgtttggccaatgccgttgagatactaaatgaagtcgtaaatgccgcaaataatgtaatgaaagaaatgaccggtgcaaataacgaccggaagtaaattcccacaatcagcattgaaaccacaaataatgtgatcaaaatgatgttggtaacttgcgcggttttttcattattgacgtcgcggacaatttccggactggtgacgtaggactttaatccagacacctggacttcaccaaccaattcattggtcaaaacgcgcagggtactgcttttggcatcgatatccaagctggcaatttgggtggaaccatctttagacaacaactgctgtttgccggccacgttggtgttgatggtaacgatcttcttgatactgtaaaatgattgatgggctttgagtttattcaaggcattgtcaatcttcgtctgctgcttagcggtgatcttgccgtttgggttcgtgtagaccacgttaatggtagacgcttttcccagattgtacccccaatcatttcgcagctgctgagcttgcgccggttgtgagtctttggaaaaggtgggctggctgtatgactgcagtgtatcggtcacgtttggagcggttataattgcaataaatgtaataatcagccatactaacagcgtgaataagcgatttttgtgtaattttgcgatagtttccttcattgattcgtcccctaaatatgtatgtatgaaaaaggctcatatattaagagtttaccattttataaaggctagtgcgatacgttttgggcgttttgtgttatattgggaaaattgttgtgaaatttagtcgaccatttttgatgggaggttcttaacgtgtgtacaagtatttttcaaattggccatgaagacggcgcccatgtgttgtcacggacgatggactggccgcagctgggagctcatcccgtctttgtgccccgcaactacggttggcactcggtatatgacgacaaacgttacgtcactaaatatgcgacgcttgggtccggccaccagcacgccaaacgaattgatatgtctgacggggttaatgaatttggcctggcggttcaaaaattgacctttaccaacggcagccagctagtcgaaacgccgggtgagaacaaaatccatctggcaccgtttgagctgtcgttctttttgctgtccaattatcgatcagttaaagacatcgaggaccatattgaagaaattgaactgatggctgacaagtacagcttaatgaagtatggccacagtgaattgcactttgctgcctgcgatccaaccgggcgaattgtcgtcatcgaaccggtcaccaccccaattgaaatcattgaaaatcccttgggagtcttgaccaacagcaaccatttcgatcggcaaattgacaaattaaacaagtatttggattttaccccggattttgtcaacggaaccgtccctctcaacacaccgcgggtgacgaccggcaacgtgtccggcaagtcaattccgcccggctcatattcaccaggatcgcgatttattcgggcagcatacctgaaggaaagaattgacatcccccaaaatgaaaatgaggccgtggataattgctggcacctgttggactcagtgaatgttcccaaaagtaaggagcaccagccgacttattccgtctaccgggcagccgtctgctgtgagagccgaaattactactatcagccatatcacgctaaatcagttgccaaaattcagttgacggatgacctgatcaaatcgaatgaagtaaagttttttaaagtagctgaccaaatcaccttcaatgagttaaactaatgtattgaggatatgagcggggagaaatcaagttgcgaaaacaaagttggcgggttattgtcatattattagtgacgtttgcggtgttgatcgcgggcgttttcctgcgtgggcagttaagtcaccatgcacagcgaaattccgtgccaactttggttcaaaaaaggcctgatcatttctcgactcgccaaaaacgaagctttatcaaccgcgttggcacgccggccgtcaagctgtacttgaagaatcggcaagtgttaccgagcgtcgtgatcgctcaagccattttggaatctcagtttggcacttctgaactgacaaccaccgccaataatttatttggcatcaaggggacttaccacggtcagtcggtccagttctatacccgagaggtcgagaacggtaaatcaatcaaagtcctggctcagttcagaaagtatccgaatttggcggcctcaattgccgatcacaatcaactggtcagcgagaagtttatcaaagctaaaaatattttgagttatcgaaagtcgacgcgcttgctgcaggccaatgggtacgcaaccgatcctcattatgccgccaaattaaaccgcctaattgtcaaatatcagctgagccgttatgatttaaaagcaattaatgaacgtgtatgactagcgattacattgttgaccacgtttaaatgaaaatttgttgaggtgaatgccacattgttgaattgggtttctaatttatatggtccattttttgatcctcataattgggaaacggtgattaccagcggaagtgactggctgattattctgtcgctagtcacgattgagtgtttgttgtcggtcgataatgcggtggttctcgctgcccagacacaggcgctgccgactaaagttcagcgggaaaagtccctgttctatggcttatggggcgcctacctgttccgtttcctgatcattggggtggggacttacctgattcatttttgggaaattaaggttatcggctcgctgtacctgttttatctggtttaccaatttttccgaaaaaccaagattgttcgaactaagaaactggctggcagcaaacgccacggcatttcactattctggtcggtggtcgcccaaatcgagtttatggatgtggtcttttcaatcgactcggttctggcttcgttggcgatttcgtccaacccggtgattgtcctgcttggtgggatgatcggaattctggccatgcggggcgtcgctgaagtcatcatgaagttgatggggattatccctgagcttcagccgatggcctacgtgttaattgccattattgccttgaaattattcctgtcgattccggcaattgacattgaaattccagcgacggcttttggcgggatcgtgatagcagcggttatcattactttgattattcactatgtaagaaaaaagcggaggattaacgatgagcacggaaataacgccgaataatttagcggccgaaaccaacaatccactcaccgtgatcgatttctgggcgccttggtgcggtccctgcaagattttggaccccattttggctgacttggaagctgactacggtgatcaaattcactttggcaggatgaatgtcgacggcaaccaggaaattgctgagaagtaccatgtcttaagcgttcccagcctggtcattttcaaaaatggcaaagctgctgaaaaggtgagtggcatttaccccaaagataaattaagaaaatatttcgatcaaaaaatatcagaagttcaatcaatttgacgggcagtctaccgaaatggtttgatgcccttttgttttgccatgggcgtcaacttggcatttaggatgtccaagccttgaagcggaaagttaaatatcggcgcgataatggctcgtttggcaggatcgggaaccacttggctttctttgagattgggcagcattttcgccaagtcggtttgggtgagatgaagtgccttgctgtaatacatgactcgctgaaagaccaggtttttgaaccacaggtagtagatgattccagcggcggcaatataccaaaagattgtccaagtgatgccaattttggctggggacaggatattggtgaagaaagccaagataataaaggcacaatatgttaaaatgctaattatggttagtttagattttgttgacatgattgaccaactttcataacgaaatttgtgataccatttagatataattatagacaagttggaaaaatatagatagtgagatgaaattgtgaaattttcagtagagacaattgatcgcaaagattatgcggctgtacgaggtattatcgcagatagttatcaaaatgacgggcccaacacagatggtgacgaggttgacatggttgatcgtctgcgcgacagtgaatcctatcatgatcaatttgaagtggtggccaaagatcacgatcatcgagtggttggccatgcattgatggtcccggccgaagttcgttctgcgacaggcaaatttccaattgtttccattgttgagattggtgttttacacggctatcgaaacgacgggattggtcaggaaatggtcatcgaattagaaactcgggcccgcttagccggctatcatgcggtcagcgcaatcgatcattctgatttcttctttaaaaacaactatgtgcctgctgataatttcaatatcctgccaacggtggcggttgatttcaatgataatttgatcaagccattgttcgacggggccctatatcaaaagggcggcaagatttactatcccgaagaattctttgggattcgcagcaccaactattaatttaatcattcaatgccacatgaagtagttcattcatctgagggtcagaaagccggtgggagatgcgaatcggtcaggatggattaacgaaataccgtggcggagtttaacggataataactagagccgatatcatctagtgagtgagctgtacatgtgcagctaaactgggtggtaccacgctgaagcgtcccttagtctatttttggattgagggacgctttttatatggaggagtatgtgtaatggaaaatgatgttaaagaaccaacgattagtttaaccgagggcattgtcgttctaatgatgatgctattgattatgggcttcagtgtgatcaagctgcaaatttcaccgcaaattccaattttgtttgtgattctgctgttgattgcctgggctaaagttcgccgcttttcttgggactctgtcaatcagggcatcatcaacgggatttcaaccgggattattccgatgtttatttttattttgatcggggctttgattagctcatggatcgctgccggggtgattccatcactgatggtctatggttttcatttgattagtgccgagtggttcctgccatcggtctttctggtttgtacgattgttggtaccgccattgggagtgcctttacggttgtctcgaccatcgggatcgcctttcttgggatggggctcaccatgggcattaatccggccatgattgccggggcggtcatttccggggcaatctttggcgataagacctcgccgttgtcggattcaaccaacttggctgctgcggtagtgggtgctgatttattcagtcacattcgcaatctgatgtggtcaacgattccggcgttcttcacatcattgattgtcttctttttgattggccgcaccaatgcgcaactcaataccgcttcaattgaccgaacgatcaacgttttgaccgagcatttcagcatttccttgtgggcatttgttcctattgtgttgatgttcttatgtgcttggcgaaaaattccggccattccaacactgtttatcaatattttggtagcggtcgggatgctgtacgttgaggaacccaagaccaagattcaagcagtcgtcaacacgttgaccaatggctatgtgtcccatactggcaataaaaatgtcgatcaattattgactcgtggcggaattgccagcatgatggcgaccattgccttgatcatttcagccctggccctgggtggtttgttgatgaaattcggtgtgattgatgctgtgatggggccattatcacggaagctgcagtcaaatggctcgctcattttggccgttatcctcagtggcattggtgtcaatgtctttgttggggaacagtatttatcggtcattttacctgggaatgcctttaaatcaacttttgataaagcaaaattagcgccggttgccctgagtcgggctcttgaagatggcggcacggtgattaattacttgattccatggggcgtggcaggtgtttttgccgccaatacgcttcaagtttccacgatttcttacctgccatttgcgatatttagtctttcttcaccaattttttcgatcatcagcggtttcaccggcatcggtttgaaacatttgaaaatgcatgaaaacggttagcattgctactttaacaacgttttacctaaatactggtcattcttaatttaacaaacattactcactcgttacattagttacgcggagacggtttttcttaatacgcgtgatattggatggtaacttcgtaactatacactatgtattgttgatcgacgaggtcaacaaaaattctagacacagaacacagatataggagtgtgtaattttgaaaaaagtattatctatgatcttcgctacttcagccgcagctattggtttattcttcgcaggatccgcatatgcttcagcaagcacagtagttacagttaagtcaggcgacaccgtttggggaatctcacaacaatataattcctcagtaaaggctatcgagagcgcaaacaaccttcaggatgcaaacgtcattcaagttggtcagcaattaacaattccttcagctgacaccgcatcaaatactcaaggtagtgcacatgcagcaaccgcaacgactcaacagactcagagttacagccaaccagctcaaactcaaaccaaccaagcacagactagccaagcatcaacttcaactagcactgctaccagcggttcagttgctgaacaagcagctcaattgatggaacaaaagactggtgtttcagcatcaacttggatggccatcagttaccgtgaatcaagaaacaacccaacagcacaaaacccaagctcaactgctcacggtttgtaccaatcactttacacaacaagtaatgactggcgcgaacaagtaaacgacgcagcacggatttaccattcacaaggaatgggtgcttgggcattaaattaagagcgtgaagagccccgggttgatcccggaacacaagggaaggcggccaatgatgaacttgttcatcgttggtcgtcttttcttgtgcagtagggatcaggaggtcggagcgcattttccactaggtagcagtggtgctgtcggagcgcattttccactaggtagcagtggtgctgtcggagcgtattttaaccaggtggcagcggtacaaggtcaaagatgccaattaccaaataaaaaatatccgcctcactgcggatatctttcctacataaaaattcaattatccccgtaccaacaactcgatttgacctttttgaggcgcgaaattaattccgacaagtggttcgcgcaaaatctttccatactcatccaaaacatcggatggcagtggggtgtgggccttgagggacgcaaccacatcaccggcatcgtgagcttcagataagtcgatgaataaattgactttgttgaccacgtcacggaacaggtcggttaaaatcccgttaggtttcccctcaacatcggtgataacgacctgcgaagaatcgaatgctaaatggttaaagcgcaccatttgtaaaacgtcaaacagcttatccattgacaacaagtcccttcatgatgattcatttaatattaagtgtagccgtttgcatattcaaaaggcaagtattatatcgttctgttgataaattcgatctaaaaaggtgccgtgacgcagccattcagctgtatcacggcacattattaccatctaaacggtgttagtcaccattcatgattgaatttttaacgatcacgtaatcaactttggtaatatcattcaacttgcggccaccggcatatgaaatcgacgactgcagatcttgttgcatttcgttcaaagtatctgagatgtgaccacggtaaggaaccaacatttgtcggccttcaacgttgcggtaggcacccttttgacgctcggatgctgacccccagtattgcttgtatttcttgccatcaatactgatcaggttaccaggagtttcttcatgaccggcaaataatgaaccgatcatcaccattgaagcaccaaaccgcacagacttggcgatatcgccattgtaacgaataccaccgtcggcgatcattggcttccgagctgctttggagcacaaacgcagtgcagctaactgccagccgccggtaccaaacccggtcttgagcttggtgatacatgctttaccaggtcccacaccaattttggtagcgtcagcgccggcattttcaatttcgcggacagcttcaggtgttcccaagtttccggcaatcaagaaactgtctggtaattgttccttgatgtaatgaatcatctggataacatagtctgaatgaccatgagcaacgtcaatcgtgatatattcaggcttctcgttgtcggcaaccaacttgtcgatgaattcatattcttctggcttgattccaacactgatagaagcataaagatcctttgaatgcatcattttgatgaaaccttcacgcttttcaggttgaaatctatgcatgatgtagaagtaaccgttttgtgccagccaaacggccaggtcatcatcgataacggtttccatattggcaggaacaacggggatcttaaatgtcttaggtccgaattttactgaagtgtcagcttcactccgactcttaataatgttcttgttagggatgagttgaatatcttcgtaatcaaatacttccatgatttacctccgaggttttaggacagctccgtcaggtagacagtttataagcgcctgactcttcttgcgactttaggacagctccgcaaagcagaagtctgcgcctaagcacctctaacaaaattccaagacccggaattctgttagaggagacttaggcactgacttctaagcgctttgctccgctcactgttttaggacagctcctccaagcagaagtctgcacctaagcacctctaacaaaattccaaggcccggaattccgttagaggaacttaggctccgacttctaaccgcttggatccgctcactgttttttaccaaactttttccacgacgttcgtctgttctctgtcaggaccgactgagaaggttgcgtaagggactccgactgctttttggacatggtttaaataattttgagcgttggttggtagttcatcaaatgtcttgcacttggtaatgtcttcgtcccatcccggcaattcgtcgtaaacaggcttgcaggcatcgagttcttttaaggttgcgggataatggtcaatcttcttgccgtttaattcataagcaacgcagattttcaaagttttaataccggttaggatatccaaacagttcagtgccaaatgggtgtagccgctgacacgcgccgagtggcgtaaaaccacactgtcgaaccagccgattcggcgtgggcgcttggttacaacgccatattcatggccgacttcccggatatgatcaccgatttcatcgtggagttcggttgggaagggaccctcgccgacacgtgaagtataggctttgcagacaccgatcacgtggtcgatccgattagggccaaccccggttccaacggcggcaccaccagcacttgggttcgatgaagtgacaaacggataagttccgtggtcaacatcaagcatgaccccttgagcgccttcaaataaaacatttttgtgatcgtccagcgcgttgttaataatataggaagcatcaacaacgtatgggcggatgcgatcggcgtattcgttatattcattgaagatcggttcaaattctaatggttcatggtcatagattttagtgagtaattcgttcttaacttgtagattgcttcgaagcttttcttcaaagatatccttatcaagtaaatcggcaattcggatgccaattctctcgtatttgtccatgtaagcagggccgattcctttgttggttgtcccaatcttagaatccttcttttgctcctggagaccatcgaagagaatgtggtatggcatgataacttgagcacggttggaaattctcaaattatcagtactgattccatcctttttcaaattgtccatttcgttgatcagggatttggggttaacgacaacaccgttaccaattacactgtacttttcctgatcaaaaatacctgatggaatcagttgtaaatgatagctgttgccgttaaatacaatggtgtggccggcattgtcgccgccttgatagcgggcaataatatcagcactttggccgaagaaatcggtaatcttacctttcccttcgtcgccccattgacttccaacaatcacaatagatgacatatgaacacctctaaattttattgccaggaatctacccagcatttttaataataccaacttgtattccattaatcaaccaaaaggttaataatttttacaagtaaaacgtttaatattcgactttgaaaccgaatacgaacgaaaggtaattattattctcataatatagtcaaaaagtgaacaatatggtattattatcctgtcattatttagtagaaaggactcgttatgatagatagatactctttacctgaaatgagcaacatttggtcactgcaaaaccaatacgcttcatggctcaaagttgaaattgccattgatgaagcatggtccaagctggggaagatccccgctgaggacgttgagaagattaagaagaacgccaagtttgacgttgatggcatcgccgaaatcgaggcggtgacccatcacgatatcgtggcatttacccgcgacgtctccaaatcacttggcccagagaaaaaatggatccattatggggttaccagtaccgatgtcgttgatactgcctggggtgttcgaatcaagcaggccaacgaaattattcgaaaagatattgatgcatttattgatgtgattgccaaacaagctaaaaaatacaaggatactgtcatgattggccgaacccacggtgttcaagctgaaccaaccacctttgggttaaagctggcgcgttggtattctgaaatgaaccgtaacaagcgtcggtttgcgactgcttctaaggaactggaggctggccaaatttccggtgctgtgggaacctttgccaatgtgccgccgtttgttgaacagtatgtgtgtgactcacttggtttacgtgcccaggaaattaccagtcaaattctcccgcgtgatctgcacgccgattatatttcaaccttggcactgattgccaccagcttggaagaatttgccactgaaattcgtggactgcagcgttccgagattcatgaagttgaagaacatttcgatgccggccaaaagggctcttctgcgatgccgcataagaagaatccaattggatccgaaaatatttgtggcttggcacgggttgttcgcggccacatggtaactgcttatgaagatgttgccttatggcatgaacgagatatctcacattcatcagctgaacggatcattattcctgacaccttgacactgttggattacatgctgcaccgcttcaccaggatcctggatcgactaaccgttttcccagaacggatgaagagcaacatgggcctgacctacggcttgatttacagccagcgggtgatgttgaagttaatcgatgccggaatgactcgtgaacaggcatacgacttggttcaaccattgactaaacaatcatgggataagggcattcagttccgtgacttggttgaaggcgataagaagatcactgatgctttgagtgaagatcaaatcaacgatgcttttgattaccattaccacattcgccatgttggtgaaatctttgcccgagttggcttggaataaccaacggacggtgaattttaaattgaattaacctgaaatcgattagtactaactgacgagggattggacaagacgatctgttttgtccaagccctcgtttagttttttcgcttttacctagcggaattgtgaaaaaataagcagcttccggccatacaagggggattaacccaatgtccaaatcctggatattgggttaatcccccttgtactctggaagctaagcgcttattttttcacactgacatttatggcagaaataccaatcgattatcgccataatcattccatttttcagcaatctggctgagtgggaaggtagtcaacggtactgcaatcttgccatcggtaatcatcttcaataaagccggcatatcatccgccaagttggctgcggtgaacgagccgaagccactgccgattaaatggaagtcaatacttcgaaacaagctgcctttcagcggtgagctctggccggccatggagccgatttgaacccaggttaaagtgtgttgcggatcttggccaagtcagcttttagttgatcatcgttatcagttaatttgatggttgaggtgacaccaaattggctcaattttgctagtttttctggattgcggccgacgccgattacttcggtcgcaccaaaactaatgctgatggggatagcaagttggcctgaagcgccggttgcgcccagcactaagactcgcttgccgcggatcttgtcttcgcccaagcgttccttgatcgccataaacgacgacattgccgggttagctgtagcggcgacaaccgccggatcagcggtattatcgattgggaacagtgcccgtcggttgacgactgctttttcggccaaagtcccataaacgttattgctgctgttgaagtagacgtgttcaccgtcggccgtttcaccaacggcatctacgccggggacgatcggtagggtgctggctgcggaatagtgagtgccgtttgccctggcgcgggcgagttggctgactgcggccgccaagatgtggacctcaacttcaccatcttcgactttgggattggggaaatcgccgtactccggaccacgggtaaaatcattaataattgctgctttcatgtgaatgctccttaattgtcatttaaatggaatcattgaaagtgtgctttcaatatggcctttatgatgattgatgacggttggttttgcaacgatattgacttttgaattggtgggatgtcgatttggcagacgttcgagttatcaaaacgcctctcgttccactctcaactatatttcgccatggcggccagtatccaaaaagcgcaccgtgtcgccgacaatttcataaattaataaccaactgcccttgatgaacaaggctcgttgaggctttctgctcttaatgacgtgatcatcatacttttcagcgactggttgaccactcaaaatctgctcttctactgttctgaaatcagcctcagtgtatcggttggcacgaatcatgttttgataatgtttcttgaatctggactggtacttgggttgatatttgcgcattaattgactccctctcgaatgatgatagctttcattatagcttttttgactggatctgaggacagaaaaaaggcccggcgggggagccggacctttcagttcaatattctgaggggaatatgaatatgataatctggacaacaaatcaatggggggattgatttgctgctcaatgttattggggggtgagtagaaataaatctcgtttatctcttgctcatggttataatatacatgataaatataaaaaaagttggacgaaagtgtgaactttttgtgaattttagcaaacttattttggcgggtaaaaaaggctgcggcgaaagattgtgaccttcgcgacagtccattttatacctaatctttttttgagggggagataaggtttaaatcaaattgattttatcatttctgacaaatatgaggtgaagagaagccttaacttctattcaaaataagcatacaggaaaagttaggctaaagtatgaattaattgtgaagattttgtgaactttttcaatcgattggatagtgggcacaaaaaaagataagacacggggatgccttacctcaagttacctatattctaggggaagaatatgaatacaaaagtaataaattaaagggggatttaatttattgccacataaaatgacgtatcactttatgtttatatctacactatatagaatgaatatgaccaaagtttgaaaaaagtgtgaagattttgtgaacttttgcgaatttcaccacaatttgtccgataaatttataaaagattaaaattgaccgtaagaaacagcgagatgaggaggatttcaaatgagctttatggctaaacggtttatcaagaaatttagggctgaaaactacaaaaaaagcgtcgcccacagcttcttgaagcctaatcagaagatcaatatttttcgtcaaagtgctgatcagtacaaaattcgtccggtcaaaaatggccagttggtcacaattcaaccaattcaaaaccccaccagccagattctctatttccatggtggggcatttacagtgccgatgaatgaagaccaactggaaatgattaccaagattgccacagaatcaaataatctgatccaagtggctgattttccactgttgcctaaacacagtgcagacgaaatcttacaatttacccaggcagcatttgacttggtgattgagtcggaactgccgacattcattgttgccgattcggctggggcaaagattgctttgcagctgctggtggataatccaggaaaagcagctggcagcagtttcatctcgccgtggttggacaccaagttgaccagcccagcgattgccgagcgggctgatgaggacatcttattggatctaccaacattgcaggagattggccgttggtttgaccaaggggccacgcctgaaaaatgggtcgattataccgatgcggatcgattaaaaggagtcggcccagttcaaatcttctatggtgaaaatgagatgctggttccctgcgatcttcagttcattgaggcattacagaatgccgagggagccgatccagaagtcattgcctttaaggatgggtatcatgactacaccctttggttcaaattgtccgaaacaaaaaagacctttagacgaattgctgaattcattaaagatcaacgtggtgcttaagcttggggaaggcatgggtgtcggaccatttcatcattgtgccttggaacagtaaggcaaagatggttccaaaaccaattgcataaagtttcccggtaaataaataggatgccgagatgatgacgaccggtggaatgtagctcagccactgggataacacggcactgccatgaatgtatttgaaacggatgatgtatgccaagtcgtcgttgggatgcataatcaagttggcccgggcgtacatcgaaactgccattgccacgcaatacaggccgatgatatccaaaatgaggcggacgtagaagtccattgccgggactcctagtgaattaaagatgaatgtgaacagcgctaccaggtaactgaacggcacggtgtaaagcaggttggagaaaaaccggcggcggtcaaaggaccccagtagtaactgattgctcaaagtaacaatgatgccgtagataaacagcgtcgttcccagggggatgttgacccatttggaaaggttaacagcggatccggtccacaccgcgcttccgaggttggaggaaattgccagggcgtttcccgcagagttaataataattgacagccccaggtaataaaggcgctgcttgaagtctttcatttttgccattatgtattcaaattctccttcaattgatcatgaattccattgtataatatttaatttggtttgaacatctttactgaaagcctcctggtcaaattgatactgttctttcacaaatcgtgttaatattcacggtagaggaggcggtcttgtggaacgagaatattcggaagtagaagctgagaagcatttcgaaaataatcgtctgtggtttcggcgattccaaacaacccgctcatttcgaaagttaaccaaacccgaaagagcagcagctggatacattactcaggcatttgttggcttagcatataaatatcaattacgaagtccgcgacaatattctgcaaagtcggtcaaagaagttgtcatggatttatttccggaaaaaattgcagcgaccaacgtctttttcacatccgttatcccagtgatgcatcgctactttgtcttcctgggtgtgcagcacaaaattagcaacgcaaaaacgctgatcaaagcgttggaaagcatcaaggtgcgtcagctgttggatggccatcgaaatgccagcaactgggatgcccacaagaaactgggcatgcaggtgctgatgggctataagcaggatgtggatcccaagaaggtctcggcgtacgaagaagattataatatgggcgtcccgctgaggttctgtttcgacttcagcgtcaatcggccgccaaagaatattattttgctgacagagaagttaagaaagaaattcgaaaatgtgatgtatgagaacaacaagtagagcgcgacgagccccgggtgaccccggagcacaagtcaaaaggaccagtgatgaacggttttcgttcatcactggtccttttgacttgtgtagcaggggtcaggggcgtcggagcgtattttggaagcagcagggagcggtagataaaataagtgctcaaatccttgtaatatcaacaccatggaactgggggggtgctgaacgggttctgttcatcttggggatttcttgtttatgcagtagggtcctggggcgtcgcccacaggactaggcaggctttcagccggccgtcggagcgtatttttaatgctggtaggcgcagatgataaacgagtggattcagttcgtgaatttcggcttaaccaaacaaactcagcttgccgataaacccacatcgttttatcctgaaattaatatcagttttaggagatgaacagaatcaaaaaaatattaatcataatcacatcactcgtcctactggtaggctcgtacttcttatggacaatggtcactttcgatgagcatgctgaaagctacatccaaagagatctcaacaagaatatccgcgaccatcaataccacaagctaaggaaaatgagtaactcggccgcctatgaatggttgagaaaagcaaatcacgtgaaatttacttttagttcggataatcaaggaagtggcaacttatattattatgctgcaaggatcaatcaccaatacaatttttttgtctcctttaaggtgaaatcatttattccaagtcggttcactttaactcggatcacctattaccctaactatcatccgcgctgattcaattcatcaaacaaaaaaagacctccgcagccaaccagccacgaagcgcccacaaataatattcagcaaacaacaactaatttaaaacctgaacgcgatcaatgctccccaacttgaccaccgtgacgcctttagcaggacgctcgatgaaagcctgatcgtcattgactgcagcgacacttcctgtcagcgtgccgtcgccggtttgaatgcgcactaattttttattcttataagcattcatcaattcatttgaaatttcttttgtcgcaatagtcaacattgtcacctcttatgataaaattaattatagttcacaattctgctggatgtaaacaatttttctcacaagcataagcttaagaataatttattaacatttttttgcatttagcgctaaagtggatatataggtaagtgaaaggggtattgaaatgactgaacgccaaatgattcaagaaattttaaataccgttgatgttatttatagttttgtcaacaccgacgatgacaagaaggaatacgaaattgtgatcaaccgccaagacggagataatcgtccgcttgagaacgtcaacaaggaaatcaaacattacttcactgatgccaactttagttatgatgaagagcttaatgacaatggcgacgacattcacgtgcaggtaaaacgttaattggtctagttgagtattacttcacaaaaagtgattgaaccagcaatttgaattgtaatgcacgttatggtatagttcataatgtgcttttttaatataatcaaaaggctataaattgatttgaaaattcgagttaccgaaaaatttttaatggaatatgtaatcgctttctagtgtttggagggaatctaatgttaacagacagaccaaaatatgttttatcaattgatcaaggtacgacttcgactcgagcaatgatttttgaccacagcggtcggaaagttattgaagcttcaaagcccgttaagcaggcaatcccacataatggctgggttgaaacagaccccaatgagatttggacatccgttttgaatgtgatttcttcggcgttcattgatgccggcattcatccagaagatattgagggaatcggcatcgttaaccaacgtgaaaccacccttatttgggacaaggagaccggtgaaccaatttataatgcaattggttggcagtctaagcaaaccgccgctttggcccgaaaattaaagaatgacggctattctggtatgattcacaagaagaccggcttgattattgactcttatttctcagcaaccaaggtccgctggattttggaccacattgatggtgctcaagagcgtgccgaaaaaggtgagttgatgtttggaacggttgatacgtggctggtttggaaactttccggtggcgagtatcacgttaccgattactcaaacgccagtcgtaccatgctgtttaacattcacaccctgcaatgggatgatgatattttaaaattactcaacattccaaaggccatgctgccagaagtgaagacttccagtgaactatatgggacgacgaagaattatcaattctatggtattgaagtgccaatcgccgggattgccggtgaccagtcggccgctttgattgggcagctggcgtttgaaccgggcatgattaaaaatacttatggtgatggtgccttcattatgatgaataccggctccaaaccagagatttcagatgataacctgctgacgacgattgcttataatttcaacgggaaagtcacctatgcgcttgaaggttcaatttttgctgccggaactgctttgtcctggttggcagacagcctgcaactcattgacaacgttcctgaatcccgtcaggcggctatgaattccgaagacgacgatgaagtctatgttgtcccagcattcaacggtttaggagccccctactgggaacaagatgttcgtggggcggtcttcggcttaactcgcggaacgaccaaggacgactttgtgaaggcaaccttgcagtcgatcgcatacggtaccaaggacatcattcagaccatggaaaaagataccagcatgcacatccctgaactgatggctgacggtggcgcttcacggaacagttacctgatgcagttccaagctgatattttaaatatcccaatccaacgggcggctgatgagaacaccactgcatttggtgccgccatcttggctggactggcagtcggtttctggaaggatattgatgaaatcaagagcctccaagagccgggccgaactttcacaccaaacatggaagattcacgccgacaaaagctgtatcgcggctggcaggctgctgtgcaggctactcggggatatcgggttaaaatttaggcttacagtttaatagtgtacaaaaatagagtgctcagtcaaaaattgatttttggctgagcactctatttatattattcatttttatcttttggctctttccaataattagcattactgagcagttccttagaccgttcatccgcgggaacaaagccaatgttgaacaggtgcttgaagtacatcatgttataaatcagcatccaaacgatgccgagaccatatgagccaagggtgtaggcaacttggaatggttcgcccattccaagtgacagcgccattccggcaatgatttccactccagccatacacagcaggttataccagtctgatcggaaaattggcacccagaggttgaataaaagggcggtgaatgacggaccaactttggcgatccgaatctgaccgttttctttgttcacgacagtagcaaagttcggtggaatcgggagtccagttggattgttaggatcattttggttattgtcatcattattgccattaccaaatgggttttgcatggggagcctcctttcgaactaatggttactttttcttgaatttaacaacacattcacaacgggaggtttgcggcatcaaatccactgattgaatatattcaacgttatacttctcggttaattttactaaatcctgcgccaaagtcgatgggttacaggaaatgtagacgaatttcttcggcacgatatctaaaatggtgtcaatcagcgaatccgctaaaccagttcgtgggggatcgacgattaatgcggtcggagtccagccgtcgtcaacccactccggaagcagttcctcagcttcaccgacctcgtataaacagttaaagatgccgttacgcactgaattggcattggcgtcttgaaccgcttcggcaatcgtatccatcccgcggacttcgcggacctgcttggccaccgaaaggccgatggtcccgacacctgaataggcatcaaccaatttttcgttgcccttgagatccagtgctttgaaggcctcatcataaaggatcgaggtcattgcagggttggcctggagaaatgcccgggcggataaatcaaacttcaggccgttaagcacttctgtgatggtttcccgaccagccagatgaatcatttcatcgccccaaatcagtgaggttctgcccggattaacattttgcatgactgaaacgacttccggtaattccgccttgatgcgttccaatagctggtgcttcttgagcagtttcttgctttgagtgataaaggtgacctggacttgatcggttgcgatggcggctcggacaacgacggttttgatgatcccggcgtttttctcttcgtcatatgcggggatgcccagttcatcaatcatcgtcacaattgcccgcatgactttcatcgtcagtgggtactgtaatgctgaggtcttgaggtcaacaacgtcatggctgcgggctttgtacaagccggcaatcgtgttgccgttctcgtcgtgacggatttggaatgtcgccttgttccggtaatgggtcggatcatccataccgatggttggcagcagcttaaagcggcgataaccggtgggctggtatttttccagcgactggcggacaacgtctcgtttgaactccaattgctttgggtaggccaaattttccaactcaaaaccgccaacgtcatttgcgtagtcgtccactggttgaatccggtccttgctcttaatcaaaatttcgacgagcttggcccggataaagttatttaaatcgttggtgacttcaacgatgactttttcggttgggagcgcaccgggaacgaaaaccagtttgcgttcgtagtaaccgatgccttcgccgttgattcccattcgcttaatttcaattgttaattgttcaccttcgttaacgtgaaccgtattattatcgttatacattgaaccgtccttaatattcttagttactagtatgatagcacatcacgagggctattcgcatgtgaagcaggcggacgcgaggtgtttcgtcaaagaatttaaggcaatcaatcgattatccttaattgcggacaaaagattgattgccttaaatggctggcggccacggttaccgcggattgagggtaacaaaagtggcgcaccaaatgaattgagctttttctaaaataaattctggattgaattgaatcaatcgacttaccaggttgcagtatcaggatcggttgccaaacctgcttgaccatggaagccgtcaatggtcttcatatcggtatttgacaagttaaagtcgaagatatcggcattttctttaatgtacttctcgtggattgattttggcagcggcaggaatccatgctgcagtgaccagcggagaaccacctgagccggcgtcttgtcatactttcgaccaattgtagccaattctggaatcttgaaaatttcaccggttccaagaggactgtaagcttcggtcaaaatatcgtggtcatcattatattccacgaccgccggctgcatgtccgacggattgatgaacatctggttaaccattggcttaaccttagccgtttccaacaatgcgtccaaatgttttggccggaagttggaaacaccaattgccttggcagtcccggctgcataaaattcttccatggcccgccaggattcagcgttggcttcctgccaattgtctcgaaaggcaaccggattgggccaatgaatcaagtagagattgacatagtccaatcccaacttttccaaggatcggccaaaggcttccttggtcttctcataaccgtgatcagcattccagagtttggttgtcacaaataaatcttcccggggaacgccgctatctttgatggcttgaccgacactttcctcgttgccgtaagctgcagctgtgtcaatgtggcgatagccggcgttaagagctgctaaaacggcatggtaagcctcatcgccattggcggattgccaagtaccaaagccgacttggggaatcttgaccccgttatataaggtgtacgtatctgttaatgacatgttcgaacctcctattgtgtctctaacactattttatagaaatcaaatatgaagtacaaagaatttatccattgaggagtgctcaccgttattcaggggatgccccaaatcggtaaagccgtattcagtgtacaggtgaattgcttctttcaaagcgtggtgggtctccaggtagaccgtctgatagccggcccccttggcaaacccgaccgctgtgtccaacaatctgtagctgagatggtggccgcgggccgagtcagttaaatacagtttctgaagttcggccacatgattggcatgatcgaactcagcgatgccgttgccacccaggacgttgccggcgtcatcgacagcaacgaagtattcccggtcatccttttggccatagaagctgctcaaatggtcaagttctttgtcgaaatacgcggtccccggaatatccagtccgtatgattttaaaatggtccgaataatttttgccagctcgaagtcatcttgttgtttaatcggccgtatttttaccattctatcagctcctgtccttaacgtttgattagcatattaccacttttggaattgcagagtaaagcccatgtgaacgctttatcgtgatatactggaactaatttggaacaagttcgggagggatcactatggatcaaagagttgcgattgtgacgggcgcttcatcaggaatcggcatgcagattgccaagaacctctatcgaaacggtatggaagtctatgcactggctcgcagagtgtatgcgatgaacgagctggatgatttgggtatccacaccatgcatttggatgttaccgaccacgatgaaatcgatcgggtcgtcagtgagatcgttgccaaaaccggccggattgatgtcttagtcaataacgccggcatcggatcgtttggctcggttgaagaagtcaccttgacggaaggcgagtacgaattcaaagtcaacgtcttcggtttagtcaaaatgattcaagcggtcctgccgatcatgcgaaagcagcatagcggccggattatcaacatgtcatccatggccggcaagattggcaacatgctcttgggcagctggtacatcggctccaaattcgcagtggaggggatcagtgattcgctgcgacaggaattgaaaccatttggcattgacgtggcaatcatcgaacccggtgcgattcagtccgagtggaaggatggtgccatggaccggatgatggatgcgtctggcagcggtccctatgccaaattggcccggcgatcggcggctttctttgcgatttcctacaagtttgctgcagccccgagggtagtggccagatctgtcgaccgggcagtcttttccagacgaccgaagaccaggtatgcgattggaacgggcgctaaaccggcaatgttaatgaagcgcttcatgccggacaagtgcctggacgccttctttgaggccttgaataagtacgctcagcaagttgtcaaccgagaaacgggtcaaaacagatagcaattgaccactgaaattaaataaagtaccattaacttagaaacactgggggaactgctatgtagcagctgagaccgacctgaaccaggtcgaaaccctttgaacctgtcagctaggactggggtagggaagcagagtgcgatcacgggcggttagtgaccggagtctaagggactttggacggaaatcgagttagattttcggccgaagttccttagatgcaggccactgcccctgggagcacgtttccgctagataacagcaaaaatccagcagaaaccaccaaccaaaaccaatcacccaggagctgcagacaccaagtgtctcagctcctatttttgtcagcaagcaaaacaacaaaggagaaggatcaaatgaaaatcgatttattagacacattacgaaaaaagaaccccatcgcttttaacatctccaactttgttaccgttcaagatgttgccaatggcattaatgcgttgggtgcatcaccaattatggctgaagaaaagaacgaggccgagccaatggtccaaatggccgactcggtgaccgttaacctgggcgcgtttaccgagggtcagttggaacagattagtgcggtaacgactttcgccaatcaatacaagaaacccatcatcatcgacccagtggctgtgggcgcggttgactaccgtaaagaacgctgcaatgaattactggatcagatcgatgtcgcggtcattcgtggtaacgcgggtgagattgctgcattggcggacgttgagtggaatgccaaggggattgatgccggtgaaggcagcggtgacttggaagaaattgccaagaaattagccaagaagcgcaactgtgtcgtggttgaaagcggcaagaccgatatcattaccgatggtgaggcggtggtccgaatctacaatgaaacggatttgttcaagctgcacgttggttccggggatatgctgtccagtaccatcggttgcttctgtggtgtcgagcacgactatttcgaagcagcccagacggccacgtcggtctttgatgtggccggtgaagtcgttgccaaatcaatgcccaaaccgctggcaggatcatttggtgttcagttgatcgacgagcttcatttgattgatactaagaccgttgagaagtatgcgaattttgagtagaaaagagtgcgacgaggcccggtttgaccccggagtgtaaggcggaaatttaaaggatgaacggttttggttcatcgtttgaatttttgccttacacagtagggggtcagggccgttggagaacgtttccacaaagtatgatatatacggaaaaacccacatgatcacaagctcaacaaagaaaggtaggactcaaaataatggttaacgaaacagttcaaactttaacaatcgcgggaactgacagtggtggcggtgccggcgtgatggccgacattaagaccatgcagatgcgccacgttttctcggcggcagtgattgtggccgtcacggcgcaaaacacgattggggttcaggactttatgccgattcccaagaaactgattgatgaacagtttgcctcagtcgcagacgatttgaaaattcgcgcttgtaaaacagggatgttggcggacgtcgccacggttgaagcagtggttgagaatttgaaaaaatatgatttggggactctcacggttgatccggtgatggttgccaaaggtggtgcccgcttgctttcagaagatgcgattaagacggttcgtgagcagttgttgccgctggccgatattttgacacccaatttgcctgaggccgaagaattgactggcatgaagattgaagacaaggatcagatgatcgatgccgccaagaagctgcaggatctgggggttaaaaacgttttgatcaagggcggccaccaaactgaatcaaaagagtcctcagacttcattctccttgagagcggcaaatccttctgggtgagctcaccgcgaattgacacggttcgaactcacgggactggcgacacgctctcgtcttgcattaccgcagagattgccaagggcgccgatgttgaaacggccatccggattggtaagaagtacgttcaagcaaccattgccaatgggattcaagtcggtcatgggcatgggccactgaaccactgggccacatttgaaggggacggtgactaagatgggcatgcaatttgaaccggggatgctgcgagcttactttattgccggcacccaagatgtgaaggatcaaaccaagacgctgcaagaaattgccaaacaagcgatggaggccggcatcaccgcctttcaatatcgtgagaagggacccggctccttatccggtgccaagcgggacgaaatggccgccgacttgcgggaaatgtgcagtgattatgagattccatttatcgtcgatgatgacgttgaattggcagttaaaaccaacgcggacggcgttcacgtcggccaaaaggatgagcgggtcaccaaagtcatcgaagcagtcggccagtcgatgtttgtcggcttgtcctgtgacaccaaagagcaggttaacatcgccaatcacattgacggtatcagctatcttggcagcggcccggtctttccaaccgggtctaaagccgacgccgatccggtgattggcgtcgatgggctggcaactttggttaaggcgagccaactgccagtggtcgcaattggcggcattaccgagcaaaatattgtcgagcttccccaaaccggggtcgccggtgtttcggtgatttccatgattgcccaaagtgatgatatctttagaacggttaaagtaatgaacgaaacctttgaaaagtaagggcttcgcaatcagttgaaatagacaattaagcggatagcgcactcctgtgattttccaggattgtgctatccgcttacgtgctgctattgagtgatgttggccaattattccatgttaaagccctcaacggttgcgtggggcaggtggttaacttcgccggtcatggtcttcatgacgtcggtattgttgcgggtgtaatacgagacttgataagggccgggcccgtttaccttacccttgtaggtttctagaaccggttgaacaaaaccggccacatctttgttggtgacccgggccaaattaacgtcgctggtgttgggtgttccaaacgctttccagtcagtcgtcgaagtcggtccgaagacgaagtagctgccggagcggtcataagaagtctcgtcagaatgaattttgacactgtgctttccaaaataaatgttagattggttgccataccaggcaccgcgaaatggttgggccacttcgcttggatttgaagccgaggcatcttctcgatgatgggagacgacacccgaaagcccgatggtgcctacaaaaatcagcgttaagataatcgtgattgtcgattttttcatgataaacgctccccaaatatgcttatctattaccatctaaagggtactccggcaatgtaaattaagtgtaaacattgggtatcaaatatgtacaaaattgatattactcgaagattacctccaagttacaattattaggtttggataaaatccatgcataaaacttgtgattttggcggaaagccgttttaatagaacatgaacacgtttttattttcaaaatatttaattggggtgagattgaatgaaaggacattttaagttagcccttacggctgcgttcctgttcgtgtccgccggcatttttggtgtcgctgcaccaactgccagcgccgacgtgattgccaatcctgggactgcgggttcgattccgcaggtcaatgcagggaacgtattgaaggactacgatgagaattcactcaacgtggttaacaactcaacaccgcagggtaacacaagcaagaagtataccaagtattcattggatccaactggttacaactacggcaactcgtacaatacaattgccggcagttcacaaagcaatacatttaagacgaagttcttcttaccagatggcttcaatgtttccaactatcaacatggtaacttccaaagtgtcacacttgatggcgatgggaacatttacttcatcgaatcaaatggtaccaacaccaaccagggggcaattgttaagttcaacatggctaagcttcaacagttaggcgttggatcggatgttttactgctgtggcgggcatttgattacttcaacccgtatacgacagacggtcaagctcataacgatgagtacaaccaggtcaacgcgcaattacaaggtgcatttgacaaggttcagaccttgacgacgactttgaatcagaataagtcctggcaaaataaccagaacaactggaagaagaacgctcaaaagtggtattactactggaagaacaagaaagccaagtataccaagatttccaagtcatataagtattcatacaatacccgggccaaggctaagaagactgtgaagacagctacttcaaagatggcaacttggatgaaatcttatcagtcacacaaggctaagattgccaagtacaataccaagatcaatagtattcaatctcaaatcgatacttatcaaggacaaattgacgacgccaaggcgcaaaaccctgacatgttcaaatacgttgatattgcccagacagcacagttgtctccagaagttgatattggccatggtcaaacattgtcatacaacccacaaaacaagcacatctatttagctgaagataacacgttgactgatttggcatcacgggatgataacaacacggttcttgaaatggatccgaataccttgaaaccaatccgtgaatacaacttcaagatgtatcatggcgactctgccaacttgcagcttcacacactggcatttgacagtaaaggaaatgcttattggggccgtaagttgaacggtggttacatgttgttctacggacggcttgatgaaaatggtgtcagcttccaggcttcatcatcaatggtcggcaagcgtggcggttccacgaaccaaggagttgccgttaaccctgccaataaccgtttgtacttcgtttctgatgatatcttgacctcagtgccaacatcaggcgttcaaagcggaaacttctcggcagacgatatccactatcaagccttcgattccggtcgtgagtttgaaagcttagcgtttgaccaagacggttacggatacttgctggcattgtggccacctgagttgatgcaatcgactaatcctttgaattaattaaataggtgagagcaggaatttcctgtttgatgtttatgagtagcagtcgcgagtttgcggctgctattttttgttggggcaaaatcgtcatctcaaaggtgacattaccaggcagtaggcctaatttgtcaaaacaattaaatagtccgccaatcaaaaaagagaccgagacataactattgtgaggttacgtctcggcctctcttgggctccaatgatatctagtttaaacgtgcaacaatcggctgatcccggccatttaagcggagaaacaagtcattccaaaaacaggaataactcgcttctccgcttaaattctgggatcaaaacgcctcgtgccgcactctcttttattaccctgcatatgcctgagccaaaccggcaatgtctgccgaagtgatgtcgttgtcggcaaccgttggatacatgatgctgtctgtatcgtcagaatgctgcaatcccaatgcatggccgagttcgtgctcgccgacgtggattctttctgtcgtcgtgtatttgaacagactacagttattggcgtaaatcgttgaagtggatggcgccaacaagaacaaattgttcttctgtttctgataatacttgacggtcgtcatcccagcatagtctaaattatccgtattatcaacggccagcgtgatatcaggattctggcttgctgcggttaaatgaacaatgttggtatcgttccacttgttgatagcctgttgccaaacgttttggtaatacgctgacccagtatcaatcttatatgtaatggttgtgtccgcccaccgatatttagcaggtgtggtgttggaatcgttggtagtcctgacggaagcctgggccggtgattctgtctgctgggttgtcgttttaacacgtttgacgtattcgatggccgtgttaatttgcggggtgtcatcggtggtttcggccacaactggatgggaaagaccaaaggttacagtgacggtgaacatagtgagcagtcggatgatcgttcttttcatgagcatttctccggattaaaatttgtaacctgatatatcaaaacagttactttaatagagcattatatcatcatattattaaaacacaatactgctataacgataaagtgataatcaaacaggtcatttatcaatcacgttctcaatcaatgatgcctcaaagtgccagcatacgccacgactaatgcggtattcaaaaaagggctgcggcacaattttcattctgtcgcagcctgatgactcgctattcaatttggtaatcagaagaaataccagtcagccagataaaggcccaagacactggtcaatgcgaagacaaccaccagcgtccagacgatattacttgccaggttatgatgactcttgcgggcaaagccgatttccaataatgcgatgacggccaggcccaagatgaccttcaggctgcccagcaccggatctcgtggtacccgataaagggccagcatgaagccggaaaccaggatcggaatgtacagcacacgggtaatcatcatgaaaatcattgaaagcttatctttcagaacaaatgccaaaattgcggtaatcattaataggatccatgaaatgagatggatattcatataaagcaaaatgtaacctcctcaactgtgtttctattttagtatagtattttgccggcaaaaagaaaaagtaatttcttgattaggttctgcaaataggctattttttaggtagttgaaacaatcgaaacgagggggttgtcatcatggacgggctgaattatacccaggaatttgtgctgtgcgtgctgaatcaaaagccaaaattgagtgcattcaaggaccgcaaagtcgctgcgtgtttgttattatcagaaattgttgaactgttgcgtgctggggcgatggaattgacgcctgccaatcgaatggtggttgcccaagtgactaaggcaccggcggattatttagtgccgctcactgaagacatcaagaaacggcagccggagtcagtcaacaattatgttcgcgacgcggttctgtcggtccggaaacgccgggtcaccaagattgccgaagcgatttgtgattcgctggttaaagcaggctatctggaagttgaccacaagacctattacgataatcaaacactgacggatcgcatcttaacgcaactgtatcaagatgcgatcgctaaaaaagaaccgtcggagaagaattccatgttggcaattttgctcgtcaattcaggtttggtgcaccaaatttttcccaagcaggaggccgaaaccatcgaactgcggcttaaagaagtcatgaagtccgaccagtatcatttgatttcagatgtgaccaaacggatcaataaagatctggctgggattattgacgcggtctcatttgccaggtgagattaatcaaaaacactgcatcatataaacacgaaaaagccgggataaagttttctttatcccggctttttcgtgtttattatttatgtgaatattgcgcctgcagtgcattaagcgctgtgacgtagttcatcgttggcaggttgccggccttaaaatctgctagtttgtcgccatcaattgccatcgtcttgaaagcatccgcctcagaaaccccggcaccttctcttgcttcattgattcgcttgagtaattcagccggtaagaggctcaacagataaaggcgtttgatctgcgtcaaagtctgccggtaagcactttccggtgcggttccagcgtagtaggccttgatttcgtccgggtcaaattcgacgatattgaaaagataatcgtccgccaagtgtagttttgcttgatatgacttgatttcagccaacatttcgttaattatcatgattcaactccattgcgttattttcaatctttcctatctatgatatgacaaatcaacgcagaattctaatcgaattaatatttggcagccaagttagcgtattcctgtggggttaaggccatgatcgaaccgtgacgcttcttgagttggccgaagtcatagtctggcgcgacctcccagtcggtgggattgctgctggttagatcagacgtcaaaattggcaggtagccgcgaccgttgtcgaattggtcgacgtaaatgcaccatttttgctgatcagccagccaaacaatttccgggccttctaccgtatcaccttgaatgcccaagtctaaatcttgaagggcggtcacctgctgccaatcgccagttagtgaaggtgactgttcaattggaattgttccgtcacgggatgcgcggacgaattggccgccagctttgaccatggtcatgtcgatcaaatcattttttggattcttggcaacggcgtaagttgcggttgattcgaagtgctggaagtctttagtgtatgcccgccagatttccattttgtgggtttgctggttgggggatgaccaaaagacaaagtaggcttcatgagccggatcataaattgcttccggtgcccaaacacagccggtgtcctcaccgaccatgcgaacggcgcgaggagtggaccaactcagtagatcagctgaatcccagaaaatcaaatccttggacccggtggtagtggctttggcctgaccccagccgccgcgatgataaatagacaggtcggtggccatgatggtgaaatggccgtcctgtctgcgcatgatgaagggatccctgacgccgcgctcaccaatcgtcgatgttagaaccggctggttgtggttgatgtcggtccagtgaagaccgtctggacttaaggcaaagtatagttgttcagcggatgggctgtcttctgttccagcaaaaaacacgaagagatagccgccgttagtggattgattattcaatgtcaaatgctccttttttagcttgttttagtaaaaactcgttgtgaataatatagcgcttacaggtggggatgtaaatgctgttttgttgtgtgaggttgattcctatggtaaaattattgttaccatagagtaacagatggaattttgaaaatgcaatttaacagagaatatgcaaaattggcaatcaatcagattgaaagtgcatatcgtaagggtgatattttaaggcgccctggacgacatggatacggacttcattctgagaagacagaagcttacttgcgagaccacggaattacctttcaaaaggcactgaaagatgctgttcaggctctgagtacctcgaagttaacaagatttcgtggcccatctcccagttattttccgggacaatcagatggggttgtgtatgactttttggtgccgctttatgattctaatatgtacatcaagttttcactcgtcgtccgcaatgattaacaattcataattttcgaatcatttcatgagtctgatagaaacgactttggaaattttattgagttgaatgtatgacaggggaggcaactaatatgaatcctgtaaaagtaaattcagtcattactgaatatgatccgatttctgaccaaaagatcaaatatcagaaaattcaaatttctgaatccgtgactgtgagaaatatatctttcaacagtccacactactaccttgtcgaagaggggctggacattcatgatcctcagaactttgaagtcccatttgacaatcctgatgtgaatttgcgggctgattatcagatctatcgtgaaaaagttggcttcctgcaaccaagagagattaaaaaagtcagagaacatctgagattgagtttacgtgaagtgtcagccattttaggaataagttatagtacattatctgaaattgagaatggattagtattacattctcaaattcaagatacacttttacgaatgcttgaacacacctacactttgtcgacgattgtcgaacagcataaaggcttgattattaacagtcatgggctgaaagcgtaccagcgaattattgacaagttaaatgctgagaaaaattgggattcatgaagattcgatgtggctttatttttgcttaactgatgtaaatcatttcccggatatgatacgatgaaagcgtagtacattcgaataaatataaggtggtaaataaattggcagaaaatgataattggcagttaatgggcgttcgtttggatggtttgagctttgaccggagtaattttaacccgcaaaagggcccgcagatcaatgctgaaacccgtttggcattgcctaacgacccggcagacaaatcaaccatgagtgtcgttcaagttgtctcgactttcaaattgtatgacgatgaattagccaaaagctatttcacagcaaccattgccggtgtgtatcaggtgccaggcagcttgacggataacgatgctattcaaaagacaattgacgatgacaaaaacttgcgagacagcttcgcccaaccggttgtcgattacttaatcgcgaccctggcagacttaagcttaaaggcatttggcacgccaaccattttgaagcgcgagcaattgattgatactttgtttggtgcaaagcagcagtagtaggcaactatctcaatattaaaggacaaatcaacagtcggcgcaaaggtgaacactttgcaccgattttttgcactcataattaccactatgaggaatcacaccgtattcaaagctggtaaattgcgttagaatgtacaaatatgttaaatgaacgtcacgaattggaggaccacatgagctacttagagctgcataacattaaaaaatcctattaccttgccaaccaggaattcccggttttgactgggatcgacctttcctttaatcaaggggagttcgtctcgattgtcggagaatccggtggtgggaaaacgacgttgatgaacatcatcggcggcttggacagtaattatgccggcgacgtcgttttgaacggcaaatcgctccgccacgatactgccaagcaattggatgcctaccggagacaaacgattggttttatttttcaaaactttgatctgatcagtcacctgactgttttcaacaacgtcatggtgtcactgcagatgaccaaactcagccataagcagcaggaggcccgtgcccgccagctgttggaacaggtcggcttgaaagaccacatgaaaaaatatcccaatcagctttccggcggccaaaagcagcgggttgcaattgccagagcattggcatccgatcctgaaatcatcatcgctgacgagccaaccggtgctttggacagccaaaatacccaagaaattctgtccttactggaccaaattgccaaagacggcaagctggtgatcaccgtgacccactcggagacggttgccaaccacgggacgcggattgtccgcctagctgatgggaagatcagcgaagacaccaccttaaagccaggttatgagaagtctcaagccaatgagctggcaactcacacgctgagatttggcgcaaccttgaagatggccttggaaaacatgcgctataacctcaagcgaaacctgctgattgtctttggcgccgccattggaatctttagtgtgattgtcatgctgggactgggtaatggggttcaaggatacatcaaccatgaaatatactcgcaggtgaaccccaacgctgttcaggtcactaaaaacgtgtcggctgatgccagtaccgatccaagcaagattaacgtgaccaccaaagacaagaaccgattcaaggatatcaaaaatgtgaagagcatcgacgatggctactttgttcagggtggcacccagctgcgacgtggtcataaaacggcttcaatctcatttatgcagacccataataaaacgatgctgaccaagagcattgccaaggggcatgcgccaaagaacggcgagattatgctgaccaaggaatacgctgaaaagcttaataaaaagcatccatattcgttgatcggtaagcgggtcacattttatcagaacacgcttaataagaagaaacgtccggttatgctgacgaaatcactgaaggtcagcggaattgccaaagcaaataccgggtcgacctcggtcacatacagcacgatgaagtcactttacaactcaaagggcatcaagattcagcctaattttgtgaccgtcgaaatcgccggtaacgttaagaacgtcaagccggtcgagaataagatcaaggcctacaagaacgacaagaaaaaggccgcttatcaaatcaccggtgtcggcggcttcgttgatacgctgaacacttatatcaccctcgcagttaacgtcttggcaacgattgccggaatctcgctgttggtatctgccatcatgatcattgtggtgctctacatcagtgtctccgagcgaaccaaggaaattggaattctgcgggccttgggatcttcaaggggaagcatccgaaacctgttcttctcagaagccttcttcattggcttgttctcatcagctttggcgattgcgttggcggaactgctgcaggtagtggccaataacattgcccagcgaggaatcaattattcaatcatgcaaatcacccccggaaatgtcattttcggctttgtggttgccattgtcatttccttactggcagcactagccccagcggcctcggctgctcgattggatccaattgagagtttaagttacgaataatagtttgaatgacaattttaagtcctcctgcgaataaacgggagggcttttttcgtatatcatgaatgtgctgatcgaaccatgctcatgttataattatgttataacatcagttgggaggagatcgaatggctaaagttaaggttcgaaaaattggcaactcactcggggttcttctacctaaggaaagcggtgtccacgagggtgatgagctggagtacactcaagagggggacaaaattattttagacacacaagaagcgcaaaatgcgagagttagagagattgttgaaaatagcttcaaagattttgaaacaggaaatgttttgactgaagatgatatggtccgcatctttggcaagtacggttggcataaataatggatccatatgaattgtcgttctcaaacgattttcaaataagcctaaaacagacaatcgccatctgggagagcattggcattgatgccggcaaaattcagacctttgtctcagatattaataccgcagtggcttcactcaagatatttccaaatcgttttgccaacgtcgatgaaaaatatcgcattccagtaccgactaagcaaattattatcggcgaccattacgcaatcttgtatcgagtaaaggaagcgacacacacagttgagattgggccaacttataatttgaaacaaatgggtattactttttagattctcctgagagatcagcactctaagaggcgcggaaataactgattgtcagtcatttctgcgccttgtgctgcactctagtattgacaacccacccacgtggtatacaatactatataaatagtattggaaactacgtaaatatcaaaggagatttcaaatgtccgaaaagattgccattctcgctgattccggttccgatgtgccggcagaattgctgaaacaatacgataatattgaagttgccccaatgctggtgaccatggccggcgaggaataccgtgacaatgtcgatattaccccggaagaattttatgcccgcctcggccaagccgatcagtttcccaagactgccgcacccactcaagggagcgtggaagctcacgttgccagcttgaaggaacgcggcttcaaccgaatcatcggcatcaccgtttcggcacatctctcaacgacatttggcattttcaccaatgtggcaagggaaaacgccgacatcaagatggacgtgatcaataccagaaatattgggattggcagtggccttttcgcggtctacgctgaagaaatgattgacagcggtcagacgtttgacgaaacaattaaatttctcaagcagtctgttgaggacagccggacgtttttctatattcccagcttgaaatacctgcgggcaggtgggcgtatcggccgagttgccgggctgatcggctcggtgcttaacattaagccggtgatcgcgaccgactctgaaggaatctatttcccggttgccaaagcccgttccgagcagaaggccatctcgaaaatggttcagttggtctctgatataatcgccagccacaagagtgtccgagtcggcgtcgctaatggtgccgacgtgcccctgcaggaaaaagtctatgatcgcttgcactcggccttcccgcaacttagaatatatcgaggaagcgtttcgcctgcgttaggggttcacactggtcccggcttggttggggttggtgtgcaggtaggcgaaggcgaataacgaaggaggggttcgatgccaaaaacgaccaccgagcttcagattagattgccaatgtgggaagaactgccggcattttcactgcacttggaccagctgttggatctgaccaacgagtatctggaaccaatcatcggcgacaaaattaccaagaccatgctccacaattatttcaaagctaaaattctggtgccgccggtcaaaaagaagtatcagcggacgcagctggccggcgcaattgtagtggggctgctgaagaacattttcacgttaaacgaagtgaaggccggcctgatcaccttattgggaaatggcacgcccaagaccggctacaataattttgtgattatgtttaacgagcaggctgccaaggccggcaaggaattgtcggaccccaccagcttggaactggcttcagccggccagcccactttgatgcagtatgatgccgtccagtcgatattgttttggctgtcggcgaagaatcgattacatgaaatgatggatccacaagaccgtgatggcgcttaggcgtttgtcacggtttttattatggcgacatatattcataatgggtcagtcaataactttattacaaatgtgtggaaatcgggtttgccgtgaactaagatagtcatgtgtgaattgaattcgttttcatttattattgaatatttatggaggggtaaatttgaatagtaatcataaaatgttattgagggagttctctattggggcagcagttatggcagcagtcgcattaagtgcacccgctctgacgaccagggcaagcatttcaactaatcaaaacgtgtcaacgttaaactcaagtaccaaagttcaatctggccattacaccaaagataattccgaggacaattatcaatttgactggtctctcagtgatgatggaacattgacgttatctaatgcaagttttgtatttggcggtaacaattcgccgattaattcccacatctctaatcaattacctgccgatgtggtgagtgccgttaagaagatcgttctgactggtagccccgttgcaagtgggaatatccaatacttgttttgtcactttgccaatgttgaaaatattgatgttcacaatttgaatgtttctggtgtaaccagcatgcaggccttgttctgtgaaaatcaaaagctcgattcggtgaacatctcatcatgggataccagcaatgtttcaaacatggctacgatgttctgggaagaccctatcacgaccattactggtttgaatgatttgaaaactggtcaggttaccgatatgcatgaactttttgcgacaagtaactctgcagacaactcgaaggtgactcagctggctcaaagttttattaacactgcagatgtacacagtgtaaaaaactttgaaggattattcgataacagcaacatgatcaacctggacatcagctcgtggcacatggatgctgccactgacacttcaaatatgtttggggattaccaaattgcccttcaaagcccattggtaagctacaccggctctaaaatgaccactttgactttgggacccgatgacaagtttgtaccggtttctgagccaactgctgttgtagcaccaacctttaacccctttggatccacacaaacttacgttccagtaagcctaccttctggaacgaccatcaatatgcctgtcgataaatcaggcaactgggaggccgtcggcagcggaacggtaacgaatccacaaggtgccacttggacaagtgctgattttgacaccaaatacgccccaaccgccacaccgcgcccagccaaggaaacctatgtctggaagcacacggcaccaaagctcaacatcaatttgaaatcgccagttactttgaaacagggcgccaaatttgatgctgacagctactttgtttccctgactgatgctggtgaaaatgccattagtgccccgattaccagtcttaaagacgctgaagcattggggatgaccatttctggcgctgacaaagtcaacactaaggttccgggaacttacaacgtcactttcaagttaggcagtcaatccgcaactttaaaggttacaattcccggttcttcaagcaacggtggcaattccagcaacagtagctcatcaactaccccagctagcaccgccccaagtaccaacaactcatggaacccaacgacaccaaatcaacccaacggcaacacgggcttaccgaactacgctgctgtaaaaggtgacgccgtatacgccactaaggccatctacatgtacagctcaccaaacttcaccaagcataaccgaattgccaaatacaccaagaagacccgggctactcggccgatgtttgttgtgaccgggtatgacaagtccaatggtggtgctttgcgctacaaggttcgtgatgttaataagggatcgaagacttatggtaagtccggctacgttactgccaataacaagtatgtcggcggcgcttattatcagactatgcccaagaacaagaagcttaccgtaattgctaagcacgggatcaattcctatcgctcagccagcttgaccggcaaatccaaacactacaagaagggtgctcgactgcacgttaagaagcttgtgaagcataatttgaccacccgttatcagttaaccaatggtcattatgtcacaggaaataaaaagtttgtcattcaaggaaattactaatatctgaacgcaaaaggacttgaagccaaattggcttcaagtcctttttgtatctgatttatttaattcgcagcaacaccaaaccatgcccggcaatcgtccagagcgccggcatgtgctgaatggccttgggaaattgatcccaagtggcctgccggacttttcaatttgtcggtcaacgcttgatcggctggcgtcagccgcaggtgccttttgtccacattgtcgatggtgtagagcatgtacaagtcaaattcgtttttggggatgttggtctcgccggttgccggatcgtactgataggttctcccggctccacttccacgtcaaattgcggggtggcgccctcatacaagcggggttcttcgggtgcatgtgctttcatggggtcctggtcgccgctaatcaggctgaaacaaattaaggccagtccaaaacagccaattgcgatgacaaataatagtccatatgtttgcatgcccattcccccaaatgttcattagtccttaattatagaacaattcgttggtaaatagctaaccgactttgacaaactggtttggcaaggtcaagtccgcgatttgaatgtgcataaaataataccgatccgagcccattcacctagggtaataaaaccgaggcaaatcatgcctaaacccaacagccagttgaattagagggcattatccatcgcgtttgcccgtaggactgatataatataatcggaattaaagtgataacatattagttgggttatggaggggattcatatgaataacttaaaaattatgggcgcacttgcaggagcatttgccattggtacaatgatccttacaactcaagccgacgcagctaagaaggtcaaagtgacgtcaaacgtacccattacagcaaccaaagtcaccaataggaacgttgcaattaccggcaagaacaagatctataacaaagccggcgtattgaaaaacgccaaggcggtgacatcagccaaacagctcaagcaactcggcaattcccagcggtcaaaagacttcttcaacgtctaccgcatggcaacgaccaacaaaggccaagtctactacaaagtcgtctcctttgaaggcaagtggcgaggctggatctacgggggaaagaccaaggccgactatcaaggtgggatccgcagcgttcagaccaccaaagatgttccgttaccagacgatgtaaaaaacgcaaaatttaccctgggaaatccaggcatttcggggacgagcaactcctggacggcaattccatggtctcaatacggtgcccggttaaagacgactgactccaggccatacgctaacgatgaattgcgggtgacggccgccaaacagctcaccaggcaatactacggcactttctactatgtggttgatgacactcatcctgagttcaacggttggttgaacagcagcagcctgaaagccgccacaacgccaccaaccaacacgaccacgaccgtgaccaattatgtgcaatcgccgcctgaggttgtgactaacacggtgacaaatacggtcacgaaaactgttgaggtcccagccaaaaatccattgacaattaactacaatgtttatgagttgggaacgtcccagaaccaagccgtttccaatcaaattttgaagatgtatcaagatcagtacgctagtgttttgagtgaattgaccaagaatcccgataccgcggccactaagctcaaggatcttggtgacgggcagacgttgaaatctaatgacccaactccgatgaactatgcctcaattgcagttagttttgacaaagacaagaatgtgatcacgatcactttgaattgggttcaaccgataatctttgtcagtgatgctcagattcttactggggacgattattatccaaaaagttacctctggtctgtgatggatgggaccggtgtcagctatcagagaggggattggttggatcgagttcaaatatccactgacgtaaatactaagcttcctggaacgtaccacaccacatatactttcaaactgatggacggcatgaccgcaacggcaacggcgactgtcactgttacgaagtgacctgtcatcttgaaggacagaacattaaattcccggttgtattccaccccgaacccgttataatcaaaactgtaacacaatataatacgtggtctggggtgccccaacggctgagatgatacccatggaacctgatacagttaggactgtcgcaggaagaccgattcaaaatgttttttataacgcaaatgaggatcatcaaacacgcaaagaccaggggcaatttagctgccgctggtctttttttgccggtacccgccacgacaggaggaaataccatgtcattatcccaagatatcttgtttgaagctcaaccctatttgattgccaacgagaaacacccatttgttcaaggaattatcaaagggcagttatcacaggaacaactccgttactacgacgagcaggacatcgcctttgagtataacgaagttgcggtcatcaatgcgctcataaaccacagcacgaccaccgaccaggcactgttgttccacaaacggcaggacatgcagcttcatatgctggatgattggctcaaacgggaaccggcgtcgatgccccatgactgggaatcattgaagcaaaccaccattcagccgattaaccaactctatcgccagcacatggcagccaccattcaaactcacagtgtcctgcagattttgccgtcatttgcggcgggggagtggatgtacgttgaattggggaaatttgttgcgactcagaccagagttaaagaagagcccttccaaagtttcctttcaatgagcggggatgattttctggggccaaacggctatatccagcaattctttgatatcatcgatcacgaagccgagtcagcgaccccacgtgagcaggagcaagccaagcagacattcttgaagagctgccttttggagtggtatttctgggacgcggcttataaactgattacttgggatgactggaagaaaaatgcattaggtggtaaaggcggagtgacgttgtaatgaagcagataaattgcttgacgatatgtgtgaatcgaatataattattgtaagacgcaggtattacacaatcaaaagaggtgatttcattggcagtggatatgaagaataagacaatttctacccgagtcaacgaaaaaatagcagaaaaggcaaaacaaaatttagccaatgtcggaattacagtctcggaatatcttcgattggcattgatctcagccgcagaagatggtgtgagcgatctattgaactccccagaagcaatgcaagcgaagtttgaagctgaacacggtcagaccctcaacattggaagtgttgaagattacaaacggtggtcggacaaattatgactcaacttcaaattaaggcaactggacaatatgtacgaagtttgaaacgattgaaaaagaagcattatcctgttgagttgattgaggactgtctccgtgcaattcttaataaagatcacgacactttgatcaaaattcacgatcatccattggttgggcaatggcgtgggtatcgtgagtttcatcctgcacgcattggaaaggcgagtagtcaacttgataagtgggtcgtggtttatcaaatcgatagcgatgaattagtgcttatcttgattgaaacgggcaatcttaatgtgctgaaatgattcttcgcaaaacctttaaaacataaaaatgagctgtatctcctaatggtaattggaggtacagctcatttttagctggtcttggtgctattaagttggctcggaatgcataaggccgaaaaggtatttgactaatgctcaaagtctaaccaatttactacgcacactatccgttcacatgcccagcgaaacttggcataaacgcactactgatcgtctcaacatcgacgttctgtcctggttgcggtgcggccacaaattggttattgccgatatagatggcaacgtgatgcgtggcaccttcatcaccccagaataacaggtcgcccggttgtgcttcagagacagcttctttggtaacgtggctttcctgagtcacggtgtagtggccgaggctgatgccggctgctttttggtagacgtagtcggtcaaaccggagcagtccatgccttggagcgattcgccgccccagacgtaggggatgttctgggttgccagctgcttagccaggctaaccacggcatcggctcttgaatcattgctgttgaccgttgccttgggtgtgccggcatttggattgtaatagttggtgctggcttgttgattgtaagttgcgttggtgttgttataagtatctgcgctggcagttgtcgcaacgccacccataatggcaccggctaccgcaaagctcagaatgaatttcgtgaatttcaatgaagacacctcgttattagatttggtagggtcatcataagcccgcaacttttcaagaaggttacaggaattttgtggtctattgacgaaagatgtcaggctgaaatagtgttaaagatttggtagcgaaaggttaaagaattttctgggagcgttgactttgttgggtgagatccgctagaaatcattaaaatgaccaggttggtttataaaatatactcaaatctttatactttttactaaaattggtcaataccaccctaaaagtattgattatcagtaagaaaacgcttacactataaaataaatttaactggttactatacttttaacaaagagggaaatgtcatggaaaaaagtaggttcaaagtactcgcagaaacgggcatcatgtcgcggccggcaacccggttggtcatggctgcccaggaatatacatcagacgtcacgttaacgtacaacgaccgcacggtgaatctcaagtcaatcatgggtgtcatgtcactgggaattccccaggatagttacattgaaattgaaattaatggcgatgatgaaaaagaagcgatggcaggcatcgaggactacctccaaaaagaagagatcgtcgaaaaggtcaccatggacgcggacgcataacgtcgattaaaatccagcacttcaaatccagtggtcggacaatccagtttgtcgaccactttttatgtggcttcaaagactaaattccagtaatcaccgcactggattggtataataaatgcatactatattaaagaaaagagtgattcatttgaggggaaagcaaattgtgatcacagcgttaagcagcctgctggtactgggtaccgggctggcaatcagcgccgatcaagccaaagctgccgagaagaaatcggttgtcaacgtgacctttaagcccagcgatgagaacgagctgaccgactacgtttacaacacggttgatccaaccagcagccagtatcatcaatatttgacaccgagtgccttcgcagacaaattcggccagtcagacagttacatacaagcatttcaagattatttagccaaatatcacgtccaggcccaggcgtttcctggcaacctgtcgatgaaattgaccgggacttcgaccagcctgcagaaggctttcaaggcgaagtacgtgccagccaagaagaaggggtatcatccaaccacgtcctacaaattaccgggacagttgtccgataaggtggttgccgtgattggcctgtattcgacgaacccaaataagaagactaagaagacgaccaagaccgcaaccaaggccaagaagacgactaagaagtctgccacccacagtgacacgaccactttgtcgacgaccgacaccaagccgaacatcaagtacaccggcaatgccttctcgaagaagtacggtgctgccaaatttgccaaagcttaccaagtcgatgatttgtacgaccaaggccttgaagggtccggtcagcgcatcgggattatcaatgatagtgacgtgcgggatgccgacatgctgacctactggaagcaagccggcgttaacgacgacatcagccgggttcaccacatttacaccgtggcgacccaggctcaggctcaagctgatttgaataagtcaatcagtgccgctcagatggaggccactttggatgctcaatctgcttcagcgattgcgccagaggcccagatcgacctttatacagccgttcagtatggcaccaagacgactttgacatcagccttttacaacaacttcatgactgcagtctcagacaacaacgacaagcagatcaccaccagtatggcgccggcctttgaaaccaaatccaactggcctgacccaagtgcttcactgagccaatacagtcacgcatttaacctgctgttggaacaggcggccgttcaaggaatcaccgtcttcaaagccagcggcgaccgtggtccatatgcactttcaggtgccaaagagaaccacatcatgtccacttcaccatacgaagttgaagtcggcggaaccactttgccataccaaaagattatcgatggcaatctgatctccgtgaacaaggaacgggcttggggcgacacttactccagacctgcctatgacaccaaatacagcagcttcgccggtggtggcggtggcttctcagacatcaacccaaccccgagatatcaaatcggcgttccgggggttaatacctttagagccatgaactacctgaccttcaagaatggtaaatactcgatcactaagaatcctcacgtcatcacaggtaccaagactggccggaacctgcctgacgttgccggtaacgccgatccattgaccggttacgcttcaattgtttccggaccgaagtacacttttaaccctgagactaagaaggccaccaaggccaacggaattctgtggcggatcgatggcggaaccagcttcaccgcgccacaaatggccgctgctaatgcagttatgaatagtggccgccagacgccaatcggtttctggaacccacagatttacaagtacgcccaagaatccgacagtccatttaacgtccttgacgacgcggacttcaacgacaacttgtactacactggccaaccgggcaagctgtacaaccaggctactggacttggcacaatcaacttcaacaagctttataacaagttcaacaatgctaataattagcaatatgtaaggtcacaatgagtgctgagcttggtagcgacgagaactgaaccccttgaattggagaaatctaattcaaggggttttatattactatatcctgctcaccggatatataatcctgtcatcgtccaaactcgaggttatggattgcaagttagccaacttttgttttatcatcactttatcttaggttataattattctagacatagttaatgtaatcaagatttatatttttgctatgaaagacttatatggaaggttaagtgatggaacacttctttacgatcggattgccatattggccatctcacaagcaatatatttttaatcaatacgtggaacgtgaaattcaaaatgatgaatatgccttcagacagctgattgtcattttaacaaaaatgtctcagcttaaatatgatgttgataccggcattattgaaaagatggttaaggatcctaaggggcatttggtgtttagcacatacgttacggacaagtttggacggctggttaattcaaaaattatcgagttgcttaatcgtagtgataggccttgctatgaaattcggattaatgctgcatacgaaaaacgacgaatcttatttattacttctaggcctacactaagtgatccaaaagaacaccaacctggcggttattatattcattttggatttaccaaaagtgaattaacggatccggttcgtatgaatgaattgaccaatggcttagccagtgattcagtggacgttattactaaaattgaaaatcagcatttctctgaagacatttttagaagatggaaagtcgcaccatattctaggaaacatttggaaggaggagcccaataatgaacgatgagattagacaacgtaaacaaaactttcaggaactttttaattcagatcgtgtcaataatttcttgaattctgagtattttgagctttcccagcaaatcatgaatcttgaacatgaattaaagcttgaccaaaaacaaaccgctaatgttttggggatgtcgttacaactttttctgcagtttgaaatgggtgtctcgactgatgtgcacgcataccactctattattagaaggttaaatcaagcaaaagaccagcaaaaagatgatttggatttaacagtcgtaatccgcaattctcagtcactctctgattcagttactgttcctgttaaagatctgggttcacaggcggctaatgagtctgtatccgcttcgtctaagagtgtcagctttgatagtagttctgagaaagtgacatctttgaccggctggaggtaatgaatgaaatttcgttataataactatagaattaacaatctacaatataagattaaccccgaagcggaccagaagagagtgaccagcccttcagactattcagaggtcggacaaacttctttgagtaacacgcatttgcgaatttcaaaagaagacgccaacattctctttacctctaccgtcaaagttcagactcagttaaatgacgaagaaaagaccaattatcgatcggtattatttgacttgatgatgacctttttaattgaggatagtgaagttagcagtgagcatgacatttttgaaatgtctcgcgaactggtcatggccgtcgtgtctgcgcgagttaaagagattgttagacaaatatcgctgttggattatttaccggcaatttcgattcagtcattttcttttcccgactcgtttgaatttgagaaggataaaaggaatccttagtcggtggcgggatgcaagtatcatcttgtaatcgatcatgtgagaatgttgccggaatcattaaagaagggggatgtgagacacatgcaaaatgaagatcacagtaaaattgatcgcaaacaattagcagaaatcgtgccggacctgaccaacgttatcagtgaccctgacggcaccttctcagtctttgactggggtcacggggaaatcattggggttatccagcaccaccaggattatcctgacacggcgcttgaagaagtcttaaccggtgccgtcccatccggtctgggttattcctacgacccggtggacgagacccacttccaagttgacggcaaagaccgccgattggagaagggcatcatcgcctcgagaaacgctgccgtcttggtcgcgccggatgtgccggaaggaattctcgattacttgggcattgacatgattaataccctccagataccaggcgttcattatgagtacccggatatcttggattaagcgcaactaaaaagtctagcgtcaccttcgattgaataaagtgaacccttaaaattggacaactttattaagctgctttctggacggtaagttcccggtattttaccggggacttgccgtccagttttgttttgatgcgccgatgattgtagaagtctatccattcgttcatagcttcgataagcgctgttttggtctcaaaatgttcatccataacctcgactttcataatgtgaaaaaacgactccatggcggcgttgtcgagacaagtggctttacgcgacatactctgaaatacatggtgctctttaagcgtgtcttgccagtggcgatgctgatactgaaacccttggtcagtatggacggttgtccgataatctaacaccggtattcgatttagggcttctttcaaaggttttaaagcaaattcaacggtcgggtggtcactgatattgaaagccagaacctctccattgaagaggtcgaggactggttctaaataaacccgttcattttgactttggttcccatatcggaattcactgacgtcggtgactaacttctggtaaggccgatctgttttgaatcgtcgcttaagtcgatttggggcgatgacgccaacagttcccttgtaagaattatactttcgtttctgccgattaaaggcgccacatagccagtcttgttcccgcataatccgtaagacccgcttatgattgattttaaagccataagcgtcatgtaaagcaccggttattcgtcggtacccgtatttccgagtatattttggatcttgttgacgaatctcatcaattgcctgaataatttgtgaatcatctaagttacgaccacgatgctccttagcataataatacgtgctacggggaatacgaacagccttaagaactagtttgatggaaacttgaaaattctgccttaactcgtctactagttcgatgagttcgtgtgttttgacttctttcgtgctaaggcatcgagtttttttaagaattcattttctatttttaacatttgattctcttgttttagctgcttcaattctgcggctggagtctgtggtttttcaggtttggggttgttctgcttgtgtttgaccatggtcttaggattccctcgtttgcgctcaagtcccgctattccagattcctggaagtgtttttcccactgccaaatcgtacttggcgacgacaagtcaaagtgtaaggcagtcactggaagcgaagcttgatttcgtttcttccagtttaatacatcgactttgaactgactagaatattcttgggacattgaccggtcttttagaccttcaatacctcgccgctcaaatcgatgaacccagtccagaatgattgaatgattgctaatgcgatacttcttagctagagacggtgaacctttaccagataagtattcagtaacgacctttattcgaagttctaaattaaattttgacatagtaaaacccccaaggttagatttggtgtccaaccttaggggttcactttagaattcgaatggtggcgctagacttttttgattgatgactcagaaatcagtggggaatgttattcaatcatcgtcggcaccttccccatggcagccaacaccttcaccaaatcagcgtaagacatcaaaatcgtcgccgtgttgacattcggatgagcagagatttccggcatcgattccagtgacttattaatcagtactttcacctggtcgtccgtgtcgtgcatcaatgccagtggggtgaccataccggagacgacgccgagcagggattccaattcttcctcgctggcgaatttcagccggctgtggcccaaccccagttgctcagccaacgacttaaagtcgacccggtgattgtcgaccagatacaaatagaactgatcggacttgcgatccttcagcagcagattcttcacctcaggtaggccttggggtgcattgggatcatccatcgtccaaatggcagggtggtccacccgccgatagtgcacgccaacctgtgccaacaaatccaatgcttcttgttccgtcgccattttcatccaatcacctcgttgaatacatattatacgcaaaagttgctaaaagtttgcgttttagcgaaaagtcgccagcactgaacacagccaaatcccacaaacccaggattaccaggcactaagccgcctaaatctcccacgttgttccgccatcaccttccatctatactcattgcttgtgacattggccaatggatcaccaatctaatcaaaggtggattcatgatgaaacgtaacaacaagcaaatcgaattgtaccaagatgcatttgacttcctattagacggcgaccatgagctggtggtctatggggtgctgaagaagctgcatatctccaagcaaaatacctactatgatgacatggttcaagaagggatgctttcttttgttgaaaaatatattcgagccatcaacctggaaaaagagcctgaatcatacctggcttacatctatcgcggcgtgtattgggatctaatcaattatctgcacaaacaaatcacgatcaccgagcatgttgaagtgccggatgacaatgttgatccgctggcagaactgcctgatgggaaaaattctgcaagctactatgacacgcatattctatcaagacagctaatgacggagttgaacccaaaggaaatcaaatatttggtacttgcttatgattatgggatgaatatctcagagattgctaaagaatgtggtgtcagtcgaaagtgcgtgcacgcttggcggaagcgggttattaacaagcttcaaaaaaacttttgaaaaaaggtaacacttttgggggttcattttgttagtaatagtgtaagggttggcgccaacgacttacaaattaagcagaatagaggagaaagacaatgcaaaaagattggatgaaatcaaatgttacctatacgttggttaatgaggatcacaagaagggcgttaagcactcttttgcgtatgttactcaaaatgtaactgcagaaaaagtggccgctttcggtaagatccttgaaagcctgatcgacggtaacatcactgacgcagccgtatcttcaaccgaccacgttgaattaagcgacgcaccaaaagcaccggccgcacctcaagcaccacaagcgtaatcatcactgactaataggaggaaacacagatgcgtaaattagaattggtattcaagacttcagacgagaagcttaagaccctgtccatcaactatgccaacggggaattaaccggcgacactgtcaacaaagcgatgactgaaatcgctaaactcaagatgtttgaccgcgacggcatcgatccatacgccacaccaatcgccgctcagtatcgtaagactgagatcgacaagttgttcgacactcgcggagaataattgcataagggtaattagctacggttaccgacaaggccgacaatgggaaattttcccgttgtcggcctttttgtgcattttttactaaatgtagaaaccaaggaactcacttacaaaaagttactgacaaacgcctgcatgatgcttaacggcggtacttgtgttacagaattgttgcaactatttcaattaaaagttttcagtacaattatgttgcgatatcagttataagaagctattattaggactgtagaaagtttaggttagctctgcttgaagcacctcttgttatggggtagactaagggtacgggttacataaacctagtgaactacaaaatattttattcatattggaggagacgcaataatgatttcttcaagcttgatttcattatcttgtctcctccaatataatatgatttgtagttcactaggtatatgtaaactgcagtccgcgttcctgaccccttgtggtgtatcagatacaagagtaaaatcgggcggaagggtggttcatgccatcccgcaccgtcctgcgtttacttacttatgtgaagcgtgttacaagatcttaatattctgtttctctgcttataacaaaataaggagggttctgcggtataatataactgtactaaatatgaatgtggaggggtattatacatgaaattgaatgttaagaaatcattattcgtatcaatcgcagcgcttggcttgtttgctgcagcggggactacaactgccaatgccaagaagaagtcatatccaacaactaaggttaaccgtgttttgaagaccaacccatatgatagaaacgttgttttcactggtaccaatgctttgtataacaagatgggaaccttgaagggtgctcgtgtggttgccactaagtcgaccatcaaagatctcatcaatgcccgtcaatcaaagaacaacttgcgggcttatcgttacggcgttaccagcaagggatccgtttactacaaggtagtttcctttgacggccaataccgtggctgggtatacggtggcaagagtaccagcaactttgctggcggcatcaagccaaccacgacctttactgaaggcactttgagccaaactcaaaaggacaccatctaccgcattaccaccccaggcattgccaacgatggtagaagcgcaacttacatggatccaatgtacacgcaatacaaattgaaccatgacgaccgttaagtggataacaccactaactacggcgaagcaagattccgtcttgaccgaatcggtactcggactcaggaaggcgatacttgggtatacatcgtcgcaactgatccggcctacaccgttgtcaacggctggatcaagctggatggtttgactgcaactggtactattacaaatcaataaaaatctgatattatgaatccccattccagctctgattggaacggggattttgcttttttgaaatatcttgagacgaattaatattcaggtagtacgcacttctttttatgtggaagtatttttgactggatactatttgagcttacgttacaagcccttttagttaaatttctccataaatatttattcatattctattgtgcttttgataatgctaatatacaatctagttagctagtgaacgaatcacatttaaacgatcattcaaggaggagtcgcaattgaatttgaaatctggaagggctttaaagctatctttgatggcttgtggttttaccatacttgtggggacagcaagtatgcaggcagtgagtgccaagagttatgatcatgtggtgtcaaacagcgtcatgacaacaccttcaaccagtcgcaatgtcaactttaccgggatctatccgctgtataataaaccagctgatgtcaagggtgcccgcgtggttgccacggcggcgacactggaccgattagccaacgccaacgtttcaaccgataacgttcgtgcctatcgggtggccgaaaccaatagcggatctgtctattataaggtagtcacatttgacggccagtaccgcggttggatttacggcggcaagaacaaagccagctttaatggtggggtcaccgcctatacgactttcgccagccaaaacttgtcagctgttcaacaaggatcaacgtataaaatcgctaatcctgggacggccaatgatggcaagaccgtgacttatcaatctcctgagtggacgcaatataagatgggccgggcaatcaccgactcaacgccttatgctaaatcagttttcaaaattgaccaaaccggtacgcggacccgtgaaaatgatcaatgggttcacattaccgatgtcaccaatgccaattcgcctgctaatggttggatcttgatgagcggcttgactcaagtcagcacaccggttgctgacaatgcgattcgggttaatttggttgatccggataacaattcgagtgtcattaaatcatttgacgtcactcgatcagccgcccaaaagggaaccaactttggttacaataccaacggcacctggacgattagcaccaatgatcaagacacaattcaaaatcaaatcagaactgcattgaatgggaccaactacggcttggaaggcttgagtgctgcccaacttgctcaggttgcccaaactcaatttggcagttcggttaacttagtggttaagaaagccgatccaattgcggataatgccgttcggatcaactttgtcaaacctgatgatacgatttacaaatcagttgattggaccaagaccggcgttgtgaaaggcaacaatctcggttatcaattaagcggcaacagcgcttggggattatcctcagctgacctcgcagccattcaagacaaaattaatggggcactggggactggctcgacttatgagctgaacgccggcaataataccttgaccagcggcgaaatcgacaccatcgcccacggccaatttggcggtcaaatctacttgaacgtctctgccgttaagaatcaagttggcgcaatccagccgtacgcattcaaaattgatgcggacttgagcaccttcaccagtttgtccggagctgctcaagcagtgttggatctgacttcgccaagtgctttgacggcggttgatggtcagtattcaacaactgcagtcacatctgctaaaggaccggatagcggcaagacctacagcatgtctgcagcccaagccgctcagaatccactgttgctggaaacttggtttgtggccaataatattgacgctactgatcaaaaggcgattaccagcagtttgatttctgccatgaaagctcaagcacgcaaagaatttatcagcaccaatgtgaactttgcggacttcaccggccttccgggaactgcctttaccagctctagtgtgatgacttatctcaatggtcataatgccaacgttctgcattcaaccaaatatccagttgcttactcagctccgggtgtcttggctgtgaccgatcagacgacttacgttgctaccagcgctgatgccggaacctatggtaaagctgccaaggcatactatgcttatgcagatattaatttaataccataagtcttgtagacaattatttaaacattcgaaacaattgagaggtagctgatagtgacgccccaacattgtttttaacagaaaggcgattcaccaggagaaagatttcttggtgaatcgctttttagatagccgatcgaattgtatgtacatatgtatcgccgcaaagaatatgttggtatatacttttcgtgaaaagaaatatggaggcgatgactgtgagtaagattgtagcattacgaaaagctgggaatagtcgagttttgacggtccctacagacttggacgcaaatattgggacaaagtatgaggttcaagtcttggataacggtaatgtcgtattcacccctgtgacgcacaaaaatatttttgacgatcctgaatggaaaaactatgattaccagaaggatttagaagaaaatcctgaactgcaaccacttaatcctgttgggaaggagcggtttgaataatgagatttccggagcaaagagatgttgtcgtgattgacgccgagccacattctggacgggagtacggtggtcataacaagcaagcaggccggcaatattcgcagatatattgcactgtggcagttgcagaactatgactttaattcacggaacggaaaaattgttaatcagattccagaacaaacttataagaaattagttccatacgtgaaagatatgcttggctttagctaacattcaaaagctcatattctacacccaccatatgagaagcggtaaaatatacgtgggtcaagaaatagattattaggaggggaatcacatcatgaaaatgaatttaaagaagtcattatttgtttcaatggcagctttaggcttggtatctgcagcgggggttgcaaccagccagactgccagcgccaagacttatgcgaaagtcaccatgaattcagttttgaattctgatccaacgactcgaaacgttaccttaactggaaccaatgctttgtataacaaggctggtactttgcgcggggcgcgagtcgttgcatccaaggcgaccgtttctaatttagccaacgctaacgtgtcaaccgctaacttccgagtctatcgggttgccacaaccaaccggggttcggtctactacaaagttgtttcatttgaccagaacttccgtggctggatctatggcggcaagagtactggcagcttcgccggtggggttgggccttacacgacatttacgtcaaccacgccaaccagccagcagaccagcacgacttacaagattactaatccaggtaccggcgacgacgctgtgacctgggattcaccacaatatacccaatacaaagtcggcaagacgatcactgattcaacgccttatgccaacgccactttcaagattgaccaaagtggttatcgaactcgtgaaggcagcaatgatgtttgggttcacattacttcgacaaccccagctaacacggttgccaatggctggatcaaatttagttcattaacaccggtgtcaacccaacaagctgacaacgcagttcgaattaatttgactgaccaaagcggcaagaccatcaagacggttgactacacggttcaaaatgccgtcaagggaactacgctggggacttattcatcaacctctggcctgtggactttgactgatcagactgctaacgacattgttaaccaactgaattccaacttggttaacaccggttaccgccttgaatccagcaatttgaacacggttcagcgggctgctttagcggctgctcaatttggcaccggcacggttaacattcccgttgtcagcaccgcaaccaacacggcttacagtacgattacaccatacgcaaccaacagtaataatgtttcaaatgggacgcgtgctttgactgctgttaataatggggttgttaacatgggtgccaactttgtggataccaatccaaacgtggatggtaaccaaggcggttatctatcagctagtgactttaacaacttcacatctgctcaacaacagaccattttgaatgcgatgactaaagccttcactaacgatccaaataactatgggccaacatacctgaccaacttgaacaatacgtttaagtcagctgctgaaggtcaatatgtggcaccatccaacttgaacttcaccaatggtaacgcagcaaatggctcaacgtttaccggcgatcaactgatgagttacatcagaagtaatccaagcttgatgactctgcaatcaccgaagtacccgcaatttgttgtgccggcatcttcaggtaataccattcaagttgtttggaacacgattaactacacggcaaacaatgcttacaatggcacgattggccagcctgtgaatgtgtactacactttcactgattaaaaatcagagtgagaaaaaagacgctttgattccagagtataagaaggtccccaccagatgcttgttcctaagcatctggtggggactttcttatacggccggaatcagtcttttttcgcaggtttcggctaggaagcatcaaagcaaaaaccaaatataaacaaaccaaccacaaactaaaatcaatccaactaccaagtagtcattgagcgaccaccaaatcaaagtgagatcaaaaaaacacccaacttccaacacgataactgttttgtcaccccaacataaggtaaaatagcggtgaacgatacccaaggggagggatattatgctagattacaagaatcaagcaaagtggccgaatggttttggcagccagcagtcaccaatcgaaattaagacagctcagacattgaagtcaaaagagccgttggactaccatgttgtgagcgactatcaattgcatcaagaagtggatgatgggacaaccgtccgcctgaccggtgagggggcagcacggatttttaatcgcgagtatcactttgtccaggttcatttccacgcgccatccgagcacgtgattgacggcaagcactacccactggagattcacttggtacaccaaaatgacattggccaattagtcgtcgtggccttgctggtttccgccggtgaattggacgatgaaaagctccagcagattatgacgacttatgaaaatggaaagaccgaaccggttgatctgaacatcagcgattgggcgccatggtatccggtgggcttccattatttaggatcgttgacgacaccgccgttgactgaaggagttgagtggctcgttttgaccaatcctgaatttaccattagcgatcgccaaatcgactggttccatcaacattttggcgatgataatcgagacccacagccgttaaatgatcggcaggttgaactttacaaatagtgcatcagttccgtaatgaaaacgtcatcaaacaataacggccttttcttgaaccccctaaattactcatatataataaagatgtgtagataatcagatattattgggcttatttaaggaggggttctacatgagatttgatcttaagagatctttgttcctatcattggctgcattaggtttcatcgcagctgcaggaactgttaatgctcaaaatgccagtgccaaaacttatgcacacgttgtctccagcgagaagatggcaatggcaccacagaaccgtaatgtgaactttacggggactaatgctttgtataccaaggctggaacattgaaaggtgctcgagtcgttgcttccaaagctactttgagcagtatcgccaactcgaatgtctccactaacaacgttcgtgcttatcgaattgccgttaccaaccgtggctcgatttattataaagtcgttacctttaacggccaataccgtggctggatttacggtggtaaagatgattctgactttgccgggggaattacacactacaccacatttaacaaccaaagcctttcaagcttaaccacggctcagcaaaacgccacatataagattgccaatccaggaactgccaatgatggcaagacagtgacctacaagtcaccggcctggacacaatacaaggttggccgtgcgattactgattcaacgccttacgccaacagcgtcttcaagattgaccaagtgggtacgcgaactcgtgagaacgatcaatgggttcacatctatgacgttaacaacgctaactcacctgccaatggctggatcttgatgagcggattggctacgacacaagcgccaatcgctgataacgccattcaaattaacttggttgacccaaccaataactccaatgtcgttaagtcagtgacgatcactagaagcggcgctcaaaagggtaccaacttcggttactactcaaacggcagctggacgatgagtcaatctgatatttcaagcattcaaaaccaaatcagagctgctcttaacggcaccagttatggtcttgacagcttgagtaccgcacaaattgcgcaaattgcccagactaactttggtagttcaaccaacttggttgtgaacaagattgctaatatcgcggacaacgcggttcgaattaaccttgttaaacctgacggcacaactttgaagtacaccgactgggttaagagcggtgccaacaaaggtagtaacgttgggttccagccaagtggtaacacactttggtcactgtattcaggcgatcagacttctattcaaaactagattaattctgctttgagtgggactaacttccagttgtctggtaatgctttgactagtgctcagatggatacgattgctcgtgggacttatggtggacaggtttatattagtgttgttcctgtagcaagtgctataagtacaattacaccgtatgtttatacagatgggaatagcaagtcactgaattcagtaaacgggaatgctgttacaacgaagctccaactggatcacactactaaaccatttaatgatgttccaagcaacgttacaagagatattgctcagcaggttgttgattattatgtaggtaccgccgcagctggtgcttccgacactgacaagcgcaatcttgccattgatggaatcaattatgtaaataagcagatttacgatgctgcacttaatgaatatacgtcaagtaatctagacttcaatgtctttaagggccaaagcgggcagcaatggactatagctgacctgactggtacattatttgctaataatttgtggactattcactcaccaagttttccactgttcactgtggacgcacaaaaccatgttcccgattctacaacaacaaatatatcctattcgtttgacagtgttcatactggactcatgggattaaccggcacctttggtaacccagctaaagctgtttatgatccttctgctgttactcagttaccacacgttaccgctccaactaagtaaaatatgtattttgatgcgagaagcaagttgcctttaaagggacttgctttttttgttatttggattaatttcattgtcatattctccagaccgcaaaattgcctcccaaaacatacctcctttataatgaaaatgtacctaaggagtagataaatgttaagttttgtaaaggaggagtacttttatgacgtctaatctcaagaaatctttattcgtgtcattggctgctttaggatttattgcagccgcggggacggcaaccgcccaatccgcaaacgccaaaagctatgctcgggtgacttccaaccagaagatgaccagcgccccaaccagtcggaacgttaactttaccggctcaaacgccttatacaccaaggcaggtacgctgcgaggtgccaagaaggtggcttcaacgaccacggttcgcaagctggctaactccaagaactcgcagaacaacatccgggcataccgggtggcgaccaccaaccgtggatcggtttactacaaggtagttacctatgatggcgcctaccgtggttggatttacggtgggaaagttcaatccgtctttggtggcggcgtgacctcgtttgacacgtttaaaaatcaaaacctgtccagcctgactgacacccagcagaaagccacttacaagattgccagtccgggaaccgctaacgatggcaagacggtgacttacaagcagccggcatggacacaatacaaggttggccgggcgattaccgattcatcgccgtatgccaacaacactttcaagattgaccaagtcggaaccagaactcgtgaaggcgaccagtgggtgcacatcactgataccgggaacgccaattcacctgcgaatggctggattctgtacagcggcttgaagcaggccgaagcaccgattgccgacaacgcaatccagattaatttggttgaccctaacaataacaacaaggtgatcaaatcaatcacggtgactcgggacggcgccaagaaggggaccaactttgggtacaacgataacggcaactggaccatcagcatgtccgaccgtgccagcctcttgaaccagattcgggatgctttgaacgggacgagctaaacactggatacgttgacgacggctcagattgcccagattgcgcaaaccaattttggtagctcagtgaacatctcggtgaacgcggtgaccaacattgctgacaacgcgctgagaattaatttccgcaaaccggatggcacttcgctgaagacaattgattttgttaaaggcggggcgactaaggggagtaccgttggttcagccgtgagtggcagtaccaactggactttaagtgatagtgacaaacaaacaattcagggacagatcaacacagccttgaataactcaggttatcaactttccggtggaaatacactgagcgatagccagattgataccattgcccgcggacaatatggtgggcaggtttatctgaatgtggtgccgatttcaaatggaattagtacaatcaatccatatggaaaacagaaggacgcaaatgataacactgctcaggccttaaagggagtgtccggattatacagtactacgccaaatggatattccattccaagtgacgttggaaatgataaatttgttgacaatccaacagcgaatggtgcggcaactcctaccaacagaactttcaatgttacggcagctcagttggctgataaggacggaactgacttgctgactaacttcttaagtggtattaaggatgacaatgttcgactagctgcatataacgggattactgaaacttatttagatcaagctaagacacaatttatttcgaccggtcttaactttgacgaatttagtggaaatcctggcgccaaatttactggcgagactgcctttgaatatgtgaaccattcagcgcttaacacgttgaaatctgtcaagattccagtattttctccggatggggaccattctcaaactccagtacagaatgctgataagtgggtccagtatacattccagtcttataaggcggacgatggaacatatggaactccagttaaagcatattaccagtatgatcagccatcctaacgactgatatccaaggtataagtagagtaaagccactttaggctttgctctattttgatattaattaacgacacactaaaacactttttctcccaattttaatccttttaatcaatttgtaagttgaaacatacgttcgtacttggtatgattgatatcactaacagacatgattttgggggtgccgacatggccgaggcaacactttaccatgcgacatcgcatgcgaatgcagggaagattttacgagaggggtttaggataccacagaatgactggggacatttttatgcaggcagtcacttcaagcagcctggaagtttggggtatgggacgtatggattcttggaggataaacaattagccggcgagttttgggcgtctatgtacaaatcactatcgagatatgatattatgagagtcgaaattgagtatcggattggaaatagtctcaattttgtcgacaatttagaagacatgaagtatttccgtgaatttcttaaagacccattcttccacagtggtatcaataatctacacacacggtttaaaaatacgtttagacagcatgctttggatggcgcactaattgaatactatattaagaatgcaatccagcgagggtggtttcatcaaattgactgtgtctgttgtgcgacttcaactaatgtttacgataggatgaatattttccttcctaatggcatcgaatattgtattcgaaataaggatattattactaggatcagcattcggagtgattgaaatggcggaatatctaaagagtcatgatgaattactaaaaattgtaaatcaggctgcaaaggacttaagacctgaagatctaattccatatcttcaagctgctgaaaaatgggacgattctaaggacacattctttgatgaggatttagatgagtctgacaaggtaaacagataggagctaaatatggcaaagtatttaaaaagtgaagaagaaattctaaaggatattcaccaaatggctaaggatttaagacctgaagacctaatcccatacctggaagctgcagaagactgggagaagaaccaccgcgatgaatttgattttgttcaagacatcgacaaaccaaaagaaaccaagtcttcgaaataatttgctcaagcaaataggacaccccacgaatgggatgccctattttgatacataagctgttttagccaacgcggctagtgccagttttgtaattgattttgacgccggcttggatatttttgatataaatattgaaatgaacttggttgctgccaaccgatttaccttgcatttgaacaccgcgggcaagcaggtcgtgacctttgaacactggtcttacctggtaccgaatgtaatgtttgtaactcccgcggagatagtaggcaacttggttttcatatttcagcatgcatggcgtgttgagtgatctggttccagtaatcagattcttggggttgttgttttgcccagttaactggtagccgatcaagtgacaacggttatacaaccagcctcccttgatccgcttgttgtgccagccggttggatcgaagtacagtggttcgcgctgcccggttggcattaacttcttgtttagtagggcattggcggtggttgcccgattcaagaaatcaagattgccatatcgctgccaagcaccatgccgacgggaaagggtactctgggaaaactttggtcgattgtgattaatgatcacaatttgtttcccgctgactcgaattggtttgttgctggtctttttagcctttttcctcgcttggttggcgcgcttgcgggtaaccttgcgcttgtgtgggttgtagtcagttttagctaacgttaaaccccgtttcctggcagttgaaagcttcacccgatagactttctttgcccggttcagcccccggttatgccggtgataaaaatagtgtttccccgttttagtcacgtaaacgtacgttgcagctgacgttgtcgtcggttgggaatagctgacgccgccgaccatcatgaccgttaacaggaaacagtagatgattttcttcataacttcactcctcaaataattgctgtgatctagtgaacattctttattctatcattaatttgttgaagaaaataatcttgaatctcgtatatttaactcactttaaatgcttgtgaaaagcgttaaaaatagatggaataccacccttaactactgtaaaataataaccgttacaaataagaattttgaggagaattttatgaacttgagggtaaaaagatctatctttttgagtgtcgccattttaggcctcactgttgctggaggctcgctaatggggcaaagtgcgagtgctaagacttacgcgaagattgccagcaatgaaacgctgacgattccggtaagcagccggaatgtcaatttcactggcactaaggctttgtacaccaaggtcgggacattaagaggcgctcgggtagttgcgacgaggtctactttgagaagtctagccagttctaaggactccagagataacgttcgcacttatcgtgttgcggttaccaacagaggctccgtttactacaaggttgtgacctttgatggtcaataccggggttggatatacggtggcaagagtacaggtaattttagtggtggcgttaccaaatacgcgactttcaacaaccagggactgtcagctttaacgacagctcagcagaatgccacatataaaatcaccactccaggaactgcaaataatggcaaatctgtcacctataaagcaccatcatggacgcagtacaaagtcggtcgagcaattacagattcgagtccttatgccaacaccaatttcaaaattgatcaagtcggcactcgaacacgtgagaacgatcagtgggtccacatttatgatccaaacaacagtaactcgcctgcagccggttggattctgatgagtggactgacgcagaaccaagtgattgtcaatcctgatgccaaaaacttaaccatcaatttgattaagcccgacggcacaactttcaagacaatcaagtggacgactgcaaccgcagttgccggacagactgtggggacatcccaaagcaataatgcccaatggatcttgaacagtaatgatcaagcggacatccaaactcaaattaacacgcagttgtctggaagtagctatcagattgcagataacaagctttcggccagccaaattgacaacatcgctcgtggaacgtttggtggccaagttaacattcagctgactgccgtcaacacgacagttcccagtataatcaatccccaaattgccattgatggtaattttcgcgaaatggaaccgttgactggggtagacagcgagtatggcacggcaaaagttacttttaagcttggtgatcagtctaaagaaattcaattgagcgctggtgacgttgctgcacaaaaggagagcgataaggacagcctggtttaccaactcaaacacatggatggcacagccagaaaagctgccgtggaacaaataaatgctgatttctacaatgccgcaatcaaacaatattcgtcaaaaggtgttgttttggataaatttgttggcacaaagggatcaacctattcagcggctgaattgggaacatacttgaacgataatctaagtacgctgacgactcctaaatacccaagtttcgatgccgatggtaatgtgacttataagaccgttaccttacacctgttgatgggcgacatttttggtggaacatatgggacgcccactggcgctttatatgtatgtgacgcgtacaaacctgaggcttaggaaattgcacaaatcattatcagtacaccgctttttactttactaaacagttatcttcacaaaatcttcacactttatacacacaatatacacatttaaaagtaccaattttcatcaagtaatacgccttaccccacgtaaacactggggcgaggcgttttcatttgtccgtataaatgtgacttttctgtgaaggtttcgctcaaatatacatttttcttcatatctgtgatattcttctagcagtgaaaaattactgggcaattaaacgtttttgccaagtttagtaattttgtttcacttcttgtttagcgcgctcaaactagatgactatctgttacacaattggaggaatggaatttgaagaacaatttgaaaaaatcactttttgtggggattgctgctttaggcttcgtggccgttgccggaactgccaatgccacacaagcaagtgctaaaacatacgccaaggtaacctctaacaaggcattatctggcgatgcaacaactcgtaacgtcaactttaccggtgacgcagctttatacactaaagccggcactgttaaaggcgcaaaagttgtcgcaggtaagactacattaggaactttcgctgacagcaagagctcacaacacaatgttcgcgcataccgtgttgcaaccactaatcgcggctcagtttactacaaggtcgtttcgtttgacggccaataccgtggctgggtatacggcggcaagtcagcaactgcatttggcggtggtgttgaatcatacagcactaccactgatcctgcagcaactactgacacaacttcttcagcttcatcagcatcttcagcaacttcaaccagcaccagcaaccaaaccaatggtttaactgctgatcaaaaagctgttacttacaagattgccagtgttggtacttcaaacgatggtactcaagtaacttacacttaccctgcatggacgcaatacaagaagggccgcgttatcaccgactctactccatacaaggacgcaactttcaaggttactgaccaaaccactcgtactcgcgaaggcgacttatgggttaagatcgaagcaaccgattcaaagaacagcaaggccaatggctggatcaagtacagcggtttgactaagaccactgataccactccttcaactgactttgatgccaacaagagtgttaagattaacttccgtgacacgactactggtaagacgttagacaagagtgctacttggaccactgcctcaactaacactaagcaaggtgactcagttgccagcttggttaacaatggtggttacaacttggctgactacatcaacaatcagttaaccgcaccaactggatattcatttgccagcaacaagaacatcacacctgatgtcacaactgctaagtttggtgatactttgactgttgacgttacaccagctgctaaagctgcccttaaagttgccttctattcagaagatgcacctagtggtactttaactgctttgaagtcatcagactttgcttttggttacccagcattgacgccggatgctcaaacaaatgcacttggcaagacaactgatacttcatttaatttgaatgatttctttggtgatgccggtaccaagaacgccaaatttgtaacagaatttgacaaagccgttaatgccgcaactgcaaaagcaggcaagttatcaaatgtttctggtactcaaacaactggcactgacaaagttggtttctttggccaatcattaaacaatggtactcaacgttacttctacgtatttaactccgctgatactcttgctaacaatgctgcatcacaatcaaagggcgcaactgttaaggttgttctccaacgttatgtaaccaacttgccacaacctaatgaagcaactaaggatgctaaggcaaacacagattacatcgcacaataatcaatagataacactttccaaacacacatccatttcggattcataacacagcacaactctacaagtaaataaagggggatcggacgaggaagcttgtccgtcctcctttacttttccaaagtttcatccaatatgatataaaatatgatttgtagtcgcatattcaatcaagcggtttatgcgagtggctgaagtacttcaagcatactttggccgaaaacagagtacatgaggggccgaggacaaacggaaattgtcttcggcccttcgtgtacccgatacatactgatttctcttcaacatttttgaaaggttggctccccatttcctgattacaatgacaaacttaaatagaccttaaaatgtgaataatttaagaatatctattcacttttgttgcattgttttattcatgtcatattcatgaaacaacttaagaaatttgttcaggtagcgtaatttcactgttcctataacaagctatactagatgtattctttgttaaggaggaatggaaattgaataaaaatttaaaaagatccatttatacaggaattgctgctttaagttttgttgcagttgctggaacggctaacgcgacttctgcgagtgccaagtcgtacgctaaggtgacatcgaacaaagccttaacgactgacgcaaccactcgtaacgtcaacgttaacggcaccaacgcactgtataccaaagcgggtactttgaagggcgccaagacagtggctaccaaaggcactttgtcgaatttatcgacttcaaagagcagtgaaaagaactggcgcgcttaccgtgttgccactactaaccggggatccgtctactacaagattgtttcatatgacggcaactatcgaggctggatttacggcggcaagtcaacaacggcctttggcggcggtgtaaaagcctataacaccaccactgatccatcggcttcaactgacaccagctcatcgtcgtcagcatcctcgtactcgacgacttcagcccaggctagtcaaacaactgctttgactgccgcacaaaaggctgccacttacaagatcgctaaccctggcaccaccaatgatggcaccgaggtaacttacagctatcctgcatggactcagtacaagaagggccgggtcatcactgactcaacgccttataaggacgcaaccttcaaggtgactgatgaaaccacacggactcgtgaaggcgacttatgggttaagatcgaagccactgattcagccaacagcaaggccaatggttggattaaatacagcggtttaacgactgctacaacgaccccaacgtcaaccttcgacgccgacaccagtgtcaagattgcctaccgtgatgtttccaccggcaagaccttgtccaccaccaacacttggaccacttcatcaactggtaccaaggaaggcaacagtgcggtgaactacacggatgccaagggtcaaaccatcggcaagttcatttacgctgaaggggccccttctggttacaagatcaacactactgataataaagatcttgcatcagacggcagcaacgccaccgttgccccagctttgtccagcgccaaatttggatcaactttaacagttgatgtgactccagttgcttcacagactaaggttaaatttgacgttgccggcacaactggcactgccaactcagcattatcatcgagtgacttcctctatggtttcccagctctgaccgcttcagctcaatcagatgctttaccagctggtggtgctactaatggaaccttcaccgttgccgattacttcggcacgaatggtaagttcaccaaggcattgaacagcactagttcatccaacagtgtccaaaccatttaccgcaacagtgatatttgggatgtgaacggtaatgaagtagccacgactggcttaaccggcttctttggtcaaactgactcaagcaagtccacggcttcagctccagcacactacttctatgtctacaacccaaccaagaccctggcagccaacgcatcaaccttggctaatggatcagcggttaccctggtgttcgataagtattcaaccaacacgacaccaaacgcactcaactctgatttgaacgccaacacagactacgtttcaaaataagttcattgcgtcacttccaataagagacatacgccaacatcgtatggatcattaaaactgcattcttcaaactagtccaaaaggggggatttagacgatgcgactcgtctgccctccttttgtgtgaacaattcttttcaatataatatggtaaagtttgcgccacggaaatttgtggttcaagccggagtgaagggatgcctcaagctcatttcttcataaaaggttctgagataaacgatccgattctgtcgggtcgtttatttttgtcctaaatctttgggtggcctttcaaaagatgatatacttgaagaggttaggtggtcgttggacttaatgaaccagaattttttaggttcaatcgactagcctttgcttaattcttaacatattggaggaatgtcatttgaaaaatactttgaaaaagtctcttttcgtgggggttgctgcattaggacttgtcgcagctgttgggactgctaacgcaacttcagcaagtgccaaatcatatgcgaaagtaacttctaacaaagctcttgggggtgacgctactactcgtaacgttaactttaccggtaagagtgcattatataccaaggctggtactttacgtggtgcccgagtgaaagccagcaaggctgttttaagcagcttcgctaactcaaagagctcacaacacaacgttcgtgcttaccgtgtcgctaccaccaaccgtggttccgtctattacaaggttgtctcatttgatggtgcttaccgtggctggatctacggcggcaaatcaactggtgcatttggcggtggtgttgcgcaatacaacacaaccactgatccacaagcatcaactgataccagttcatcagtgaactcaagtgcctcaattaacactcaaggccaaacaactggtttgagtgctactcaaaaggctgcaacctataagattgccaaccctggtacttcaaacgatggtactgaagtaacttatacttacccagcatggactcaatacaagaagggccgggtaattaccgactcaacaccttataaggacgctactttcaaggttaccgatcaaacaactcggacccgtgaaggcgacctttgggttaagatcgaagcaactgacgctgccaacagcaaagctaatggttggattctttacagtggtttgaagcaagctactcctgctacaccagctgagaactttaatgctgataccagtgtgaagattgcttatcgtgatgtttcaactggtaagacactttcaaacaccaatacttggacaacagcttcaactggtaccaagcaaggtaacagtgttggcgctttggtaaatgctaaggcacaaaaccttggaacattcgttgctgctactggcgcaccttctggttacaagctcaatacaactagtggtgatctcaagggcgacggtagtaacgttgttgttacacctgcactctcaagtgctacctttggtgctactttgactgttgatgtaactccagtttcatcagcaactaaggttaagttgcaaatgcctggtactaatgggactgtaaaccaatcattaactgcaagtgatttcctttatggttatcctgatttgaccaccagtgcacaaaatgagtcattaccacctgttggtactcctaatggtatgttcactgtcgcaaaatatttcgactccaacagccaattcactaaggatatcaacgattcgacaaagtccaatactgtgcaaacagttcaaagacttcatagtgatatctggaattctaacggtcaagaaacattcggagatgtcacaggattctatggtcaaaaggatcctaacagaagcacaacagcaatccctgtttactacttctacgtatacaatccaactgaaaccgctaaagccaatgcatctcaattgcaaaacggatcttcagtaaatttggtatttgatcgttattctactaaccgtacacctgatccagttagaactgatttaaatactaatactgattttattgcaaaataagatatcatcgattcatagttttacccattccagctctacaaacttaatatgtaatgtcgaccaaagtgatttggccgtccgctttatggaatcaccgttccgtcaatatgatttgtagttgcacacaggtaacgaataaattgctgggcggaagggatacttcaagcatatttcttccaggcaatttgaaaataaaccagcgatccgatttacttcgggtcgctggttttttgtctggatacagttaaggggccaattgattctgcgttcgatttggaattttccaacgatcggtggagttcttctaattcgttactttcctccaaaggttagtcgttatggaaaaacggattggggtcagccgttggacccaaaaactcgtaatctgtatataagtagggaacgttattattcattttgtgctcgatgccggcgttgtaaactttccagcgcagttcgtcgatttccttcattattttgtcgtaatctctcaatgacaaaagaaccccgagcatttggtcatgtttgataacaaacacaccggtttgattcaattttgctcgttggaaagctttagttggtgactttttcaattcggaaacagatatgagtggcgtatttaaaactgtcattgtatccctcctcgtatttgttcttatgatatcaattttccccaagagatactagtttggtggctctcgattaatggacaagaagatgctttcatgggctgaatacaaaaaatgcctgaaacataaattaacattcatgtttcagacatttttcgtagttttagtaatcagcagctgtgttagtagaagttgttttcttcgtagcagtggtcttgctggtggtcgtcttcttagtagaagtggtcttcttaatctgatcctttgggaaattatcaatcataaagttagcgatgtctctggccattaactgatacgtcttggcagccggatgcaagcggccgtcgttaaatcggtcaatgtgattagcgtcagtgatcaaattaggatcgacgtcctgccagttgaggtatggcacgtcattttgctgatagacttcagcttcggcacttctcaattcgttcatggtgtagccgccttggccgacaacgtcatcggagttctggttgttgtcataacgggtgattggcaggatgccatagatgatcaggttcttattttcagctttcatcttcttaatattggtatccaaggtgttcttaatttggtcaatggtcgaatcggtatgaccgtaatcgttggtcccataagcgatggtggccacgttgtatttggcaaaattggtatcctcaaccgtggtggttaagtcccccggtgtcgacatatcgccggcgtcacacaagaaggcaccgttgtatgcggcgttatcaactttcacattcaggtaacgggccagccaggtcgggtagccggcatccaaggtctcgtagccgtcataaccggcggtaatggagtcgcccatggtgataagcgtgtctgatttgaagtagtcactatttttcattgcgatgtcaaacgttccttccgaaatatcttgtaagttgccgcgccagacccagccgttttgcttgccggaaccactcttcacgtaataccaaacggagttgcccttgccctgggcggatcggtcgatgacagcttttttataagtgtaccaggttaccttggcaaagtctttagcagatcccaaagtcttgttcaaaccggaagtcgtgtagacgtagccgccctttaaatggtagggaagtggttggtcgtagtcttcggtagaaacaagggaagcagctggaatcgtttttttagtggtgtcattagttgatttggatttggtgcttgatgaactcgtcgaagtcggggtcgttggtgtcgttgtggcagcactgccaggtgccatgatcgccgcaatccccaaagcggctgtgatggcagtcgttatgtaaaaacgtttagtcatatcaattatctcctcataattttgaactatgtattactttagcatgatattgttacgaaacccttacatgccgcttacactcaaatgaagagttcgtgcacaacttgcttatttttagtaaatcaattatgattacttttagcaagatactaatagaacgatttgactagaatgcaagcgggggagtcaataaatgaatatcaaagtaaaatgcaggttaacactgttattttcattgatggtttttggcggtttggggatgaatactcaagtcaatgccgccactgatgattcaaccacggctgcgcctcagattcaatcggtcagcaaagccgattcatcggtcacggtgaatccggctgaggggacctcatccaacgtttcggcggatgagtcaagcgacagcgcagcggcaaagattgacgattcaaaagtgaacaaggattctggcagtagcgtcacaactacatatggggatgccaaggataaccaggttaaggccaatagcgatagtgataaggatgctgctaagggtgactcttcaacggctgcaagtgacacctccactgatgtgtctcaggattcatctgctcaaaaggatagttcatctgaccagaatgccaccagtgattcgtccagctcaaccgatgatgccattgacaccgatactgacacggcggacgtgactgaggatactgactcgagcaaggttgtgaagccagcctctgccaaggcggacgctgatgtggataaatccagcacagatgctcaaccaacaacggctgccagtgacgccgatgccccggatgacagtccaacggtcttggaatcgctgacccaggatgcatccaaatccgaccaggcgccagagacactggttgtgccggatcaaccgattattgagagccaaaatgtttacaacgacatcgttggggatacatttgccgacaaagtgacgaagagcgatcccaaggcagttaaggaagcaaccgcgattgccaataacaagactaagctgttgaccttcaatgctttctcggacaaaatttaccgtcacgtattgaagacagctcagaagcctgggacggtcacgacgacctctggccataaagtcaccttgaccacgcctgtcaagcacgtgaaatacaccgagcatgattcaaccggtgtttcagagactctgccagtcatggcaaccttggcgattattggggtagcaggcattacgtttattgcgtttgacccgcttagatttctctttaaataaatggacgaagcacggtcgggtttgtcggccgtgctttttgctgtctaaaggcgcgtcaatctaacgtttagaaataaattcaaaaaagagtatttaatacttgcaaacgcttacagatatgatattatatagtcaaggaagggaaaagaagttcgaagcataggggtttcagcctactttgaatgttcttcgatccaagattaatatgttgttatgtcacaggattattttcaaatgtttcacatgtagaacgcatagttgtttattttaagttttaagagtttgaggttcacgattcacagaagcatggatgtttgaataaatgatgttttatttagccgattgtttcagagattcatagagtttcaaattgttacagtttaaaataacagaaggttaattcaggtgattaagtgtttgaatataatgttatgagtcacacatgttcaaatatgaattcgatgattcgctattgaaaacctggtggagtaattgaaaagggttatgtacagaggtcacttgtagtgaatctgagagattcattcgaatatcaaattgatgtgatatcaagttgatgaaagatccaatgaaataggttaaggttcacaggttttaagtaccacgcaccttaggtttatgtatcacgtatcaagcagttgcaccaagtatgatagtttcacgtagaaccaaaatgttgaccacacggcaaatttatcaataaagtaaaaacgtgaaaatgattaaagtttgcggcagttggatcaacaaatagttagattgaggcgataagacattaaagttttaatgaagtgggtattaaccccaaagttcccttccgtataggatttaagcttgcagtacttagatgcgagtttgaatcctatttttttgtagagtgcgacgagacccgggagacgcggtttccaagtgggctttgattaaagttcctggttttggggactttaatcaaagcccacttggaagttagcgtctgggtcgtcggagcacgtttcaataagagtgcggactggggcggttagtaaccggagtctaaggtgcttcgaacggaaatcgagtttgattttcgtttgaagttccttagatgcaggttgctgccccagggagcacatttccactagagaaaagggaaccacaaaataaccaatacataaaagaaagaccaccaagaaagaccaccaacaagcaccaccaccagccaccccggcaccaacccaaaaccaaacaaattccataaatcccccacgctcgaaaattccctatttacgccagcaaaacactttgatataatgaaagcgcaatcaagaaagtaaaaggtattacttaacgccatttcttgatttctatttacaggactttctgcaatgaggtattctattcacatggaatatttttttctgagcaaagttttgatttggaaaggaagtttctcatgaactttcgtcgtgtcattgtacttgatctggcatcattgggtgtcggcgaggccagcgacgctaatcgatttgaatcggttggcgccgatactttaggtcacatcgcaactcttgaaggaactgactttcaactgccgacattaagtcgactggggttgggcaacattcgctacagcgacccggttgtcggtctgccgccagttgaggaaccgatcggcttttttggcaagattagaagccagagccgggagaattctcaattaagtggtctgcgggagatgtttgatttccagacacccacccgaacaaccagtgtcattgacggcatcgtcggccttttaggggtccactcaatcttgatcagcaattaccagagctacctttccaatcagaaccaagcggaagtcattccggtcaatacggatgagggtggcttggagcagcttcaccagcaggtgattgcgccgaataacggcctgctttattttcgggcattagggttgtccgaacacgcacaaacggggaaccgcaaaggctgcatcgattcacttaaattggtggatcagcatttggcacggttgatgcgggaactatacagcaccgaccttttaattatcacgtcttcgtatgccaacgatccggccatggacgttacaccaacgcgcgaatacctgccgttgattgcctacacgtcctcacttccagagggcaaggccttgggaattcggcggacacttgcagacattggggcctcaatcggggagatattcggccttgaagtgtccaatgaatccactggcagcagttttctcggcgaattgaaataagtcgccgcattatttagggtttaattcataaaaccaattccattacagagggggatagctagccatcttcatcgttgtttagcaattattgtcgttaaaattcagaaaagaggatttcagaatatgcaattatcatatttactggtcaatattctgggtgtcgccgtataccttggaattgctttcttgttttcaaataacaaaaagggtatcaactggcgttcagttggtgttgttttagtaattaacctggttctggcatggatattgactagtttctcctggggccgtgatgcggttaaagccgctgccgacggatttaactggttggtccaagtcgcttaccaagggatcaacttcgccctgcctaactgggttaccccacaatttggcggaactgccaagtcaatgaactttgtcacgagtgcgttactgccaatcctgatgattgttccattgtttgatacgcttacatatattggcgtattgccgtggatcatcaagtgggtcggccgtggactttcatttgttaccggcgctccaaagttcgaatcattcttcgctgttgaaatgatgttcttaggtaacactgaagcacttgctgtttcatcactccaattaaaacaaatgtcagcaaagcgtaacttgactttggcactgatgtcaatgtcatgtgtcaccgcttcaatcatcggggcatatacccaaatggttcctggccaattcgttttgactgccgttccactgaatgtgttaaacgccttgattattaccagcttattgaaccctgttaaagtcactcctgaagaagatacggttgctaaaatgggtggctcaggttccagtgaagccgctgttgaagccggcgacgttcaagctaatggtaaacgtgaaccatacttctcattcttaggcgactcaatcttgggtgccggtcgtttgatcttgatcatcgctgccaacgttatcgcctttgttgccttggctgctttgattgacaagattttggctttgttcaacccatggttgtctttggaacatatcttaggaatcatcatgttcccatttgcatggttaatgggtctggatgtcagtcaggcattccagttcgcccaattcatggggatgaagttggttaccaacgaattcgttgttatgggtaagattgccagcaccattcacaacctcagcatcttcccagctcactaccaagcacaattaacggtcttcatcacttcattcgccaacttctcaactacgggtatgattatcggtgccttcaagggcttggttgataaggaaaagaacgatttgatcagtaaaaacgttggtaccatgttgctttcaggtattctggtatccttaatgtctgctggaattgttggtctgtttgtttggtaaaatcagttctagaaagttaggttttatgtttggataagttacaaagagaagaagaggcggctaaccggctgcctcttcgtgaggctatacgggataaagccaccgtcaaacgggaaatcattgctgggattaccggctttttcgcgatttcatacatcatcattgtcaatccaatgatcttaaaagatgccgggattcccactgatttgagtgtctttgcaacgatcatttcttcgttgatcggctgcttgattatgggcttttgggccaatgcaccggtaattttgacgccgggaatgggcgtcaatgccttcttcacttataccgttgtcgttgccatgggtctgtcctggcaagaagcgctggcaatctcgattgtctccagtatcatttatgtgattatcgcatttacgaagttgagtgagattttggcgaagggaattccagagactttgaaagcggggattaccgccggcattgggctgttcttagttgaaattggactggaaaaagcgcaattgattcagcaggggaagaactcgattctggctctgggcgatttgaccaagccggcgacgctgctggcgttgtttgggttactgctcacgctattcctgttcgtccgcaatgttaccggcggcttctttatcggtattctggtcacctcggtggtcggaattctgtttggcatcaaagatcaagtctcaccgtcagttgaaattggcgatatcactcgttactcggggattgtggccaaaggaaattttgacaacgcgttaaccattccatttgtgctggcagtcttttcgatgaccatgatcttggtatttgaatcgatggggctactggaagggattatgccaaatcctggtaagtttaagaaggcgtttcaagccagttccgtgaccagctttctttccgggattcttgggaccagtcccacggttgctgcagccgaaagcgcttcggcaattgaaagtggcggtcggaccggcttaacctcgattgttgccggattgatgtttgcggtttcgttgttctttattccgttgctggcatttgtgccccaagcagcgatcgcacccgtgattatcattaccggtgcgttgatgatgaatcagctcagccgcattaatatgtttgatttttccgattggttcccggcatttctcatcgtggtcttgattccatttaccagtagcatttcgactggtttggcgtttggatttgtcgcttacccaattttaaaaattgccgctggcaggcaacacgagctgactgtcgcgacttatgtcttaggatttttattcttgtgtgatttggtgctcagtgcactattatagaagtaacaagcgggcggacttcaggttcgcttcttgttaggaactaattgtaagcgtttgatattaacaaatattgtttggaaaggaacttatcatgaccatcaaaattattatggataccgatcccggaattgacgatgctgccgctttaaccatggcgttgaacgatcccgagattgacctgaagttgattaccagtgttgccggcaacgttaccgtggacaagacgactaagaatgcgcaaaagattgtccgcttcttcaataaaaaggtgccggtcgcagccggtgccaaacagccgttgattaaagaatttgaagatgctgcccggattcacggtgaatcagggatgccaggctatgatttcccagaagatctgccaaagccattggatgttagtgccgttgaggctttaagagaaacgatcatgagcagtgatgaaaagattactttggtcccaactggttcttataccaacgtggccttgctgttcagtgaatatcctgaagtgaaggaccacatcgaacggatcgtcgcaatgggtgggtcacttggaaaaggcaacatgacttctgctgccgagtttaacgtcttcaccgatccggatgccgcacgaattatgtataattctggaatcccgattacgatggttggcctggatattacgatgaaggccctgatcaccccggactctctcagcaagctcgagcacatgaacgaaaccggtaagatgctgcatgacatcatcattcatgatggtgataacagcgctgaaggaattgccatgcacgacgtcaacaccatcttctacctgcttcatccagaagcaattaccaccaagaagatgtggatcgacattgtcactgacggtccagccattggcgaaactgtcggcgatatccgtggtgcttaccatgatggcaagaccaacgctaatgtttgtgtggatattgacgctggggcctttaacaagtggttcttggatgaagtttctaagattaataagtaaattttctaggcagtcagatattttttctggctgtttttttgttggacggctgtaatagtttttctgcaccctacgtcttgacactttcccagttgattggcataatgaatctaacattaaaaacacatgagaacaatgcgatgacgaggagagtagtgatcgaggcgatctaaagagaagagccatttggtgagaggcttgattgtcaagatgatgaagatgagctccgagcaggtgaccggtagaagccagtgatccgtcagcaaacgttattttgccggatatcgattttaaatggtaccgtcgaggtgtattttagatacacgaagatagggtggtaacgcgcaggagcgtcccttagtccgtagttgggctaaggggcgctttttgttttctcataatccaacatacattgcaaagtaggtgaaatcattgagcgaaataactgattatgattctaaattaatcgaggaactattcatcaaatatgccaaagtcaacacgagatccgatgcgaacagtcacacagtgccaaccactgtcggccaggtcaaactcgcgaaaatggttgaaaaagatcttcacgatttggggatcgcggatgccaagtacgaacctgaaaattcctatgtgattgggagcttgccgagtaattctgataaggatttgagtgcgattggatttattgcccacttggataccgccgattataatgccgaaaacattcaacctcaggttcatccaaactatgacggtggcgagattgtattgaacgccgagaagcagatggtgttgagcccgaaagaatttccactgcttaagcactatgttggccagcgggtcatcacgactgatggcaccaccttgcttggcgcagatgacaaggccggagttgcagcaatctttggcgctctcaaatattttctaacccatcctgacgttgagcatggagatgtaaaagtcgcctttggccccgatgaagaaattggccgtggcgctaaacggttccctgccaaagaatttgggactgaatttgcctataccttggataacggccagcccggacaaatcgaagctgagacctttaatgcttccgaggccaaaattgatatccgcggcaccgcggttcatcccggggatgcttatggtttgatggtcaatgccgttaccttggccaatgaaattatgagtgcattgccaaaagacgaggttcctgaaaaaagtcgcgatcaccaaggcttcattttggtcaccgacatgactgcaacagtgggggaggcccatctcaatctcattattcgcgagtttgatacgcagaaataccgtcgtaatttggcactgttacatcagattgtcgaccgaattaatgatcaatatgattctccaagagtcagtctgaagattaatgaacagtatcaaaacattggcgatacggtcaaacagcatccatacatcgtcaatctggcattgaacgtctatcatcagctgggaataacgcccagcattacaccgtttagaggcggcactgacggtaatgcgattaccgcaaaaggcattccaacgcccaacttatttaacggtggtgacaattttcatggcccttatgaatatgtcagtaccgaagcgatgaccaagacggctcaggtggtcagcgagattgttcaggaacacgtccgcgaatatgggcaccgcgacgagagcccagttaaattaaattaacaccagacatcagcaaccagtcaatccgactggttgtttttatttgcggattgatcaggttgacaacttcaataaccttgatttacaggtgaatttactaaactcaataaattcatggcaaaacatgttaaaatcttatatgtatgcaaccgacaaatgtctttggacaccttgtcagtcaagctattttaaggtaaagtataataagacgtgaaacagattgtttcacacatcaggagaaatcaagcatgaacaatgatcaattcaaaaaggcgcttttggataaaggtatcgaagtcactgaccagcagatggatcagttcgatgcctattttaagctgttagtggccgttaacgaacacgttaatctgacctcaattacagaaaagcctgaagtgtatctcaaacatttctacgattcgattacaccagccttttttgtttcacagattaaaacagcgccattgtcgatttgtgatgtgggagcgggggccggatttccatcattaccgttaaaaattcttttcccacaactcaaagtgacgatcgttgattcattgaataagcggattaactttttgacaaccttggtcaaagaattgaatttgaccggcgttgagctgtttcatgcccgcgccgaagaattcggcggtaaaagatctgagcatcgtgagcagtacgatctagtgaccgcccgtgccgtggccagattaaccgtcttgagtgaactttgcctgccattggctaaagtcggcggcaaaatggttgccttaaaggctgctaaggctgaaggggaactgtcggatgctcagccagcgattcaactgcttggcggcaaagtctcgggggactttgaattttcactgccagtttctgatgaagaacggcacgttattgtgattgataaggtcaaggagacacctaagaaatatccacgaaagccagggacacccaaccgtgagcccctggatcaaatcaaacgatgaggagggatgaaagatgacatacgtaatcgcgcttgcgaaccaaaagggcggcgtcggcaagaccacgacggccgtcaatttgggtgccgggatggcttcgctggggaagaaaatcctcctggtagatgccgacgctcaggggaatgcgaccagtggagttggcgtctcaaaggcagacatcaccaaagatatttatgatgtcttggtgaatgaagaaccgatggcagaaacaatcgtccacacctcacatgagggtttggacattgtcccggcaaccattcaactgtctggtgcagagattgaattaacaccccagatggcccgagagacccgtttgaaggccgccctggatgccgtcaaagaccaatatgatttcgtattgattgattgtccaccgtcgcttggtttgattactatcaatgctttcacagccagtgactcgattctcattccggtgcagagtgaatactatgccctggaagggttgagccaattattgaacaccattcaattggtcaagaagcatttcaatccaaatttgaagatcgaaggggtattattaaccatgttcgacgcccgaaccaatctgggcgaacaggttaataccgaggtccgcaaattcttcaaggatgaggtttacgacaccattattccaagaaacgtccgcttatcggaagcaccaagctatggtctgccaatcatggattacgacccaaagtcaaagggtgctgagaaatatatgaatctggcaaaagaggtgctggcaaaccatggctaataagaaaaaactaactggtcttggcaaggggattgaagccttgttccaagacaataatgtcgatacgagtaaagaagatgtcgttgacctgaaagtcagcaccatcaagcccaatccgtaccagccccgccaccgttttgaccaaaaagcgttggaagatctggccctttcaattaagaactccggtgtcttccagccaatcattgtcaggcagcccgatccggaagttgactcatttgaattattaactggtgaacgtcgactgcgggcatccaaaattgccaagcaggagacgattccggccatcatccgcagtgtcaatgaagagcagatgatggaaatcgctgtgatggaaaacctgcagcgagaggatttgaccacgcttgaagaagcggaagcctacaacatgttaatgagtcgactggacctgacccaggcacaggttgctgcacgattgggcaagagccggccatacattgccaactacttaagaattctgggcctgccgaccgaagttaagaaaatgctcgaagacaagaaactctcaatgggccaggccagaaccctgctttcggttaacaacaagcaggaactcatcaaattggctcgcaagtcagtcaatgaatcattaactgtccgtcaactggagcaggctgctgccaagattaacggcaacaagccggccaaaaagaaaaaggcccccagaaaatcaccatttgtcagggcgtcagaaggtcaactccaagaaaaatttggcacatcggtttcgattgtcaattcatcacgcaagaagggtaaaggtaagattgaaattgagtatacctcaactgacgatcttaaccggatcctggaaatgtttggggtcgatttggactagtcacgttgccgaaaggagacttcatttatgtatgatttaaacgatttagttgaaatgaaaaagcctcatccatgcggcaccaaccgctggcagatcattcgaatgggtgcggatatcaaaatccaatgtaccggctgcggccacattgtgatgatgccccgaagagaatttgatcacaaattaaaaaagatccttgaaaaagctgaaaaataaaccagaaagaagcgtttaagttatgtctttaacagcaggaatcgtcggcttaccaaacgtcggcaagtcgactttgttcaatgcgattaccaaggccggagcggaaatggccaactacccatttgccaccatcgaccccaacgtcgggatggttgaagtccccgacaagcgccttgaccgaattcaagaattaattccagccaagaaagtggttccgaccaccttcgaatttaccgacattgccggtatcgttaagggtgccagcaaaggtgaaggacttggtaacaagttcttggaaaatatccgtcaagttgatgcgattgtccacgttgtccgtgcatttgacgatgacaacattaccacggtttccggcaaggttgatccactggacgatatcgacaccattaatttggaattgggcattgccgacctggactccgtcaacaagcggttagggaaggttcaacgcgctgccaagggtaatgacaaggaagccaaagcggaattggccgttcttgaaaaaatcaagccggttttggaagacggcggttcggttcgttcaatcgactttgatgacgacgagcaaaagattgttaagggtctattcttgttgaccagcaaaccggttctctacgttgccaatatcgctgaagacgacatggctgacccggagaactccaagtatttcccagaaatcagggaattcgctgccaaagagggtgccgaagcaattgcggtcgctgccggtcccgaagaagaaattgcccaattggatgacgacgaaaaggctgaatttctggaggctgaaggagttaaggagcccggtttaaaccggcttatcagagcctcatacaagcttttgggcctgcagaccttcttcactgcaggtggtaaggaaacccgtgcctggacctttaagaagggtaccaaggcccctcaagctgccgggatcatccattcagactttgagcggggcttcatccgtgccgaagtcatggcctttgatgatttggacaaattggagacaccagcagcagtcaaggaagcaggtaaactgcgtcttgaaggaaaagattacgtcatgcaagatggcgatattgttgaatttaggtttaacgtttagacgttattttaaggagtgaagctagtgagtagcaacgatgacacacagcgcaatgccaacagcaaagcgcgtcagaagaatgcccaggtgcatcaggatcgggatcatgcggccaaaattgtccattcccagttcgataacattgggttaaccaagcggaatgctgagtacatgttcaagtttaaccaggcacttggcgccaccaaactgtctgcagacaagaagaacgaagccgtccagacaatggttcaggaattgctggagggccagaagtcaggcaaaactgccagaaatatgtgggggactgtcgatcaaaagattgaaacgacggttcatccaccggcaaggccagctgatccacgcagagactattggaagaatgccgggtacaatgctgtcctgtttttgacgatcttcttcttgatgtatggggttctgtggttcctgccaacaaagggcggccaacactcaccaatgatgggcatcactggaattctcattagtgcggcagttgccggcttgggcattccaattgtgacgatgatgttcacaccaggtgttaagcatcgtttctcaatttggattcgcatcatcctggtcgtcttgttcctgatcgtgtggatgggaatcttcacgctgtcatcaattctaccgccagttttgaacccagtcttgaatccaatcgtctacatcgtgttgggtgtgttgtcaggagtggcagccttcttcgtcaagcgccgattcaacattaccggtggtgtattctaaaactaataatgcatttaacgatatggtttggtcagatgatttgtcatttgatcaagccattttttgtccatgctccaaacacgaacaataaaatgtaaatttttgaaataaatgccagacgacgaaaaaagatgaacgatggtctttatttattcggaagagtcgtgtataatcaatacaatttcagaaaacgatttgcttaagggcctcatcatttttatgagaagcgtatgagaattctttcagagacgttgaataactaaaatgaaaatgataagttattaagcaatcaacatttaaaaggagcgagatagatggttagttgggatgaaaaattcggtaaaaaaggtttgacgtttgatgatgtgctgttgattcctgcagcgagcgatgttttaccaaatgatgtggatttatcagtacaattggcagacaacttaaagttgaatgttccttttctaagtgccggaatggacactgttaccgaatcgaagatggcgattgcgttagccaagcttggtggcatgggtgtggttcataagaatttgagtattgaagatcaagccgctgagattgccaaggtgaaggcagttaagaagactgccgacacacctaaagctgcggtagacgacaacgatgcgttgttggttgccgccgctgttggggtttcatccgatacttttgaccgggcatccgctttactaaaagccggtgccgatgcgatcgtgatcgataccgcccatggccattcagccggagttcttcgtaagattgccgaaattcgtgaccactatcctcacaccactttaattgccggcaacgttgccactgccgccggaaccgaagcccttttccaagccggcgttgacgttgtcaaagttggaattggccccggctcgatctgtacgactcgggttgttgccggcgttggcgttcctcaaattacagctgtctacgatgcagccagtgttgcccgcaaatggggcaaggcaatcatcgctgatggcggaatccagtattcaggcgacatcgtgaaggcattagctgccggtggtagtgccgtgatgctcggaagcgtcttctccggaactgacgaagctcctggtgaagtctttgaagatcatggtaagaagtacaagtcataccgtggcatgggcagtgttgctgccatggaacaacaacatggttcagctgaccgttacttccaaggcggtgtcagtgaagccaacaaattagttcctgaaggtattgaaggcgaaaccgaatataaaggcagcatcaacgacatcgttttccagatggtcggcggcctgcgttcaggaatgggttacactggctcagcaaccatcaaagatctcaatgacagcgcccaattcgtgcaaatcaccaatgccggcttgagagaatctcacccgcatgatgtcaacattactaaagaagcacctaactacaaaccagaagattaatgcatctcaaacacctgcaggtcaaccgctatccgcgattgacctgcttttttatcttcaaaccaagtttggttaaaatgtcgccgggttccagttcaccggctccgcctgctgtagtggcttggatttcgagcctgtagtctcgaaatgccaagatgctgtaatcacgacttgcagtcgtttcaacagcatggacactacagctggcaatgccggtaaactggaacccggctactggcagcatatctatgagtttggataaaagtgattgaaaaggaactgcacgattcgtgaatcaaacggaatgaggccgaattttgctggtttggcattgacagccatagtgaaagtgttgttgaagccgatgaaatcggcaattacaacacctttgtatttcaagactacaggcttgaaatcaaagccactatggcaggcagagccaaaccagcaaaatttcccacttgagctgcctcttagtacttacaggacgagaggaatgctaagttttcatcaatatcgacaacaattatcatttttattactaaataggagtattatgattctgttagtaacattaatcatcaaggcaggaggcataccgttggactcacaaaatattcttgaacggccatttatcaccatcactaatttaatctggagcttcgaccacgccaccaatcgggtcaatattctgctggtcaaacgcgataacgatccttacaacaactactgggcattaccggaaacctttatgcgctcccaggaaagtgccgaagagactgcgttgcgcctagtccgagaaaagattggcatggatttgtcaggcagtcacactgaacagttggcaacctttaccaatcctctgcggacacctggcgatcgggcactgtctttggggtacatgacatttttacccgataaaccgcagctcaaggcgggttatggtgcctcggatgcccggtggttcaccatgggatatacggataaaacgtacacctttagcgattcggatcatattttccaatccacagattgcccggttcaacggacgtactatgcagaatttggcgggaccaacgctgatcctgacaaacacctggcatttgatcatcaatggattttgaaggttgcctgtgagcgaattcgcaacaaactggattatcagcctaatatcctgttgattcttgggcgacaattcacgctcaaagatgctcggcgggtctattcgccatttttaaagcttcgggtggatcaaatcgacaactcgaatttcaagaaaagccaccaagatctctttactgatattggttccagcgaggtcaatggtcccggtcggccggctcggttgtacaaattagctcatttgcgggcgtaaacgcttgaaatgttatcggagtcgttgtaacgtagaataaaagtttggaacacttttattttaagaatataaaagttaaaggtacttttaatcccaatgaaaagagtcgaaacataatgagtaacttatcaatgttgacagatttatacgaattttcaatggctaacggctatcgacagacgattaccgatgagcagggggtcttcgatgtcttcttccggaaggttcccgataacggtagttttgtgattgctgctggcttggagcaggccgtcaaagcgctgcagaatttccactttgacgatagtgacatcgagtatctccggtcactgaacctgtttcaagagaattttttgacgtatttaaaagatttcaaattcgattgtcaggtatccgccattccggaagggacgcctgtctttccacgagaaccgatgctgacaattcgtggaccgctgctgcaaacgcaattatttgagacaatgattctcaatattttgaatcatcagtcactgatcgccaccaaggcccgtcggattacctactcggctgatggccggccggtgatggagtttggtgcccgacgagcgcaaggccccgacagtgcgacgtatggtgcccgagctgctgtgattggcggctgttccagtacttccaacgtgttggcagccgaagcatttggcatcccggccgccggcaccatggcccatgcttggatcgaatcgttcccagacgaattgacctcttttgaaaaatgggcagaagtttatccagacaatgccgccttactggttgatacctatgatgtgttgaaatctggcgtgccgaatgcgattaaagtctttaaagaattgaaagccaacggccacaaaccagttggaatccgaattgattccggtgacatcagtcaactttccaaggctgcccgcaagatgctcgacgatgccggtttgccggaagttaagattacggcttcaaatgccctggacgagcacgtggtcgcttcactccttaatgagggtgcgccgttggataactttgggattggtgagaagctgatcactagtgcttcttcaccggtcctcagcggggtttacaaactcgctgccgttattgagaacggtaaaatgattcctaagatcaaagtcagtgccagccgggaaaaggttaccctgcctggtctcaagcaggtctaccggctttatcaaccggggactgacaaggcctttgcggatgttatcgccctcagtgatgaatccttggatcaaccgattacggtggtgaaggctaacccactggctaccaaacgggaacagcgaatcgagaagtttgacgccaagccactccaaaatgaagttttggccggcacggatttgaagatggcttttccaagtgtctttgatattcaaaagtattccaaacaaaaactaaccgagattccagctgccactcagcggttggtcaacccggacgaatttccaatctatgtgaccaccaagctggctgccttgcaggagagtttgctggaagcggatgctcagtagttgcatgacattttaagaaatgattagagctgttggtaaagttgttgcttttccggcagctctttttctcccaaatcggtctgggtaaatttgaccctcctgaggtgggatgggtttataatacccctgtaagcggttacatgacagatgtgctttagaagggggcatatttatgtattattctaatggcaattatgaggcctttgccaaacccaagaaacccgctggtgttgccaacaagtcagcctatttgatcggttcgggtctggcgtcactggctgccgcagtctttctggttcgtgatgcgcaaatgccgggggaaaatattcacgtcttagaagagctgtcactgccaggaggcagtatggatggcatttataatcctgacaagggctatattgtccgtggcggtcgggaaatggaacagcactttgaaaccttgtgggacctgtttcggtcaattccaagcttggagaatcccgacgtctcagtcttggacgaattttattggctgaacaaggatgacccgagtttttcacatgcccgggcaatcgagaagcgcggccaccgaattccaactgacggcaaattcaccctgtccagaaaagcagtggaagaaatcgccaagttagtgatgacacctgaagaccaattggataatttaaagatcaacgacgtcttttccgatgacttcttcaagtctaatttctggctggattggtcaacgatgtttgcctttgaaccatgggccagtgctgcagaaatgcgacgctacctgatgagatttgttcaccacgttggcacgctgccaaatatgtcgtcactaaaattcaccaaatacaatcagtatgagtcgctgattaaaccgatggtcaaatacctggaagatcggggtgtcagtttccaattcaataccacggttgaaaatgtgattgtcgacactactgatgggaagaagaccgctaccaagctggagattattgaagacggggtggagaaaagcattgatttgacgccaaatgatttcgtcttcattaccaacgggtcgattactgaaagtacgacctatggggataacgatcatccggcagcgaaggaacatgcggttggcgcagcttggacgctttgggagaatctggctaaacaggatcctgcattcggtcacccgaagaaattttaccagaacattcctccggccaactgggtgatttctgccacgaccacgttcactgacgatcgaattgtgccatacattgagcggattaccaagaaagatccgcacagtggtcaattggttaccagcgggccagtgtcgattcgggattccaactggttgatgggactaacggttagtcgtcagccacatttcgctcagcaaaaaccaaatgagctggttgtctggacttatggcttgttctcagatttacctggaaactatgttcaaaagaagattgccgactgctcaggaattgaaatctgcgaggagttcttataccacattggcgtccccgttgatgagatcgaagagattgcccaatcagccaacacgattccggcccacatgccgtacattacctcgtacttcatgccgcggcaggcaggcgatcgaccgctggttgtcccagccggttcaaccaacttggcatttatcggtaacttcgctgaaacaaggcgtgacacggtctttaccaccgaatattcagtccggacggcaatggaggcggtctatcaactgctgaacgtcgaccgtggtgttccagaggtctttgattcatcgtttgatattcgatcgatccttagttctgtgtactatttgaatgacgaaaagtccttattggaattacctttgaccccaccggaaaaaatggttattcagcgattactgaaacatgttaagggaacttacttggaagaacttttgaaggatcaaaaactcatctagggagatggcaggtatgaaagcaagatcagtcatttgcggtggtttattgtttgcggtcggcgtggcaacggggatgcacgtggatcattgggcacatgaaatgcaccatatgcatcatcacggccatggcccgcatatgggtccgggtcacttccacgaccaaccttttgaagatattggtgatctaccttatgttcgcgagacgcggactgatgggggaggtttgaggaacgaagtttagagtgcggaacaagccgtttagcttttgagcattagtgtgataacgggcgttaacgctggtcctgcgttaacgcccgttatcggactaagcggagaaagctggcttgtggagcgcatttctgctaggtaagagaagatcttaaaagagaatcgtcaacatggtagaaccaccaagtaaaaccaccagatacaagtaagccaatgatgaacggtctgtgttcatcgttggctttaattgtttgtgtggcagagtcctggggctttgagcacgtttctgataggtaagaggacacatccaaagagaatcgttaacacagtagaaccactcaataaaaccaccaagtagccggaggccaacaattggggggccaaaagcttcctcattcagaagtttctagcccacttcctggaattacttggtggtttttgtgtgaggatgattttactgtgctattgtccttgtttcctagcggaaacgtgcgacgagacccagatgctaacttctaagagtgctttggttaaagccccaagccctggggctttaaccaaagcactcttagaaaccgcatctcccgggtctcgtcgcactctctttttttaagttccccttaagcttccgatgctatccttgtaaacgttgtgcaaacgccttacagtaacatttcagacatgcttgttgaatttattaaaaagtgtaaaatcaaaactggatgctaattgataaagccagacacataataatgataaaataatagtaaatacagacgataatgaggttgattacactatgaaaattttagttgtcgatgacgataaagaaattgctcagcttctggaaatttatattcgaaatgaaggctacgagcccgtttccgcttacagtggccaggaagccctgacccgcttacggactgaatccgacattggtttgatgatcttagacatcatgatgcctgggatgaatgggattgaagttgtcaaagaagtgcgtaaggattctcagattcccatcatcatcttgtcggccaagaccgaagacatggacaaaattcagggcctgatcagcggtgccgacgattatgttaccaagccgttcaatcctctggaagtcatggcacgggttaagtcgttgctgcggcggactgaagagcacgtcactaacgatacgcccgatgttttggacattggccccttaaccatcaataaagattctcacgaagtcaaaacgatcaccggcacgccgattcagctgactgccttggagttcggtattttatacctccttgccagccatcccaaccgggtcttttcagctgacgaaatttttgagcgggtttggcgacaggagagcattgtctcggccaaaaccgtcatggtccatgtcagccatctgcgtgacaaaattgaagaagccactaacggtgagaaagtcattcaaactgtttggggtgtcggctataagatcgagtcccattaggccaaatcaattttgaaatgggggatgccgcatgaaactgacaggtcgtgagaaaaccgagctgtttttggaaggtgtcgtaacagtcattttgcttttgctgctcaacctttcagtgatcattttaattaaccaatcaatctccaccaacccagggctgcgggacggaattttcattatcaaacgatcgattttaattggccccgaccacatgcatctctggagctgggagaatatttttattgtcctcctgctgctgtttgatggtgcggtggtttattggcggctgatcagacgttaccaccaaatgcagttgcgtcacatcatcagtgagctgcattacattgccaatggtcatttgaatcaccgaattccctttaaactgagtggtaatactcaatcggtggttgaaagcatcaacgccttggttgacagtgtcatcaagtcaatggacgaggaacgggcaattgaaagttccaaggacgaactgattaccaatgtcagccatgacttgcggacgccgttaacctctattttgggctacctgggcttgattcgggataagcaatatcacagtcaggaagatttgctgaaatataccgagattgcttatttgaaggccaaacaaatgaagtccctggttgataatttatttgaatataccaaggtcaaacagaccggaacgccactttccatcagtaagattgacctcaatcaaatgatggaacagctcgtggccagttttgagctggaagctgataaaagcgggctggcaattgctgctaaagaaacggataagcccttatacattgaggccgacgccgaaaagctgggccgggttttcaataacttgatttccaacgccatcaaatatggcaagggcggccaccacatttatttgagtgccgcagtcggccaacctggcgaagttgtcattcacgttgccaatgatgggccggagattccgcaaaaatcacttgatcaaatttttgaacggttctatcgggtggaaagctctcgcaataaggataccggcggctcaggtctgggactggcaattgcccagagtatcatcgatttgcatggtggctacattaatgtcagctccgatgaaaagttgacgacctttgcgattcatttaccggttcaacatggtgataaattaagcaaaaagccccgccaaaaaattgctgaataaaaggagaactttatgaagcatcgaatcaaaattttaacggccttaatgggctttttttgcgttttaacactatcgatgacggttgatgccaagtcgacagttaccccggaaccagctatttatgccaaatcagcgattgctgtcgacgccgacagcggccaaattttataccagaagaacgccaatcagccgcgggcaattgcgtcgatttccaagttaatgaccgtctatatcgttcatcagcaaatcagggccaataaactggcctgggatgacaaagttaaaatttcatcggaacttgccaaattaagtacggcatccggtctcaccaacgtaccgctgaccgccggcaaagcctactccgtccgccaattagtcaatgcgactttggtcgaatccgccaatgcagccgccttggcacttggccagaaagtggctgggactgcaactaaatttgccgcgttgatgaacaaaaccgcccggaagataggcatttccgatggccacttctacaatgcttccggtttgaccaacaagttaaccggtaaattggctttatcacatgtcagtgccaatgctgaaaacttgttgtcggcaaaagatgttgctttgctggctcaaaagctgctgcaaaagttccccaaggtgaccaatattaccgagcagacgacgtcaacattttatgggaccaccatgacgggacataatcaattgattgatgatcacaatttgggtcagggtgttcgcgttgatgggttgaagactggaacctccgacaaggcaggggcgtgttttgttggctcggccacgacaaatggaaagcatcggattatcacagtggtgttaggtgccagaaacaagtccgccaacgatccggcacggtttattcaaaccgccaagttgatgaaatgggtttatgctactcatcaaccgattaagttggcagccggagcgacgatcgctggggtcgataaagctaaaattcccgatggcaaacagacgaccatcttgccggttaccaaggcgacccactgggcttgggccgacaaaggcacttctgccaagcagatttctggtcaatacgttaatcagcctgccaaactgacatcgccgactaaaaagggcactcaggtaggccaggctcggctgagcattgacggcaaacgattgcaatacattggccactcggctggcaagctggtgatggtgaccaatcaatctgtgaaaaaagccaatttctttgttcgcctatggcgcgcgatattacggctgttttaaaattcaattacacaaaaggtgtttattaattgagtcatatcccatataattgtatttggattgtgtttacattatttttacacacatgtcacgaatgtgtgagatgggtttagatggaggaatccttttgggaaaagctgtcgcaaaatctagggagaagctgccatattggcgaagaattcttgacgcttctttgcctgtagatttgagttatattccaattgggctggcatgcggtattttattgaacgcttccggctttaacgtttggaccactttaatggtttcaatcatggtcttttccggtggggctcaattcttgattgcgtctcttctggccactaatgcgccgatgctttcggtcattttaatgatgttctttcttgaactgcggtacgcattgctggggtccagtctttccaagtatctgcatggagaatccttggggtttactgcattgtttgcggcatcaatgaacgatgaaaactacgcgttgaactatttaaaattttcgacggataagaagtttacccctcatgaagcactacatgttgaacacatgacgctgatcttttggacaattagtaacattatcggcagtctaatcgggtcggccattaacattgatttaacaattgtccattttgcactgaccgcgcttttcctgtatatgattgtggttcagctgaagaatgggttgattattgtaatttgtattttatcaggattcttggcggctttctttatggtccttaccaaatccacgttggggctggtcttatccactttgacagcatccttcattggttttttggtcgaagcgacgatcagaaagtacaaacccaagagtggttggctgcggccgatgaaaaaccctgccggatcgcctgaagacgccgacgaagacgctgatgactaggagctatctttatggaatggaacacaacacagcatgtatggttaatcttggggtgtttttgtgtggcttttgcgccgcgactgattcccctgatgtttttccgtacccgaaaaattccagattggtttaacgaatggatgagatatgtcccaatctcgctcttcacggcgttggttgtcaaggacattttcatttcacctgaatataccgttaccatcgtcaaccgggcacctgagatgattgcggccgtcattgtgattgggattgcttattggactcgttccatggcaatttcggttgttttggggctggttgctgttttcctcttggcaatggtagtttgatgagcgacaagttacatacaaaaaggtcgagggaaaggtgattttacctatctctcgacctttttatttctggtcattaatctagttggacttgtgtgggaatctatttggattaaattcttacagtaaaattcttcttttaattttctcagtcggattggccaccaccaggccaaagtcgtcgggactcaagcgttggtcgacccgcatcccgttttgcacgagaatggtgtacttgtaattttctttaatcgcaatgtccatgaatgggtcgatcaagtcctggtccatccggccgttgatgtagaggcggtattccggatagttttttaagatcttagtgaccatttccgccgtgccggcttgctggagctggccgatcgtcagcgctaaggcgactcgttctctgaagttgccaagaaatgcccgtttctcatccggcttgatctgaggattgccaaacatgtgctgcttaatatattcttctgaactgtcagccatttgcatgctcctttcaaatctttaaaattaatataacaaatattttgatcaaagtctcgatctgtcatttgttataatagtctctaatgattgtttttccaaatatcgtgaatcatggcatgccagtgaaaatgccaattagggaaaaatgttataataaatttgaacaaattttattaggagggcttcaatttgaaaaaatggatctggattgtaatcgccatcgttatcggtgcatcagttggtggttacgcatatgcccgtcatagccaaaacgaaaaaatttacgctgaagctatgcagcgaggccgccttcaaatttcgaatgaaaaatacaccgctgctgaaacatcgtttaccaatgccttaaaacgcaaaccgaatgatgataaagcggataagatactgaaccaaacgcaatcgtttatttccgccaacgatttatttgacgaccttaaattcggtcaggcaaagagtgagtatcagtcagtcgtcgacaccaagaagggtaatgaactactgtctgatcgtgccaaagcacaaattaccaagattaaaggcatccaaaagaaccgtcaaaactacaacaagatttataatcaagccttggatcaggccggtaatgggcagtacaccgagtccaacagtacgctggataagattttctctgataaatcaattcatcaaaagtactatgccgatattctgaagaaggccgaaacattgcgggataagaacaatgatgccatcagcggcaatgcttccgctagttccaacagttttgactccagcacatcagacagtaacaccagcaataatcccaacgtttccggcgctaagggtgctagtttgacgtcgtctgagaagaaagctgccgctgcctacaagggctcaaatgaatacaccgtgaccaagggcgaccgcgatcttgacggcaaaccgattacggctgctcagatcaccagtgccagaaagcaaatcagtgctgctggtgtcgattccaacgcaatgagcgaccaggatgtcagaaacgtcatcaagggtgctcataagaatggcgaaacaatcggccagtacgtgaaagcccgatattaagattcggtaaaggggttgtgacaaaactaacgttttgacaacagcccctttgcttgtttcattttatatagctggaacgtgtgccaaaaggccgcttcctaggcataacctagaataactttccgagcttttagctcaaaaagtcattctaggttatgcaacggaagcaagaccgccttttggcacactccctttctaagtaataatacttgtgagaaaccgtcttctaagagtaaaattaattttaattagaaatcacgagggggttgggtatttgtcaatttgggcaaggttcgtcaacaacgtaccactgagaagatttaccgtgttgatgctggtcatttttgtgctttatgtaacccggagcatgatcagcacagtgctgttaacctttatcttctgtttgttggtggttaaattaaccaatgcaatccgcaggcacatcaaaattccggcaggcattatcgtcacggtcgtttacttgttggtaattttggggttgtactttgcggtgaccaagtatattccaaagattgctgatcaaaccattcgaacgacacaggacattatcctcttttacaccgaccccaagaatctaccggatgatactacgatgagctggttgaatgaactgattaagcaaagtaatatcatggctcagatgaaaaatggcgtgtcgctggtttggaaatatgtgaccggcgttgggaccatgggaataacgctgttcttgtcgatgattttgagcttcttttttgccattgagcagcgaaccatgaccagattttccaaactgtttcttgaaagtgattttggttggttcttccaagacttgtacttctttggcaagaaatttgtcgcaacgttcggtgttgtgattgaagcgcaattcttcatcgccatctgcaacacagttcttaccaccatcgtgatggctttcatgcatctgccgcaactggcagccttggcattgatggtcttcatcttgagcctgattccagtggccggcgtgattatttcctttgtgccgttgtcattggtggggtattcagtcggcgggtggaatgatgtcttttacctgttgatcacgatcattgtcgtgcacgcgtttgaagcttacattttgaaccccaattttatggcctccaagaccaacttaccaattttctatacttttgtcgtcttattgatcggcgagcacttctttggcatttggggattaatttgtggggtgcctattttcaccttcttcctcgatattttgggagtcaagaagcatgaaggcaaactcgacaaagtcccaaccaagccgggggaaccatagaaaccggattcactttataaaagtttcacaattaagctgaaaaaattttccatttggtgtaaaatcaatctgatagagataaagaaagaggtaattatattggcaaaacttgtgttaattcgtcatggtcaaagtgaatggaacttatctaaccagtttactggttgggttgatgttgatttgagtgaagaaggggttaagcaagccatcaatgctggtaaattaatcaaaaaagccggcatccagtttgactttgcgtttacttccgtattgactcgagcaatcaagactttacattatgctttggaatactcagaccaactttggattccggaagttaaatcatggcgtttgaacgaacgtcattacggcgctttgcaaggccacaacaagaagaaggctgctgaaaagtatggtgacgaacaggttcatatctggcgtcgttcatacgatgtattgcctccacttctgaaggccgacgacgaaggttcagctgttcatgaccgtcgttacgccaaccttgatccacacattatccctggtggtgaaaacttgaaggttaccctcgaacgggttatgccattctgggaagatgaaatcgctcctaaattacttgacggcaagaacgtgattattgctgctcatggtaactcattacgagcactttcaaagtacatcgaaaacatttctgacgaagacatcatgaaccttgaaatggctactggtgagccagtggtttatgactttgatgacaaattaaacgttgtcagcaagactaagttggactaactagataatatttgaagcactgttgttgggtaatcctgataatagtgcttttttgttgcttaagattcacccaactctaatggtaaatggggaaactaacgcttatcaacggatgaaccggtttcaattttaatggagatttaaccttgttcctgactcttgttggttaattttaataatggcatgctattctttagtttgatttttaacaatcaccagaattacatatttcaaaatattataattggggaatctagctatgtcgaagaaaaagatcacgttagttggtttaatcttaatgatttttaccacgatttatggttttgccaataccaccgttgcttatgagcaaatggggtatgcaagtattatttggtacgtattggccgcaatcttgttcctgctgccaactgctatgatgttcgccgagtatgggtcaaccttcaaagatgcccatggcgggatttattcctggttagccgggtcaattggcgaagagtgggcctttattggcaccttcatttggttatcatcctggattatctggatgatgtccaccgcttctaaagtctggattccgtttgcgacaaccttattcggtcacgatacgactcagagctggagcttctttggcttgagctccaccaagacgattggtctgctggccattctttggattatcaccgtaacctggtttgccgttcgcggaatggactcgatttccaaaatttcgtcggtgggcggaatctttgtttctctgctgacggtgatttttgcaattgccagtgtcaccgttttgattttaaacggcggtcatttggcccaaccggttaccgggatgcacagctttattcaatcgccgaaccctgattttcagtcaccaatcgctttgatttcattcatggtttatgccgtctttgcctatgccggaactgaaactcttggtggtgtgaccgataatatgcatgaacccgaaaaaacatttccacgcgggttaatcatttccactttggtaatcaccgtgatgtattcactttccatcttcctctgggggatcactgccaattggcattcagtccttggaaatggtcacgttaacctggggaacattacctatgtcttgatggccaacctgggtgttgtgctgggccagagtctgcatctttctgcagctgccagcaccatcttggggacgacttttgcccgctttgccgggttgagtatgttcatggcttatatgggctcgttcttcgtgctggtctactcgccactgaagtcattcatcatgggctcaaattccaacttctggcctgctaagatgactaagctgaataagaaggggatgcctggatttgcaatgtggacccaagcggtcattgttgccgtcctgatcttcttcgtgacctttggtggttcaagtgctaagcagttctatgtgattttgacgaatatgggaaacatttccacttcattcccgtatatcttcctggtggctgccttcccattcttcaaacgcaagcagaacctggaacgaccgtttgagatttataccaaacggtggatgaccgataccatctcaatcatcgttttgattgtcttgatcggtgggattgggttcacggcaatttacccaattttggaacacgattacgtcaacgccttctggacgatcatcggaccaatcttcttcggtctggtcgcttgggcattcttgacttatcaatcacacaagcttcgcaaacaagcacattaatatttttcaaaaaaaagagtgggatgcgaggcgttttgatcccagaatttaagcaaaaaagtgggccattcctgttttggaatggctcgcttttttgcttaaatggccgggatcagccgatcgttgcacgttttatcaatatacaagtggtaatcaaagttgcaatgaaagccaccgtagcaattaacgtcccaacctctttgttgtctaaaataaatttgatttgagatgaatgtcatcgtccgcggtaattgttcgaatgacccgacacggattgccgaccgctagggaattagcggggatgtctctggtgacaacagaaccggcaccaatcacactgccagcgccaattgtgacgccaccaatgacaacgacgttgctggcaagccaacaattgctttcaattgtgatcggtttggcgtactcatcatcgtattcggacccgtctgagcgctgtttgaggttgcgatcctgatagcggagtggatgcatcggggtggacaaggtaacgtttggaccaaacatgacgttgttgccaatcgtgaccggacagtcgtcaaggattgtaaggttggcgttaccatagaagtgggcgccaatcgttgtataaatgccgtaatcgaagaaaattggcccttgaagataaatacccttatcggcattaggaagcagctcagccacaattttggcccgttcttcggtgtcctcgtcaaaggtatcgttatatcgtttggaaagtcggtgcgcttggtgctgttgagcagctaagagtggatcggtgggatcatatatttttccggctaacattttttcttgttcagtcatagtgtcctccaaattagtgtgataccctcagtatagcgtacttaactgtggtagcgctaccacgaccgaaactgttatactgattgtagctgattttaggaggtgtctccatgattaatccggtaccactttacaaggagatgttccaacagatggggccacagcactggtggccggccgattcgaaaatggaaattgtgatcggtgccatccttgtgcaaaacaccaattggaacaatgtcgatatggctctgacaaatttaaaagatgagacgcatttggacgtgaaacagattttgggcctgccaactgaaacgctgcagtcattaatccgccccagtggtttttacgtcaacaagacccgcagcctccaagccgtcctcaaatggtttgaccaagacgactgcaactttgccttaatggtagataagtatggatccaacttacgtcggacaatgttaaagctgccaggagtgggggaggaaaccgctgattcgctgttggtctatgtatttgatcagccggcgtttattgccgacaaatatgccagaacgctttttacggatctgggatttcgcaatctcagcaattattcgaaactccaaaagcgaatttggctgcctgaatcatttacatatcaggatgctcaggaattccacggcttaattgacgagttcggcaagcggtatcttaagagtcaccgagattttgatgccagttttctgggtggctttgataggcaccagcttgatcggccgtgacagataatcttgcgaattagaaataggagttggttagatgaatgtactgttgatgctgctgccggcagttggctgggggcttttgggaccagttgttgcccgcatcggtggcaagcccgcaaatcaaatctttggaactgccgttggcacgctcttggtggcagcggtgatgacgcctttttatcatccacacctttcagtgccgacatttttagcagcagtcctagctggcagtttctgggtcattggtcaagtcggtcagttcattagttttaaaaatattggggtatccaccaccatgccaacttccaccggattccaattaattggcacctcactggtcggtgtcgtgatctttggtgaatggtcgacgataatggaaaaactgctgggtgcagggggcatcctgattttgattgttggcattatgctgacatcggtcaccgataagccactggttgcccaaaggacaccgcaaaagaagctgccaactattctgatgcttttaacgacgactttgggatacgttgtgtatatggccattcctcggggactgaatcattcgggactggcgatctttttcccagaagcaattggtatcctgctggcggttctggtctatgttttcgtcactggtcagcagcggattattaaagagccggtcagctggttgaatatcgccggtggactggtcttctccctgggcgcaatttcttacattggttccgttcaggcaaatggtgtcaattcagcctttgtggtttcgcagttggctgtggtcatctcgacgttgctggggatgatttggatgcacgaaacaaagacgcctcgtgaactggcgtttacaatctttggtttattgctgattgtctctggtgcggttatcacgacagttttttgaccacaaaaaaatgcgctggaacctgaattccaacacattttgggcaaaataaaagaccctcacaggggtctttatttattttgatttaattattcaacaacagtaacgttagcagcttgtgggccacgatcgctgtcttcaacgtcaagggtaactttttgaccttcttcaagggtcttgtaaccgtcagcattgatagctgagaagtgaacaaaaacgtccttgccgtcttctaaagtgataaaaccgtaacctttgtctccattaaaccatttaacagtaccttgttccataagaatgaaacctccgttgcgcatagcgcgataaattttgcatttgaaacttgaaaagtaaggagtcattcttattagaacgatggaccttgtttcgaagctaaatacattatctatactttaacaggtcatcgtagaaattgcaaatataaacgctcatcgactctttttacagagaacttggcttgagtgggctataatgaaattaacgttaatgtcgaaaggggatcgtcttatgagcaaatcagttaattggaaagccgccttaattgccgggggtgttgccggcgttatttccggtctcgtcaaattgggctgggaaaatgttttgccgccgcggacacctgaacggaataaaaccaacccgccacagcgtttacttgagcaggccggaattcctgaacaggtgactcacgcaacttacacctattccgatcaacaattaccatgggtcagctacatgatccactttggtttttcaacttcgtttgcaatgttttacagtctggccggccattatgttccggtgattaaaatgggcgacggcacattgtttggcctcggtgtctggggtgcctttcatttgggcatcatgccggcaatgggcacggttccgtctgctaaagatcaaccggttgaggaacatgtgtcagaggctttgggccacgttgtctggatgtggaccaacgacttgattgccgatgaggtttatcgtaagttaaccaaataagtttaattgaacgggtcaacataaaagaggtcggattataggcaatcaatgtctatgtccgaccccttttaaatttaatgattattttgattctgctaattgttcttttggcgcatcagttgatttaatttcttctgaatcttccgtggcttcagagacttttcgattacccattaccagattaataatgatggcactcaaagcggcaatcgtgatgggtgaaccgagcaggtactgaaccatttgtggcgtttcactaaccactttggctggcaagagaatcacagccattgtcaagacgattggaatccctaagacataaatggaactttcatcagtggccaggttgcggataacgttcaatccattcaacatgatgatgacacaaatgatggagaagattccgccgattacagcggcaggaacagctgacaggaacgctgataatttaccaaagaacccaagaacgacaaaccagataccagctgagacgaagacgcgtttgctggcaacaccggtgatcgaaaccacccggcgttggttgagtatccggtcattggggttgtcccgagcagggcggcaaacagacagctgagtccttcaccaatgattccgcgattccattgtttcttggtgatcttttcaccgacaacggcactcattgcgaaccaggtaccggtggtttcagttgtcaataccatataaatcactacgaaggttaaaattgccggcagtgagaaatgaatcccgtaatgtaatgaagtaaagtggggcagactgatccaagccgcgttgttcacgactgaccaatcgaaacggcccatcatcgaagcaacgaccgtaccgacgatcaaagcgataatgattgaactgactttgaacaatcgttgaagttgggggatgcggatgccgattgtaatagcgaccaacattgccaaagcggtgatggcagcaatttcaatgttttggttgacgttgccggctgccttgaagatattgtcattcaaagcggacggtaataacgacaggccaacacaggtgatgatggtgccgccgacaattgctggaaccaatgtgttgataatcttttggtagacgcctgaaacgccaagcagaattaataacaatgctccgacaatcaaagatcccaggacagtcgccatcccgccgttagcggcaccgtttgccaagtagaccccggcaaccgcaccaattggcacaaatgatgggccttgcgaaacgggcagcttcatgaagtaccgggtttgaagaattgttccaatcccgcaggccaagaaagccgcctgcaagaagccggtcttctgtgccagactcattgacagcagcccggcaatgatgatcggtggcacgtaaacatccatggccaacacatgctggagtcccagtaatcctgattggaaatatgaaaccttatcgtctggaccgtaaagcaaaccgttatcattgcgtttcattaagaattctcctcaatttgttaaatttcggctatacacgaacattaatttgaaataaaaataaataattcgcatcgctagttaatgcttagtataaacactagctttgtaattatcaacaataattcgaaattaattttttgactttaatgttcgtgtttggagcccctaaattgaacacgcaagatgatgattgtcatagtggggatgaaaccgttatccgatcaaataatgattgagcaaattatcattttccacattaaaaaagctgaaattcatcattgaatttcagcttttaatattgtgaagagttatctggcaagagacttgaccaacgcgtcgatgatgtgggtgatttctcgctgctccagaggttgatcaaacaataggtaaccaatgatcacgccgccgacaaccgaccaaatgattttgagaatttctaggttgtcccagttgacgattaaatggttgtctttgagttgattcaaatttttgttgatgttgtgccaatatagaggaggaaatttggtcagcagttcttttctgacagtctcattatataagacctcggagacaaaaattttgaggacggctgcgttgtctttgagaaattgaattctgtcgcggaccaatgaatcaacaaaggcatgtaaagtgacaaattgcagggggagctgatcagtcttaaattcggtgaggacggcgggaaaaatcgagttgatcaccggttcgatgatggcattcagtaacccgcgtttattcttgaacttattaaaaatatttccctcggaaacgcctgccttggtggcaatttctttggtgcttgcgttggcataccctttttctgcgaatacttcgattgctgccaataggattttgacctgcttgtcggtcattgcatttagcacgttggcatcagcaaataattttaattcggtaccattcagcattcattgtggctccttactgtgcattgaatttaaatttcagattaagtatacactcaatctagtattttaaaagtcgcttagctgatttttatgtaaatttttgataaatgccatgaaaacggcttcttgaaaacttttgagagtaatggttgacctttatatctccgtgtgtataataagtgttggtaattgactgagtaactactcaaacaattgcccgaattcaaaccaatgaaagagggctaatacatgcgagagagtgtggaaatgaaagaacctaagaagaagtttttcagtagtacagaagatgctggcgacagcaagagcttagatgaggttaacggtagtatcatcgtgccgcaagatgcaggattttggcggacgttgataacttataccgggcctggaattctgattgccgttgggtatatggatcccggtaactggatcacatcaattgctggtggggctcaattcaagtacagcctgttatcagtggtcttgatctcaagtttgattgcgatgttgttacaatccatggcagctaaacttggaatcgtgaccggaaaagatttagctcagttgacccgtgaacgtaccagtaagcgagttggatttatcctttggatcatcactgaattagccattatggcaacggatgttgctgaaattattggttcagggattgcgttggaattactgttcaagattccattagtagttggcattttgattaccagtgccgatgtgttgatcctgttgctcttgatgagattaggcttcagaaagattgaagccattgtggccaccttggttgcagtgattttactggtcttctcatacgaagtattcttggcaggaccgaatatgcctgaactgttcgccggctatattccttcaacatcgatcgtcacgaacaagtcaatgctctacctggcacttgggattgttggtgcgacggttatgccccatgatttgttcctgggatcatcaatttcccagacacgtcgggttgaccggaagaatcgccaggatgttgccaaagcaatcaagttctcaacgattgattccaacatccagttgtcactggcatttatcgttaacagcttattgctggtattgggagctgccttgttcttcggtacgaacagttcagttggtcggttcgttgatttattcaacgctttgcaggattcacacattgttggcgccattgccagtccaattctgagtatgctgttcgccgtagccttactgtcatccggacaaagttcaacgattactgggacactttcaggacaaatcatcatggaaggtttcattcatctaaagatgccactttgggcacaacgattgattactcgtctgctttcagtcacaccagttttgatctttgccatttactatcacggcaatgaggctaagattgaaggattactgacagcatcacaagtgttcctgagtattgctttaccgtttgccatcatcccactggtcatgttcaccagtaacaagaagttgatgggtgagttcgccaatcgtacttgggtcaagtacgctgcttggttcgccaccattgtgctggtaaccttgaacgtctacctgattctccagacggttggcttgctgaaataaccgtttaaagacctttataaaaaataagtaggtttccgttatattctttataaaagtgtttagcagttgggagtcgttgacaatttaaaaatttgtctgcggcttcttttcttttagtctaagatagaggttaataactaacagggggattactaaatgatcaaacccgaaaagacaatcaatggaaccaaatggattgaaacgattcaaatcaatgccgaagaacgggcaaccctcgaagatcagtatggcattgatgaagatattattgagtacgtcactgataaagatgaaagtactaattatgtttatgatatcaatgaggacgaccaattattcatctttctggcgccgtatgcactcgataaagatgcactgagatacattacccagccatttggcatgctgcttcacaagggcgttttattcacgtttaaccaaagccacattcctgaagtcaacacggcactttactcggcattggataatcccgaggttaagagcgtcgatgcatttattctggaaacattgtttgcagttgttgacagctttatcccaatttctcgcggcattaccaagaaacgcaactatttggataaaatgttgaaccggaagactaagaacagtgatctggtttcactttcccatcttcaacagacgttgacttttttgtccagcgcagttcaaaccaatctcagtgaactcaatcgtttgccaaagacccattttggtgtcggtgctgaccaagataaaattgatttattcgaagacgtgcaaattgaaggagaacaggtccaacgaatgtttgagattgaaactcaagtcgttgaccgaatcgatcacacattcaacagtattgccaataacaacctgaacgatacaatgaaatttttgacaatttggtcactgaccatggctgtaccaacgatcattaccggattctatgggatgaacgtgaaactcccgttagccgggatgcaatacgcttggatgctgacgctggggatttctgtcgccttgattgtggcgatgctgattatgctgaaggtccggcggaagatgtgatgggtgagtgacttgctgctgggtgggggacttttttggagtgtgtatagttgagcagttatgctattttgagcacccttcggcttctgaaatacgctccgacgcaactggggctaacttctaaggggactttaattaaagccccaagaccagggccttcaatcaaagtccccttagaaaccgccccacccattgctcgtcgcgctgtggcgcgtttgttatgttattttgagcacccttcggcttctgaaatacgctccgacgacccaggacccggccacataaacaaaaacttccaatgatgaacaaagaccgttcatcattggaagttttcgcttatgttctgggtcctaaccgggtctcgtcgcgctctaatttttaccatttctttacccaatcaataccaagcaaaaacattacccttctatactaaaagtgttacattggaagttgcgagattgacaatgttgggagggttttacatgaaagaacaaaatgaatcatttgtcgcttcggccttatcagaaggagcaatccccgctgccggggaggccaccaacactttttccgttagtcagcctgctttgcgaaccctgaaaagtgtgaaagaacatgaaatccacttgcaaggggctttcaacgtccgcgatatgggcggctatccaaccaaagacggtctggtcgttaagagccacttactcctgcgatccgccaggttgaatgctttaacctccgcagacgtcaacacacttattaatacttataatttgggcgtcgactttgatctgcgtcgccccgaagaagtcagtgagttgcccgaccgctccttgccgggcgtgaaatgcattaacgattccgttgacactcgcgagacttactattatcaaattaatgctgaaaacaaccgcaagcactatcggacttatgtcacgtccgaacatgcgagaaaggtctatcataatctatttatggctttactggagaagcccatggggaaatcactgctctggcactgtgcgtctgggaaggatcgcactggtgtcgctgctgctttgatcctctacgtgttaggggttgattccaggaccatttttaaagattacgtggcctccaacgattttctcaagccacggattgacgcccgaatcgctcggctcaaagaaaagggtgccacccgttcagaaattaagtttgccaaagtcgatggcggcgttgatttgtcctacttgaaagctgcgatcgatgaagttaaacgtgattatggatctgttgctgatttcatcacaaatgggttgcacatcaccaaagaacaacaggcacgactacaagaaatgtacttggcataacaattgaataggtgttgaatcaggctattgggcagttatcgtccgatagccttttactttactaaaaaataatgaaagaataaccgatcttttcaggaagtacaataaatcctaactgacatatcaatttgcaaacctatgtaaatcgtccgcactaaataatataagcgcatacaacgttgttccaatgcaggaactaatggtatagggaattaaaaccttttgccaaaaatattttagtaaaagttaggaaaaacatattgacagcgctttcctataacgttattatgaagtcactgatatataagtgttcaaattttctcaggacgttcaaaatcgttgaatgtcgcaccggcacagacatacagccatttattatcaatcattatcaattgctgggtgaactttgggaaatgaatgcttttatatttgaagtgaaatgtaagcggttaatgcggttccaccgactaatcgcttatcggatgattgaactgaggaggcgtgaccagtaagtgattgattgaagtttgcgtaaaacttttggtaccacaataatattttatcgggagtgaaattcatggctaagaaagatgaagaaaaagacgctgtcaaaacaactgttggagttgttaccaacgccaaaattaaggatgaacaacaacccaagctaccttggatgatttcatccgcaatgtttttagcaccgctctgttggtatggtccaattggatcaactcgaagcgtgttaatcccccaattgtttgctcaattggatccggcacataaagtttgggcagttggtattttggcaacgattgcctcaattaccggtgcggttaccaacttactgtttggtgccttgtcagatgttacccggacacgatttggtaaacggaaaccatacattgtcttaggaacgattgccatcgcgatttcgttggtcttaattgccaacatgaaatcaattgttgccattattgccatttggatcgttgcggctgcggccgaaaacgcgattgccgcggcgatttacccgcagatttctgatcgggttgcgccaaaatggcgtgggacggtttctactttctacggtgttggctttaccatcgcccagcaagggtttgcgttgttagcggcccagttcctcggcaacgttaaatttggtatttacttcatggccggatgtaccgttattttggccctgatccacgagctgctgattcaagaaaagggtaatttggacgagcctaaagtcaagtttgacaaggacagcctgaagaaatatttcttcttcccaacccatgatgcccgcgacttctatctggccttatttggtaagttcttcatggttgttggttcaaccattgtcacaactttcctgctgttcatctttaccgactacattggtcaaagtactggacaagccggaacgtcaatctcaatctttagttcgatcatgctcttcatcggtgtcttctttgccttggttggtggcccacttgccgataaacttggtcgagttaaagccccagttgtgattgcaaccttcgccttgggtgctgccgcattattcccactgtttgtcaaagaaccatgggcaatgtttgcatacgccgttatcgctgcgtttggtaatgggttgtacaactctgttgatggtgccttgaacatggatgttttgccatcatccgatactgccggaaaagatttaggtttgattaatttggccaacacattaggtcaaatgcttggtgccatggttgcttcagcaattgttgaagcctttggttacggcgcaatctttatcttcgccattgggatggaactgattggtggaattgcgattgccatgattaaacgggttaagtaatcactgtttgatgaaagaaggataaataatgtctgttaattcagaagattggaaacaagctttacagtccaaagaggcgtttgccgattttatttacgattacttcaaggaccacaaagatttaaccggaaactatgagactcccagctattacgagtactacgttgtcactttggatagcaaagaaggcttgattatcacattgaagactgggttaaaccagaacactggtgatatcaatgcgccgctaccattcaaggatgttgaacatatttcagtcgaagacttccgtcaactggtcttgaacaagaaatttgaagatcaaagcgagagtttgactgacgtattctccaagatgttagcttcagagcccaacgcccgctttaaccgcggtcaagacggaaaatagctttgctcaaatgaattagaatcaggtcccgtattttggggcctgtttttttatgcccaattaaatatttagtaaaattaatgaaatgtttaatgaataatctaaatgtttattgacaaaatactgtaaagcgcttacattagaattagtgttcagactaagcaagaggagtgtgataaattcatggaaccagacattaaatggttagacgatcctgaaactttcagggtcggtatgctgccagcccacagcgatcatcaattttatcagagtgctgatgagattcgaaataatcacagcagttacgtgcaaagcttgaacggccagtggcaattcgcctatgccaaggatccaatgcaccggatcaaaaacttttatgctgctgattttgacagcagtgactttgatgcgatccaggtaccacagcatattgaatttgccggttacgacgattttcactacattaacacgatgtatccctgggaaggcaagatttaccgccgtcctgcgtacgcgcttgatcaaaatgatcaggaagccggtcaattcagtgaagcagtcgacaatccggtcggccactacattaaaaaattcactttgaactcagcattcaaagataaaaaggttcgcgtccgtttcgatggcgttgaaaaggcgatgtatgtttggctcaacggtcatttcttaggatatgccgaggacagttttaccccgtcagaattcgatttaaccccatatcttcaagatggtgagaatacgttggccgtggaagtcttcaaactcagcacggcggcatggctggaagatcaggacatgttccgtttctttgggatttttagggatgtttccttgattgcccaaccagaagctcacattgaagacctgtccattaaaccaaccttgagcgatgatttgaaagatggcactttgaatgtcaccacaaaaatgacagttaacaaatcgggtgccaccgccaaagtgtcggttaccgatgcagacggcaatggactgtacgcggattcccagtcggtggatgacgccatcactttgagtaacgtttcatttaaaaacgttcatttgtatgataaccatgatccttatttgtatcagctgacgattgaaattgatgatcaagatggtaacgtcttagaaatcgtgccttacaaatttggctttagaaagattgaaattaatcaagacaaggtcattacccttaacgggaagcgtttagtcatcaacggcgtcaaccgccacgagtgggattgtcattccggccgggtggtttccgttgacgatatgaaagccgacattcgaactttcaagcagaataacattaacgcggtgcggacctgtcattatcctgatcacacgctgtggtatcacctgtgtgacatcaacgggatttatgtcatggccgagaataatttggaatctcacggtacttggcaaaaactaggtgcagtggaaccatcttacaacgtgcctggatcggttcctcagtggaaagctgccgtgatcgaccgcgcccgcaacaactatgaaatgctgaagaatcatgccagcattctcttctggtcattaggtaatgaatcatatgccggcgatgacattgcggccatggaacaattctacaagcaggctgacccaaccagactggttcactatgaaggggttgttcaaaaccgcaagtatgaagatgtgatctcagacgttgaaagtcggatgtatgcttccccagacgaaatccaggattacctggatcataatccgaagaaaccattcctcttgtgcgaatacatgcatgacatgggtaactcacttggcgggatgaaatcctacattgatctgattgacaagtatccaatgtacgctggtgggtttatttgggactttatcgatcaggcaattgaagtcaatgacgaaatcaccggccaaaaagttctcagatatggcggcgatttcgatgaccggatgtctgactacgaattttccggtgatggattaatgtttgctgatcggaccgagaagccggcaatgcaggaggtgaaatactattatggacaacacaaataaacaattgcacttggtatatggcgatggtggcctcggcgttggcggtgacaatttccattacatcttcaattacacccgcggcggcatggaatcaatggtcgtcgatggtcgtgagtggatgtatcgtgagcctaagccaaccttctggcgggcaaccaccgataatgaccgtggtaatggtttctcgaaacaagctgttcaatggtatggcgccgatatgtttgccagtgccgataaagtcgatattaaaattaacgaccagttgattgaatttcccagtgcaccgcggaataatcagtattccaaccatgagtatgccgacaaagtagaagtgatttatcattttgcaaccctgacaattccaagtacggatgtcgaggttcactatacggtgacaggtgatggtgtgatcagcatccatgcccattatgccggtaatgatcaattgccggatttgccagtctttgggatgcgctttattttgccgactgccgcaaccggctacgaatatgctggcttgtccggtgaaacctatccggatcgcatggctggcgggattcccggcgagtatcgaattgacggcttgccagtaaccaactacatggttccccaagactgtggggtgcacatgaagaccgattgggtcacagtgacccgcaacgctaccaaagtcagctcggatcactcggacacaccgtttagcattaaatttgaaagtgacggccagccgtttgcctttagctgcctaccatatacggctgaagagctggaaaacgccactcatcaagaagaattgccattgccaagacggacggtcgtttcaatcttgggcgcagttcgtggtgttggcggcattgacagctggggtcgggatgttgaagagcagtatcacattcccgcaggaaaagatattgattttggttttaagattacgaaagcttaattgtttgaagcagccacgattggctgctttttatttaccataaagcacaattgaattaggaaaagaagtgccaaatttacttgtgttttagtaaaatgtgcagtatgattaacgctgtaaaagcgctttcaaaatacaatgatgaggtgattttaacagtgaaacgaaaattatttaatgaacaaattaaagacaacccactccgcagtaaagcggatgtcaaagctgccctggtcgacattttagcgcctgccatggaagttttggcgcaacaaaaacgaaagggccgcttccggatgagtgacagtggggccgtttacctccaagacaagaccgaagtggaaggtttcatgcgcctgctttggggcttagggccattctttagtgataaaaagcgggtatacgaacgtccagactggtacgagttggtgacgcaaggcatcttagccggaactgatcctgatgatcctgattactggggtggagatcttggtgactatgaccaggtcttcgtagagatgggcgctttgactgccttcttgtatgaaacaaaagattatttctgggataatttgaccgttaaaaagcaaaaaacgattgtcaaatggatggatcaggtgaaccacaaggtgattccaaagaccaactggttattcttccgtgcgatggtcaaccaatttatcactgattccggctacatggataattcagagttgatcgatgctgattatgcgatcaccaataaacattacctgggtcatggctggtcctacgatggttatgtcaaccagatcgataactacattccgtttgcctaccagttctttacgatcctaacggttggcttggcacacactgataacaagcaaagtcaattattgaaagaacgcgcccagaaatttgtcccaagttatgccaactggtttgccgctgatggtgctgccttgccatacggacgcagtttggattaccgatttgcccaggcagccttttgggcggcttatgcctatgcgcatgttgatatgcctgaagggtatagcttaggtgatatcaagcacttgctgttgaacaacctgcgttggtggttccagcagaacatcttccagacggatgggttgattccaatcggctatgcttatcccaatatgaattttgctgaaggttacaacgggccggcttctgcttactgggccttgaagacctttatcttctttgccttacctgatgatgatccgttctggaccaccaaagaaagtgatgacttcaagtttgaagctttgaagaagcagccggaacctagaatgctgattgcccacagtcaaaatggtttggaagttcagtcatttactgccggtcagcactcccacgagcatgcccatggtgaagccaagtatgagaagtatgtctactcaaccacctttggtttcagtacgcctaaaggatccgttcttttgaaacagggggcttatgataataccttggcagttgccgaatcggaaaacttctggcaaaccgccttcaagtacgatgattacgcaatccacgacaactacgtctactcagactggaagccgtacgatgatgttgaaatcaagaactttgttgtgccggcaatgccatggcatgtgcgggttcatgaagtcaataccggccgggagcttcatttggctgaaggcagtttctcagctcctgacagtggagcacctgatgaatatgaaatgaagaccagagcagctaatgccgttttctatcattcaagagtcggcattaccggattagtcggcttgtcaaaggaattgacaactgaattgtcaacgccggaacccaacaccaatctctacttcaataagaccaagattcccctgcaaactggtgttttggccccaggcaagtacaccttgatctcactgtatcttggtgatcgtgagctcgagagcctggatgatgatggcaagattgtgattccagaagtgaagttggatggcaataagctgacgatttcatttaatgatcacacggttggtgccgacttcgatgagttttaatggtaaatattgaacgaaatgtgcaactaaccaatggccactatgtcaccgcaaagaaggccatggttatcgaaaaatagttaaatgaaccaaaatgatttggttggttatttttatgattttttgggaagtggggttgtacattttgtactttgcccattttcgggagtcggcaagcggggcagttgttcagccgcagagtgccattaatatgattatctttatcgtatcgggtggcgttggcttgatgatcgtcttggcaatgctgtttgtcggccgctttcatctcagcaagaagacattcatggttctttctgcagaacttgttcgtctgcaaaagggcggtagtatgagtgatgtggatccacaccccaaggcagtttgtgaggatttgaccggcgttaaatatgattcaattgaggtttggaagaaagatgaccaaccgcaaaataaatcacggggttagccggttttgggattaaatctcctcaagtcgatttgattgaccacaacctgcttcgggtagatacttttgttgaaataacaagttatctatttggggaggattcacatgacaaatttagtgattaaaaaagacgttgaatatgatgctgttcaccaccagttaactgacatttattatgatggcgaaaaggcgcaaagcaaaggcgcaatcattgatatccatggtggcggttggttccgcggcaacaagtccaaagatgaggattcctcgatccggtttgtggaagccggctacctggttgtaacgccggcttatcgaattacgtcagcggctttctatccggcacctttggaagatatggatcacttgtatgaatggttgaagaaatccgacttgccgttcaaccacgaccatatcggggcatttggctcgtccgccggtggcaacatgaccgtcgaattggcaatcaaatatggcattccgattgcctcactgtctggcattttggatattgataagtggttgagcgagcatgaagatgtggttgccgcagaaggtgacacgagtggctttaattcaaccgccagctcgaatattaaccagactggggccaacgatccgttttataagtggtttgtgaccaactactttaacggccggaccgaccaatacaccgaagccactccggttcatcgagtaaccgaccagactggtcagatgtatttggccaattcactgaatgaatttgtgccaaccagtggagtcctggacatggctcaagctttgaccaaacaccaaattccttatcgaacccggatgttaaccggtagtcgtcacgctaagggatacctggatgatgtctgggatgacgtggttgggttctttgctcaaaccttataatgcggtacacttaataggagcgcggtgacagctgtttacctggatgactaggctcagctggtaactgacgtcatcgcgaaataatcagtgtacgcaaaagtggccgaaacgaaagttttgcttttgttcggccgcttttttacataatgaaacggggtcacaatggatgattaagaataaaatgtcttggggaaaggaattctggttggcagccctttttctggtcctcttgatgggtgtcgacttttcggtccggggagcagggccactggtttgcggcggtgcccgactgatgtttgcgctggtcgttgccggaattgttttctatgtactgggaacgatgaaaatttttcagactaaagtcaagttggggacttttgccaaaatctggggattcatttttggcatttgcctgggtggattattcctattgattagcattctcggtcacacggctttgatgatgcatgccaaaacggtggttgccgataccatgatggcattgtcagcgggaatctttgaagaattcctgtgtcggggattgttgttctcggcattcctgagcgtcttcaaacaggccaaatataagtttaccgaggccgcgttggcttccggaatcttcttcggcctctttcatttcatgaatctgatctcagggcagggctttttaccaacccttcaacaggcgacctacgcttttgtgattggggcgatttttgcatcaatcaggttgacgaccaataccttaacctgggtggttctgattcatgcgttaatcgattggcagccgggaatttcggtgactcatacggttagtgcactggcgtcgtggccggttttcctggcagtttggggaacaattctggtcgtgaccgtgatttttctgatttcgtttgatagtagttatcggcagagtgtgaaagaggacgtctagcaattggattttaagcccctccagacggaaaccgagtcaggttttcggctggaggggcttaaaatccgattgctgtcctctttcacacgtttaatcaagataaaagtgagacacaacgaaaccgagtcaggttttcgggtggaggggcttaaaatccaattgttgtcctctttcacacgtttaagctctaacataataaaatgcggctgaacaaaaggatcaccttttgcccagccgcattttgttgaggaaatttttaagctgttttgatctttaccagtaacccaaaaccttggttaacttggcacgattaatatctctggaagataatttatcctggaaaatcgcgtaatcatcgttgactactttggattggctccaggagtacttcgcgtcaccgctcttagttcccgaatcagcttccataatatcattggagtacggggtgtgatccaagccaaggctgtggcccagttcatgggtaatcactgatttccagtaggtgtcatagagtgcctggtaatctgcactgtttggctgatcagctgatggcagtgcatgaccggtctcagctttgtagacagccggcaggtacttggtgttgtcgaagaaattatagttgatgtaaagcttgctggtaatgtaatagccatcccagctgccttgcccggtcccagcatttttaaagcccactgtaatcgtgtggtcagctttggtgcctaatttaaacgctttggttttgagggccttgttccaattctgcatcgcggcgtaggtataagacttcaatgattgattggctacgtagacctttgccgtatgatttttgaagatgccctgggcactcattggttggacattgtaccagcggtcaaagacctgccaatatttgtcatagatataagcggggtatttgcggacacttgatgttggattcaaatcaggggtgcttttgatggccttggcaaccgttttgccggcaatccgctgagttgatttggcataagtaatcggactttgaggcatgttcaacgtcaatggcaccgctaaagcaaaggtggcactggcgactgcggcgagaatgaaacttctttttttcataaggaaccctctcttgaagttacataaaatcattttgcctgaataatagcattccaatcaagatcgttcaagaaatcttgcttcaaaccaagcggtcttaatgaaggcttatgaattattgcaggggatagactaaattgtaccaagtttccccggcatgactggatgctgaaatgccttcgttttgatagccattgctttcataaaatgggatcaggtctgccagacaggtcagggtgatagccactctgctttgtgctttggcaacctgagccaattcgctcagcaggcggctggcaatgccatggccgcgaaaatcgggatggaccgccaagctgaggaccgtttgataaggatcatctcgacggttggcgtgggcctgttcaaatagttcatctgtcagataccgttgtgaaaatgccggaccgacgatgtaaccgaccacttgattggcctcatttgtggcgacaataaatgtgtccggatacaaccggattctttccgccatcgcagttttggtggctgcctcggccggcgaaaagcctgcttcttcgatcaccataattgcggtcaactcatccatccttgccggttgataatgtaatttcaattcggacctccattagcttgtggtatcattaattgcgtaccattttattaataatgattatcataacacgataggggtcttcacaaaatgaatcattcaaatattggacatcgtaatcgcggggtgatcctgatcgcggtctttatcgcgacgtttatgacttccgttgaagtgaccatcgtgacgacggcactgccctcaattattagcgaacttcatgggctggcttatcaaagctggattatgagtgcctatctgttgacgactgcgatcacgacaccaatctacggcaagttggccgatacgttgggccgacgaaaagtatttcagtggggtgtgaccgtcttcaccatcggctcgcttttaagcggattgtcaccttcgattttattcttgatcgtcgcccgggcaattcagggaattggggccggtgcggtcatgccactgacgtttacgatcatcgccgatattttttcgtttgaacagcgggcaaatgtgctggcactcaataataccgcctggggactgtcagccttggtcggcccgctgattggcggttttttagtggaccatctttcctggcactgggtattcttcgtcaacgtgcccttgggcatcatcgtcgccctgctgatctggctggggtatcaggaaaatattgagctcaagaatcagctgatcattgattggctggggattatctggctggcaatttcactggtcagcttattgctggggattcaggcattggacacgctgccgctgattgcagccagcctgttgatagtgacgattgtggcaacttggttatttcttcgccatgaaaagcatttcgcagacccgttaatctcaccaaaaatgtttcattccaaaacctttaccattcaaattatcacagcaacaattttgagtggggtcttaattggttatcaaatgtatttcccaatttggctgcaatcattgtatcgggtatccgcaaccactgccgggttagtcgtgacctccagctcaatcatgtggctggtcgcctcgttttttgtcggtaaattgattgcccactttgttcccaaacaaattgcagtgaccttgattggtgtgatgctgctcagttatttgtcactgatctttgccagtcaagcatttccggtctgggcattttatgtgattgccatgattaatgggattggaatggggatcgttgtcagcatgaatacgattcttagccagcatttggttcccaatgaaatggtcggttcggcgacttcagtcctcacccttggtcgttccttgggccaaacggtgatggccggggtgtatggtgcaatcttgaatttagtgattcgattgcagctgcacggcggaatcaccttttcaaaggtcaataacgtcatcagttccaaaggggccgccgtggtggccaatcggtcgctgattgatccaatcatcctgacagcccttcatatggtgtttgtcggggtggtcgcgatgttggtagttgtcttggtaatcaatattttagatcctaataaaaaaattattcgttgatcgttgtggaaattagcacgaaaaaagaggtcggacatcaatttgtccggcctcttagcgtattgtgccgttcaaaagcaatcggcattagctgggaatttgatttgcccagcttattttgtggatcctggcaccccggcaaccgtctgaaagacgtcagccaatgaggtatgcatgtcggcgaatttcttgttgaggataagctgacggaattcttcaaccgagatggtttcaacatctttgaaaggaattgtcggcgcatcggcgttaaccgttggattaatcgagctgaccaaggtgatcactaggcccttttcgctgttcaaagtgacagtatagtactcgtagtatgaaggagtttcgtaattaccggtcagttccttgtggtccttaaaatagttgatgataaagtcgttgaatgcctttggtgattttaatgatgctttccaatctgtgtttgtcatagtcaaacttcctttcgtgtctcaatcagtttcaaaatggggtaagaggtggataactaacatattagagctgatatttctctcttgcttcaattgttattctaaacacttctcaaattaatacaagtggaaacatcaatgaaaacgttgacagttatggatttgttttaatttgttgattggaagcgttattttcgtcagaatgagctgaatcatcagaaaacactactgatatgttagtatcctgctgggagcttcatagatcaacacgcgattagcttgctttgtgagccgttttgtaagaacataacagcagagattcagattttttcgagaaagtggtgatgaaatggcaacaggctatattggtcggattcgaaaacgcgtgggccacatgcctttaattttgaatacggccgctggaatcctattaaatgatcagtaccaagtactcttaaatttaagaaccgatagtcataactggagtttgccgggtggctacatggagttcggtgaaacatatgcccagacttgtgtgcgtgagtatcaagaagatagcggcgtaaaagttgagattgtccggccgctcggattattcgatcagggaatcttcgcctatccaaatggtgatcaggtgcagacaattgatcggctgtttttagtcaggaaagttggcggccaattgctgtccgctgagactgacgagaccattcgactggactatttcgattttgatgacctaccgccactgctgaatcagcagacggaaaagatgctggcatttgccaaagaaaatgtataggggggacttgatgatggctgataaagtactcgttccggctcaattgcatccggacggaaaacgttatttacgtgagcacggcctggaagtcgtggaattgatgcgggctaacgctgaaaatattttgaagaatggcaaggatgctgccgcaatgattttatttttggatccagtcggcgagaatgtgatttctcacatgcccaatttgaagattattgcccgacacggcgtcggctatgacagtgtggacttggatgccagcgccaatcacggtgtttgggtgaccaatacgcccaatgccaatgcggcaactgtggctgaaacgactttggcagagatcatggacgtgtctaagcacattaccaaaaactcgatggaaatgcgggatggcaactttacctacccgttggctcatttgggattcgatcttgaagggaaaactttggggattcttggttacggcaaaattggccgtctggtggccaaaaaagctagtgcgctagggatgcgaattatgattcataaccggaccccacgggaatcaccatacggggaatttgtcgatctcgataccttagtaaaatctgcggatattttgaccctccatttagctgccaattctcagacccgacacattatcggtcgaaagcaattggcagagatgaagccgaccagtgttttgatcaacctgggtcgtggtgccctggttgataccgctgcgttgattgatgcacttaaaagcggctcgattagtggtgctgctcttgacgtctttgacgaagagcccttaccaatgaacagtgggttattcaagctggataatgtgttattgacaccccacattggttccagtacggttgaaagcttttcaagaatggccacggatgcggcaagtgaagtggttcgggtcttgaatggccagcagccgcagtggccggttaaccaaccccattagttttctggaaaatttaaataaatagattgtacacaactcatatagcgcgtatagttaggttggatcaacaaattatacaagggaagcgtttctcatgacaaaaacatacaaagcagaaattacttcattgaatggcgacaagattggtactcatcctactggtgaggccacatttacgattgatggcgatacactaactgttgaaatcacgatggatcatacgtcaccaaacacccaacactggatgcattttcacggtttcccagatggcagggatgctcaaccggcaactgccgcccaagacaccaaccatgacggctacgttgacttgccggaaaccgaaccagtgtccggaacgacaatggtcccgtttaacgacgctccggagaagatggatatcccaactgacacttacccaacttctgatgccgacggtcatttccactacgagaagacagtgccgttgggcgaaatcagcgagaagttcaaggaagtctttaatgatgccgacctccaccttgagaagcgggtggtttacattcacggggttcctcagtcgatggatttacctgataccatccaaggtgccgttggtaaatatgatcagcatacgacgttgcctattgctgttggcaagattgttgaagcctaaattaattcagatctattcaggagttgaaatgattcgactactgaatagatcttttttgattgcttcctccagccagcagcaagtctgccatttgccatcatttttggtaattgatgcaaaggtatacagacttaagaatgtttgagataatcaaattgatggtatagaaaagaggggcgattatggaaaataaattcaatcttactctcaaacaaaatcgctttcttacgaaaaagaatcttgtcaatatggtgtattctaattcaaaatttgagggagttaatacgactctgccgcaaaccaagacgattattgacggcatgagtgtcgctggtgtttcgattgatgatattcaggtcatcattagtctcaaaaaagggttggaatttgtattaagtcacagtgaaccatttcgattagatatttgtcggcaaattaatcgaatcgtcgcggccgaagatgccctcgtccccggacaaattcggactggaagtgtccagatcggcggtgttcagtatgtaccgccagttccagatgtcaataatgtcaaaagcgtaattcaaaaaataatgggtgatgatcagactgctactgaaaaggcgcttcaaataatgtatgagattatgcggcagcagatcttctgggatggtaacaagcggactgctattttgtctgccaattatattttgattaattccggtgccggaattgttaatatcaatgaaaaccaattagaaacctttaacacattactggccgattattacgaaactggtgatttacaggccatcatgcagtggacatacgataattgtttatatggcattgaatttaaataactgtcatttataacccattcagccccaatcaaaaagtcttcgggatttttgattggggctgaatgatttgattattcaattaagtagttagttggtggctttaaattctttaatcccttgttgcagccggttcaagccatcttcaaccatggttttcggactggcaatattcattcgcaagaagtggttgccatcaccgccatacacatcgccggcagaaagatacaggccggtttgggcgcgaatgaaagcggctaattttgccgagtcgtcggtcagttggctgacgtcgatccagaccaaataggtggcagttgacggaaccacgacaatttcgtgaatgtttgcctggcagaatttgacgaccatttcgtaatttgcccgaatttggtttctcagttcatggacccagtcgcccgctttggtgtaggcggcaatggtgcccggaatcgccaagaggttgggttcgccgagttcatcggtgttaattccccggttcactttgctgcgcagggcttcgtttggaacgatgaccgttgcggcgtgcagggcggcaacattaaatgttttgctgggtgagacgcagacgatgacgttttgcagcagctcatttggcaatgagaacactggcgtgtagtcagcacccttaaacaccaagtcgccgtgaatttcatctgacagcagggtgacgctgtgtttgagacagagctggttaattttaataagttcagctttggtccacacttttccaattgggttgtgtgggttgcacaagatcatcatggtggtcagcggctcggccagtttggcgtccaaatcatcccaatcaatctgatactggtgggctttttgatcatagaccagatcggatgacaacacatggcgaccattgttcacgatggaattatagaaaatattgtaaaccggcgcttgaaccaggacgttatcgcccacattggtgacgcggcgaacagctgaggatatcgtcggcacaacgccagtcgaaaagaacatccaatcccggttgattgtcgcatgatgttccgtttggtaccagtgggcaactgcatcaaaataatcggtgtgcggttcctcgtatccgaagatgccaaagtcaactttttgacgcattgcatcgagaatctcgggagcgaccttgaagtccatgtcggcgacccacattggcagctcattaggtttgacatcccatttaactgaatcggtatttcgccgcgaaatcattgaagtaaagtcatacattaggctgtctcctttttagatgttttgttatcagtaatgatagtcgttttacttggatcgactttggtagggtcaataataacctcaccgattgaacgagcatgaatggtgccgctgattggatttttgacactcatgatgtttgagttgatttctgcgtcaatgtcagaacagtattcaaatgccaaatcggtccgcagtaagcggcagttacgcatcgtgaggtgatcaatgtagcataacccctgatcgctttcaatcgtacagttgatcagcgtgaggttcttcgtattccatgccagatattcaccgttaattgtggaatcgacgatcttgacgttttcgcagttccagaaagcatctttggacacgagagttgaatgatggacctcgacatttttggcaccgtcaaagacatagttgccaattagattcagatggtcaacggaaatgttttcactattcatgccaaaataatctccgttggcctggacgttgttgatcttgatgttttgacagttccagagggtttctttggcgtcggaaaagtggtcgttattcagcgtgatatcactgcagcgcctgaaaattttgggcgcttgaatcgcactgtcgttgatttcaatatcgtgagtgtaccagattcctgaacgggccatggtttctaagatcgagtggtcaaccttgacgtgtttgctgtaccacagtgggtatttgtaggtaaaaattgaatcgattaagtgaatgttgcgactttctttgagaggggattccccggtgccaaatgtggtgccggaaatgtccgcgttggtttcggcaaacagtggtcgttcaccgtcaaaatattgatttgtgtattgtttcattatgactccttattattttgattaattaattgttttctgaaaaggtcttaatttcagtatactcgtttccaacaaattggtgactaggatttaaatgggattggtttcactataaactttgaagtggactctaagtcaagggcgtttcagcgataacttttgattaatgtcatcagtaccaaaaaccactgctataatgtaagtggaggtgcagattatgacaacaatttatgttgacccttccaaaaagaaggaacagatcgttaaactgtctgatggcacgtttggtttgatgaaagctgaaaagcaaaagtctgggattggttatgagtttgactttaccagccacatgcaccccagcttcagaatcccgcatgcaccggttaatggggatgaagaaaccgttcattcgattgacggcgagcagcagtttaagattcagtggttgagcaagtgattcttcagttagcaggcggcttggctgacagatttaaggggataaatcgattatttccggcttgaaataatggctttatttgcttaaatgctgatgagttgtcaagatcgccgttttaactgaaaatccggctgaattgaatccattctcactttcagggtctgagcacgcttgataatgctcaggctttttttacacccattttttcatggttcttattcctgttcacttatcgttttggccttataatcaaggtgttaagaatcagctatctggatgggaggcattattatgcgagcagcatatattacacaaaatggtgaggcaaaggacatcaagattggtgagttgccgaagcctgaaattaccaatgatgaagtgttaattaaagtgaatgcggtggccgtcaaccatgtcgacacgtttgtccgttcgggatcttttaaaaccgataccaattttccgtttgtgatcggcagggatgccgttggtcaagttgaagaagtcggagctgacgtcaccggtttttccaaaggcaactgggtttggaccaacagcatgggctatgccggccgccaaggggtgaccagcgagtacgctgccattcccgcggccagactattccatgtgcccgaacacgtggagccgactcaattggtggccgccgttcattcagcggcaactgccgcaatcgtgttgaccaaagtgtttggggccgtctccggagcatcaatcctggttgaaggcgccgccggccacgttggaacaaagtttgtccagatggcccacattatgggactcaaggtggtcacgacttccaacacgagcgactttgacctgctggatcgcttgggaagcgatcaatgtctgaattacgataagtcattaaagaaacagctctccaaggctgaaattcaaaaagttgactatgtggtcgatacctctgggcaagttcaactccaggataatttacgggcattgaagccgggcggcaaagtctgcttgattacagcaccaaagagcaatcaattctcgtttgacgtccgtcagttttatacccagtcaaagacaatcagcgggtttgtgatcagcaacgcgccactggatcaaattcaagatgcggctaagtttattaatcggctgatggctgacggttatctgctggaggacccggttttggagaagtcctacgaggatgctgcgtgggctcacaagaagttggaaaagaatgccaagaagaaaaagattctcctcaaattttaataagcaaaacatttaggaaattaaaataaatcagttatactgtacttgtagataggaaacgcttacaaggaggtatgacatatggggaaattagataacaaagttgcaattattactggtgcatctcaaggaatgggcgccagtcacgccaagatgttcgttaacgaaggcgctaaagttgcgcttaccgatattaacgcagaaaaagggaacgctctggctgatgaattaggcgataacgttatttttatcaagcaggatgtttccagtgaagatgattggaagaacgtcattgatgaaacggtgaagaagttcggtaagctggatattctggttaataatgccggaatcagttttaacaaaccgctttccgatatcactctcgatgactacatgaagatctttaagatcaaccagctttccgtcttcttggggatgaaatacgcagctgaagccatgaagaagaatggcagcggcagtatcgttaatatttcatcaatgaacggtctggttggtggtgcgattggttacaccgataccaagtttgccgttcgtgggatgactaaagctgcagcattgcagttggccggttctcacatccgggttaactcggttcacccaggggtaatttccaccccaatgattcaccaaggtgatagtgaagaagtcatcaagcagtttgcaaaatcaattccgctgcaaagagtggcagaacctgaagaagtatcaaaaatggtgctcttcttagcatcagatgacgctagctactcaacaggatctgaattcgtgattgatggtggaatgacagcgatgtaactgaatgcggtggtgttgggatgccaacatctaactgaattcaaaaaagccgttggacaaaagaaatcaacttttgtctcaacggctttttagattgtttaatggccaaacttcaaatgcaacgtatagatgaatttatacgaacgcatcttttcagctctggaatggactgcgtggccgaataaaggctttttggccggttccagttgatgcagctctaacagcattcgagcctcaccatcaccatgaatggcgcgatacttcaattcgttttcagctgctttggcgaccagtgcttcagaccagcaacgcggactgagccgtgtgtataggtcataattgctttcattttccatgattatgtagacgctcccccgaaactcaactatttgtataatgaaatcactatctataagattatgattttttcgccaataagtcaattagggtttgtaccaattcaaaaaggatcaggcaatcatttctagagggaaataattgtctgatcctttactcaagatgctgcatccacacagtactaagccagattctggttataaacgtaattcatcaaggaccgggtttcggtaaactcgttttcgtcatgcaggacaaccgtgataatccggtcatggcctgacttacgaccagttccgacgaagcagtaacccgccggatcggtgtagccggtctttaagccatcaacgttcagggacttttgataatactttcgtcctggcagcaggttattgtagttgtgaagcgtttgaccatcgaccttcattgatttaactgaagcgtcggtcaaaatatcgttgtaatcaacaacgaagtgacgggaaatttgagcaatatcgctggctgaaacgtaattggcattcttggaagcaccaatactgtaaccataaggagccaaactattctgttccatcccggaagccgaaacaaatgatgagtgcttcaatccccattccttggcttgattattcatcatgccaatgaattttttgttgtaatcaggcgttgaaccgccggcaacccattgtccaagggcaattgcggcgttattggatgattcaatcagacctgccaggtacaactgacgaacagtgtagctgttgtggttaaatttaaagccgccgaagacattggatttacctaatttcttcaaaccggcattactcgtggtgaccttactggaccaagtacctttgccttgagaaatcttttgacgaaccaggtagagggtcatcagtttggaaagagaagcgatgggtcgagcagtgttggcgttttttgtccacacgttattattggtattgacatccaaagcgaccgcagacttggcatatttgagcccaaatggtgaggtgccggcctttaagtacttatgccaaacaatgccagaaactgttccggaaccatttttcactttatagtagagtgcttttgaactgccatgcttcaaagtcaccttggccgtcgcgtaccaggtggtgtacgggtaggtctttaaatttgcaaccttcttggtgtgtgaagcgttatacaccgcgcccttggtcgaacttttgtgatagggcgtcttctttatcgctgtggttgagacagttttataggaacttgaactggcgttgaccgtacgcgtctgcccccaaagtcccattccaattgtgattgtggttgcacaggtaaccagtgccaatcgcaaaaattgattcattttcatatataatctcctcctcattcaataaaaagtgtaacattcaacctttgcccactttgtctttttaacaaaactgtaaaagaactgtttgatcggagtaattctgtgagttctaattaatattggtgaaatagtctggaaatttatcaagcactgattgttgttcgctgagcattaaattgagatggctataaaccagttggtgtacctttgccgcatcatggtcactgaaggcattgataatatctcgatgttcttgggtcagtctgttcatgggcaggttggcgtcataaactctgagcagccgatagcgattcaggtcggtactgaaactgattagccaattccaaatattttgtttgttggcaaactcgtaaatcttttgatgaaaatggttgtccatttgaaagaatcgttggatctgatcacgtttggaggccgtttgctgttcttcgaccacagctgacagctgatcgatttggtcatcggaaacagtgccaccgattgacttggcgatgtctgattccaacaactggcgggcatagcgggcatccagtgattttttcaggtcaattcgagtgacgtaagtgccgctttggggaagcgagtaaagcatgtcgtcccgccgcaaacggagcatggcttctctaacaggggtccggctaaccccaatttcttcttcaaattgtttgtcggagacttgttgaccggggtacaaatccagattcatgattttggtatagattgcgttataggccttgtcttgtaaactttccatgtcatctcatctttctttttttaaaatcgatccactgagaatatgttaccatattaattattttcctgaaccgtcaaagtgaatgaaatggggtggcagcgactttgaccgggaattttaaaagtgatatattagtagcacattaatggtttggaaaggacgattgtcttgaaaatagggttcagatggttcggcgagcagaatgatccggttcaactggcggagattcgccaaataccaggggtttctcaggccgtcacggcactttatgacgttcctgtcggtgaggtgtggccaaaggatcgaattgctcagctgaagcaagcggtcaccagtgccggcttgggttttgaagtgattgaatcggtcaatgttcatgatgatatcaagaccggtcagcctggacgggatcaatatattgaaaattatcagcagaccatcaagaacctggctgaagccggcgtgaaggtgatttgctacaattttatgccggtatttgactggctgcggaccgatctaacctatcagttgccggatggctcgaatgccatggcttaccagcctgaaatgttacctgatgatccgaatgaactgattcaccaaattatgtcgggctccaagggctttgaaatgccaggctgggagcctgaacgcttggcccatgtccaacaattatttgccaaatatcgggatgtggacgctgaccaattacggtcaaatttaaaatattttctggatgccatcatgcccacttgtgaaaagtatgacgtccgaatggcaatgcatcccgacgacccgccatttccattgtttggcttaccacggatttataaaaaccgcgatgatatgctcaaaattgagcagctgtacgaatcaccctataacgccttcacgatttgtaccgggagcctgggagagaatccacaaaatgacgtgccggcaatcatccgcgaatttgttcaaaaaaaccgcgcaccgttcattcatgctcgtaatatccgcttcatgaaccagacaaaaacagccttccatgagtctgctcatttgtcgtcggccggatcactggatatgtatgagattgtcaaggcactggcagacaacgattatgagggctatctccgaccagatcatgggcgaaatatctggggtgaacagggacggccagggtatgggttgtacgaccgggcactgggagtgacctatttgaatgggttgtgggaaaccatccggaagaatcaataggactttggacagatgagcttaattatatttgttttaactatgaacgagtatatattaaaggggttgccggcaaaatgattagttttgtcgcaaccccttttgcattctcttagtgtgtaccgattaccgagccgaacagtgggaaaacaagcagcttccggccggataaggggattatctaaatatccaaaccctggatatttagataatccccttatcctctggaagctaaacgcttgttttcccacgctgattgttatctattaactggatttttccctttgccattgttagaaatcatcgccgccttgatctcggcatctgaagaaaggttaaagtccccagggatggtcagcttcaaaactgcagccgccatcgcataatcaagctgatactgcggattgaaattgtggccgattccatggacaatggccgcgccgaatgcgtcaccaccagcaacctcagggagaacttcgacatcgtaaatcgggctctcatagaattgaccttgataattcatgattcccatccattggctgctttggggactatgaatgttccgtaagatactggccacggttgtgatgttggggaacttcgccacgagggtcgtgattgcttgcttaaatgtggccttttgatcgatcgcttggtggttggccgattgaaaggctttgatgccaaaggcctgctcgatatcttcgtcgtggaccagacaaacatcgacgagcggcagaatttgtgggttaaacgcaactgcttgatcagacgtccagagttttcctcgaaaattagcatcgtaaatcactttgatagcgtgattgcggcagaacttaacggctgataaaagaatcatctgtaggttagttgaaagggcagcggtgatccccgaaatatagaaaacatccgtctgatccagtagttgattccacggataatcagccgcttctgatgttgcaaaggcactggtcgcccgatcataaatcacgtcactggctcgttgactgacgccttgctggagaaaatacagaccgattcggctgccgccgcgacgaatgcggctggtgtcgacgccgaacgcctttagttttgaaatggcggtgtcgccgatttcgttgttggggagtttggtgataaaggccgcttgatcccccagcaaagccagtgaaacggcaacgttggcttccgcaccgccataattggcattgaacgaagtcgcctgaaccaacttctgattatccggaaccgtcagccttaacatgatctctccaaaagttgtcacccgcatcgcaaaaatctccaatcgttatcattacttgtatctgtataataccatattaattggtgccaaaacgcgcgactgatgcggacgttgacacttttaaactgattgtgacagaattaattgagataataaaaggtccgaccactcagttagagaaggccgaaccttatttagatggttattgatttgatgagtcgtccgaatcgtcattggattcattgtcggattgatggcttgaatcgttggtggttgtgggttgatttccagaagtggctgccggtgtaacattgattcgatcggcttcttgatggacctgcgcttcgtgttcatccaccaactcgcgatagaaattggcaaaactgagttgcatataaggttgaacccagatggccgcaatccccagggtaatgccaaccaacagtccccagccaatgaagctgagggccattacaaagtaatcccacttatggccgtccattaattgacgactgcgggtaatggcatccaaataactgattttttcgccccggtcaacggcatcgcggtagatgtataatgcctgggagtaggcgacggctttaataagcccaggaatgatcaacagaatcatccaaagaataatcaaaacctgctcaatgatgtaaatgacaatggttcccaagaaatagtcaacgttgttgaagatggtcatcgacttttgcagcggctgatcataggtcaacttttgtcgcatcgcgtcgatacagataaaggcgacgccaatggcgaccagagacccgagcagaattagaatcatgccgaaagtctgggcactggtccagattggttcaccgttaatatcgtaaagctcttcttttggcgcatagatatagccgccaacaaattcaagaataaatactggtaaaaatagcaaaaagaaaaatttaaaatgagcatttaataggctcttagagtctagttttaacgcttttctatccataatcacaacccccgtcaatttaaaatatctttacaagttaattatagtgcaacctgttgaattcacttagtaaaacgtcctttatgcctgcttactcgtctggataagatcatccaccactaatttgtacagcagtgacttaattgccattgattggtactgtttagctgacaaatgatcagcgtccacatctgtcagctcctgattgaacaggtcaatgaactgatcataagctttgggggcggagtcgagtttgagggcgattttcattgcctggtcgatggtatccagcgataaaattggcttgagcagactcaccaccagaattttggccaagtgaacccgtgagtagcgcttcttggtcgggcggtcaaccaggccttttttaacgtaactgttgatcatggatttggtaatctcagtgtgggtgattggtgccaaatattggttgacctcgtcaatcacttgatccatatacaaatccaaattaggtaaatcttcaaagtgcggcatggtcatcgccgctaattttttggtaaaattatctttagtcatggtattccccttcgaattgaatactagtattattgcataggatagtcgaaaaataaagtacgtagactttaaaactatgttatcttgacttagaaaatagaatagcttattatgatgctaaggaggcatcgtgatgaatgaattaatggctaaaaggcgtcatcaacaaattatctatgaggtattaaatgctgtcacccacggtgtttcgttttttgtggcgatttggttgtccattttattagtgaacaaagctttacgtgatgggctttcgatgggggcaattgtcagcttgatcatctacagtgcgacagttctctcactctatttggcgtcaacgttgctccactgttttgtttttaccaaagccaaacgcgtctttcagatcctggatcatagcaatattttcatcttgattgccggaacgtacactccttattgtgtcatttttgtccacaactgggctggcaaccttctgttggccagtgtctgggtgttggcaattggtgggatcatcagccacgttgtctttcatggcagatttcaaaagactgaaaccaccatttatgtggtgatgggctggttatgtatgttcttgggcaaagcgctatatgacaatttgagcaccagcggtttttggctgctggttgccggcggcgtgacttttaccgtgggagcattgatttacagcattcccagagttccagggatgcacttaatctggcacttcttcgtgatgggcggcacactgaccatgtttctctcgattttctttaatatttaaagattattaaattaggcttgacttatttctcagtggtggtaaattacatgtatcaacaaattaaaaataaataataaacatgaagttacgattagaaaagtaattgcttaactcacataaagagagccccgctggtgagaaggggatgtgagtggcagtgaacacacatctatgaactggttagctgaaccaagtaggctatcccgctagtgagcgttaccacggctactgtaactgttctccaatttggacgactagttacgagcagcgtaaggtcgtttttgtaagaaaacgatgaacgtgaggtggaaccgcgaaagatcgtcctcagatattgcttcggcaatgtctggggacttttttatttcataggatttgattgtaatgaatgtttggttatctgaaatggagagtggcttatatgcaaattattgaagattccttagaccaattattgaaacaggttgccatcaggaccaacgcggttgctaaccgtgaagaagttgaaaaatcagtgcgggaaattatcgccaatgtcatcaaagatggtgatcaggcagtgaaaatgtacgaacagaaatttgataatgtcgagctggagagtttgaaagtcacccaacaggaaattgacgatgcctatgaagcgactgatgacacagtgattaaagccttggaacttgccaaagctaatattacgtcatttcaccaaatggaagtggaagacagttttattgatgcgaaaaagaaaggcgttattcgcggtgaaaaaatcgccccactggcagcagttgggctctacgttccaggtgggacggcagcttatccgtcttccattttgatgaacgtcattccagccaagattgccggggtttcaagaattgtcatggttacgccaccacaaaaggacgggttaaataaggcggtcttggcggctgctaaaattgccggggttgatgaaatttatacggttggcggtgcccaagccattgctagtttggcatacggaactgaaacggtgccacgggtggataagattaccggacccggtaacgtgtttgtcgcaacggcgaaaaagcaggtgtttggtcaggtcgacatcgacatgattgccggtccctcagaaattggtgtgatcgccgggtcccaggcggttcccagccaggttgcttcggatttattgtctcaagcagaacatgacaaattggcccgaccaattttagtcaccgatgaccgttcactggccgaagctgtcagcaaggagatggatcgccaagttgatttactgcccagaaaggaaattgccaaagcagcgatggataatgaaggcttcattgccgtcgtagacgatattgacgatgcctttaccctgatgaatgccgttgccccggaacatttggaagtccaattacccgatgccattgaatacttgaaccaaatcaaaaacgccggctccgtcttccttggattttcagcttccgagcccctgggcgactacctcgcaggccctaatcacatcttaccaaccgggggcacggcacggttcttctcgccgctcggagttcaagattttgttaaacggacacaatttgtttcctatactagggatgccctgaaaaatgaaaaggatgccatcacgactctggcacgggttgaaggtctcgaagcccacgccagggcaattgaaagccgctttgacgattaaagtgtaaaaggttgtcgtgagttcgtaacattgtttacaaaaacagtcatcagccggttgattcgatgcaaactgatcaaacaaatagttttccaatccagtgccctattgcctttgacagaacctttatgtcaaaggctttttctgtaaagtaattgtagtcggatggaaaaataacttttcggtaatcgatgatatacttgttataactcatgggaggcggaataatgaaacaattcaaaatttttatgtttgcactggcaatcgttttcggaattcagttagcagctcttccagccaaggcggatgccagcacttcaaccacgacccccaaagcattgcggggcacctggtacgaatatcgtggcagcggtaagtttaatgtcatcaagattaccacgcacagtttcaccaccaatggcaaatcttacaccccttcaaaaaaggatgaccgtaagcttcaggtcagcaaatgggggtcttggtacctcttcaataaatcaaagtcttcgaaaaaagacctgggtcagtacaagaccactaagaagttgattggcggatcctacaagaaagtcttaatcaaatatcatggcattggcacttatcatgtgtttccaaaccataaatatgaacacaaatattcatacactgttttagactgatgagacggtctcttcgaagcggtttgttagaatttcgttacctgatcatttataataaagacaggtattataacaaacgacttcgtcaggaggccagcgtatgaaaaaagcattcatcaccgggttgctgctattaattctgccgttgaaattgtttggctgttcgaatcagtcaaataattcgagcagtgaaagttccagcagcacgaagacagagcagtccagctcgacgacttcttcaactactaattcggcatcgacttcgacgacgattactcacgccaagcgggcagtcaaagttcgctatgaaaaggccaattttacaacctcccttgaccgggagtatcgtgaagaatatttgtatcagaatgtcccgggaaccgttgattcgaacaaagtttactcgtgggataacttaaacgtttcggaaaacaccaaggttcacgtcaatcaaaaggcgatcgcaaccttcaaagatgacgatgataacgagtacgatcatgaggatttctatcgaattacgttgggcaatcagtccggcaagcagtattgggtaggcgatgatgtcctgcagaacgatcatgaaaatgactatgatgactgacgattcaaacagcttgcattttattttgattggttgtattctattaccaatcaaaaaaggaggtgatgctttttgaatagtggaatatctcttaaggcatcagctgtggagaacgaattaaaatagttgatgcatttgagaagggaactcgcaaatagtgtgcgggttccttttttgtagtgtgcgacaagcaacgggtgatgcggtgtgtagaggggcggtgattgaaatcctgattttggattttaatcaccgcccctttacacgttagcatcagttgcgtcggagcatagctcaaaggccgaagggagcaggaaataatagaagaacctcaagctctataaaatcgatgcaaatgcaccaaacatcacgtacgaactttgttcatcgttggctgtctttttgtgtagcaggggtcaggggcgtcgccgagtaggctaggcagcctccaaatgcaaaccagaatattacaaccacattaaatccaacatcctcagaacttttccctggaaaacgctagataatttctaccaaaacctgtagtatgaaaaagttgtgcttttcagaaatcaataaaggggatgagaaatcaatgaaaacattcaagtttcaaagcttcgttttagttcttattgcatttgtattggggttcagtgaattcctaattgtcgggatcctggatgacttgagtcaccaattcaacgtgtcggttgcgactgttgggtatctggtcacggcatttgcgatcgtctatgccattagtacgccgttcattacaatcctgattggaagattcaatctattctgggatttgatggtcgcaatggctgtcttcacgtttggcaacattttaagctttttggcacccaacttcttaatgctgacggtgtcacgagtggtcactgccatggtggccggcgtgtcgatctcacttggcttgacctttgccggttatgtagcgccaatggctaaacgcggctggctgttatcttgggtattttccggtttctcaatcgcctcggttgtcggcgtgccacttggaacctggatttcaacccagtttggctggcggatctcgtttctaacggtcattgtgatctcagttttgacgatgggcctcatttttgtcagcctgcccaaggacttcaaacaaaagaagagtaccatttccgggcagctggcactgctgggcaatcaccggatccaaatcggtatgctgctgccaatgtttaacctggccgcaatctacgtcttctacacttaccttcggcccattattaccaatcaactgcatttttcagtctcaatgctgaccattttgctggccgtctttggaattgccaacattattggtaaccgtgccagtggccgcttaagtgaaggtcctgggatgaaagggatgccgtttgtctatattggccagttcattttaatgatgctgatgccatttgtcttcaacttcagttggccgggagcactgcttttgacgctggtcatcttcaccatgccgctgattaattcaccgatccagttgttcttcttgcaaattgctgaaaaggattatccacagtcaattgtgttggcttcgtctctgaattccattttttccaacttcgggattgccctgggatcagcgactggtggggtgattgtcagtaacctcagccttgacgcggttggcccgggtggcgcggtctacgccgttgtcgctcttggactggtgttgtggttgaaccacttgacctcgaaagggctttcatctcgctccactaacctgtaaaatgtgattgaatacaaaaattttggtgggtgagaatatgaatggatttatcggtgagctatttggaacgtacgtgttgattgtgctggggactggcgcctgtgccggtgccaaccttaagcaaacttacgccaaaggctcaaactggacgtttatcagtgtggcttggggaatggcggtaacgatgggggtctatgtggcctcgtcactggggtcactgggccatttgaatccggcagtcacgattccttatgctatttttgggctctttccctggaatcaggtggtgccgtatttattgggccaatttcttggcgcatttcttggggctgcgacgatcatgatgatcttttatccacatttcagaacgacaacggttgataatggcaacacggttggcatatttgcgacccgaccagccatctattcgccggtttccaattatctatccgaagttgtcgcaacctttgtgtttgtctttgcgctgctaaacctgggagattttacccaggggctgaaaccgttagttgtcggcctattgatcatggtggttggtcttggcgttgggacgaccaccgggtttgcgctgaaccctgcccgtgattggggcccgcgatttgcctattccgttattccggttcccaatcgtggcagcggtgaatggtattattcctgggtaccgatgtttggtccattaaccggtggtatcattgcggcaggcctccaagttatggttaaatagacagtatcaattattttggaggtacttatggatcgtgttggaatgaaattagaagccaagcgtataattggcagtcattttccgttttttatcttattgttcctgccggcagtgattattcagctgggatactcagtggcttattcgaccaatcccctgcacgaggttgataccaaccaggcctttaatcaaattattcagggaactgcccactttggcagtaatgaactgttgaatttgtggctgatttcgactttgatctcaatcgtttccggccttctcttgtctggaatgatgtttgtctgtattgacctaattcgcaacaaagtaccgtttgaccaaccagtgaccaggtcgtttactatcttgaatcatggccaatacttcatcggcgcgattatgattggcattatcacgactgtactgacactgttatggtccgtactgttgattgttcctggaattatcaagggctttgcctattcacaggccttaaacatttaccgggattcagtggatgccggcaagccgattgggtatctggaagcaattacccggagtcgaaaaatgatggtcggccacaagatggattactttgtcatggaattgagctttattggctggtacatcctcaactcgttcacctacggcattttgttgctgtggctgcagccatactaccagttatcgtttgccaatttttatgtaaaaatcgctcaaatgaaccaaactgaacaatgaaaaatactcatcattccaattgctggaagtggtgagtatttttattatggctcactaatattaattatcgaggtgccagactgtggcggatcagtccgaaacgcgacttaatcacccagggcttgggtcaaatcgttggccaaatcttttgggttctccaatcctgtcgacagtcgtaagagttcatcagtaatcccaagctttaggcgatcttctttggccatgtcgctgtgcgtttgaagagaagggatggtcagcagactttcgacaccacccaggctttcagcaaatgaaataattttgaggcgtttaaacagccggtcaacttggtccatgttttgtagataaaagctgatcatgccaccgacgccaggatacaggactttttggacttgaggcaatttcttcaaacacgctgcgacatatttagcgttgctggtgtggcgttccattcgcacggccaacgttttgaggcttcttaacagtagccaggaatcaaaggggtccaaagtgacgccggttgtattgaaattgaattccagttcactggcaatttcttctgacttggcaatcacacagccggccaacatgtcgttatgccctgaaaggtatttggtggcactgtggacgacaatgtctgccccctcacggagtggctgttgatacacaggcgttagaaaagtattgtcgacgcagaccaaggcgttctgattggccgcatgaatcagatcagccactttttgaatatcaattattttcatggtggggttggagggtgtctccagccaaactgccttggttttggcagtcaccaagtcacttaacttttcgtaatccttcccgttccatttactgaatttgacaccgtagtggtctgccaggtaatcaaagtaacgaaacgagccgccatacaaatcgtctgaggtgatgatttcatccccagacttgaataacgaaaagaccagttggatggccgccattccggaactgaccgcaaatgcattggcaccgccttccaggtcggcgagggtcttttgaaggacgcttctggtcggcgttgataagcgtgagtaggagtactgtttgtgcggatcaaaggtctccgcatcctccaagtcgcggtgacgaaagtttgacgtgagataaatcggggttgaaaccgagtggtactgatcgtggttatcccggtttccagcttgtgcaagtaatgtatcaatatcgattaatttgtcagacatatgctcattctcctttaaattttttcaccaaaaaagccttcatcctaaacgatgcgtgttaacgctgttcagggtgaaggctatttcactttaccacctggcttcactgagatttcacaacctcagcctcattaagtacgccatcttgatggatgggatactcggcaaagtaacgcttgctgacgtcgaattagccaaaccaaaataacttggtgaccgattcggagttcagagatcatcttcacatttttaaccagtcttctctcaccaatcgaagctctctttatcagtttaaaaatgctactcttctcatcaacacttaagtaaattaaaatttacataattgtagaatatatttcgttaaaggtcaacggcctatcgaaaatttgtggttcgttatttcacaatatggacagttttacgctgtctgttcatttaaacgatcgcgacaacaaaaatgaagtcctgaaataaagcctttatttacaaaggattgtgggttaatttaggccttaaaaaaggtcgaacttttttgttgagcctatttacatatttttcacaaggtgttaggatgaaagcggtttaagaatatgaataatcattggaggaagaactcatgaaagaaaattttgattttttaatgcctagtgtgaacttttttgggaaaggtgttattaaaaagattggtgatcgtgcgaagatgttgaacatgaagaaaccgttaatcgtcactgacaagtttcttcggggaatggacaacggtccggttgctcagacactggattcattggatgctgccggcgtttcatacgtgatctttgatggtgttgaaccaaatcctaagattcgcaatattcaagctgccaagcaagtatatttggacaatgattgtgacagtattatcacggttggtggtggttcttcacacgattgtggtaaaggaaccggaattattttgaccaacggcgatgatattaccaaattggccggaattgaaaccttggagaatccattgccaccactgatggctgtcaacacaactgccggaactgcttctgaattaacccgccactgtgtgatcaccaacgaaaagaccaaattgaagttcgttgttgtttcatggcgtaacattccgctggtttccttcaacgatccgatgcttgaattggatgtgccagccgcaatgactgctgcaactggaatggatactttcgtccagtcgattgagccatatgtgtcaaccaaccgcaacgaaattaccgatggtcagtgtattgaagcaatcaaattatgtgaggaaagtttgcgcgaagctgttgccaacggtcacaaccttgaagcccgaaccaagatggtcgaagctgaaatgttaggcggcatggcctttaacaatgccgaccttggctatgtccatgcaatggcccatcaactaggcggccagtacgatgcgcctcatggtgtctgctgtgcaatgctgctgccaattgttgaagagtataacttggtggcatgcccagaaagatttgctgaattggcaaaagcgatgggcgaaaataccgacggcctgtcaacacgtgatgccgcagaacttgcgatcaaggcaatgcgtcaaatggccgatgatgtccatattccacgcagtatcaaggcaattggtgccaaaccagaagactttgaactgatggctgagaatgccttgaaggacggtaacgctttctccaacccacgaaagggtactaaagaagaaattgtccagttgttccagaaagcttatgacatgaagtagagcgccgagacccgggtgacccctgagcataagcgaagaatcccaatgatgaacggttcttgttcatcgttgggatttttcgtttatgcggctggggtcagggtcgtcggagcgtgttttcaaggccgaagggattacaaaatggcataacaaacgcgccagagcgcgacgagacccaagtgctcccaccaagtaggctagaccatttccgcccgtcaaagtatatttcgaggattcaaaagttgtcttccggatccacaaacccaaaaaccttccaacaatcttcacactttcttcacaacttggcgagaatattaagataaaattatggtgtagataagatattacccaaaagaatcagaatcaattttcaatattggagggcgtttattatgaaaaagtttgatctggccgatgcagcactgctacttattccattgacgatgatcggcttctccgctagtattcatacccgtgatcacgatatttctaccaccaaggccgcccaggtgaataagatcggtgaaaatatcgatacagaatattcgggtgattccgacttaaacaagggcaacatcagaccgctgtattttcagccgtcgcgggtttttagcgtgaagtaccggacggttagctttaaaacggttttggacgaagactaccgggaagaaaaattatatcgttatgttccgggggctaagaaaaacaatcgcacttatcgttggtcaaccattaaggcccacaccggcaaacgggtttacgttgataaaaaggctaaagcctactatcgggacgatgatggcgaacgcgaaagcgaagatttctaccggatccgcgtttctacaaacaagcatgcgacgcgttactgggtcaatgaagatgcgattgatgactgatttttaatatatttgattggattggggtgagtaatccctgccaatctggcaatcaaaaaatgaccaattatttcattttgaaatggttggtcattttatgtgaatgatgaatcattttgcggctgattatgataaattagatgtataaattcgcttaactggaggtgcaatttgaagatactagtaactggtggtgccgggtttattggatcaaatttcatccattatcttctcgaaaatcatccgactgatcaggtgaccaactttgatgccctgacttatgcgggtaatttggcaagtttggcggatgttcaaaatgatccccgataccattttgttcagggaaacatttccgatcggcaggcggtcgaacaagttatttcaacctatcagattgattcagtcgtcaattttgcggccgaatcccacgttgaccgctccatcttacatcccgatgcctttgtccgcagcaactttgtcggcgtcagcacattactggatgtggtgaagcaacagcacgttaacaagtttgttcaaatttccaccgatgaggtttatggcagctcacgggggcatgagcagttcaatgaggcggcacacctcaatccaagttcgccgtattcggcgactaaggccggtgccgacctgctggccctttcgtactacaagacgtacggcatcaatgtgtcaattacgcgatccgccaacaattacggcccgtttcaattcccggaaaaattgattcctttgatggtcaccaatggtcttcggggaaaatcactgccggtttacggtaacggcaaaaacgtccgcgactggctgcacgtgtttgataattgtcgcgcgattgatgccgtcttgcgtcatggccgcccaggcgggacttataacattgccgctcacaattacgcagaaaacattcaaattgttgaaaaaattgttaagcagttggaattgcctcagtccatgattgactacgtttccgaccgaccggccaatgatcagcgttactcaatcgatgatgcactcattcgcaatgaattaggttggcagccgaccattgattttgatcagggcatttcccaaactgttgattggtatgtgacacatgaaaagtggtggcgaccgctgttaggcgccgtccacaacagataatggggtgaaatcatgaaaatcggttttattggtactggtgtgatgggcactgggatgattaaaaatttactcaaggcgggctacgacgtcacggtgtataaccgcaccaaggaacacgccgaggatgcgcttgatgcgggggccacttggctgggtacgccagcggaagtgaccaagaacagtgaggtggtcattaccattgttggttttccaaaggatgttgaacaagtctattttggtgacgacgggattttaggcgttgcccacgctggtcaaacgttgatcgacatgacgaccagctcacccagtcttgccaagaagattgccaaagctggggaagccagggacattggggttcttgatgcccccgtttccggtggggatgttggcgctgccaacggaaccttgacgattatggtgggtggctctgaaagcacatttgagaaatcaaaaccggtgttatcggcaatgggcagtacgattacccggtttggcggggctggtcaaggtcaaaatgccaaaatggccaaccaaatcatggttgccgggacaatgaccggaatgatcgagtcacttgaatatgccaaacatgccggcatcgacctgtcccagatgattcgaacaattaatggcggggcagcagcaaactggagcatgactaattatggcccccggattcttcagggggacttccagcctggatttgcggccaaacattttttaaaggacttgcggattgcgttggatacagctgatgaaatgaacattaatttgccggcgactaaagtggctcgggacctctacgagaagatgaccgacgagttgcatttaggtaatcttggtactcaagggttgcttaaggtttatgaaccagataacatttaggcgcaaaacggggctggaacaaaatttttagttttgtcccagcccctgtctatccgttcgattatttttgctgatttttgcgttcttttctgctttggttggcagaaaccaggttgatgataactgaaaccaacaaacaaattcctgctaaaataaccaatccgattttgacatcgtctggaaatgatgacttttgaatgaagaaggccaatgcaattgaaatcacaagggcagcatctgccacgatcagtttcggcgaaaatcccattgtactcacacctttcaaaaagcattataacaaatcggctgtccttgtcacggttatttgaaaattttgtctggcaggccaaagttgatataataagattataaatgaaggttaggtgaagatcatggcagaattggacagtaacgacgcattcattgatacgaacaagttaatatttggcattggccaggtgcaacagatcactggggtttcaggaagacaattgcgttactgggaagaacagggctacattcaatccatcagccaaaaaaagggtgcagcacgagaatattcgctgcacactttattctttatctttcacgttactcgatttctgaataacggctttactcttcaggcagccgttgacagagctaaaaaatttgatcgccaattgccggtccttcgacaattcttgcgcgcccaactgcaaggcgtcaacattgatgatgaccaaagtgttctggatttcggctatgttgattcctcacacacacaacgaatctatggggttgttaaagatggtgagacgttctttcaaattgaaaatgttgattaagcatcacatcacttatcgaagcgctggctgtggccagggctttttattgtgcgctcaatcaatcgtcttcgttatcgaatttcttatataagccaatgattgtcttatcttttaattcgactggcttaccatccaacgtgacgtcgacaattttgtaatagtcttccaggtcagggacctccaaacgctgattggccagaaagtcggctgcagacttgtattcaatggactcggtgccgccgccattttcgtatttgatttttaacatgatgccactttctttctatatagtttaactaacattgacaacttaattttagattgaacatttttgaaatacaactaactgcctttatgaaatttctgtgaagaatgtttgtcttttttgagactttaaattcgactgaaaaattgggccatgatatattattgatgaggggatggctgtcgtaacatcctaaaatttaatattgtaatgacgacgtttaattagggggaattgaatgttgaagtttaagcatatttttgttcttgtgttaaccacgttgattttagtgattggcttttcggcatttggcggtcaatccgcttcagcgcaaacaatcaagtttaccagcgcgatgcacaccagcaagaatttgacttacaacggcacaatcaagtactacgttaaagcggacgcaaaaaaatattcacctgaaatcacctatgcaacccaaaaatggaataaagcccttggcaaaaaggttttccaacgaaccacttcaatcagccgttcccgattggtcttcaccggaactaataagcttaaccggaattacgcgggggtcgcagaaattaatagtggcgtgattgcattgaacacctcatggatgaatcgatacaatcagcagaagcgccgggcagtgatcattcatgagcttggccacacgtttggcaccaaggatttgtacaattatccaaatggggcactgcgaagtttgttcaagcagcagacgatcatgggcggcaactatgccaccagcattaaatcgtttgatgccaaattagccaaatggactttgcgaaaaaccagaagcatgtctcaaaccgagtttcgccactatcgttccaatgcgggactctactaccaacagatgcttaacggacagctttaatttctgctgagagaccattgacaagcgattgtccaaacactatgattaacttattgttttatagacgttgacgcagtccggtagtcgattaacttgagaagtcagaaactcagcggtagatgtgagctgagcggttaatcgacgaacatacagctgctgagtcttcaactatgtgagacggatcatctcgttaccgatgaattgagtggttggcgatttttcgccagtaacttgggtggtaacgcggaaaacttttcgtccctgacaattaattttgtcagggacttttttatttaggaggaattatggaatgaacattttggaagatttgaaatggcgtggcgccatcaatcaagaaactgatcatgaaggcttaaatgaattggttaatcaaaagtctgtcgggatttacgtgggaattgacccaaccggcgacagtatgcatattggccatttgatcccgttcatgattttgaagagattccagctggccggtcatcatccagtcattttgatcggaagtgggacgggctcaattggtgacccaagtggtaagaaatctgagcgggtccttcagtcgatggataaaatcaagcgtaatgaaattgcgctgactgctcagatggaaaaattgtttggagaagacggtaagtttgagattgttaacaactacagttggctgtccaaattgtcactgcttgattttctccgcgattacggtaagttgttcaacgtcaacactatgctgaataaggaaattgttgctagtcgtttggaagtgggaatttcattcactgaatttacctaccagattctccaggccattgattttcttcacctttaccgacacaatgatgttcagcttcagttgggcggggctgaccagtgggggaatattacctccggaattgatctgattcataagatagaaggacccgatgccaaagcctttgggttaaccattccactattattgaagtccgatggtaccaagttcggtaaatcagagggtggtaatgtctggcttgatcccaaaaagaccagtccatacgaattctatcaattttggattaaccaagatgataatgatgttatcaaataccttaaatattttactttcttgtcacaagatgaaattgccgacttggaaaagaaagttcaaactcaacctgaaaagcgtgaagctcagcgtaaattagccgaagaagtgacggagtttgttcatggcaaagaagccgttaagcaggctgaacatatcactgcagcattattctcaggaaatgtggctgatttgacgacaaccgaaattgaacaaggcttcaagaacatgccatcagttgaggtttcatcagaaccgttgaacattgttcagtggctggtggatgcgactaagattgaaaagtcacgccgtcaggccagagaagacattaccaacggtgccatcagaattaacggtgaacgcattgaagatgtgaattacgaaattaatccggcgaagaagtttgatggcaaatttgtcattgtccgtcgtggtaaaaagaagtactttttagcgagagttaaatagaagcaaagacagatcgaacgctgatctgtctttttttagttgacaatgttcatcaaagtcggtatattatttagtgcggcttttgcgagaatgacttcttcgcagagttacaaattttaaaaagtcattgacacacattgcgcgtcatgataatattaaatagttgtcaaaagcgagaaacaagcgcttccgacaaccaagtagacctttgaaaactgaacaaaattttcgacaaacaaatgtgcagggcgtttcaattcttcggaattgaaaccaaacatttgcgaagtcaattcgtaaaaacaaataataaatttaaatcatgagctatcacaggcttatcattttaaacaatttaagatgagagtttgatcctggctcaggacgaacgctggcggcgtgcctaatacatgcaagtcgaacgcgtctccattaatgattttaggtgcttgcatttgaaagatttaacattgagacgagtggcgaactggtgagtaacacgtgggtaacctgcccttgaagtaggggataacacttggaaacaggtgctaataccgtataacaaccaaaaccacctggttttggtttaaaagacggcttcggctgtcactttaggatggacccgcggcgtattagcttgttggtaaggtaacggcctaccaaggcgatgatacgtagccgacctgagagggtaatcggccacattgggactgagacacggcccaaactcctacgggaggcagcagtagggaatcttccacaatggacgaaagtctgatggagcaacgccgcgtgagtgatgaagggtttcggctcgtaaaactctgttgttggagaagaacaggtgtcggagtaactgttgacatcttgacggtatccaaccagaaagccacggctaactacgtgccagcagccgcggtaatacgtaggtggcaagcgttgtccggatttattgggcgtaaagcgagcgcaggcggttttttaggtctgatgtgaaagccttcggcttaaccggagaagtgcatcggaaaccgggagacttgagtgcagaagaggacagtggaactccatgtgtagcggtgaaatgcgtagatatatggaagaacaccagtggcgaaggcggctgtctggtctgtaactgacgctgaggctcgaaagcatgggtagcgaacaggattagataccctggtagtccatgccgtaaacgatgagtgctaagtgttggagggtttccgcccttcagtgctgcagctaacgcattaagcactccgcctggggagtacgaccgcaaggttgaaactcaaaggaattgacgggggcccgcacaagcggtggagcatgtggtttaattcgatgctacgcgaagaaccttaccaggtcttgacatcttctgccaacctaagagattaggcgttcccttcggggacagaatgacaggtggtgcatggttgtcgtcagctcgtgtcgtgagatgttgggttaagtcccgcaacgagcgcaacccttattgttagttgccagcattcagttgggcactctagcaagactgccggtgacaaaccggaggaaggtggggatgacgtcaaatcatcatgccccttatgacctgggctacacacgtgctacaatggacggtacaacgagtcgcgaaaccgcgaggtcaagctaatctcttaaagccgttctcagttcggattgtaggctgcaactcgcctacatgaagttggaatcgctagtaatcgtggatcagcatgccatggtgaatacgttcccgggccttgtacacaccgcccgtcacaccatgagagtttgtaacacccaaagccggtgaggtaaccttcggggaccagccgtctaaggtgggacagatgattagggtgaagtcgtaacaaggtagccgtaggagaacctgcggctggatcacctcctttctaaggaaaaacggaatcctgcacattgtcgaaagttttgtttagttttgagaggtctactcccaaaagtggttacgctttttgggcctatagctcagctggttagagcgcacgcctgataagcgtgaggtcgatggttcgagtccatttaggcccatccacggcctgatagttagctatcaccggagtaacatggggaattagctcagatgggagagcacctgctttgcaagcagggggtcagcggttcgatcccgctattctccattgacacgagagtgtcagacttggttctttgaaaactagataatattaattttctgtaataattttttgaaattgtatttatataatttcaaccgagaacaccgcgttattttgagtttgttaactagaaaaaaatcgcaaatactcaattaactttacatcacgtagtgatgtacaggttaagttaaaaagggcgcatggtggatgccttggcactagaagccgatgaaggacgggactaacaccgatatgcttcggggagctgtacgtaagctttgatccggagatttccgaatggggaaacccagcagttttaatcgactgttactatatagtgaattcatagctgtatagaggtagacgtggggaactgaaacatctcagtacccacaggagcagaaagaaattttcgattccctcagtagcggcgagcgaacggggaacagcccaaaccaatgagcttgctcattggggttgtaggactgaacatttgagttaccaaagttgttgataatcgaacaatctgggaaggttggcgaaacagggtgatagccccgtaggtgaaatcaatgaccctcagttcaggatcctgagtacggcgacacacgtgaaacgtcgtcggaatccgggaggaccatctcccaaggctaaatactctctagtgaccgatagtgaaccagtaccgtgagggaaaggtgaaaagcaccccggaaggggagtgaaatagttcctgaaactatgtgcctacaagcagttagagcccgttaatgggtgatagcgtgcctcttgtagaatgaaccggcgagttacggtaacatgccaggttaaggtttaaaagccggagccgcagcgaaagcgagtctgaaatgggcgttttagtatgttgctgtagacccgaaaccaggtgatctacccatgtccagggtgaaggtgcggtaaaacgcactggaggcccgaacccgtgtacgttgaaaagtgctgggatgaggtgtgggtagcggtgaaattccaaacgaacttggagatagctggttctctccgaaatagctttagggctagcctcggacgtagaatcatggaggtagagccactgtttggatgaggggcccgtcatgggttactaagttcagataaactccgaataccattgatttttatccgggagtcagacggtgagtgataagatccatcgtcaaaaggggaacagcccagaccaccagttaaggtccctaaatatatgctaagtggaaaaggatgtggagttgcatagacaactaggatgttggctcagaagcagccaccatttaaagagtgcgtaatagctcactagtcgagtgattccgcgccgaaaatttaccggggctaagcatattaccgagactgtggacttgaccttcggtcaagtgataggagagcgttctaagggcaatgaagccagaccgtaaggactggtggagcgcttagaagtgagaatgccggtatgagtagcgaaagatcagtgagaatctgatccaccgaatgactaaggtttcctggggaaggctcgtcctcccagggttagtcgggacctaagccgaggccgcaaggcgtaggcgatggataacaggttgagattcctgtactagttgatgatgtttgagcgatggagggacgcaggaggctaagttgtgcatccagttggaaagggatgttcaagccacgagtcagtcaaagagtcaaatgctttttggcgggttgacaagtggtgatgaggaccgaaatttaagtagggaagcaaccgacgtcacactgccgagaaaagcttctagtgagtcatcaactacccgtaccgcaaaccgacacaggtagtcgaggagagaatcctcaggtgagcgagtgaactctcgttaaggaactcggcaaaatgaccccgtaacttcgggagaaggggtgctgtgcgcaagcacagccgcagtgaaaaggcccaggcgactgtttatcaaaaacacaggtttctgcaaaatcgtaagatgacgtataggggctgacgcctgcccggtgctggaaggttaagtggatgagttagcttcggcgaagcccagaaatgaagccccagtaaacggcggccgtaactataacggtcctaaggtagcgaaattccttgtcgggtaagttccgacccgcacgaaaggcgtaacgatctgggcactgtctcaacgagagactcggtgaaattaagatacctgtgaagaagcaggttacccgcgacaggacggaaagaccccatggagctttactgtagcttgatattgggtgttgacacagcttgtacaggataggtaggagccattgaagccggaacgctagtttcggcagaggcgttggtgggatactaccctcgctgtgtgaacactctaacccgcgccactcagcgtggcgggagacagtgtcaggtaggcagtttgactggggcggtcgcctcccaaacagtaacggaggcgcccaaaggttccctcagaatggttggaaatcattcaacgagtgtaaaggcagaagggagcttgactgcgagacagacaggtcgagcagggacgaaagtcgggcttagtgatccggtggtaccgtatggaagggccatcgctcaacggataaaagctaccctggggataacaggcttatctcccccaagagtccacatcgacggggaggtttggcacctcgatgtcggctcatcgcatcctggggctgtagtcggtcccaagggttgggctgttcgcccattaaagcggtacgcgagctgggttcagaacgtcgtgagacagttcggtccctatccgtcgcgggcgtaggaaatttgagaggagctgtccttagtacgagaggaccgggatggacataccgctggtgtaccagttgcgccgccaggcgcaccgctgggtagctacgtatggatgagataaacgctgaaagcatctaagtgtgaaactcacctcaagatgagatttcccattcctatatggaagtaagacccctgagagatgatcaggtagataggttggaagtggaagtgcagtgatgtacggagcggaccaatactaatcggtcgaggacttaaccaagtagaaatggtgttcaagggcagaaaattaatattagctagttttgagagaacgaagttctttcaaggaaaatagtgtggtggcgatagccagaaggatacacctgttcccatgccgaacacagaagttaagcttctgcacgccaagagtagttgggggatcgccccctgcgagggtaggacgttgccacgcgattttatggaggattagctcagctgggagagcatctgccttacaagcaggaggtcacaggttcgatccctgtatcctccattccttgagccgttagctcagttggtagagcatctgacttttaatcagagggtcggcagttcgagactgccacggctcattacaattgaatattattaagcgcataatatttgtatgccgacttagctcagctggcagagcacctgtcttgtaaacagggggtcggaagttcgaatcttctagtcggcattttgcggaagtagttcagtggtagaacatcaccttgccatggtgggggtcgcgggttcgaatcccgtcttccgcttgttatgccggggtggcggaattggcagacgcacaggacttaaaatcctgcggtcagtgatgaccgtaccggttcgatcccggtcctcggcatattatgcacccatagcgcaattggatagagtgtctgactacgaatcagaaggttgtaggttcgactcctactgggtgcattgttttaacgggaagtagctcagcttggtagagcacctggtttgggaccagggggtcgcaggttcgaatcctgtcttcccgattgatagcataactatcatttttcatcgcggtgtagctcagctggctagagcgtccggttcatacccgggaggtcgagggttcgatcccccctgccgcgatataggtcttggacctttagctcagttggttagagcaaacggctcataaccgttcggtcgtaggttcgagtcctacaaggtccatcgactcaattatatactggagtttttatacagcttttatggaggattacccaagtggctgaagggggcggtcttgaaaaccgctaggtgggtcaaaccacgcgagagttcgaatctctcatcctccttattatcgcgggatggagcagtctggtagctcgtcgggctcataacccgaaggtcgttggttcaaacccagctcccgcaattttggttcgttggtctagttggttaggacgcctgcctgtcacgcaggagatcacgagttcgagtctcgtacgaaccggttttggctcggtagctcagtcggtagagcaatgcattgaagctgcatgtgtcggcagttcgattctgtcccgcgccacttgtttttaatattgtttttgcgggtgtagtttagtggtaaaaccacagccttccaagctgttgtcgcgagtccgattctcgtcacccgctttttcatataatgggcctatagctcagctggttagagcgcacgcctgataagcgtgaggtcgatggttcgagtccatttaggcccatattttggagaagtactcaagtggctgaagaggcgcccctgctaagggtgtaggtcgcgtaagcggcgcgagagttcgaatctctccttctccgttttaaatgacccgttggtcaagtggttaagacaccgccctttcacggcggtaacatgggttcaaatcccgtacgggtcattcaagagaatcttattatattatcgcgggatggagcagtctggtagctcgtcgggctcataacccgaaggtcgttggttcaaacccagctcccgcaattttggttcgttggtctagttggttaggacgcctgcctgtcacgcaggagatcacgagttcgagtctcgtaagaaccggtggaacatcgaaagttttcaagttacttaggtagcttgttttttttacataaaattctgatccaacacaaaaaccgttaatcagtgaagtcatttgcacttcatcaattaacggttttatttgaatgaaccttttattgcgtctttttggtcttagctggtgtgtaataagcttcatgtgagtagaagtttggtgaatcacggtactcttttggaatgaattcatcagaactgttcttccaaagttcgaagtcggcgtaatcatcccaagttcccaaaatgattcgttggctgatgtccttgtgataattaagggaataaattgaatgcatgccatcgggaaggccatttgttcgcagcttgttgatgcgcgcatcaaaaaccttctgttgatcaaaatttaaatctaatgtggagaagctaatgaagccgtcccacttatcttcaccactgtgacttaaaatatcatagaaaaccggtgccttgaagactgaatctttacctgaatggtccagcagcataaattcacctggttggctgagagcttggtacatcatcaaatcccgatcaggatgcgctgccttgagttctgttaaaattttttcatttccaaatgtaatgacgatctgttcgttcatttgacccacctcctatatacaattttattatactttctttcaatattggaaccaaacatttaccccaaattagcgtaaaatataaattggataaagatgaaagaggaggaattcttttgaaactaacagtgattggttttcttggcggctatccggatcatggtgatgccaccagcagttatcttttggaatcgggtgattttaaattactgattgattgtgggagcggcgcactgttgagcttggaacaggttgtcgaccctctgaaactgaatgccgtcattttgagccattaccatcacgaccacacagctgacgtgggcgtcttgcaatattattggcaattgcatgaaaaaaggtacagcgagcccgtattgccgatttacgggcacaccctcgatgagatcaacttcaagggacttagctggcccaaatctactaaagggatcgcctatgatccaagtcaaacactgactgttggcccgttcacgattacatttttcaaaacccatcatcctgttccggcatttgcaatgcgtattcaagaatcatcaaccggtaaggtactggtgttcactgccgatacagcttatttccctgaattgacccaattcgttcacgatgccgatcttttgatgactgatacgaacttctttgcgacaaaaaccggccagaaatggcatatgacatcgactgagtccgggcaactcgctcatgacgggaatgttcaccgattgctgctgacccacttacctgcaaatggcgacatggagcaattaaagacggaggcgcaaacgacggcgggggagaccatgccaattttggttgccaaaactcatctttctgtggatatctaagccaaatttgcccaaaataaggtctttgtttgtctattctgtgaatcttatgatttatataacattttccgatataatcaaagcatcaaatgattactaggaggattcacattatgacagtcaatttattaacaacccccagctgcacttcctgcagaaaagcaaaacaatggctcatcgatcacgaggttgattttgtggaacgaaatatttttgccaagccactttctgaagttgaactcaaacaaatcttgatgctgtctgaaggcggcaccgatgatgtgatttcgacccggtcttttttgtacgaccaatacaaatcaaagatgtcttcaatgaccatcagccaggtgatttccttgctggcaacccatccagaactgattcgccgaccaattttagtggatgccaaacggattgagtttgggttcaatgaagatgaaattcgttgcttcatgccacggagcactcgaaaatgcgaattggaaaagatggtcaaaaaagccttatagtcttggaatcttaattgcttgttaatattcatgtttagccgtattatttacttagacaataatatgatacaatgttattattaattaccctcagatattgaaaggggtggctaaatatggaaatggaacggattaatgagaatacgattcgtgtgttgattggtaatgatgatctcgacaagcgcggcattaccgtgcttgacttgctgggcaaccacaagcagatcgaaagcttcttctacagtattctcgaagaagttgataaagaccatcaatttcaaaataacgatgccgtcactttccaagttcttccaaaccaaaatggcttggaattgtttatcagtaaggatgtagatatgtctgataacgacatgttcgatgcaggtgactctgattcagatcaccctgaaaaacgtgatcgggtttccaaatatatcgcagaacatgccgataataacaaaccgcaacctgtaagtgataaaaagactaacgatgaatttggtcatcaaaagcggactgtaattcttgagttcgaccaattagatgattttgtgtcgctcgccaaggcattgcgacttgaaaatggcacatcggatttgtacttgtatgaaggaaaatactacttgaagcttgaactattcagcaatgaccccgttgacatggtcgtcagtgatgaagttgcaattgccaatgaatatggcaagaagaccgctgttactgaagaggttctcaacgaatacggtcagcagttgatggaaaacagcgcattggagttaagcaggtactatttcaaataaagttcaaccaactaaaaacgacagccgttaatggctgtcgtttttagtgtgcagattattgttggtacgcacgtcctttgatcgttgttcgatagtacgtttggcgactgttttgactttgtggggtgcgaaaccccaccgttttggaaacgatatacagtggccgtttacgtgatgcctcaaagactcgataaaggtaagcgcccaacatcccaatggtcaatagagtgatgccgaccattaagaatagcgcaaagaccgcaaagtgaatggtatccatcgtggtaaacagcgaggtaaccaagtagccaacactaaatacgattgacaaggttcccagccagttggccaactggaggggaaatgatgaaaacgaggtcacgccatccattgccaaacgaatcattttgcgcaacgggtatttagaagtcccggcaattcgctcttgacgctcgtaagtgacgtcggtctgcttgaaaccgacccagctgaccatgccgcggacaaagggatcggcctcgttcatttgtcgcaattggtagaccacttgcttgtccattaaccgaaagtcaccggtatccagcggaatattgacgttggtgattcgttttaaacctctgtaaaagagggccgccgttgcctttttgaaaatactttcgccatctcttgaaagccgcttgccatataccacatcgtagccttcatgccatttatcgatcatatccacaatgacggcgggtggatcctggagatccgcatccattaccacgacggcctcgccttgggtataacgaatgccggcagtaatcgcgagttggtggccaaagtttcgtgaaaattcaaccaaccgaatattgttgtgcttggcttgctgattggaaatcagttcgacacttctatcggtggagccatcatcaacgaaaatgaattcaaaggtctgcggttgattggcagcaaagttttccaaggtgttgatggtggtttcaatgccttgctcttcattgtaaaccggtaggacgattgaaattaattcctgttttttgtccattaaatgacctcctatttataaattgacgacaagtcatacagcacgccggatgaacccattccgccaggaccttgcatggttgtctgtttctgggtagacttactgttcgattgaccagctttttgagtggattttagtttgggattgctcttcgttgaaggcttggctcccggcttaccagttggctttttcttgcctgacggagctcctgctggtgcctgtttgctgttaggtgctttagcttgtttggtggacttggtggtcgtcgtagctcctgggccacccatgccggcttgagaaccgttgctgcttgaagattgatacaagctggttttgactttggtagcgtgtttcttaatccaattgataatcttggtattccccgatctgccggagtaatagaagtacttcaagtcaccgtttttgacgagtttcttgaattgagacaaggtaattgccggatcagttccgttaaagccacccatcgccatgaccgccttcccggttttgatgatgtaaggcgctgcggttgtcgaatcactggtggcaaacagatatttggcgtttccttgatgcttttcaacataattgagcagtttggtgttgactgagctgttgcccatgccgccaccgccgcccggcatgccgttgctgctggatgtgagcagcgatggtccggcggttggaatcatggctgattcagcggcaatcgtgggcgttaacgaccaccaggttggagctgccatgatggaaatgagaccgccaaccaacagcgcttggaatgcgcgaccccgtggtaaaacagccatcccaactgaaaagccgattgcggcaattagaatcacccaggtgagccatggatagtaactgtaaacgtaccaggattgaagcgccgcagttgccacgattgcaatcgggagcagatagaatttccagctggttcgtaaactgtttttaaacaggccgaccagcgcagtgacgccagttccaaatagtgctgcgattggtggggccaacatgatcatgtagtagggatgaaagaaactggcaacgctgaagaaaccgtagaccggaatcagccagctggtccacaggatcaactgtttttgttgcttggacaggctaaaccaacgtttgcgacggtctctaaagaagactaagccgccaattaagccaaagagggcaaatggtaataaccaactgacttcaggcccgagggctgattggaagagtctaaacggtccggcagtgccaatgttgaaggcgccaccgccaccaccgccgttacccatcttgccggggccacctttgccgccgtttggctggcccttcatttgcttaccgccgggtggggtttggtgtttgccggtttgcttcatgccggtaggggcttgaccacccggcattccaccaccttttttgttggtcgttttgctgttcattccggcaccaaatgtcccgccggttccagtggtttgaccaagcagtcgttcacttccgttataaccaaaggccagttccaacaaggagttggtttctgaaccaccgacgtaaggtcggctgctggcaggggtcatgtcgacagaaattgggtaggccagggtgaagactaagagcgacacggtggccaacgttaatttggtgattttctttttccaggtttcgttggctgccaaccagtaaaataaatacatggctggcaggatcatgaacgcttggagcattttgacgttaaaagcaattccaattaacgcaaagctgatcaacagtgaccaaattttgcggctgccaatggccttttcaagaaagtaaagggccaacattaagaagaaaactaacgtggcatccatgttattggttcgagaatcagccacgacgatcggtgtcagggttaatgccaaggcgctcagacgagctgcgttttgaccaaagtacggctggatcaatcggtacattagatagaccgatctgactccgaaaagaaccgatggtaagacgatgctccagccgtgcagaccaaagattttggcactgattgccatgaaccaaagtgcgactggcggtttatcaaccgtgatgtaaccggccggatcaaaactgccgtaccaaaagttgtggaaactttcggtcatacttttaatggccgcggtgtaaaaggcgtttgcagaacccgccttccagatttgccagccgtagaggaataacgcaaggacgaggattacgcctaaaatccagtcaaacctgaatttgcgttgataacgattttgggtattttcaatagatagattattggttgccatagtggcggacctcctttaagtgatgttggttgaatacccaaaactttgaaagcaaaaaattggtgggtacggtgatcatcaaactgacgataggaattagtcggctgtcaagaatcggccaaccgctggcaaaatgagcgaacaaaacactgatcagccaggtgaaaatgtaagtggcgtagtatttccatgcaaccgttttaactgaagcacctgtctgaaacacccagcggttatttaacgctaaccccagcagagaggtaatgccgtaaccgattgccatggcaatggttgcgttggttggatgaagtaataacagatagatgacataggtcagcacggtattaatgaatccggtaatcccaaattttaataattgctttgtactagtaatggatgactcactcctttctgaattgatgaaatgagtttatatgtttaaccataaaacaagcttaaaacatttgatttatgataaattgtgaataaccgagttgacggaatgcgtaaaaacctttaatttagtgtcaacgacaaaaggagaacattcaaatgaaagacttacacatattaataattgaagatgatgaggacctggcgaagagtctgcagctgtttttgggcgaaattgcgcaaacgaccgtctcccacgatggctttgaaggccagatgctggggcaggagggaatctacgatctggttgtattggatttgatgctccctcaagtcagcggctacgacattttgaaacactggcggaccgaggaccatttgagcatgccggtgctgatcttgaccgccaaagacaccctggacgacaaagtgcacgggtttgaactgggagccgatgattatttgaccaagccctttcaccgtgaggaattgctgatgcgggtgaaggcccttttgaagcgaagtggccaccttggtgacgacaataccctgtcagttgggccatttaaagtgaacttaagcaatcggattgtggaagttaacggcaaagagttggcactgaatggaaaagagtttgacctgctggtctacttcattcaaaatccggataccattattaccaaggaccagatttttgatcggctctgggggtttgagtctgaaaccgcgatttctgtcgttgaagtctatatgagtaatttgcgaaagaaaatcaagcagagctcatcgctccagccgatcaagaccttaagaaacgttggctatatgtttgaaacggaggaatcagattgaaaaaaggtgatccgcagcaaaaacaacagctgagccttttcctaaaggaattggtcgggttcgcactgttgtttgctgtacttggtttagttgttttcttcttatttcaccaatcgatttataaaaatatcgaccagggattggtcacgcaaaagcaaaacgtgttaagtaaccgcaaggcccctcaatttcggacgggcggcaatgcgcaaaatccagccccggccaagcccaataatggtgacacaccatttagaaccaacattttagtttttaacaaaaaagggcagattatcaatgctcaaatgctgggcaatcggatttacaatctatttatcaataccgaactggataagtcgcaagtcaacaaggtccgcgaagtaaccttaatgtcgaccgacaacaccttacattatttccgaaccctgttgattaaggtgcccaagtccaattccaatccaatttatgccggtaactatgttttgattttggaaaatattgataccgatttgatggcggttaacagttttaagcgctcactgctgacaacgctggtcttcttttggatcgtcgccattgcgattgcttatttcctatcccgatcgagtatgaaaccgatcctggacgcctggaaacgccaacggcaatttagtgctaacgccgcccatgagctgcggacgccgctgaccgtcatccaaaatcaaatggagtatatgttaaccaaacccaagaccaaggtcatcgaccaggtcgatccaatctcaacttctttggatgaggtcaggcacctgcaaacgttgaccaaccggctgttgatgttggcccgttcagattctgggacaattgaaatcaacaaacaggaagtggatttgaaaccttggttcagccaaattctcaaaccatacgacgatatcgccgccagccaacataaatcgatggtgacggtccttaaagccgatggtaagggacgcttggataaggatttgattcgccagctcttaatcattttgttggataacgcgatcaaatacacgcctgccggtgggacagtcactgtgatgacggcattgaaccgtgatcgattgacgattgaagtgcgcgataccggaaccggaattcccgatgctgacaagaaacgaatttttgaacgcttctatcgttccgacaaatcaagaaattccaagactggtggtaatggcttgggattggcgattgccaaatggattgttcaacagcactcggggaccatttctgttaaggacaattatccaaagggaaccgtgtttgatgttttgatcaagctgtaaaatgataaagtgattactgtgcacaaagaaagctcggagtaaaagtgatttgacttttacctcgagcttttttgtgattgggttccactagatcaatgattgatcctgcttatcggccttgttaattcctggaaataattcgtgcagatattcaagcggttcaactttaccgactttgtcagtgtatacaacttgagtcacgttgtcataggttaaggtgatcagtgactcaccgtcttcatctttgaccacataataacgaataccgagttggatggcgtaaaagatcaaccgttgggcatcaaatgagattttcccaattgatggcagaagggtcgttgcgcccaaacgttgggcccgccagcgcttggcgaccgtggttccgaagtccatcaagctaccatttttgatgtgttttaacaacattgccgaagctgtcagttccgggtgggtaaccacttcactgaagtcgtccagtgcctggagctgttcggaatgggcatgaagtgacttggccatctcaatcaactgatcaaagatttggatgccttcagccattttgaaagtcggctggttggggttctccaacgccacctgattgttatcagtgaaagattgttttaaatcagcggcaatattttcatggtcaactggggtgactaagagatacattaagaagaattttaaaaagtacattgcgtgacgactgatgccattaggggtaaacggcgtgttatccagtactcggaattccagataagagatgcctttagtgcgataatctttaatgtcgtcttggccgcgaagtcggaccggtccataaaattcagctgtggaatatagataatggtcgtcgattgcatgattaatgccgtcaatgtaatgatccaagctggtataaatggtggcgtcaacctgatcttgtggttcgttgacatagccataaatgctgttgcggatacttctgaccggatgggtgagttgtttttgatcctcagcggataaaaagcctttctccgcaattgggctggcaccaaacaaataagtcagcagccaacggtgaaggacaaaattttgagctagctggaagtacaatgcatttttgaaggccaccaaggtactgaactggtcttggtagtggacatacagccgattgatgaccggttcggggatgctgaagttgacgtgaacgccagtaatgatttttctggcgaccccgtacttttcggttaagtaatcacgatatttggcgtaggcgggccgaccaaaatggcctttgataaagtcgacgtcgtcttcgtccattgctggcggcatactcagcggccaaaaggattctgatttatcaatcgaccgatataaaactgtctgcaaagtatccaattgatccaacacgccgccaatattggggttgggatcggtaataatttcgctcattgattcggaaaaatctgattgcaaatagggatgataacgtctggaaccgagattttgcggatatggcttgcggcttaatcggccgtggtcatcgattcggtgttcttcgatttcaatgccgattaggctatggtaaagctgttctgcaacgcgttcttcttgaatgtgttttaataaatttttcagcatagtagtcccccagccggatttagttatacataattataaacaaaaatcggcagaatggtagccatacggccgttctgatgaaaacgtaaggttatttttaacttcttgaaaatcattgccatcggtttcgtatttaacccatagaaggtgatgaaatgctgatagcgatgattaataatcaattagtgaatgcggctgaattcaagggccaaaagaatttagccaatcgactggtttgcccgggatgcaggcaaacagtgatattcaagcgcggcaagtaccgcattccccattttagccataaatctaatcggatttgcggtagtttcagtgagaatgaaagtcaggcccacctccaaggtaagctgacttttcaacggcagctgcgagccatggcgacagaggcggtgttggaatattatctgccaacaattgagcagcgggcagacgtttatttaccgtctccaaagctgattttagaatatcaatgcagtcccatttcatttgccgaactttctcggcggacggcgaattaccagtcacttggaattgacgtggtttgggtgctgggagatcgccatttaaatgccgccaaacgattggatggtgttgccaagtttgctcgttttagcacccaactgggcttttacatcatcttttattctgctaaaaatcagcagttccgaattgattttcagattcgcgaagttgccggtaaactcactagtcatatgcgactatttaaaactttagccgagttgaagcgattcattgaccacccgccttcagctcttcaacagtattcagttcgagctactaactcggcaattttgcaccagcttaaccggattcagcggagtattgttttgaaaaatcccacttacctggacatggtcacgcgctgttatcaacgaagaaaagtctttgtcggctgccctttgatttgtcatggaaaagagggtgagggatggccgatctttcggcggactgctttgtgttggcgagtgtggattgttttgcagctgtttacgagcagtaatcgggaaatttccaatcaggagttaaatcaggttttcaaacaatcggttcaactttttggccaacaatttgcccaagtagacgattacgtccgtttctttcaaatggcctttaccagttttatctttagcctccgggccggcggctatcttcgacacacagtagccggcgtgcaaatcattaaacaaccggtgtggtttgccgattatgatgaaaaacggcaatatatcatgaccgccaagccggaggtgtgctaatctattggtaactaactatttgaaggaggacgttatgccaaaaccacaagaattaccgcttagaaaagatgttccagaagaactgacttgggatctgacgacgatttatccaaccgatcaggaatttgaaactgactatgaagctgttcaaaccggtgccaaacaattcgctgaattagccggaaccattgagaagagcgcggccgcgctgctgacggcaactgagcgtttgatgaccttaagccgaaagcttgaaaaagtctatgtctacgcccagttgaaaaatgaccaggataccagcgaagacaagtatcaggccatgtattcccgtgcggaatccttgggggctcagtttggagcggcgactgcctggtttgaaccggaactcctcaaagtttctgacgatcaaatcaagcagttttatcaggatcaacccaaactggccgattatcgacggtttttcgatcaaacctttaaacgccgtaatcatattttaagcaatgatgttgaagccgtcctggcgggggccggcgatattttctcgtctggagagaaaacctttggcattttggataacactgatctttcattcccagcagtgactgatgagaatggcaatcaggtgaagttatctcaaggtgtttatggtattttattggaatcgacaaagcaaagtgtgcgtaaagaagcgtttgaaaaattgtatcaagtttatcgtcagttccagcacacgctggcggcaacactgaccactaatgtcaagaatcacaatttcaaagccaacatccgccactataacaatgctttggaggccgctttggctgataacgaggtgccgacagacgtttataataacctgatcaaagtggtcaacgagcacctcgacctgctgcacaggtacgttgctttgcgtaaaaagattctgggccttgatgaactgcatatgtacgatatgtatacgtccctagttggtaaaaaatcacccaagtatacgtttgaacagtccaagcaaatcgctttggaagctttgcaggtaatggggccggattatgtcagccacgttaaagaggagttcaacaaccgttggattgacgttgttgaaaatcaattcaaaagaagcggcggctattcctcagggacttacgataccaatccgtatattttactgaattggaaggataatttggataatctctacacgttgatccacgaaaccggtcatagtatgcacagctactattcccatcataaccagccttatcagtatggtgattactccatttttgtcgctgaaattgcgtccacgaccaacgagaacatcttgacggattatctcttgaataaatttaaagatgatgatgaaatgaagaaatttattttaaattactatctggatggatttaagggaacggttttccgccaaactcagtttgctgaatttgaacaatacattcatgaacaggatgcaaaaggtcaaccattaaccgccaactttatggatgattactatcgcaatttaaatcaaaaatactatggtgatgccgtgatttctgaccctcagattggccttgaatggtcacggattccacatttctattacaacttctacgtttatcaatattccaccggctttgctgccgcatcgacattggctgatggcattgtgaacggcggccaggccaacgttgataaatatttgaactacctcaaatcaggcagttcggacacgccaaccaacgtcatgaaaaaagccggcgttgacatgacgcaaccggaatatcttgagaaggccttccagatttttgagcagcgtctggatgaatttgagcgtttgtacaacaaatagtttcgctaataaataagcgtaaaaaataccgacatttgggaaatcccagatgccggtatttttatggattaaattagttgaatcgcaagtttgatttgggatacggaactgtcgttggtttctttgaagcctgctcgaagtgagcggccgatcccagactcttggcacaaaagccaaagagagaattgtaatcaaagtccttgatacgaatgccactgtcagcaacgtcggaattaaacaaaacggtggttgatggatcgcggacttccatttcgtggactactcgctgatcacaacgaaacattttttctgccaaatcagagcggcggtctgccatgaacatctcgacatccaaaccatttcgttctgcgagcttggcaaccagttcatctgagtatggtactgaattaatcagaagttctttttgcaggtccatcaagaagcgtcggccaaacttctttccctgaaatgaagctgccttgaaatccaaaatggtatcgtagggcaggttgtgatcaagatggctgagttgctcgttttttgaaaagtcgtgcaggattttgatgttgagcatcgaaacaaagcgcacgctgatttgtttgtttaatttttgtgaaatccgttcaatcgttttttcggcgtcgtaacaatgtcgattaagtggatcaacgaataaataaatctcaagtaccattattgcccctccatgtgtaaccgacaacaaaattaatatactaattattttctccattaagaataccaaattttcacgtaaaaacaacaattttgcttgaagtgtgtatgattgattgggaaaggttgttgaatatggtaaaattaagtctgattgaattttaccttgaagcaatagagcgttcgtttgagcgcaacagattggaagtgttagcttggttgagaattgggatgactttttagttccttacaaacaagctgttgatgaattaaaagtaaaattacgtggcatcagagcgcaattcttaaaaattgatggtcgcagtccgattgaatttgtgaccggtcgggtgaaacccgtcgacagtattaaagaaaaaatggttagaagacacatttccgaagatcggcttgaagaagatatggaagatattgccggtttgcggatcatgtgtcagttcgttgaagatatttatcaagttgtggatttgcttcgcaaacggactgatattaatattcttgaagaacgggattatgttcataacaagaaaccgagtggatacagatcataccacattatttttgaatatcctgttcagatgcttgacggcgaaaaagtcattttggccgaaattcaagtgagaactttggcgatgaacttttgggccaccgttgaacactcattaaactacaagtatcaaggcgaatttccagatgatttgaaaggccgactggaacgatctgccgaagccgcctttcatttggatgaagaaatgtcagaaattcgtgatgaactccaagaaaccaacaagcatgagccaggcaaagatgtaaggaagtcgtctgatgaagatagccatctacagtaatcttggtgagtcgtcaaacattgtggcgacttcattaaagaaaaaaattgaagaatcacccgatttaagcatcgacggactgaatcctgaaattgtcatttctgtcggtggtgatgggacactgctgtctgcatttcaccactatcaagacattagtgatcgaattcgattggttgggattcatactggccatttaggcttttataccgactggcgggattacgaagtcgccgaactggtggacagcttggaacatgacaatggtcaaagtgtcacgtatccactgctggatatccgggttaattatgtgagtggcggcccagctgattatggcttggcgcttaacgaatcgactctcaaacagattagcggttcgatggtggctgacgtctacattaaggacacactctttgaaagttttcggggtgacggtctttgtgtctcaacgccgagtggttcgacggcctacaacaaatcagttggtggcgcaatcattaatccaaccctcaatgccattcaaatggccgaaatctcctcgattaataaccgggtctttcgaacgctgggctcaccgttgatcatttctccagatgagtgggtgaaaattgtcccgaagagttccaaccggacgattttgacttgcgatcaccaaatcatctccaacgaagccgttgaatcggtcgaataccggatttctaaacgccggattgcttttgcccagtatcggcacacgcagttttggcggcgggtaagcaactcgtttattggtaaggttaatttagatgactgaatttacgtggaaatatacaggccaggccccgatcaaggtccggacatttattatgagttacgggatcacccggacattgttgaaaaaaattaaatatcatggtggaaagactttggtgaacggtgaagcctcactggttaaccgaatgcttcaaaccggcgatacggtcaaagtcgtcctgccgcctgaaccggaaaacgatcatgtcggtgtctccaacgttccaattgaaattgttcatgaagatcccaattttttggtggtgaataagccgtacggggtggcttctgttccggcacacaaccatgttgattcattggttaatcgggtaaaaggctactatcagcgccagggctatgccaatcaaaaaatccacattgtgactcgactggataaggacaccagtggtttggtgatttttgccaaacaccactttgctcattcagttcttgataagcagttgaaggaccggacaattcaaaagacgtacctggcgattgtcgctggtcgcatttcaatgcctcactttgaaatttatctgccaattggcagagccgatgattcgttcgtcaaacgccaagtggttgattccggcaagatgtcggtgaccgaagcttggacagtgcgtcgattagccaaacagactttgttaaaagttcgactgcacaccggtcggacccatcagattcgggtgcatatggctgccattggtcatccgttgattggcgattggctttacaattcagatgaccattcaatgaccaggcaggcacttcactgtgccgagttgactttttatgatccatttgccggtcgcctgcttcattgcgaagcgcggttgccggaagatatgcagtcctacattaatttgcataaactttaattgacgattaaccaatctgtttcccgcaaaacgtgtttgagaattttggccaggaagcttttttggttggctgctgtgatataatgaactgcgtttgtggaggattttaagtgaaaaagattgattttggccaaaaatttgtgaagcagaatttacagttattccgttgtcccgtctgtcaaacaccattcgatgaggtggtgggatatagcttaagctgtccccatcatcatacttttgacatctctaaaaaagggacgctgtttttcctcaccaaacaggcaaataacgaatatgacaaatcgatgcttcaggcacgccacaagattttacaggctggccttttcgacccgattgtcgatgcgatcgcaacgtatttgggcccggaaccggaaaccattttggatgtgggctgtggtgagggcacgccgctggcacgattgctggcgcttcgagatggccaagataccgcaatcggctttgatatttccaaggatgggattaatttagcgacacaacagccagtcgatgcttttttctgtgtcgcggatttggctcggctgccgtttaatgaccacacaatttcgaccataattgatttgttttcgccatctgcctatgatgaatttaatcgggtagccaagactggcggccgattgattaagattattcccaacagcgactacctgcatgaattacgggtcgctttatttggcactgggcaaaagaacagttcttattcaaatgacaaagtatttgatctgttcatgactcactatcccagtgcaagcattgataagcttacatacgaattttcaattcccaaagggatgcagcaggaccttttgacgatgacgccgcttcactggggcaagggacggcaagataacgcccttcaactggttaatgcactcaagacgattaccgttgatgtttctgtgatggtcgcagatttttagaatatttggaggaaacaatgactaatcatatcgtactatttgaacccttaatgccggcaaataccggtaacattgcccggacctgtgccggaaccgacacggtccttgacttgattgaaccgcttggattcagcattgatgataagcacctcaagcgggccggactcgattattgggataaggtccagatcaattatcatcaaaacctgcctgaatttttgaagtcggtcaagaatccccaaaacctattcttagtttctaaatttgccaaccaggattacactgatccggattattctgacccaagtcaagattactatcttttatttggtaaggagacgaccgggttaccggaaccatttatgcgtcaaaatcctgaaaaggcgattcgaattccgcaggatgacgacaacattcgggcactgaacctgtccaacacttgcgccattgtgatctatgaagtactgagacaacagaacttcaacaatttggaacgaacgcatcaatatgaacatgataagctgaaataatcaacagccattctatgggaaggggggaacagcatgaaaaccaagcgaaccaagcaaaccagtagcaagccggttaaaaaacgcggccgtccacgaaagacgaccaagaagactggcggccagtcgagctttcttcagaaatatacggttaatgtcatcggtggtgtcgttgccattttggccttactgggattgtttcaagccggaattgtcggtaccttaatgatcaatattgccaaactgtttgtcggcagtctttatccggtctttcttttggttggaatcgttgtcggcattttcctcgcaggcttttcccggttccccaaaattccagccaagtatacttggggaacggtcctgattttgctgggcgttcttctttggctgaccttaattgaatacattcaggctgcccagccggttgactttatcaattttaactggcagaagctggttgatgatgttgtttcttctaacagtgattccaacattggtggcggcattctggcaacgattgggttttatcttgcccacgtactatttggcaaaatcggcaccggaatcgtcgccagcctgatcattttgatcggtggttttattctatttgatatttcatttgcaaaaatttttacgggtctgcggacttgtttgacatttatcaagactcgggctgcagctatccgacagcagacggaccagaaacggtctaagaagtcggctaggcagccttcaccgacaacgactgccaatcatccacaaactgtggaacagcctcaaaatgatgattctgagccaaataagttgtcggcgtcagcgatcacgatttctgggatgccagtgagtgatgaagctaagcagtcatctaaaactgtctctaagccgacacctcttcaagaatccgaaaaagcggacgattctgccgacgttaacctcgtcgatgtcaaagaagatgatgcctacaagttgccgacaaccgacctgctgacgcaaatccctcaggatgatcagtcaagcgagttgcagtcaattgaccataacgctcaagttcttcaaaagacgttggacagttttggggttaaagccgaaattaagcacgtcagtttaggcccgtcggtcaccaaatatgaattgcaccctgatattggtgttaaggtgagtcggattgtgaacctagccgatgacattgccttggcattagccgccaaagacatccggattgaagcaccaattccgggtaaatctttaattggcatcgaagtccccaaccgaaagattgcgacagtttccttcagagatgttgttgaacatcagcctgataaccacggccacgtgctccaagtgccgcttggaaaggatgttaatggcaatgtgattacggctgatcttaccaagatgcctcatttactgatcgccgggtcaactggtagtggtaaatcagttgcaatcaatggcattattaccagtattttgctgcacgccaaacccagccaggtcaaattaatgctgattgatcctaaaaaagttgagttgggcgtttataagggcattccccatctgttaagcccggttgtttccgagcctaagaaagccgccagagcactgcaaaaggtggtttccgagatggagaaccgttatgaattgtttgccaaattcggccagcgaaagattagcacttataatgattttgtcgcgaaaaacaatcgtgaaaatgacactaaaattcagccgatgccctatatcgttgtgatcgtcgacgaattggccgacttgatgatgaccgtctccaatgatgttgaagctgcaattatccggctggcgcaaatggggcgggctgctggaatccacatgattttagccacccaacggccatccgttgacgtgattaccggcttgattaaggccaatgttccgtcaagaattgcctttgcggtatcaagtgggattgattcccgcacaatcatcgatactaacggtgctgaaaaattgcttggccgtggtgacatgctgtttttaccaattgactccaacacgccgattcgagttcaaggggcctttattcccgataaggatgtctccagagtcgtcaaattcattaccgatcagcaatcagctgattatgatgaatcgatgatggttagtgatgaagagatcaaagaagaggatcaagaagattccgaagacgatttattcaacgatgctttggcctttgtggttgatcaacagaaggccagcacgtcgcttttgcaacgtcacttccggattggctataatcgggcagcccggttaattgatgatttggaaaagcgtggctatatcggtccacaagatggcagtcggccgcgtcaggtctataaggaaaaacaagaataagtttgattgacaaaaaagaggctggcacaaaagctttcacttttgtcccaacctctttaagtcgtttgtttataagaatgtcatgattgctgaaatgaccagcgaactgatcgttgcaataatcatgatccaaacaaataccaatgtaattttttgaaatctggttctctttttacgcgccaatattcgcaccactttctcttgtattccatacacagtttaactatcattatcgttcaatgcaatatgttttgtcaaaatcaggagggtaactcatgcatatttctccttggatgactgacacggtaacctttataacgcaatttctgattctatttgcagttgccgggtttttagttgttttaagaaaaaatcaatttttcaggtcgaaggtgccgattaaaccactcgatttttggccgccaattttgctgtacttcattcacgagattagtaaaaagggtttgtcggggtcattcattcccgaagtggtgattgtttggttagggctcacattgattgtgttgatctggcaaatttttgccaatccgaatttaacctacaagaaattttttatcaccttttggcgattcagtgatttatttttattcggttgttggatcgtcgtggggatttatgtcatttttgagtctatctgaatcactagctgttcatcggatcaaagcagatttttatgctttggtctttttttgtgcagaaatgggcaaatctccccaccactttcttattgccgtcagatcagtcctggacggatttttagttgaatatgaaaacggtttataacaaaaaagtgacaaattttgaggaggcgtggttgatagtggtggattgtggtagaatgtgattgtaaactgaaattgggggtgatgacgacatgttcatgggtgaatatcaacacaacattgacgccaaaggacggatcatcatccccgctaagtttcgccaggatttgggcgacaaactcgttgtcacccgtggaatggatggctgtttatttggctatccgatgagtgaatgggaaaaggttgaacaaaagatcgacactttgcccgtgaataaaaaggatgctcgttacttcacgagattctttttctccgctgcagttgaatgcgaatttgacaaacaggggagaatcaacatccccgcaactttgagggattacgcaaaaattgagaagaaatgtgtcgttgtcggtgtctccaatcgttttgaaatttggagtgacgatcgctggaacgactttagtaatgacgccgaagagaactttaatgaaattgctgaaaatatgattgatttttagataagcagacatgctggaaacgggggtgatcgaatgtctgaatttaagcatgtaactgtcctcttaaacgaggcggttaaggggttgaatattaatcccgatggtacatatgtcgatgcaacattaggtggtgggggacataccaccaagattcttgaacagttaaccaatggccatctttattcttttgatcaggacgaagaggcgattgcttataaccggcagcacttggctgaatacattgaagccggcaaattaactttgattcacgataacttccgtcatttaaaatcagctctccaaaacgttgatgtttcggggattgacggaatcgtttacgatttgggcgtttcatcacctcaatttgacgaagccggccgcggattcagttatcgctttgacgcccgccttgatatgcgaatggatcaggataatccaatcgacgcctggaagattgtgaatgaatggccttacgaaaagttggtccggattttctatcgatatggcgaagagaagtttgccaagtcaattgctcggcggattgaaactgttcgacgagaacatccaattgataccactaacgatttagtcgaagtgattaaagaaggaatcccggcagcagccagacgccatggcggccatcctgctaagaaagtctttcaagcggttcgaatcgctgtcaatgacgaattatctgcgttggaagattcactggaacaggcgttggatttgttgaatgtcaacggccgaatcagtgtcatcacttttcaatctttggaagatcgcttggttaaaaccatgttcaaagaaaaaacgtccttgccggaattaccgcctaatttaccgatcattcccgaaggcattaaaccaaaatttaaaagtattactcgaaaaccaattgttccaactgaagctgagttagaagagaatcatcgatcacatagtgccaagttgagaataattgaacgaattaaaaactagataaaggaagagtacatattatggcacaaaataatttagctcgtaacctaaccgaacaaccgcaaccgtatgtttccagccctgatcaggctaaagtaaaacgggtgagcattgcaaaagccctcaaactttcgtcctttgaaaagctgttaattgtatgtggcagcgcagtcttaactgtgttaatgttagtagttgtatcgtcaaaaattgccttgtctaattcacagcatgaacttcagcatttagacaaccaggttgtgacggttcgcaccagtaatactaatttaaaacaacagattggtgagctgcaaagcagtacccgtctggacaaaattgcacacaagagcggcatgtcactctccaatgcaaatataaggaatgttactaaatgaaagagccatctgatcgttccgcagacaaactgaatgcccgaaaaagccggaaaattgttggaataagtttgttcctcgcatttttcctgctttttgcatttttaggcagtcgtttacttgtcattgcggttgggaaaaatgttaaaaatgtcaatttaaatgaccgcgccgaaaaactttatactcaaactcagaccctcaaagccaaacgaggatctatttatgatgcaaacggtaacccaattgccgaagacaccagtacatattcgctatatgctgttttggacaagcagcaaaaagggctgaacggcaaaccactttatgttgtgaataaaactaaaactgccagggtgctcgccaagtatttaccgatcaccgaaaagaaggcattgaaaattttatcccccaaggataaacagccattccaagtggaattcggcagcgccgggaccaatatttccttactgactaaaaagaagattgaagcagccaaactgccagggattgactttgtccaaaagcaggcccgcttatatcccaacggcgtcttttcatccaatttgattggggtggcggtttctgaaaccaacaagaagaccggtaccgccaacttggttggccaaatgggtattgaaaaagccttcaacaaaacgctagccggacagaatggctttaaaaacgcccagtacgatgtctacgggtacaagcttcccggtaagcagcaaaaagaaaagccggccaaaaacgggaataatatttacacgacgattgattcacggattcaaaccctgttggagagcgagatgaactctgttcagtcacaagttcatccggctggaatgaacgccgttttgatggatgccaaaaccggaaaaatcgttgctgcttctcaacgaccaactttcaacgcggcaacgctgaaaggcatcggttcggcttggaccaacacgttatcctccgatatgtacgaaccggggtcaacaatgaaagtctttacgctgtcatcggccattaattcgggtcattataacggcactgacacctatgagtctgggcgttattcaattgacggcaagattgttcccgattggaatcctgccggatggggctatatcacttataacaaaggatttgccttgtccagtaacgttgccatggctcatttggaacaacaaatgggtcccaagacttggaaaaaatacattaagcgatttggttttcttaagagcaccaatagtggccttccgggagaactcaccggcagaattcagttcaattatccgatcgaacaggctgacacctcatttggtcaaggaattgaagtgaccactttacaaatgatgcaggctttatctgccgtttcaaataatggtacaatgatgaagccgtactttatttctaaaatcacaaacccggcgaataataaaacgattaagcaatacggcaagcaagttgttggtcatccgatcactgctgcaaccgccaaagctgtcagaaagcacatgcaagacgttgtctacaagtcttacggaatcggtgccgattacaaaatcaagggctaccgggtggctgcaaagactggtaccgctcaggtcagcaacggaatgggcggttatgcttccggtgacgacagctatctctactctgtggctggaatggttcccgccaataatccacgctacgtgatgtttatcacgatgaaacagcccaaactgactgggaccaagacagctacacaattgctggcagagattttcaaaccagtgattacccgtgcgctgcagaactcgaataccaaacaggcaaccgtcaagcggcaggtaccaacggtgacctatcagacaacgacctatgccaaacgggtgatgaatgaaaaaggctttaatgttgtgacaattgggtctggcgattcgattctcaaacaatcgccgagcgctggaacaacacaagccgaacaaaagcgggtctttttactgacaaataaaggctggaagatgccgcgaatcattggctggagtaaagccgatgttgaaaagttctgctcgctgacaggcttaaaacttgagtctactggtagtgggtacgctgacagtcaaagcatcaactttgagaagtcaattgatacgggcgatgttttaaaagtaaattttgaataatgaaggatggtaaatggcgactatgggtaattggttaacacctttattgagtacatttgtgataacggcaatttttatgccaagtttgattaaatatttccgaagccgacatgaaggtcagatgattcgagaagaggggccttcgtggcacgaaaagaagtctggcacaccgacgatgggcggcattttgttcatcgttgcgatcgtcttatccgacttggtcttcggtggggcaaaagggatgttgaacccgacgcttctcatcttactgtttgtcctgatcacctatggtctccttggaatgtgggatgacagtattaaactgtttcggcgtcagaatgaaggattaaaggcctggcagaagatgctgggacaaattgtggccgccgtgattttctcggtggtatacatacacgaaggctttccaatggcgattaaaatcccgtttggcggcgaccttcgattaggctattggtacattttgttcattgtcttttggctggttggcttttccaatgctgttaatttgaccgatgggttggatggactggttgctggtctgggaacgatttcctttgcggcctacgggattattgctgccgttcaaaagcagacggaagtggccgtcttttgtttctcggttgtcggtggtttgttggcattcttcattttcaatcacaaaccagccaagatcttcatgggagatatggggtcgctggctctcggcggagccttggcagccgtttccgtgctggttcaccacgagttctcattgttgatcattgggattatctacgtatgcgaaacggccagtgtgattattcaggtggggtcgttcaaactgactggtaaacgggtcttcaagatgacgccgattcaccatcattttgaaatgagcggctggtcagaatggaagattgatatcgttttctggctgattgccttggtggcatccgccattagtgtgatgacgatagtatagaggttgggacaaaacggctggttttgtatccagcctatttgactattcatatgatgaaaaacgagggagtaaaatgaaaaaaattgatgattataatcataagaaagtattggttttgggtgctggtaaaagtggcacccacgctgctgaactcttaaaagaattgggggcaacagttgttttgagtgattccaaacccagttctgaactgcctgaagtcgctgagctgcaggacgccggcattcaaacggttactggtaaacaggatccggccatcttagacgatggttttgacattatggtgaaaaatcctggtattccatacgataacgcggttgtagctgctgccgtcgatcaccatctaccaatcattactgaagttgaactggcttcacaaatcaccgatgccgaaatcattggtgtgactgggagtaacggtaagaccacaacggtcaccatgataactgaaatccttaaccaggaacgtgccaaagggcatgcctatgctgccggtaatattggcatttctgcgaccgaaactgccaagaaggcgacggccgacgatacgatcgtgatggaactttccagttttatgctgctgggaattaagactttgcacccacatgtggccgttttgaccaatattttctccaaccatttggactaccataaaacccgggaaaattacgtgaatgccaaaatgcggatcaccatgaatcagacgcctgaagatttctttgtggtcaactttgattctgatgaatggcgcggcttaagcaaacgcagtgctgctaaggtcgttccctttgccagaacaactgagattgacaagggcgcttacgagaagaacggcaagctgtattacaacgacgaattcatcatgaatgccgaggatatcaaagttcccggaaagcaaaacgttgagaatgccttggcggcaattgcctgtgcaaaagtgctgggcaaatccaatttggcaatcaccaatgtgttggaaacgttcaccggcgttcgccaccggcttcaatttgttcttgaagccaacggccgcaagttctacaacgattccaaggcaacggatattgaggcgactcagatggcccttgaaggttttgacaaaccagttgttttattggctggtggacttgaccgcggttatacgtttgacaaactgattccgcaatttaaggaacatgttaaggctgcagtcttatttggcgaaactgccgatcttttggaagactccctgaagaaggccggcattcaaaatattcaaaaagttgataatatcgatgaagctgttccagcagcatactcatttagtgatgaaggcgacattgtgttgctttcaccagccaacgccagctgggatcagttcaagacctttgaggagcgtggcgatcgttatattgcagatgtggagaaattgacggataagcaggaggggcactaatgcgtttaatcatttctggtggcggtaccggcggtcacatctacccggcactggcaattaccgaggatttacttaaacaggaacctgattcagaagttctctatgtcgggtctcagcgaggcctggagagttccatcgttcccgagcagggaatcaagtttgttgccttggaaattcaagggttcaagcggtcgctgtcattggagaacttcaaaacggtggcgttgttcctaaagagcgtgcatgaatccaaaaagatcattcgagactttaagcctgacgtggtcattggaacaggcgggtatgtttccggagcagtggtttatgccgcggccaaagcccacatcccaaccatgatccatgagcaaaatagtgcggttggattaaccaacaaatttttgagtcgctatgtggacaagattgcgattggctttcatgaggcagccagtcaatttcctaaagaaaaagttgtcttcgctggcaatccccgcgcccagcaagtggctaatatgaagagtactttcaagtggtccgatgtggggctgcaagatggtgaaccgaccgttctcattttcggcggcagccagggggcaccggcaattaataaggccgtgatcggcgctgtcagcgagtttaacaaacgccagtaccaagtggttttcgtcaccggtcaaaagcgttatcaaaacgtgatgaatttgctggataaaacgcggatcagcagtaacttcaaaattctgccgtacataaacaacatgccgcaagtcttaccgaaagtttcgctgattgtcggtcggtcaggagctaccagcattgccgaaataacggccctggggattccagccgttttgattccaagtccatatgtcacggctgatcatcaaaccaagaacacgatgagtttggttaaccgcggcgcggcattgatgatcaaacaggaagatttgaatcctaaaagtttgttaaaggccgtcgatcagttgatgcacgattcaacggcacgtgagaaaatggcagagaattcaaagcagctcggcgtcgttgattccgctgacgaaattttgaatttagccagaacactgaccaagtagtctgataatcgggggtagagatcgttgggagcacaagaccaaaatgggaagaatcacggaggattgtttcgcgatttccaaaataggaacgtcaaaaaaatgtggccgttggtgatgccgattaccatcattttgttggtcatgatctttatgatctcgtcatacagtcgcgtgaaaaaggtcaccgtttccggtaatgagattgtcagcgatcaacaaatcaaggctttttcccctgttaagaagggaacgtcactgtttgctgtctgggggaaaacggacaagcttgcccaatccctcaaacaacgcagcagacggatgcaatcggtgaagatgaagctggtcaactttaatcaggtgaagattaaagtcgaggaatatccaacgattggctatctcttcgttcacggcggctatcagccaattttaaagagcggcgtgattattaaggggaaagttttgaatcccaaggccggttttccggttctgaagaaatttcaaaatcctaaaaaactgcggcggacgatcaaacagtaccgacgaatcagtccaccggttcgcgcagttatgaacacgattagcttttcaccgactaagagtaaccccgatcgaatttttattcagatgagtgacggcaacaaagtctatgcgtcaatcagtacatttggcgacaaaatggactactatccaagcatcagttccaagctgaaagtcaaaagtgtcatcaatttggaggtcggcgcctattcgtacccaatcccccaaaaacagacttcaacaaaaacgaccagtgtacagggctattagagctaattaatctttttcgatgtttatgattgtgttaaacttatgttatgttcagaaaatattctagatgtggaggttccttacatatatggataattcgggtttatatgtgggacttgatataggaactacctcaataaaagtaattgttgcagaaaaagtaaaagggcaattgaacgttattggtgtgggaaatcagccttcaaatggattgagccgtggtgtgatcgttgatattgaccaagctgcagacgcaattcggagtgctgtaaatcaagctcaagaaaaagcaagtattgagattaaagacgtgattgtaagtgttccggcgaacatgttacggattgagccatgcaatgggttaattactttggatgatcaatcacgtgaaatcactgaggaagatgtccgaaacgttgcggcatccgcacttggcaccagtttgccacaagaacgagagataattgatattcagccggaagaattcattgttgacggattcgacggcatcaaagaccctcgggggatggtcggcgttcgtctggaaatgcgcggtaagttaattaccggttcaaaaggcattatgcacaacctgcaaaaggccgtgaataaagccggtttgaatattatttcaactgttttaacgcctctggctgaaagccacgtggtgttaaatgacggtgaacaggactttgggacgattattgtggatcttggcggcggacaaacaaccgcttcagtcattcatgatcatcaattaaaatatgccacaaccgatcctgagggcggcacatttattactaaagacatttcaattgttttaaatacatcaatggaaaatgctgaaaagatcaaacgtgattacggttacgccgattcattgcaggcatcggcagataatgaatttccagttgaagtagttggccaatcagaaccaacttacatcgacgagcgttatctcgcagaagtgatcgaagcgcgtttaagccagatttttgatcggatcaaagatcgtttgaatcagattcaagcgcttgatttgccaggtggaattgttctgactggtggtgtggctgcacttccaggaattgccgaattagccgctgaccaattcaacactaatgtcagggtctatattcctgatcagatgggattgcgacacccatcgtttacagctgcactttcactagtgtcatactttgccgatctggcagacgttgatatgattgttcgatcggccgttggtgcaacattgaccaaagcgcctaagttgagtcagcctgagcagacaccaatgcctgcagctgggaagactaagaagaccaagaaaccgacacagaagaaaaaacgcggtgaaggaatcaagaatttctttagtgatttctttgattaagcacttaaacggagggaaaagacaattatggaatattcattagattccaccgataaccatggtgcaaacataaaagttatcggcgttggcggtgggggaagtaatgccgttaacacgatgattaactcagatgtaaaaggtgttgaatttatcgttgccaacaccgatgttcaggctttggcaacttcaaaagccgaaaccagaattcaattgggacccaaactcacacgtggtttgggagccggctccaacccggacgttggtgccaaagctgctgaagaaagtgaagaagcaatcactgaagcacttgaaggtgctgacatgattttcgtgacggccggaatgggtggtggtaccggtaatggtgctgcaccaattgttgctaaaattgctaaagaccagggtgcactcacagtgggtgtggttacccgtccatttagtttcgaaggaccacgtcgggcaaaatatgccgatgaaggagttgctcaactaaaagagaatgttgatactttaatcgttatttccaataaccggttacttgaaatggttgacaagaagacaccaatgatggacgcctttaaggaagccgacaatgtcttgcgccaaggggttcaaggaatttcagacttgattaccagccctggctacgtcaacttggactttgccgatgttaagaccaccatgcaggatcaaggttctgctttgatgggtgtcggcactgctaacggtgaaaatcggactgccgaagcaaccaagaaagcaatttcttcgccattgttggaagtttcaattgatggtgctgaacaagtattattgaacatcaccggcggaccagatttatcattgtttgaagcccaagatgcttctgacattgtgtcacaggctgcgacgagcgatgtgaacattattttcggaacgtcaattgacgaaaccttgggtgacgaggtccgcgtgacggttatcgccaccggaattgataagaaaaaggctgaacaggatcggatgtcaacacggcggacccgctctgctcgtccacagccaactgcccggccacattcagaccgtcaagctccagaaaccaatcaatcacaggattcttcaaatgctaagagtgatccacttggtaattgggacatcagaaaacaaccagcgccaactcgtcctgctgctcaggatgaatttagcgacgttgagaaaaaggatttcgatcctttccaacctgatgttaattctgacgatacaagaccagataccagtgatgattcacaagacgacattccaccattcttcaagcaccgtcgtcggggcaagtaacatcagctgaccggtgccgatgtttggtgaaatgtgaaaggacacgaaatgccaaaatttaatttagctaatttttttgggatggatacagaccaaccagaaaatcaaattgataagccggcggacaacgttgtattgatgaatcgacaagaactagaaaccagcagcattgttgttttggaacccgttaattataccgatgttgacaccatcgcccaaaaactattggaggacagtgcggtcatcatcaaattggataaattggataacaattccgctgcccggatggttgatttcttgaacggtgttttgtttgccattcacggatcaatcaatcggctcggtaggaacatcttcatttgttcaccgaagaaatttcaagtaactgagtaatctcgagaaaataaggagcaacctattggtcacatttgttatgtatgcagtttggtttatcgacaaggctatcaacatttatatgctgtgtattgtcgtgtatgccctgatgagttggttcccgaatgcttatggaacagcaattggccgatttttggctcggattgttgaaccatttgaaagcttgtttaattttgccacgattgggatgattagtctcgctccgattgttgcattagcggtgctgacgttcgtccaaatgggcgtcaactatcttggacaattgttaatcggctactaattggggtatggacatttcagccagagggggaaatatcttggtagactcgaatgtttcgcaacactatcgacaggctgaattgccttttttagagtcaatcgacagtttgagcggcagggttgcgaatgaatatcgaccgatccttactgattttttaaatcctagacagctttatatacttgaaacaatcgtcaacagatacgagggtgtctcatttcaaacttttggtgggtatccctcagctgaattaaaacgagcggttgcctttccggattactttgttcccaaggccgatgattacaatattacggctttccagattgactatcccagtaaatttgccacgttatcccacggacaaattctgggatcgattatgggaagcggcattgatcgagatgtcatcggcgatattgtcaccgatggtttgaattggcaatttatgtgtgaatctgagatggccgattatgttcaatcacaagttgaccggatcggcaagatcaaaatcaagttgaaacaaattcagcctgaggagattattgcgccggttgatgaaggtgaagaattaacgacaaccgttgcttctttgcgggtcgatgcactcgttagtgaaggattccacatttcccgtcatcatgccaaggaattgatcgaaggcggcatgattcgaatcaattgggaagatgccaaccgaccggatcttgaaatttccattcaggatattatttcggttcgcggtttcggcagactggttgtccaagacattgccggtatgactaaaaaaggcaagattcggatcggattaaaagtatataatcgaaataaataggaggattgaatcattatggtattaagcccacaagatattcataacaaggaattttcgacaaaattacgaggttacaatgttgatgaggttaacgattttcttgaccaagtcatcaaggattatcagatcgttttgcaggagaacaaggatttgaactctcagctaaacgaagctaaggacaaactttcctactttaacgatttaaaagattctttgaaccagtccatcttggttgcccaggaagctgctgataaggttaaaaccaattcgaagaaggaagctgaaattaccagccgtgaagctcaaaaaaaggctgacgatattttgaatgctgccaacgaaaaggcggatgccgttttggaagaagcttcaaaacgcgctaagaagttagcgattgaaacagatgatttaaagaagaacaccagggtattccgtcaacgacttcaagtcatgttggaaagccagctcgaagtcatcaaagggtctgattgggatcgcttggttgaagaaaagccaaccacaacttacgaagatatcgaaaaagttgttggtagccttgacaacattggaaacccaggggtacaatctgaaactaaacagagtaatggcgctgcagatgttgaagaaacaccggctactgtggatgattcaaaccagaccgtcgtgatttatccagatggtcgcacacaaaatgaataattaatcgattagagaaaagaaagttattggctgaaacaacagcgagctgaagatagtgggagttcagcagtcaccaaccggtaaatcgatcacctctagtacataaatcgattatctgaagagatagaattttaaattctaaaattgggtggtaccgcgaagacttcgtcccttgtgacggggtctttttttgtagagtgcgacgagggttgcgttttagcaatactacccaaacttcatccaccaaccaaatttctcaacatcaacacatcatcactccactaaatatctccatgaaaggaagtccagcaatgcgggtaaaagatacattaaacttaggcaaaacaaagttcaaaatgcgtggtaatcttcctgttaaagaagtcgatcgtcaaaaggcttgggaagacaacgatgtttatcaacaaagacaaaaattaaacgagggcaaaccaacatttgtccttcatgatgggcctccatatgccaatggtgacattcatatgggccatgcgttgaacaaaatttcaaaggatatcattgttcgatacaaatccatgacaggttaccgggccccttacgttccaggttgggatacccatggcctgccaattgaacaaaagttgacgcaagccggatatgaccggaagaagatgtcgaccaatgatttccgtaaattgtgtcgggattatgcgttgaaacaggttgaccgacaaaaagaagaattcaaacgtctgggtgtttcaggtgactgggacgatccatacctcactttgaagccagaatttgaagcccaagaagttcgggtgtttggcgccttcgctaaacgtggcttgatttacaaaggtaaaaaaccagtttactggtcatggtcctcagagtctgccctcgctgaagccgaggttgaatatcatgacatcacctcaccaaccgctttttatggtgaacacgtcgttgatggtaaaggtgtcttggatgacgatacctacatggtggtttggacaactacgccatggaccattcctgcttctgaaggaattaccgtggatgccggatttgattattcagttgttcagcctgaaggcgaaactcggaaatttgttatcgccactgagttggttgataaagtcgccgatctcattggctggaccaacgtcaagacgatcaagaccgttaaaggccaagaccttgaaggcattttggcagaacatccatttgatcatagtcgtaaattattaacgatgttgggcgatttcgtggaccttgaagaaggaaccggattagtccataccgctcctggttatggtgaagatgactttaatatcggccgtcaatacggtctggatatttttgcgccagttgacgacaaaggctacttgactaaagaatccggtgaagactttgccggcgttttctatgatgatgccaacaagattgccttggataaattaaaggacgctaagttgttgcttcactacatgccgttgaagcatagctatccatttgactggcggaccaaaaagccgatcatcttccgggcaacgcctcagtggtttgcatctgttgataagattaaagatgaaatcttaaaatcattggacgatgtccaattcttccctgattggggcaaggttcgactatccaacatgatcaaaaaccgtggcgactgggttatctcccgtcagcgggtttggggtgtgccactgccaatcttctatggcgaagatggtgaagcaatcattactgaagagaccgttaaccatgtagctgatttgttcgaaaagtatggttctgacatttggtttgaaaaggatgccaaggacttattacctgatggtttcacaagtgagcattcaccaaacggaaagttcactaaagaaaatgacatcatggatgtttggtttgattcaggctcctcccaccaaggggtgcttgaagaacgtaaagagctgacttatccggctgatatgtaccttgaaggttcggaccagtaccgtggctggtttaactccagtttgattaccagtgttgcggtttctggtaaagccccttacaagcaagtcgtttcccaaggatttacccttgatggcaatggccataagatgagtaagtcacttggtaataccattgcaccaatcgatgtgattaagaagatgggggctgaaattgtccgcctgtgggttacctccgttgatacttcagctgatgtgcgggtaagtaccgagaacttcgtcaaggtttctgattcttataagaagatccgaaacacgatgcgattcttgttggccaacacgtcagactttgatcccaaagaaaatacggttgcctttgacgacttggaatctcaagatcaatacatgctggtgctcttcaataaattcttagccgataccagaagctatatggaacgatatgacttcctggactggaacaagaaggttgttggatttattaccaatgatttgtccgcattctatctggatatcgccaaggacattgtctacattgacaagcaggacggtcacaaacgccgttcgatgcagacggtcatgtatgagattgccgttggcttaaccaagttaatgactccagtgttgcctcataccactgaagaaatttggggcttcctccacgaacccgaagaatttgttcaattaaccgatattccggaacccaagaagtacgaccacgattctgaaatcctggccaactggacgaaattccgaagctatcgtgatgacgttttgaaggttcttgaagaggctcgtgacgccaagaagattggtaagtcatccgaagccgctttgacgatttacgcaaccagtgaagtggctgacttgatggacagtttacagaccgatttggcaactgttttgatggtttctcaattgacgatgaaggactttgctgatgcacctgatgacagtacgaaatttgatagcgacggcttggcattatcagttgaacccgctgaaggcaagacctgtgaacgctgccgtttggttcgccaagatgttggtgcagacagtgactacccaaccttctgtcaatcctgtgcccaaattgtccgtgaccagttccctgaaaccgcaactgaaggttttgaggaaaagtaaagcggcctttgagacgttgatcgtttaaatttcatcaaaagctgttccaatcttcatgattaaacattaaaatgagactatgacttaaatgttgtagtcttatttttgtattttaattaattgaaatgtgctctggctcacagattgtgccaaacaccttggaggatattttgcttaaaggaaaaattaaaagttacaacccacaaaatgcatttggtttcattacccaagacagcggtgaagacgatctgttcttcttcaaaaatgcctttcctgaagatcaatacggcaccattcaagttggcaagccggtagaatacgttgtcgttgccggacaaaagggaccgcaagctgccaaggcgcacgtgatcgaagattagccgtcttgattgcaatgacccggtattatttgtaaaatgatattattaactaaaaaaggtgatcgagttggactttgaagaaaaagtaattggcacagagaagatctacgatggcgcaattatcaacgttgaaaaacagacagttaagctgcctgacggacagacatcatttcgagaaattgtccaccattccggagcggtcgggatcttagccctcactcacgataataaaattattcttgagaagcagtggcgggcaccggctaaaaagaccaccattgagattccggcaggaaaagtagacggacgggatgctaattttcacgacaccgtcattcgggaattgaacgaagaaatccgttatgttcccaacaccatcaaagaactctatggcttttactcgtcagtcggcttttctgacgaatacatgaaattataccttgccgaaggcctgaaacctgttgccaatcaattgccgcgggacaaaggtgaattccttgaagtgtttgaaaaaacgctggatgaagctgtggcaatgattgcggatggcgagattcaagatgcaaagaccattactgccattcaatattggcagttaatgcaaaagtaggtgaccatttaacttggcgatcgatgataatcacaaaaatgacggaaaaccgttaacgcgagaacagtatcgaaaattaaaattacagcaggaagcagactttgaggcccgcgacaaacggcgggttcaagtcgaacgcgaatatgcaagaaaacaccaacagccggtttccgaagcgacgcctgaacctcaggaaacgacgcgggcacgtgaaaatcatccagcagatgacgatttcaaaacgccgcgttggcaccggattaaccgcaaactgaattggacaatcacaatcttaattttattgatggtgatcgtttttttagtgttgttttttgtaaattaaggagaatttgaatgacttacggaattatttgtgcaatggacgaagaactggcaatcttaaaagaagccttgtctggcgaagaaaccaagcattacggcaatgctgattattatttgggaacaattcacggccaaacactggtcatcgttaaatcagggattggtaaagttcaagccggcatcacgacctcaactctgatcaatgaatttcacgtggatgccgtgattaactcgggttcagccggtggcatcggtgaaggtttatcggtcggtgacatcgttgtttcgaccgagacggcctatcatgacgtggatgtcaccacttccggttaccaaatgggccagctgcccggctttcccgcccgctttaaagcctcagaggaactcgctgacaagattgtcaaagcggcccaacaaagtggcgtgactgcccacaaggggttaatcgtttccggtgaccaatttattgccgattcaaacaaaattgctcaaattaagcacaactttcccgatgccctgtgttctgaaatggaaggggcagctgttggccaagtggcctatcaaaacaaagtgccatatgcggttatccgggcaatgtctgacgttggtgatgaagaggcagaagtcagttttgacaaatttatcatcacggccggcaaaaagtccggtcagatgttgattgacctctttaagaacgagtgactttaaggagtgaaaataatgaaagagatatatcttgataatgctgcaactaccccggtttctgatgaagtatacacagaattaatggataagtataaaaacatttacggtaacgcttccacgctttacggcctggggagagaatccaaagccgtcatggaaaatgcccgggatgtgattgctaaaagcattaacgctgatccagacgacatcgtctttaccagtggcggttctgaaagcgacaatacggcgattacccaaactgcgattgcccgcaagtcactgggcaatcacattatcacaaccgccattgagcacgaagccgttatcaggccgtgtgaggccttggagaaaatgggctttcgggttacctatcttcccgttgacgagtatggcaacatctctttagacgactttaaggctgctttggacgatcagacgatcctggtttccatcatgactggaaacaatgaggttggttcaattatgccaattcatgaaatcggtgaaatcttgaaggaccatcaggcttggttccatacggatgctgtgcaggcatatggtttgttggatatcgatgttcaacgtgaccatattgatatgctgtcgacatcggcacacaagattaatggtcctaagatgattggttttctctaccggcgtaaaggggtgaatttccctagtttaattaagggcggcgaccaagaggaaaagcgacgtgccgggactgagaatgttcctgcaattgccggatttgccaaggcggtccaaacgatcacaccagaagagaaggcgcaccgacaagccaaatatttgaaatttaagcagtatatcgctgataaattgaagcaaaacggagtcgagttcgaggtcaacggtcgaatcaccgaggataatttgaaccacgtcttcaatatttggcttaaaggcatctcgacttatgtgatgcaaactaatctggatctggcaggaattgcggtttccggcggatcagcatgtacggctggtagtatcgagccatcgcacgttttggtggcaatgtacggcaaggatagcccaagaattagtgagtcgattagaatcagttttgggcgttacaatacgactgaggacctggataagttggtagatgcaattaccaagattgttaatcgggtcaaaaccaagggggtaaagatgtaatggcattcgcaaaaacaggtaaggttaacggtgatgatacagtgtatgaactaagggataacgttaaacggttcacactgcgtgatttgggatttattgagggcaagaccggtgtcttttcactggaaaagtcattagacccaacatcgccgtataatgccaactataaattcaaaatgaaggttgataaggatctaagtggttttagaatggcgatcaccacgggaaatggtctggaaaaagtcaacatcttcaagaatccggatacccaaccaagtgtcgagcaatatcaatttattattaacgatttgattgatagggatgtgctaaaaagaagagtgtgacgagagccggttagggcccggaacataagtgattaaggccaatgacgaacgctttttgttcgtcgttggccttaattgcttatgtggtagggccctgggtctcggaacacgtttcagctgagtaacagtgaactaaacactatatgggaggaaaaggccaaccaccaatttaaacaagtaattgtacatcacaatcaaacaaacccaatttgcaacattcaatcgttgggcccgggcaaaactaatccttttgcctgggcctttttacagtctgccattctacctagtcgaatcttgcccccatcagcagcttccggccatataagcgggggacactgttttttccaagattaacattgacacgtccacgtaaaagcgataaattagattataattaagatatgatgataaacggataagtgatgatcttatgaacaatttgtgtttcacgttcgtctgatgatttcttacatatctgaattgtagaaaccatacttagttacaacgcttatcacctgcttaatcaatattttaaggaggacacatatacatggcaaaacaaaagttagaagatttagattggaccaaccttggattcgcctatcgtgatttaccatacagttacaacgaggaatttaaggatggcaagtggcaaaacggcgggttaaccaccgactcaacactgactttcaacgaagctgctgaagatttgcattatggtcaggaagtttttgaagggatgaaagcctatcgtaccaaggacggccgaattcaacttttccgtcctgacatgaacgccaagcgctttacgaattctgccaaacgtttggtaatggaaccatatcccgaagataaatttgttgaagccgttaaagaagttgttaaagccaacgctgattttgtgccaccttatggttcgggcggctcgctttacatccgtccgttcatggttggaaccgaaccactggttggcgtttcaccttcgtcaacttacaccttccacatctacgccaccccggttggtgcatacattaaaggccttcatccaatgccatacatggtcagcaaatatgaccgggctgcttacgctggtaccggtcaggctaagactgccggtaactatgccggaagtttgttagcagctaaggaagctaaagataacggctttgccggcgaactttatttggacccacgtcaacataaatacgttgatgaatttggcggtgccaacttctatgcaattggcaaggacggcaagttctacacaccaaaatctcattcaatcctgccgtcaattaccaagaaatcgatcttgcaaattgccaaagacttaggattagatccttctgaaaccaacatcgatgtcaatgacttggatgaatacactgaagctggtgccatggggacggctgcggttatttcaccggttggctctttaaccaacaatggtaaaaagcacgtcttttacagtgaaaccgagccgggacccgttacacaaaagctttacgatacattatttgggattcagtcaggtgatgttgaagataaatatggctgggttgttccggttgaataaagagtgggacttaaagcggttagtttccacgtttccgcaaggtaatatttaaaatcataaaagttcaggtgagacaaacaatatttttgtctcacttttttgaccgccgaatcccttggaaagtgtttgacattttttctggcaaacattagaatattagaaaatggttagaccgatgacaactatttactacatatcctcaggagggacactatggcaaaagcaaaaccggcaacagaaattgattgggaaaacttaggcttcgattatatggacttaccgtatcggttcttagcgcattatcaggatggtcagtgggatgaaggtcaactcactgaagatggtactttacacatcagtgagggctcgaccgggcttcattacggtcaggctgatttcgaaggcttgaaggcttatcgaaccaaggacggcagtattaatttgttcaggccggatcaaaacgccaaacggatgactaaatcctgtgcccgtttattgatgccggcatttccggaagataaatttgtggcagcggttaaaaaagtggtcgctgccaatgccgactatgtgccaccatacggaacgggcggaactctttacttgcgtccgctgatgattggtgttggtggtaacatcggcgttcatccggctgatgaatacatcttcacgatttttgccatgccggttggggcttactataagggtggtctgaagccaaccaatttcacgacttcatactatgatcgggctgcgcctcatggcactggtcaaagcaaggttggtggcaactacggcggcagtttgctgcccggtgaccaagcccacaaagccgggtattctgacgtgatttatttggacccggcaacccataccaagattgaagaggcggggtcagccaacttctttgggattaccgcagacaatgagtttgtcacaccaaaatcagattcgattttgccaagtattaccaaatattcactgttgtatctggcggaacaccgacttgggttaaaggccgttgaaggtgacgtcttcattgacgatttagatcgattcgaagaggccggcgccatgggaacggccgcggtgattgcaccgattggcgggattgaatataaggacaacttacatgtcttttatagtgaaacagaagttgcaccgattaccaagaaactctacaacgaactaaccggcattcagtttggggatgtggaagctccagaagcttggattcaaaaagtcgaagtttaattgattaacaaatgatggcaccagaaaagagggctgggacaaaacgaacggttttgcccggccctttgtgttttaattggcgatttgctacacaccaggttagtcgatggtctatgaaaggatggtcattgtgatcaaacgagaaggtcattcccacacagaattttgtccccatggaagtggggatgatgtggaattaatgattcaaaaagcgatcaagctgggttttgaagaatacagtattaccgaacatgccccgttgcccgaaggactggctgataagtatgccgggaaaacaaccggactcacggaggcctcaatggcggccgctgatttggacgcttattttcaaaaagccaaccaaatgaaggccaagtatgcggaccaaatcaaaatcaacattggctttgaagttgacttcttgcctgattttgtcgattggactcgcgactttttgaacgaatacggcccgcgaacaactgataatattttgtcggttcacttcatgcaaggggcaaacgataaattctggtgtgtcgatgatactgtggaagatttccaggccggattattgagtcagtatcccgactcacaagtcctatatgagcattattttcaaaccgtcctggcctccgtgaatgctgacttgggtccgtacactcccaaccggattggccacatgactttggttaaaaaattccaagattattttggcttggatcgtaacttttctgagaacaatctaagactggttgatcaaattctcaaggcggttagcggtcaacaccgtgaactggatttgaacgctgccgggttgtacaagccctactgtaatgagcagtacccgtcctattcagttatccagatggcaaaatcgttaaacattccatttgtttatggcagtgatgcccatagtattgccgaagtcggtcagggttacaatggcgtgatttcattagttgaataaatcgcttgacaatcgatggtttggtgatagtatatgaaactaaataaagcaaaagttaatataataaagttttgattagaaaaagtaaccagtggtaatttaaaagagagtgccattgttgaaaaggcacattttacactggcgaacacacatctatgaactaaccggttgaaccaagtaggccggttcgcatgtttagcgttatcagggttaccgtatctgttatcagaggatgactagatattggcaacgtaaggccgactactgtgaggtagcggcaaattgaggtggaaccacgactttaaggcgtcctcgaagactgaatacagttttcgaggactttttttatcgaaataggaagtgacagttatgaaaaataagaatttaccaatcggcacccgtgacgagtttggcacggaagcggaagtcaaagaaacgattcaaaataaactttttcagggcttttggcggcggggatttcgtaagttaaccaccccggttttagaatattcagatgtttttcaacctctgaatgccgaaaattatcgtccctaccaattattggacgagcaaggcgaaccactggttttacggcccgatttgaccctcccggttgcccgagtcatgagtacgaccggcattgagctgccagtgaaatggtattacggcggcgacgttttccgagtaaagaagcagttatccggaagttataaccaattaactcaggccggaattgaaattgttgggtacaagggcttgaaagccgattgggagtgtctggaagttgctttagcaggatgtcgggacatggccatcgaaaatgtcacgattgaactcagtcatgccaagtttgttgatgtgctgattgatcggctggatttgccggagcccaccaaagctggtttgaagcaagcgttgttcgccaaagatctcagcaagtacaaccaactcgcacatccactggcagaaacaccgttttcatcgttcgtcaatgaatggccgtggttgtttggcaattttgatgaggtgatgacagtcgttgacacattaccgccgattgaggagttggcggggatcgttaatcacttaaaatcaacggcggccttcatccaagagttattccccaaagtcaacgttaccttggacttaagcattccttctccacagagctattacaccggcatggcttttcgcggctttaccgataaatcctcaggctatttgttcagtggtggtcgctacgatgacttattaaccaatttccaaaatgtcaaaacgtctgccgtgggggtggcattcgacgttgatgccttggtcgaacggaccagcttccctgatgacacaccaaccacgctgatcttctttgaggacgaccaatggcaggaggcagaagcggctttatccaagttcgccaatgcgaccctctgtctgaccgacgattttgaagctgctaaacggctggcagccagtaccaacagtcaactcattgatttaacaaaagcaggtgaaaaatgatggaacgaattaaaattgcccttactaaaggccgaaccgaagatcaagtggtcccattactggaagcagctgggattaactgcgaggggattcgcaacaagcaacggcggctgattttcgatgaagatccccgttacgaaattatcctggttaaaggcccggacgtcctgacctatcttaacagcggttcggttcaaatcgggattgttggcagcgacatcctggccgaacaagaaaatttccaatacgcaatgttggatctcaacgtcggcaaatgccggtttgtcttggcatcaaccaaagatttcaatccccaggcccaccggcgcaaaataattgccaccaaatatcccaacattaccaaacggtattttcaagggattggcgaagacgttgaaatcatcaaaattgaagggtcggttgaactggcgccattgattggcctggccgacgcgattgtcgatattgtcgaaaccggcaacaccctgcgtgaaaacaatctccaagtcttcgcaaaactacagccagtcaacaccaaagtcgtggttaatcgattggcacttcgccagtaccaacctcaaatcaaaagcttgattgccagcctcgccaaggccgacgatcaactgatccaatccaaattaattaaggagtgagcaaaatgcgaacagcaacgatttctcgcaacacaaatgaaacccaaattgaattaagtctcaacttggatgactattcaaagattcaaattgataccggaattggctttttcaatcatatgctggatgcatttgcccgccacggccgcttcgggttggtggtcaaagccaaaggagatttagatgttgacccgcatcacaccacagaagacgttgggattgctttgggactggcactcaaacaggcgttaggcgataaagcaggcatcgaacgatttggctccgccttaattccgcttgatgaaactctcagtcgagtggttatcgatttgtccggccggtcttatctggtatttaaagccgaatttgccaacgaccacctgggcggctacgataccgaagtcactgaagacttcttccaagcattcgccttcaacgctgaaatgaatcttcacgcagaagttttatatggcagaaatacccaccacaaaattgaaacacttttcaaggcgctgggcagatcccttcgagcagctgtgaccatcaatccagaaatcaaggggatcccgtcgactaagggggttatctaatgatcacaattattgattacgacactggcaatacccgcaacgttaaaaacgccttggatttcttgggcgttcccaatcaattatctgccgatcccagtgagatattgacggctgatggattaattctgccgggtgtcggcgcctttaaaaaagccatggattctttaaatgaacgtggtttagttccggtgattcaacaggctgccgatgcaggaatcccaattttagggatttgcctgggaatgcagattctgtttgataaaagttatgaatttggtgagtcaaacggtctggggttaattgccggtgaagtggtgccgattcctgagaatttgggggtcaaggtccctcacatgggctgggatcaaaaccagtctcagcagaccgatgcacttggagatgggttcgacggtcagttcagttactttgttcattcctactacgttcaaacggcggccgaaaacattgtttcgacagtcgattatggcgtccagattccaagtatcgtgcgaaaagacaatgttattggttttcaatttcatcctgaaaagagtggtgaagttggactgaatggtttggcaaaattcaaggagatggttgaaaatgcagattattcccgcaattgacttaaagaatcaacaaagtgtccggctttatcagggtgatttccaacagacaaccgttattagcaagtcgcccttacaacaggcagtggcaatcgattctgccggcttgaaaaatttgcatctcgttgacttggatggcgccaagtcaggacggccggtcaatcgggcattgatcgaacaaatctgcgcccaaactgatctcaaagttgaagttggcggcggaattcgctcactctcccaaattaatacttacctgacatcaggcgttaaccgcgtgattctggggtcagcagccctgaacaaccccaagttggtgcagcaggccatcgaacaatttggcgctgatcaaatcgtcgttggcattgacggcaaggatggtcgggtggccgtttcgggctggctggaacaaagttccgtggaaatgggtgaactgatggcctcaatggtggcctttggtgtcaataccttcgtggtaacggatatttcccgggatgggacgatgactgggcccaataccgctcagctcagtagcctgcaagccaaatttcctcaagtcaccgtggtggcttccggtggcatccgtaacgtttcagatcttgaggatttgcaaaccgctgggattaaagcagcgattgtcggtaaagcaatggcaacgggtgatttaccgctcgatgtcttggcggaggtgaataccagtgttagctaaacgaattattccttgtttggatgttgaccacggccgagtgaagaagggggtcaactttgtcaatttgcaggacgttggtgatccaaccgagattgcggctgcctatcaacaacaaggtgccgatgagctggtgtttttggacatcaccgcgaccaatgagaagcgtaaggcgatcgttgagaccattgaaaaagtcgccagccaagtcttcatgccgctgacaattggtggcggcatccatagcgtcgacgatatgcaaaatctgctgaaagccggcgccgataagacagccgttaattcagccgctgtcagtaacccccagttaatcacggccggagctgaaaaatttggcgctcaatgcgttgtgttagccattgatgccaaatggaatccagaatccgggcagtatgatgtgtacgtcaacggcggccgtcaacgcacgaatttaaatgcgattgagtgggccaaaaaaggggttgcgctcggagccggtgaactcttagttaccagcatggataaagacggcaccaagagtggttatgatattaacctgtacaaacagctaaccgctgccgtgaacgtaccggtgattgcttctggtggctgtgggcaactgggtgactttgctgaagtctttgaccaagcagatgttgacggtgctttggcagcctcggtctttcactttggtgaactgacgattgctgatgtgaaaactgatttacgcaaagacggggtgatcgtacgatgaaacctgattttgaaaaatattcagacggcctggtaccgacaattgtgattgatgacaataccaaacaagtgttgatgatggcctatgttaatgaagaaagtttcaatttgagtatgcaaaccagacaaacctggttttggtctcgaagtcgccaagaattgtggcacaagggtgaaactagtggcaatacgcaagaaatcgtttcaatcgatattgactgtgatgaagatactttattgatgaaagtgattccggccggaccggcatgtcataccgggcacaccagctgcttttaccggaccattttaccggaaccaaccaaggaggaataatatatgcaagatttagacgaactttatcaattaattttggaacgcaaaaacaaccccgagaagggctcatacaccgattatttatttaccaagggtctcgataagatcctgaaaaaagtgggtgaagaagcaaccgaagtggttgtggctgcgaagaatccgtccgatcccgactttattttggaagttgccgatttggcctaccatgtcgaagttctgatggcccaacgcggaattacccccgaccagattaagcaggagcttgccagccgtgaaggcaaaaaaagcatcaccaaggatcgtaaacaaattaaggagtggtaggaatggtcaaagaagccgtcaaaaatctggaaccgtacgttcctgaactcactttggaacagatgaagaagcaaaaggggctggataagttagtcagaatgtccgccaatgaaaacgcctatggcacctctggtgacgtggccaaggcactggacaagtggcactatcgcgatgccaatctgtatcccgacagtaacgctgatgagctgcgggaaattattgcttcccagtttgatatcaacgccgacaagttgatctttggcaacggcttggatgaaattatcgaattgctgtcgcgggtgattcttgaacccggggatgaagttttggatccggcaccaactttttcagaatatgccctgcatgcagaaattaagggtgccaaaatcaaatcggttgggctggacgactccggccggattgatttaaaagcaatggcccgctcaatttcttccaagaccaaaatgatctggatttgtaatcccaacaatcctaccggaacttttctggaggctgatgccatccgggcatttgtcgaagatgtttccgaagcgatcacggtaattgttgacgaagcctacattgattttaccggcggcatccatgactcggtcatccagttgaccaaggaatttaagaacctggtggttttgcggacattttccaaggcttatggtttagccaatttcagggtgggctttgccgtttgctcagatccattgattggctatctgcaggcagcgaggttaccgtacaacctgagcacctttgctgaaattgcggcaaccgcggcatttaaagaccagtcattcgtcgacaataccgtcaaaaaagtcattgccgaacgcaaaaagtgggaacatttcttaatcaaagccggcttgccgttttatgactcggcaaccaactttattttcttccaagtgaagggtggggatgctgatgcgcttcatgaatatttgttggaaaatggttatttacttcggaacggtttacgcaaggactggctgcgagttaccatcggcagaccggaagacaatcaagccgttcaaaaattgattgccgattatcttgcttaaacatttacttacaaaaagtagcattcatttcgagaatgcgttaatattagttttactggaaattacgaccttcaactcgtggattctccagaatctaattgaaatgatggtggttttatgcaagacaacagtcaaacacgtgttgttgttggaatgagtggtggtgtcgactcctcagtcgtcgcttatctgctcaaacaacaaggatacgatgtgattggcgttttcatgaagaactgggatgatactgatgaaaacggcgtatgtactgcaaccgaagactataaagacgttgctaaagtcgctaacaagatcggcatcccatattattctgtcaactttgaaaaggagtattgggaccgcgtgttcacttacttcttggatgagtataaaaagggcagaacccccgatcctgatgtgatttgtaataaggaaatcaagttcaaagccttcttggattatgctttggaattgggtgccgattacattgcaaccgggcattacgcccaattaacccgtgatgcagacggtcacaatcatctgctgcgggcatccgatggcaacaaggaccagacctacttcttgagccaactttcagctgaccagctggaccgggttatgtttccaattggtaacctggttaagccggatgttcgaaagattgcccgtgaggccggcttggcaactgccgacaagaaagactccgttggtatttgctttatcggcgagaagaacttcaagaacttcttaggtcactatctgccagcaactcccggcaagatgatgaccgttgacggcgaagttaagggccaacacgatggtttgatgtattacaccatcggtcagcgtcgtggacttggaattggtggcgatggtgttgataaccagccatggttcgttgtcggcaaagatttaaagcagaatattttatacgtgggcaagggttatcacaatccattgttgtatgccgattaccttgaggcttcagatattcactgggttaataacttggaccgcggcaaggacttccactgcaccgctaagttccgttatcgtcaaaaagataccggcgtgaccgttcatatcagtgatgacggccagtcggttcgcgttgattttgacgcaccggttcgtgcaattacaccgggacaagccgttgtgttctatgatggcgacgagtgcctcggctctgcgattattgatgcggcttacaagcaggctaaagaattacaatatgtttaatctgaaaaagttgacgattgtcgtcaactttttttgtgggctgattgcgcttgttaggaaatgcaacagtgattcctggataatcgttatcatcagttgttacttttaattgagcttcaaaataaaaacaaatttttcattataaatctcgttaggcttttgaaatcgaaccgttttcctgtcataatgtaagaagataacagcagtttggaggaatgtcatttgactaagttgtactttgttcgccacgggaaaactgaatggaatcttgaaagccgttatcagggtgccggcggcgattctccgctgctggctcagagttatacggaaatggatctgttaggcaaacattttcagaaaaccgattttgcccacatttattccagcccgattaagcgtgctcgggtgacggcggctcgaattgaccgcaaattaaagagccatccggatatttcactcttatccaggttggaagaatttcacttggggaaaatggaaggccaaaagtttgccgatgttgagcaggcttaccccgaagagtttgaggacttccgcaaccatcccgatttgtacgatccaaaggccatcggtggggaaagttacttggatgtgattaaccgcatgacgccggcaatcacttcaattgttaaggcctacccggatcaaaatgtgatgatcgtcagtcacggggctgcgcttaacgctgagatcaatgcgttgctgggtgtgggactgcccaatttacgaaaacgcggcggcctggcaaacaccagcacgacgattttggaaagcacagatgaaggacaatcctatcaactgattgattggaacgacaccagttatttgaacaaaaaattagacccgacagatttggtataggtgacaatatggcaaataattcagataaaattaaaaaattacaagcaaaaaatcaagcaaatcagcgtaaatatactaagaagcgcgaggctgaagaggcgaaagccaaagccacgattcataaactagttgaaaaagtggatcacgaacccgacaattatcacaattactatgatttagcgacgttcctggttgaagctaaagattacgagcaggccgaagagcttttaatgaaggcactcggcttatttgacaagtccaaccaagacgtcaaagataccctgaaatttggtcttggaaatgtctactatgccgcggcggaatacgataaagccatcaaaatcttccaagaaatcgaagacaaaaagcttcaggccgaatcctatattatgctggcccaaagctatatggccaagggtgacaacaagcgggcaatggtctttgctttatcggctcaaagtgcccggcacgatgaccctgacgtcaaccaaatgattggtgacaatctcttggccctgggtaactttgcccaagcgggggacttttacgatatcgtcttgaaaacagagcctgaaaacggcaaagccaactttaatcgcggcctggttgccatggtgaatggcgaagattttgaaaactattttgcaaaagccaagcaggctgatccggcttattttgaaaagggtcaacaaaagttgaaagatattgaaaaagtgatccagatcaacaaagacaagccgaagaagtaaatgtcagcatgagtaaggaggaccgtcttggaccattcaatagatttatttggctcagaacagaataatcacgaaccacaatatgtcgatggccgattaaaggcgatcttcttttcgagtaatgacagtttttataaagtcgtcttagttgaaattacggagaccaatgtcaattggccggaagacgaaatcgtcgtcaccgggaactttggcgatttggttgaagaaaacagctatcatttcaccggcaaattagtcgatcatccccgttatggcaagcaatttcaagccagcaactacaccagtgtgatcgccactaccagagaaggggtcgtcaaatatttatcaggcgatcagttccccggcgttggtaagaagactgccgaacgggtggtggatgttcttggcgatgatgcgattgaaaagattaccgcggataaccgtgtcttggatgacgttcccatcagcgccaaattgcgatcggcaattattgaaaatcttgacgccgatgataacttggaaaagaccattgttggactgaacagctatggtttttcgagtgcgattgcttcggcgatttaccaaaaatatcatgaagatgctttgaaaatcatttctgataatccctaccaattagtcgaagacattgacggcatcagcttcaaaaaagccgacgccattgcccttcgattggggattgtgccggattccaacgaacggattcgtgccggattgatgtatgcgattgatgaattatgccttcaaaatggggacacatataccacaaccgccccattgattcaaactgccacgagccttctggaggggaattcccagcagcagattcctgggaaaaagttggccgagagtttggttgaactggctaaagaaggcaaggttgtcggcgaagaagaccgcatttatttaacccggctatacaacgccgaagtccaaattgccgatcatttgaaccgggtgatcaaaaatcaggatgatgaagatcatctcaaagaagatgcgatcaaaaagcaattgcgagtcgttgagaagcagtttgatattaattatgatgattcccaagttgccgcgattgtccaagccatccagtcaccggcatttattttgaccggtggcccgggaaccgggaaaaccaccattatcaacggcattgtcaacacatttgcccgactacatgagtattcactggatattaattcctataaagacaaaccgtttccaatcgtgttggccgcaccaaccggtcgagccgccaagcacatgactgaatctaccgggttgccagccagcaccattcatcgactgcttggtttgaacggccgtgagtccaacgacaccactggtacgaaggatattgaaggggcactattaatcattgatgagatgtcgatggttgatacttacttgttcaggtcgttagttcgggcaattcccaaccatatgcaggtggttttggttggtgaccaggatcaattaccatcagtgggaccaggccaggtattccacgatttgctggtttctaagcagattccggccatgcagctgaatacaatttaccgccaggagaagggctcatcgattatccaattggctcacgatattcatcgggggcagctgtcggaaaatttcactcagaaccaatccgaccgctcgtttatcccatgtaacgagtaccagatctcttcggtcattgaacaggtcactaaacgtgccaagcaaaaagacttcggcttgatggacgtccaggttctggcaccgatgtatcgcggtcgagccggaattgacaggctaaatgacgtggttcaagaagtctggcagggtgatccaactggtaaaaagtcggttgcgatcagagaacacacttatcgaattggcgacaaagtgctccagctggttaataaccctgaaaataacgtcttcaatggcgacattgggatcattgtggggatggacgcccctaaaggacagcaagttcccaataagattacgattgattttgatgagaccgaagtgacttatgagaagaatgagtggacccaattcaccttggcttactgcacgtcgattcataaagctcagggtagtgaattcaagatggtgattttaccaatcgttcggcagttctcccggatgcttcagcgcaacttactgtatacggccgtgacccgagccagcgactttttgattatgctgggtgaaaaagaggcctttgaacaatgtgtccgcaacgtatcggttaaccggcagaccagtttggtcaaacggctggtagatacaattggcattcagccgcaatcaaaaagcgctgacggagagccggaagctgaggatcaaaagcaattgccgactggcacgccatcagcccaagagactgatgatgctaaggccgataatctgcccgatcatttaaccacagcggttatcaatcaaaatctgattgacccgatgattggcatgggggatgtcactccccgcgatttcttgaagtcataggtttatcagtgaattcttaacaagttcaagccgaaattatggtagaatttaaataaataggtaaagaagaatacttggaggaaatcatggccgaatcaaaaacgcatcccaatcttaaattattttctttgaattccaaccgccacttggctgaggaaattagtaaagcagtcggtgtgccgcttggcaagtcaacagttgaaaagtttagcgatgacgaaattaaaattagcgtcgatgagagtattcgcggtgatgaagtttacatcatccaatccgtttctgatcccgttaattctaatttgatggaattattgattatggtggatgccgttcgtcgggcaagtgccaagtcaatcaacgtggtgattccttattatggctattcacgtgccgatcggaaagcgcgctccagagaaccaattactgccaaattagtcgcttcctttttagagatggatggcgttgatcgcgtggttgcccttgatctgcatgctgaccagatccaaggcttcttcaacattcctgttgaccatttgaaagccgatacgctgttggcagactattttgttaaaacccacaagagttccgatgttgttgtcgtttcaccggaccataccggtgtttcgcgtgcacgaaaattcgctgaacttctgagtgcgccgattgcgattattgacaaccggtcgccggaagatgccaccacggttcccgaatcagttatcgggaacgtgaagggcaaacgggcgattattgtcgacgacatgatcgatacggcatttaaattgacaattgctgccgaaaccttaaaaaaggccggcgcaaccgatgtctttgcgattgcaacccacgctgtcttttcaggggatgcccaacagcggcttcaggattcaccaatcaagaaggttattgtgacagattcaattagtatttccaaagctgaccaatttgaaaaactggaagtggtttccgtgggtcaattatttggtgaagccattaacttgattcataatcacaaatcggttggtaagctgtttggaagataaaatattttacgaggtggtttaatttatgtataaggcaaatgacgatcgttatgaaaacgcagtggtacgcagagctggaaattccgggctccaactgccggcactatcatttggattgtggcatagctttggcgatgacgccaactatggcgacagcgagaaagtcattttgaaggcctttgacttaggaatctttagctttgataatgcttataattacggcccaagtgccggtgctgctgagcggatgttcggtgaagtttaccgtgccaacctcaagccgtaccgcgatgagctggtgattaccactaaagccgggtttaatatgtggcccggaccttatgggaacttctcatcaaagaaaaccttggttaatgcgcttgacggcagtttgaagcggatgggcttggactatgtggatatctattacagccaccggtttgatcccaataccagccttgaagaaactgctgaagccttggatgagatcgttcgttccggaaaggcgctctacattgggatctccaactacaatgccgcccaaaccgctgaaattatcaaatatttcaaggaactccatacaccattcgttgtgaatcaggcatcttataatatgctcaaccgtggtattgaagaagatggtctgctggatacattgagccaaaataataaggcgctggtcgcatacgggccattggctgaaggcctcttgactgacaagtatttaggcggcatggatgataacgttaagattcactggagtaatgaatttgtcatcaaacatggtaaagacgagttggtgaagaaattaaatgagctcaatgacattgccaagaaccggaaccaaaatctggctcagatgtcattagcttggcttttgcacgatccaacggttgtcagcgtggttactggggcctcgaagattaatcatctggaagataacctgaaagcactcaacaatcttgactttacgtccgatgaattagctcagattgataaaatcgttaaagaataattattaggttgttcatacatgtttgaattaagcattaaattgggattaaaccggtttaatgctttttatttggtataatctaatcaaagacatttgtccgtgaatggagaataattatgacaaagaaagtgacaattactgatttagccgctcgtgcccaggtctcagtgacaacggtttcacaaattctcaatggtaaggctgcccgttttagcagtaagaccgttgagaaagttaagcagttgcaaaaggaaatgggctacgttcccgactttaacgcccaaagcttgattcgtaaaagcggtcggacaatcggtgtgatcattcccaacatgaataaccctttctttagcagatttttacttggcattgagactgaggcaattaaacaggactatgtgccccttatttttggctctaacaacagtcagtcacaagagacgcactatctcttcgaatctgttcgaagggccgcagacggcatgataatcgcttcagcggtgtccgacattaattatattgataatatcttgaatcaaaacggcattccctatattttaattgaccaggcaccggtggttaagggtgatcgggttgatgccaataatcaaaagggcggggctttactagccgattatttaatcaagaatggtcatactgatgttgcggttgtctgtgccaccaaaccaaccctcaatcttcaggaacggctggctggatttgtggaagcctacaaaaacaacggcaccccaattcctgaagaccgaattattacgactgagatgaccaaaaaagggggttacgctgctacgaaagcagcgttagccaccaagccaactgcgatttttgggatcaatgacgaggttgccattggggtctatcgtgggcttgaagaagccggcttgaaaattccaagtgacatttcggtggttggatatgatgacattgatttgggagagtacatttcccccaaactcaccaccgttcatcagcctgcttttgaaatgggaaccaacgccgctcaaatgatcatcaagcgaattgaagaccataatgagccaatccaacaggtttccctgccggtatccttggtagaaagagagagtgtccgggcaattaactaactgggatagttgttaaatttcaggaaatttgatagaatttggttaaaggttttaacacactatactaagggatttagaggagcttattatgacaaataaagtggttgtgctcggaagtctaaacgttgatacaacattgcacattgaccaaatgccaaaaccgggggaaacgattagtgccaagagtaaaaccaattccgctggcggtaaaggggccaatcaagcagtcgcagctgcccgttccggtgctcagacgagttttattgggcaagtgggtgatgatagcaacggcatctttatgatcgatgctttgaaacttgacggcattaataccgatcatgtgggtatcaatcaggtcgatgggaccgggtctgcggtcattcttctggacagccagggtcaaaacagcatcatggtttatggtggggctaaccaagccatgaaaaccgaagtcatcgccgacagccaagccctgattaaaagtgccgatattttaatttccgaatttgaaacgccccaggaagtcacctacgaagcgtttaagttggccaaacaacatggtgtgaccacgattttaaatccggcaccggcttcaaaaatcatttacgggttgctcgaagtcaccgatttgattgttcccaacgaaaccgaaagtgccacattgaccggtatcgaagtcaacgatactgattcaatggatcaaaatgccgctaaattcagcgagatgggtatcgataacttgatcattacggtgggcgatcgcggcgcgtactatcatactccaagcaacagtggctttgtgccggcattcaaagttaaggcaaaagacaccacggcagctggcgacacatttatcggggctttcagttcacaaattaaccaagatttatccaatattgaagcagctttggtttatgctcaaaaggcttcatccattacagttcaacgtttaggggccttaccttccattcccacggccgaagaaatcaaagcggaatacaaataaaaattatcttaagtattagtttaatttttcttccaaactgttttgcgagtagggtgttgctttctcgaattttatctggtagtatatccagacgttagcaggaaatgttaaaaaattgataacattcccacgttagaaatcaggattgacgattcgaaattcaaatttcatgttcaaaggagtttatagctatgagtaataagttagaaattctgagagaataccaaaaggcatcctcgaagcttgatcaattaaagtccgaagaagcagacaagatcaagtctaccccagtgaatacgagttctaccgaagtaatcacaccacagtttggaaacgaaatgacgcatttgaatgaagaatgcatgcagttaaacatgatcttagaagcaatggatgcttcggaagactaggtcgtgtggacgcgggatcgtctatcgacggtgccgtttttttgttacaatcaagtgcccaactggtccacagaaagccaaaacagggcagataacggtgaatgcactcatcgttatctgccttgttttggctttcagtttttattttttgaattttaatgggcaacagccacccgacttcagaaattgtccgatagtaacgccactgacaccgcacttttaatctgatttcttccctggagctttgacagccagttttcagggaacgtcaccggcgcaaagagcagtgatgccagcatggaagtaattgaaccgatagtatcggcgttactgccaagattgacagcctttgacacggcaacgttatattgttccgaattcatcaggcaccagaaaacggcgttgagggtggcgatcacatcgccggagggccttagcttcgtactcgactgtcggaggaagtgaggctcctctaattgctcaaaaaacggcacctgagcggcgaattgatcttttgagcggtaatagtccagggcttccttaacggcccttagcatggcgtatttgttgggattttgaatcaggcggataatgacgttggttaaaaccccggaaccaataaatgtcttgggggttcggttggtggtagccgtgtaatcatgaaccatgtcggcaatggtttcattaaaggtgtactgctggttcttcgttaaaatataaaaggccaacggcatcaaccgtttaagggcagtattgtcattgtctgaatccaaagtgccgccggacaaaaccggtggggtgccggtatcaaagcgttggatggctgctttggtggtctcatcaacgtcgtatgcataattaaagggcgtgtaatcaccaaaatggacccattgcgaataacgtgtcatgaggtcataaagattatatccaaacgttaagctaactaaagaagcaattgatagtgatgtatcatcagaccaagtgccggctgggatttgattcgtccggtgttcgaccatctcatggattggatcatcgaaggggttcaggcgggtatcgtgttgaatcggatatccaagcgcgtcacccagggcaactgctgttaatgattgaaataaaaggtagctggtggaatacatagaattacctcgtcgttagtttttcgcggtacagaaacttaccgaatccagaagggatatttaaccgtgtcgagcttcaggttaaaagtccgttcgccaagttcttcgccatcgatttgacccaaacgattaccatttgtttttataaacagctctttttcatgataatgatgaataaatttaagccgtaagtgtctctttaaaaatatcatagatacaaataaaatcaattgccaaaggctggttttttcgaccactactaaatccagatggtcgtcgaacactgatgcgctgggcacgatgttgatgcctccgccgaaataaggaatatctgttgtggttaataaaaatgtgttatcgaatgtgactttaggcatatttcccgggagaatttcggtcttgaaccctttaaagtggatgatcacgtttaatatagccgccatgtatgaaaattgtccgaagaattggtgactttttaaagaagaatgatttgcgaggtgcacaacagtggcgtcaaagccgatgccaaaattgttggtgaagaagccttcggaatgatgatcaaggtctgtgtagtggccgacattgatggttttagcagctgattgggtcaaaatgtcagccaatgctttctcccagtgcaaaggaatctttaatccccgcgcaaaatcatttccggaaccgaccggcaaaaaggcaattggaactggatgatcattttgatgggtgcggtaatagtgctggcagcccaacagtgtttcgtgaagggtcccgtcgccgccagcggcaatcaacacagcgtcagtttggttggcggtgtcaatttcactgagagcttgttcagcaagttcaacagcatgatttgggtaggcggtatagagtgtctgataatcggcatgtgcagccgccagttgtttttggatatccggccaaacctttttggcgttagcaccaccggcatgcaaattgataatgatgaaatatttcattggtgaatgagcccccaactcagatggttttatgtaaaaaacttgagaatcgaatataaaatctatccgcttctcaagttttcgaattagtcacgttcagttttgttaatctttaccattcatgatgagcattggcaaaatcattggatggcgttcggtcttgtcgtaaaggaattcttgaagatcatcaataatcgcatttctaattgaagactcggttgcttttttagcacgcatcgactttcgaatggtcttaaatacacggcgtcggccttcatccaaaagttcaccggattctcgcatgtagacgaagccacgtgacaagatatctggaccggattggatttcctggttggccaagttgattgttgcaacaaccacgacaataccttcctcagaaagcagttgacgatcgcgcaagacaacgttgccaacatcaccgatgccgctaccatcgatgtaaacatctccggcagtgaagtgaccagccatacgagcattatcttttgaaagggcaagtacatcaccattttgcatgataaagctgtgatcaagcggcacgccacattgttcggcaagctcagtatgaattttcagcattctgtactcaccatgaatcggcatgaagaacttcggcttcatcaagcgcagcatcaatttctgttcttcttgaccaccatgtccggaagtatgaatgttgttcacccgaccgtgaatgacattggcgccggcttcttcaagcttgttgatgacgctgttgacactggtcgtgttaccaggaatggggttacttgaaaagataaccgtgtcaccaggctgaattgaaatctggcggtgggtaccgttggcaatccgtgaaagggcagccattggttcaccttgagagccggtacacaagatcaaagtcttgttagctggcagtgactgcagctcgtgtgcatcaacaaacgcatcatcaggaatatcgagataacctaattcgcgtccattcactatcgctgcatccatgctgcgcccaaagacggcaatcttgcgaccgtgggccatggcattatcacaagcggttttaatccgtgaaatgttggaagcgaaggttgcaaagatgattctgtcttcaatattatcaaaaatgtgggcaattgaagttccaacccacttttcagatttggtccaaattggcttttcagcgttggtgctgtcagacatcaaacaaaggacgccttctgcacccaaacgggccatttcctgaagatcaggcggctggttggtcactggtgtgaggtcgaacttgtaatcaccagtttccacaatcacgcccaccggtgtatgaacggcaattccaaccgtatcagggatcgagtgggtggttctgaagaatgaaactttcatttttcggaacttgagaaccgacttgtcactaatttcgtgtaattctacagaatttagcaagccgtgttcttccaatttattcttaatcagcgccatcgcaagtggtccggcataaatagggacgtttaaaaccttcatcaaatacgggacaccaccaatatgatcttcatgaccatgggtgatgaccaaagctttgatcttatccttattttcaaccagatactgatagtctgggataacataatcgacacctaagagatcatcttcggggaacttaattcccgcatcaatcaggataatttcatcctgaaactggatcccgtaagtgttcttaccgatttcacccaaaccaccaacgccatagatagctgcttcgttattcttgacgtttagttttttcatttattattaaactccgttactttgtaatcaggactactttgctcatactccaagtgctttccttggaggggttcgatgaattcaatatcataatcagtattgtcttcaactaacgcgtgagcttcaacctctgtgtcggcctcaacatagagtgaatgagtcgtttcccggcgagggctttccttcttgctgggttgatataaaaccttccaaatcataaaaaaaactcctttaaaattatacaatttttttgcagaaactcgaggtttccttacggacaagtggttgtgaaaacacaactaataacgatattctaccataatctaaaaaataagtatataaacatgaaagtaatcaactcgcaccattgcatggtaaaattaaatcaatgaaaagaaatggggctcagttatgaacattgatttgattattcaaattatcatcgggttggtcgcagcatttgctgtttacaatttgattcattatatctttgtaacgagacccggcagaaaacggctggcgttggcacagcggattgccaatgaagccgtgaaaacttcgattaaccagctggttgaacaaaaggcagttttgccctttgatgaaagtgattttaaatctgaagatattgccgaagtgtggggcagaggtgtgatggcgtttgaatatcatctgcccaaggcaaaaattgaaagttcaattcccgatttccgaaaggccttggcaacgacgcttgagcaatacggtgatacacaccacatgcacgcgcataccgatcaggctgatcggccggcgtttatggtcaccgatgtctggcagctggatgatcgggtgcactttgatgttgcctacctggtgaacgtgacgacgattgaatatgtggatgacttaaagcggctgcactgaaccattatggactagtcaacggcgtttgcttttcgatactgtttggccagtcgcttgcgtactttgatgattgcaagcagattatgatccactgtcggggaatagagattttcaacagcgaccagcttggcaatcagtgccaggccttttttctcactgccaaaatagagctgccagaccgcggtgatcaattgttgttggaaccggccattccaacttaaatccagggtgttgacctgacggattttgtttagaatttcttttgcggattgatactgagccaagttgagctcgatttgaaaaagagaaagataaagatccattaattcatcagcaatatgaaatgggtcatccactgcttgaaggtattgtcgacagttgttttcaaatctgtcaacaatctcggaaataagcgcttcttgatgccggctgaccgcaattggcagtaaaatttgggcctgcctaatttcttcaagtgtccaggtctgtgatgcaaaaagggtgtcccagagattttccattgccggagtgactgtgaatgtttttgaataataagtgacgaccaatatttgacccatagcagcaaccgatttgtaactgaggcggctgcttttttgcgtttcagcgatgatttggcccattgtttgaaggtcgtggccgttataggcccgtagcaggcgccttttcagggatgttgcagtgggttcgtgataatcgttttggataaaacggaattcgttggctgaaatggacagattatctaaaattttaaataacttggcggcactgatgtcgttctccccattttcaaagcgatgagcaaatgaacgtgacatcacgcctgagtacacttcgctttgggtgaatcctttaatttgtcgaatcattttgactgtctgcccgattgttttcatgattgcctcccaagctttgaatgtggcatatatgcaacgcattttacatctatcgctttaataatggtagtaggcttcagttaatcaaaattaaagcgggtgctgacaatggaaattagtgatcatgagtcaaatatgcaggttataaaagatgtatcgagcaacttcaccagtactttttgtggtgacatgttttcatttgctctggggctcatgctgctgcgggcgacgggaatgtcgttaagctttggactctcaatgattatcatgccgattgtgactttgatcgggttggtgccgattggcaacttggtcgacacttatccccacaaacggctcttgattattagtctggtcgtccggatcggcgcactattgatttattcgatcgcaattggtcacttcgatggcagtggtaaattaatcccaacgattgggtttttgatcatcaattacgcatctgtcaatctttcaaattccggctacatggcgtcggttcacgaattagtcaacgagggtcatattcaaaaattgaattctttgagccaatctgcggcatcgtttgcctcgaccttttcgccgattgtggctgccggattgtatgtgatagttggctttaggctgtttatcgtctttcagctgactgctcacgtgattgccttggtaattcttttgacgatgaattttcattatttgagctatccaaggaaaagcagtcagacaccgcaggaatcccagtgggcaaaattcaaactggggttaaattatttgatggcccacgactttttacggtatctcatctgtattgccctgtttttgaattttatttttgcggtcattaacgttggcctgccatttatgattgtggaacatttacatttgggaaacgtgacgctggggattttgaattccgccgacgcccttggcatgctgatcgggaatttgatcatcagtgtctcgaaagaattgaggcacttggcaaaaatattagctgtcacgatggtcatcattggtacggggttggctggagttggcgctttattgatggctgctcccgaacaattagtggtccaattggtgggctcgttgatgttgtttgcagtggggatgtcactggcttttatgaacacgccttttggtatttacatgcaaaaaacggttccgactgaactgatgggcagagtctcgtctaccgaaatgtctttgaatatgatgtcaattcctttggaaaccgtcttttattcatttgtcttccaacagattccaagcggaattgtgttcatcatatctgggatggctctgattgccgtcaccggattgacaatgccagcttttatgcacgtccagatgccaaggactgatcatgccacccaaaaggctgatcgtcagcgtctctaagttgagtttgtcgggtaatatgtctataagtaaaacggtttgttacaaattcaatgaaaaagaaccagtaacttacaaaaagttcatttgatatttgttcacaaggcataaccaaacagatctaattcaggaaaggccactcgccacaattaaattggataagaaaaaaaccgggcaaaagtttttccttttgctcgattttttaatatggatgcttattgaaatttcttagatcggcatatgaacaactgatttagtgcaccgatcaatacacaaagatttcgtcatctgttttggcaaatgggttgtccttattaatgtgatcataaaagagtgttccatgaaggtgatcgatttcatgctggcagacaattgccgggtaatttttcaatcgaaccttgtgctctttgccgtcaacgtcttggtattttaaggtaattctggcagcccgagggacatagccgggaatgtccttatcaacggacaggcagccttcgccctctgtcaatgcgccacgctgaaccgaattcgacacgatcaccgggttaataatgacatctttgaaaaccggttcatctttttcatcctcgtcttcacttggaaccaacactgaggccatcatttcagagacaccgacctgtggggcagccaagccgacgcctgcacgcagacctaacttttcacactgttccggatcctggctgacttccagatattccatcagatcatgagccagttgtttatcttctttgctcaaagggaatttgaccttttgagcttgtttacggagaaccgggtctccatctcgtacaatatccttcattaaaaacacgctaaagacctccgaaaatattttaagcattaattgaataacttctattctaacttaattttaagaaaaaaacactattcacaaagtgggtgaaatttcacaaagtatactcccgcaagcggtttcaacccaaaatttgtcaagtgaaaattatattcaaaaaagttggtttcatcacaatgaaagggcttgcaaacgttgctgaaaaatgctaaatttaacttgtggtttagaagtgatcagtttgtacatcacaagtctagctttacaggaaaggaaagtgttatctatggcagcaaagagtaagcatgttgttgattttgccaagatcaaatcaacgatgagcgatccatataagaaaccggttcaagttattgatgaaaacggtaaaatagttaatcaagaattatttgaccaattcagcgatgacgaactagttacgctgatggaaaagatggtttgggaacgtgcattgcatgaacaaacaatgaacttttcacgtcagggtcgattaggtttctatgctcctacttacggtgaggaagcctcagaaatggggattgcccacgcaatgaagaaacaagactacctattcccagcatatcgtgatttaccacaattaatccaacacggtgcaaccgttaaagagggttacttatggtcaaaaggtcactaccaagcttatgactacgtacgacgcggtgtacgtgcatttatcccacaaattattattggtgctcagtatgttcaatcagctggtgctgcattaggaatcaagaagaacggtgagaaggataccgttgcttacacatttaccggtgatggtggtacttcacagggtgacttctatgaaggaatcaacttcgccagttcattccaagctccagaagtattcttcgttcaaaacaacggctgggcaatttcagttccacgaaagactcagaccgctgctgaaacccttgcacaaaaaggtgttgcttccggtgttcctggtgttcaagttgatgggatggatattctggcaacttacttggttgcaaaagaagctcgtgactttgttgttgccggcaatggtccagcattagttgaaaccttgacttatcgtttcggtgcccacagttcagccggtgatgatcctagtcgttaccgtactaaggaacaagaaaaaccatggttcgaccgagacccactaattcgtttgagaaaagttttgactgacaagaaactttgggatcaagacaaagaagacaaattagttgctcaatacaaagatgaattcaaggaagcaatgaaggatgccgaagctgctcctaagcaaaaggttagtgacttcttgaagaacacatttgaagttccaaccccagatgtagcagctgacattaagaaatacgaagcaaaggagtcgaagtaatcatggctaaaatgacatatattaaagcaattaccaacggacttgaccaagtattacaagacgatcccaagactctgatttttggtgaagatgttggtaaaaacggtggtgtgttccggacaactgaaggacttcaagataaatatggtgaagaccgagtattcgataccccacttgctgaatcaggaattttaggaatgtcaatcggacttgcattaaccggttggcgtccaatcccagaaattcaatttatgggattcacaatggaagctgttgattctgtcggtggtcaaatgtcacgtaaccgattccgtttctcgggcgacgttacgatgccgatcacaatcagaactccatttggtggtggtactcatactgccgaacttcacggtgactcacttgaaaacttgttcattggcatcccgggactgcgggtagtaactcctgcaaatccttatgacgctaaaggaatggttatctcagccgttgaaaacaacgacccggtattattcatggaaaacctgaaactttatcgttcaatgaaggatgaagttccagatggccactacactgttccgctagacaaggcaaatgttgttcgtgaaggatctgacattaccgttgttgcttacagtgccgaagttaacgaagcacttaaagtagcagataaattagaaaaagagaacatctcagttgaagttattgacttacgttcattatcaccaattgacgatgaaacaatctttgcttcaatcgacaagactcacaaagtagtgattgcccaagaagcacaaaagatggctggtgccggagcaaaagttgcttcagacattgctgaaaacgacattatgtcattggacgcaccaatcggccgtgtttctgctcctgacagtatcttcccatttgctatggctgaaaatgattggcttccaaatgctgatgatatcgaagctaaagtacgagaaattttgaactactaaaattctaatttgttacagaaaggaagttagatcccatggcttataagtttaaactaccagagatgggagaaggaattactgaaggtgaaatcgctacctgggatgtaaaagttggcgataccgtcaaggaagacgatccgttagttgaaattcaaaacgataagtctgtccaagaaatgccatctccagttgccggaaccattaagagtattgaaaagcaggaaggagaaaccgcagaaaagggcgacgttttagttgtcattgatgatggttctcctgatgaacctgatgatgccgcaccagcagctgcacctgcaaaagaagaagctgctccagctcctgctaaagaagaagcacctgcaccggctgccgcaccagcacctgccgctgctccagccgcagtaactgctgcaccagctgcttcaaatccaaacgcaattgtcaaagcgatgccatctgttcgtcaatatgcacgtgacacaggcgttgacattactgctgttcctgccacaggaaatcatggtcagatcaccaaagctgacattgacaacttcaatccagctgccgctccagccgcaccagctgccgctgcaaccgctgctgcaccagctggcgaagcaaaagctgccgcaggtcaagctatcaaaccttggaagtctgatcaacctgatcttgaaacccgtgaaccaatgtctccaatgcgtaagatcattgctaagtcaatgcgtacatctaaggacattgcgcctcacgtaacttcatttgacgacgttgaagttagtgcattaatggctaaccgtaagaagtacaagcaagcagctgccgaccaagatattcatttgacattcttaccttacattgtgaaggcattggttgccgttatgaagaaatatcctgagttcaacgcttcaatcgatgacaccactcaagaaatcgtttacaagcattacttcaatgtcggtattgcaaccaacacggaccacggtctgtacgtaccaaacatcaaaaatgctgattccaagggtatgtttgagattgctaaagaaattaccgagaacacccaagctgcctatgacaataagcttggcccagatacaatgaagggtggttcaattaccatcagtaatgttggttcaattggcggtggctggttcacaccagttatcaaccaacctgaagttgctatcttaggtgttggtaagattgccaaggaaccatatgttgatccagaagacggcgagattaaagtaggcaatatgctgaaactttcattgagctacgatcacagattaattgatggtgcccttgcacaaaatgctttgaattacatgaatcaattgcttcatgatccagcaatgctgttgatggaaggatgatcgaataatggctgatgttgaaaagaaagaaacagtaattatcggagctggccctggtggctacgttgccgcaatccgtgcatccgaattaggacaaaaagtaaccctgattgaaaaatcagatacacttggcggtgtttgtttaaacgttggttgtgttccttccaaagctttgatcgctgctgggcatcgtctgcaggaagctaacgatgcttcgacgtatggaattacaactcaaccagctacaatcgattttgcgaaaacccaagagtggaagcaaaagaaggttgtcgaccgaatgaccagtggtgttaagatgcttcttaacaagcacaaagttgaaatcattcatggagaagctgttcttgacagtgatactcaattacgagtaatgcctacaggaccacaacaattcatgagtgccgataccggaaccacgattcagtttgacaacttaatcattgccagtggatcacatccaattgaaatccctggtttcaagtttgacggtcgggtgattgactcgactggcggcttgaacctgccagaaattccaaaagaatttgtcgttatcggtggtggctatgttggaaccgaattagccggtgcatacgctaacttaggtgcccatgtaacaatcattgaaggattggattccatcttgaatggatttaccaaagacatggtttcattagttgttaagaacttgaagaagaagggcgttgatattcataccagtgccaaagcaatttcttcaagtcaagatgacaacagcgtgtctgttacctacgaagaagatggcaagcagaccactatcaaagctgattactgcatggtcactgttggtcgtcgtcctaacaccgatgatcttggcttggaatacaccaaggttaagttggacgatcacggcattgtccaaactgatatccaaggcagaaccgattctgagcatatcttcgcaattggtgatattgcttcaggtcctgcattggctcataaagcattcttccaaggcaaagttgctgccggtgcaatttccggtaagaatactgccaacgattatgttggcgttccagcagtctgcttctcagatccagaaatcgccgttgttggtatgactcaagcccaagccaaggataagaacattgaagtttccacttcgaagttcccattcgcaggtaatgcgcgtgccgtatcacttgatgaagccgacggatttgtccgtttgatcttcaccaaagacgataagacgatcgtgggtggcgaaattgttggaccaggtgccagtgatttggttgctgaattaagtttagcagttaacagtcacatgaatgttgaggatattgccctgaccattcatccacacccaaccttgagcgaaccagttcaagaagctgcggatgttggattaggattcccaactcatatttaaaaagttctgttttaattaatccggttaattccggaataaaggattcaatgatgaatgaagcttgttcatcgttggatccttttgtttatccagaattacgatctgttaagtcctccgagaaatgaaaaactcacataacttcgaccttttctatttcacaaagtcttcaactatcatataataaagtcaacttggtaatgatcggagtgaagaagatggccgaggggtatgagtacccactaattgatggtttggatgttgatgaaattattgacgttgttaatttttttgaggcaattgaaaaggcgtatgaggaagctgaaggcattaaacgagcagactttatcaaagcttatcggaaattccaagaggtggtccctgccaaaatggaacagaaacaattggagaaggaatttgccaatcgttccggatatgattcctacgaagtcatcaagctttccaaggatgggcaggcagctaatttgaaggtacgtgaggcataggatggaaattaacgaactcaaacaaattgataaaacggttaaaggttggctgcatgagtcacgggacaacgttctaagaaaaattgacacccgactggaagttgatactaagaccagtcgacgtgatttggtgaccaacattgataaacaaaatgaaaagtttttagtcggtaaaatccgtgaatttgactccaacgccaagattttgggtgaagagggatttggcgaccaggttcattcaacagaaggacggatctggattgtggacccaattgacgggacgatgaactttgtcaagcagcggaatcattttgctatcatgattgccctttatgaggacggcaaaggcctccttggctatgtaatggacgtcattggtaagcatttgttgtctggcggaccggatatcggcgtatttgacaacggccacccgctgccgccggtcaaggacacaccgcttcgagaagggttaattggcctaagtgggccgatggttcttcacaacgattacaatatggtagacattgcccaacagtctttgggaatgcgcatttatggcagtgctggaattgatattatttccgttctccgtggtgaattggttggatacatttcttatctcaagccctgggattttggggcaggcagaattctgtgcgaaactgccggacttaagatgacaactattgacggacagcgattagatgtgttatcatcaacaccagtattgttagcaacacgaaatgcacatcaagacattcttacaattgtaagtcaatgatcggactgtgacagttgtcacagtttttttatgcgaataatatgatgtacaatattcggtttgatttaaatgaagggaagcaaacgacttggatactaaattaaaaacacgcgacgacattcgtaacattgctattattgcccacgttgaccacggtaagacgactctggttaacgaaatgttgaagcagtcagatacgcttgatcaacacgtacaaattgaggatcgggctcttgactcgaatgcgatcgaacgtgaacggggaatcaccattctgtcaaagaacacggccgttcgatatggcgacaaacaaatcaacatcctggataccccaggacatgcggacttcggtggtgaagttgagcggatcatgcgaatggttgacggctgtttacttgtcgttgatgctttcgaaggcactatgcctcagactcgtttcgttttgaagaaagctcttgaacaacacttaaccccaatcgttgtgattaacaaggttgaccgtgaaggtgcccgtcctcaagaagttgtggatgaagttcttgacttgttcatcgaacttggtgccgacgaggaacagcttgattttccagttgtctatgcgtcagctatgaacggaacttccagttatgatcctgatatcagcaaacaggaacatactatgaagccaatctttgacaccattgttaaagacattccagcaccaattgacaattcagatgaacccctccaattccaagttgcaatgcttgactataatgacttcgttggtcgaatcggtattggccgaatcttccgcggtacaatcaaggttggtgacagtgttactgttatgaaacttgatggttccaagcagaacttccgagttaccaaattaatgggattcttcggtttgaagaaggaagatatccagtccgctaaagccggtgatttgattgccgtttccggaatggaagacatcaacgttggtgaaacggtggttgatcctaaagatccagagccactaccaattcttagaattgatgccccaacactgcaaatgacctttggtaccaacacttcaccatttgccggccaagacggtaaattcgtgaccgcccgtcaattgggtgatcgtttgaagcgtgaacttcacaccgatgtttcattacgtgttgaagataccgaccaacccgggtcatggattgtttccggtcgtggtgagctgcatttgtcaattttagttgaaacccttcgtcgcgaaggctttgaattgcaagcttcacgtccagaagttatctaccgagaaattgacggcacaatgtgcgaaccatttgaatccgttcaaatcgatactccggatgaatataccggttcgattattgataccctttcacaacgtaaaggtaccatgcagaacatggaaacaaccgacaatggtcagactcgtttgacattcttggcaccatcacgtggtttgatcggttattcaactgaattcctgtcattaacccgtggatatggtatcttgaaccatactttcgagaaatacatgccagttatcaagggctggaaccctggccgtaccaagggaaccttggtttcaatgaacgccggcaaagcaacgacctatgcaatgatgggtatcgaaagccgtggaacattgttaatcgatccaggtaccgaagtctacgaaggaatgatcgttggtgaaaacaaccgtgagaatgatatcactgttaacatcaccaaaggtaagaacctgaccaacgttcgtgctgccggttcagatgatatggcccggattaagacaccaactcatctttcactcgaagaatcacttgaattcttgaatgaagatgaattgtgtgaagtaaccccacacttcatccgtttgagaaagaaaattttgaattcaaacacccgtgaaaaagaagctaaaaagaagcgtcataactaaaatcagtaaatcatcaggaggggttgggacaaaactaaaaattttgttccagcctctatttgcgcctgaatattatctagcaaaactgtgcgccaataagcagcttccggccatataaggggattacccaaacatccaagttctggatgttcgggtaatccccttatattctggaagctaaccgcttattgtcccacgctcttttgtattgaatggagtttgttgtaacttcttaaattcccctaaaccgtttagcaatctctgaatccggttttttaattatgatataataaagctcgatgcacctacatataatttgaaaagtggagttggaccaatggggaaagcacgtttaaaaaatctcgactatgttatttttattccgtatattgtgatgtcgattatcggtgttgtgatggtctattctgccagcgcaaatatttcgctgcagaacggggggagtccgctgagttacctgatcaagcagttattctttgtcgtccttagtgttattattgttggcgtgatgacggcaatgaacattaagtacttacgcaaacccaaatttttgaaattcttactgtatgctctgattgttgttttgattggtctgctgttagttggcaaaaccatcaatggcgcagctgggtggattcacttagggccaattaacatccagccggccgagttcgtgaagttctttttgatcatttggcttgccgacacaattgataaggctcaaccagagatcacgctgtcttttcgggactggtggaatcacatgaaatggccgttgttctttaccgccgttttgattgcgttgattctcaagcagcctgattcaggtggtgctgccattaatttggcaattgcctttattctgtttaactgtagtggcttttcatggaaacgagctttggcaatcatttatggttgtatggtggctgccgtgctggcatttgaatttattctggtaccaatggccaaatcggattcgttctcccattcctatcaactgcaacgaattgtcgcgtttaccaatccttttggtcacgcgcaggggacaggtcaacaggtggttaactcctattacgctataagtaacggcggccttttcggtgtcggcctcggaaatagtgttcaaaaaaccgggtatctgcctgagcccaacaccgattttattatgtcgattttaaccgaagagctgggggcgattacggctgtcattgtgttggcattattgacagtgatcattttgcgaacagtccaaattggtgttcgcagtaacgatacttatcaaagcctggtttgctacggcgttgcaacttatatgagtattcaaacattctttaacatgggtggtgttttgggggtcctgccaattactggtgtgaccttcccgtttatcagttatggcggttcaagtattttgaccctttcgttttgtttgggactggtactgaatatcagtagtcgtcagcggatggaacgaaaagcacttatcgctgccagaaattaaatttgaggagatggcataatggctttaactgttcaacccacgaccgggttaatcgtttatttacattcgattcgtcattccagaaatctgaagtcatatggccgactgtattacgtctccaaacggatgcgctatggtttgatctatgtgaacaaagatgatgaggaagagattactaaaaaattggcttctcaaagttgggttaagcaggtggtcccttcacatttgaatgaattggtccaagaagttgaaggtaaaaccgagttggacgatgacgattcggttgacgaagattattagagttgaggtaaactatgaggattgtatcaggaaaatacggtggcatccgcttaaacccggtgaagagcgatcaaactcggccgaccactgataaggtgaaagaatcattattcagtatgaccgggccctattatcatggtggtcggttcttggatctgtttgcgggttcgggagcagttggcatcgaggctgtttccagagggatggatagtgctgtgcttgttgatcgacagtatcaagcgatcaaaacaatcaaagacaacattgccaaaattcacgctgaagatcagtttaccgtgattaaaggtaacgccgagatggttttaaaacaattagctgccaatggggatcggttcgaccaggtttttctggatccaccctataagcttcaaaagatcgtgaccactttggaagaattgaaaagcctcgatctattgactgaaggggcgacggtaatttgtgaaactgataaccacactgaattgccgctcaatctcgatggatttcacgcagccaagcaaaaaaattatggactcacaaatttgacgatttatgactatcaaatggggaatgcgcaatgacaaaagctttatatgcaggtagttttgacccgatcaccttcggtcacattgatgtcatcaaacgggccagccgaatttttgacaaggtgtacgttgctatcagtattaacacccacaaacatgctttgttcaccgatgaggagcgggctgagtttgcccgccaggcattaaatcagttacccaatgtcgacgttgtggtctctgaagagctgaccgtccagcttgcccattccttgggcgcaacggtcttagtcagaggcgttcgcggcggcagtgacctggattccgagatgtcaatcgcggggcttaacgagaagttggccgacgatattcaaaccatttttatcccaaccgcggccaactatcgcgacctctcatcgagtatgatcaaagagatcgctaagttccatggcgatgtatcaaaatttgttccaggacctgttgcacaggcattgaatgacaagtatcaacaataaaatagcttttagagagtggtgaactaatgaaaaagtgggttaaaaaatatttaatttggtttgccattttactttttgtggcgatcggctttttgtggccgcttcccaaatacattgagggacctggtgacgccgctaatctgagtaaaattgtgaacatccaaggtcatcccgaccgacagaaaggtcagtttatgctgatgtctgtcagcatctctcaagcccgaccatttacttatctttatgccaagctcagcccatattattcgattgagccggaagaagacgtgaccggtggccaagatatgaaggagtatagtaaggtccaacaaatatacatggacggatcgatcaatagcgccatttacacagcctatcatcaagcccataaagccgttaagattaagtattccggcatttatgtcatgagtttgatgaaaaattccaactttaaaaataagctgaaggtcggcgacgtggtggttgctttggatgggcatcattttaagagttccttgggcttcatcaagtatgttaagcagcaaaaatatggtcagaaactgacggtcacctataaacgtcacggcaaattgcatcaagccacggcgccacttggcatgattgccaagcatcgggcaggtattggcatcactttgaccgatgatgttcaagtgaagcctaagattccaattaaggttcaccctggtcaagttggcgggccttccggtggtctcatgtttgccctccagatttatagtcagttgaccaacaagaatctgcgtcacggtcaaaaagttgctggaactggaacggtcgatgggttgggcaacgttggcgaaatcggtggaattgataaaaaagtcatcactgctaaaaagcatgatgcgaaaattttccttgcaccatatgtgaagccaaccaaaacaattttgaagtatgaggaaggccaccagacgaattatcaactggcaaaagcaacggcgaaaaaatatgccccatcaatgaaagtgattcccgttaagacgtttgcccaagcggtctcaattttagaaaaaaatcaataagcaaaatcaaaaagggttagataatctaatcctttttttcgtatgtattttttagaagggaggcacagtatggataggatacgtgagtttattgatgaatatctttatcagatactaattggtttagtagcagtcattgttgtttttatgtttgtaattggtgggctgttgattggtaaaggcggtgaaactgcaagttccgaggaaccggttgctgtccaaagttccagtgcaagttcagatacgggatcggccgcgagttcatcgcctggtgatcaacccaagcaagttgctgcaggcactaatcaacaaatgtatgttgacgttaaaggggcagtgaagaatcccggtgtttatcaggtcagcagcaatatgcgggtagtcgatgccattgaattggctggtggttacaatcggtctgcggacaagaagaaaatcaatttggcccagaaactgaccgatcaacaagtcatttatgtaccgattcgtggtgagaaggggacaccggtcacgtcaacggttgcggccagccccacgccatctgagactccagcagattccgggtcggacaactcagcgccatcggcggacggaacttcaggaacgtctcaacagatcaatttgaatacggctgataagtccaagctccaagagctaaccggaattggggacaaaaaagccgatcagatcattgcttatcgccaagcacacggccaattcaaaaacattgaggagcttaaggaagtccctgggtttggtgataagacctttgccaatctgaaggcatcaatttgcgtctagcccaaaaagcgtttttgagatatgatttacaccagagaaggtggaatgataatggataagcgaattaaatgggaccaatattttatgatgcaggcggttttactggcctcacggagcacgtgcgaaagattgtcagtcggagcagtcattgtcagggacaaacggattatcgccggtggctacaacggatccgtcgcgggggatgatcactgcattgacgttggctgttacctggaagacggtcattgcgtgagaaccatccatgcggagatgaacgccattctgcagtgcgccaagttcggtgaaagcactgacaatgctgaaatctacgtgacggattttccgtgtcttcagtgcaccaagatgctacttcaggctggaatcaccaaaatcaattacctcagaaattaccataataatgattacgcccaaaaactgattaggttgaaaaatattgaattgaacaaaattaagttaactcaagccgatatggatagagtgccattcggatcctatttgtctgactagttatcaataaaaactggctcatttttccggcactcgtcatgcttttgatgagcatggccatgtacgggaaccggctgattgcggcagctttattaagcattctgattatgcgaatttattttctgcgggacgttaaggttgttagtacatgtatccttgctggcctgatctttgcctttggtgggcttttgaccaatcgacaggtctctgcaccagtcgcacagcaaaattatgtggttaaagtctatccagataccgccaaagtgaacggggcaaatttgagctttattgcccgtcctgagggtgcaaagcaaaagatggtgttctatgccagattgaagtccagtagtcaacaacgtcgtttagcagccggtattaacccaatgatgcttaaggtgagtgggaaaacagccccttttttgccggcaaccaacctgaatcaatttgatatggaaaaatattatcatcaccaaaagattcaaagttgctttttggtcgaccatttcgttcttctgccgccaccagctaaactgtcaattgtcgatcgaattcatattattcgttcgaaattcaaccagtattgcagtcagctgcccaaaactctggggatctatgccaccggattgattagtgggtatcggccggtgaacttcttcgatgaaatgacgggggttaagaagctggggttgctgcatgtctttagtatttcagggatgcatgtggcctattttctttcgattgtcgaccagctgctggcttggctggggttgtcgaggtttaaaaaatcaatcatctcaatcacctttttaggcgcctattttgtcttctctggcggatcccccggattgctgagggcagtgatgatggccatcattggcattcttaatcggttgtttaaattcggtctttcccaactggacatttggagcgggtcattaatcattaacctgcttcttttacccgaggcgatgtttttaatgggggttcaactcagttatggattgtctttggggttaattgcctctgagaagctttcatacattaagcaaacgattttgctcaattttttaaccgtgccgattttgttatttcatctttacgagtggcatttcttaagtgttgccgttaatctgattgtcttgccgctgttcggccgggtcatctttccgctggttatcattggcgtcattgtcggactggttgcggaaacgttggttctgccgatcgacatgtttttgcacatctttaatgatgggttaaatgcagtgagccgtttgccggggatgttgacctttggtaaaccggcattgccgattgtcctaatcatgttggcggtgacaatgctattggccgttgttgatcgtgttcgggcacccaaattgattggcatcttggcagctgtttatctggtgacgtattgttggatccattttccgctcaatggtgaggtgaccatgtttgacattggccaaggggacagcttcttgattcgggagccctttaaccgttctgtaaccctgattgatactggcggcaaggttcaattcaatactcagccatggcaaaagggtgctcaaacctaccaagctaagcgactctcgattaattacctgaaaagtattggcatctcaaagattgacaatctgtgtgtgagccatcaagattcggaccattgtggcgatttgccggcattcattgaagaaatggaaattaagcggatcattattcctttgggaatggaccaaaaccccagttttatgaagagaattgccaaccgcagtcgatctaccaaagtgatccctgtcactgatgagacgcaagtaccaggtttgccggctcaaatctttcatccctatcttgccggtaagggtgagaatcatgactcaatggtgatcggtactcaaaaaggcggtttgcggtggctatttacgggggacttggaccgcccaggagagctggacacgcttcaaaggcatccgggcttgtcagcagacgttcttaaagtcggccatcacggaagtaaaacatcctctgaccctcagtttattgctaccgtcaaaccacggatcgccttaatttctgccggtcgaaacaaccggtatggtcatccaaacgacgaaacacttgtcacattgaaacagcatcacgttaaaatatttaatacccaaaaacacggtgtggtaagatatatctatcgaaacaataccggtcatttcgaaacggtgttagccggtcatgaagggaatttataatgaactattctcaattaattcaacagttaaaccaaggaaacctcgccccggtttatttgatcttaggggatcaggagtatcttgccggtcgaattaaggatgcttttgtcaaaatcatcccggacaacgagcgttcgatgaatattggcaattacgatatggaagataccacgatttcagccgcggtggaggatgccatttctgtcccatttttcggtgagcgtcgactggtcatgattaaccgaccgtattttttgactggaatgcgtacgaagtccaaattggatcaaaatatcgacgactttttggaatatttaaaacaccccgaagagtccacggttatggtgatctttgccccgtatgacaaattggattccagaaagaaagtcaccaaagccctgaaaaaggtcgccaccaccattgaaattggaaaccttcgtgaaaatgagattaaaaaactggtcacggataagattgctgctgcgggattcaaaattgatcacgatgcattggatcggatggtcgaattaaccggtggtaagctaacggcgatgatgagtgacttgcccaaattgattttgtacaacaatgatacgaaagtcattgatcttgcatccgttaatggattggtcagcaagtccatggagcagaacgtttttgacttggttaatagcgtccttgcgaagaatcccaaacagtcaatggacatttatcatcaattaattctggaaaatgatgaaccaattcggattaacgctgttttaattcagcaatttcgattgttgctgcaggtcatgattctgcagaagcacgggtactcacaaggaaacttagcttcaacactcaaagtgcatccgtatcgggtcaagttggcgatgcagacgatcagaaagttcaattacgatcaattacgagaagcttatattggcctggttgatactgaacgtcagatgaaatcaacccagcgcccacccgaattattatttgaactatttgtgttgaaatttatgaaaagtgtcagttaataaaaaataggagtaagcaaagtcggtcgaccttgcttactcctatttttgtgggacaaaaaaagttgttagtctgactaacaactaggaaagaattattttgctaactttgaagttaaacgtgacttgtcacgagcagccttgttagctttaattaagccctttgattttgcgcgatcaattgcgctgattgcgttaatgtataaatctttaacgtcgtcagaaccggcaacttgtgccttttggaacttcttaacggcagtgcggtatgcacttaattgtgcagcgttgcgacgttgtgctttttcgttagttttaacacgttcgatagcagatttgataattggcatttgactcacctccgagtattattctaagtaaaaattattaaatttcaacaagcatcattatacaaaaaccaacgactgattgcaagccaaactgtcaatgaatatcggcggtaagcttgtatttgtcagagaaatccgttatactattttttgtgtgttgtacaagaccttcaacttagtttgtcgggtaccacttccgcatactcagttgttggcgtcaaaaaataaaaaggtggttatacattatggcaattacacagactaagaagaacgaaattatcaacaaatttgctcgtcacgaaggcgataccggttcagcagaggttcaaatcgctgtcttaaccgcagatatcaacgaactgaacgatcatatgcgtactcatcgtaaagattaccattcacaacgtggactcatgaagaagattggtcatcgtcgtaacctgttggcatacttgcgtaacaaggatgttacccgttatcgtcaattgatcaaggatcttggtcttcgtcgttaatattaacatcaaggagagcggataatatccgttctttttttatacataattattttcctcaattgtcaaatcaagtgcaacactaagaatctattcttagaagtggtctagttgctaagctagttcaggcattagatcggctgggcagcgatagttcaatgaccgccgtagccggttgtttaaggtatcttgagccagctgaatgtcaatgagtgaggccgaagccaaggatctgcccttcgggaagaactcgcgcaaaaggccgttagtgttctcattggttccacgttcccatggtgaataaggatgggcaaagtagatgtcagttcccttgacttgactcaagcttgagaactcagcaccattatcaaaagtaatggttttaaagtgctcggttccatagtcatataaggtattctggagggctttcaagcaagtgtcggcatgataattgggaagtttaacgatgatctctaagcgactaacacgttcagtcaaagtcattaatgctggctcagattcaacccgtttgcctttgaccaagtcaccttcccagtgtccaagctcttgacgcgcttgaaccatggcgggacgctcttcgattgaatggcccagatttttcttattgattcgatgatgctttgccccggggcatttaatccggcgacgtagtttagctggtaggtctgaattgcggatagctaaacgctggtcatcaatataccggtacaccgtcggtgttgaggggcagacaagccttgggtgatcagtcttgaattggtggacaaaagtatccacactatgcatcctgggacgcgcttttaaagctgtcaccaaagcattacagaaggtttgacaatgatcaaagagtccacgataacagctatttagtcggtgcttacgataaattgcttcaccagtttctgccagatatgactgttcaaagatatgagtactagcgttaatctgtgtcgttgtcccacgttttaattcacgtgaaatcgtgctgggattacgatgaagggcctgggcaatccggcggatagaccaatctaagtcccttagaagctgtccaagatctatgatttttgatatacttctatgtaaaaagcgagtttaagctatgaaaaattatcccagcaatattactcggcaacaatttgaattaattcgaccagctttagaaaattttcgtaagcgaactaagcctcgaaaatatgacctctacgaggtcttctgtgcggtcctatatgtcttgaaaaccggttgccaatggcgtcaagtccccggtgatttcccagaatggcggtcagtttacaactattacaaaatttggtcaactaaagctgagcctacggctgattctttattggaacaagtttaaaaaattgtcattgctcggcgaacttaccaaggacgttcagctttaacttcctttattatcgttgacgctcagagcgtcaaaaacaccgctactgctgaaaacaaaggttacgacgctggtaagaaaatctcggggattaagcgccatctggcagttgatatcaatggctttccgcaggccattcacatgacgcgagcgaacgtctctgatcgagacggggccagtgcaatgatcgctttacatgccatgcatttacgccaggttcaaaatgtcttagttgatggtggttattcaggcgttaattttcagctcgatgtagccagtaatttaaacgcaaccgtgcaggttgcgaagcgcaatgagttgcatcgattcgaagtcatgccccaacgttgggtagtcgaacgatcttttagttggctagagaattgtcggcgactttggaaaaattgtgagcgtcaattaaccaccagtctgcaaatggtcgttttagcgtttttagcactattacttaagagattttagacagcttcttagggattcaattcgaccacgttcagctaaattgagttggtgatactgattagatatgatattcttaattcgggtcatgaagatacctctttcttgtttgtggtgaattaagaataggtcttcatggcctttttgactagtctgaataaagaactggtctagtagagcaggtgttgcacttcaattttaaatcgaggtacataattattttaagaaagcacaatgttttttgaaaaattcggtttcaacaaaaaatatgttaaactaaaagaagctgaaaacgaacgtaaaaaagaacatattaatttttgaggtgaatcatgaaaaacgaaatcaaagtaatggcgattggtggggcccgcgaaaatggcaaaaacatgtacgcggtcgatatcaatggcggtatttatattttggactgtggtctaaaatacccggaaaatgaattgttgggaattgacgttgttattcccgattttagctggcttgaagagaataaagatcgcattgtcggtgttttcttaacacatggccatgcagattcgattggcgcaatttcttatttcctgagcaaattcgatgttcccgtcttcggatctgaaatgacaattgaactcgctaaaattaacgtctccgactctgaagaagttaagcacttcgatgactttcacgttgtcagtgatcgcagtgaaattgattttgaagacattaaggttactttcttcaagacgacacactcgattcccggttcactcgggattgcgttgcatacatcaaatggaatcatcgtttataccggtgactttaaatttgaccaaacagcggcgccaatctatcaaacaaattattcagcgttgacccagcttggtgatgagggtgttttggcattacttgatgattcaagcaatgctgagaacccaaatcccagtgcctctgaaaagaagatcgcagaatatatttatgataccttcaattatcaaaacagccggattattgtcgccggtgtcgcctcaaacattttaagaatgcagcaggtcttcaatgccgccgccagaaccggtcgcagagtctatttaaccggccatgacctggaacggattgtcaagactgccatgggattgaatacacttaaactgccagaagacgatttgttgattagctcactggacgagcttaaaaaaatggcccctgataaagttgtcatcattcaaaccggcaaaatgggcgaaccaatcaaagcgattcagcggatggcgaataaagaacaaagtgatattaatattgagcctggcgatctggtctttatcacgacaaccccgtcaactgccatggaaacaacggttgccaagacgcgtgacatggtttaccgtgccgatggcgaagtcaagatgatttctgatgagatgaattcatcgggggatgccagtcaagctgatttacagttgctgatgaatttattacatcctaagtatattatcccagtccaaggggaataccgattactggaagccaatgctcaactggccaaagaaatcggctatactgatgatcaaatcgttattcctgccaagggtgatgtgatctcgatttcagaagatgacattcatttgggcaagggagttgaccttgcggataccatgattgacggtatcggtattggtgatattggcaacattgtccttcgcgatcgaaaggtactctcggaagatggcatttttgtagcagttgtgacgattgaccgcaaaaagaagcggattgtgtccactcccaaattgacatccagaggatttgtttacgtcaaagccaacaaagacttgatgaaggacgccgccgggattatcgaaaagacggttaccaacaaccttgaacacaaagagttcgattggagtaaccttaagcaggacgttcgcgaggatctgagtgattacctgtataaacaaaccaagcggcgaccggttattttaccagttattatggaagttaaccaacaccataaacgttcaaagaaaaagcaaaaagcagctgaaaaaaattagccaactgagcgagtaattcattcttttgaattgctcgttttctatctctacacggtatggaggaaaagatgactgagatgataaaaaacgatcgcgtcatcctgttgagtgctcaagaggatttgcgggatggccgttataatcaggtcgtaaataaggcagagcatttgttgggaaaatatccgcaatccgtggaattgaacgatttgtatgcaaatgcgttgtaccatttgaaaagatatgccgatgccggacaagttgtggccgattttgccgggagtttcatcgctcaaccaaggtatcaaggccatgcgatggagatccttttggccaacaatctgttcatgtctgcccgagaggtgcttgcccaggtatcgacttcaaagaagggggagtggaagcaaagaatcgtgactgctgaaaacgattatcgtcaacagcattcaaccgagctggcggcgaagtcacgtaaatttgcctatcttggggcactttccgtcactgagcaggttcatgaggttcaagcagcgcttcatctgccactaaatgaatatttgtcggccgccaagacattactgaatgatccgtttgggtggcaggtttcgaaaacgcaggtcttgttacaattaatgaaagctcaagtttctgaaaacgttgatttgatctggttggatggaaagacccatacgataagtttggacgaattaaaaccattggagaaaatcgatgcttttgtgcgtgttcttcaaattgttgagcaacaatttgctgctaaggacccaatcaaattggatttgctggaaagagaattattcactcagagtaattatatttacccctattttgatgatgtgatgactgaacccaacttctgggcacaggcaattattgcccaatcgtttggtgagccgttgcccgccaagacacaacagcagcaaagaatgttatcttggatcaaccagattcatgatcaggaaattaaaattggtctcatataactgaattattttcggaaaataaagggaatctgtttacaaacattaccagtatcgatataatacttaaggattcttcgaaaattgactactttgtcttttccagaagatgtagtataataacacttagaaatgcattgatgcgaaattgatgtaattcttgaaaacaacaggaggtttcattaatggcaaaagaacattatgaaagaacaaaaccccatgtaaatattggtactattggccatattgatcatggaaaaactactttgactgctgcaatcactaaggtattggctgcaaagggtctcgctaaggctgaagactatgctgatatcgatgcagctccagaggaacgtgaacgtggtataactatcaacactgctcacgtggaatacgaaactgaaaagcgtcactatgcccatatcgatgccccaggacatgctgattacattaagaacatgatcactggtgccgctcaaatggatggtgctattttggttgttgccgcaactgatggcccaatgccacaaactcgtgaacatatcttgcttgctcaccaagttggtgttgattacatcgttgtattcttaaacaagactgatttagttgatgatgacgaattagttgacttggttgagatggaagttcgtgaattactttctgaatacgattatcctggtgatgatattcctgttctccgtggttcagctcttaaagcacttgagggcgacaaggaacaagaacaagttatccttgacttaatggatgttgttgatgaatacattccaactccagaacgtgatgacagcaaaccattcttgatgccagttgaagatgtcttcactatcactggtcgtggtactgttgcatctggccgtatcgatcgtggtactgttaaagtcggtgacgaagttgaaatcgttggtttgaacgacgaaccattgaagtcaactgttactggtttggaaatgttccgtaagactcttgatgaaggtcaagccggagataacgttggtgttcttcttcgtggtatcgaccgtgatcaagttgtccgtggacaagttcttgctgctcctggttcaatccagacccacaagaaattcgaaggccaagtttatatcttgactaaagaagaaggtggccgtcatacgccattcttctcaaactatcgtccacaattctacttccataccaccgatgttaccggtgttatcgaattggaaaagggcgtagaaatggttatgcctggtgataacgttacattccaagttgaattaactaagccagttgccattgaaaaaggtactaagtttaccatccgtgaaggtggccatactgttggtgccggtgttgttagtgatgttaacgactagtttttatcattagacacacttaagctgtgaggataattcctcgcagctttttttatgtttttagttcgtttgaaattaattttacattttatgattaatacgttaaaataacaatgttatgcaattatgaaattgtaaaaaattcttttggtctcggaggaaaaaagatgtctgcaaaatgggaaaagaaaggtaccaatgatggcgaattaacattcgaaattggtacagattcaatcaaatcaggattagatcgtgcatttaaaaagaataagaacagcattcgggtacccggcttccgtaaaggaaaggttccacgtcagattttcactaagatgtatggtgaagaagcattgtacgaagatgccctcaacattctcttgcctgacgaatatgaaaaagccgttcaagacgctaagatcgaaccagttgaccaacctaagattaacgttgagtcaatggaaaagggcaagccttgggttattaaagctaacgttaccgttaagccagaagttaagcttggcgattacaaaggcttgagtgtgcctaaacaaaatacccgtgtctatcaaaaagacgttgacgctgaattggaaaagaagcgtgaaagccaagctgaattggttcttaaagaagacaaggctgctgagaagggcgatactgttgttatcgacttcgaaggaagcattgacggcaagccatttgaaggtggcagtgctgaaaaccattctcttgaactgggctcaaactcatttatcccaggctttgaagatcagttaattggtcacaaagccggcgatgaagttgaagtaaaggttaccttccctaaagattaccaagctaaagatttagcaaataaggaagccatctttaaaaccaagattcatgaagttaagacaaaagaattgcctaaattagacaatgactttgccaaggatgttgacgaagatgttgacagtcttgatgaattgaaggaaaagatcaaagaagacctcaagtcacaaaagaagtctgaagctcgtgatgccatcgaagacgctgcaatcagtgaagcaactgataatgcagaagttaaagacatcccgcaagctatgattgacgaagatattcaacgtcaaatggatcaatatcttgctggcatgcaacaacaagggatcaaccaggacatgtacttccagttaactggaactaagcctgaagaccttaagaagcaatttgctgacggtgctgagaagcgggttaagactaacttggttcttgaagcaattgttgccaaagagaagattgagccatcagaagatgatgttaaggctgaggtgaagaaccttgccaaacaatatggcatgaaggaagacgctgttcgcagtgccttgactgaagacatgttgaaacatgatattgcaatcaagcaagcaattgatatgattgttgattcatcaaagcaagacgccaaagcaaaatcaactgaaaaggattcaactgaagccagctcagaaaaatagctttttgcttaattaaaagacccgttattttgacgggtctttttttaaggataaagccgattaattgcaatttgtatgtgatatggtaaagttactcttagttgattactactaattgtatttaaagtccatctcggatggaggagtgaataatttgtttgaagataatgaatcaagcgggcctattacttgctcgttttgtgggaaaacacaggatcaagtgaaaaagatcgtcgctggtcctggcgtttatatttgtaatgaatgtatcgatttatgtaaagaaatcatcgatgaagaattggcacctgaaaaatcatcagacgatttactcaaagttttgacgccagctcaaattctggacaagttaaatgaatttgtgattggtcaagaaaatgccaagcggacactttccgttgccgtatataaccactacaaacgggttaacgaaatgattagcgaacctgatgatgatttggagcttcaaaagagtaacatttgtatcatcggcccgactggctcaggtaagacttacctggctcagacaatggctaaaattttgaatgtcccatttgccattgccgacgcaacaacgttgactgaagctgggtatgttggtgaagatgttgaaaatatcctgctgaaactgctgcagaacgctgattatgacgttgaacgagcagagcatgggattatctacattgatgaaattgataagattgccaaaaaatctgaaaatgtttcaattacccgtgacgtatccggtgagggtgttcaacaagccttattgaagattcttgaaggaacaattgccaacgtgccgcctcagggtggtcgtaagcatccacaacaagaatttattcaaattgatacgacgaacatcttgtttatcgttggtggcgcctttgatgggattgaaggaattgtcaagagtcgccttggcgataagacaattggtttcggtaccaactcagatgaagctgctaaggtcgatgccaaaaacatcatgcagtcggttattccagaagacttattgaagtttggcttgattcccgaattcattggtcgtctaccgattttgaccgcattggataagcttgatgatcacgatctggttcgcattttaactgagcctaagaacgctttggttaaacaatacaagaagttaattgaacttgatggtgccgaactggaatttgcgcctggcgcattggagaagatggctcaactcgcaattgcccgtgatactggcgctcgtggccttcgctcaatcatcgaaggcgtcatgcgtgacattatgtttgacctgccgagtcgaaacgatgtctccaaggtcatcattaccccagagactgtgacggatcataaggaaccggaattaatcttaaaacaagcatcgtaattcctagaaatctgatgtagactttagatagcttactgtcagatttcttttttattcacacattttattcattgaaggagtggtttcatggaagttcacaacgtcgaccttacgattagtgctgtcgcagaaaaacaatatccaaatacacaatttccagaaatagcattggtaggtcggtcaaatgttggtaaatcttccctgaccaatgtgttgatcaatcgcaacaaatttgctcggacgtccagtcagccggggaaaactcaaaccctgaatttctacaacatcgaagataagctgtactttgtggatgtccctggatacggttatgcaaaggcatccaaagccagtcgggaaaaatggggccgcatgattgaaacctatttaaccaaacgtgaacagctgcggggggtcattaccctggttgatggtcgccatgcgccaactgacgacgatgtttcgatgcataattggttgaagtattacaatattccaatgttaacggttgcgaccaaaatggataaaatctccagcgggaaatggaacaagcaggaatcattgatcaaaaagacactgcagttggatgcctatgaaccactcattttgttctccgctttgacaaaaacgggtaaaaacgagatttggcgttggattgaggggagaatgaaacgatgaattttgatgactatcaaaaggcagccaatcggacactgatgggtaacgagcaggttttaactaactgtgcactgggactcaccggagaatccggtgaagttgctgacttaattcggaaatatacttttcaaagcaagaggctcgatcatgatgaattggttaaggagatgggggacgtcttgtggtacctgtcccaaatctcagagtgggccgacattccatttgatgaggtcgctaccgacaacatcaaacggctcgaaaaacgttatcctgagcaatcaggtggcgttaatcaagtgaatatttaaggatcaatttagaagcagtcattttgagatggctgctttttttgcagcaatttctggcaaaatgacctcttatttgcatattcgacataatattttcacaaataatgaataaaacataaaaacagttgcattaaatgaatattggtgttaatctcaatacattgaatttttcagaagataagagggaatatatatgtcagaaaataataaagtcattttagcttactccggtggccttgatacctccgttgcaattgcctggttgaaagacaaaggttacgatgtcgtcgcttgctgcattaacgttggtgaaggaaaagatctcgatttcatcaagcaaaaggcactgaacgttggtgctgttaaggcttacgtcatcgatgccctggatgaatttgccgacaactatgctgctgtggctctgaaggccaacgcgatgtatgaagggtcatacccgttgatttcagctttgtcacgtcctttgatttctaagacgttggttcaaattgcccatcaagagcatgccgttgccgttgcccatggttgtaccggcaaaggaaacgatcaagttcgttttgaagtggccatccacggcctcgatcctcagcttgaagtgttgagcccagttcgtgattggcactggtcacgtgagcaagagattgaatacgcaaaggatcacaatattccaattccaattgatttggactcaccatactcaattgatgccaatatttggggccgtgcaaacgaagccggtattttggaagatccatggcaaagtgcccctgaagatgcatttgcaattaccaatccaattgaaaatacgccagatacccccactgaagttgaaattacttttgaaaagggaattccaactgaattaaacggcaagaaaatgaaatttgctgacattatccaagaactcaatgaaactgccggtgaaaatggagttggccgaattgaccatattgaaaaccgtctagtcggaatcaaatctcgagaagtgtatgaagccccggctgcaacggtgctgttaaaagcccataaagagctggaagacttaacatttgaacgtgacttggcccatttcaagccaactattgaaaaacaactgagtgaacttgtttataatgcactgtggttctcaccactgatggattcaattcaagcattcattgataaatcacaagaggtcgttaacggcgtcattaaattgcaactgtttaaaggtaacgtgatggttcttggtcgcaaatcagattcttcactttacgacaagaatctggcaacttacacttcttctgattcatttgaccaagaagctgccaagggcttcatcaagctttggggactgccaacccaggtttatcaacaagttgccctgaaaaataagaacgcacagttcgttcaagcagttaccaagtctcagttaaaggacaaagtgacggttcatgaacacaattctgcacatacaggagctaagaaataaatgagtactaagaaactatggggtggtcgatttcaagaacaagcagcgcaatgggttgatcaatttggggcctcaatttcgtttgaccagttaatggccgatgaagatattgagggctcacttgcccatgtcaaaatgcttgggcacactaaaattttgccaacggctgatgtcgaccagattgtcgccggcctcaacggactccgagaggaccttcatgcaggtaaattgcattttaccgttgaaaacgaagacattcacatgaatatcgaagctttattaaccgagcgaatcggatccgttgccggcaagctgcatactgcccgttcacgaaacgatcaggttgcaaccgactttcatttatacttgaagaatcgcttgccacaagtcatcgatgaaatcacgacgttgcagaaaacgttggttgagatggctgaaaaaaatgttgagaccattatgccaggctatacccatttgcaacacgcccaaccgatttcatatggtcactatctgatggcctattatcagatgctcaaacgtgacaaggaacggtttgctttcaatatgaagcatacggacatcatgcctttgggcgctgccgcgcttgctgggacgacttttcccattgatcgggaatacactgccaaagagttggatttcggtcaaatttatccaaattccctggatgctgtttccgaccgtgattttgctttggagtttttaagcaacagttcaattttaatgatgcatctgtctcgtttctgtgaagaaatcagcatgtgggtcagccacgagtttaagtatctggaattaagcgatgcttatacgactggcagctcgattatgccccaaaaaaagaatccggacatggctgagttaatccgtggcaaatctggtcgggtatacggccacttaattggcttgttgtctacgatgaagtctttacccttggcctataataaggatcttcaagaggacaaggaggggacttttgatacggtcaaaaccttattgccttccttaaaagtgtttaacgggatgctaaaaaccgccaaacccaacgttgagcggatgaagcaggccactgagaatgacttttccaatgccacagaactggctgattatttggctgccaaggggatccccttccgtgaagcccacgggatcgttggtaaactggttttaaagggcattgagacccaccagaacctccaagacatgtccttagaggaactacaggcagcttcacctaaaatccaagaggacgtctatcacgaccttaaatcagaggtggcagttgaacgtcgtcattcatatggcggcaccggatttgaccaagtgcggctacagatcaaaaatgccaagaaggaacttggcgaatagttattgtgtaaatgatatatattttctgacaaaaataaaacgaggcaccgctgaatcagcggcgcctcgtttttcattgtgtatatattggattgagtggtgagaatgctgttggtggatccttaagcagttgttcgttacactctgattaaaatgtgttccgacgggtcagatgctaacttctaaaggcacttcaattcaaatcccaaaaccagggatttaaatcaaagcgcctttagaaaccgcatctcccggccctcgtcacactctgatcgaaacgtgttccgacgcaactggggctaacttctaaggacacttcaattcaaatcccaaaaccagggatttaaatcaaagtgcccttagaaaccgccccaaccgttgctagtcacactctgactagaaccatctcttcttcttttccggtttttcttcattcttgcgttttttatctttatcttttttatcgtgttttaagaacttatcacgctttttatcttccggatccatttcggcaaacttgccgaacatcgcatccatgtcgttttggcgattgacctttaatgccattgagattcatctccttacccttttcgtcataactatagcaaatctgaccgcaaaagtcacatttgttggccattactcactttttgatgcataaatgtattaattatgtataaatacgacttaattaagatttttcttgcataaaatatattttgggtgtaatgtattggttattataaatttggaagagggaaacttgatgaagaagagtcttaaagcaattattcagacattgattatgattgccgctgtatttactttaaccacagtattttcaaatcctgcctccgctgcggacacgtcactgcaacgagttaagcagcgtggggaactgattatggttaccagtcccgattatccaccatacgaatttcaggtgaataaaaatggcaaggataaaatcgttgggatggatatcgacgttgccaaaaaggtggccaaagatctccacgtcaaactggtgattaagagcatgaacttcgattcattgttggtggcgattcaaaccggcaaggcagatatggcaattgggggtattaacccaactgcagctcgtcgtcaaagtgttgatttttcaaagatctattattcaggcggccaaagtttcttgattaattcaagcgatgtcaacaaatacaagagcgccaaaaatttgaggggtgcaacaattggtgcccagaccggtactttgcagtatggtctggccaagaaaaaaattcccaattccaccgttaaagggatggacaagtcaaccgacttggtactggccctcaaaactcataagattgatgctttgggaattgaaaagcccagtgccgaagcttatgtgaaaaatgatcccagcctaaaaatgatttcatccgggtatcatttgaacaaaaatgaaattggcgctgcgattgcctttaaaaaagggtccgggagtttagttgccgccgtcaataagagtattgaccagattaaaaaacagaacctcaccgaacagtacctggctgacgccggcaagtatatgaaggttaatacagtaaatacctccatgttccattattggaagtattttgccaaaggggttgagtacacaatcctgatctcgattgtttcgacgttctttggggtcctgattggcgttatcctggcactgatgcgtttttccaaacagaaatggcttcggggtctggcaattagttacaccgaatttattcgaggcacgccattaatggttcaagttttattcgtttactttggaattggggttgtcgtcaatattccagctttgatttcagggatgattgccgtatcactgaatagtggtgcttacgttgctgaaattatccgtggcgggatcaattcggttgccaagggccagaccgaggccgctgccagcttgggcttgtcaaagggtgacctgatgcgttttgttattttaccgcaagcctttaagaacatttggccggctttggggaatgaatttatttccctgatcaaggaaagctccattgtttcgattattggggtgaccgatttgatctatcaattaaacatcgttcgtgcggatacgtatcgtggtgtcatgccgattttcgtcgccatgctgctgtacttcatcatgacgtttgcattgaccagagtcttgaaccattttgaagggaagatgaaacatgcaggataagaaaattcttgaagtaaatcatttaaataaaaaatttggtgacaatgaaattcttaaagacatcaatgggaccgtcaaatccggcgaagttatctgcgtaatcggtccatccggtgcgggtaaaagtacctttttacgttgcctgaatttattggaaaaaccgacctccggtgaagtgaagtttgaaggaaccgatctgactcatgttgatgaaaaacagttgatcaacttgcgtgagcgaatgggaatggtatttcaaagcttcaatttattccccaatatgacggtgattgagaatctgaagttggcaccaattcgggttaaacacatgaaggatgatgaagcccaaaagatcgccatgcacctcttggatcgggtcggattagctgaaaaggccgacgcctatccaagcagtctttcaggcggtcagcaacaacgggtggcaattgcccgggcattggcgatgaatccggaagtgatgttgtttgatgaaccaaccagtgccttggatcccgaaatggtcggtgaagttcttgaagtcatgaacgagttggcgaaagaagggatgacgatggttgttgtgacccacgaaatgggatttgccaaagaggttgccgacgaggtttggtttatggccgacggctacattttggaacgaaataaacccgaggagttgtttgacaatccgcaaaatgagcgggccaaagactttatcggaaagattattcaaaatgtatgacgcaggcttttaactattagaaagatcggtgagatgaacctagatgtggttcattgtcgccgatctttttgcttgtttaaattgccctggcagaaacatcaggtccaatccctggttcaaagtaaaaagaggcagatagatgaaattcattgtcgaatcttgtaaaatctattgataccagatggttatgaaaatcccgcgaatgttggttggatgaaagaatggtttgatccctctaagtcagacactctctgggacacaacggttgaaccaaacatatattcgatgtataatttttagatgaatattatgaaaggagtgagttttttggcgagtgaatatatcgaacataaattggctttactgcctgacatgcctggctgttacctgatgaaggacattaacggcaagattatttatgttggaaaagccaaaaacttaaagaaccgggttcgttcttattttaagagcagccatgaaggcaaaactgcccggttggtctccgaaattgccgacttcgaatacattgtggtttcgagtgacaaagaagcttttctgcttgaaatcaccttgattcaaaagcatcggccatacttcaacatcaaattaaaacagggaaacggtgggtacccctacattaagattacgaatgaacgggaccctcagattaaaatcgtcaatacgttactcaaagatggcggtttttattttggcccttatccaaacgtctatgctgctgaagagacggttaactttctgcagaaggtctatccattgcgccgctgcaacggatttcagaatcggccctgcctgtattatcatatgggacagtgcctcggggcttgctttaaagtggttccggaagaaacgtacgccaagcagattaaacggattaagtcgtttctgaatggcaatgtgtctcacgccaagcagatgctgacgactagaatggaaaaagcagctgccaagatggagtatgaacgggccgcagaaattcgagatctgatcaagtacattgaaattaccgttgagaaacagaaaattatttcgaccgataatacgcctcgcgatatttttaattactatatggataaaggctggctctcgattcaggttttcttcatccgtcaatcacgattgatgaaacgtgagaaacgtctctttccgatcattgatgatcctgaagaagaaatggtcagttttatctcacaattttataagcagaaaaatcagattctgcctaaggagattctggtgcccaaatcactgccaacagatgtgattagtcacgtggttgaagatgttcccgttagaaccccccagagagggcagaaacgcgatctattggagatggctggtaagaatgcccagatggtcctagaggagaaattccgcctgttagagcttgatgagagcaagacgaccggggccatgaaagaactcactgatgcaatgggaattgcgccggggcacaaaattgaagcatttgaccattctcatattcaaggagccgatctggtctctgcaatggtggtctttgttgatggtcagcccaataagaatttataccgaaagtacaaattaaagaccgtcgatcacgcagatgaagccgccagcaccaaagaagtcatccgccggcggtatacccgactgctcaaagagcacgctgagatgccggacttaattttaatggatggcggggtcatccagatgaacgccgtcaaggatgtcctggtcaatgaacttggattgaatattccggttggtgggatggttaagaatacgcatcaccaaactgccgatttgctttttggtgataatgacacgccactgcagttggatcccaagagtcagggcttttatctgctgcagcgaattcaagatgaggtccatcgatttgcgattacctatcatcataaagttcatacaaagaactcattgagttccaggttggattcgattgccggtgttggtcccaagacacggaacaaacttctccggaaattcggatcgctgaggaaaatttcaaatgccccaattgaggaattgcgtcaattagggatttcagagactgtggcgcaaacaatcaagttctcattgagtaagattgatgaagaacgaaaagtgaccaattatcaagataaaaaattgacgcattaaaatgattcgaaagggctttcttctcaagattattttgacctgatgtaggaaactcggtatactgctagagtattgaacacgtaactaacgacttgggattaattagaattaattaaatggtgataagatgtttgttgatcaagtaaagattaatgtaaaagctggaaacggcggaaatggcatggttgccttccgacgggaaaaatatgttccaaatggcggccctgccggaggtgacggtggtcgcggtggcaatgtcatctttaaggtggattctggtatgaacaccttgatggactttcgataccaccgaaagtttaaagccaagaatggcgggaacggcgccaacaaatcaatgaccggccgaagtgccgacgatttggtcattcctgttcccgagggaacgacggttaccaataccgttacgggcgaagtcattggcgatctggttaagccggatcaagaattagtggttgccaaagccggccgcggcgggcgtggaaacattcattttgccagcccgactaatccagccccggaaattgctgaaaacggtgaaccgggtcaggaagtgtctttgagcctcgaattaaaggtgctcgcagatgtcggcctggttggatttccgtccgccggtaaatcgacgctgttatcggttatcactagcgccaagccaaagattgccgggtatcattttacaaccttggttcctaaccttggcatggtgagattagatgacggccgtgattttgcagttgccgatttacccgggttggttgagggtgcttcgaatggtgttggacttggattccaattcctacgtcatgtcgagcgaaccagagtcattcttcatttggtagatatgtcaggtcttgagggccgtgacccatttgaggattatttggcaattaataaagaactggaacaatatgatgagcgcattttgaaacgaccacaaattattgtcgctacgaagatggacttacccgattctgccgataatcttcaaatcttcaagcagcagttggccgagcattcagatgcagataagacgcgagagatctttccgatttcttcagtgacccatacgggattaaccgaactggttcgacgaacggctgacttgcttgatacaaccaagctttcagacatggagcagccagcggaaacgaccaaggagtacgcttaccaaccggctgagaccagcgatttccatattgaatacgataaagaatatgagtcatgggttatctccggtgataaaatcgagaaattattcaagatgactgataccgaacatgatcaaagtatgttacgatttgcgcgacaaatgcatggaatgggaattgatgatgccttgcggaaggcaggggccaaagatggtgacacggttactgttttggacttctcattcacatacgttgagtagttatttggggaaatacaaattcatatagggcagggaatatttcgatgcaacaggttcaaacaaaaaaacaaggcaaacggcttaaaaacagccgttatatatccggttttgacgggatcagggcactggcggttgttggtgtcatcatttaccatttgctgccgtacaagctgcaaggggggtacttgggtgtaccgaccttttttgtcgtttcagggtatttaattactgatcttttgttacaagagtgggagcaaaacggccggattgatttttgggcattctacgcgcgtcgtctgaaacggctgtatcctgctctggtgtttatgctggtgggaaccggcacatacataacgctgtttcaacgctcactattaaccaatttacggtcaatcattactaccaatatgctgtacgtttacaattggtgggaggtcggccatggccagagttattttgaccggtttaacggtgaatcaccgtttacgcatttgtggtccttatcaattgaaggccagtattacttaatatggccgttaattctaaccgcgatggtcttgattattcgcaaacggcggacaattgccaatattcttcttgtgttggcaattggttccggtgtcttgatgggactgttgtacactggtccggatacgttgaatcgagtttactacggcaccgacacgcgaatgttttcaatcgtttttggtgctttacttgctgttatttggccatctactcatctgaagaaaaacgtgacgacgcgatcgcgttggaccctcaatattattgggctggtgtcaatcgcaatcattgcttacctgtattttgaactctctggtcaaaacacgtttacgtatcgtggcggaatgttcattatggcaatcgcttcgacaaccttgattgcagcctgtgcccatccgggagcggacgtgaaccgctggctgaccaatccggtgtttagatggatggggaccagaagctacggaatttatctttatcaatttccagtgatgattttttatgagatcaaagttcaaaatattgctgcccatccactgatgaatgcaagcattgaaattgctttgattatgattattagtgagctgtcctatcgatatattgaagcaccgttaagacattaccgctacaggaacctcggtcggtcaatttacgagtttgttcaaccgaattcggaatacggctggaaacgattgtggctgataccagcaattttgctgattgggatttcggcatatggaagtgcaatttcacctaccaaagatgccaagaatgtactggaagaaaacatctccaagaacgaaaagaccgctaatgcaaataacaaggcagcgttagctaaacaaaagaaggcttccaagctcactgccaatcaaaagcggatgaagaaactgctgaagaagaaattgacggttaagcagtataaaatcgccaaacactatggcctgaacaaacgtcagtatctgacggtttatcaacaaccgttaaccgccattggggactcgattttagctgataacagtcacgatcttcaaaatgtctttcaaaatgcctatgtttccgctgccgttggtcgtcaaatttggcaggctgggcaggttttgacccaaatgaagaataaaaacgagctggcacctaacgttttaattaacttggggaccaactcaccaatgacttccgcccagattaattcggttatcaagtcaattggacccaagcatcaaatcttctgggtaacgactcacgtgccaaccagaaattgggaaaccgaagttaatcacacgattcgagctgctgctaaacgccataagaatatgcatatcattgactggcacagctatagtttgaatcggcgggattggttctggaacgacaacgttcatcccaatccaaaagggaatatttattatacacatctcattgcgacgtcgattagcgatttttatagtaaaaaataaaagtttgaaggccttcattccatgcaagcagctggattgaaggctttcaaacttttttggcttatttcaaattaatggtgagtgttgaatccggtgagggggcaactttcttttgagtggtggtgtagatggcaccaaactgaatggtgagtttggttgccggctgagtcgcataattgtgaaggtagccggtcatcgcaaagctgacggctcgattagcaccaattttattgccggcagacgagtcggttaattgattagctgtggtcaacatttgcccttgattggttttaacataattgacaccgtttagtgcaatttcaaagttgtgatgattcgtcactgtgtaattgagaacgaaggtgtagtaagtgtctggaatgctgcgaagattgagcacctgttcggcggcctctttagcttgcggcgtcttggcggtgttcttgatgactcttacctggttgactttataagttaatttgtcagctttgatatcaaccggtttggtggtcacgtcggctaattgctgtcgagtcccaaaacggtcaaaagtaaattgatgtttcgtgctcaagtcgccatttttgacatagtgagcattcttttggactgatttgggaactttgtattgataatcactccacgattggctggaacttgaactggttgatgagctggaaggctcgtttgacatatcagcactcaatgactttttctcagttgcttgattgcttttattaccaccgcaggctgctaatccaaccgacaggatggcaaacatgatgattaagtatccttttgctttcatatttttatctcctagtaaaaaacaattgatttattgacaattctaaacccaaatatcaattggcggtcgtttaaagttcttaaatctgtcttgagggagagccgtttggttctggtcatgaattgatccaacgttattgtagcaaatccaccctgagatgggctcgatttgcccaacaataacgaatttttatcaattaacagctgattaaccggcaaaaagtgctgaccttctgaaattaatagggtcaactttgggtttagtgtactgctggcgcggaaaaactcatctaaattcatggctgccattcccttctaatgattattttaacggatttatgatacaattgaaaagtgattttaagcggttggcaggtgccaatcactctaactcgattttaaaaataaggaaacgataataatgcagattgaatttttaggcactggggcagggtctccaggcaaatttcgcaacgtgtcaagcttggcgttacggttacttgacgaaatcaactcggtgtggttatttgatgtcggcgaaggcacccaacaccagattcttcgttcaacaattcgcccccgcaagattgaaaaaatttttatcagccatctgcacggcgatcatatttttggcctgccggggttgttaagcagtcgctcgtttcaaggcggcaacacgccattggacatatatgggccaaaagggattaaagaatatgtcaatgtgagtttgaagatttctgaaagtcggctctcgtataaaattaatttccatgaattacccaaggacaccgatggcaaaatttttgaaggtaagaagtttactgtttatgccgcgcctctggaccatcggattaccagctttggctatcgggttgttgaacatgatcatccaggcgaattgatggtcgagaagttgactcagttgcatattccatccgggccggtatatggcaagttgaaaatgggacaaactgttaaactgacggatggtcgggtgattgatggtaaagaaatgatcggtcgtgcccaacccgggcgaattgtcacgattatcggggatacccgaaaaactgacaacgccgtcaaactggcagagcatgccgatgccttggttcatgagagtacctttggcaagggtgaaaacaaacttgccaagaattattatcattcaaccaatatgcaggctgctcaaatcgccaaacaagctggcgcaaagatgctgctgttgaatcacatttctgcccgttataccggtaaaatggcccatgaacttgaaaaacaggcacaaacggtatttcccaataccaaagttgtgaaggattttgatgtcattgagatcccgtttgagaagcattagcgaatcatttctggggggataagattgaaaaagcaaattagcacaattatcagcattatattgattatcatcattgcaatttttgcattgatgaattttgaatctgttgaggttaactttggcttcgcatcatttcaggtgccactggtacttttgattttgatttgtctcttaattggtgccctgattatttttctgttctcgtcgactcagaatgtcaaaaagaatcgtcaatataagcaattggcatctgaaagccaaaaacgacaagacgatttaaacgccgagattggcgaactcaataacaatctcaaagaattagaaactcgtttgaaaaattcgacgggtaaacaggagattggtagtcgagatcaacaaatcagtgatttgcaggatgagattgccaaattaaccgagaaattatcatctcaaaagtaaggtagagtgttttaatgattgattccaagtataagtggcagcttgatcaaccagctgattcgtcagtagttgacaagttggccaaggatgcaaatattgacccatttatcgctaaaatgttaattcagcgtggcattaccagtgctgatgttgtcgaggatttcttgaatccttctgtcagtgcctttcatgacccgtttttgatgcatgatatgcataagggaattgaacgaattcaacaagccgtcgaaaatggggagcatattactgtctatggcgattatgacgcagatgggattaccagcacaaccgttatgtacgagacattgagtgatctgggtgctgacgttgattattatattcccaaccgatttactgaaggttacggcccgaacgtcgaagcttttcaaaagattattcaaaagggtacatcactgattgtcactgttgataacggggttgccgggaatcaagcgattgcagctgcaaatgagttgcattgcgatgtggtggtaaccgatcatcactcgcttcctgaaaagttgcctgatgcgtatgcgattattcatccgcgggtaaaaaatgaaaatggggatgcttacccatttggcgatctttgtggcgctggcgtggcttttaaagttgctcaagcgttgatggacgaagtaccgtctgatctgattgatattacagcgatcggaacggttgccgatgtcgtatcgttacgtgatgagaatcgcgcaattgttaaattcggtgttcaggcgatttcaaatagtcaacgtccggggctgcttgctttgattaaggaagccggcattgatttggggagatttagcgaagaagatattggctttgggattgctccccgtttgaattcgcttggtcggatcaaagatgccacagtcggggtcgaattattatcgacatttgacgaggatcgcgcaggtgaattagccaaatttgccaatcagcaaaacgacttacgcaagtcacttgtcgaccagttcttcactgaagcggttcagtccgttgaagatagtggcgacatttctcaacggcacacgctggttgtcgtcggccataactggcaccagggggttctcggaatcgttgcaagtcgactggttgacaaatatcagcgcccgacaatcgtcatgaccgacaccgatggtagcgaagaggttaagggatccggccgtagtgtcgacaattttgatttatttaaagcaattgaccccattcgcgatcaaacgattggctttggcggccaccattctgcagttggattgaccatcaagaaggacaaagtgcctgttttgaaggaccagttggaaaaagctgcggaagagcagcaattggatttatctgttaagcccaagttggccattgccggcgttattccggtctctcaggttacagcagtgttatgtgaccaaatcaaaactttggcaccgtttggccaggacaaccctaagcccatttttcaagtccaatttgatcagctcgccaacgtaaaggcaatgggtaagaccagtgatcacctgaagttttcactggttcaaggcaataatcggctcactgcgattgcctttggtcgaggaagtgctgccgttgagcttcaaaattctcaagcagccgttcaagtggttggcgagattggggaaaacacttggaataatcgaacgacgctccaattaatggtcgatgatctgaagcagacattaccgccggtgatcgatgagcggacccacgagctgcaccgaaagatgtttgcgacagtcggcacttacgttttcttccacgaaaaagtcttaaaacagctgcaaggatatgtgggtgaccaatcgcaagttgtgatgtatgaccaagtcaccgaggcatcggctaatggcaatcgcttgtatattgttgattgtccggacgtgcttgacgatttggttcagctcttagccaaagtccaaccacaaaccacggtcctatatctttacaaaaaacaacttatctccaaaatagggatgccagatcggaattcttatgctaaactgtttaggttcgttaaagaacattcaaacgttaatattgcgacgcagttaaaacaaatttcagagcacttacacatttctgcacggacaattatttttatggttcaagtctttttggagttggatttcattacgattcaggatcgggtgattaatttgaatccgaattatactgcccgtgatttgaaaacagctccaagttaccatcttcgagttgaacagcttgcagctgaaaagaaattgttggtttcaaatactcatgaattagtcagcttcgtcaaggactgtttgggtgtttgatgaaaggaagaaagaatatgccaatcgatttttcaaaatatattgcatcatatccggactttccggaacccggaatcctatttagagacatttcacctttacttgaaaacggtgaagtctatcgggcagcaaccgacaagatagttgattttgccaaggaacggaacgttcagatgattgtgggtccagaggccagagggttcattgttggctgtccagtcgcctacaagttgggggttggtttctcaccagctcgtaagaaaaacaaactgcctggtgaaacgattgaggaaagttatggcttggagtatggtaaatcatcactgtacttacgaaccaacgctgttaagccgggtcagcgggtcttagtaacagatgacttattggccactggtgggacaattgatgcaactattcgtctagtagagaagttgggcggaattgttgtcggcaccgcatttttgattgagttgtcagatcttaaaggccgtgaaaaagtcaaagactatgatttctttactttgctaaaatattaaaccaagttcattactgctggttatccagtggcaatgagcttttttgttacatttgaattcgtacttagttaaacaaaaaagcatctcagcattggtacgctgagatgcttactgtcatataaggtgagtacaggatttgaacctgcgcgccggtattagccggttcgccggatttcgagtccggtgcattaccactctgccaactcaccacaacagttttaattatatcaagagttattctgaaagtaaattactgtctacttggaagaggcaaattttgttttaacatagccaacgactgccggaatgagcgagatcgcgacgattccaataatgaccatcgagaagttttctttaacaacggggatgttaccgaagtaatagccggcaccacaacagatggcgacccatgagatacatgcaatcagattatacttaatgaatcgtttataaggaaaatcactcgtagcggcaacgaaggggattaacgttctgatgattggaatgaatcggccaaagaagatggccattgccccatatttgttaaagaactcccgggccttggttaaatccttttccttaataaattttcccaggattcgatttcggggaataatttctccaaatttgtttccaaagaagaagttgagtgaatcgccgccaattgaagcggccaaaaagatgattacaaacaagccgatgcttaaaccgtagtttacgttggctgataatgccgccgcagcaaatagcagtgagtcaccaggcagaaatgggaagatgactgcgcctgtttcaataaagatcactccaaagagaatgaggtaggtggagttcccaaatgtattcacgatatttattaggtgatcgtcgatgtgtaagataaaatcaatgagcgtgctcaagtaatcattcctttcgaaaatttataattgattttaccaaattccctgagaagttggcgagttattacctgtcctttaacaaaaaataagttttgttgttaaatcaagggatccacgctacaattattaacagattacagataggatgattattatgagttttaagataggcatgaaggtccatggaaccgtcactggtattcaaccctatggcgtattcctggatattggtgaacatatgcaggggctgattcacatctctgagtgtcaaacaggattcgtggatgacctctataagatctttcgggttggacaaacagtttccgcgctcattattgatattgatgagtattctggcaaaattagtctctccactcgcagcactgatgttaatcttgaaatccttcgccggccaaaaagctttcgtccgaagagaattcactactggactgattaccgattgaatatcggatttacgtcacttgccagggctaaaggtggttggatgagggatgcccagaacttttttagttagtttggaagaaagttcttgacccagctttcacaaattggtagaatattttctgttgtcaattatccatttgatctgccagtgacaattaacatttgaaaaatcagttaaaaatcacttgatttcaaaccggatatctgataatattaaatagttgtcaaaagcgagaaacaagcgcttccgacaaccaagtagacctttgaaaactgaacaaaattttcgacaaacaaatgtgcagggcgtttcaattcttcggaattggaaccaaacatttgcgaagtcaattcgtaaaaacaaataataaatttaaatcatgagctatcacaggcttatcattttaaacaatttaagatgagagtttgatcctggctcaggacgaacgctggcggcgtgcctaatacatgcaagtcgaacgcgtctccgttgatgattttaggtgcttgcacttgaaagatttaacattgagacgagtggcgaactggtgagtaacacgtgggtaacctgcccttgaagtaggggataacacttggaaacaggtgctaataccgtataacaaccaaaaccacctggttttggtttaaaagacggcttcggctgtcactttaggatggacccgcggcgtattagcttgttggtaaggtaacggcctaccaaggcgatgatacgtagccgacctgagagggtaatcggccacattgggactgagacacggcccaaactcctacgggaggcagcagtagggaatcttccacaatggacgaaagtctgatggagcaacgccgcgtgagtgatgaagggtttcggctcgtaaaactctgttgttggagaagaacaggtgtcagagtaactgttgacatcttgacggtatccaaccagaaagccacggctaactacgtgccagcagccgcggtaatacgtaggtggcaagcgttgtccggatttattgggcgtaaagcgagcgcaggcggttttttaggtctgatgtgaaagccttcggcttaaccggagaagtgcatcggaaaccgggagacttgagtgcagaagaggacagtggaactccatgtgtagcggtgaaatgcgtagatatatggaagaacaccagtggcgaaggcggctgtctggtctgtaactgacgctgaggctcgaaagcatgggtagcgaacaggattagataccctggtagtccatgccgtaaacgatgagtgctaagtgttggagggtttccgcccttcagtgctgcagctaacgcattaagcactccgcctggggagtacgaccgcaaggttgaaactcaaaggaattgacgggggcccgcacaagcggtggagcatgtggtttaattcgatgctacgcgaagaaccttaccaggtcttgacatcttctgccaacctaagagattaggcgttcccttcggggacagaatgacaggtggtgcatggttgtcgtcagctcgtgtcgtgagatgttgggttaagtcccgcaacgagcgcaacccttattgttagttgccagcattcagttgggcactctagcaagactgccggtgacaaaccggaggaaggtggggatgacgtcaaatcatcatgccccttatgacctgggctacacacgtgctacaatggacggtacaacgagtcgcgaaaccgcgaggtcaagctaatctcttaaagccgttctcagttcggattgtaggctgcaactcgcctacatgaagttggaatcgctagtaatcgtggatcagcatgccacggtgaatacgttcccgggccttgtacacaccgcccgtcacaccatgagagtttgtaacacccaaagccggtgaggtaaccttcggggaccagccgtctaaggtgggacagatgattagggtgaagtcgtaacaaggtagccgtaggagaacctgcggctggatcacctcctttctaaggaaaaacggaatcctgcacattgtcgaaagttttgtttagttttgagaggtctactctcaaagttggttacgcttttttgggcctatagctcagctggttagagcgcacgcctgataagcgtgaggtcgatggttcgagtccatttaggcccatccacggcctgatagttagctatcaccggagtaacatggggaattagctcagatgggagagcacctgctttgcaagcagggggtcagcggttcgatcccgctattctccattgacacgagagtgtcagacttggttctttgaaaactagataatattaattttctgtaataatttttttgaaattgtatttatataatttcaaccgagaacaccgcgttattttgagtttgttaactagaaaaaaatcgcaaatactcaattaactttgcatcacgtagtgatgtacaggttaagttaaaaagggcgcatggtggatgccttggcactagaagccgatgaaggacgggactaacaccgatatgcttcggggagctgtacgtaagctttgatccggagatttccgaatggggaaacccagcagttttaatcgactgttactatatagtgaattcatagctgtatagaggtagacgtggggaactgaaacatctcagtacccacaggagcagaaagaaattttcgattccctcagtagcggcgagcgaacggggaacagcccaaaccaatgagcttgctcattggggttgtaggactgaacatttgagttaccaaagttgttgataatcgaacaatctgggaaggttggcgaaacagggtgatagccccgtaggtgaaatcaatgaccctcagttcaggatcctgagtacggcgacacacgtgaaacgtcgtcggaatccgggaggaccatctcccaaggctaaatactctctagtgaccgatagtgaaccagtaccgtgagggaaaggtgaaaagcaccccggaaggggagtgaaatagttcctgaaactatgtgcctacaagcagttagagcccgttaatgggtgatagcgtgcctcttgtagaatgaaccggcgagttacggtaacatgccaggttaaggtttaaaagccggagccgcagcgaaagcgagtctgaaatgggcgttttagtatgttgctgtagacccgaaaccaggtgatctacccatgtccagggtgaaggtgcggtaaaacgcactggaggcccgaacccgtgtacgttgaaaagtgctgggatgaggtgtgggtagcggtgaaattccaaacgaacttggagatagctggttctctccgaaatagctttagggctagcctcggacgtagaatcatggaggtagagccactgtttggatgaggggcccgtcatgggttactaagttcagataaactccgaataccattgatttttatccgggagtcagacggtgagtgataagatccatcgtcaaaaggggaacagcccagaccaccagttaaggtccctaaatatatgctaagtggaaaaggatgtggagttgcatagacaactaggatgttggctcagaagcagccaccatttaaagagtgcgtaatagctcactagtcgagtgattccgcgccgaaaatttaccggggctaagcatattaccgagactgtggacttgacctttggtcaagtgataggagagcgttctaagggcaatgaagctagaccgtaaggactggtggagcgcttagaagtgagaatgccggtatgagtagcgaaagatcagtgagaatctgatccaccgaatgactaaggtttcctggggaaggctcgtcctcccagggttagtcgggacctaagccgaggccgaaaggcgtaggcgatggataacaggttgagattcctgtactagttgatgatgtttgagcgatggagggacgcaggaggctaagttgtgcatccagttggaaagggatgttcaagccacaagtcagtcaaagagtcaaatgctttttggcgggttgacaagtggtgatgaggaccgaaatttaagtagggaagcaaccaacgtcacactgccgagaaaagcttctagtgagtcatcaactacccgtaccgcaaaccgacacaggtagtcgaggagagaatcctcaggtgagcgagtgaactctcgttaaggaactcggcaaaatgaccccgtaacttcgggagaaggggtgctgtgcgcaagcacagccgcagtgaaaaggcccaggcgactgtttatcaaaaacacaggtttctgcaaaatcgtaagatgacgtataggggctgacgcctgcccggtgctggaaggttaagtggatgagttagcttcggcgaagcccagaaatgaagccccagtaaacggcggccgtaactataacggtcctaaggtagcgaaattccttgtcgggtaagttccgacccgcacgaaaggcgtaacgatctgggcactgtctcaacgagagactcggtgaaattaagatacctgtgaagaagcaggttacccgcgacaggacggaaagaccccatggagctttactgtagcttgatattgggtgttgacacagcttgtacaggataggtaggagccattgaagccggaacgctagtttcggcagaggcgttggtgggatactaccctcgctgtgtgaacactctaacccgcgccactcagcgtggcgggagacagtgtcaggtaggcagtttgactggggcggtcgcctcccaaacagtaacggaggcgcccaaaggttccctcagaatggttggaaatcattcaacgagtgtaaaggcagaagggagcttgactgcgagacagacaggtcgagcagggacgaaagtcgggcttagtgatccggtggtaccgtatggaagggccatcgctcaacggataaaagctaccctggggataacaggcttatctcccccaagagtccacatcgacggggaggtttggcacctcgatgtcggctcatcgcatcctggggctgtagtcggtcccaagggttgggctgttcgcccattaaagcggtacgcgagctgggttcagaacgtcgtgagacagttcggtccctatccgtcgcgggcgtaggaaatttgagaggagctgtccttagtacgagaggaccgggatggacataccgctggtgtaccagttgcgccgccaggcgcaccgctgggtagctacgtatggatgagataaacgctgaaagcatctaagtgtgaaacttacctcaagatgagatttcccattcctatatggaagtaagacccctgagagatgatcaggtagataggttggaagtggaagtgcagtgatgtacggagcggaccaatactaatcggtcgaggacttaaccaagtagaaatggtgttcaagggcagaaaattaatattagctagttttgagagaacgaagttctttcaaggaaaaatagtgtggtggcgatagccagaaggatacacctgttcccatgccgaacacagaagttaagcttctgcacgccaagagtagttgggggatcgccccctgcgagggtaggacgttgccacgcgattattccggcatagctcagttggtagagcacctgactgttaatcaggttgtcgacggttcgagcccgcctgccggagttattatttttaatggagagttgtccgagctggccgaaggagcatcattggaaatgatgtaaacgggtaaaagcctgtttcaagggttcgaatcccttactctccgtaaccgaataataagtttatgacccgttggtcaagtggttaagacaccgccctttcacggcggtaacatgggttcaaatcccgtacgggtcattatggaggattagctcagctgggagagcatctgccttacaagcaggaggtcacaggttcgatccctgtattctccatttccatagcaacattggttcgttggtctagctggttaggacgcctgcctgtcacgcaggagatcacgagttcgagtctcgtacgaaccgttgttatgtatttgaaaattgaatgcacaacataggtattattatactcaagatggttaatggctcggtagctcagtcggtagagcaatgcattgaagctgcatgtgtcggcagttcgattctgtcccgcgccattcatggaggggtagcgaagtctggctaaacgcggcggactgtaaatccgctccttcgggttcggtggttcgaatccactcccctccatcttatagggatatagtttaatggtagaactacggtctccaaaaccgtcggtgtgggttcaactcctactatccctgttaataatactatggcggtattggtgaagtggttaacacatcggtttgtggatccgacacgcgtgggttcgattcccacataccgccttttgattgggttatagccaagtggtaaggcaacagactttgactctgtcatgcgctggttcgaatccagctaacccagttgggttagccaaagttatggcggtatagccaagtggtaaggcagaggtctgcaaaaccttcatcgtcggttcgaatccgattaccgcctttttccatgtattggccaatcaaatattattttgccggagtggcggaattggcagacgcgctggactcaaaatccagtgatcgttgagatcgtgtgggttcgaaccccacctccggtatcactaacaaatattaataaaaaaggaatcattgaatatcaatcaatgattccttttttattgacttgaaattgaatcaagaacaaaaccacaattaccgatacataccacaaccacgctcaacacgaggctgtgattgatgcggcgttgtacaataatgagtgacaccaacggcacccgtacacagcgttaaggcggatgcacatacaattaaaaatttcacggacgttcaccaaccttcataagttaatttaggatagcattctacgtgatcattttaacatagagatcaatgcgagtcattaccaatcaataccggaccgattaacgatagtaggatgtattgggtgagggagggtaagaaaattagtgagcctccattaccattgcctcgctaccgtttttttgtttaaataggtcatctataaataatcggcgacaatttttaaaagaaaaagattgaagattatcgtcttcaatccaaagttatcttgattcagctagggtctagcatattgattaccacgcgatgcttgggttgcaccactggcatttgcttgagaaacactctcgtaatggtaattattgggattcttgacctcagaataatacttgtcactatcagaaacaaataccattccggatctagcaattgtccaaccgccatttgtagttgtggctgtagcactctgatgtgaattggaactcccagtcgaagtagttgaacgatgatgtgtataagccatcgtcgagctgcgtcggtgatattgtttggcgttgttgctgccatcttggtaattaattcggataccttcagcgtcattgataaccacaacttccgtgttcaaggatttatctgatgatcggacatcgacaattgatccacggggcatcgtttcgcttcccttgtacaggggagttgtttggtaataaataacgtggtgagtattggggttgtcttcccagtaattttccgccgcttcctctgtggcccgcattccaccattttgatcggcgcccacattttgcggtcgggtacccgttgtgaaattgtagtttgatgtatatgatttggcccccagcaaactgtcaccaatcgagtggctccgattataaaggtagccatgataggtccgccccgtcagtccataggtaattgataccattttgttttccggccaggcaggaggttccagtggatctccttgacggccgccctgggacagatgatattcagaataagtcagcactgctcgggcagtcgcagatctgccttgggcatcagctgagaaatgatagtcaccagctgccagcccggcaaaatggctaaaatgagcttttccagttgtccaataataatcaccagtcggcccggcggattccttgttggtataactcaccagcttgttcaaaatggcttggtgctgttggcttgccgacgcagttgaactgtggtgtgaatgagtatgaactttttttgctgattgggtggcatgagaactactggttgtagccacctgcgatgcgtgatgatcggcggcctgatgactgccactgccatcgctgcaacccgccaagccgccagttatggcaatcaatatgacggctgttagcaggatatgttgatgtgatttcacgttgtgatccccctcaaaaaatgtttcgttgaccaaatcaatcggccacataagtcgtaatacgataaaatgcgaacaactattcatttttattatacagttgaatctcatctgttaacagacgaactggaagatcgatttggttaaagctagaataaggatcaagaaacttgagcactgatgggggacttgcttctagagacccccatatgaggatccgaaaatgtctgacgatcctttcgtagtgtatgccattgaacgacacactaaaatgtcaactgacgataaaaaagcccgtcacgaaatatttcgggctctacaatatctgttgttggtaatagatttttatctattactgatgacagattttttgtttttcattagaataaaaaaagcggacatttcctgtccgttcatcaaaaccaacaaccacgaagattttagagaaagaaggaaatgccctatgtcaaatgatactacgaaaatgttgttaggaatagatgatgaacacttaaaaattgagaatggcaaaataggtgatgatggggtaatcagattaaatggatcactgaactattctcccaaggcctgccgcaattgtggggttattaatgatcaccagatcattggctatggttggcggaagaccaccattagattcgctaaaacattgggcagcacggttatcctatgcctcaatcggcgaaactttcactgtaaggcttgtcataccaacttcctggcgcagacgagtgcagtgccgaagcactgcacgatttcaaatacaacccggaaacaatgtttagagaagttaacggaaccagtgagcctcaaacacattgccaatgaattgtccacttcggattcattcgttggtcggcagctcttgcgcgctgaacacgactttcaaaccaactggcactacttacccaaagttctcctcatggacgaagttaaaagtactaagagcgccaccgacgcgatgagctttgaatttatggacgcggaaacccacgaattgattgacctgttgccctttagaaccatctatcagcttcaaaagtacttccaacattatgaccaagccgcgcgagaaaatgtgaaaattatcgtcaccgatatgaactatacctatcccaaattggttgggcagatcttcccgaacgccatcgttgtcatcgatcccttccacctggttaacgctttaaaccgggcttttaataagacgcgagtgcgtctcatgaaaaccctggccacttcctcacgccagtatcacgccttgaaacgctattggaaactattattaacgccggccaatcaccttaactacgaggctttccgtaagtggacaaacttcccttatccggcaactgccacggatgtggttgatgctttactggacattgatcccgagctcaagcaaacttacgacgtgatgaatcggttacgtgaaaccatcaaaaaccgcgactggcccaactataatcaagcctttcaccacctgcaggggtgctcggaagagatgttggcagccctccaaaccttggcggctcatcatgatgaaattggcaacactttcacccaccactacaccaacgggccattagaaggttcaaacaacaagattaaagtcattaagcgtactggatttggttaccgaaacttcttcagattccggctaagagtgctgttcgcttttcgagttcatacaaaaagagccctaatcaccaagtgattagaactccaatattttgttcaccaacaacagttgacgaagaaccatatttcgtaacgggctgatcaatttaatcatctaatctattagacgttcaaaattttattcaagaaatcctgtaatcgttcattctgcgggtgttcaaaaatttgttctggggtaccttcttcaaggatttgaccgtcatctacaaacacgacccggtcggctacttccttggcaaatcccatttcgtgggtaaccacgaccattgtcattccttgcttggctaagtccttcataactgccagaacatcgccaaccatttcgggatccagtgctgaggttggttcatcaaacaacatgatgtctgggttcattgccaatgcccgcgcaatggcgactcgttgctgctgaccaccggacaatgattgaactgtcgcatcgaacttctcctgtaagccaacggtttccagtaactttttagcctgaactgctgcctggtccttggtttcctttttgagttcgacaggagccaacataatgttttcaccaacggataagtttttgaacaaattgaaatgctggaacaccataccaatattttcccgtaccgcgttaatatcaacatcatttctggcaatgtcgacattgtcaataacgatcgatccagaagttggttcctccaacttattcaggttgcggagaagggtactctttccagatcctgaagggccgatgataacgaccacttcatttttttgaaccgttagattgatgcccttgaggacttcattgtcaccaaaggttttgactaaatttgtgacttttactttttcgctcataccttagttctcctttgtacccaatttgataaccaagttaatacagtaataataatcagataaattgcggcaacgattgtccagactttgaatccttccaagtttctcgcaataataattttaccggtctgggtcaattcaagcaaaccaataattgataggattgacgtatccttcaaagtaataatgaattggttaataaacgacggcaccataattcgaatcccttgtggcaggataactttacgcatggcttttccaaacgggagccccaaacttctcgaggcttccatttgtccgggatcgacggcttgaatgccgcctttgacaaacgcggcgatatacgcaccttcgttaaaggtcagcgtcacgaccccggcgacaaaggcaggaattttttgccccgtcaaactcggaattccagtataaatgaacagtgccaaaaccagcaggggcattcccctaaacaggtaaatcaacgttgtcgaagttccctgactgaatttgttaggcaccacgcccatcaatccaaccaaaacaccgaagatggttgcaaagaagattgataccactgtcagccaaagggtttcttgcagccctgaccatagggcacctttattttgcttaattaagccgataaacgtccggtcttcggcgctgttgccagatgtcttggcagctgtcttaatctcatcagcacccaaatatttggccttaatgctatcatctgtgccgctggccttcagatctgccagtccttggttaaacgcctgcagaagtgcttggttatgaccttttttaaccgcaaagccatatggtgcatttaatgcgggcttggtgacaatcttcaacttggttccttgcttgattgcgtattgcataactggatgatcttcaaaacaggcaactgaattcccggttgagacatcttgatacatattgttggaatcatcgaatgtaaccactttaaagccgtatttctttttgatactattggcataatcggcacccgaggttccggttttaaccgcaacccgtttacctttcaactctgacaatttatgaatcttgctgttcttagcaacagccatgacaactccagaattgaagtacggtttggaaaagtcaaactgagctttccgttcgttggtgattgacattccggcaatcacaccatccgcttgaccagactcaacagcttggacggccgcgttgaatcccagggctttaattttgactttaaagccttgttcgttggcaatagctcgaattaaatccatgtcaattccgacgtatttgttattcttgttggcaaattcaaacgggggaaaggtaacatcagttccaataacgaaagttttgccttttactttggaattatttgcgtttcccagatacttaccgacaattttgtcgtaagtcccattcgcttgaatctttttcaggccggcattgaatttcttaattaatgccttgtgagtgccctttttaacaccaaacccataccaaccttggttagcaggcttgctggcaatttgaagctttaaaccgtgtttaatgccatactggagaacgggttggtcgtcgaaacaagcaaccgagttgccggtcgtgacgtcttgatacatattatccgaatcatcgaacgtcacggtcttaaacccatacttcttcttcaaactattggcataatccgcagcggccgttccggttttgagagctacttttttacccttaagttgtttgaaactggtgatgtcactgccttttttgacggccatgaccgcaccggtcttatagtagggtgttccgaaatcaaacttatcttttcgttccggggtgatcgtcatcccggcaataattccgtcaagctggccggattgaacggattgcaccgccgcgttaaatccaaccggcttaacattgactttaaagccttcctctttggcaattgacttgataatgtcaatatcgattccgacgtatttattttccttgttggcaaattcaaatgggggataagtaacatctgtcccgatttggtacgtcttagcttgtgcttcgctgcctggtagcgccagacagaacaagatcgtggcaaaagctgccagcaatccgaaagccgttaacactttgcgcttcatgaattattcctcctagacatatgtaataaaacataacatataataatgagaacataataccagaaatttgtgaatctgtatagcattaaccaatttgtgcaaacggtgccaagcttgctgtgacattgcaaaacactgagaattattaattttaaattagaaaatgtgttgacattgatttggcagtttatcataataatcattaaaattcatttagcatttttatgatcatttatacataccacattggaggaaatcagttgaaatttgaagaatcgaatgtattacagcagttgccgaaacaattttttgccggtctggtcaagaaggtcaatgctaaagtagccaccggtgcggatgtcatcaacttgggtcaggggaatccggatcagccgactcccgattttattgtcagatccatgcaggagcaaaccgccatacctgccaatcataaatattcgcaattcagaggtgacccggaactaaagcgggcagcggccaacttctatcaacgtgaatatggggtcactttagatcctgataaggaaatcgccattctcggcggttcaaaaattgggttggtggaactaccgtttgcactgctgaacccgggggacacaatgctgctgccagatcccggctatcccgattacctgtccggcgtttcactggcacaagtcaaactggagctggtgacgctgcgtgaacaagacgactttttgcctgattatcggaccattaaacccgaagtcgtggatgcggctaagctgatgtatctcaactatcctaacaatccatccggagctgtggccacgccggaattctatcagcagacggttaactttgctaagaccaaccatattggtgtggtgcaggattttgcttacggggcgattgggtttgacggccgaaaaccggtcagtttcttacaaactccaggtgccaaagaagtcggaattgaaatgaacactttctctaaatcctataatatggctggctggcggattgggtttgcggccgggaacgccgatatgattgaagccatcaatctgattcaagatcatttattcgtgagtgtcttcccagccatccagaaagctgccattacggctttgaatagcgatcagcagtccgttcatgagttggttgccctctatgaaaaacgccggaatcaatttttcaaggctgctcgggcaattggctgggaaccctatccatccggcggttcgttttatgcctggatgccggttcctgagggctataccagcgaatcattcgccgatctactgctggatcaagcagcggtggctgtcgcccctggtaatggttttggcaagggcggagaaggtttcgtccgggtgggcttattaattgacgagccgcgatttaccgaagcttgtcagcggattgccaagctgcatttatttgattagagtttactagcaacctcgttttgcgcctaaatgttatctagcagaactgtgcgccaataagcagcttccagagtataaggggattacccaaacatccaagttctggatatttgggtaatccccttatactctggaagctgcttatttgcccacgctcgttttcctaaatcgttaaaattagccgttcgcgcagctttattttagataatcgtggaactcaaagccaagcatctttggcctgcctccatagttaccagtaaccaagaagtttggtcaattttgcccgattcaaatcgcgattggtgatcgtggccatttcggtgccgtccaatccattgatggatttttcgaccggcttctgccatgcatatttggcaatcatattgccggcactggtcgctgcatacatcaagtctgcctgatagccggtgtggtcaagcccaagggtatggccaagttcatgtgccaggacaccatcccaatattgatcaatcgtaaatttggcagctagactgggtttgatataccccagcggatatttggcatcgtgatagtgggttttatcgataaaaatttgcctgccgtcgtaaagaccatcccagccttcttttgtcccgctgccaaatgaaatctttaaggtatagtggctttggcttcccatctgaaagacagtttcacccaaggcagtattccatttgttcatggcgttttgaacgtgctggttcaattccggattggccacgtaaatcaacgcgtgatgatccttgaacattgaggttggcgaaaaatgaaaaacgttatatgccaagtcaaaaacagcttcatgggtttcatagttcaccggcttcagacttaggatagtttcatccggattcatatctggggctgcattaatcaatttcatcagcgacttctgagacattgccacttgcgttttggttaaatagccgtgccaaatataccccgttattgttttgcttttattggcaacataatagtagactgccgttttaccattcggttttctgacggtcacccgtttagtagcgtagaagatcgtttccggataatttttagcgctgtgaagtttttgcgttagcgttttatccccataaataatccctttggctgctcgataggctgtgcttttctggggagtgacccggacaatttttgccgctgtggtttttgcatcagccgaggttgcggcaacatcaatcatcaatgctaacgaaagcagtccgactgccagcaacgttaatttttttacgacccgactcatttgaacgtgcctcctcaaagctgcaagtgtttccattaatataccatatccgattgataatttgctacttatggccttggcaggttctcagaagttgtgaccgtggattttatcagtggtaatctccggcattggttctaccagatgggtcgtatccctgtattcgatgcttagatgactcatgtttttaaggtcggagagaacctgctgatatttgtggggatcgtgaaccaacgctaataactcatgtgagcggaccaacttggtttttaatttccgactataaatgaagaagtaatagcggtcattaaaatggttgtcgacgatcaccaaccagtattggtagttgggaagtcgcttgaagtattggtggtacttgtcaattagttctcttgattctgccagcatggtgaagacctccttgagataaatcgttaagcttgatgaccgccaaccaaaccggcacggtcgattgcagtgccgcctttggttttggacgaagctctgattagtgctttgtaaccgtattttttgcggataatgtcgatggtttgctccaatttttccttatccaaggtagtgatgggatcctcaaacaggctgaagcgggtttcacgcttttttgaaagccgattgcaacgaaccccgacgttacgaactgcgctgccgtcccatttactttccaataaatagtggacggcattggcaatgcttttggttgagttggtgggttcaacgtgcatttgggctgagaagtgggttcgtccctgcttgtctgtggtggccatcccgatgaaaatactgacgacttcagcgacgacgttgttttttcgcaggcgggtcgcgacttgatcggcaatttcaccgaaaacagtttttagatcacccaattccgtgtagtcgcgcattaatacctgtgaattgccgtaacctttattgtctgaacggggaagataacgcttctcaaggttggagtagtcaatgccccacgcgtggtagtaaagctgttcacccatgacaccaaatttcttctttaacaggttaacgtcggcgtgggccagttctttaatggtataaatgcccaactgattgagtttgacggcggtgtggctgccagttccccacatatcggcaagatctggaatctgccaaatagtatcggggacgtcggcgtagtcccattcggcctgccaaggctcttttttcttggcggcgttatccagggccagtttggccagcaggggattttgtccgatgccaatcgtcgtgacaatgccggttgctttaaaaactttgtcttgaatcaatttggcaatttgggcattggaaccaaataatttgtggctgtggctgacatcgatgaagctctcatcaatagaataggggaaccagtgaatatcatcggtaaactgacggtagatgcggttgattcggtagttaagggcaacgtaatcggccatgtgcggttccaccatttcgatatccatctgatcattgacttcaaatcgtcgagtccccagtttgacaccaaagtttttcttggtgtagggactggcagctaaaatgagtccaccggaggattcttcgcggctcatgacggcaattttggtggaaaggggatgctccccgcgcttgatggcctcagtggaggcaaaaaaagacttgcagtcaatgcacataatgtcgtggctgggcaaaaggctgggattatcaagaggtgtttgcataaggatcacctgcgattggaaaagttttattgagtatctatataatacgaacatttgtttggtgtgtcaagaagaacagagcgcggaccaagccggttagcttctgagcatttatgtaatcacgagtgttgatgcgggttgggcatcaatactcgtgattggataaagcggaggaagctggcttggggagcgcattttgaaaacagagcgcgacgagacccgtttagggcccagaacataagtgaggaatgccaatgatgaacggtctgggttcatcgttggcattcctcacttatgtggccgggccctgggtcgtcggagcgcattttcaaggccgaagggagcagtaaatataataagcgcaacaaacctggtggaagctagcccaaaataacatgggaaaaggaagttgatttatgtataaggaaattgtatctgggtagaactaaccccaaaaagatcagtaactccacaaaaaagcgcccctcccaagttttccgccttgagaagagccgcttcaatttcatttttatcaattatcatcaatttcatcaatatttcaaaaataatcagacgctaatttgctgcttaaaaaatatctgagttaatcacctgcaactttcaagaacacagcgccaagccccttatcaaaggttgctttccagtcgccattgctgagtgattcaggtagtaggaaggtaccgcttgaaacacgttgaccagcttgtagcggcattccttgtgattcgagtttttcaaccagccagtgtaaggattttaacggattgcccaacacttctgatgaagcgccgtcctttagcttcttgccgtcatggaatagttcacatttaacgttggctagatcatcgacgttgtcaaataggagattggtatctttttcatcaccgtagacgacgtaaccaccaacagcagcatcggacatgaccatatatttggataggcttgggaaccagtcactgaagcgtgaatcaggtacttcgacagctggggcaaccttggtctttctcatgagatcttctaaagaatctttgctgctgagatcttctttagcagtaaagagcatttcaacttcagcaagtggttccatgagttcgccacggtgaagggtaactggggattgtaggaaatggctcttaacctgggcaccatatagtggtgagtcggagtcaaacatatcttgagtttgattactggtaagcgatactttgtagccgccaacgtcttcctgcttgagttgggttagtcgtctttgaacccgataggctgacttttcatccttaacgacaccatcgtagtcggactcttttaatggcttgtgtgtctcgtaagcgttaaataatttgtttgctaattcattttccttagttgttaattccatcgttgcttgttcatccataagcgtttcctccataaattgtatttaatctgtggatcctcaactgtatgtacagtgaggaccactcagtgacgtgaaatatatgtgttgttatgtcaatggcactatgtcggttaaaattatgtgtttgcaaaatctgaatctgaccagggttttcattggagctgctaatcaccgattccataagtcctcaccaccttaaataattaattaaattcaaataaaaaggcgtcctccaactacccgaaaatggatagttaaaaggacgcctattgcgcggtaccaccttaatttgtagtgctattactagcattacctcacacgtacagctttcgcgatacgctgacacaataatgggtgcacccaatgcgatctactaaaactttgatcacatagctcggagatgataatcatctaaggacgtaaattgcttcgcaccaaccagcaactctcttattacgaacggaaaatgacgtttctcttcatcgctttttaattttaatttaatgattgtcattaatttacaccctgttattttgattgtcaacagcaaatttgaaattaattattctttgttgggattttctcgaatcacgcgggcaggattgccggcaatgatgaggttatctccaaatgatttggtgacggttgaattagcgccaacgatgacattgttgccaagcgtaacgccggggagaatcaccgatccgccgccaacccaaacgtcattgcccaaagtcaccggtttgcccagacccacaaagttcgcccgttgtttgggatcaaggggatgataagcagcgtaaatttgcacgtgtggagccagcatgcagtgattaccaattgtcaccggtgcaatatccaagatgacgttatcgtagttacaaataaagttatcgccaacgtgaatattgtagccaaagtcacagcggaagttcggttgaacccaggggtcttttccgactgagccaaacagtttgcggaccagggcctctttttccgcaccggcagtgtcgtccagttcattcatcatcttacataagcggcgggctttagtttcgtcgttggttaattcgggatccatcaccaagtatggttcacccgctaaaaatttttccttttcagttgccatgtgattttccatcctttattgtaaattaatttatattatagcattatttgtaagtataaattgtctctaggcataatttattaggatgaattagaaattgccgagtgacttaatatcgggtatgataaatgcaattaataatagataaccaaactcacggaatttgaaaggatgcagacaatgaaagcagttattacagtgattggtcatgaccaaattggcattgtggcaaaagtttctcaacggttggcaactttgaaggttaacattaccgatatttctcaaacactgatgcatggtgattttaccatgatgctcatgggcgaatggaacgatgctgatgtgcagtttgaagttgtcaaacagggcttacaggatttggcaaatgagaccggcctatcgattaatattcagcgtcaagaattattcgacgcgattcaaaagttgtaggaggtcgccaaaatggaaaccaaacaaattttagagaccattctgatgatttctgaagaaaaacttgatattcgaaccatcacaatgggaatctcgctatttgactgtatcgatagcgatggtgttaaggcccggcaaaagatttatgataaattgacgaccagtgccaaagatttggtgaaggttgctgatcgaattgaatcagagtatggcattcccattgtgaataaacggatttctgtgaccccgatttcaatgattgctgctgcgtgtcacgatgataattatgtcgcctatgcgcagacaatggaaaaggcagcagaaaccctgggggttgatttgatcggtggcttctccgcgttggttcaaaaaggctaccaatcaggtgatcgaaaattgattgcttcgatgccggaagccttgagtgagacacaacgggtttgtggctcggttaatgttggttctacaagagccgggattaacatggatgccgtcaaacaaatgggccaagtggttaaagatttgtctgaaatcgatccggtcagctgtatgagtctggtggtctttgccaacgcggttgaagacaatccgttcatggccggcgcctttcatggcgttggtgaagctgataaagtcattaatgttgggattagtggtccgggcgtggttaaacgggcgcttgaacaggtcaagggggaatcaattgacacggtttccgaaacgatcaaaaaaacggccttcaaagtcacgcgaatgggccagtttgtcggtaatgtggctgctaaagcgctgaacgtgccgtttggaatcgttgatttgtcgctggcgccaacgccaagtcaaggggactcagtcgccgaaattcttgaagaaatcggtttggaaagtgtgggcgccccgggaacgaccgctgctttggcattgttgaatgatgcggtcaaaaagggtggcgtgatggcttgtgaacatgttggcgggctgtcaggtgcctttattcccgtgtcagaggacagtgggatgatcaaggcagttgagcacggtaatttgaatttggaaaaattagaggcaatgactgctgtttgttcagtgggattggacatggtggcagttccgggcgatacgccggctgaaacaatcagtgggatgatcgcagatgaagcagctatcggtgtgattaacaataagacaacggcggtgcgggtgatcccggcgaagggcaagcaagtcggagagcaaattgacttcggcgggatattcggctatgcgccggtaatgccggtaaacaccaatagcccagcgaaattcgttcaaaggggaggaagaatcccggcaccgattcattcgtttaaaaactaagagcgcgacgagacccggttgaccctggtatataagtgaaagacaacccctgatgaacggtctttgttcatcaggggctgtctttagcttatatgttaggggtcggggtcgtcggagcgtatctcaaaggccgaagggagcagtagataaaataagtgcatcaaaccttgtaacctacaaaacaaaatagaatcgaggagctcttgatgaacgtattttgttcatcgttgcctgcttctgcttgtacaatagggtcctgggtcgtcggagcgtatcgcagaggccgaagagagcagtaaataaaataagcaccacaaagcctggggactacaaatccttctccaccacaacacaaggcacgccgtcctcataaaacacatcggacgtgatctcataacccaggcgttgataaaatttgacggcgtccatttcactatgaatcagtgaatgagtgaaacccatttgtttggccttgtcttcaagggcactgacaacttttctgccatagccatgtcctcgcgcttcctttaaggttgcgactctgccgactttaagggtgtggtcattgtaagtttcaaaccgacaagtcgcgactggcactttgtcatcaaataagaccgcataaaccatgctgtcggaatctttgtcatcgaattcatctcgaaaggcgattccgcgctccaatacaaaaacggacattcgaatgtaagcagcagccccacgagctggtttggaactttccacgattaatttcataataggctcctcaaaatagacttcttgaactttaatattgagctggttatcatctgatttacgatacttctggaccggcaggccaatctttgccgacatcaacccaacggtcggcgtttgcatatttgctgagctcatcgacagacaatttgactgcgctgtgggtgtcacctgccgcagggtagatgaattcaaaccgctgaagggaaacgtccagatagactttaacgccttgattgagagcaaatgggcaaacacctcctggttgatggccaatatattcttcaacttgatctcttgggatcattctggcgcgcttgtgaaattcggccttgaactttttgttgtcgactttggcatcaccggccaacaaaaccagcagtgggtgggaatcaatcaagaacgacattgttttggcaatatgttccggttcacaatttaacgcttcagcagcttccataaccgttgcgctggattcatccaagactttaatgcgatcggctaagccaacctcgttaaagtactgtttcactttttcaaacgacatacctatcactcccgactgataaagattaagactaatatacaggttcacggaagaatagtaaataagatcttgattattccagaatgaaaaaaatgaatgggcagttaaggatttgtctgggactgaaaagtggctccagttctgactggaatgggaattccaacagctacaaatggccttttcaagctgccaatcctgatcgggacttaattaattgtcagattaatggtaacatgaaaccctatgatccaaaattatgagagaaaactgaagatttgtttaagtattgatttggcgagagcttttgctagattgaagtgctaaaacttcgtaaaatatgcttagagacagataaagggggttggcattagtaatgtcacgtaaagagaagttcgctaaaaagcctaagaaaaaattatggacacgaatcctggtggggtttgtgttggttctttttggtggcttcgtgggctctcatttctattttcaaaatcatttcaagttcaccaaaattaacgacgttgatgtttccggtttgacggtcgctcaggcaaccaagaagttgaatacctcacatatcgatgaagacggcaattatttagtggttcgggatttaaaaatcaatgtgaattccaaggatgttaagaaattattcaaacaccgtagttcaatgagtgcgatgacttctgccaagctgagtgccaagtctgatgtaaccaacaagcaactcaactaccgcttgaagacgttactgccgaagtttgaaaaccgggttgatcaaatcaataccggtcgcaaacagaccatcgattcaaaagttattttgaagaatggcaaaattgttgttcaagctggccagcagggaagcactctggataaggccaagatggtcaaagactttaagaagcaggcaaaatcgagtttattgatttcggttaaaatgactaaagatgcgtacgtcaagccgaatagtactcaaattgccaaacagaagaaacagttagccaacatcttggacaacaccgtcacgttgaatacctacaataagacctataagtttgttgccaaacgctgggttgccaatggttacccaactgctaacgggacctataagtttgattcaaccaagattaagaattgggtggcaaaatttgccaataaagtcgatacccttggcaagtcggtttggattaccactcatcaaggcaagagggttcgtgttcatgctggtggaacctatggctggaaagttaatcaatcggctttaaccaagaatatcatgaagaatcttggccgatcacattccgtcacaatgaacttgaagcactatgcggtcggaaccggttatggtgttaaggggtctggtaagacctatgtcgccattgacctgcagcgccttcacgaatacgtttataaaaacggcaagctgatggctaatattccaatcatgtctggaacgttgaccggtggtaaccgaacccctcaaggcgccttttacattatgtacaagcagcgtcacgcaactttgagagggaggaacagtgatggttcaaagtatgcatcaccagtcagctactgggaaccattgaccaattcaggggttgggatgcacgattcaccatggcagcccgcctcggtctatggtaatccaagtgctcgtgcacaataccattctcatggctgtttgaataatccaccgtcgcgaatgggtgaggtgtggaagaacacgcacactttggaacccgtatttatttattactaagaagtcaaatgactgttgacagggaatcgcctgccaacagtcattttttgatttaatatatgttaaactgatgataaatagcaaaacggggtgaacaatcgtgcatttatataaacacgttgatattagcaataaccgcaatttggtttatggtctaaatgtggtcgccgttattgcctttttaggcttcctgtggctgtttggtcccattgtcggctcaatgactgtcaacttcactgaaagctacttcgtttggctgatcgtggcattattagtgattgtgacgatccacgaggttttgcacgggattctttataaagtgtttaagccaaatgggaaaattaaagttggtttcaaaagtggcatgttgtccgtttccagccccaagtccctctataccaagcagcaatttatttggattggggcgaccccatttatcgtcatttcactcgtcctgattgcgatatttcttttgggatggcttcctggcgaattattcttaccgttggcagcccttcatggggcaggttgtgtcggtgacttttatcttttatggctggtgataagctcaccaaagcactattacattagcgatcaagaaaatggcatcgacatttattcccccaactgaattgttggatttcaacggtgtctcagatacaataaagggattgcaaccaaagtctgagctttggcggcaatccctttattggatggttaacgttaatcttggaccaaaattttaattcctaaatacagattataaatgaacatggccagatccaccaggataactaacgcgattagcgccaggaaaagaaatccagcaaaggcggccttttcggaaatcacaccactgataccgacaaccaggatggtcagcacaagggggattaaatgcaaaataagcgcgtgtctcgcagtgctgtgcatatctggattgttatcgctgacgatccaaacaatcagtggaaaaataaatggtgcgaaaacaattgaaagataggataaagcattaacaattcgatttgtcgacatgtgagtaactccttagtgattggaataggatttgtagaccggcgagcggaaaagatcgacgaatgcaccaccaccggaataatcccggagaacactgatcttttggccctcaacggttcggtgggtcttccgccagccacggtcactctgataggctttggtcgcataggcgttaaacgtgtaccggttcgtgccggagattttagcaaaagctaattttcgatagcccttccaagtggatttataaagggtgtgctgcttgccgttgtatttttgggtgactgagtacttgttaatctgggtcaaacagaacttcccgttgacgtatgaataccaattcccgcgccagctggtcggcgttgaactgtgaatggtgccaacatgataataagtgtcagcagcttgagcaggctcatgattgacgaaaacggtgaaaatgaaactggcagctgtgataacagcaaccttcaacaatttgttcatttaaattctcctaaaagtctccggatcaaaaacagaattattttgataaagttggctaattctttagattatactaaaaaatgatagcgtaccaagtgcggttttgtcaaataagcagaaaaaaggctcgctgactttggtcaacgagcctcaacaatgcaattattgtttatctttacttcttctgattggatgttctttttcttctttatcaacggacttttgatacattttatcgttgacgtacggataagtccacttaaccatcgctgacatgataattggcaaggtcaataccaaaatgatcaacccaacaatcacggtcatcgcaacttgaatcaaagtcaaaacgtttgacggaatcaacgcggcaaaagttccacccaagatgatggcagcggaaatgacgactgtcccaataatggttgccgaatttaaaattcgtcgacggacatccggaatggcgccggcatcaccacggtacctcatcatcaagaagatactgtaatcgactcctaatgccaccaacatgatgaaactaaagaacggtgtgttccaagtcagcatgttctggaacagcagatatcccgaaagccatttggtaatctgcagtgatcccatataggttacgattaaggtgccaataatggtaatggcttgaaccagtgagcgggtaaccaccatcagggctaaaccgattcccaccagcatgatgacaactgttcggaagaaatcgccattagcaatcttttgaaggtcagaagtttgagaactttgaccgccgatagcgaccttagcatttttcaaactggtgtccttcattttggcattcagatcgcgagtgattgtccgaatccggttagccgacttggtggtacttggatcggaattcaggaccacggtaatcttggtaatcttccggtcttttgacataaatgcgtcaagggaaggggtgaatgacgcactcttgatacttgcggcaggcatatagaaggtgttgcccaagtaagacttttgcatttccttcaagtatttgttaacagtggtggttccgcttgaaacttgatccaatcctgaattggcagaggtcaaaccagtttgtaattcctgcatctgactctggagctctttcattttcgaattcaatgtttgaacacccgaattaacttgagaactgccactagcgacactttgagccccggaaaccagtgatgaactgtttgaattcagtcgactagcgccacttgtaatctggttcaggccatttgagaacggagcaacttgtgaattcaagcggccaagaccggaagataactgtcttgatccggactgcaatgcggccatccgggcacgaagcgcctttagcttagcggtttggcttctcacttgagaaattcccgtgttcaatcgttgactgccagctgacaatcggccgacaccggattgaagactggaggtgcctgagctgagttgttgcgaaccgctggccaagttgctgacaccggcagtgtatgaggtgacgccttggctcagttgttgggcaccggcctctagtttgctggcaccatcagctaatttctcaacttgggcgatgctttcagaagtgtttgagttggctaatttttcgttggcactctttaaacctttttgaactttcttgatgccttgattggcttggtttaagccattagtaagactttccagctgacttcttaaatacagtgaattgatttttgttccacctggacgggtaactgaggcaacactcttgaccccggcttcagaattcaggtagctggttaattggtcgatttcagctaaatgttgttgggtatccagtggtttcttgttttgaatatagacggtcgtcgggccggacatcccagcagggtagtgatcctgaatgatgttataaccggcttttgactgaaccgagttgggcaattcatcggcactgttaaaattgagtttctgactgccaacgaacaacagtggcaaagcagcaatgattaaaatcccaaccataatgaaactgtgtgagagggtgaactttgagaggaaattccacaggaaacttcggtcatgggcagccaggttcttgcttggccaaaagagtcgttctcccaaggtagacatgaagaacatattcagagtcaacagaaccattaatagaatggcaactccgacagcgaccgcaacgcctgaacggtagaaagagaacttggccaatgctaaggccgcaaaaccaattaagaccgatgaaccactatacagaatggttcgtccggcatgccgccgcgcacttcttgcggcgtcggttgcgccttgacccttacggatttcctctttaaagcggtcatacaataaaatgttgtaatcagtcccaattccaaacagaactaccaccagaaagacttgggtaaagttggagattgggaaatcccatcgttgtgccaaattcatgaccacgtccaatgacagcaggtaggagacaccgactgtcagtaatgaaatgacaggaattaagaaggaacgaaagacgatgatcagcactatgaagatgaagattgccgcaatgatttcggtcttttgaagtccctgctcagtaaccgttgaaaaatcttcatttaagacgtcactaccggttacgtacgttctcattcccggcgttttaatcttatccaagattttatcagtctggccacgaaccttgtcttttttcggcacggtgatcatgaccatctgggtggtactgtcttttgactgcagctgctgtttggcagcttggttgtcacttggggctgtgaccgagataatgtgcaggtccgggtcgttcttgacggcgttggtggcgtcttgaatctgtaaggtctgctcatcactcaacttgccgtgcttgttattgaaaacggcgatgagggttctggcatttttgccgccctcatattttttctcaatcttattggcaacttcactctgcaccgaagcagggagctgaacagtccctttgtcatggaccagctgggaaatatttggcaacgtaaaaattgcgaccaaaattaggccaatccacacaatcagtgataacagatgcttctctttgaatttctgcattaaaattcttcctctcattccctagtgataaaattattctcttgttcaaatttagacacttgtataagcaatattaaaatgataaactcggcgtgaatctgacgcaagggacattttgctgcgttagtttaaatttagacaaaattcgataaatgcaaacagaggctggctcatgaaatatgacttaacaaagaaaccaacgcgtggtgcgcaacgaaccttggaatcattttcgacgacgatgatcgcgcttctctccaaagagccgttcgaaaaaattagtgtcaacgagatttgtgcggttagtaattttccccgggcgactttttataactactttgacgataaattcgacttggcagcgtattgctggtatgtaattgcccaagaaattgaagtggatcaggcgaccgaattgaaagctgatcgaacattgatcacgtattttgatcgactttacgacgtgttcaaaaataaccagacgttactcgataacgtgcttcagtacaatgatttttccggacagctggttaacagttttattaattactttaaaaataagctgcaggaaatcctcaccaaatcaattgattattccaaggcgggcctaccggttgaattgatcgtcgatcattgcagtcagacggttgtactggttttaaaatggatctttttaaagcatcatgattccgacaaacagcaggctcatgaatatttggagaagttgttgaatattgaacattttatctgaattgacacatcaagtgaatcattcaatgactatatagtaccatgaacgaccttttcgtgaattgaattttcatgaaaatatcgagcgaagcaacttctattatagcaaaagtggccttcatttgtgcgttaagttgagatgtgttagcatgctatttaagtgttcccaaagaatgcttaaatcagttcaatgatgaggaagtgacagaatggtcttaacttcagatgaagcagctgcaactaagcaggaactccaaggcaacttcgagttgtcagggatcactttgcaaatggcagccgttgatttgaaaagcacgcctgaacatattcaggacgttttaaacttgaaaaattgccaaaaagaagaaccttggattctgcgtaattacctaattaagctcattttgcttcaggaaaaagaaccctattcattctccaaattaataggggatcccaaacgttatcagtttttgaacagtcgcctgattgatcgtggcgaattggcctaaggttttaataaagtgaatgattgtgtcaaatgaaaacaatccaaaattagatccagttaaaactgcttgaatttcagttttaactggatcttttatattactccgaggatgaatgttgggacgtcggctaattattgctatatattgcttaaatggctagaatcaaaaccgctcgcactcgcctgaatcccaccgttgtttagcttaaatgtgtgaaagaggacagcaactaaattttaagcctctccagccaaaaacctaactcggtttccttgtgtctcactgttatttggatgaaatgtgtgcaagaggacagtaattgaaatttaagcgccgccacccgaaaacctgactcggtttccgaccagcggcgcttaaatttcaattactaaacgtcctctttcacactctcatcttgaagtggtcacatcactttgcttaacccagccattgacttgaggatgggcagcgtctgttacatagtagtatgtggcattgccatcgcgattattttgcttggtgccgaccttggtcacggtcagtggatccttgtaaaagtctgccgttgcgctgagattgcgccccactttatattgggtatagtcaggggcaacgtaggttaacgtggaagcttttggtgtcgtaaagtacattgtggtgttggcaaaataagttggcaccgttgattcctggaaggtcgtcgttgcctttaagccaccggaaacatcactgggattgattgtcggatcggttgttccggcaaatatccagccccgataggttttatcgaaggaaacaactttcaggtaccagtcgccatttgaggtctgagctgcccgataacctctgaagtaggtttgcccggcatcggcagttgtgccaagggtctttaaaacggctgccttggtgacaacttttgcactcttatagaccggcacttttgaatagagtggtgctgttccggttgtcaggtaattacgggaattgccatccgccacgagcgcctggttgctggttacagtcgtcgttgatttggcctcagtgttggttggcgttagggtaaatgcgccgatggcaagtgtcaggccaagtcccaatatgagtttgctggtgattgttttcaaattaatccctccaagcacaatctttattcaaaaagtatacacccatttgaaaatgaatcatacaatcgaagtcaattaaattaaaaaatgattagtttattttcgaatgacagttgataaaaatacatagttacctgatatacatcaccaactccattcattgaacagtttactgattagaatatttttaattttaagtatattttcgaggccattcgttgtatcctagttgtaaatattatttaaaatagtggatattcatacaaggagtgacgacatgaaaaaacacgaggggttattttcgcaagttcgctggttgttcattgtgatcgcatttgtcggaatggtgatcggcctgaatacacaattggtgcatgcaaaggccagttcgctggaaacggatttccaacgagcggctgccaagtaccaggtgccggtagatctgcttaaagcggtggcttataatgaaagtgcgtttgatagccacaatggtaagcccagtgtggccggcggctatggtgtgatgcatttgactgataccactggcttaacgccaagcggctcagattccaaagcggttaaagtgccaaataccgcttctctgcatacgctgcaaaaagctgccaaattgaccggtcacagtgttggtcaactgaagaccaattcagctgccaatattgatggtggggcggctttattagcagcctatcagaaatccttgggcaaagggctaacgtcaaatattggtagttggtctgcagccgttaagaaatacagccagtcggattctcaggcagctgctgatttcttcgccgccaacgtttataaaattttggcaaaaggcgtcaatcataacggcgtcaaaatctcaccccagaaggtgaatgcattgaaagatgaagcaatcgataccaccggtgaatcgggccaaaccgatgggcctgccggcctgccaattgaatggattcccgcattatacaaaacctttgatgatcaaggcgactacggaaactatgatctggctgaccggccaaacgacgaaaagattaattatatcgtgattcacaacaccgaaactagttttcaagaagcactgacactcttctcgacaccgacgtataccacggcgaactacgttgtcagttcggtcgaagggacagtcgctgaaatggttcgaccgcaaaatgttgcttggcacgccggcaactggtacattaattctcattcaattggcattgagcacgagggttatgcggcagttggcggctactggtacaccgaaaacatgtacaagtcctcagcagccttggttaaatatctggctgataagtaccagattccgctggatcgtcagcacattatcggccatgacaacgtgcccggtttaacacctgcagctcaaaaagggatgcactgggatcctggaacttattggaactggaatcactactttgaattaatgggcgttgatttatcaaaaagtgacggcagcacggatagtcacattatcaccattacccctaatgacaagacgaatttgacggccgattcgggacaaaaagtgactgatgacggggtcaaccttccgctagccggatcaaattttgtctacctctacgagcaacctagcttcagtgctgatttgatcgccgacaaagacttttcttccggtcaatccggcaccactgaaaaggatgactggggcgataaagccgtttacggccaacaatttagtaagatcgatcagcagggggattggacagaaattgattatggcggtcaaggtgcttggttctacaatccgggcggtgctaattcaactgatgccactgggaagctcgtaacggctaaaggatcaaaagccgtgccggtgtatggcagtgcctatccaagcgacagtattttgaagaagaataaagttaccggcattaagccaacaccaatttatcaactgcagccaggtcaaaaatacgtttatggcggcacagtcacctctgattacttcaattcacacttcaattcaaactcaccgaagaacgtcattcatggcaccgatgattattatcagattcaatttaatcaccgaattgcattcgtgaaggcgtcagataccactctttcagacgattgacagattaatcgatagcaagtgaataacttggaaaggccgaaacagcaaccaatgtttcggccttttttaatcgctattaatgtcatcaaatatcacatcggccaaaatttgctcattttcccgcaaaattctgataatggtgtcactaggatgtgaggtattggtatacctgtaatttgaggagttttaacgaagactgttgactttctgaaaaatgggtatatattaatacccgtaagtaaatgtcacaaaacattacatgaaatgagggaatagaatgagaattgagagagattgcatcggagaaatgtttgtacctgataacgtcctttatgggattcactcactgcgagcgaaacacaactttccaatcaccaacgaaaaagttgatccagccatcattcaaagctatctgcagattaagaaggccgctgctttggctaacgagcaggccggcaccttggataaagaaaaaagtgctttgattatggctgcctgcaaccaattgctattctcaaatgactacagtgcctttatcgtgccagccatccagggtggtgccggaacgtcaaccaatatgaacgtgaacgaggtcgtcgcccagcttgccatgcaattaagcgcccagggtggaaaagagcccttggtaatcaagcccaacgatgatgttaaccagtcacagtcgaccaatgatacctatccgacggcaggcaagatggcgatgttaaaacggttggcgccattgacgtcagctgtttccagtttggttgacgccttaaccgataaagccgcagaatattcgtcagcaatcaaagttggtcggactcagctgcaggatgctgtgccaacgacctttggcaggacctttacagcttatgcttcaatgtttaaacgcgatctctcaagattaaagcacgctcaaaaggttctttctcaagtcaacctgggcggaaccgcgattggtaccggaattaacgcgaccgctgaatacgaatcagccattattcccattctcaacaaatattctcatctttcgttgcatcaagccgctgatttggtggacgccactcaaaacagtgatgctttcaccacgatttcttcggccatgaagtcattagctgctgatttatccaaattcagcaatgacttgcgactactttccagtggccctcaagccggcctgaacgaactggagctgccaaagaaggctgcagggtcctcaattatgcccgggaaagtcaacccaatcatccccgaagttgttaaccaggtggcatttgaaaccatcggcaacgacgtcacggttacaatggctgctgagagcgggcagttggagttgaatgcatttgaaccaatcatgttcaagagtattttgactagtgagcagcatttgaccaaggcaattgagacgctggttgaaaactgcgtcagcggcatcaaagtcaatgcagcatattgccgaaaggaagtcgaacactcatcgatcgcggcgacggtgctttcaccgctgctgggctatgaaaagacgaccgcgttgattaaggaagcattagccactcaacaatccgtcaaagcactcgtcaaacaaaagcagctgctcccggattcattggtcgatagtctcttcacgccagaagttttgacgaatgttcgcagagtcaagaaagaaaagtctgctgccggttcaaatttaaattaaccacgttttaccgaaagtcagcctgatgagggggggctttttctttttgaccaaaacagaatcatcaccacgctctccaatcgcgatataattgagttggttaggtcaacaatttgaaaaattggggtgatttgacaatgaaacagaataaatcaacgctgattgacgatgatgccaaggctgatcccactgatttgatgaaccagtttcaaaccagtaatggtggtctctcgcaggcagaagccgagaagcgtttaggaaaatatggaccaaatacgattcgacagggcaaacgaaagtccgaagtgttaatctttttggaaaactttacctctttgatggcgattcttttgtgggtatccggtgtgatcgccatgtttgccggcatgctggaacttggaattgccatttgggcggttaacgtcatcaatggttgcttttcatattggcagcagcacgccgctcaaaaggcaaccgactcattgaagaaaatgctgccatcttatgttaaggtccgtcgggatggcaagtctcagcagattaaagttgaacagctggtgcctggcgatatttttgatattcaagcgggggattcaattcctgctgacgccagggtgtttaatgctgccaacctccaagttgacgaatcttctttgactggtgaatcggtaccggttgaaaagcatgacgcttaccaacacggcgatggcgaatttgctcaacagaacatcgtctttgctgggaccatttgtaccagcggcactgcgacagctctctgcttggcaaccggaatggatactgagttcggccgcattgccacgttaactgagtcacagaaaaagaccgtctatccattggaacgggagctcaatcatttaacccggcaactaacgattattgcgattatgattggcgttgcctttttcctgctggcaattttcttcgttaaatatccggtgaccaagtctttcatttttgcattagggatgattgtcgcctttatcccagaagggcttttgccgacggtaactttatcgttggcgcagggcacccaacgaatggcgaaaaaacatgcactgctcaaaaacctgagtagtgtcgaaacgttgggacagacgacggttatctgctccgataagactggcacgctgacccaaaatcaaatgactatcaaccatctgtggctgccaagtcaagaatacgacgtcactggaaccgggtacgtcaccaatgggcagattcagttaaatggccaccaggttgatctggcaggacagcctgacctcgagaagctgttgattaatgcaaccatcaataatgataccgaggttactgaaggtaaagccggtgaaaaatcaaaaattctcggaactccaaccgaggccggcttagtgatcctgtcacgcaaagcagggattgatgccgccgccgaacgccaaaagtttcccagattaaaagaattaccgtttgattctggccgtaaattgatgtcggtcatcactaaaaatgcggacggtaagttggtcatcaataccaaaggggcgttaggcagtgaattaaacgtttgtgaccggatcttagataatggtcatattcgacctttaacggctgatgatcaggctaaaattatgcaggtaaatgaaaattacgccaaacaaggcttaagaaccctggcgttttcgtatcgggtggtggatgaaaatgatccactaagtcagcagtcacttgaaagctgcacgattgaaagtgctgagaagcagatggtcttcattgggctggcaatgatgtcagatccgccacgaccagagatctttgatgctgttcgcaattgtcgacgggccaacattcggatcatcatggttaccggtgatagcccgacgactgccaaaagtattgccactaagattggcattacttcggacaaggtcagagtcatttccggcgccgaactggataagatgtctgatgccgagctgcaggaagccgtcaaaggggaagccatttttgcccggattgcaccggaacataaatttaggattgtttccatgtgccagaaaaatggtgacgtggtggcttcaaccggcgatggcgtcaatgacgcgccagcactcaaacgtgcggatatcggcattgcgatgggagtgactggaaccgacgttgcaaaagacgctgccgatatgattttgaccgatgataactttgcctcgattgtcagcgcgatcgaagaaggtcgggccgtttacagcaatttgcagaagttccttctatatatactcactagtaatgttcccgaagccgctccatcggtcatcttcttgttgacccgtggactggtgccattaccgttgacggttatgcaaattttgacggttgatttgggaactgatttactgccggcattgggactgggaaccgagaaagccgagccaggcatcatggatcagccgccccgtccattgaacagtcacttgttgaaccgatcaattatctggaaagcctttggttggtacggcttgattgcctcggcaatttcgacgtttgcctacttctttgtcaaccacgtcaatggctggcctcaagtacccttggccggatctggtttggtatacgcggaagcgacgacgattacattggcagccattgtcttctcccagattgcagcggcgatgaactgccgaacgcagatttcatcagtcttttcaattggattatttagcaatcaccgcattcttttggggatcgtcgtggaagttgtcttagtcgcactgttgatgtatgttccatttctccagggcgtcttcaacaccggaccgctaaacgtcacagaatggggcttcttattctgcattccggtgccgatattcctggttgaagagctgcggaaatatgtggttcgccagattaaaaagcgacgggcgaagatttcagtctgataataatgttgcatttacaacaaaaatagtttagaatcaattctatcaagaaagggctgattaagtggcagagattttacgacccatcggtgcgattgccagagccttggattcaattgccaacgttgaatttaaacggtttgatcttaccaagggccagtatttatatttggcccggatttgtgagcaccccgggatttttcaagaccaattggcagaaatgatcaaggtcgaccgaaccacggctgcccgagcaattgataagctggcggcaaaggactttgtggttaaacggcctgattcgaccaaccaaaagattcggcgcttgtttccgacagaaaaaggacaggcgacctatccgaatattttgcgggagaatcagtattccaaccaggtggcgctaaagtccatcaccgacgatgaggccgaccaactggaacgccttttgcataaagttagtgccaacattgacgatgactggcattatgttaaaaaaggcaatcttagaaagtattgaggatgaacttgtgacaattgtgattagaaaatgtactttggcagatctttcagaactgcagcagatcagcagagagacttttgctgacacgtttggtccggaaaatagtcctgccaacgtgaatcagtatttggatgaatcgtataatcttgaccggctcaaacaagaactcaccgatgcggattccgatttctttttcgccttggtggatggccaagtagccggttatttgaaggtcaacgtcggcaatgcccagacagaagcgatgggcaaccatgccttggaagttcaacgcatctatattaagccagctttcaaacggcagggaatcggatcgaaattgatggctcaagcattggcggtggcaaaagataaacaccgttcgactgtttggctgggcgtttgggagcataatcttgtcgctcaacagttatatcaaaaatttggtttcaaacaaactggcgatcatgtcttcacgctgggcgagagccgccaacgcgacctcattatgagccgaacaattgaaggagagagccagcattcatgaaaaaattcattttagatcccaaaaccatcgaattatttccagacatccatattgacgtgatgaccttacatggcatcgataatcacgtgaatgaaaaggacgacccgtatttccagaaactcctggatgagggcaccgaggcggccgaacaatttatcaccgtcgacccattccgtgataatccggtggttgccgagtggcgggaagcattccggaagtttaaaaccaagaagggcgcccgctcaacgattgaggccttattaaaacgggtcagtcacggaaaacgattttcaccgattgcaccgttagtcgatatttataacagccaatcactgaagtacggagtctccgttggtggtgaaaacgtcgacgccattgctggggacatgcacctgggagaagccaagggtggcgaatccttcctgccatacggtgagaccgaagatatgccggctttacccggtgagatttgttatatggacgataaaggcgcagtttgtcgttgctttaactggcgcgaaaatcagcggactgaattgaccgaggacaccaccaatccgatcatcgatattgaatcgattaatgaggatcagtcggcccgctcagatgttgccatcagagaaattcaacgtctctgcaaagaatattttggagttgttggtcagcttcaacaattgaatgctgaaaatcctgagattgtcattgctaaataaattcaaaaggcggttatcacattcccttgcttggggatgtgacaaccgcctttaattttggttccgagcttatttgtgatacttgtcggcaatattatacttaatatcatatcaccgctatcaactttcagcaaaactttctttttatcatgcttatcaattactttgaacttagcgtaggcctgattagcgtaaaccttgtggaaagccttcgaacggttacgcgagcgattaaccaaatagttccacttatcgggcttaccagccttgagttctttgactgcttggctgttctgactgaccttgatggtaacgcccttgttcttatcggcttcaacggatggtttcttgccgtagggcgtcttatcttgggcattgaacagatactggttcagttcacgagccaccgttttatgacccgggccatcctgtagggtgaatagactgccgacaaaataaatgacgagcgcggcagcaaccagtgagataaacttgccaaccggtttttggtaccacttcataaattgttcaacatctttattctgaacttcatcttcttcaagccatggctgcttggcgccacagtatggacaaaagtttgagtatgccgggatggttttcccacacatgacacaggacttagtcttttcttcagacatttctcatgctcctccaatatgtacctttgcgaatataccaattaattatagcaaagatttgcttggtgggaacaggtaagtgcaaaattatcgttaattaggcaggtgtttatcgataaattctttcaccggcagccggaaatcgaggtaatatttctcaagatcctctctagaccaattccaccaggcaattttttccatatcggttttaatttcgtcagggaaacgatccttaattggtttggcagggatgccgccgacgatggtgtagggctccacgtctttggtcaccacggcacctgaaccaataacggcaccatcaccaactgtcacgccagcttggatgatcacgccgtggccaatccagacatcgttgccgatggttgtccgcaggtgggttcttttttccaagaattcggtgtctggatgatcgaaaccgtaagcgccgccgttataggcaaagatgtgttgggcaggccggtcgtagggatgattggtcggtccgattcgaatcatcgctgccatactgatgaactttttcaagtcactgttttgaataaaacaatattggccggtgtaggtataatcaccaattgaactattatcgattaaattgctgcttcctatttccacccattccccgaatgtagtattcttggtttgagtcatttttccaatcgttggtttatcttttgacaactttacaaaatcaatatgcatacgaccaacctctttctcaaaataatttctaaaaactattataatatgttttcacactatttagttaaaaggagcttacaaatgtttgaagtaaagactattgatcggtttgacctgaccgattttgctggagacgtctttcgtacctccaacaccgataccccggatgccattttagtgcggagttccaaggttgatgatagcttgatatccaagcgattgctgctgatcgcccgttccgggactggcacgaacacgattaacgtcgatgcggcaaccgccaacgggactgccgttttcaacacgccgggggttaacgccaacgccgtcaaagagctcattattcaaaaccttttcagatgtctgcgtccgctgaatggtgccgttcaaatgatgcagcagctcaaagttgccccgggtgaggatttgcaggccgctgccgaagccaaacggggcgattttattggcgaggaactttatggacggacacttgggatccttggcttgggaacgatcggccagcggttggcggatgcctgctaccacatggggatgcagattatcggctataaccgcagcttcaagaatctacgtcacgtccagcaattggataccattgatgaagtgttagagcaggccgattttgtggtgattttactcccgctgaccgatcaaaccaaccagctgttgtctaccaagcaatttgaaatgatgaaggatagcgcttatctgctgaattttggccgcggcgagattgtcgataatcaggcggtggtctcggccttgaatcataacgagtttgccggttacgtgtgtgactttccgaaaacggaactccaggatcatccaaagattactctgctgccacatttaggcggcaatacgattgaggcgctgacccattctgcaaacttgattttgcagaacctgctggactttttggaatatggcaccgtcagaagctcggtcaactttccccgggttgatttgccgttcatgagtaatcaacggctgacgtttttcttccacgccagagacacattctgggtggatgttgccggtattatgagtcgctatgacttgccggttcaagaaatgatgggaaacaccatggacggttatggctatacgattgtgaataccgatttggcggaaatcacgcagcaacaaacacagactttgttaaatgaacttaatcagattgacgggatgattcgggtcaggttgttgaacaacccaacccagggagaatggcagtaaactttagtaagtgtttcacaaccttcgaacttttttgaaattatgagactgaaagtgggagtacgggtctcgtgatttgacgagctcgtttcacaaataaaaagcaaaagaagtattgaaattaattttcagccgcctataataagcattgtaagcggttgttagttaaaaaagcaaatgattaattcacatattcgcactcatttaagcgctggataatcatttgcttttctgttgtttgcaattgctcactaaataacaaatatagtatttggagatgtgattatgcgaattaaagcagctgttgttaacaaaaaaggcggagacttcgaaatgaaagatgacgtcgaattagcagatatgcaggctgacgatttacaagttcatatggttgccagtgggatctgccattcagacgaagctttacgaaaaggaactgccgaaattggttacccaatcgttcttggccacgaaggatcaggaattgttgaaaaagtgggccctgaagttaaagacttcaagcccggtgatcacgttgttctgtcattttatggctgtggcaactgtatcaactgtttaaagggaattccaacccaatgcttgaattacgcagcaaacaacttgtcaggtgttcgtcctgacggtagtgcccactttactgaaaatggtcaccaagttgccgacatgtttgaccaatcctcattcacgacgaccactgttgtccgtgaacgtaacgcggttaaagttgataaggacttggatttgcgtcaattaggacctcttggctgtggctatgtcacaggtagcggcacggtcttcaacactttgaagccggaaccaggttcaaccattgctgtctttggtactggagccgttggcctggccgcaatgatggccggccgaatttccggctgcaccaaagtcattgccgttgatatcgttcctgaccgcttgaagttagccaaggaattaggtgcgacagataccattaacagtaaagacactgatccggttaaagctattcaagatttgactgacggctatggtgttgactatgcggttgataccactggtgttaaatctgtcatggaagcatcaatcaaggccttggcacaaggcggcaccactgcaacaatcgccgttaccgaccaacacgttgatctggatacttggaacgatctatgtgtcagcgaccggaaagtcgttggtgtcaacatgggtgactcaattcctcaagtcgatatccctcgtttgatcaagttctacaagatgggattgtttgacttcgacaagactgaaaagttctacaagttcgatgatattaaccaagctaacgctgattctgtcagtggtaagacgatcaagccagtactggttattgacgaagactacaagcctggtaagtaacacgtttccacaaactcacatcaaggcatccaaaagtttcattaaaacaataaaaatatttgttcctgccagatggcgttcaattacactgttttcgacaggtatcttgaaagggagcaactattatggcacaaaatgctgttgcattaaaacattatcaaatgtacattaacggaaaattcatggattcaaagtcaggtaacgaaattactgttttaaacccatcaactggtgagaagatttcgacagttccagctgcaactcgtgaagaggccaaagaagccatcgatgctgcatacgaagctgaaaaatcatggaagaaagttccagctgctacccgtggtcaatatctacacgatgttgccactgaaattcgtaacgagaaggatcacttggttgaaatgctccaagaagagcaaggtaaaatcaagtcattagcaaccactgaaatcatgttctcagctgactatttcgattacatgggcagtgctgctcgaacttatgaaggtgaaattcttcaatccgacaacaagaatgaaaatatcatgattgccaagcagccaatcggtgttgccgccggcatcttaccatggaacttcccattcttcctgattgcccgtaaaatgggtccagctttggtaactggtaatacgattgtgatgaagccatcttcagacacaccaaacttgggacttgaatttgccaagattgttgaaaaagttgggattccaaagggtgttgtcaacattatttcaggtcgtggctcagttgttggtgacgaactcaccaagaacaagaagatcggcattattagtttgaccggttctgttgattctggtaaacgggtcatggcaggtgctgcaacccacatggctaaagtttcattggagttaggtggtaaagcaccagccattgtctgcaaagatgctgacattgatttggcagttcaatcaatcattgactcacgtgttgataacaatggtgaactttgcaacaactgtgaacgggtctacgttcaggaagatgttgccgatgagttcatcaagaagttatcagacaagatgtcaaagatcactgtcggtaacgttatgaaagatgaaaacgttggtatgggtccactgattaaccaagaagctttggacaaagtctctggcatggttgatcgggccgttcaagctggtggcaaggtcacagccggtggtcacaagttgaacatcgaaaatggcttctactacgaaccaacggttatcaccaacgtcaaacaagattcagaaattgtgcaagacgaaatctttggcccagtactgccagtattgacctttaagactttggacgatgccattgaaatggctaatgattctgacttcggtttgacttcatcaatctacaccgagaacttggacaacgcaatgcgtgctgccaacgaactcgaagatggtgaaacttacatcaaccgattcaactttgaagctatgaatggttcacactcaggctggaaagaatcaggtatcggcggcgatgatggtcgtcatggtatcgaagaattcttgaatactcatgttatttacctgcaagggcatccggagaaggctgaaggctagagcgtgacgagggccgggagaggcggtttctaagggtactttgattgaagttcctgggtttggaactttaattaaagtgcgcttagaagttagcctctggcccgtcggagcacattttatccaaataacagtgaaccacccaccaaaaaggcacccacagcaaacgcacaagaaagtttgtcggtggatgccttttatgtatgactaaaatagctgaaatccgaacgaatattaaccgatgtgataaatagaaaaaatgacactcccacaccatcctggcatataataaagccaacaaacccacaggaggcagacacaatgacaccatccaatatcatcggcgggatactaacatgtggtgttggcctatttttgattgtcgcaggcttaatggtgagcaggggaaaatggtcaggaatcgttgctggaaatcttttccgcgatgatcaaaagtcggttggtcggcataagaaagccattggtattttatatatcatcctcggcgtcctgtgcctagtcttttattttgttgtctttttgaaagcttgaaggttcatatcatatcccatcaaaatagcggcctgcactggtctcaaccaagcgcaggccgctatattatacatacagtaaagattgaatcattgaaccaggtaaaagacgccactgaccccaatcaacacaaacacgcatttttgaatcattgagatattcatgtggaccgtaatccggttggcgatcatggttccgatcacgccaccgacgattcccaacaatatgagggggacgtcaattaaacctaaaataccgttatagaaacgaatacttgtgatatacaattgatcaatcaagaagaaagcctgaatactggcgagatattcctcttttgtatctgccaaggacaggaagtagagcgccatcaacggtccaccaattccaaacaagccgttgaagaagccggaaacgatcataaagataatggcaatataaatgggataatgtttccggccttctgatttgacgaacaaaaagtacagtgagagggcaaccaacagaccacccagcatggatttcagtaaatggacattgattgagttgactagttgtaatgccataaaggccacactggcatagacgacaaacggccagatgattcgtttgaattggatgctgtgccgataacgccaagccaacatgatgttggaaaccgacataatcagggatgcgaccccggcactttgggggatgggcaagattgtcggtaaaaagaccatcaagacaattgctgagccaaatccggtaaccccctggacaatcccagcaaggacagcgggcaggagcacgaatatgaaattagtcatgaccatcctcctctcaagtcatctccgttacgagacgtgtgataagttcctctgagacttccggtgaagctttggtgattgtttggtgtaaagttttcgggacataaagagcgcgacgaccaagaaggctaaacacatggtaaagccggcctgaatgcccatttgttgataattggcgtggccagcaaaaaagtgactggcaatgttgatggtggccacaataatggccgttccaaacgatgccgcgatttgtcgcaaggtgttgaaggcagcgaccccgtcagcgattagttcattggggagataggatagtgcctgggtctgaattggaatgagaattaagaccagtccaagctggcggattgtctggcccattgtcaacatcagcaccgaagcgttaacgtcaatgaatgcctgcatcatggtaccaaaacaatcgattagaatacccgtggtcacaatgatccgcaccggataacgatcgaacagccggccactgattggtgacataaaaccagttagtagcgctcccggcagtaaagagagtccggagatgatggcactcttacccatgatcgtttggattagcagcggcaacagaatcgtattaccatacatcgtcgagacaatcagtgagttgaccaaagtggcagtggtgaactgactgtttttgaagacggccaaattaacaaacggatggtcggattttccttgagtgacggcaaacatcgtgattaagacaacaccgacgacgaatggcagccagactgttagagatgtgatagggaactgactcacgtttgaaaaactccatagaagtcccagtaaaccaaaactgatggtcatcaggccttcggtgttaaattgaggttcctggttagtagggatcttgggcagggcaatcgtggccattaccaaatcaatgacgataaacggcagcaccaaaatgaataggtagcgccatgagaaatagttcaaaataacaccggaaagtgttgggccaatgatcggcgaaaagttaaatgccaagccgacgattcccatcacggcaccttttttgccgggctcggcgtagcggattgccagggtatttaccaggggcatcatcattccggcaccgattgcttggatcatgcggccgatgatgagagtgaagaaattaggtgccaaggcaccaaaaatcgttccaactaaaaagacgctgacgaaaaaaataaacagagaacgaaatgtgaacttcttggtcagataagcactgaccggaatcataatcgcgttgaccagggtgtagccgttgctaatccattgaaccgtaccggacgaaatggcgaacaccttcataaaggttggcaaagcgacattcatgagcgttgaacagagaatgccgaagaaggcaccgaagatcataatgatgagcgaataacgattttgctttgacattaacaggacttccaaatatgtattttttgcatttcgaaaaatagcaactctaaatagtgtaattttaataatggataattgcaataggaatatagttaatcactaatcgcagaataaataaaaacgtggaattgtaatcatgcaattccacgcttttattaagctttcttagatacccgataaaagttcggtgaaaatggcgtttctgccgcaatgttactaccgtcataatacacgtgaacgtatccgtgaccaactcgtttgaaagtgaatcgggcctggtgcaatttgttcagttcgtttctgccgacgatggtgtaggcggttttaccaatcgctttccatttggtatcggtaatgtgccagcccgctgactgcgttaaataggcattcacactacttttacgaacccggacagattcatagctatcaaacttcttcatgccaaagtatttaccgatgttaatcgttttgtctttccagtgaccgcgtagtgctgttggggttcccttgtgccaggttgccgcttgtgttgatgtcgttactgctcccaaaaagccaagtgacgcaatcgccgttacgattaactgcgtgcctttgttcatgactgtcatctccaattaatttgcttggtcaaatttattaaccaattgaatgaccatgcttggctcactgccggggactgcccgatagacgacgtagtctcccggaaccaaatcaacggatgccagctgggctttttgggcgacgctaaagccggccacttcgtagtaggcgtgaccgtcgacgtcttcgtcggttaacgtgacgttgacctgttcgagtggggcaacgtctaaggatgcccggcgtaatgccaggtactggtagttgatcgagtcaaccataatggtgatttcattgttggtgcagggaacgctcatggtctgtttcaaattgatttacttccttctttgagtttcgcgtggcgaatatcattgacattgatggtcaccagcttgtcggtttgaagatagattagatcaccattagtgccaattacaatgccacttatattataaacgtttaagtagccgtcatcatttaattgaagggtaatttgtttggaattctgccaactgtcctgcaaaacgcggtcgatgacttccggatcctgttccggcaatcgatgagtcgagacctcgtcgacttttttgtcagccatatcctgggtatggtcactcaaaaagtaacccagccacttcaccatgccgcggtcgttgtagagccattggtcgcgtggaacgtctcgaatcatgttgaacacccccatacgtttaatatacgaacatatgttctaaacgtcaaggggaacagtttaaataaatgaagcctggagccgaagtgattgctggccttgggattgggaaaatgttacagtttatttggctaattcacaatttattcatatttttaggggacaatgaatttataaaatacattgaataggagtgaagcaattgcgcacggtctatattttcaccatcattattgcgtcgatcgtcatgtttttgattgattactatgtgtcattaccacatgtattgtgggcttgtacctggttgggattcattgtaatcgttggaatttgcagttatcaaataatggctcattggcataataatcaataaaattaaattcgaatttgcttctcatccgtcgagatcgggaagcccttcttaaacgcagtccgcaagaagttaagcaggggcggagttacctttaattcgtccaaatcccgcaatgagaaggtatagcgaattgccttttcatcaccagcttcaactttttggacccacttgggctcacggatcaactcacggcccatggcggcaaattggacgccggcgtcaatcaacttggcaacttgagctggggatgccaaatggccgacaaccatcaatggtaaatcatccgccaggactgcttggactttttcgaagagcggctgctggtcatcgcgatcgacaattgatccctgccaggcatccgccaatgacatgtgcagataatcaattggcttttgattgagttctttcaccaaggccagggtgtcggtcattctgataccaggcttttccagttcctcaggcgaaatccggtagcccaagataaactttgggttatcagaacgcttgatgacggctgcgcatgcatcaacaaccgccaaagggaagttcatccgtttttccaaggagccgccccagtggtctgttctgcggttggaatggggactgaagaattgctgaatcaaataggtgttggcaccgtggagttcgacgccatcaaaaccggcgtcaatggccaattgagtggcgttggcgaagtcctgaatggtctgctcaacttcttcagcggaaagcgcccgaggggtttcggcacccaagcgttgtggagcgaccgcgctggcagagacggtttgatggccgcgcagtacccgcgagttactcattcgaccggagctgaagatttgaagaattgctttggtatgattgattttgatggcgttggcaagccgcgacaacccgggcagcatgttgtcatgtgcgacactgagttcgccttcaaagcctttgcccagatcattgacgttggcgcagccggtaataatcatgccggggccaccggcacgcaatcggaagtagtcgatttcgtctccggtgatcgaaccgtcttcaaaactggacatctcggtcatcggtgacattgcgatgcgatttttaatggtgacaccgtttcttaattgggttggttgtaggaaattatattttgtcatatgagacctcctgatgatgattaataccttgagtgtaccaaacaaacctaaaatttccaggtgaaaatgtttggttcattttcctaaaaaagcgtttacaatagaagtggaaacaaaattggaggagtgatagttgatggaaacattgaaaatgattcagtcacgtaaagcagttcgtgagtattcgggccaagtgtccgatgatcagctgcacgaaattttggttgcagccaacgccagtccggttgggatggggcgctatgatgattatcgattgacggtgatccaagatccaactgttttgtcaaaaatgactggcatttatgaagccccaacggtgattgtggtttcagtgaaggaagagagtgcctccgatgagatttcagccggcgcgatcgttcacaacatggaattggccgctgaagatcagggattaggtgccaactataatatggccagtttggaatccattccaagcggagtcgttccagatggttttaagccggcatttgccttgacccttggccagaccaacgatacattcacaccacgggaaattccgttggatcggattaagacaaatactgtgaaatgatattcaaaaaaatgggttagctctcaacgatttgttgggtgctaatccatttttgatttgacagttaagctggggattctttatctgacgaattgcgggtcgtggaccggttataattccccgcctttttcaaaggttggtaccatcttttcagctcgcagcaacagcaattgatgcagcaaatccttcacgttctcagtaattgcgtgagcgatcttgtcgttaacctgattatgccactcaggtaacttgtccttggcaatgtttttaaattctgcatctgcagtcgccactgcagcccggccgttggcaaagccaaacttgcggctttcagaaaccgcagtcattgcttcgagatcatgctcggcaaagaaggggtcagccaacatggcaaccaacttattcagccaataaaagctttctgtcgtggttcgcagcggcgtgtgcttaaagttatccggggtatcagtgcagttggcaaagaatggtactggcgcgttgaactcattgacaccttcggccagccaatgaatggcggcgtgttcggctggaaaatcgggacgaatttgcaggatatgtatctcttggttgcggttcataccaattggtcgatagcgcaaccgtgattcttcagttccggtcttcccataaggatcaaactcggtgccttgatagtggctgctcaaaaagaaggcaatgtcttcaactgaaatcaaatgatcggcaactctggtaaatggcattgtccgactttcgggattctgctggatttccgggttaaacattttttgaccgtaccaaacccgcggggtgttgtagtagtgatccgcttgaacgtcctcaccgaaaatatcacggaagttaaagccggaacgggccttgttcaagtgatacttatcggcaaatgctttcaggtcgtcgctgtacatatagtggtcaggatcatcaaagttgatttcttgaatgccggtttgattaggtgcgaccgcataagcgtcatccggaattcgttcggcagcccaatggtgcccaccgactgtttcgaagtaccagacctcatctgaatctgaaaaggcgatgccgttgctttcacaagtgccaaatttggtgaccaaatcgctcagacgtttgacgccttcacgggcattatggatgtaggggaggacacaagtcagcatggcctcttcaccgataccgtcagccaccagcgggtccaaccccagcatggtggtgttggtaaattcggtttcagttgagctcatggcaacgttgtcagtgttaatcccggattcgccccagaggccatcactaacgtcagcgttgggtgtttcggtgtagcgcagcggattgtttgggagcttaacccgaaattggttaaaggtcgaaacgtattcgctgggttgatctgtcgggttcaccaccacaaagcgcttggcattcacgcctccgccggcatcttcatttctggcaatcatcgtcgatccgtcagttgtagcattctttccagctaaaaatgcggtacagctggaagtcgtttgaaatttattcaatcaaatcattccttctcaatttaatacatcgattcgattgggaagcggtgcttggtacggtagaaattttagtaacttaaagctaactggttggtgattgatttaggaagtaccagtgcttggccgtaaatccaatatttttgaactttggtgtgtttagtggccttcttggttgagtatttggtgatccggtaccagttgaactgcaatccctggttggcgtacaaatcaacgtggactttggtgccagcctttaagccgctcttcttccatgaagtggttttaatgtttttgtagctgctgttgggggcgtgattagtgagcttaaatgatttgtagttggtgccgattttggcattaaaattagctttgtgataactcaaggatccgggcatgctggcagcgcttgaaacgggggattgagtgacagatacgaaaccaccaaggcccagggctgttaccgccaacaagatacttttcttaaacatctaaaaaatctcctttcaaaattcaactaattttagtataaaagtctggttaaaaaaattccagccgactagctggaattttagtgattagcctaagaacttacgcaagattgcctgacgactgattaaggtggtcttggtttctttatcagaaatcttaaccagatcagcggctagttgggcatgcttctcttgttcaggtgtctgtgggccggcctgaatatcgaatagtcgttcaactgcttcaatatcttcgtcaaccgctttccaggcagggttcttggcttgaagagcagtcaaggcgtccttgctgaagtatttggcaacgtgggcataatcgtgtttgatatttggatagtatttcattaaggtgttcagttctttgtcactgagcttgttcaagatgcggccagttccaaggaattctggcggaaccccaactgagtacagggcaccggtaaaggtgatcgcacgaggcatcttatagccatcaacgtcacgtgagtaaccgatgattccgacgtgttggtgacggtcccgacgctttggaaaggcatcaaataccggctgtaagtcgttaatgagtggatccaaagtttcgtgatattctgcagcggcttttttagcgatttccaagagaatgtcttggtcgtcgtgatcgataatttcaaatttgctcttttgaaggccgtcgcgcagtttgatgatcgctggttcaaccacatccaatgggtaatcgtaacggaatgccgattgaatcgttgccgtcttcaaaccggggaattcttcgaggtaacggtcaatcatcattggtgataggccgccacggaagatggtgcttccggttccggcaattggatagatcggcaagccagattcttgttcaaattctgccaagccggtcaaggctaatttgttaccaatgatactgttcaagaaaccgtttgaaagggcggaatcggatcccgccaagaagacccgcatgtagcttaattcacggccaaagtggtctttgtacatttcaaggtattttttcaggatttgtggggcgtgtaactgggattcgaatccttcaaacaatggaatcatttgcagagtatctgaatctttgtgcccggtattaaattcagttgacttgtagtgggaaaggctggcgaacttgtcttccatggaaatcagctggtcggctgattgggtcatgggcaagatagcttcgaataacggtcgttccttgaatcccaaatcgtaagcaaagtcttcagcggacaagatggtggtcattgcctgcatcaaactgtagcccttttcttcccaaatgtttggcagacggaaagtgaggtacttatctttgccaaggggatgcttttggaaatattcgtagtgctcggagtacaaacggtcaatgacggatgcatcggcgtgtttgccttcccagtcccacatatactcatcggcatcgagcttggaaaagttttggtaagcttcatcaatttcacgaaatgcggatacaaatgcattatcgttgtgcttgaagaatggaactcctgcgttatctggatgttgagtacccataatattagggatttttctatccataaaagaaagcctcctgagatttgattaagttcatttagaatgattatacagtaaaaaatgtgaacatgaaaataatattagcaaattgtgcaaattcataaaacaattaaatacccgaatattaatgaataatttaaacagttaattaattatttcaactaaatattacagcttatttgaaaacattaccagctttttagatgagattgagaacattatcgcaatcaaagaggttgggacattaattgttacgctggctttcattgcaaccttcattaccacttttatatagataaaacttgcaacaaacggctgatcccggccatttaacgaataaacgcagtcattccaaagtccggaataactgcgtttattcgttaaattctgggatcaaatcgcctttcgtcccaatctctttgggttaatcaaagctcgtaactgtttcagcggtgtagttcccgctgttcttaagtaattttgaaactgggcagcggttttcagcttcttgtgcaaattgatcagcggtttcaaagtcaacacctttgaccatgatctgagcgtgaactaagaattggtattcagcccgctcaccaatgtaagccactttgacgtggacctcggcggtgtggggggacaccatgctctctttcaacggcttgaagggttgcctccaagcaggtggccaaagacatgcccaaaagttgttccgggttggtgcccggctttgaattcaatgggctgctggtttccactttgatgccatccggcacataagcatggccgttcagaccttcatcattcacagcttcggtttgatacaacgggttattccatctttcatcttgcattctgttagtacctcctacatttctttaacctcgattataagcgctttcaatgaaattaaaaagaaaaaggttggtatcaaaaaaagagtgggactaaaggcgttttgatcccagaatttaagcgcacagatcgattattcctggttttggaatgattgatctgtgctcttaaatggccgggatcagccgattgccatgtaggctaggcaagcatgctggccgtcgtcgcacgtttttgataaataatatgggatcacaaaaatagaggccgaggcaaaagcgtatacttttgtcccagcctcttgagccgttattcgttataatccattcgaatgatcacaggatctttagtcaaaaagtcgccaaccccggataaaaatttttggaaatggggcgtattgttgtggaattcaacagctttttcatcctgccaatgttcaataatttcatactcagtgtcactatggagcttcttgaaatggtcgtagctgacgttgcctgcttcgccacgggagccatcgaccaattcatcaataaatgcttcgtagtccgattgcatccctggtttaactgacaattcaacgttgataactttcatctttgcagcctcctatcaaatgtttgggcatgtacacccttagtatatcgaagttttgaacttattgttcaatttatcatccgtaaatgtgagatcgtacgccgtcccgtttttatcggtgacatagagtaagtatttggctgacatcggtccctggccgataatcgactggccgtttggtgtgcccaacgcattaatcgcagcttgatatgtagttccaagacccaactggttaatttttgatttggcagtgattcgctgcttgcgcttggcagctggcgtataggatttcccgacagctttgtgattgagaaactgtactttgaccttggcaaccgggaaagtcgcagaaacatccttccaggtatactgcgtcgtcttcttggtgacgccgttgacggtgaccgtgccaacgtgggaaggagtcccgaagagtttgaggacttggtcttccgaggaaccataggcggcatcggtaatgtcgccaatattaatccgattaaaattggccagattgatcccttcagcttctcgatcgtgtttatattcggcggcggttttttgactgtcaaaatgatgatcaacctgttttttggctgaattcgaagtgccacacgctgatagcaacagcgtgctcattaatgcgagtgtaactgtaattggttttcccataaaattccccctgacaagatggttctaaatgttggctggattgacaacattatatacttatttgggcggcgagtcgtggactttttaaccgtcgcggccagttttcgaatataatgaacatacaaagttctcaatgaaagacaggtgaatcaattggcaaatcaaccgttagtatttgattatcaagcggctcaaggcaagccggagaatattcgccatccggaagggtactgcccgttttgtgatgttgagcatttgaccaacattttggcacaggacgacgatcgaatttggctggtcaataagtttcggacccttgaagatacctttcagactgtggtgatcgaatccagtgaccatcttggcggaccctccacttattcagttgagcagaatcgtcaagtgttcgaatttgcgtttaaatgttggcaccaaatgattgtgtccaataaatatcaaagcacgattatgtacaagaactatggcccgttatccggcggcagtttacgacatccacattttcaaattgtcggattggataattatgatgtttatcaaaatattgatatcagtaattttaccggagttgaagtgattcatgatgagcgctgtgaaatcacattatccacgcaaccgattattgggtttgtcgaaatcaatattgccatcgacgaagttggtcatattgacgatttggccgatgctgtccaagtgattgtcaaatatctgttgaacgattacatggctggccggctgtcatcgtacaacttatttttctacgaaatggccaataaattttactgcaaaattgtgccacgttatgcgacctcaccatattttgtgggctataaaattgcccaagtccaaaatgaaggccgactggaaaaaattgcggcagatatttcagaacgtctgtcggctaatcaataacaataaagggaacggcattttgccgttcccttttattattcatgaagttggttaaaccgcactgactaatggaaccgatggatcgtcattaacgacagtcacacgggtatcctgggctaatgcctgcttaatcatctggttgattttagtgtaaacctttggatccgcagccttgatttcgttacgggaagcaacgaataggtgacgaatttctctggactttaagagattttcaatattctggaagtcggtgaatagttggtccttaaatatcttggtaatggcttcagctgtgttttcacggttgtaggtctcaatggccgtgttcaccaatttggcaatctcagtggtggtgtcattttgaacggactgatccacctcgaagtcggctagttgtaagccattattgactttcttgaataggttaatattttgagataggcccatcaagacgaattggtgttgtgccaattccacgtttccctttaggaagtccattatgacccggtagtaacgttcctggtcgattttcttttcctgggtggtttcgttatgaccgtggtattgggcgttgccgccgcgggcactaaagttcagttcaccgccacgcaattcctcaccgagggcttctttaacattggctggatactctttgacatcaagtgcggtgacccgcttgttggaaagttgatagagtttactgttgtcacggtttaattcgatcaatgtgtaatcctgattaggtgcttcactgagtaataacaggaagtcaattgcatcttcaattcgatagtccggctcatcgacactggttcggatcaaatgataaacatttttgccaaggtgatcggcaatcaccgtcatgccttcataaggcagctgctcacgggtcaggtcattgacatcggcaataaatggcgcaatatcgtctccgacttctttttggatttttttcagcatattcttaactcggagttgttcactttggtcaaacgacagcttacgcaagttaagattcaaagtaatcaccggtgcttgtaagtcaggtaacttcgccaaatctgaaacagaaataatagttgccataagtaggacactccttcattttttatattaggtataactatttaattatataacctacttctattataacagatccaggatccaaagtcttattcggcgatttgataaaaaaagcaatcctcatgggttcaaggattgccgtattggagattcgtaataattgacattaagccgccaaaaagagtgaaaagtagacttaatactgccagggcgacgaacaggtggcgccatttgaaaggtgccggctggccgcgggcatttttataaatgagataaaaggcaccaacgacgatggtaaacaccgctgtggccagtaaaatccagacaactgctaaaacaatatccatgatagcctccgtcaataatgatacttgtaaagatagcattcacaactggcaatggcaaccaggggatgatcattacgtttttctaaaaccgattatgatcgcttaaggtttaagtttcagttaaccacgcctttctagaatgaatttaacaaatgaaatttagtcacgaatttgctcgaagaaaggtgggagacgatgattaaatggttgccatatttattaaatattactggtgtattggtctggttgaagattcaatcaaggaacttgaggcaattgacctggtgccaactgttcacaattgtcacttcaatcatctatattttggttgtgagctatcttaccttggcgccgacatcatacgcgttcgtgggaccccaacaagtctcaccgatgatgatcggttcggcacccattaatttgatcccattttggagtaccactgctgatttttatcaaaatgtggtgatgatgctgccgatgggcgtgtatttgggattgctgctgccaaagttcaacctgcgaaaagtcttattgaccgggttgagtgtcagcttgaccattgaaagcctgcagttcgttttggatctgtcggtcgggctgtccagatgggtcgatattaacgacgtgttgaccaacacgtttggggtgatcgtcggctggctcattttgaaaggcttgatgcacacgatctttcagcgactcttgagtcattttgcgattacagcattttcacaccaaaagggtaaatgattgccctttcaggagtgaggcactaaaataagcttactttaaattaatgggagatgttatgatggctaaattgaaccaggcaatgaaagacatgattgccggagaattatcgtatatttcaactgttgatgcagatggtaatccagatgttggacccaaaatttcgatgcgggttctggatgatgagcatctgatttataacgaaatgaccggcggccaaacccaagcaaacatcaataataacggcaaagcaattgtggccgttgccaacgccaaggcattaaaaggattccggttcggtggaacggcgaaactctacacggacggtgactactttgatcaagctgccaaatgggcagaaggtaagttcccagctcccaagggtgccggtgtgattaccattgaaaagatttggacattggatccaggtcctaaggcaggaaagctatttgaagaatagtggcctactttactcttaaataataaataaaaccagcaatgatgattatttcatcgttgctggtttttgtgtttcaaggttacgtgcaaataaagactattatgcttgttattacgagtcaggcttgataactgatactttctgagaaacttgatccatcagaaactgtatctaaagattttgaatcgtcagactcatctgtaatgatcttaatacttttgggcttcagtgtcgtagtggactcagataataagactaagtcatattccacccgcttggcatggggagccaactcttcttcagaacctgtatcagccatcgcatcgtcatcgaagtttatttgataaccgttggaaaatacaatttgcttgattccgccaaagtcaatcgttgttgtggaatgattggtaacaacatactcaattttcattcgcgtgtagtctttaggcatactatctttgttaaacgaagtcagtgcctgatcaagctgatcttctgtatttgcatgaactttgtcgatctcagcgtgtttaaatttaacagaaagcggcccattttggattgtcgtatccggtttagttcctagtccggtcatggaaatttttcctagaacttcgctatttttccattgcccaacttttgacagatggataagagggtttgaagagacttgtttggatcctttttcttagccttcgctttggtcttagcggtcttcgaactcgctgcaggctgcatgacaaccgttgttttcgcactattcaatagggcgatacagattaccaggccaactcccaatacgataatggcccaaatcatccagtttttataccaaagttgtctttgagatgctgccacgggtgtccgttgctttaaagtgggcgatggtgacgatggttgattttccaatcctacttgtggtttgccacagtagggacaatacgatgcagcaaatggaatctctttgccgcaacttaaacagaactttgtttcttgattcatgataatcccccaaaatatgtattcagctttttgcgtcgtcagttttggacaaaatgactcaggagcatgactggatgcttctgagttttcaagtgcattcagctggtcgttgaaagtgccatttaactatacccaaaccgcaatacctgcgtcaactactttttgacgattatttaatggtttgatagccggaaagttatattatcatctcttgggaatccttttataatagccgattaaccgctttcaatcaaaaagtcgttttaattgtattttcgattgcacaaaactaatatgatgttaatcagtaattggttacttattttacagggaggttttaattatggctgaaacaattaattcggggattgctgcattacacacacttgagagctggggtgttgatcacatctacgggatcccaggcggaaccattaacaatttaatgtatgcattagatgctgaaaaagacaaaatcacttatgttcacgttcgtcatgaagaagtgggtgccttggctgccgttgccgattcgaaactaaccggtcacatcggggttgcctttggctcagccggccctggtgccactcacttgtatcaaggggcttatgacgcaatggctgacaaagttccggttctcttgattgttggtcaaaatccacaagctctgatgaaccaggacttcttccaggaattcgatgagaacccatggtttaaggatgccggggtttatgctcgaaccgtcatgactgctcaaagtctgccccacatcttagacgaagccattcgtcgggcgtttgcgcaacacggtccagccatcgtcacgattccaaatgatttggctaacaaggaaattccagcagatgggtattatagttcagctgccaattttgccaaaccagaactaggtgccggttcagacgagcaggtccaacaagcattggacttgattgatcaggctaaaaagccagtcctgtacgtcggccagggaacttacggcgctgccgatgaggtaatggagtttgccaagaagttccaaattccagtgatcacgaccgcactgggcaaggaaattatcccttatgactttgaatccttactgggttccgctgcccgggttgcttccaagccagccaacgaggcgttacagcaaactgatttgatgctgtttgtcggctcgactatccgtttgcagaagccatgttcaaaccggacgttaaattcattcaaattgataacaatccacaagtgcttggcaaacgtcacaagacggatgttgccattcttgcagatgccaagaagacattacagaaattcatcgatatgggtcaaactaaagagccatcagattggtacgcagccaacgttgataacgtcacaaattggcacgaatacaatgaccatatgatgaaccggacggaaggcaagctgcgtttcgaaccggcatttaaagagatcaatcggatcgctgaaaaagatgccatcttctccattgatgttggtgatgttacccaaaatgctgttcgtttgttgaagaccaacggccatcagccttggattacttccggattatttgccaccatgggcgtcggattaccagggtcaattgctgctaagttgagctacccagatcgtcaagtattcaacctgaccggtgatggtgccgcagctatggtgatgcaggacctgagcacccaagttggctacaagctgccagtgatcaacgtcgtcttttctaacgaagcactgggcttcattgaagatgagcaagaggatgacagtcacgagtggttcggaattagtttgccgcagaccgatttcgccaaggtcgccgaagctcaagggatgcttggaatcacggtgacatccgttgatcaaatgaagccggctttcgataaggccgttgaagagaccaaggccggtaaaccggtgctgatcgatgtcaagattaccaacgagcgtccgattccagttgaaaaattgactttggatccggataaattcgatcaaaagacgattgacgacttcaagaaacgttactacgcagaagacttggttccgttgagtgcctttttgaaacaacacggagttaaataaatcgttctatagctaagtgagaggctaaagcatcagtgtcaattgatgttttagcctcttttgtgtgtcattttgatactgattaaatatgctggagatgactgttttcattcacaaaagattaaaaggcctcaatcatgcaagccggataccattgaattataattaattgtatataaatgaggggagtcaaagattatgggaaaatggaaaagtgcactcttagtgctgactggattcgtaactttgggggcagtttcaacgacagcttcggccaaggcaaaacagaccccggtgacggtgaatgttgtctttaatgttcgcgaccgtaatgcaatgaatacttatgtcagccaaacggtagatccaacatccgctaattatcatcagtacttaacaccacaacagatggctgaccgttttggccgaaccaacgccgaaatttctgattttaacaggtacttcagtcaatatcacctcaaatcggcggcttatcctggcaactttgtgatgaaagtccagggatctcaaaagaatctggtgaaggcctttaaggcgaccccagccaagaccaacaaggactgggacgtgaccggcactaaattgcctggtaagctgtccagtcaagttgcgtcagtcttgggattgtttgttgacaagaaaaagacttcaacgaagaccgacaagaaggcgttaaagtttacccataacttaattgaagacgacacgccaattgtcgccagcagtcaaaatcagctggcgaagaaatatggtccgactaagtttgctgatcgatatggggttaataagctgtacgaccagaatctccatggagccggccagcgctttggggtgattgtgacttacgacttcaacccaagtgatgttgccgactactggaaacaaatgggggtcaacagcgacgtttccagaattcacaagatttacaccaccgataatactggtgggccaaagccaaagaacaatgatgatgtgacctcccaggaagaagccagtttggatgttgaacaagccggaggaattgctgatcaagcacaaatcgacgcttatgtcggggtttccagcaacggagacaccacgccggatgttcaatatttggacgcatttgccactgcgattggtgataaccgtgacaaacaattgacgaccagttcgtcctttggtaatgaattgaatggcttcggtcgtggcgggctgagtgaaacagcttcagaattcaatgatgctatcaacctggtttttgagcaggcagccattcaaggaacagtcatttttaacgctgccggtgacagtggaccgtatgaagtcgcaaataagtcaaccaacttgccattcccaacctcggaatatgccgttcaagtgggcggaacgacgttgccttataccaaaattattggcggccaattggttcaagttaaaaaggagcgtgcttggggtgattcctattcacaaggtacggttaccaagccaactgtcttccctggtggcggcggtggtttttcaactctcaatccaacccctgcttatcagcttggtgttccgggcgtcaacacttacaacgcatttaacatgttgaaatataccaagggtggttacttggtcaacccagatcctgaaatgatttctgggactcatcagggacgaaatgtaccggacatttccgggaacgctgatgaaaaaactggttatggcgtatacattacttataaagccgggaatacccaggttcccatctggatgaatgcaggcggaaccagctttgttgccccacaaatggctggcgccagtgctgttatcaacagtggtttaaagacttctgccggattctggaacccacagctgtataagtttgctgttcaatccgacacaccgttccatgttttagatgacgcgacgatggataataccaatctgtactataccggccagccgggcaaggtttataaccaagcaactggtctgggaaccgtcgacttcagtaaactgtttacgaagtttaatgctcagcaataaagcaaattgaaaaaacaggacccccaacatgcaagatgatagcgtgttgggggtcctgtttttttggatatttggctgaaaagtcgacttatttaatactgtaagtttgtaccccgatgatttggttggtgccggctttcacgccgtggatcttgattggagatttggtatcatacagattccaggccattgagcctttggctgattgatttttctcgatagccaccttgtatttgggcgctaaatcttgatccggaagtggggcggcgaccaactgctttttggatttagcaggctggtaggcgcggagcacggaagcggcagacactggcgagactttatggttgccagtgtttttaatggtgtaccaaagggcaaaaatgggtttcttgccaaattcattaccagtctcaccagctggaatcacagcggttttggtaattttcagctgaaaattcttaacttgaagaaagttcttccgaaaacttgccgtgtctgaagaacttttattctgaccgctacatcctgagagggagatgacggcgattaaggtcaatgcgagtgcgaatatttttttcatgttctgagctccaatgcttatgtatttatgaaaatgatgatttattaatattttacatgtttttttcaataaagaaactcaaaatgaggaaagttgacattggataaaatgatggcagataaaaagcaacgccatgaatggacgctgctggatgatttgatgcgattatttgttgattggtttgccgaggacaatccctgggtattggtcaacggcttcttgatgatgtttgtcaaaatagaagatgccaatttgataatcctttaaggtattgcgtttggcttgattgtagcccgccttctccagtgcggccttaaccaatttcaaacgtttttgatcggaaacgtcctgtttatagaacgcccggtcaaagtatttgtcgacagatgggaacacaataacatcagtgaatgaaggaagcgacttaaccccagtagttggattggtttgaacagggaaggcatccctttcgctggttagtttccacgataatggtgtatttggaaatagttttaagaccattttagagaaatgctgtgaaggagattcctgaatgtatttggcatattcttgattatttgaaaagttgcccggctgtaggttattccacactttgtaatttgtgttatagccgggacgcagataaccacgccaaacgattcctttttgggtgtattgattatttggagtccagccattgatgccatagtagacagacaatttaccattatgcctgtacgtataagtgtgatttcgataccagttggtgttggggtaattgtttaattgaaggattttcttagtgtgcgtgctgttccaaaggtagactttacgattcttatattgggatttgacttggaaaacgtttggggaactctgccaagtcgttttgactcgttgatagccatcagcaaaagtagcaggagctgatgccatcatgcccagaccaagcgcgactgcagtggttatcatggccaaaaatgatttcaatttcataattattccccctgaatgctactgatttgaattatctaatgctcgtagttcagacataatctgcatgagcttggcatgatagatgtctgatctcaacgcgtcgttctgctggctaaaccagtactgcttggcaggggcgacgtaggtttccggcacctgatacttgtcagcaatctgctggaaagtcgttgggttgtcggctgcctgctgcaggcgatagagcggttcttcctggatgattttgacaacttgtggacggacctcttcgggcagcttgggttccacaaccttcacgaccgtattcttaattggtttatccaaaattgtattggtttgccgctgagcgtcggttaattcgtgaacctgatgaccaacgtaaagaaaaccggccaggacaatcaccaagacgcttaaccaaacaattaacttggtgtgcttagattttttctgttcttgtttggattgcttctgctgcaatcgtgatggtgtttgattttgcatgttgaatccccctcaaacaatttacgatacgattataacatttttaatcatgattcaatctgggaaggaaaccaggcatgcgaatttaaaagttccttaaaacaaaaaaatggcaagcagcttcgaccttctgaacgcatacgcgccgatcgttacttactcaccgtggtttggcaccagaaatgattatagcatggctgacttggcagatgcaagcaaatctatgaacgggggctctgatttcgacaaatgcaactgtttgctcgattgaggtataaccacagtgccagataatgtataatcgtttttgataaaattttttgacgcgggggggaaacacatgaaatcacttaaagtgcaaagcttcattctcatttcaattggatttattctagggatgagcgagtttattattgttggaatcatcaatgatctggccgattcttttgatgtgggcatttccaacgtcggcttcttggtgacgatgtttgcgattgtttacgcgattgtgacgccaattttgacgattctggtaggggagcatcgactcaagcgggtgatgttgctgttgttgagtgtcttcaccgtttcgaatgtcatgacggctctggccaactcattctttattctgtccttgtcccgagtgctgaatgcggtggttgccgggataactgtttcaattgcgattacctttgcggcggttattgcgccgcgggataaacgggcctggttgatttcttgggtcttttcggggtacagtgtcgcctcggtttttggggtaccgattgggacttggattagtgatcaggtcggctggcgttgggcattttggttaatcgtcctcatctcagtcatgattacggtcatgttcatgttgtcgctgcctggagatttgcggcaagggaaagcaaagagtttgggtgaacaattcagccttttcaaagatccccgcattctcttggggatttgtctgccaattcttaatttaggcggggtctacgttgtttatacctaccttcgaccaattgtgacatccggactgcattttccaaccagttttgtgacaccgtttctgtttgtctttggactggcatcgttgttcagtaatcaatacagcggccggttggcgaatcgggatggcttaaaatcaatggtcacggtgtttgtgattcaagctttgaccatgttggcgatttcgctgttattcgggttgccgtgggctgcactggccgccttaattatcatgggcctgacgatgtacttgctgaactcaccaatgcagattttctacctggcggtggctgaaaaagactatccgcagtcgatggtcttggcctcatccttgatttcgatttttaataacgtaggaatcgcggtaggatctgcaaccggtggggtcttgttcaatcacttaggattaaaatctctgggatacagtggggctgtgtatacggttgtggctttggcaattttaattgttttgaaccgggtacgaaagagttttgattaacgattgcaagacgacatttctcgtcttttattattttttctattgctactttgaatgaccaaatcaatgtaatcataaaaaggtcagccatgacaatgctttgtgcactgtcatggctgaccttttagtatattgatggagtcggcgggagttgaacccgcgtccgagcatattgccacctagatatctacgttcatagatatattatttgaatttcacctactgaaacgccataaatcaaggcacccacagcaggctaacctgattagtctcttcagttcacttcaggtgggagcaaactgcgtgagcccactaaatttaggacccagatctaacccatgggcgagattaggaggatctacgttaagcgcttattaggcagctaaagcgtaagaattgttattattttttgcagttataataaactgggcggtttaacgtggcgctgcacgaaacgcaatccagactcaacctatacccgtcgaatccataacgaccccgatacaatacgtatcatatcataaatcacgggaactgagaagaattgtgtcttacaacaggtcaaaatgtttgaggccgttaatgataccatgatcagtattcttggtcgtgataaactcggcatactttttcacctgtggaagcccattttccatcacgacggggtggtcaacgaaatccaacatcggaatgtcgttgttgccgtcgccaaacgcataagttgggatgccggagagattggcgttggcaatcaactcctggatgccttttttcttggaactgcctttgtgaacaatatccatgctaaacggggtatttctgaagaatgtcagggtgtcggcgaaccggtcaatgtatctttcgtcaggccccttggtgttaatcagcatcatgatcacttcttgattctcgatgaaatcatccacgcccaagtttggcatccgggagttaatgaagttataattgccgcggacgatgtcattgataaaattaatcttggcaccctggctgttcataaccgtggttgcttcgtggttggatttggcaaacgccacaaaatccttaacaacagatttttccaggacagctttgtaaaccggctggccttcgaaaataacgtaactcccgtttgcggaaaccactgtgtcgatcccagtcttttgcattgtattggggatttcaaataaatttctgccagtcgaaatcaccgggagaacctgatttgcttttaattggtgcatcgcgtcagccacttcgtcgtcaacacgcgtgtgttcattaaataaagtatggtcaaggtcaaagaacgcaattcctttatacatagataagccatccttttcattatcaattttataatcatatactttactatcataacaatattgcgactttccaagcaagttcttctaattattggtaaaatgggttatatatggggtgagacgattggaaaaaacaaccattgcgaatgaaaagaccagccgtttcttcgttcgactaagaagaattcccggcgaacattggtatttagcaaacggtaacgaaaaaaatgtaaatccaaaaaataaaattaaagttccggacagcatcaaggcacaggattttttgattgatgagattagcttcttcaacaaattagtctggtaccacttcacttgtggtgatctggaaggctggctgcccaaacgaaatattcgaaagacatttcgccgattggacgttgaaccgattaagcagcccacccaatccgatattgataatcaatgtacggcgattttaatgctgctgaacagcgccggcattagtgtcgacgtcagtgatatccgagacaaagttgagaagtggcacgcgcaatcgggaaccctaatggatttgagtgacttaattatttcgttaacccactcaattcgcgatctgaacggcgttgattttcgcaaattagataagcagcttttgcgcagaagaccgattttagtcaaagttgccggcctcgataatttaaagtccagcttgatcttgttgaccggttttaacagaaaactttactactacaacgatccgtggaccggcaaactagagtcgatttctcaaaatcatttaagaaagcattggaaacgcgggaacttggaagcaatcagttattgaaggtggggttttagaatgaaattgttgatgattgaagataacaaatcagtgtcggaaatgatgcagatgttcttccaaaaagaaggctgggatgtcacaattgcttatgacggcattgaggcaatggacaaatttaacgaagatcctgatagttgggacatgattactctggatcttaatttacctaaaaaagacggaatggaagtcgccaaagaaattcgggccaagtcacaaacagtcccgattattatgctgaccgcccgtgattcggacagtgatcaggtcttgggatttgagatgggcgcagacgattacgtcaccaaaccattttccccaattaccttggtggccagaatcaaagccttgcagcgacgggctcacactgaaactgaggaggaatctgaggacgagaaggccaaaaatgtctttgacgttcaaactgatcactttaaattgaactccagtacccgagaagtgtatttggatgacaagcggatttctgatctgactcccaaagagttcgaactgttaaagacgttggcccaaaagccacgtcaggtcttttcccgtgagcagcttttggaaacggtctggaattatgagtactatggtgatgaacgaactgttgatgcgcacgtcaaaaagttgcgtcaaaagattgagaaggttggcacccaggtgattcaaaccgtttggggcgttggctacaaatttgatgatagtgaagtgggcaagaagaaatgaaaatgatttatcagcaattattggcgttctttttggtaattggctgtacaattttattgctgggtttttcatttagccgcatgtcaaaaacgtttgtatatgaccaaacctggcataacttggaaaagtattcggatagtttgattcaacaatcgctgacgattagctccaaaaataaggccaaagtgacctttgacgaagaaaagttgaagaactctgaagccttgttggagaaccaagcggtccattttaccgtcttcagtccacaagatcaggtgatctatcccaataacggcgttgccccccgaattacccagaaagactgggagcatttgcggcgcaatcagatcgttcgcaaggtcaataataagaatttcaagctcagcaatggcaagacccggcctgcaatgattgaagttttaaagccatactattataagaaaaaactagtggccgccgtgacggttggtgcctttatttcggatgttaactccaacgtcaagcggattaaccgcgatttgttaaaggcgctgtttgtggcgttgctcatttcgatgctcattagttacttcatcgccagacggctgaatcgacggattagcaaactgcgaagtgcggccaatcaggtttcaaacggcaattacaagattcgcttgaaacccggtgggaaagatgaaattggtgaattgatcgtcgatttcaaccacatgacccaatccttgcagcaggccaacaatgaaattcagcggcaggaagaacgccgccaggaattcttggccaatgcggcacatgagatgcgaactcctctcacaacaatctcgggcattttggaaggaatcaagtacgatgtgattccccaggagtcaagggccaagagcatcgacttgatgagcagtgaaactcagtggctgattcggttggtgaatgagaatttggattacgaaaagattcgctccaactctattcagctcgataagcgtcattttaacgctgctaaggtccttgaaaatgtcatcgaccagttggacagtaaagcagaagaatcgcaggacaagctcgttttgaacgcccctaaagacctgtcaatttatgcagattatgatcggtttgtccagattgtcttcaatatggtgaccaatgcgatccagtttactgatcacggtacgattaccgtaaccggtgaacggggttacaacgagaccatcatcaaggttgccgatactggtattggcatgtccgaggatcagcaaaaaaatatttttgaacgttattataaagccgatgcctcacgaagaaccggtaagtacggtgagtcggggctgggattggcgattgttcaccagttggtgaagtcccatggcggcaagatttcggtttcatccaaattgggtgagggcacgacgtttaccgtgattattccggatgcgacagctgccgaaaaagaacaagaaaatcactaaattaaaagtcatcattttgcatttgcttgagagagtctcaaggatgcaaaatgatgactttttgttagctgtttgattcttgggatgcatgggcttcgtaagccttggtgcccttttctgttaaaccattgatttcgttgtggtcggtcacgatgtacccggctgcgaccagtggcttgggatcgccgccaatgacgttgtcacaataatcgacgaagtggttgaccggggtgccggatgatacccggccggtataaattgcctttaaaatttcatagtctgttgccgttaattccatgatgaagcctcctaatcttgatgcatttatgataccaccaggacgggtgtgggcggtgaattttgtttggtggcataagacactgacttcatcccttaaagattgggattattagcacggaccattgcgatgagcaagttgtcaccgcataaatggttaaagtgatacaatattttaaaattagtagcgttttcattaaatgtccacaactgctcaccaaaccgaagttgcgcaaatcaaaatatcaagatagtgagaaggctaattatgaaactagcaaagaaatatttatatagcaccattctcggtctctcattaggagtgggaatgtccaccaacgtggtgaaagccgccccaagttccaatagtgccgtggtttctcccacgagtgacccttcaaaagacgagcaggcaaatccagacctatcgggaaaggtcgaagatgtctcctacacggttaaggatgaccagctgactttatatggcggcacgatcaaaaaaattcacgagaacttttcacttccttggcaacaggatggggtccgtgaccgcattaaaaagcttaagattgatggtccgcttcaatttgaacaggatggtgcctatgaattttttgaggcgttggggaatcttgaaagtatatccggcttaagaaacgttgatacatcaaaaaccgaaacgctgaattatatgtttgctcaagatggcaatttaacatccattgacgtctccagctttcggacacccaatgtcatcacgatgagtggcctgttttttggtgattggaagcttgaacaagtcgatctttctaattttgatttttctcaattaaaaaatacggatcacatgtttgggggggattatgtattaacgaatatcacttttcctcattcgaaagcttctaagattgataatatgctggatatgttttacgggaatcactccttgaaaacattggacctttcagactttgacatgaccaatgtcacggctattggcagtatgttttccgaggatacgttactatcgaatctgaaactggggccaacctttaaaaattcagctttggccactctcccgccgcatcaaaaaggcgatgaaatccccattgatcccttgaaggacgccaccggtccaggatggcaagcagttggtaccaatggaacggtcaacaatccacagggcgagctctatccaacccttgaggactttgtggctaagcggcctgctgaagacgaaacctatgtctggcagcaagacaccacgcccatcaatcaatatatgctgaacctgactaatagttcggcttcagtatatgagggccttcaagctaagaattgggatccgaccagtgtgattcaattagcgactcacaatggaaccgatgataagtctgctgttacgattactgatgacaatagccagccggtcacccaggcaactattgatgcactggctcctggaacctactcgctgacttatcagaatggtgatcagaaacaaccatttaccttaacaattaaggccgatcaggccagcttgaagacgacggatattgatctttatttaaaccaggcgttcactgaagatgtgttgaaaagtaaaattttggcggtcaattccgatggccaggctcttccgtacacttacaccatcaaagatgcaactggcaaaactgtttcgcttgatgacgtcaaatcaaaggttggtcaatacacggtcgacattgttaccaatcagctgctaagtggtaacgagcccctgggagggaagctcaccatcaacgtgactgacagcagtaccctcaatctcaagtatggcaagctgacaatccccgttaatcaggtatggaaaccggcagatgcatttgataatgccaaagatgccagtggaaaagacctagcctttaaagatattttggtgacggctaaagacagctctggaaagatcatctcagacctgagtaatctgtataaaacgccaggcgtttacacaatccattacagtaatgggtcagcttcaaaggacgttcaattgacggttacccagccgacgccaacaccgtctccactgccaaccccccagcctgtgccaaatccgcaaccatcaccatcgcccaaccccatcaatccagtcacaccaacgcagccaacggttccgactcaaccaactaatccaaagcttcctgattacgcggtgacaaagggcgcggcagtcgctgccattaataatgtctatttgtatcgaacggttaacttcaccaaaggccagcgaattgccaaatatatcaagaaaccgcgcatttaccggccaatgtttgtggtgacggggtatgctcgttccacaagtgggaagatgcgttaccatgtccgtgatgtcaaccacttatcgaaaacggcgggcaagaccggctacatcaccgacaattggcgatatgtccgtccaatttattacgctactctgcacaaacacattacggtcatttctccggcaggggttaatgcctataagcacaaagacttgactggtaaggtcaaaagttatcaacagggaaccatcctcaaagttaaagggatcgtgaagcacaatctgaccacccgttatatcttgacgaatggcaggtatgtcaccgctaaccgaaagctggttaacatgggtcggcatcggaccgttaagaaggttcgtgccaagacaaccattcatcgttatcagaacgtgaacttgagcggacggcctcacactattaagaagggccagatcatcaaagtatccaattatgattactcccatggccataatctacagaagcacggtgccttgcgataccgtgtggctggtgggtatatcaccggtaactctaaatatgtcagaattattcgataatttacattagacagtgcgacgagaggcgttttgatcccagaatttaagcaaagaagcgggctattcctattttggagtggctcgctttttggggatcagtcgatcgccaagtaggccaggcagggtttcagccggccgtcgctgcacgttgtatcaatacaaaagtggtaatcaaatccaccgtagcaattaatgtcccaacctctttattttttttgcaaccagaaattgcatcagtgtgaaatttttgttgtggcattttttgttagacaatttattgaaactgtctagcggattttgcaacaaaaaaggtgttagccaaaaattggctaacaccttgctgatccttgtcaaatcaacgattatcacccgcacggggctcgaacccgtaactccgccttgagagggcgacgtcttaaaccagtttgaccagcgggcaatgctatcaaactcactataatagtgtatctaaatcagaaagatttgtcaacaaaggaaactgaaatataaagttgacaaaacgcagaaaaatctttaatatatttagttgtgatattcattgggtattcgccaaatggtaaggcaacggactctgaatccgtaatttactggttcgaccccagtatacccaatcttttgcaaggtctgttatgtttctctctaatcagagacaatgtaacagacctttttatattccataaatcccactatcatcctgtgcagaaggggatctttaaccgttacccgttcatactcgtcccagattgaaattgcttacaccacagtgacccaaagtgtgctgatctagaattaaatggttaatgattcacgcatattcatgcagataggagccgatattaatggatcaatttacgttagtcaaagaaacgctggataagatgggaattccctatgagattgttgaacatcctgctgcccacaccactgaggaagccgatgagtacattaagggcaaagagggcgttcgtacagaacaatgtttatgaccaacaagaagaaaaccgagttttacctgttggtaatggacgatgccaaacgtctagactttcatgaatttcaagacttgaccaacactaaacggatcaagatggcctcagcggaatcacttaaagaacaaatggggttggagccggggatcgtctcgatttttggattgatcaacaatcacgagaagaatattcatgtttatttcgatcgggccattttagatgaaaagacaatgaccttccatcccaatgtcaacaccagaacaatttttgtcgcttccaaggacgttttaaaattcgtgaaggaaatgggctatgactaccagatccttgacttggaatcctttgattaatcagagaggttacgaatgaaataccaagatgttaccaactatgtgattgaaaaatatcatgttcaccctgaatacctgtggaaaaagtatccgagctttaccgttctgcgtcacaaggagaaccggaaatggttcggcttagtcatgcaggttgaaaagtcgcaacttggacttgatgggcagggtaaggaggacatcctggatgtcaaattggatcccaaagaagttgagtttcgacaaaccagtttggagtttctgccagcttatcatatgaacaaaaccaactggttagccattcggttgaaccaggtggatccaaagcaaattcacgacctaatcgaagctagttatcagttaactcaataaccaaaaatgaggcatccgccaaggtaaacttttccttggagggatgcctcattttattgagggtttatttaatttcatagtaatcatcggccttagattttaactgattagtctcaagcttgttgagatccagcttccgcagcgtctgtttggtcaccatggttttgacaatggttcgtttccgaccgttgccaacatttcgattgaagataatggtgaattgatcataacggtcatagtcggtctttttaattgccttcaaaataccaatcgtggttaaccgaaatgactcggtcgtatcgcttttatcggtaacggccactgtgagtgctttctggctggcatgcagcttgacttgatgatcaaatagaagcgtgtgggtggcgttcagttctttcttgacggcagtttcagtattttgagtcgactttttagccggctttttcacggccttttcggtccgctcggcctgctcggcattgccctttttgatgacttcttttcctttgggggaattaaaaaacaacgtgccaaacacagccatcagcaccaacgaaatcagtgcatacttgccgtatgggtatttaccgtgcttgccagtggtcttaaagtagacaaacatggcgaaaaaaatcaccatcgcataagacgacagcttggtaatgacatcaaacattgtgctaatcaaagtgaaggtctcctttatttggctggttattcaaatgacaggtccaccaggtatttgtgttggtccactaaatgcgaggtggtgatccacaattcgtgataattggcgtctttgacctgcgtcatctcatgaaaatagtccagcaaatcactgtacattgacagaaaatctgaagacattcgattaacctcgagtttttgttcagggaaataaatctctggattccctaatttaacggtgtcatcaaggtacatttccacgacgttgtcataggtgtccggcttggtgaatactttatccggatgggccttaatgtatgataagacgtgataaattgtgtctgagttacttgccacttgaacttcctccgatcttaaaaatcctacgttcctattgtaacaaatctgagcagagtggggaaaatgttttcaagcaaccgccagtgggctcctttatccagttgtggattagcggtacaatgaatgcatctcaatgcgaaaggatgctgtccatggattatccaaacacggtcacaaaaattcatcagtttgtggacgccggaattgtccccggcgtgagttacgcgattattgatcgggatggccttcaaacaaacgtttttggtcaacaggaactgttaccggaaagattgccgcttcacagtggtgaattgtacgatctagcctccttgaccaaagtgattgggaccaccaatttaattttacgactactggcttccgggaaaatctcactagatgattccttgaccaagtattttcctcaatggcagtcgccccaggtcaccatcagacatttgctgacgcatacctcagacattgtcggctatattcctaaccgcaatcaactgcccaagtcggaactgatgccggcgttgttggccctgaaaagcggttcagatatcggcaaagttattcactatcaagactacaattttatctttttaggctggattgcttcaagggtgatgggcgagcccgttcaacagctgattagtgagtttgtgttaagaccgttggaactaaaccaagcgacattcaccccggatcaggttaacaatgtcgtcccgaccgaattaattcccagtaagggtttgatccgcggcaccgttcacgatcccaaagcgcgaatccttggtcctgactgtggttcagccggcttgtttgcgccgctcagcgatctgattcatttttcaaagtggttgttgggcgatgtcaaatatcccaactttctgccggcagactgggttgaccagctcttcgttgaccaaacgccgggacacatgaagaatcgttcgtttggctggatcctgcgtcattataatggtcatccatacattctccacacaggctacacgggcaccctgattgtggtcgatcgctattcgcataaggcgttggtctttttgtccaaccgggtccacccggatccaagcaaccagttgtttttgccatatcgcagccaactgattcgaacctttgtgaaagaaaacgagattgcatatcaataatattcagacaaaataggagtcacagcggatgctgtgactcctattgttgtattaaaatgttgcgccaactttcagattctcttgtgctgttaaatcggcgtcaggatattttcgcttcagcgcgttcatcaaaacgtgtttagcaatatcattgtttctggcaagaattggaccatggaaataggtgcagtagacgtttttgtaaattgccccttcagtcttatcttggccgttgttgccgtgaccctccagaacctttcccagtgggcgttcaccgcgacccaagaaggtaattccctgatgattttcaaagccgtgatacttttcgccggtttcttcattttcaatcacgacgttaccaataaaacggtggtccttttgtttgtcggtatagtgattcaacgcaccgatgcccatcagcttttcaccgttagcgccgatatagtagtgacccaacaattggtagccgccacaaattgcgaccacggagccgttatcttcaataaagtcggttaaagcctgctttttggtttggatatctttagaaataattgattgttcgaaatcttggccaccgccgaagacgacgatgtcatatttgtcaggatcaaatggttgatccaagctgacaacttcagacgtcagttcaacgcccattttgttggccagatacttgaggaccaaaatgttccctaagtcaccgtaagtgttcatcaaatcgccgtaaaggtgacagacgtttaaagaataggtcattaatccattcctcccttgataaagcctttggctgcaaatacttttcttaagtgtagcatagcggtgtaagttgcgaggatataaacctttttggttggtgccttggggatcatttcgacaactttgtccaaatccggttcaaccaagtgtttctttgggtcgactccggcaacttggaggcggtaggtgatatctttgtaccgctcaccgccagtaatgaactgtttgatgttcatcttgggcagtcgttcaaaatcgccatcccaaatccagctggtatcaatgccatctgcgtaattggcattgaggagcccgatgaaggtaaacgggtccttgtcagtggaaatcatgtcgatcacctgattgaggccgacggggtttttaaccagaatcagcgtcaccagcttgccgtcaacgttgatctcttcttggcggccaaagatccgttttcctttttcaaaggctttcttggtctgagcaggggagactcccatgaatcggccaactgaataagctgccagggcattgtagatgttgtaaaccccaccgatcccaattttaatcggctcaccatcgatttcaaaggtagatgatttcggggtcaagtcgttaattttgttcagcgcaaaattcaattcgggccgctcaaaaccacagttggggcagaagtacttgcccagattggaatagctgatgaaatggtagtgcaggacatgctgacattggggacagagaacgccgtccgtgttgggcgtcgccttaatgtcgccatctttttgattgtcgaagccgtagtagacgatcgggttcggcagttgttttgaatgaaaaatcggcgcgtcaccattggcgataatggtggcgttgggagctaaggcgaccccattcaaaattttattataggtcgtatagatttcgccataacgatccatttgatctcggaaaatgttggtgaaaacaaatgcttttggtttgatgtatttggtaaccatgatgacattggcttcatcgacttccagtacagccaatggccgcttgccctttgactttggtgcatgaaggaaagtggtaatgatcccttgctccatgttcgagccggtggggttggtcaaaatgttatcatacttttctttgagtacttgaaccgtcagagcggtcgtcagcgttttaccgttggtaccggtgatgacgatcacgtcgtagtcacggcccagggttgccaaaatttctggatcgagccgtttggtgattttaccgggaagcgaactgccgcccttgaaaaatgtatgcagaaaccagtaagacgacttaccggccgcagtcgcaattgaactttttaatgacataaactttactcccttaaaatgaagtacataatgaacctaatcaaacattaagtgtagcatatgctcaactgtttgaacatatatacgctcgttctttaaggggtttacaataatgagggtgctggcgaattttctcattattatcgattttcaaaactttttctgtataatggaagagaagctcttaaggaaaaaggtggatattttggctcaactattttatcggtacggtgcaatgaatagcggcaaaacaatcgaaattatcaaggttgctcataattatgaagagcaaaataaaagtgttatcattatgaccagtgcgttggacacccgagaaaagcagggcatgattgaatcgcgcatcggtttggaacgaaaagccgaaccgattcgcgaggataccaatgtctttgatttggtacaggaactaaatccccacgccagttgtatcttaattgacgaggcacaattcttaaagaaaaagcacgtcatggaactggcccggatcgtcgatgagctgaacgtgccggtgatggcatttggcttgaagaacgactttcaaaacaacttgtttgagggttccaaatacctcctgttatacgcagataagatagaagaaatgaaaaccatttgctggttctgcggcaagaaggctatcatgaacctgcgttttcacaacggcgagccggtgtatgagggtgaacaaatccaaatgggtggcaacgaatcctattatccggtctgcagaaagcactactataatccacctattaagtaacaaaagtgaggaatattaaatggacgaaattttcgacaaattacaatcggtcgttgatcgatatgatgagttaaacgagttaatcagtgatccggaagtgattgccgatactcaaaaattcatgaaactatctaaggaagaagccgaccttcgagacactgtggctgcttttaagaagtatcaaaaagtcagcaagcagctcgatgatgacaaagagatgcttcgagaaaagattgatgatgatcttgaagcgatggtcaaagatgagattaccagcctaaccgacgaaaaagacaagctcgaagaccaaatgaaggtcatgctgctgccaaaagaccccaatgatgacaaaaacatcattatggaaatccacggcgccgccggtggtgatgaaggtagcttatttgctgccgatttattcagcatgtattccaaatatgctgaacgtcagggctggaaagtggaaataattgataagaacgaaactgaagttggtggtttcaaggaaattgttttgatgattaccggcgataaggtctattcaaaactcaagtatgaaaacggtgcccaccgagttcaacgggtgccggtgaccgaatctgccggccgggtgcacacttccacggcgacggttggtgtgatgcctgaagaagaggatgttgatattgatatcgatcccaaggatatccgggtggatgtttaccgttcatctggtgccggcggtcagcatattaacaagacttcctcagctgtccgaatgacccacttgccaaccggcattgtagttgcgatgcaggatgaacgatcccagcagcagaaccgccagaaggccatgaagattttaaaggcccgggtttatgattactatgcccaacaggaacaggatcaatacaacgctgaacgtaaatcggccattggaaccggtgaccggtccgagcggatcagaacttacaattacccgcaaaatcgggtgaccgaccatcgaattggcttgactttgaacaagttagaccggatcatgaacggtgagctggacgaaattattgatgctttgattgtttctgatcaagccaagaaacttgagaatttaaccaatgaataatcaagagaacgtgacctactttgaagcccggaagtgggcttcttttcgtattaaggaatctaatgacattgacatgtacgacgtcgattttttgttagagaaactgtttaagatgtcggctgccgatctgttgattcattaccacactcagatgccagtcaagcagtggcgagtatttcaagacgcgatcggtcaattgctaaaaggggtgccgccacagtacgttgttggcgaggcagatttctacggtttatcattgaaagtcacaccagctgtgctgattccccgagttgaaaccgaggagttggttgactggatattggcagacaactcggattccaagttgaaggtcttggatattggtaccggtagtggggcgattgcgattgctctcaagcatgccagaccccactggcaggtatttgccagtgatatttctctgccggcaattaaagtggctcggcaaaatgccattgccaatcacacggcaattcattttatggtgagtgatgtttttgccgcaatcgatgagtcatttgacgtcatcgtgtcaaacccgccatacattgccaaagatgagcagtcctatatggatgccagcgtgatcaaaagcgaacctgatttggcactatacgcaaaagatcagggacttgctatttacaaacaaattgctgccgatgcggagagtcacttaacttcaaagggcaggttgtacttggaaatcgggtttcagcaacaatcggctgtgaccgagatcttccaagcagcgatgcccgacgctcaagtaattgccaaacacgatgtctccggtcatcagcgaatgattcaagtaaagaaatgaaggctatataatatggaaactttaattttaaaacagcagcaactagaccaagcggcggactttatccgtcaaggcgaactggtggcatttcccaccgaaaccgtctatgggttgggggccgacgcgaccaatgaaacggctgttaagaaagtttatgccgctaagggacgtcccagtgacaatccgctgatcgttaccgtatctgacatcgcgatggtcgaaaaatacacccaaccattttccgacgacgccaaagcattgatggccaaattctggccgggttctttgacgatgattttcaagctgaagccaaacgctttatccaaatcggttaccggcggactggacaccgcagcgttcaggttcccgaaaaaccaaaccacgctggatttgatttcaaaggccggcgtaccaattgttggtccgtcagccaatacttccggcaagccaagtccaacgactgcccagcacgtttatcatgatttaaacggcaagattgccgcaattgtcgatgatggaccgaccacggttggtgtcgaatcgacgattcttgacatgtctgtggcaaccccgtcgattttgcgcccgggtgctgtgaccaaagaggatattgaggccgttattcatcgaccggtgattgatgaactccaccatgtgggcgccaaacaaacccctaaagcccctgggatgaagtacaagcactatgcccccaatgctcaggtctacattgtcgatcctgatgatgattggcacgatgtggtcgcctggatcaagcagcacccgcagccaattggggtgatggcctttgatgacatcatcaagacgattaattggccggataatgtcgatgtgatttcacttggcaacgacgcccgcacagcagctcatgacctgtttgccgaattacgggattttgataaccaccctgcctataaaattatttttacccaaggaattgatccaaagggaattggtgaggcttacatgaatcgtttgaataaatcagctgggcaaatgcatttcaagcagttataatttatttgtaccaaataaattagtgaggtgttgcagttgaactacgattataaacagcaggatccagaactttgggatgccattgccaacgaagagaaccgtcaggagcataatatcgaactgatcgcgtctgaaaatatcgtatcaaacgctgttcgtgccgctcagggttccgtactgaccaacaagtacgctgaaggatacccgggccggagatattatggcggctgtgagtacattgatgttgttgaacaattggcgattgaccgtgccaaagaattatttggtgccgaatatgccaacgtgcagcctcactcaggttcacaagcgaaccaagaggtttatgccgcattcctaaagcccggtgatcggattttagggatgggattagacgccggcggccatttgagccacggtgccaaagtcagcttttcaggcaagctctacgactctttctcgtatggtcttgatccaaagacccaattgatcgattacgatgaagttgccagaattgcccaaatcgttcaaccaaaactgatcattgccggagcctccgcatacagtcgaatcattgactggcagaagttccgggatattgccgattctgttggcgcttatctgatggttgacatggcccacattgccggtttggttgcagttggcttgcatccaagtccagttccggttgcagacgttgtcaccacgacgactcataagacgttgcggggacctcgcggcggcttgattttggccaaagaaaagtatgccaagaagctgaactcagctgttttccctggcagccagggtggtcctttggaacacgtaattgccggaaaagcggcggccttttatgaagacttacagccggcattcaaagaatacggcgagcagatcattaaaaatgccaaagcaatggccgacgtattccagaattccaagtcagtctccgttcttaccggtggaactgacaatcatttaatgacgcttaatttaacgcagacctcattgaatggtaaagagctgcaaaacctgctggatactgttcacatcaccactaataaagagtcgattccaaatgacccattgccaccttcgaagaccagcgggttgcggttgggaacgccagccattaccacccgaggcttcaaggaagacgatgccaaagcggttgccaatttgattttacaagtgattgacaaaccaaatgatgaccaaaacttaaaggatgtcgctgccaaagttgaacaattaactgcagctcacccaattaatcaataattttgactggcttgaaactaattgtggtttcaagcctttttgtatactttccgatcgcgtatatgtgatacaattatttcggaatacaaaaaggagttggaaaataatgggtaagtttcaagttatggatcatccgttgattcaacacaagctgtcaatgattagggacaagaattgcgggactaaagagtttcgggaaatcgtcaacgaaattgccactttaatggcttttgaagtttcgcgggatatgcctttggaagatgttgatattgagacaccagaggggattgcgcatgcgaagcagatttccggtaaaaaggtcgccatcgtaccaatcttacgggcaggtatcggaatggttgatgggatgcttgatttgattccagcagccaaagttggtcatatcggtatgtatcgtgacgaaaagaccctcgaacctcacgaatattttgtaaagctgccatcagacattggccagcggcagatttttgtcgttgatccaatgcttgcaactggtggttcatcaatcatggcgattgatgccttgaagaagcgcggcgcatccaacatcaagttcgtttgcttagtagctgctccggaaggggtcaaagcacttcaaaaggctcatcctgatgtggatatctatactgctgcacttgatgaaaaattaaatgataagggctacattgttcctggactcggtgacgctggtgaccgtttgtttggaaccaaataattgattgaagctgagacaaaatgaaaattttgtcgtcagctttttattttatttacaaaaggattctggctttgatagccaacgaattaagtctaatcaaagacccttgggtgacattcgttgtgcatgccgttgaacactactgctcacgcgaagtttccctgtcaagattgttttgaattttgtaataaatggtggtatgatttcaattgtatttgaacacgggtctgtgttcagtaccatcgcaatgtttcactttggtattactgtcttctggaccaaaaccagattgatttgcatgcgtgattatgtggaggaaagaggtgagattttgtgggagaagctgcttctacttttgaattcttaggactgacgtttaacgttggtaatttaatttcgatattactggctgcttgtgtggtttttgttctggtgtatgctttatcaaggcacttgacaatcaaaccgggcaaggcacaaaacgttttagaatatgcggtggactttaccaatggtattgtccgaagctcgatttccggtgaaacaagtagaacactaggtttatggggctttactctgtttatgttcatcattattgcgaatttgcagggactcttcttgcatatcgacatttctggtgtaacatatgtcaaaagtccaacttctgatccggttgttactatgactctggctctgatgactctaacgcttgcacaattccttggaattcggcagttaggttacaagggacattttcagaattatttaaagccattcgtatttttcctgccaattaacttattcgaagagtttactaatttcttaacgttgggattgcgactatttgggaacatcctttcaggtgaaatgcttcttggaataatccttggcatgtcgcatggtggagcagttatgtgggtcgtttcattcattcttgaattggcctggacaggtttctcagtctttatcggatgtatccaagcctatgtttttgtgacattatcatccgtatacatttcacgaaagctcgagcttgaagattagcaaaaatatttttggagactataaggaggatttttaattatgggagcaattgctgcaggtattgcaatggccggtgccgctatcggtggagctgttggtgatggtattttaatttctaagatgttggaaggaatggcacgtcagccagaattatccggacaactgcgtagtaacatgttcatcggtgttggtttggttgaagctatgcctatcatcgccttcgttgttgctttgctggttatgaacaagtaataaccggtttagtcaaatacacaaagaaggaggtgccaattgatgttttcatattcagtagttggagctcagctttatgttggtgatatgctgtttgtcatgatcacatttcttgttttaatgtggttggtcaagatcgttgcatggaagccaattacgaagatgatgcaagaccgttcagacaagattgttaatgatattgattctgccaaggaatcacggactaaagcagctgaacttgctcaaaaacgtcaggctgaattagacaaaacgcgtgatgacgcaaataccattattaacactgccaaacagaatggacaaagacaacaagaacagattgttgaagatgctagaaatgaagcatcgaatcttaagagttctgctgaaaaggacattgaacaagagcgacaagaagctttggctaattctcgaaaagatgtggcaagtctttctgttgaaattgcatccaagattatttcaaaagaattaaacgaagatgatcaaaaaggacttgttgactcttatattgaagggttgggtaagcagaaatgacattagatgatatgagcgcttcaaaaaaatacgcaaaagccatgtttgaagttctgagtgattctaatgaacttgaatctggttacgctgatttgcttgaattacgtaaaatttttgctgctaatccaaggttgattgaaattctcgatgatattcgagtttcagatgacgagaaaaagtctctgctggctcctatcacccaaaatgcatcagactttattaataactttttaaaggttgttgccagctatcgccgtttcccacaggttctgagcattattgatcagttccaaaaggtttacgaagatgacaagaagattgtccgggcgcaagttgtttcggcaacgccgcttgatgacgatcagcttgatcgtttggcaaaagcgtttgagaagcgggtaggtgcggttaaagccatttttgataccaaagttgataaatcactcatcggcgggatcgtgattcgatcatccgatgtgattatcgatggaagtgttcaaactcgcattaataaagttaaagaattattgttgaattaacgatatctatttaaagaggtgaaacttatgagcattaaagctgaggaaatcagtgctcttattaagcaacaattacaaggctataagaacgagctcgacgttcaagaaacaggtatcgttacatatgttggtgatggtattgctcgtgctcatgggctcgaaaatgcgttgtctggagagttgctcgacttcggccacggcgtttatggaatggtacaaaacctggaaaccaatgatgttggtatcatgattttaggtgatgacacgaatatccgtgaaggtgattctgtaaagagaaccggccgaattatggaagttcctgttggggacgagatgattggacgagttgttaattcactcggtgaaccaatcgatggtaaaggtccaattaaggccgacgatcacaaagcgattgaacataaggccccaggtgttatggaccgtcaatctgttttcgaaccattacaaactggtattaaagcgatcgattcattgattccaattggtagaggtcagcgtgagttgatcattggagaccgtaaaactggtaagacttcaattgccattgatacgattttgaaccaaaagggtcagaatatgaaatgtatttacgttgcaattggacagaaacaatcaactgttcgaactgccgtaagtacccttgaaaagtacggtgccatggattacacaactgttatttcagctgggccatccgaacctgcatcattgctttacattgcaccttatgccggcgcaacgatgggtgagtacttcatgcacaagggtcaacacgttttgattatctacgatgatttatcaaagcaggctgatgcttatcgtgagctgtcacttattcttcgtcgtcctccaggtcgtgaagcttatcctggtgatattttctatacccattcacgtttgttggaacgggctgctaagttaagtgacaagttgggtggcggttcaatgaccgcgatgccaattgttgagactcaagcaggggacgtttcagcttatatcccaactaacgttatttccattaccgatggacagatcttcttggatgccgatagtttctattctggtgttcgtccagccgttgacgctggtacttctgtttctcgtgttggtggtgatgcgcaggttaaggcaatgaagaaagtttccggtactttgcgtcttgatttggcttcatatcatgaattggaatcatttgcacaatttggttcagatcttgatgaagcaactcaaagcaaattaaatcgtggtgcccgaacggttgaagttttgaagcaaccacttcattcgccaatttccgttgaaaaacaggttgtcattctttactgcttaacccatggattcttggataaaattgcaattgatgatattttgagatatcaaaccgagatcttcgattacttcgatcaaaatcacaaagatttgttggaagatatcgctaagaccggtcaattgcctgatacaagtaaaatggatgctgcaattaaagactttgaacaaactttccaaccaagcaagcacgatgatcaacaatcaaacgatgatcaatcagctgcttcaaatgactagttttaaggagggtgagattacatgggtgcttcgctaaacgatgttaaacatcggattacttctactaagaagacgcgacaaattaccaatgccatggaaatggtttctcaggcaaaactgaaccagatccaaaagcatacggttagttatgcggaatatgcaagccaaatcaaatctgttgtattgcatttagcccaatctcacattttagatgggctaaacaaatcctcaggtcattcagctgatcaagatcaatctaagactaagagaagcgcatatttaattatcacctctgatcgtgggatggttggtagttataatagtaacgttatccgtgaagccaatgagtttattgagaagcattcgggatcgaatgattatcaaattctcgctgttggtggaaccggatccgacttttataagaaacgcggcgacaatgtttcttatgaataccggggcgttagcgatgtgccaacctttaacgaagttcgtcaaatcgtcaagatggtgacatcaatgtacgataaaggtcaattcgatgaattgtacgtttgttacgagcatttcgttaaccgtcttatttcccgtttcagagctgagaagatgctgccaatcgatgatgaagccattgcgtcagctgccagccaggacattgaagttaagccgatgagtgctgaatacgatgttgagccttctgaaaaagaagtcttggatgttgtattaccacagtattctgaaagcttggtttatggggcaatccttgatgccaagacttcagaacatgcttcaagttcgactgcaatgaagtcggcatctgataatgctgacgatttgatttcctcattggaattgcagtataaccgtgctcgacaggctgccattaccactgaaattactgaaattactggtggtcaagaggctcttagtcactagaaagatttgaatggaggaattaactaacatgagttctactggtaaagttatacaagttattggaccagttgttgatgttgaattctccttggacgataaattaccagaaattaacactgctttagcaattcacgtcagcgaagacaagaatttgattgtcgaagttgcccttgatttgggtgatggcgttgttcggacaattgctatggatggaaccgatggtcttcgtcgcggtatggacgttgaaaacaccgaatcttcaatcagtgttccggttggtaaagatactcttggtcgagtattcaatgttcttggagatccaatcgatggcggcccagaatttggccctgacgctgagcgttggccaattcaccgagatgctcctaagtatgatcaattaaacccatcaactgaaatccttgaaacagggattaaggtgattgatttattggaaccatacactcgtggtggtaaagttggattgttcggtggtgccggagttggtaaaaccgttttgatccaggagttaattcacaacattgcacagggacacaatggtatttctgtgtttactggtgttggtgaacggactcgtgaaggtaacgatatgtactacgaaatgaaagggtcaggggttctcgagaagacggccatggtttatggtcagatgaacgagcctcctggtgcacgtatgcgtgttgccctgactggtttgacaattgcggaatacttccgtgatgaagaaggccaagatgttctgttgttcattgataatatcttccgattcactcaggctggttctgaagtttccgccttgctcggccgtattccatcagccgttggttatcagccaacgttggctactgaaatgggtcaactgcaggaacgaattacttcaaccaagaagggtgccattacatcaatccaggccgtttatgtgcctgccgatgattataccgaccctgctcctgcaacgacatttgcccatttggatgccacaaccaacttggaacgttcattgactcaacaaggtatttaccctgccgttgatcctttggcttcaacatcatcagctttggatccagcaattgttggtcaagaacattacgaagttgccactgaagtccaacatgttttgcaacgatatcgtgaactgcaggatattatttcaattcttggtatggatgaattgtcagacgaagagaagacggttgttaaccgtgctcgtcggatccaattcttcttatctcaaagtttctcagttgctgaacagtttaccggcttacctggtaaatacgtatcagttcaggatactgttaaaggctttaaggaaatccttgaaggtaaatacgatgatattccagaagatgccttccgtaactgtggccctatcgaagatgttgttgaaaaagccaaggctatgaaacaggaatcagacaacgaaaagcagcgtgctgcaaactaaggagggattctaattggctgataattcagttattaccgttagtatcgttactcccgatggaaaagtttacgagcatactgctagtatgatagttgtttcaactcagtcgggacaactaggaattatggctaatcacgttccgattattgcaacacttgacgttgatgaaacgcgagttaaatacgacgacaaggaagacgatattgctgtcaacggtggctttatcgaattctcaaacaacgttgcgacaattgtggctgatagtgccgaaactcaaaatgatattgatattgcccgtgctgaaaaagcaaagaagaacgcgcaacaaagaattgccgaagcccgtcaacgacaggataaggccgctcttgatcgtgctcaagttgctcttcgccgtgcaattaaccgaatcaacgttgccgggaaataaccgttatttctgattgcggtttccggaaactgaatatggtacttcaaaagctgcgcccatttgggtagcagcttttttggttagtcggagttaatccttgaaattaccggtgaatcaggttagaattcctttatcgtgatttgtgaatgatgtatttatgtttgcgtttttctccagtttggtcggaatcatatacagtcattgttatccgaatgtgccgattagatagcaattctgcttatatttttgtaaaagaaaccgaaaaggtaagacaagttcgcgtctttatgatatagttgtctgtgaattgggggaagactcaaatgaatacgattggcattcaagcgctgattacattgattacatacattttgtttatcgctatggcgttttggacagttcaagaaatccacatcgagcgttatatcccattgagggcaatgccggggaaattactgatcgtgctcgtttcaattgcgattgggtacgcatgcagttcatttttcctctctgtaatatttaacattcagaatttgatgtatctaattaagtgatgtaggaggcgttcttgtggaaaaaattattgtacatggtggtaagccacttcgagggaaagtacatattgatggggccaagaatgccgttttaccaatccaagctgcaactattttagccggtgagggaaagacggttatctcaaatgtgccattgttgtctgatgtgtataccatgaataaagtgttgcggttcttaaatgtgaaggttgattttgatgaagccaataacgaaattacgtttgatgcttcaaaagatatctccagtgaagcaccttttgagtatgtctcaaagatgcgtgcctcaattgttgtcatggggccgcttttggctcgactcgggcacgcaaaggttgctttacccggtgggtgcgcaattgggtcacgaccgattgatctgcatttaaaaggatttgaagctttaggtgctcggatcgaacagcatgacggctacgttgaagcttacgccccggatggccttaccggcgctgaaatctatctggattttccaagcgttggtgccactcaaaacattatgatggctgcaacattagctaagggcaaaacagtcattcagaatgctgcccgcgagccggaaattgttgatttggccaacgttttaaacaagatgggggccaaagttgtcggcgccggaaccgaacagattcgcgtggaaggggttcctgaacttcatgggaccgatcacgcggtggttcaagatcgaattgaagccggaacattcatgatcgctgctgcggttacccgtggtaacgtgatgattgatggtgctattcccgagcataacaaaccactgattctcaaaatgcgcgagatgggcgttaccatcaacgaaagcgatgatggcattcaagtcatcggccacgataatctcaaaccggttgacgttaagacaatgccgcatcccggctttccaaccgacatgcagccgcaaatgaccattttacagttgacggccaatggcagcagctcaatgactgaaaccgttttcgaaaatcgtttcatgcacatggaagagctgcgccggatgaatgctcaatatacgatctccggtcgaacagtcatcatggatggcccaactgattttaatggcgccgaagttgcggccaccgatctgcgggccgccgcatccttggtgattgccggcttggccgctagtggctataccaccgttaccaacttacagtacctggatcgtggttaccacgatttccacaagaagctcgctaatttaggtgctgaaattaaaagagtcaacgttgaagacgactcaatcgtcttgaatcaatcgctcaagaatcgttcataatttttcggggttgggatcgttacttgatctcaaccctttattgtttggagacttattagaaacgcaaactttatgtggtataattattttttgagattaaagtttttcaggaggaacctacacagatggcaaaagacattggaattgatttaggaactgccaacgtactcatttacgttgccgggaagggaattgtattgaacgaaccatcagttgtcgcagtcgatactcggactggtaaagtcttggcagttggctccgaagcctatcggatggttggtcggacgccaagtaacattcgtgcgatccgcccattaaaagacggcgttatttctgattttgatattactgaagaaatgctgacatatttcattaacaaattggatgttaaaggatttatgtccaaaccaaaaattatgatctgtgcaccaaccaacgtgacggaaattgagcggaatgcgatcatgcaggctgctgaaaaggctggtggcggacaagtctatctggaagaagaacccaaggtggccgctgttggtgctggaatggatatcttccagcctcgtggtaacatggtcatcgatatgggtggtggaaccagtgatatcgccatcatttcactgggcgatattgttgccagcaaatccattcgagttgccggtgataagatgaacaccgagattgccagctatatcaagcaaaagcataacctgattattggtgagcatactgctgaaaagattaagattgaaattggaaccgctaagaaagacgattcagatgttaaaacgttggaagttcgtggtcgggatgccgtttccgggatgcctcgggcggttacgattgatagcaatgagatcgctgaagcaatcaacgataccgttcaattaatcatcagtggtgccaaagaagttctcgaagtgattccacccgaattggcgtctgacatcgttgaccgtggaatcatgctgaccggtggtggtgccttattaagaaacatcgatcaagtaattgccgatgcgctaacagttcccgtgattatttccgaaaatcctttggacaatgttgccaagggtgccgggatccttttggagcactatattaagaaccctaagttgaaggcaaaagatcaaaaataacaggagtcaaagtgaaaaacattctgattagtcttgttcatggttatcagcgctttatttcgcccttattcccgcctacctgccgttattatccaacttgcagcagttatatggtaactgcccttaaaaagcatggtgcgttcaagggggccgttatgggcattgcccgaattctgcgttgccatccgtttgttaagggcggctatgatccggttccggatcactttaccatttttcggaataaggacgcacgcgatgaataccggaaatccatgcacctgaaatgatctttgaacaaggagaatatgatgagtaaagcaaataaaagtatcaacgttgaaattaaagatcgaacggatcaaaatggagaatcgatctccgaattatttatcggcaagaaattgattggctcaattaagcagttgagcgaaactaaatttcaagcagtcaacactcacgacgaagcgtttcatgttaaaaccttcgatgagggtgtgacacaattaatcaaagattttcatcttcaccattaatttggcgatcgaaaacgaggagggtctaatttggatagcagtcgcagaacctctaaagacgaccaatcgcgaattgactggggaattattttctgtgtcttaatgctggcgttgattgggctggcatcgatttacgttgcagccacccatgattcaagttctaccagcgtcatgagacaggtggtttcgcaattggtttggtacgtcatcggaattatcgccgttgtcattattatgcagtttgattccgagcagttatggaaagttgccccgattacttactggctggggattgccctgctggcgagtgtcttggtgttatacagtcggacctattacattaatacgggtgccaaaagttggttctccctatttgggttgacctttcaaccgtctgaagtgatgaaaccggcctatattttgatgatggggcgggtgattgttcaacataacgataattacccaatcaggactgttcgaagtgatttcctattaattgggaaaatgttgctgtggacagttccggtagccgtcttgttaaagctgcaaaatgattttggaacgatgttggttttcttcgccatcttaggtggcttgatcatcgtttcaggagtgacatggcggattattctgccagcggtgattaccatctttggatttgccggaaccatcttggctttggttattccggagtccgggcgtcatctgttggagaagtttggttttcaagcctaccagtttgcccgagttgacacttggctcaacccgtcagccgatacttccaatcaggggtatcagttgtggcagagtatgaaggccatcggatctggtgggatttttggaaccggatttaatcagtcacatgtgtatgtgccggtgcgagaatctgatatgattttctcggttattggcgagaactttggatttattggcagctgtattttgattttattgtatttcctgttgatttatcaaatgattaaggttacattcgatacgaggaatgttttttacgcttacatttccactggcgtgattatgatgattctgtttcatgtttttgaaaatgtcgggatgagtattggcctgttgccattgaccggtattccattgcccttcgttagtgccgggggatcggcgttgattgggaacatgattgggattggcctaattatgtcaatgcagtatcataataagagttacatgtttggagaagacaaagaattctcataatttttagaaaaggtggaattaatgatggatacaaaatattattggactgaagaaaataacggggaagtcacagttggcttgaccgaagcaggcaagaacgaactgggtaacatcacctttgtttcccttccaaaggttggtgctcaattaaccaccagcgatactttattaaacgttgaagctgacaaagccgtttcggatattccaagtccagttgctgggaaagtgactgctgtcaacagtaatgccgttaatgacccttcagtattaaacgggactgacaaggcaacttcatggattgctaagattaaaaaataaaagttcttgacgctaggactttttttaggtacactaactgatagtttgatgatagaaaaattacaagatgagtagataattagagattgtcaagagagcccggctggtgggaaagggtcaatcatcgttattgaagatggtcttggttaaaaatgtgtcggtgagcaattgcaagccgataatgggtaacgaccattatttcgttgagtatgaagatactcatgaggcgattgttgaaagacaatcgcgaataaaggtggtaccgcgaagtttttcgtcctttcataagtcaattaagacttatggaggatgaaaagctttttttgtctaataaggggtgaaaagattgattcgatttaaagatgtatccaaacagtacagtaccaaggatggcggtctaaccgcggtcaatgatgtcaacattgagattaacgatggtgagatcttcgggattgtcggctattcaggcgccgggaaaagtaccttggtgagaatgctggacggacttgaagcaccatcgaccggtgaaattgacattaacggaacggatgtttccaagctccacggcagccaattaagaaagcaacgtcaaaaaattggcatgatctttcagcatttcaacttattgtggtcacgaacggtgctggacaacattgctttaccgcttgagattgccaaagttcccaaagccaaacgaaagcaacgcgcagaggaattgatcaagttggttggtttggagggccgtgagcattcctatccttccgagttatccggtggtcaaaagcaacgggttggcatcgcaagagccttggcgaacgagccgacaatcttaatttcagacgaggcaaccagtgccttggatcctgacacaactaatgaagtccttgacttattactgaagattaataaagaaatgaacctcacaattttattaatcacccatgagatgcacgccatcgccaaggtttgtgaacgggtggcagttatggacagcggcaaagttgttgaaaccggatcagtgtttgaggtcttccgtcatccacaacaagaaatcactaaaaaatttgtcagtgaagaatttacaccacaacaaagtgacaacacgatgacccttgatgaattggttaagaaatatcctgatgggcaaatcatccgactgattttccatggaccacaggcggaactgccaattgtctcggatgttgtcaaacggttcccggaattaaccatcagcattatttccggtgccatccatcaaactcaagaaggcgcgttggggtcgctggatctgcaatttgtcggcgatgacaatcaaattaacgatgccttggaatacctgaaaaagatgcgggttggaacggaggtgattcatcatggctaattcaactggattcaaatcttacttccagtttcataacgtcgattggggttcgatgatgtcggcaacttgggaaaccgtttggatgaccctgttatcaatggttgcaattgttattttaggaattattttggggctgatcttatacgagactcgcaacaagccgggcattggctatcgaattctcaattggctggtcggcttgttcgttaacatcttccggtcaattccatttatcatcctgatcattttgttactgccaattaccatgaaattggctggaacgatcattgggccgcgggccgcgttaccatccttgattatttcggcggcacctttttacgctcggatggttgagtcctactttcgtgaggttgattccggggtcttggaagctgccgaatctatgggtgccacaacctgggaaattatcaccaaggtcctgttaccagaaagcaagccggcattgatcgccggagctactgttaccaccatttcgttgattggctacaccgctatggcaggtgccattggtgccggtggccttggaaacttagcttatcaagatggtttccaggcaagcaacaacacagtgaccttagtcgcaacggtcatcatttgtttatttgtatttgtcgtccaatttgtcggcgatgtctttgtcaagattaccgacaaacggacattataatatttgggagggtttcaaatgaagaagaaattattgagtttattcgcagttgtctttaccgcctttttgttggtggggtgttcatcatcgtctaattccagcaaaaagacgaccacattaaaaattggtgcttcagccgtgccccatgcacaaattttgcgccacgtggctccagaacttaaaaaagaaggcgtcaatctgaagattaccactttccaagattacacgatgcctaacaaggctttggccaacggcgaactggatgccaattacttccagcatgtgcctttcctaaagctttggaacaagcagaaccacggaacattagtcaatgccggtggtgttcacttggaaccgatcgctgttttctcgaagaaagttaagaagcttcaagatctcaagaagggtgccacaatcattgtcagcagcaatgttcccgattatggccgaatccttcagatcttcaaagacgccggtttaattacactgaaaaagggcattgacattacttctgccaacttcagtgacattgcttcaaacccacgtcatctgaaattcaagcacagctatgaaccaaaattactgccaaccatttataagaatggtgaaggagatgcagttgtcatcaacgccaactacgctgttggtgccggcttgaatccaattaagcagtcaattgcgattgaaaaacggaattcaccatacgtgaacatcatcgccacccgtaaaggtgatcagaacaagccagccatcaagaaattagtcaaggttcttcaatcaaccaagactcaaaaatggatcttgcatcactataaaggtgccgttttacctgagaagaatgttaagtaattaatatcaattaaaagccgtccgctatatacttgaattagtaattgtttactaatccgagtttatagggggcggcttttttgaaagagaaaaatgtatttcatgttaatggttatgtgggcttaattattgccttgattttgctgggagttggcggttatctgctctggattggcggggaaggcagctcaattggctcaatcgtttttgggacaatcatcattgttttggatctgttatttgcaagttcattaacgattatccaacctaacgaagccaaagtgttgaccttctttggtcgctacattgggacaattcggacttccggattattcatgaccgtgccattgaccagcaagcagacgatttcactgcgggttcgcaattttaatagttcaattatcaaagtgaacgattcaaaagggaacccagttgaaattgccgctgtcattgtctacaaagtcgttgattctgccaaagcaatttttagcgtggaagattatgaacaattcgttgagattcaaagtgagtccgctattcgacatattgccagccagtatccgtatgacagttttgatgatagtacagacaaattgaccttgcgggggaatgcaaccgaagtgtcggtcgcgttacaaaaagaattacaggaccgtttggacgtcgccggattgcaaattattgagacccggttgacgcatttggcatatgcaactgaaattgctaacgccatgctgcagcgacaacaagcaaccgccattttgtcggcgcgaaaaattattgttcaaggagccgtggcgatttccgaggatgccgtttcccagctgcaaaaggatttgggatcatcgattacagatgaacagcggatgaaaatgatcaataacgtcttggtctccatcatcactgaacgagggacccagaatgtcattaatactgataatctagattaattaacgcttttagacgattaagaggctgaatgttatctagcagaactgtgggccaataagcagcttccggccgtataaggggattacccaaacatccaaattccggatattcgggtaatccccttatactctggaagctaaccacttattggcccacgcttttttgtttttggttgacatccggattcttagcatatatagttagttacataagtaattaactaacacacggaggaacacttatgacaactaaaatcgttcaaacagaagatttacacaaaacctacgataaagacagcgcaaaaccatatgaagctctgaaagggatcagcttgtcggttaacgagggcgaatttgtcggaatcatgggcgcctccggttccggaaagacgactttgctaaatattttggcaactctcgatcaaccaaccagcggttcggtcgaaattgacggccaagacgtaactcatttaactgccaaccagatggcagattttcgttctcaaaaattgggcttcatcttccaagactttaacttattggaaaccttaaccgcccaagaaaatattgctttgccgttgtcgcttcaaaatgccaaggcggctaagatccaaactgctgtcaaggaagccgccagcaagttgggaattgatgacttgctgagtaagtacccaacgcaattatccggtgggcaaaagcaacgggtcgccgctgccagagccttagtgtcaaatccgtcaattatttttggggatgaaccaaccggagcgcttgactcaaccaacgcccgtgaattactggacaccttaacgaacatcaatcaacagggggtctcaattctcttagtgacccatgacccgttctccgctagtttctgtaaacgaattttatttatcaaagacggaaaaattggcgatgaggtagacgccggcgataagccgagaaatgaattctatcaggaaatcctcgaaaaactcggtacatttgaacagtaatcaatcaaaggagcttagcgatgttatttaaaatttcaatctcaggaatcaaggctcgttggaaagattatctggttctgttttccgggatgatcattaccacagctattttctacatgtttgaagcaatttcaacaaacgataaatttaccaccagcagtgcggtgggacaaaatgccaagatcgttttcatcttcggatccatcttactggcaatcatcacactggtatatgttttttacgcgaataatttcttgatgagtatgcgtgaacatgattatggactcttcatgatgctgggtgccaaatcaggagtcatcagtaaattgatcatccttgagaccattgcgatcggtttaatttccacagttgtcgggattgtcattggcattggctttacccaagtgctcagccattttctggccagcctcattcacatgtcattgactaatttctcggcattttatatgccagctatcattgcaacgattatcctgtttgcgattttgtttctggttgctggtttcttaaatgccaggacattcaccaagacctccgccctgcagcttttgcgttccggacaacaaagtgattggcagcagcctaaggccttgacacttggcgttcaagcaattcttggagttgttctcttggccggtggatattatgcgatgtatgacattcaaaaactgaaagttatgtctattccaatcgcgctcatcacgattgttctagggacctactttgtcttcaactcattttttgtgatgctgctccaggcatttcaacgttctaatatgagcaccaagggcctgaacagtttcacattggcccagcttaaatttagaattcgtgattataccaaaatcctttcagttgtctcactgctgtttgcattggcactaggcgcaattactgtgggaaccggttttcaacacatggtacctaaattagcttctggaaatggctactattcagttgctattaccaaccccaatcaggaaatgcgttcactggttggccagattcaagataaatccactgtcacttaccaacaaaaagttgatccgacgaccaagcgggtttattaccggagtgaccagcttcagcgccaaccattgaagtacgcggcgtttgtgagtcgaaagacactggcgtcaaaagctttcaccgccaaagtttcccagttcaagcgaagcgattcatcggcataccaagagctgtggggactacaggtaccaacggttaaagcctaccaaatcaaagtggtcagttctcagacattcaatcaaattaatgccaagaccaatcaattattgttggttcgcgcaaatgatatggacgctgccgcaacgccactgaccaaaattaccaacattcagtccaagcagtacggctatcgaaacggggaacaggtcggcggttcgtttacgatgtatcaatccctgaagagtgtctttggcagtcttgagtttatgggaatcttcttaggaattgcctttctggccatgcttgccagctgcttaatgtttaagattttgagtggggcagccagtgacaagatccgctttgatatgctcaataagattgggactcgtcgatcagtcttaaaccactcaatcgttgttcaaatcctgggcttgtttgcactgcccggaattttgggaattgtcgacgttgcctttggccttcaaatgttcgccaagagtggtctattgatgggtggcgcctaccaaacctttggactgacgacagtcggcttcttggttctttacttgatttactttgccgtgaccgtcctgatttattcccgaattgtggttccaaagacgaaggtggagcgttaaatgaaagaaattatagaatgggttgataaatatgaagtttgagtttaatagttcagagcccatctaccgccaggttgccgaacaaattgaggacgcgattgcttcgggaggctttgctgaaggcgaccagattccgtcgacaacagaaatttccaaggagtttcatatcaacccggcgactgttttaaaagggatgaacatcgttgctgctaaaaatttgatcgaaaaacggcgggggctgggaatgtttgtccaggcaggcgccaggcagcgaatcttggtagaaaagcggaatggcttttttgatgagtttgtcgaaaatctggttcgggaagcccagaatctggatatttctgaagatgagttattgaatttagtgaaaagaggttaccagcaatgagcgtattggaagtcagtcacgtctcgaaatcatttgggtctaagcacgtcttgtcagacattaatttgtcatttgacggcaacaaaatctacggcttacttgggcgaaatggtgccgggaaaagcacactgctcagtattattaccgaccggatttttgccgacagcggcgaagttaagattgattctgaggatgtcagcgataacgactcaaagctaggtttgatgtatttgatgagcgaggccaatctttacgctgacggctggaaattgacccaaattctcaaggattccgaatctctgtatggcggattcaaccatgaattagcggatcacttgatcaaagaatttggcttggatatcaatcaaaaatttggtaaattatccaccggttacaactcgatttttaaactcattttggccttgtgcctcccagtcaaatacgtcttgctggatgagccggttctggggttggacgccaaccatcgggaactcttttacagtgaattgattcaatcttattccgataacccgcggacatttatcgtttccacccaccttatcgaagaggttgccaatattatcagcgacgtgatcgtcttggatcaggggcgagtgattttaaaccagccggttgaagacgtcttggccaagactcattcggtcgtgggaccagaaaaagacgtcgagcaatataccaagggcttaaacgtcattggccacgacatgatgggcaccatccgggccaactacgtctatggtgaccttgacgaccgcatcctgcccgacacagtccagctgtccaactttgacctgcagaaactgtttattttcctaaccaatcaatatgaggggagtgccaagaatgaagacaaataaagtcaccaaattcctgtttcgacgacagattatcggcttagcggaaatgtatctgttcttgtttgccgcctttttggtactaccgtttctgttttctgccatctcaggatctctgaatgattattccttaaccaatcagatgcaggggtcctgggtgacagcggcgtttggcctgtatatgtttgttatttcaacgctgtcctatgaaaatttcaagtttttgattcaaaacgggatttcccgagaaacttttttcaatgcgcaagtcattgtcaatggcttgttaatcctgatcggcaatacctttaacttggtgtatcagtacgccgtcttgatgccattggggcatgccagagacaccaacatctacatgtcctcgtacgctggatactttaataacccaattgtcgcatttttgttcaactttatttttagcggattgttgttaatcgttggcgctttgagcgggatggttatcgggaactttctaacgttattctctaaatttgtccagcggatcattttgatcgccacgccggtcatcggctacatcaccgtgatgtacactgcatctcgggttattttggatcgcaattttcagatgacttgggttgccaatttcgccaaatttgtcctcggataccgggcaacgggtgcctacgatccatttccgatgattgtgagcatgctgatcgtttctgtgatcttgttgttgatcacccgctacttgttcagtaagaaacaattaaaacgtgaataattgtgatcggtgaattcaacctaaaaatgtgatgagaagcgtttgtaaatgttttcaactgtgaagttccgtgatatacttaagtttctggaaactatacgaatttataaaaggatgagaattcatggaaaaacacaaaaagcaacacattggcctcatttttggcggtaactcttcggaacatgatgtctcaaaacgctctgctcataacatttatgacgcaatggataaagaacgttacgatgtgagtttgtttttgatgaccaagaacggctacttcctggatcatgaagcttcctctcgggttttcgacggagaaccggaagacgaggttgccaagcaggaattagctaaattggacctcaagaatcctttggctcggataatcaacctggctgaagaatccgatattgacgttttcttcccgattattcacggtaatttgggtgaagacggaacgattcagggactattacgtctcctgcacaaaccatatgtgggaacggcgatcttagggtcagccatgtcatttgataaggatattaccaagaagattgtcaaactggccggagtaccaaccacccgctatgaagtgattaccccgctgacggccgagcagtacagctatgactctctcagtgatgaactgggacagactttgttcatcaagccggctaaccagggatcttctgttgggattcacaaagttgaaaatgccgaggaatattccgaagggattcgcgatgctttccgatacgacagcaaagtcctgatcgaagaagcgattgaggggccggaagagctggaaatttctattctgggtaatgatcatccaatcgcatccaagattggggccattcgcgtacccaaagacgacgccttttatacttacgacaataaatttgttgatgccagtcaggttaaatttgacgttccagtggacatctcggaagaacttgcccaacagatcaccgaaatgggcttgacgacttatcgggcattgggactcaaggggatggctcggatcgattatctggtttctaaagatgacaagccatatatgagtgaggttaatacgctgcccggattcaccaacatcagtttgtatccgcagctgttcgccgcctctggcatttcatattctgaattaatcgatcgcttgatccaactcgccattgatgagtttgaacgtcagtcaaaaatcttatatgactttaagccattgccaccacgcgatcaaaatattaacaagtagcataatcaaactggcgcagaattctgctgccggtttttttgcatgtagggaagttttttgatggggaataatgaaacgaaactttatgattatttaacgggggcattgatcgtccttattttgctgttgagacgttttttggacacttaccaaagcttcgcaacggtggtattttgttcgctgacgatgtttttactgttggtcggtctattttattatgggatcgtccaaaccgttcacaagacaattttgagccgaccgtggtcactattggcgttgctgggaagcggtgtttacctgtttgttctgctggtgccattaggcctgtttggcttctcaaatttcattaagttttcggtgccgatttctggaaatcagttttcctggctgacagtcaatcgctatccgcttgcgctgacggccattgttggctattttggcctagtgctggttgggatttatttttctcattttgcgttgaacttgcttgctgcggatggcgatcatccaattcaaggtttgaaacagactgttaaattgatgacgttgaaaaagtatggccaaaagctgctcttattattttcaatgctggttggcatctgcctgttgattcttgggctgggctggttgaacagattgcttcccaattccgtcctattctttttgtcacaaggaacgattgatgtggtggctccatttgtcgaaatcgttgtgattggtcgcctgctgggcattcagtttgcccggctgacaggaaaggggctgattactggtgtgggcggatgtctgattatcttctcagcgctgtttgccgggatcaatcccgcgttttccgttcgaccggtcggccatcccacgatcattgttcaccgcggggtcattaatcataacgctcagggaaacacaattactgctttgaagcgtaacagccattatcactttccatttgttgagatggatattcaagaaaccaaagatcatcactttatttgtgcccatgataacgatgtgccaattccaggccacggggatcaggagattaaccgcctcaatctggcagaaattaccagattccatcacgttgatatgttcgctgattatctgcgaactgcgaaccgattaaagcagccgctcatcattgaattgaaggtaactaacagcagtgacccacagatggggactcgatttgcccaacagtttgcctctcaactgacggttttaccacaccgggttcattcggttggttatccatttctccgacaaattaaacaacggattccacaaatcaatgttggtctggtgactatgcttaattttggtaatattggcaagtacaaggtcgatttttacacgctgcagcatctgaccgccaatccattcttgatttcctcggttggcagaaccggtcggccagtctattcctggacagatgatagtcagttatcaatgatgcgaatggaaatgctgggcatcaccgggcaggtcaccgatcaagcgctgcgtcttcaaaaattacgggttaactatcaaagggaccgttggattctacttttgaactcgttgcagaattatttgtgactttttcgtaggtttatagtaggaggtgtagtgatggttaaaagatgcccttgggcaactaccagccctgaactattggtttatcacgatacaatttgggggcgggtacaaaaggatccgcaaaaactattcaaagccctgtgtcttgagacgatgcaggcaggattgtctttttcaacgattttaaaatttgaaccgggaatggatgaagtctttcaccacttttccctggattatttggccaagtgtgaccagtcagatgtcgaacggttttgtcaagatcgtcgaattatccgtaatcatgcaaaggtcagtgcgataattgccaacgccaaagtcattcaaccgaatcctaaaatgttagttgaagcaacctggggaccagttaatggggtttcactggatcatttactaaaagcagcgccagacccaaaaatgtatcaaaaatttaccgaaaagtttgtgaaggcctttaaaaatatgggcctccaacggattggcttaattactgtgtacagctatttgcaagcggttggcgttgtgaatgatcatctgatcacttgtgattttcatgaggaatttcccaccaaaaatgaggaaaaatcttcttgattgtcgattataaatataatatgatactcaggttgtatgttaagcatgttaactatagggagtcgttgtatgacaatggtgattactggggccttgatcaaaaaggcaagaaaagataaggggatgtcccaagttcagctcgctgaagggatttgtacccaagcaaccatcagttccatcgaaaatcaaaatacgtgcagcagtgttgacattctggtcaacctctgccaaaaactggatttaaaaattaccgatgttgccaagaatacgcgatatggtgataaagtcttctcttacattgaagacgatatgcggaatcatttgtatgccgacgctaatagacaaattggtcggattgactgcaaaaagttgaatacccgatatatgttgggcaagtatcattgctatcggggattcattgaattgtatatcaatgatgatattgatgaggccattttcaacttcaatcttcaattgacgcagtattccgctgatgaatttaccttttaccaagcctggtccaatttgggcattggtctggcttatcaaaagctggggaaattggatcgcgccgaagggttcattgattccagtgccaaaattttggctaaagtcaaaaaggccggcaagcacgatatgatcgtgattgttgacctctatgtggacattattgccgcgtacgccgagttgggtaaatatgatcgggcgctgccgctcattcatgaaattttacacgaattgacggagcaggatttgatttataaggtggacgtgctggcggagttggaatcaaaatgcctgtatcccaaaggacaggtcgtccaggccactatgaagcagtttgcagcgatgtttattgcggaacttcgcgggaacacggaattggctgagaaaattcttaagcgcaaccagtcccatattgtcgagatggtcaaaaacgagcttgcaaaaagtgaggggcatccgacctttgttaagtgatggctaggatgttagctgcaaaaaggcagttaaaacaaaaggatttgacttttgttttaactgcctttttagcttgctttaatcaatttgatgatcgaaattggaaaaattaaacgtgcttgcttggattaactgccggcttattgtccaaatcagttctaacgaccaggacatcgcaaaccgcagttctggtaacatattcggtaaccgaaccaattaagagtcgttcgacggcattcaaaccagttgcaccaatcatgatgaggtcgatgttgaggttttgaggaatgtctctggcaatcacggtctttggtgcaccatattcaattgagtaatcaacatcgttgagccccgctttttttgcatcttcgatgtatttgtccaaagtttcctttgcagtatcggtcacttgttcgaccattgatgtgtcaaaacttgaaatattttgaaatgcacgtgtatcaacaacgtggactaagtgaagagatgcattattacggatcgcaactgctacaccttttttaaaagctaattcagcctcgtaggaaccatcaactgggaccaaaatttgtttatattgttgttgtaacattatgcccaccctcatttctatctgtttaacttaattgtactttactttcggcaaaatacaaaggaataaatctattaccgttgtttatggttaatgacgttgagaattgcgaattcaacaaccagaccatgtgcagtcatccacaaaagaaccactaaaatgagaatatcattttgaatgattaatgccagaacgcccaaggctgccaaaatgatgaacatgatgccgccgtttttggcagctcctttcaggcggggatcatcttgaactgaaatattaaacatggttttgtgaaggtgggaaagtaagtagtagccaatatatagggcaattaacacggcaacagctactaaaatattaattatcattattacactccaatactatttatgaccggctatttatgaccggcagattttctaagcttggcatattgttctttaaacgcggcctcaattcgaccgttttctttcgggtggtaatactgagcatttttgattttatcaggcaggtattgttgtttaacccagtcgttgggaaaatcgtgggggtatttgtaggtcaccccgcggccaagtttcttggcaccttgataatgcgcatctttgaggtgcagtgggacatcaccatagttaccggatcgaatgtcacttacggcaccatcaattgcggccatcgcggaattggacttgggacttaaacaaagctcaatgattgcgttagcaagtggaattcgtgcttcgggaagccccagttgacgcgcagcgtcaacagcagcaaccgttctttgacatgctcctggattagccaggccgacatcttcataggcaattaccagtaatcgccgcatgatcgaaaccaagtcaccggattcaatcaatctgccggcataatgtagggctgcatccgtatccgagccgcgaatcgatttttgaaaagcagaaatgacgtcgtaatgggcatcaccatttttatcggaattgagtgcttttcgctgaaggcattcctcgacgattgcctgggtgacggcgatttttccctgatcatttttgggtgtcgacttcactgcaagttccaaggcatttaacgatgagcgcaaatcaccattagtggcagttgccaaaaagtttaacgcttctttggtaatcgacaccggataattacccaaacctttttctttgtcgtttaacgcgcgattgagggctttttgaatatcagttgcggtgaggggatgtacctcaaaaatttgggttcgcgatcgaatggccggattgatgttaatgtatgggttctcagtggtggccccaattaaaataattgagccgctttcaagtaatggcaatagaaaatcttgttttgttttatcgagtcgatgaatttcatcgagcaacaggacgaccgtgccgctcatcttggcttcctcggcgacaacctgtaaatcttttttggtgtcggtagcagcgttgagaactcgaaatgcatatttggtcgagccggcaatggcgctggcaatgctggttttcccagttcccggcggcccatataaaatcattgacgacagcatcttggcacgcaccatccggtcgattattttacctgggccgactaaatcctgctggccgacaatttcttcaagcttggtcggtcgcattcgataggcaaggggttgttgcatactcatcctcctctcaaattgtgatggttaaaaatcaaatcctataaattataacatgatcgtgagggcacaaaaaaagcgttttgcataagcaaaacgctcgctgaatgattaacccaacttgttgtagtattcaacaatcagtgattcatcaatatcagcatcaagttcttcacgttgtggaagacgaaccaatgatccttcaagcttgtctgcatcgaagctgacgtattgtggacgacccacaacagcttcaacagcatccttgataacttggaggtctttagacttctcacgaacagagattacttgaccaggttgaacttcatatgatggaatatcaacacgtttgccatcaacagtgatgtggccatggtttactaattgacgagcttgacgacgagtagtggccaaacctaaacgataaaccatgttatccaaacgctcttcaagtaagatcatgaagttaacaccatgcttaccttcacggatcttgccggcacgaacgaacaagttactgaattgacgttcagtcagtccgtacatgtaacgaagcttttgcttttcgtgtaattgcaaaccatattctgaaagttttgaacgacggccttgaccgtgatcaccaggagcataaggacgacgtgagagttctttaccagtacctgacaaagagatacccaaacgacgtgaaattctccaacttggacctgtatatcttgacataagtaatcctccaatatttttttggagtaaaataagccgttgcagacttagtattcgtgcatgttgctttgctctttcgctcaagcagccgattgagttacttgcagaaccaattgaatggcaacaacatgttgacgagcttaccgtctactgctgcgttattttacacaaccatcattgtataaagatttctactgtaagtcaacatgtttgacgaagatgtcggcaaactggttaagaacctgctcgtcttcactcgaaaaacgatcaagtgatggcgaatcaatatctaagacaccaagggctttgccgtctttaaacagtgggacgaccaattcagaattggaattggcatcacaagcaatgtggccggcaaattgatgaacgtcggcgactcgtagtgaatgcttttgtttgagagccgttccgcagacaccatcaccatttttgatgtgcatgcaggcaacatttccctggaaggggccgaggatcagttcatcgttagcgggcacataacgataaaagccgacccagttgatatcttcgaggctgacttggagcaatgcagcggcgttagccatgttggagatcaaatctgtttcattttctaagagtgaatcaagctgttgattcactaaattggtaacgttttgcataattgttttcctcacttcaaaaataatatggtgaaaaggacctactatgatataattcaacttagagcacattaattgattattcatacatattaaattgttttgggcaattttactaccataatgttcaattatatatctttatttctgaaggatgggatcgaatgcttactttgttgattggaattatcgtgttggttggggcgggttatcttggttttgttttctaccaaagaagaacaatcaagatggcaaccgatgtttacgagaacaaacgggatttaaacaaaattccgttggatgatgagtttgcgctggctaagaaaatgaacttaaccggtgaatctcacaagaaatatgatcaattatacaataagtatcagcactacaagaaccaaatgctgcccaatattgatgaggggattgcggcagtcaaagaagacggtaagggcattaactttttaaagaccaagagtgactggcagagtgctaatcaggccatcgccgacgccgacgccaccttaaaagaaattcaggccggccttgctcaactatatgatttaaacaagcagcacaaattagcgctggaagaacttgaaaagaagtacaaacgcttgcgagaggacatccttaacaagaacgagtcatttggcccgagtatcgacagcttggaaaaaatgctctcggacattgagggaactttcgatgaatttacgcaacttaccaagagtggggatcccaacagcgccgaagaagtgttgagtgacctcaacaattcgactgacaaattagaatcctatatggggcgaattcccaaactatatcaactactttcaaaggaatttgttgatcaggttgacgaaatcaccagtggttacaaagaactcaaaggaaaacagtataatttccccaacgataagttcgatgaaacgcttaaggggatttcagatcagataaaagtcaacaccaataagttaaagactttggaagttgattcagtggaaaaggccactcaagatattgccgaccggatcgacaaattgtatgatgcaatcgacaaagaattccaagcccgtcccaaggtcgagaagaataccaagattatcggccaatatatcgaacatgtccgtaaacagaacagcgacttgcagctgcggcttgaaacattaaataaaagctatattttgaaccatcaagaaattgagaataatcatcaatttgatcaacaaattgccaccattgaaaagaagtaccaggatgaagtcaacgccatgcaaaatgggacggctgtttattcaacgattgacgccgaccaaactcacatgatcaaagagctgggtcagatcgagtctgaacaaaaggatttattctccgcaacagttaagttgccagagcaagagcaggcagccagaaatgcattggccaaatttgatttggcaatgcgcaataccaaacggcgaattgataatcacaatcttcctggactatccaacgattatcaagatgcttttgcagcagtcattagggaaatcaatcacctggacgatgccatgaatcagccgcagattgatgtcgatgacatttccaaacagttaacaattattcaatcggatatggacactttggatgaaaagaccaaccagttgattgatgatgccgctttggccgaacagacaatgcagtatgccaatcggtttattggcagcaactctgaaattgcggcggccagcaaaacggcccagatgtattttgaccaaaaatacgattatgagcagagtttgaatatcatttccaaagcattggaaaaacaatcgtcggggatgtttgccaagatcaaagatgattatttcaatgccaagaaacatttaaagacagaaaaaaccgatgaagatgaatcataatatgacgtatgagacgaagctgaatgttcaccaacagcttcgccttttgttttccatcattgattgcccagcgacaatgcttgtgagactcacagtttgggtgtatcatcgtgggagttatatttgttggagtcgaaccaataaatttagagaagaaggtttcaaatgatttattttgataatagtgccaccacaaaagtcttaccagaagttcttgacacttataacaaagtgagtgagcagatttggggcaacccatcgagcttacacaactttggtgaacaggcgtttaatctgttggaacagtccagaaaacagattgctgatttgttaaacgttcacccagatgaaatctactttacgagtggcggaactgagggtgacaattgggtcatcaaagggactgcaattgaaaaacgtgaatttgggaagcatctgattaccacctcagttgagcatgcagcagtgcgcaactcttttgagcaacttaaacagctcggatatgatgtgacttatttaccggttgatgatgaggggcggatctcgattgctgatttgaaagcggcaattcgtccggatacaacgctggtgtcaattatggcggtcaacaatgaaattgggacgattcagccgatcaaagaagcgggcgaactgctgaagaactacccgaaaattcattttcacgtcgatgctgttcagggcctcggcaagggaattcaggatcagattttcaatgaccgaactgactttgcagcattttctgggcataaattccatgccccacggggaaccggctttatttatggtcgacgtggccgtcgaattgcaccgttaatgaacggtggcggccaggaaaagaatcaacgttccggtactgaaaatctgccgggaattgctgccatggccaaagcgatccgattggtgcttgaaaaagagcccagtgcaattgatactgagcgccagattaagcagttgattatggatcacatcagtcagtttgataaagtcaccattttttctaagaatgatgatacttttgccccgcatattctttgttttgcaatcaagggggttcgcggagaaaccatcgttcatgcttttgaaaagcaggggatttacatttcaacaaccagtgcctgctcatcaaaggatcatactgaatccggcacgttgaatgccatgcaggttcccgatgatattgccaccagtgccgttcgaatttcacttggagatcacaacacacttgatgaagccaaacaattcgtaaaagtatttgaccagttgtatgaagaatttgacaaattaagttaggagtaactatgcactatacagaaattatggttcgttacggcgaactgtccacaaagggcaaaaataaaaaagactttattaagcagcttggcaagaatgtgcgggctgttctccatccatttcccaagcttgaggtcaaaccgcaacgggatcgtcttcatgtggctttaaacggtgaggatgaccagcaggtgatcgaaagcctgaagggtgtttttgggatcgaaaatttctatccttctgttcggcttgaaaagaatatggcaatcatcaagcagaccgcccttgaaattgtgaaagaacagtatcatgacggagcgacgttcaaaatcaacacccgacgtcaggataaacattttgaatacgataccaatcagatcaacaaccagttaggcgattatattctcgaaaatgtgcccggaatcacggttgatgtcaaacaccccgatatttccattcgagtagaaattcgaatgaatggtgcctttctctcatcagaaaagattcatggtgccggcgggttgccggttggtaccggtggtcgggccacaatgatgctgtctggtggaattgattcgccggttgccacgtatttggcaatgaaacgtggtgtcaaaattgatatgattcacttttacagtccgccatataccggcgagcaagccctgaataaggccaaacagttaacctcagtgttgggcaagtactcgggtaatattcagttcattcaggtaccgttcaccgagattcaagaaaccatcaaggaaaaggtccctgaaggttatttgatgaccatccagcggagaatgatgctgcggattgctgcccaaattactcaaaatcgtcattgtaccggcgtctttaccggcgaagcactgggacaagttgcctcacagactttagagagtatgatggcaattaacgacgtcaccacgatgccggttcttcggccgctggtctcaatggacaaaacggagattattaagatttccaagcagatcaagacttacgacctgtcaattctgccatttgaggactgttgtacgatttttacaccgccggcaccaaagactcggcctgatttggccaagtcacgtaagtttgaacagtatatcgatgttgaagggttgatgaaaaaagcaatcgacaacattgaaattaccgatattaaacctggcgaagaattcctaaaccaaaaccaggacgtcttcgctgagctgctttaatgatcggggacttgcgtattccgtttgtttaggctacattatgtataaagtcgttagaccaagggagtgcttttatgaaaatcacgatcaatggtaaagaagagagtatgtttggcaatccacccgaagtcggtgaacaactgccaaagtttaaacttgaggatgcagatggcaataaggtgaaaactgctgacattattggcagaattaccctgctgtcaacggttccggatattgataccccggtttgttcagttgaaacccgcaagtttaatcaagaagcggataagtttcctgatgtccagttcttgacggtttccaacaatacgattgaacagcagaagaattggtgcgctgctcagggagttgccaatctgcagatgctgtcggacgaaaacctctcgttgggatacgcaatgaaactttatctgccaaactttggtgcgttggcgcgaacaatttttattattgacgccaccggtaagattatttaccgccagattgttccggaaattggtaatgagcctgattacgatgatgcactaaatgctttgaaaaaagttgctcagcgtattgacgattagcagatatttagttaagattaaaattaaattaaagtgttgagcaagagagtagccaacgtttcggtttcagaaagaaaatcattgctgtgagatttttaccgggcgttgagtgaaggtagcttgtgagctgcttatcttcaattgaagatgagtcggtattatcagaccgttattatgatattaagtggggcttttcagcccaatttaggtggtaccgcgaacacttcgtcctaatttacaggatggggtgtttttttattacataaaaacgatttgaattttggaaggagtgacgttatgtcagacaaattgcacgaaatgtcaacgaagtatgatccaactgccgtcgaaaagggcagatatgatgaatggcttgatgaaggggtatttacaccgagtggggataaaaaggccaaaccattttcaattgtgttgccgccgccaaatgttaccggaaagctgcatttgggccatgcctgggatacaacccttcaagacatgattatccgccgcaaacgaatgcagggatacgatactttatggctcccaggaatggatcatgccgggatcgctacccaagctaaagttgaagccaagctgcgtaaacagggtatttcccggtatgatttgggccgagaaaagtttgttgaaaaggtttgggaatggaaagatgattttgcccgaaccatcaaggaacagtgggccaaattaggtctttctctggactacagtcgtgagcgattcaccttggataaaggattgtccaaagctgttcgtaaggtctttgttacgctttacaataaaggcctgatctaccgcggtgaatacattatcaactgggatccgcaagcaagaactgccttgtcagacattgaagtgatccataaggacgataaaggtgccttttaccatgttaaatacccatttaccgacgggacgactttcaacggcaaagattacatcgaaattgcgaccacccgtcccgaaacgatgatgggtgataccgcggttgccgttaatccttctgatgaacgttacaaagatatcgttggcaagaaagtccgcgttccattgattaatcgtgaagtgccgattatagccgatcagtacgttgaccctgactttgggacagggatggtaaagatcaccccagcccatgatccaaatgactttaaggttggtaatcgtcacaacttacaacgcattaatacgatgaacgaagatgcttcaatgaacgaaaatgccggtaagtataaaggcatggatcgttttgaagccagaaaagctatggtcaaggatttgcaggatgaaggcttgatgctctcaatcgacccaattgtccattcagttggccattctgaacggactggggttcaagttgaagcccgtttgtcaactcagtggttcgttaagatgaaaccgctggctgaacaggccattaagaaccaggataccaataacaaggtcaactttttccccgaccgttttgaaggaacctttgaacagtggatggaaaacgttcacgactgggttatttcccgtcaactttggtggggtcatcaaattcctgcttggtacaacaagcagaccggtgagatctacgttgggatggaagcgcctaaagacgccgaaaactgggagcaggatccagatgttttggatacctggttctcgtctgccctgtggccattttcaaccatgggctggcccgatgatacagaagacatgaagcgctatttcccaaccgacaccttggtgaccgggtacgatatcatcttcttctgggtttccagaatgattttccaaagcttggaattcactcatgaacgaccctttaaagatgtattacttcatggtttaatccgtgattctcagggacgcaagatgtccaaatcccttggaaacggtattgatccgatggatgtcattgataaatatggtgccgatgcccttcgctggttcctgtcaatcggtgggacgcctggccaagatttgaagttcagttatgacaaaatggactctgcttggaatttcattaacaagatttggaatgccagtcgttacgttattatgaaccttgatgggattgacaagccggaattacccgacaagtccgagtggcaattatctgacaaatggattttaagtcgactgaacgctactgtgaaccacgtttcagacttattcgagaagtacaactttggtgaagccgaccgttatttgtatgacttcatctggaatgatttctgtgactggtacatcgaaatgagtaaggaagctctcaacagtgacgatgagaagttgaagaagaacacccaaaacattttggcttacgttttggatcaaacccttcgcttactgcagccgatcatgccattcgtcaccgaatatatttggcagatgatgccacacgttggcaagtcactggtaaccgccgactacccagtggaccacaaagaatttgacgacccaacttctgagcatcaaatgcagtcattgattgatttgattacggcagtgcggaatattcgaaatgaagccaacgcaccgctgtcatcaccaattgatatgttaattcaaactgacaatcagaccctcaaatcaatctttgaatccaaccgcgactacattgaccggttctgccacactcaggaattgcaaattggcaaagatattgaagcgcctaagctgtcaatgtctgcggtgattacggatgcgactgtctttgttccattggccgaattggttgacttgaaggatgagcaggctcgggttcaaaaagatgtggataaatttgaagccgaagtggcccgttcagataagaaactggctaacaaacggtttgtggagaacgcgccggatgcagtggttgctgaagagaaggccaagcaggctgattaccaatcaaaattggatgcagccaaagaccggctccaacaaatttccagcgagatgtaaagtgatttaactgacttaaatttttaaaaacgtgggactaaatgctgtttcctggcacatgccaggctataagccgcatttttgcccacgttttttaaggagaaaataatgattaacacatatgatgaagccttggctttcattcatggacggaccaaattcaagaaaattccaaccttaaaacggatgcggcgattcttagacgaattgggtgccccggacaaacatgtcaatgcgatccacattgccggcactaatggcaagggatcgaccttggcatttttacggaacttgtttcaagcggaaggcaaaacagtcggcagctttacctcaccgtttttgattaaatttaatgagcgaatcagcgttaacggcgtcggcatttctgacgatgaaattctaagactcactcaggaaatttatccgacgattgccaaacttgacgccgagttgccggaaggcggcccaaccgaatttgaaattgtgacagctatgatgttcaagtactttgctgaaggacacgctgatattgttttgattgaagtgggtcttggtgggctgtatgattcaaccaatgtcattatccccaaagtctcggttattacgtcgattggctgggaccacatgcacattttaggggatactttgtccaaaattgctttccaaaaagcagggattattaagccgggcgttcccgtagtcgtcggcggagttgaccccgaaccgctcaaggtgatcgtgaaccaagctgagcacaagcaaagcccgattcagattctgggacagaattttaaggtcaatgatcgcggtgagcacaattggaatcaagaatttgactttagttccgctgactttcaattgcatgatttaaaaacagccttaattggtgattatcagactcacaacgctgcgttggcgatccaggcatacattgactaccaccagctcacaaagcgcgctgtggatgtcagaaacattcaaaagggaattgcagcaacacggtgggcgggccggtttgaaaaaatttccaccaagccgaccatcgttttggatggtgcgcataatatctcggcagttaacctgattgtcgataccttgcagaacgattttccccagggccatatttatattttgatgggcattctggcagacaagcaggctgataaaatggtggacaagatggccaccgttcaaaatgcatcgatcatcttgacccggttcgccggaccaggaaaacggctcgcagctaatccagaaaaattggaaagtcaactgaaaacccaaccggaaaatgtttccgctattgatgattggcaagacgcaatcagggaattgagacggaaactgacgccggatgatatgctcttaattaccggatcgttatattttatttccgatgctcgaaagttcttgttgaatcccgatcacaatttcaaataatctattaaatcgggcgtcgtttcacttgattttatttatttttggacgcgttatgatatacttgtttcgttaaacaataataaataaatctataaaaatcgaactaaattaagttgatagacaacgaagggatggataacgtgtttggatttggggaaaaaaacataggaattgatcttggaaccgctaatacgatcgtttacgtcgagggcaaaggaattgtccttcgcgaaccttcagtggttgccaagagcactaaaacaggcgaggtaatcgccgttggtgcagaagcgcgagcaatgattgggcgcacaccagcaagtatccaagctgttcgaccaatgaaagacggtgtcattgccgattacgataccactgttgccatgatgaaatacttcattcaaaaagccttgggacactcatcaggtaagccatacgtcatggtttgtgtgccaaccggcattactgccgtggaaaaacgggctgtcattgatgccacccgggtcgccggagccagagatgcctatgtcatcgaagaaccattcgctgcggcaatcggtgccggacttccagttatggatccaaccggtagcatggttgctgatattggtggtggaacgactgacgttgcaaccatttctttgggcggcattgtttcaagccgttcagttcgaatggctggcgacaagcttaacgaagcgattgctcaatatgttcgccaaaagtacaatttgttaattggtgaacggacttccgaacagcttaaaattgatatcggttccgcttctgccaaggaagctaaagaaatcaaagccgttccggttcgtggccgtgatttggtaaccggtttgccaaccacagttgaaattagtggaacggacgtcaacaaagcaattaacgaatcagtgttggccatcattgccacgattaaggaaacccttgaagaaacatcgcctgaaattgcagccgatgttattgatcatggaattgttctgacaggcggcggcgcattactcagaaatattactgatgtgattgcggaagccactcaagttccggtttccattgcatcggatccacttgattgtgttgccatcggtactggagaatcattaaagagcattaatgtaatgaagaaaaaacaataattaatcgtttatatcgattcattattgaataacgaatggaggcaattatgcaaaaatttttctccagtcgaaagcttgtgattgtcgtaatctgtttgatcgtcagttttggtttaatgtcgttatcggttgccattcgggacaagcggagcacaccaccgttggtacaacaatttggaaatgatattgttggttttgctgatcagattgttgccgccccaatgaacggtattcatcacggatttgtttcaactaagaatcttttgaacacttatcaggaaaaccaacgtctcaagtcaaaagttgatcaattgacccaaacacaggtcaaggatcaggttttgtcgcgagaaaataaacaattgaaacgtcaattaaacgtcggcagcactttgaccggatatgaaaaaatcaacgcagctgtcattacccgaacaccatcatcatgggcaagtcaggtgatcattaataagggtcaagcttctggtattaagaaggatatgcccgtgattgccggtcctggtctgatcgggacagttgctgaagtcaacaaaaccaacagcaaggtggttttaatttccaacaccgccgagaactctaaccggtttgccatccaagtgcttggcgataattccaaagttgttaatggtattatcacctcgtatgattcggctgccaaccggattatcatggggaatattacctcgaacgccaaattatcagttggtaatcgggtgacaaccagcgggctcgggggcgtcattcccaagggaatttacgttggaactgtttcaaaagtgacccaagacgattatggccttgccaaaaaagtttatattaaaccggctgccaacttaaacgacattgaagttgtttcagttgcaatcagagattgatgggagggacaattaagtgaaacgaaaagttcccattgcagtttactttgtaattggtcaaatcattgcgttctttcttgatggttccatcagccagacaatgtccggtattttgtttaaatatcccaacacgatggtgccgtatttaaccgtcctctggttgattttggcagccttctttggtaatggcaaaaaattacatctatacacttggtccgctgtgattggctttatttttgatatgtactacactggattgcttggggtatatgtgtttatttttccattagtcgtttatttatgccaattggtttaccaaattttgccaccaaatttcatgagtggctttttggtgtattttttaggaatcacagttctagttagcctaggatacatggccaatgtatttattggggagacggactcatccgttgctcagttcttagttaacacattggctcctacactggctctcaatctggtgttattgacaattgtttactttccggttgaggcactctataggactcataggcaataagaaggggagtagacaatgcaagatgcagctgtattaaagggcaccaaggatggttatgaaatcattctggatgaaaatgccaatctaaaggatattttttcttcacttcgaaaacttctggacaacttgaaaacgcagacggcatcaactaatccgcaaaccattgcttttgatatttataccggaatgcggttatggccagctgccgaccgttctgagcttgagaaaatcttttcggattattcgacgttttcagtgcataagattacgtcagatgtgatcactaaagaggagtccaatcggattttggaacagtccagcgtccacattgttgatcgggtgattagaaacggccaggaagttcacatccaaggtgacgtcttatttctgggcacggttcatgagggcggcaaactgtttgtcggcggtaacatttttgttctgggtaacgtccagggaattattcaagccggcgcaccggaccttgaggacaagatgattattggggatgtacataacgcacaacaagtccggatcggcgaacagttcgaaatagttgctgacatgaagcgtgaaatgaacagcggcacggtgatttatgtgaacgacctgcatgtactggattatggtaaagttgagaatcttaagcagattaatcccaagttttacaatcagataggaggagtcatcaatgggtaaggcttacgttataacatcaggtaaaggaggagtcggtaagaccacttcttctgctaatattgggaccgcactggccatgctcggtaaaaaggtggttcttttggatcttgatatcggattgcgtaacttggatgttgtcttgggactcgacaaccggattatgtacgacattgtcgatgtcgcagctggacgagccaagctcagtcaagcactggtcaaagacaagcggtttgatgacttgctttacctattgccggcagctcaaaatactgacaagacggccctaaatgaagaccaggttcgcgaaattgttgatgaattgaagcctgactttgattttatcctgattgattgtcctgccggaattgagcagggcttcatgaacgcaattgctggtgccgatagtgccattattgtgacgactcctgaaatttctgcggtccgagatgctgaccgggtggttggtctcttggagcagcatccgcttcaagaacagccgcatctgattattaaccgaattcgtcaacatatgatgaaagacggttcggtgatggatgttgatgaaattacccatcatttaggggtcgaactattggggattgtctttgatgatgatgcagttatcaccacttccaataacggcgaacccgttgttcttcaagcggaaaatccagctggtcaggggtatcgagacattgcccgacgactagtcggtgaatctgtgccattgatggaaatcaaagatgaacagcagccttcgttctggcaaaaagtcagtcattggttccgtaaaggataaaagtccttgacgggaagcagaattaatattattataaatctaacttaattaaagatttttaaagacgttgatcagaaccgattaacgaatcaaatcacagagagcttatcaaggtgggagttaagcatttgagcgttaatcgtcacatctgggagtcatttttctgaagctgagtaggaaaaagcggtaagcacgttattgctgaagtttagtatgttgcatattaaacccattgaggcctttcatgtgagtgagaggtgaatcagaggtggaaccgcgaataatcgtcctcttaagtcatcatggcttaagaggattttttattttaaaacaagactaaacttcacgaggcagcaggtgtgaatctgttgcgaattgaggtggaaccgcgaaaaccatcgtcctcttgagtcaatgtgtactcaaggggatttttttatggagggatgtcaaatgattcaatatatacaagaaattttaccggccttattatctggaaccaaaatgactttatcaattttcttctggacattgatttgttcaattccattaggggcattagtcggattaggactcatccaaaaatttaaaccgctgacctggctgcttaacttttacgtttggattatgcggggcacaccactgctattgcaattaatttttgtgttttatggcttaccgattattcacattgtgttccaacgttacgatgctgccatgtttgctttcattttgaattacaccgcatatttcggtgaaatctttcgaggcggtttccaatcagttcccaagggccaatttgaaagtgccaaggtgctgcgattgagttatggccaaacgattcgaaagatcgtgattccccaggttttcaaaattgttctgccatcaattggtaatgaagtgattaacctggtcaaggattcctcattggtctacgttatcgggttgggcgatttactgcgagccggcaacgttgcgacggcaagagatgtcacgctgttgccgctgatattagtcgggattatctatctggcattaaccgcggtatgtacgattgtgttgaagttaattgagaaacgtgaaaatgtttggcgttaggaggggattacgatgttagagattaagaatttaaccaaacgatttggcagccgaaccattattgatgacttgtcaatgaccgttaaagataatgaaattatggcaattgttggcccttccggtgccggcaaaacgaccctgttacgttgtattaccggtttggagtcggtgaataccggggaattttactggaatggcactcaatttgacccaaccaacacgactcaaaaagacacgatcatcggggtggttttccaagattatcagttattcccaaacttaacggtcctgggaaacattactttggcaccaacgatggtcaaaaaagaaccgatggcagacgtcaaaaaatatgcacgggaattattgagtcgcttgggcttggaaggcaaagaaaatttatatccttatcagctttccggcggccaaaagcaacgggtggcaatcgttcgtgcactggcaatgcgaccgaagatcctttgttacgatgagccgacgtcggcccttgatcccgctttacgagatgaagttgcccaaattatcttggatcttaagaagcaggaaatgacccaaatcgtcgtcactcatgatatggattttgctaaaaacgttgcggatgaaattcagcaggtcaaacaaattcagtaggaggggtaaaatgttaaaatctttgaaacgattattactcattaccagtctcctactcgtgaccattgggttatccggttgcggggtacgctatgtcagtcgccaaggctctcaggaaaatccggatacgtggtcgacggtttccaagcaaaaaagaatcgtggttggcctggatgacagttttgtcccaatgggctttcagaccaagagcggcaagattgtcggctatgatgtcgatctggcccgtgccgtgtttaaacagtacggcatcaaagtggactttcagccaattgattggtcgatgaacgtcaccgagcttcgaaacggcacgattgatcttatctggaatgggttctctattaatccccagcgagcaaagaagattactttcagtgaaccctatctaattaatgatcaggtattggtttccaaaaagaatcaacatatcaacagtttcgcagatatgaagggaaaagtcgccggcgtccagagtgggtcggcaggggccatggatattgataaccaacctaaattgctgaaagataagatcaagggccacgagccaatcttatacgacacctttacagacgcgttcatcgatttgaatgccaaccgaattcagggattgctgatcgacagcatttatgccggttattatttggaacaccaaccaaatcaatccagttttaagtcgattcccagtgaatttcctaaagaagaatatggtgtcggcatgcgaaaaggtgatacggtcttgaagcggaaaattgatcaaggtctcaatcgattagccaaaaacggcgagcttcacaaaatcaacatgaagtggtttggaactgatcgtgacagtccgctcattaagaatactaaataagttcgatcattagtagtctgtggcaaatgtgatttgtcaacagactatttttgtattcagatccactgccgatcaattctctatttttccttattattggcagattatattgagattttaatgattttattttatgataaaatttgtgactaattgaggaggaaactcagtgaaatacgagattgcaaaagggattagcttgacgacaattcccaccacaaaattcaaaaataataaattggtgatgaatttcacctttccagcccaacatcaaaactacgccaaattggcactgttggctgaactgctggaaaattgctcggcccaatacaacagtgagttgttggtttcccgccaactgtcaaaaatgtacggggacagttttggtgtgactgtcttacggtatggcaatcagcataccctacaggtgtcgattacgtttccaaatgacaagtacctaccgccaaaaagtgagctaactactgaaatattggcatttctaaaggaaatgattgaggatccctttattgaaggcgatcagttcaatcaagcatactttcaaattcatcaagggaatatgattcattatctggattcgatccaagacaacaaggagttcttctcaaccctggagcttcaacgtttgtattaccaaaatgatcctgaccatggtcacttcctgatgggcagtcatcaagaaatgagccaaatttctgctcaagagctgtacacattttatcgatgggtccttaacacagcgaagattaccatcctggctggtggcgatttaattgacgaccaactagtagcgggatttaaagaatttgcctcatttactgatcgaatgccggaagactaccaattaagagttgtgccggcaccaatatcgaaggtccaacaaggaaccaaagtgattgccggttctcagtcagttctcagcatggcttacgaactaccaatctattttggggacgatgattactttgctgccgtcatttttaatcagttatttggtgggtcaagcagatcgttgctatttacaaacgttcgtgaaaagaacagtttggcctacgacattcatagtggctataattcattagtcggaatggtaaccgttcaggcgggaattgattttaaagatgaaaatcgcgttattcagatggtcgccgatcaattgcagcagaccagcgacgggcagtattccgatgaattgctcgacggtgtcaagcaggcattgattaaccaacatcgttcagaagccgatcacctcggatcattaatcgagaagcaatatctccagcagatgatgggctttagtttgagtgataccaaatgggagcaacaggtcgcttctgtgacgccttcgcagattgcccaagttgccaagcggttgactttacgagccatttatcagttgaacagcaggggggatgcataatggaattgattgactatccaaactacaatgaaaaactatttgttcagaccctctcaaatgggttgaccgtttatctccaacccaaagcagggtttaataagacgaccgcggttttgggggtgaattatggctccattgacagtcagttaatgctcaatggcgaaaaagtcgttcaacctgcaggaattgcccattttttggagcataagatgttcgataaaaaggattacgacgtttttgagctgtttaataaaaccggagcgcgttcgaatgccttcacaagttttaccaagacgaattacctcttctcaactgccgaatccgtgaaagaaaatttggatattttgttggattttgtccagattccatattttacccaagccaaagttcaacgggaaaagggaattattgatcaagaaattaatatgtatcaaaatgatccggacaatcaggcatactttaaaacgattgccagtttgtatccaaactcagtgttggcaaacgacattgccggcgacattcagacggttgataagattaccctggaagatgttgagttggcctatcgaaccttttaccggccggaaaatatgagcctgtttatcaccggcaaactcgatcctagcgaagttatgagctggattgaggataatcaacggcgaaaatcgacaccggcacccattagcctgcaacgccgactgacgctccccgaggcatccaaagaaaccgttctccacacgaaaatggatgtttcccgccctaaaataacgctggggctacggggaagtgatcaggtgccgacgggccgggatggcttaaagtacgaaatcgccatctctgtgatgtttgacctgtttttgagtgaaaactccgtggaatatgataaactgtatcatgatgaaatcattgatgacacgttttcatgggaatttgaaaatgagcgtggctttcattttgccgtgattaacggcgatacggataaaccattggaactcattgaacggctcaaacaaatcattgcggatattccaaccaaaattggtcacctccaaaccgaatttcagttgcaaaaaaacgagttatttggcaactacgttgaaatgatggattctgaagaagcaatcagtggccagtttgacggatttatcggtgaacctgttacaatatatgatgaggttgagattctcaaatcattaaccttggaggatgtttttgaggcggcccacagttttttggaccaagcagcagttcaagaagtgatgattcaaaattttgaccagccaaagggatagttgataaattatagtttatgaattacttaaaataatcaaggttttccttatgatatacttagtggagaatacaaaaaattcaatggagaatgagtatgagcgacgaaaaagataatttaacaattgggaaaaaactacatgacgcacgagtggctaaaggttacacgctggatgatttacaaaagaacactaagattcagaaacgctatctaattgcgatcgaagataatgactttgacgccttaccgggtgatttttatgttcgagcatttgttaagcagtatgccgattcagttggtctggacggaagtgagctgctaagccagtttgatactaaattgcccgataccgaagacccggaatatgttgatcgggtcaatgatgacaaccctgagacgagatctgctcaacgaaaggttgaagaacgcaatgataaactgcggcgctatattccaattatttcggtgtccgtcgtcgttttaatcatcttgattgccatttgggtggctgcggccagaagtacccgaaacactgccaaaacgcaaattgagaccagtaaagtttccgtttctggtgataaatcttccagttctaaggcttccagttcaaagaaggccaagacgactaagaaggccaaggggattacctttaagaaggttactgcttctggcagcaatctgacctaccgagtcaccggaacttccggtacaacgccactgaagatttcagtaaccggttccgggagtgcctggacgtcggtttctgcagatggaacttctttatggcaggcttcattaaccagtggtaattcacatacaatctctcttccaagctcgaccaatactgtcacgattaatactggcaacgctgaagcgactcggattaccgttggtggcaagaagttgacgttggcggcaccgttaaatggcggttcaactcaggtgagagttgtcacattgcagtttggcaagtcaagttcatctgcttcaaccagttctagttcaagtagtgcaacgacgggtgcttcaactaccagtagcacaaccgggacgactggcaccactggaacgtcctcaacgactggtactgacacaaccggcaacacgaatgcaacaactggcagcactggtacgaataataataccggtaccaccaatggctattagtcagctggaggtttaacatgaatttaccgaataaattaacactgtttcgaatcatcctgattccgttctttatcctgatcctcgcggtcccaatcctttccggcagcgttgtttgggcgggcactacgatcagtatgaccagattgtgggcgacaattatctttgtggttgcctccttaaccgatttcttagatggtcagattgccagacgaaatcatttggtaaccaactttggaaagttcgctgatcccttggcagataaaatgctggtaatgacggcatttctgtttttggttggcttgggggatgttccggcatgggtcgctgcgattattgtctgccgtgaattggcggtaactgggctgcggctaatcattgtcgagaacgaaggccaagtcattgctgcggcctggccgggtaagatcaagacaaccactcaaatgctggcgatcattttactgttcttgaacaacgttttatttgatgcattcaacattccaatgggcttaattctgttatacatttgcctattcttcacgatttactcaggaattgattactttgtaaaaaatcgctcagtattttcagattcattttaatcacagctgccggagggttcatgaaaatgagtcttccggtatttgtgtcttgttagataaaaaccaagtatttaacgtacttatgaactagagggagcaactaagatgacattggaagagacattagtaaatgaactattatcccgacacattacaattacagcggctgaaagtttaactgccggtgaatttcagagcactctcggtaatgtgcccggcgtctcagaagtttttgaggggggatttgtcacatactcaaatcaggttaaagaacaactactgcagataccaagtgaagtaattgatgaaaatggtgtcgtgagtgaaccgactgccatttggatggcaaatcaggcccgaagcatcatgaataaagatctgggcgtatcctttaccggagtggccgggccggacacattggaaggcgatcctgctggcacggtctggattggcattgcctatgggacccaacatacttacgcgaaacagtttcatttcacgggggatcgaaatcagattcgggctgctgcagtcaaggccggcttggagatggcgttggacatgattcatcgttattaaattaatcgaacttttgttcgcgttttgattgcttttttggataatcattagtatagttagtaagtaaacttttccgttaaggatagtgggaggaatttaatggctgaccaaagaaaagtagctttagataaagccttaaagaatattgaaaaagaatttggtaagggatccatcatgagaatgggcgacaaagccgatactcaaatttccacaattccatctggttcattagcgcttgatgatgcactgggagttgggggatacccacggggcagaatcgttgaaatctatggacctgaaagttcaggtaagaccaccgtggcgcttcatgcggttgccgaagttcaaaagcgcggcggcacggctgcctacattgatgccgaaaacgccctggatccggtttatgcaacccacctgggtgtgaatattgacgatctgttactttcacaaccagatactggtgaacagggtcttcagattactgacgcattggttaccagtggggcaattgatatcgtcgtcattgattcagttgctgcattggttccccgagctgaaattgaaggagaaatgggggatgctcacgttggtctgcaggctcgactgatgtcgcaagctctccggaaactttctggaacgatcagtaagaccaagacgattgccattttcattaatcagattcgtgaaaaagttggtgtgatgtttggtaatccggagactacccccggtggtcgtgccttgaagttttatgcgacaattcgactcgaaattcgtcgggctgagcagattaaggacggtaccaacatcattggtaaccgtgtccgcatcaaagtcgttaagaataaggttgcgccgccatttaagcgtgctgaagttgatatcatgtatggcaagggtatttctcaatctggcgaattggttgatatggctgttgaaaaagacattatcaacaagtccggttcatggtattcatatggtgaagaaagaattggtcaaggccgtgagaatgccaagacttatctcgaagaacatcaagatatgtatgacgaggtgatgaagaaagtcagagctgcctacgacattcctgatgaaactgactcggacacctctgatgctaaaaccagttccgataagaaaaccgataaaaaagccgacaaaaaggattccaaaaaagaatcggcagccggttcttcaaaagaaaccaaagttgatagcatcgatcttgacattggtaagtaattggtactaccaaatgcaaatagatttcgttaatgggcactcagaggagttgcccattttttgtgacttaatcaaggcacagcaggcttttgtgaaacattttaaaagaaaatatggtcactcaaaaatcttgttatatacaaataccaaaaaccgcaacgtaaagatgattgacactagtgttaacaaacattaaaataagaattgtgtcaataatcaaataacatctaattggtttacaaataatcattttttgatgatttggaggtgaaaagccatgaccatggctgggataatcctcgcaatcatcgctataattgttgttggttttgttggtattttaagctttgtaatcggcaagtctgcacaaaagaagatccacgagaaagatcttgactctgccaatgggtcggctaagaacattttgatcgaggcccagaagaaggctgagacggttgtgaaagaagcaactctatcagctcaggagaagaaccaccgttaccgttcatcggttgaaaaagaactgaagactcggcgtgcggagattcaaaaacaagaggatcgtttgctgcagcgagaagaggctcttgatcgtaaagacacggctttcgaacgtcgtgaaagttcgttgaaccgaaaagagcagaagattaatcgtgaacaacagaatttagttacacaacaagaagaagcaaactcacttatcgcaaaacgccaggccgaagttgagaaagttgctgctttaacgcaagaagaagcccgggacctgattttgaaagaaactagcgaaaagttggctgacgaaaaggctcggatggtaaaagaaagttattaccaagcccaaacagaagctgatgaaaatgccaaaaatctgataattgaagctattcaacagagttcagcggacgttgtctcagagacaaccgtttccgttgttagtcttcctaacgaagacatgaagggacgaattattggccgtgagggccgtaacattcggactttcgaaacgttgaccggcattgatttaatcattgacgataccccacaagcagttgtgctgagcggctttgatccgattcggagagaaattgccaaaatgacacttgaaaagttaatcaaggacggtcggattcatccggcacgaattgaagaaatggtcgaaaagagccgtaaagagcttgacgaacgtatccaagaaattggggaagagacgctattcgaccttgggattcattcaatgagcccagatatgatcaaattagttggacaactcaactttaagattgatcatgggcagaacttgctgagtcattcaattgaggtcgccaagttggcgggtgcttttgcagcagaattaggtgaggatgttactttagctaaacgcgcaggattattacacgatatcggtaaagctgccaataatggtgttgagggatcacatgtacaggttggtgttgatttcgccaagaagtatcatgagagtcccgttgtcattgatgctatcaaaggttatgaagaaggccacaatccagaaacaatcatttctgagttggttgctgttgcggaaaagatcgcgatttcgcgtccaggcgcacacagtgaatcacttgaaagctttgttcatcgacttgatagtcttgagaagatcactgacagctttaacgaagtacaaaagagttacgcaattcaagcaggtcgagagatccgtgtgattgcaaagcccgaagatataacggacacacaggcaattgtgcttgcccgtcagatcaaacaaaagattgaaactgagatgaagtatcctggacacattaaagtaacggtgatcagggaagttcgttcagtcgaatacgcaagataaaagatcagagtctctggtcttttttcttttataaatgttagaattattttatattattcagaaagtatcgaggaaaaatacatgcgaattctttttatcggtgacgtggttggcgacaagggtgtttcaatgattggcaattatctgccaagactcaagcaggatctgaaaccccaggtcacaatagtgaacggcgaaaatgcaacttcaatgggtcgcggcatcactttgagtatctataagcaattgatgagtgatggtgtggatgtggtcacgcttggaaaccatgcttggagcaataatgaaattctcgacttcatcgatgatactaaacggctgattcggccgtacaattttcccaagcgaacaacacccggaaaagggtataccatggtcaatgtcaacggcaaacagttggctgtcctgaattttcaagggcgcgtcttcatggacaaccttgacgatccattcgagctggctgacgaactggttgaagagattcgaaagacgaccaattgcatttttatggattttcatgccgaagccaccagcgaaaaattagcaatcgcccgttatttggacggccgaatttcagcggtggtggggacacatacccatgttcaaacaaatgacgcacggattctccaaggcaagacggcctttttaaccgatgccgggatgaccgggccggctgacggcatgttgggcatgcagccggacagtgtgattcaacgcttcttagatcagcgaccagcccgatttaaagttatggaaaccggtcggggaatcatttccggctgcttcgtcgatattgacgataagaccggtcacgcgacccacattgaaaccgtgtcgatgactgatgatcaaatttaattgtgttttataatagtttagacgatactgaaatcgaattcagtgagaatttaaggggactttcagttggcaaaaaaagaattaactccaatgatggtgcaatatcaaaaaatcaaggaccagtatccggatgcttttttgttctaccgtctcggtgatttctacgagatgttcaatgaggatgccatcaagggttcacagttattggaattaactttgacgaaccggagccggaatgcggccaatccggttccaatgtgtggtgtgccccacaaagcggtgcaaaattatattgatattctagtcgaccagggatacaaagtcgcaatctgtgaacaaatggaagatccacgattggctaagggaatggtcaaacgagaagtcattcaattggtgacaccgggtacgcaggtggatgttggcagtgaaaacgccaagtccaataactatctgactgcggtggtggatgatcaaaaaaaccatgagtttgccttctcatacgccgatctttccactggtgaactcaaagttgccaaattaaccacacaggctgaatttgttaacgaactggtttctttacagactaaggaaattgtcgttgatactgatttaccggagtcaattcaagatacgattcaaaagttggggattttgatttcccatcaatcggttctgccggtcaatgcctcagtcagttacttaagccaggacgttgatgacgacttgatgaaacgggttgtcaaactcctgttggattatatccaggcaacccaaaaaagaagcctgcagcatttaaagcgggcagtgatttatgaaccctcagattttttggaactcgaccacaattctcaatacaatttggaattaatccgcaatattcgcacaggtaaaaaagccggcactttattgtggctgcttgaccaaaccaaaactgcgatgggcggccgaaaactcaaacaatggattgagcggcctttggtgaaccgcaaactgattaatcaacgccatgatgcagttgccgtgttactggatcactatttcgaacgaaatcaactccaagacgagttaatcaaggtttacgatctggaacgattggcaggtcggatttccttcggcagtgtcaatggccgtgatttgattcaactcaaggcttcgctcaagcaggtcccgaagattaaatatattttggagcaaatcgccgacaagagttttgaggatatgctcaaaaatctggttccattggatgatgtcgtcgacgaaattgattctgcgatcgtcgaggaaccgccaatttcagttactgatggtggggtgattaaggatggctacaatcaacagctggacacttaccgggacgctaccaataacggtcaaaaatggttggctgaactggaagcgaaagaacgtaaaattaccggcattaataacttgaaagttggttttaatcacgtttttggttactatattgaagtcaccaaggtcaacttaaacaagattcctgcaaaccgttatcagcgcaaacaaaccctggccaacgccgagcgattctcgacgccggagctgaaggaaaaagaagcgttgattttagaggcccaggaacaaagtaaaactttggaatacaagctattcgttaagatccgtgatgacattaaaaaatccatcaaacgaattcaggatttagcagatgccgtagcgtcaatcgatgtcttacagagctttgccgccgtcagcgaggagtaccgatttgttcgaccaacgcttacgacgcagcatgtggttgaagtcaaagacggtcgccacccagttgtcgaaaaggttttgggccaccagcaatacgtcccaaatgacgttaatctgggcgaagataccagcatcttactgattaccggtcccaacatgtctggtaaaagtacctatatgcgtcaaatggcactatgcgtcatcatgaaccaaatggggtgttttgtgcctgccaaacatgccaaactgccggtgtttgacaaaattttcactagaattggggccgctgatgatttaatctcgggccaaagtacgttcatggtcgaaatgaaagaagccaacgatgccattgagaatgccactcccaacagtttgattttgtttgatgaaattggtcgggggactgcaacctacgatgggatggcgttggcccaagcaattatcgaatatgttcataacaacattggtgctaaaaccctgttttcaacccattaccatgaattaactgttttggatgagtctctcaaacgcctgcaaaatgtccatgtcggcgcgactgaatccaatggcgaactggtctttttgcataagattcagccgggccctgccgataaatcatacggaatccatgtggctaaattggcaggtctgccagaagggttattacaccgtgctaacgacattttaaccaaccttgagcaacaggccgataaagagcatcaaacggcctccgcaccaaagcaggcgcctcagcaggcagctgagcagcagacgtctttatttccccttgagcaaattgatgataaacaagccgaagttgtgtcacaattaaagaaattggacttgatggggaagactcccatgcaagtgatgaatcaagtttacaaatggcagcagaagataaacggagactaaggtgattgatttgaatgaaattcataagctaccaacaatcctttccaaccagattgccgccggtgaagttgttgaacgaccggcatcagtggttaaggaattagttgaaaattcaatagatgccaagagttcggaaatcgatgtcaccgttgaaaattcgggcttgaagttgatcaaagttgtcgatgacggcaacggaattgacagctctcaagttcagacggcctttttacgacatgcgaccagcaaaatttctgagcaacgggatttgttccgcgttcggacactcgggttccgtggcgaggcactccccagtatcagttccgtcgctaacgttcggatgaagacgtcaaccggttcgattggaacggaagttgaatacaaaggcggcaagcttgtcactcaaaaggcttctgaatcacggaaagggaccactgttgaagtggcatcactgttctataacacgccggctcgtttgaagtatttaagttcaccgaatacagagctttccaaaatatcagacattgtcaaccgcttggcattgagtcatcctgagattgctttttcatttatcagtaacggccgtgaattgttaagaacttccggacgtggggatttacgccaggttttgggcgcaatttatggtgtcaagacggtttcaaagatggcggcaattaagggaaatgatttggacatcaaagtcagtgggtatgtgagtttaccggaattgacccgttcaagtcgaaactatatttcactgattttaaacggacgctttattcgcaactttccgttaaccaaagcggtgattgcgggctatggttccaaattaatgattgggcggtttccaattgccgtaatcaacattgacgccgatcccgctttgatcgatgtcaatgttcatccaaccaagcaggaagttcggattagtgacgaaccgatgattggtaaattaattgccaatgccatttacgacatgctaagagacaagcagctgattccagatgcaaccagggatttcaaacagccggttcaagctgcaccaagacagtttgatgtttcgactgccactcaggctcaaacaaatccaccgctgtttgccgtcgacacaccaacgacgccttcaatttcccaacctgaagtaacgccggtggtggtcaaaaccagagacgaccttgccagctcacaagttgctcaatttgatgactttcttaaaaatgagccgagtggcttgcctgcatttgaaggaacccagccaaaaacgattgacaatcaccagccgagtgccaagcctgagcagtctgaactggtagtggaaaccggttttccgcatctggactacattggtcaaattcatggcacctatctggtggctgaaacagccgataatatgtatctggtggatcaacacgcagctcaagaacggattaactatgagttttaccgtaagcaaattggcgaagtttctgatgaccaacagaaattattggtgccaattgtgctcgattactcaacctcggatttcttgatgattagcgaccgtttggacctgctggacaaacttggaattcatttggagccgtttggacagaacagtttcatcgtccgtgagcacccaatgtggtttaaggccgggcaggaagaagacaccattaaagaaatgattgactggattttatccgatcataaaatttccgtggccgccttccgcgaaaaaacggccatcatgatgagctgtaagcgggccattaaggcgaaccatcatcttgatgagctccaggcaaaggcgttactgaaacggctgcctgagtgcgagaatccatataactgcccccatggccggccggttctggtgaaatttaccaatgaggatattgaaaaaatgttcaaacggattcaagacccccatcatacagaccaagaaatcatctagattgttgcccagtaccgagtgagatatggtacaatttattggcaaacatacgttttagtgaagaggagaagttgatgtttgaatttttggaagggacggttgttgatatcacacccacccacatcgttttattagtgggcggcgttggttatttgatcaataccgcagacccgtaccgttttaatgttgatgagaaaaaagtcatcagagtctatatttatcagtcagtgagcgatacggctatcttgctgtttggctttgcgaccattgaagacaagcagatctttgaaaagttgatttcggtttccgggattggccccaaaagcgctttggcaattttggccggcaacgaccgggatggattgatcaccgcaattaataatgaagacgtcaagtttttgacgaagttccccggagttggtaagaaaactgcccgccagattattttggatatgcaggggaagctcgacgacattgcaactaatggtgtttcgctggcccaaccgcttggcagtaacgaaaagtctcctgaattggccgatgcgttatcggcattggaggcgctgggttatggtgccaaacagattgccgccatcgagccggatttagttaagcaagctgatttgtcaaccgatgaatacttaagtttaggattgaaactgttaatgcattagggatgaggagatgatccattggccaatgaaaaagatgatcgattggtttcaccagagaatgtggatgccgatgagaacagcattgaaaaatcgcttcgtccccgagttttaagtgagtacattgggcaggatgacgttaaaaacgagttaagagtctatatcaaggctgctaagcaacgtgaggagtcactagaccacgtgctgctttatgggcctcctggacttggaaaaacaacgttggcgatggtgattgccaatgaaatgggcgttaatattagaacgaccagcggtcctgccattgataagcctggggatctattgtctttactcaatgaacttcagcctggtgatgtcttgttcatcgacgaaattcatcgactgcccaaggtggttgaagaaatgctttattcagccatggaggacttttttgtcgatattatcgttgggcagggttcaggcgcccacccaattcatttcccactgccgccattcactctgattggtgccacgacccaagcaggaatgctgtcggcaccactgcgtgatcggtttggaattgtagagcacatgaattattacaatgcgacggatttggaggatattgttcgccgaactgcggatatttttcaaattgatattgaggactccggtgcccatgagattgctttgcggtcccgaggaacacctcgagtcgccaatcgcttgttaaaacgggttcgagattttgctcaggtatctgacaaagaccaagttgatttgtcaattgtcagatacgcgttggcaaagttaaaagtcgacgacttagggttggatgcaaccgacctgaaactgttgacgacaatgatcaagtattatgacggtggaccagttggcttaaacaccctggccgccaatattggcgaagaaaccgacacgattgccgagatgtatgagccttatctgctccagatcggtttaatcaaacggacagccagaggaagaattgtgactcccaagggatacgctcatttgagttatccaatgccacctcaggacgaaaggaattagaatcttgaaaacaaattatacccttgaagactttgattatgatctgccacatgaattgattgcccaaacgccgattaaagatcgcgatgaatcacgactgctggtgttggataaagaaagcggtgagatgcaggaccgtcatttttacaacatcattgattatttgaatcccggggatgccctggtgatgaatgactcaaaggtcatgcccgctcgaatatacggtgtcaaagccgataccggcggccacatggaagtgttgctgcttcataatattgagggcgaccgttgggagactttgatgaagccagccaaaaaagccaaggtcggcacggttatcaattttggtgatggccagcttaaagccgttgtaaccaaggaattggatcacgggggccgggaaatcgaatttcaatacgatggcatttttatcgaaattctggagcggctcggtgagacacccttaccgccgtacatcaaagaaaaattagatgatcctgatcgttatcaaacggtttacgccaaagaaatgggctcggctgccgctcccacggctggtttacactggaccaaagatctacttaaaaaagtcgaagataagggcgttcatttggtttatctgacgcttcatgtcggcttggggacatttcgcccagttgatgaggaaaatattgaagatcacaaaatgcacagcgaattttaccgtttatcagaccaggcagcggccacgttgaatgctgtccgggataatagcggaaaaattgtggcaaccggaactacgtcaattcgaacgctggaaacggtcgggaccaagtttgatggccaaattcgccccgactccggctggacggatatttttatcaaacctggataccagtggcgggtggtcaattcatttatcaccaatttccatttgcctaaatcaactttggtgatgctggtggcatcgtttaccgggcgagaaaatatcctgaacgcttatcagcatgcaattgacgagaagtatcgcttctttagttttggcgatgcaatgtacattcactaggaggattattatatgcaaccagcgataagttatcgcttgattaaaaaggagaagcacaccggcgctcgtctgggagaaatcaccacgcctcacggaaccttcaaaacgccgatgtttatgccggtcgggacccaggcaactgtgaaaactctggctccggaagaattggagcaaatggggtcgacaattattttggcgaacacctatcatttatggctgagacccggagaagacatcgtcaaagaggccggcggtctgcacaaattcatgaattggcacaagggaattttgacagattccggtggttttcaagtcttttcactggctaagaatcgtgatattactgaagaaggcgtgaccttcaaaaatgaaattaacggttcaaaaatgtttttgtctcccgaaaaggcgattcagattgaaaatgatttgggtcctgatatcatgatgagccttgatgaatgtccaccattttttgagtcttatgattacgtcaaaaagtcagttgagcggaccagccgctgggcggaacgtggactgaaagctcaccaaaatcctgactggcaggggttgtttgggattgtccaaggcgccggctttgaagatcttcgcaaacaatctgcccgcgatttggtcagcctggattttccggggtattcgattggcggattgtcagtaggagaatccaaacaggaaatgaatcgcatcctggaatccaccagtccacttttacctgagaataagccacgttatctgatgggagttggagcaaccgattcactgattgacggtgtgattcggggcattgacatgttcgattgtgttctgccgactcgaattgcccgtaacggaacggtgatgacgtcacatggccgactggttgttaagaatgccaagtatgcccgtgacttcacaccgttggatgatcattgtgactgttacacctgccgcaactacacccgggcatacattcgtcatctgatgaagaccgacgaatcttttgggatgcggttgtgcagttaccacaatctttattatttgatccatttaatgaaacgggttcaacaggcaattatggacgataatctgttggacttgcgggcagaagtttttgaacagtatggttataacaaaccaaatccaaaaaacttttaggtgtagactattcagggcttatttggtaaagtattactatggaaagtgtgggtgaaaaattttgaatcaatcttattactcaattttaatgattgttgtcttgtttgcggtgatgtacttcttaatgatccgtcctcaaagaaagcaacaacaaaagcgtcgggatcaactttcaaagatcaaggaaggcgaccaagtgattacgattggccggctccatggtgtcgttgacgaaatcaacgaagccgaaaaaaccgtgactttggattgtgatggtatctatttggtatttgatctgagcgcaattgcttcggttaagcagcctgctgttgctgcgcctgcagcaaacaacgatacaactactactgcaaatgatgatcacaaagatgatgctgcttcatcaaagggcgatcaggatgctaccgaagattctgataccaaagatgaaacaaagtcggaagacaaatagtttgacgaagtcggttgggaagttgatttttatgaatcccgaccatttttttacccggcaaagaacatacgtttgattggggtgatctcagtgaaaacatcggctagaaacatcatccatgtggatatggatgccttttatgcgtcgattgaggaacgcaaagaccccactctcaagtctcaacccctgattgttgccaaggatccgcgcaaaaccggcggcaggggagtggttgcaacggctaactataaggcccgtcaattcggggtgcattccgcaatgagtgccatgaaggcgctggaactttgtccccaggcggtttttcggttctctggatttgatctttaccgctcagtttccaatcaaatccacgagatttttcatgagtacacggaagtgattgagtacgttgccttggatgaggcttatttggatgtcactcataataaaaaacatctcacagacccgattcaagttgcccgaatgatccaaaatgaaatttgggatgccacccacttaacctgttccgtgggagtatcttacaataagtttctcgccaaagaagcctctgattacgccaaaccagtgggcattacagtgattggacagcgagatgcattagaatttttaagccgtttgccaattgaaaagttccgcggcgtcgggaaaaagaccgttcccaagatgcatgaattaaatatcaataacggtcaggatctgattcagtggtcgcagatggatttgatcaagcactttggtaaatttggttacgttctctatcagcgcgctcgaggcattgacgatcggacagttgagtatcagcgggttcgaaaatcgattggcaaggagcggacatttggcccggcgattgacacacaaaccgaagtcgatgacgaactccagcgaattgctgcgatggtggtcaaggcaatggatgacaaaaagaagcacggtaaaacattggttcttaagatccggtatgccgacttttcaacgtttaccaagcgggtcacgatggataactatcttaaaaatagccccgaagaatactttacccttgccaacgatttactggtcgatatgccggatatttcaaaaggggtgcgcctgttgggaatcaccattaccaacctggatgatttaacttacgagaacattgttcttcacctgtttgattaattcaccaccccaacggtttatcttattcacaaagtaatgtatacttaagtgttcgacaataaagttatggagcaaataaaatgtcaattcaagatcaaatattaagtgaaatcaaaaaatttaaaaccattattattcatcgtcacaaacggccggatccagatgcgatcggatcacagatgggactggctcaactaattaaggggtcatttcctgataagacagtcctgtgtgctggtaaacaatatgatagttttgcctggttgggaaccaccgatgaaattgccgacgagcaatataaagatgctttggtgatcgttgttgatactgccaatcagccgcgtgtcgatgacgaacgttatacgacgggaaaagaattgattaagattgatcatcacccaaacgacgatcagtttggtcacattatgtgggttgagccggattcatcaagtacatctgagctgatttatgatttttatgatgccaatcgtgatcaattaactttgcccgatgaagttgcccgactcctttatgccgggatcgtcggtgatactggcagatttatgtatccttccacgtcgccacatactttggcagttgcttcaaaacttgctgaatatcatttctcaaccagtgaagtcaacaaaatagaagacgagatcgacattccactggcacggctgtccgcttatgtttatgagaacctgaatattcttgatagcggtgccgcttatctggttttgtccaataaagtattagagcccttcaagttaggggacgaaagtacttctgccgtcgtgccattacctggcaagatcaaacaagtggtttcctgggcaattttcgtcgaacaaaaagatggctcctttcggattcggttgcgctctaaaggaccagaaatcaacgaattggccaagcagtatggcggcggtggccatccactcgcaagtggtgctgttgtcgaagatgaagcccacatcaaggaatttgtgagcgatttgaatgatttagtcgccaaaaacaagtaggagattatatgagtaatttttcagagtttaatttaaagccattcttattggatgccgttaaggagctgaacttcagccacccgacacccgtccaggaaaaggtgatgcccgttatcatgcagggaagagatgtcgtgggccaatccgctactggtagtggtaagacccatgcttttctgctgccgatttttaaccagcttgatcccgcaaaagatgaggttcaagcggtgatcaccacccccagccgggaattagcctatcagatcattgatgccgctaagcagttggctaagcactcaccagaaccaatttctaccggtgcctacattggtggaactgacaaggcgcgtcaggaaaaaaagattcaacatgagcagcctcaactggttgtcggcactccgggtcggatttgggatctgatccaaaacggtggactggatgttcacacggcttctcagttagttatcgacgaggcagatatgactctggacatgggattcttggatgtggttgataacatcgctgccagtttcgggaaacatgttcagatgatggttttctcggcaacgatcccacaaaaaatcaacgtctttttgaagaaatatatggttaatccttttatcgaagagattccggtgtcaacgattatcagtccgacgatcgataattggttgatttcgacgaaggggcaggacaaaaatcaactcatttataaattgctgaccattggggaaccttatttggtcctgatttttgccaatacccgcaaacgagtcgaggagttaaccgagtatttgaagggccagggattgaaagttgcgatgattcatggcggtctcaagcctcgtgaacgtaagcaaatcatgaagcgggtcaaaaacctcgaatttcaattcgttgtcgcaactgatttagctgctcgagggattgatattgaaggggtatcggatgttatcaatgatgatattcccaccgaggatttggaatttttcatccatcgtgttggtagaaccggccgaaacgggatgtccgggacttcgattacgttgtattctcctgatgaggaaaaagaagttgaagaacttgaagatatggggattcatttcaagccgaaagcccttaagaacggcgaaattgtggattcttatgatcgaaaccgtcgaaagactcatcgaaagaaacacgataagctggatccaacgatgattggcatgatcaagaagaaaaagaagaagatcaagccgggctacaaacggcgaattaaaaataccattgcccgaaaggacgagatggatcgtcgggttgctaaacgtgaggaagcacgggccaaacggaaacaacgtaagaatagttcttcacggtatcaataggtctgtattgacaccatattcacaaaaaagtatactttgagatgtgttaagaacatgccgtttaattttttgtttcagagacgttttggttggtgagaaaagcgacgaaaattaaacggtgctctcttaaaagttaaattatcaaacgcaactctgcgttatagagatcaagtggttaacgataaacatcgttgcaatcagagtggtaccgcgtcaatgggcgtctctgtgagcaacggtgttttaattttgtcaaaggagaagagaacatgaaacagttaagcagtggtcaaatcagacagatgtacctcgattttttccaggaaaagggccataccattgaaccaagtgcctcactcattccagtcgatgacccaactttgctttggatcaattcgggtgttgccactatgaaaaagtattttgacggttcagttgtcccgaaaaacccacgaatgaccagttcacaaaagagtattcgaaccaacgatattgaaaacgtcggtaaaacaccccggcaccataccttatttgaaatgttagggaacttttcagttggtgactatttcaaaaaagaagccattacctgggcctatgaactgttaacttcacccaagtggttcggctgggatcccgataagctttatatgacggtttacccgaaagataaagatgccaaaatgtattgggaaaaagtgggcgttgcgcctgatcatatcattgaaattgaggataacttctgggatattggccagggaccatccggccccgattcagaaatcttctatgatcgcggcaaggactttgacaatctagcccctgatgacccggaaaattaccccggtggtgaaaacgaccgctggctggaagtttggaacattgtgttctcacaattcaatcacaccccacaagatacttatgaaccacttcctcgaaaaaacattgataccggaatgggtcttgaacgagtggtttcaattttccaacatgcccgaaccaacttcgaaaccgacctctttttgccgatgattcgcaagactgaagaattaagtgacaataagaaatacgataccaacaagaaggataacgaagccttcagaattattgccgatcatgcccgggcaatcacggttgctatcggcgatggcgcattgccttccaacgtcggccgcggctacgttatccgtcgcttgattcgaagagcaatcgttaacggtcagcggcttggaatcaacgaagctttcttatacaaattggttccagttgtcggccagactttggaatcatattatcccgatgttcttaagcaaaaggattatattgccaaagttgtccgttcagaagaagatcggtttaacgaaacgctgactgacggcttgaaactgttcaatcaagtggtaaaagacgccaaagcaaatcatcaaacgaccatcgatggcccaactgccttcaaactctacgatacgtatggtttcccagttgagttgactgaagaagaggccaatgatgccggcttatccgttgacaagccaggctttgaggttgaaatgcaaaaacaaaaagatcgtgcccgaaaggccagaagtggtgccaagtcaatgggtgttcaacgggatctcttaattgaaatcaaggatccaagcgagtacgttggctacgataccttggatgtcgatcacgccgagcttttggaaattgtcgagaacgaaaaactggtcgatcattcaaagggtggctctgttgaagtgatctttgacaaaacaccattctacgcggaaatgggcggccaagttgctgaccggggagttgtccttgatgaagagggagacaaggttgccgatgtcgttgacgtccagcatgcacccaatggtcagaacctgcacacattaaaaactcaggaacccctcgaaaagggcaagacctatcacttgattgttgacaaattattccacagtcgcgttgagaagaatcacacagcaacccatttgttggaccaatcattgcgaaatgttttgggtggacacacccaacaagctggttcactcgttgaacctaactatttgcgatttgattttaaccactttggccaggttacggatgaagatttacagaaggttgaagatatggttaaccgccaaatcttcaatgaaatcgatgtcaacactgttgtcacggatcctaagaccggtaaaaagatgggtgctattgccttatttagtgaaaagtatggcgataaagtacgtgttgtcagcattggcgacttctcagttgaattctgtggcggaactcatgttaacaatacccgcgacattggcttattcaagattgtctctgaatccggagttggggctggtgtccgccgaattgaagcggtcacagccaaagatgctttcaagttgctgaacgatcatgaaaaggaactgaaacaaattgccggcgacttgaaagtcacccaaattaaagacacacccaaacgggttgaccaactgctgggcgaaattaaggatcttacccaaaaacaacagtcactggaagccaaattggctggacaacaggctcaaaatgtttttgccgacaagaaaactgccggtaagtattccattatcaccggaatcatcaaagatgccggaatggatcagctgcgccaattagctgatacttggcgctctaagcatttgtctgacgtcttggttcttggaaccggcagcggcgacaaagctaacttgattgtcgcagtggcagatgaacagatcaaggcgggcattaaggctggtgatctgatcaaatcgatcgcgggcaatattaaaggcggcggcggcggtcgtccaaacatggctcaggctggtggcaaagatcctgctggccttgataaagcgatgagcgcagcggttgattggttggcaaataaataattattacaccacggttacatgtcggttacattggcttacttgattgtagtttcacttataatcagttaaaattaatacaaatgaccttaagtcatagaggtgaattgtatgagttcgttagataaaaccatgttttttaattttaatgaagatcagccaaaagacgtccgcgaaacattgttgactgtgtatgcagcactggaagaaaaaggttacaatccatataatcagattgttgggtacttgatttctggcgatccagcatacattccacgtaaccttgatgcgcgaaatcttatccgccgacatgaacgtgatgaaataatcgaagagttagttcgtttctatttggataatcatccaaccgaaacgaaaaaaggtaaaaaatgagattaatgggtttagatgttggttcaaagaccgtcggggttgctgttagcgaccagttgggctggacctcacaaggggttgaaataattcgaatcgacgaggacaacaaggaatttggtttagatcgggtttccgagttggttaaaaagtaccaagttgatggatttgtcgtcggccttcccaaaaacatgaacaattctttaggcccccgggctgaagcttcgcaacagtatggcaaacgacttgaagacaagtttaacttgccagttgattttgaagatgaacgattaacgactgttgaggctcagcggatgttgacagaagaagcagatgtttccagagccaagcgcaaaaaagtgatcgataagctggccgctggcttgatacttcagaattatttggaccgcaatggtaaattaactaaaatatagcgaggtaaacaattatggcagaccaagaaccagtacaacaacaaattacattagtcgacgaaaacggcgatgaaactttatacgacgtattattcacttttaaatcagaggactttgatcggtcgtacattctgatttatccagatggcaaaggtgaagatgaagaagtcgaaattcaagcttatgcactgccaaagggtgatgatccaagtgaccctcaaggtggagaacttcaagcaattgaaactgacaaagaatgggatatgatcgaatcagttttgaacaccttcttgggtaaagatggcgacgatcaggatgatgacagcaacgacaatcaataattaaagattgtccctattgcgaaaggattgaggcgaagcatcgttgagtctcagtcctttttaattgaaagaatttaggatgtgatgtaatgtctagtaacgaaaaacgtcgcttcaaaacaaccattgatggcaaggattacgtgcttgtcggtaagggatcggttgatcatatgcaggcggtgtccgatttattaaatgagcagctcaagcaacttcatgaggcgatgccaactgccactgatgagcagcgggcaatcctaattgcctttaatgcaatctccaaacaatttgatgttgaggaaaaagcacacagtaaagaggttcattagatgatttttacaattgggatcattctgattttaatatttggctttttccgcggccttcatcgaggtttcgtgaatgaagtcttaagtctgattggctttttggcggcaaccatcgtcagtatcgttggaaccagtccaattgctgactttattaatcaggcaatttttaaaaacggcggcaatcaaactgctgagttgattatcaaatgggtgatctttgccttcctttttgggtttgtttggcggattgttcgtttgctgagtgatctattatctccgatcacccgcctgccattattacatcaattgaaagcactactgggtgcagccgcagatcttctcatcaagtatttgttcattttcatcttgctgaactttctgctgatgttccctgatcagagcattcaagaacagtaccaacaatttgacgtttcccagtggattgtgaaaaaaacaccgattctctcagataaaatgattcagatttggaatcaacattctagtgaggttaatgtatgaacgaaaaagttttagaaacattagagtatggaaaaatcaaggagcagctggccaaatatctgacgaccgaccgtggccgacaaattgtcgatttattgacacccagtccttcctttgaaaccgtttctcaacgcttggcacagacggccgatggggctgacattgtccgcttaaagggagaaattccgattccaaaactcgcagatattgcaccgtatatgaaacgcctgcggattgaaaatgcgtcattaagcggaactgagctgtctcatatcaccaaattactacgcgctgtgcaggtcgtcactgaattttttaggggcttggcggctgaagaagtgactttaaaatccgttccctcaattgtcgatcggctcacattgatgcctgaagtgaccaaacgaatggtggcttcggttgatgaagacggccgcattctggatggcgcttcttcgcaattacgttcaattcgccggaccattgcggccactcaaagtaatattcgttcgaaaatggggaagtttattaagggatcggatgccaaatacctttctgagccgattattaccgttcgtgacggcaggtttgtcctgccaatcaaggccgaatataagcagcgatttggcggcatcattcatgatcaaagtgcctctggccaaacgttgtatgtggaaccaaacaacgttgtcgaaatgaacaatcaattgcgtcgggatcagcttgctgaaagagctgaagttcggcggattttggcagagttaaccaatttaattcgcccgcatcgtgacgagttgttggccaacatggatttggttggccaattggactttgtgaatgccaaagccaaatttgctcatgccactggtagtgtgatgcccaaagtatcaccgaaaaatgttattaatctcagaaaggctcgccatccgttaattcccagagatcaagtcgttgccaacgacattgaacttggcgatcagtacaatacgattattgtgaccgggccgaataccggtggtaaaacaattaccattaaaactgtcggcctcctgcagttaatggggcagtcaggcctgtttattactgccaatgaagactcccagattggtgtgtttgataacgtctttgccgatattggcgatgagcagtcaattgaagccaatctgagtaccttttcatcacacatggacaatatcatcagcattctaaaacagaccagtaaagacagcttggtcttgctggatgaacttggtgccggtaccgaccccaaagaaggggccgcactggcaatggcgattattgatgcctttcatcaaattggcggcgaactgattgccacgacccattatcctgaattaaaggcgtttgcttacaaccggcaggggattatcaatgcatccatggagtttgatgttgagacactccagccaacttatcgatttttactgggaattcccggtcaaagtaacgccttgaacattgccagcaaacttgggatgccagcggccattattgaccaggcacgggcgtttaccgactccgagaaccaagatatcaataatatgattgaagagcttacagcgcaaactaagcgggctcacgatgaagctgatgaattagatcaacaactgaaagaatcaacccggcttcagcatgacctgcaagacaagtttaccaagtacgaaagtcagaaggaacggctcgtcgaacaggctaagcaacaggctaatcaagtggtcgaagaggctaagaagaaggccgaccgaattattgatgatctgcatcaaaagcaggcccaggtcggtaaagttgccgttaaggaaaacgagctgattgatgccaaaggggcgctcaatcaattggaatctgctccgagtctgacaaagaataaggttttaagaaaagaaaaggccaagcacgatttccatcccggcgacgatgttttggtcaaatcttatggtcaacaggggacgttgctgaggaaggataagaaccatacttgggacgtccaaatcggcattttgaagatgcagattgaagaatctgatttggaaaaggcaactccagccaaacaagataagaatcagtatcagacccacgtgtcccggaccaggtcgactgggatgtcaccgaccttggatctgcgcggtcaccgatacgaagaagcaacgacagaagtcgatcgctacattgattcggccctacttgccggctacccttcagtgacaattattcacggcaagggaaccggggcgcttcgtaaaggggtcaccgaatatttgaaacgaaacccacgggtaaagagttttggctattctgcaccgaatgctggtggggatggttcaacggttgtgaagttaaaataaaaatgattgtgtgcaatctgtttgctttttgctaaaaaattgttagtattaaactattaaaggattggagtgttttaatatgcttaaagaaactacggatcaaacttttgaaaaagacactgccgaaggtgtcaccttaaccgatgtttgggcaacttggtgtggcccttgtcggatgcagacacctgtcatcgaagagctggcagaagaaatggataatgttaagttcactaaaatggacgccgacaaaaacccggaaactttatccaaattcggtatcatgagtatcccaaccttgttggttaaaaaagacggcaaagtcgttgataccatcgttgggtatcacccaaaggcccaagttaaaaaagtgcttgatcaatatgccggctagtctttagaatgacttcggtgtctcaagcggtttgacagtcaaaaagcccaccgcaaaaccaaatcaggttttgtggtgggctttttgattggttcttcgtcaactgttgttggtgaacaaaatattggagttctaatcacttggtgattagggctctttttgtatgaactcgaaaagcgaacagcactcttagccggaatctgaagaagtttcggtaaccaaatccagtgcgcttaatgactttaatcttgttgtttgaaccttctaatggcccgttggtgtagtggtgggtgaaagtgttgccaatttcatcatgatgagccgccaaggtttggagggctgccaacatctcttccgagcacccctgcaggtggtgaaaggcttgattatagttgggccagtcgcggtttttgatggtttcacgtaaccgattcatcacgtcgtaagtttgcttgagctcgggatcaatgtccagtaaagcatcaaccacatccgtggcagttgccggataagggaagtttgtccacttacggaaagcctcgtagttaaggtgattggccggcgttaataatagtttccaatagcgtttcaaggcgtgatactggcgtgaggaagtggccagggttttcatgagacgcactcgcgtcttattaaaagcccggtttaaagcgttaaccaggtggaagggatcgatgacaacgatggcgttcgggaagatctgcccaaccaatttgggataggtatagttcatatcggtgacgataattttcacattttctcgcgcggcttggtcataatgttggaagtacttttgaagctgatagatggttctaaagggcaacaggtcaatcaattcgtgggtttccgcgtccataaattcaaagctcatcgcgtcggtggcgctcttagtacttttaacttcgtccatgaggagaactttgggtaagtagtgccagttggtttgaaagtcgtgttcagcgcgcaagagctgccgaccaacgaatgaatccgaagtggacaattcattggcaatgtgtttgaggctcactggttccgttaacttctctaaacattgtttccgggttgtatttgaaatcgtgcagtgcttcggcactgcactcgtctgcgccaggaagttggtatgacaagccttacagtgaaagtttcgccgattgaggcataggataaccgtgctgcccaatattttagcgaatctaatggtggtcttccgccaaccatagccaatgatctggtgatcattaataaccccacaattgcggcaggccttgggagaatagttcagtgatccatttaatctgattaccccatcatcacctattttgccattctcaatttttaagtgttcatcatctattcctaacaacattttcgtagtatcatttgacatagggcatttccttctttctctaaaatcttcgtggttgttggttttgatgaacggacaggaaatgtccgctttttttattctaatgaaaaacaaaaaatctgtcatcagtaatagataaaaatctattaccaacaacagatattgtagagccttttgattccaatgagttaatcatcaggcttggaattgtcatcgggatcgggttgaacgatttcaaatatagcagaagcttcttgaccatcagttggcttgtcagggctcaaataggtgcttaaaagcacaaatcccttattaacattggccttttcgagctcagcttcggcttgttggttaagaatatactgacagctttgagcgatgaatccggattccagataaaaatcaggatcatcaaatgcgttgagacgctgggcgacgatcttgccgcttagctgccagctgatctggttaccagagcgtttaagcagctttaggtcgccaaatttaaattgtttgaaaaaggtttccaaatcttcataggttgccagacgatgatttcttgccagatgcttgccggcccaataggaaatttcgtggacgtctttgcctaaaatctcaggaatcagtgaatcgcgaattaattcctggcccagtaggtctctcattgtatcgtcagtcataaaatgcttgtatacttcgttatccattttttaatctccatcaatgcaaaatgtaataaataaattatacaataaaatcattaatcttgttttgtaagttgaagtaaagattcttttgcaagataataatgttattgagacaaaggaagaaggaattctgttggataatcggccgattggcgttatggactcgggggtcggcgggcttaccgtcttaaaggaaatcaccaaaatcctcccgaatgaatcgtacatctttattggcgatcaggccaatttaccgtacgggcaaaagagttctgaaaccgtcagaaaactcacaaaaagaattgcagactatctggttgaacaaaatatcaaaatgtttgtaattgcctgtaacacagccactgctgcggcatatgaatatttaaagaaaattttaccgattccggttatcggcgtaatcgaaccgggtgcccaaatggccgttgaagcctccaaatccggggagattggtgtgattgccaccaacggcaccgtccgctccggagattatcagcgattgatcaaacaagccaaccgatcagcagttgtgtcatcgttaggctgtccggaatttgtcacgatggtcgaagaggggcttgccggaaccgttgaagctcaggttgccgtgaacaaccgactggcttggtttatggataaaccgattgatactttggtcatgggctgcacccattttccaattttaaaaaatgaaattcaaaatgtgatgggcaatgccgtcacgttgattgacccgggagtcgcaactgctcagcaagtcaaggcaaagttagcagctcatgatggttttgcccccgcacaaaaacagcgtgttcgaagattttacaccaccgggaacccggcggatttcgccaaagttgccgacaagttactgggaacaccgattagtgccgttaagttagatatttaaaggagtttgataacgtgaaaagacccgaatcgattgtgattgcctcacaaaacgctcataaaatcattgagtttgaggatgcttttaaaccaaccggaatcacgattaaatcactgaagcattttgaaaatgtgccgacgatcgctgaaaccggcacgacatttgaagaaaatgcgaccctcaaggccaccggcatcatgaactttacgcatcaagcggtgatcgctgatgattccggcctggtggttaaagcactcaacggccaacccggtgtccactcagcccgttatgcaggtgatcacgatgatgacgtcaacaacgataagcttttgaaggaaatgcaaaacaaaacggatcggacggcttactttgaatctgttctggtctatttaacgcctgagggtgacaaggtggttgccagcggtcgaatcgacggcgaaattttacgtgaacgccgtgggaataacgattttggatatgatccattattctatgtgcccagccagcagcgaacactcgccgagatgagcacccatgataaaaatctgattagccatcggggcaatgccatccgcaacctgatccgtaaattgttggggttgtgggactcatgaaaattgttgttgttagtgatagtcatggagatcgcgccattatccaagaattggtgaacaaatacgccggtcaagtggatgccattttccattgcggcgattctgaattactagcggacgatccattagtttctcaactgcggattgtccaggggaatatggactttgccgaatttcccgaccacctggttcaagaaattagcggcaaacgaatcctcttgactcatgggcatcatcaaaatgtgaatggtggcctgcttaatttggaattatatgcgcggagcttatccgccgatatcgtcctttttgggcatactcatcaattaggagctgtttttgacgatcagatgctgtttgtgaatcctggaagcattgcctatccacgtgggcaatacgccgggttgggcggtacctatgccattatcagcatgaatcaacgtaattacaccgttcaatattacaaccgccaatttgaaccggtggcgaatttggaacttcgttttccgttctaaccaaaaaggagtctaggattacatgatcgataaaccaattgagaccgtgatgcgtgaaagtcaccgggatattttaatccccgctgatttggtcgcaactgtcaatcaagacaatgatctccaacacgtcttcatggttttgacgaaagttaaatacgcaaaaattcccgtgttagataacgataaccatttcatgggactggtttctttacccatgattactgaactcatgatgcaggataccggcattaccagtcgaccgcttgagtcagtgaaagttaagcaaatcatgcaaaaggatgtcccaacgatttacgagcgggataacctggaagccattctcaggtatttggtggatgaaaactttctggtctacgttgattctgaaaatcactttaaaggaatcattacccgtcgggaactatttaaagaaattaattatttggctcacaactttaataaacactacatcgctttgccggtgtataatcacaaatccaaaaacgaaaccaagcacgccaagattcaaggctccaagggtctgattaatcgataatccattgggtgaatatcgttgatggttacaaaattgaattaagtcaaaaaacgagattactgacaaaatttgccggcaatctcgtttttctaagaattggtcactttattcaaacatcagttggcttgtccatttaccattgttgggctcgccggcagttgaatcccggcttcattaattgcagctagatagaaggccaaaaagttatgggcaacttcgtattggctgccgttttttgtggtgatatttacctgaacgaccagtttgccgttggggaggctaatggtgccaagaatcttgggatctccgataatatccggatagtgggggatctgttcttcattgacctggcggataatttgggtgactttatcaactggcgtttgtgggaaaatgccaacttgaatcatcgccgtcatattgtttcgagacatgttggcaatggtggtgatggttcggttggggatgaaattcaacgtgccgtcgtcgccgacaacctgcgtggttctcagtccgactgcggttaccgttcctctaatcgtgccaatctggacgtactcgccaacttcaatttccttttcaagaagaatgaaaaagccactgacaatgtcagtcacaaatccttgggcaccaaggccaattgccaagctgaagatcccagctgaggcgaccagggttccaactggcaccccaaccgttgagagaatggagtaaatccagaagaaccataggcagtagttcaaaatgttcagcgtcagggtgtgaaaggtcttgatccgtttttctgccacggtattttgatatttgcgccgatagcgtttgaaaaaatgattaatcagtcctttaccaatccgacgaaagagtaaaaataacagactgaataaaattaataatccgactttttccagaatcgtcatggccagctgatcccagtcaaccatgttgagatatttttgccaattaatggctaaaactgtgaattttaaggtatttatcattgggattcctcgctttgtgtataatatcatcttagcaaattggttctgcaaaagaaaccactcttcgttcattttcattgtcaaaccattgctggaatgctattcttaagtaaatgttgcacaaggaggaagatcaatgactgctggacaaatagccggccttatcgccgcaattgcatttttgcttttggtaatcttcattggcttattcttaatgaaggtaagcagaactatttcagaagtgaaccgcacaattaagacaatgaccagtaatgtggacgtcattgccaaacaaactgataatattatggcaacatccaacgatttactgaaggatgttgatgacaaattgaacattgtcacaccggtctttcaagccgccgctgatttgggtgagagtgtgtcaagtttaaataccgctactcaaaacctcactaaacgggttaaagatactggcaaaaagggtgtttcagcagggctcgccggtaagtttggcaagagtgcctggaacatgtaccgcaatcgacacggttcaaaggatacaactaaataaacaatcgaagggatgatcagaatgggtaaaaaattagcatttggcttattcgctggtgcattgggtgccggtctatatgcagcctaccaaaaattggatgaagcaaagaaggcccaactcaaacgagacgcccgtcaaaaggctgatgagttgcgggatcgggcagttgactacgcgttttacgccaacgatgccgtcagcgacttaaaagatgtgattcatgatgaaatgcaaaataccaaagggactgtcaatgatgccaaaacgcaattcgctgacaaagctaaatcttttggtaccgaccaagcagccgatgatgacgacgctgacgacaatcaggatgatattgttgttgacgctaaagatgccttccaagataccggaattcccaaggctgctgatgatttggattcacaatctgaccaggatgacggcgataatgagattccaatcactgacgactccgataacaacgataacaaataaaaaacaacctcagtgtgcaatttatccaaacagtcaaagtcaaacttcagctgttgagataaggcacaatgaggttgtttttttgatgctgttaattattgttcaatgtagcgtaattccttggttgtgtgcgtaaatggttcgcagccatcttcggtaatgtgaacacaatcttcaattctgacaccagcaacgtttggaatgtaaatgccaggctcaattgagaagcacatccccggttgaagttccatcttgttgccagccatgatagatgggaattcgtgctcactcatgcccatcccatgacccaaccgatgaatgaagtattccccgtagccggctttggtgatgacatcgcgagcaatcttatccagttcctcagcggttattcccggtttagcagcttcttgggcagccagctgtgcttccagacaaacttgatagatgtccattgatttttcatccggtttaccgactgcgatagttctcgaagcatcactaatgtagccgtcccagacagttccgagatcaaataagaccagctggttattctggactttattttcactggttgccccatggggttctgcggcgtgggggccggcttgaacaagggaagggaaactgagttccatgatcccgtttttcatcagtgcatattggagatcggcggcgatttggtcttctgttttaccaacctggacggcttcaaatccggtttgtaatgcaaaatcgtcccacttgccggcaattttcaatttttcaatttcgtcagccgatttaattaaccgcatttgttcgatcaatggggtcaggttcgctgagaaatccgcgttgggaagaacttgttggagagcttccaatcgttctacctggagctgggatttttcaattgcaaaatgactgtcgtcggtatttctggcatgaatttgatcggcaatcatcacccaagggtcttcgtggtcgaggtagccatagactggggatgaaaagccggtatctttaatggcttctgattccagtgccgggccaaagataaatggttcctgatctttaaaaatggccatcagtaagactctttcaaccggatcactataaaatccggtgaggtattggatcgttttagggtcggtaatcagtgcgatgtcttggccgttatcagccagccaccgttgaatttgttctatcttgttcataggatcactccttcattattttatccacagtatatcatacaaaattcttctcaattatcgccgtaaagttccgttttcacttgaattttcagcaatcttagtttatgatttaactgaaaacgttttcaatttgctgaaaacctttttatttggtatattagatgatgttttgaaaatcgatgaaaacatattctaacgagaaagaaagggctatctttatggataaacaaacaattacaatttatgacgttgccagagaagcaagcgtgtcgatggcaaccgtttctcgagtagttaatggaaatgccaatgtaaagccggcaacccggaaaaaagtgctcgacgtaatcgaaaaattggattacaggcccaacgccgttgccagaggtttagcaagtaagaaaaccacgactgtcggcgtcattgtcccagatgtaaccaatatgtattttgcctcattggcgcgtgggattgacgatgttgcgaccatgtataaatacaatattatcctgaccaattcagactccaataacgaaaaagaagttaaggtgttaaataccttgctctccaaacaagttgacggcattattttcatgggtaacgaaattaacgataagctccgtgaagaattcaagcgaactaaaacgccaatcgtgtttgccggatcagtagatgaagaagatctctacgcgagagtcaacatcgactacgttgccgctgtccaagaagaggttaagaacctgattgatcgtggtaatcggcgagttgccttcgtttgtggccccttggagcaggcgattaacggcaaattccgtctgaaaggctacaaacaggccttaaagagcgctggaatcccttacgacgagaagctggtctttgaaactgatgatacatacaagaccggaaccttgcttcagccagcattaatggcagttaacgccaccgctgcgatggttaccgatgacgagttggccgccggtatcatgaacggtatgtcagataccgatgtcaaagttcctgatgactttgaaattatcaccagtaacgataccaagttaaccgaaatggttcgaccaaagatgtcttcaattacacagccattgtatgacattggtgccgttgccatgcgtctgttgactaaattgatgcacaacgaaccggttgacgaaaaaaatgtgttgctcccatacggtttgatgaagcgtgaatctaccaaataatcaggtatcaaatcaaaggagtggaccgtggcgattcgctctttttgttctggaaactggtttgaaaagccgccacatatttggccgcgctttcttgaaagaggggggcgtatctggtagaatattgacgtatgtttgtaaccagctaataaattttagaaaagaggagttattatgtcaggacattcaaaatggcataacattcaggggcgtaaaaacgctcaggatgctaaacgtggaaaaattttccaaaaaatatcacgtgacttgtatcaagccgctaaaaaaggtgatcctgatccagaaaacaatcctcagttgcgtctagtgatggaaaaagcacgggctgccaatatgccaaaggataacgttcaacgtgcgatcgataaggcttccggtattggtggagctaagttcgaagaaattacttacgagggttatggtcctggtggtacagccatcatggtttctgctttgactgataacaagaaccgaactgctgccgcaattcgttctgcattcactcatcatggcggaacccttggaacaagtggatcagtttcatacatgtttgatcgaaagggttatattgtgattctgcgcgatggtcttgacaccgacgaagacacaatgttgatggacgcgcttgatgccggtgccgatgatatgaagaccagtgatgatgaattcgaaatcttcactgatcccaaatcaatggacgacgtccgcgacgctttgcaggaaaaaggctacgacttggatactgccgaagttcgtcttttccctgaaaacacgacagaagttccagaggacaagatttctcaatacactggtttaattgacgaactcgaagaaaacgacgacgtccaagacgtttacgaagccgctactttaccagaagaataatttaatatgatttcagtgtctcaatggccgatcatttgatcggtcatttttttatgctttgataaataaaattcaacttttcattcgtatgtattacatgtgaggtgaatgaaatggaaattagtcagcaagttaatggtcttttgaatgaagccattaaaacacaagccagtgatctttattttttacctgaaggagacgaatacctggtaaaaattcgtaatgcaaacgaagtcgttgtttgggataaaatcggctatctgcaggcgagacggatgatgaactattgcaagtacatcgcagatatggcattaagtgaacaacggcggccacaaattgggtcgatggattggcattttggtgataaccaatattttttacgattatcctcggtcggtaatttcacggggttggagtcactggtcatccggattatctatcagcttgatgatgtgcacgcggcattttttgaagaaaaacaagttcaactaatttccgaaatgagtcgaaaacgcggactcattgtcttttccgggccaaccggctctgggaaaacaaccaccatttataatttggtaaatcagatggtttccgaccaatttgtgatgacgatcgaagacccgattgaaattagggaaccgcgttttttacagctccaggttaatcacgatgcagggatggactacaccgacttgattaaggtgggcctgcgtcatcggcctgacgtctttatcgtcggcgaaatccgtgatgcaatgacagcagaggcagcaatcaaagccgctctgagtggccatttggtctacaccaccgttcacgctcaggatccggttggggtcattgatcggctcaaacagctcggaatcagcgacgaatttattgcccaagccttaaccggcgtcgcttatcagcggctgattccaaccaccgacggcaaacagcgggcaatgttgatgggacatgattattcagagttggtcaatatgaatacatacgattggggtgaatggcaggatggactcaaaacagctgttaaagcaaaactggttacaccggaaactgcacaacgattcgagttcggttaagaaatggccggtggttttccaagctaatttttttgactctttggcgaatcttttgtcaattggattctcactgactcaagcgttgaaatttatcgccgacactgacaaacaattgtcccgaggcgttaatgtggtgattggatcgttaaagtccggccgggaattttcggaaagtgtccgacccctgattgaaactcaagcttatcaccagctgttaatcgcggagaagcacggtcaactcagtgacattttaaacgaactggccaactttgatcgattgcggctcaaacaactcaaaaagatcaaagcgatgttggtgtacccattatttttgtgcctgatcttaggaacgttgatcttgatgattcgagtctacgttttgccacagattcaggatttaatgcccacagccaatcatcagcaaccggttacgtactggcagcagctgattcgactttcgccaatcccaattttgatcggcatcattggcagcacagttcactggagtcggcaggatgccataacccaggcccaaatgattgtcaaaatttcgggcgtcggcaaattgtttcgaaaatatattgcttattatctggccagcaatttggccactctgctgaaaaacggtttgagtgttaaggaaatttatgccacgttatccgagttcaaggagggatcactgattcatctcttaggtgaaaggcttcatgccactttactttcgggagggtccttaagaaaattggtagaccggcacaattttattcccaatgagattatcaaatttatgagctccggcaacacgattccggaaatggccaattccatgacggcctattcacggttgatgtttgacgaaatgatcctgaccaccgataaactgattgggtttattcagccggctatgtttgtggtgatcggtgtgacgattatttcgacgtattttcaactgctaattccaatttataactcagtgaaaggaatgtattgaaatgaaaaagcgcgttaagaaaatgagagaaggctttacgctaatagaaatgaccatcgttttgtttattatttcattattgattttaatcattattccaaatctatccaatcaaagaaaacatgcccagtctgttcattcatcggcaatgaccgaagttgttcaggcacaaattgacgcctatttcagccagcacccaaccgccaaatcagttagttttccaggcctgacaaaaggtggctatctaaccgccaagcaggttaaacaagccaaggatgaaggcctgaagattactcataatgaagtgcaaaaataggggtggctttaccgttattgagctggtggtttatttaggcgtggtgttaggtgtcttgatgattaatttgatgctgatcaaggtcgtccagtctggaaatccaagtgaggcgttgttttggcggtcatttcagagtgcttggacccgcatgacattaaacgcaaaggccgagaacatttcttatcgaatctccattcgcgataaagatgttattttctttccgatgaaggtaaagaaaactcactatgacgaggtaaatgaggagcggatttcggttccgccttccattcacgtgagatcacaacgaagcatgattgcccatgacgatgggtttgcatcaccaactaagcttatttggcttgattcggatggtaacgtcaaatacaatcaaaaaattcaaatgggatggagtggctatcatgtggaaaggtacaaataagcgggcttttacggtgatcgattcattaatcgggctgaccatcatctgcaccttcagtttgttctacatccaaaccacccatcaaatgaatgagacaattaccaacgcagaaaaagtgatgacaattgagaggcaaaaatatgaaacagaaattgtccgtgagtaaggttgatactcggccgggctacttattaattgagggcctgatcaccttggtgattggtgtattcgccatttggacgatcatgacgatgatcgtatatgccgggaacgaaaaaaagcaaaacgtgatcaattttcattcttatctcagtataatcgaatctgaccgttatcggtttgaaatcaagcagtgtcaaccctctaagtgcgtgatgtacagtccggtcacgaaaaaaacttatcgaattgaacggtatcaaaacatggttcgattggccggtgcttacaagggtcacgtaccgtcgttgacaaatgttcaatgggtacgctggacaaagagcggggggtgtctaagaactgatgttactttcgataatggccaaaagtgttcagcttattcaaaattaccgttcaaggattgataaatataagcgtggatccctaacggtggtggccgtcatttttgtcggtattttgatgtcatgcttgatgtttcaactggctgcttataagcaggagttgggatcaattaatcgtatcaccgagcatgaacggcaaatgagacggcaatttcttgaaaagccaatcaaaaaagatgttcacccaaaacgcacaagtggtcacgaatagtggcctttttgtggttgtgaaataacaatctaacttgaattattgacagcttatctggtagtatttaatagtgttcaactattgaataaaggggttgagagttctggctcaagggaaaattgagcagctttttgatatcttgaatcgttcgacagaattgattcaaaaagccaaggatcaatcgtatcttgattctttcatcgaaacactgggatttatccagagtgacgatgaagaagatgacgaactgactgaagttgataccaaaaagctgactaatatttatgcagactttaatccggatgacttcactgccgaaactttccggaaagcaattcaaatggctgtgctcaaggcgattcgagttgacacaattcaggctaattaccaactgacgcctgataccattgccaacgttattggctatattattgccggaattttccatgaccgcaaagaattaagcattcttgatccggcaatgggaactgccaatctactaacagcaatttatcatcagcttcaaaccagcattggcgttacaccaaccatttccggaattgaaaatgacgatgcaatgtttgaattggctgcagactcagtcgagctgcaaaagattcacgctgagcttttccacgaggatacgatccaaaatgttttagctcccgtggtcgatgcagtcgttagtgatttgccgattggctactatccaatcgatgctaatgccaagggatttgctacccattcagagacgggtcattcatacgtgcaccatttgctgattgaatttggcatgaagcatgttttgccgggtgggtttggtttcttcctggtgccaagtcagcttttccaaaccagcgaagccaagcagcttcttaaatggatgcaagggaagatttacctgcagggattacttaatttaccaaaagaactctttgcaaacgctgcggcccaaaaggcaattttgattcttcaaaatgctggcgacggtgccaaacaggtggatccggtaatgttgggggaatttccatcatttaaggaccaacaagcctttaccaagttcttgaccgagattgatgattgggaacaaactgatttattataaaattgtttatcaagctttttaaaaaatacagaggagcattatttattatgggaaaatcaattgcaattaacgctggtagttcaaccttaaagtacaagttgttccaaatgcctgaggaaaccgttctttcaagcggtgctattgaccgaattggattgggcgcatcagatatctcaatcaagtacggtgacggtaagaagttcaaagatacccaagatattgataatcatgaacaggccattcaactggtccttgataagctgttaagtttggacatcatcaaagactatagtgaaattaccggtgttggccatcgaattgttgctggtggggaactcttcccggattcagttgtgattgacgatgaggtcatcaaaaaaatcgagtcactaacggagttcgcaccactgcatgagccggctgcattgcttggcatcaaagcgtttaagaagattctcccaaatatcattagtgttgccgtctttgatacttcattccatacaacactcccagaagtcaactacatgtatagcttgccttacgagtattatcagaagtatcaagttcgtaagtatggtgcccacggaaccagctatcgttatgtctctgccagagcagctgcccttttaggtaagcctctgaaagacctgaaattaatcgtccttcacttaggtgccggagcttcaatcgacgcaatcaaagacggcaagtcatttgatacctcaatgggcttctcacctgttgccggcattacgatggcaactcgttcgggggacgttgatccttctgcattacaatatgtgatgcaaaaagccggtattaaaaacatggatgatatggttgatattttgaaccacaaatcaggtttggtcggtttatcaggtgtttctgcagatatgcgtgaaattgaaggggttatgaagactaatcaccgggcaatgctcgctcgcgaaatctttaagaatcgtatcatccgctacattggcagttacattgctgaaatgggtgggattgatgccttggtcttcactgccggaattggtgaaaacgacattatgattcgccaggaagttaccgataagttgggctacttcggtatcaaagttgatcctgaaaagaataacatccgtggcgaagaacgtgacctgtcagctgctggttcaacggttaagacattgttgatcccaaccgatgaagagttaatgattgttcgcgatatcgaaagattacgcaaaacacagaaataatttttggacgttcgtcattaatacccaatcattacgggcgaagatcgttgctttttcaagcatagaatccgttgagccccatttgaattcggacgtcgcgggttacaaacgaggctgagacaaaagggttttgccttttgtcccagccttattgtttaataaaccaaattgtcattttttagaaacggaggcacattgtggaaaatcaagaagacgacaaccaactgtcccggggcctcaagaatcgacatgttcaattgattgcccttggtggaacaattggaaccgggctgtttcttggtgccggccagtccattcatttagcaggaccatcaatcatcctggcatatgggattgccgggctggcttgtttcctattaatgcgggcgctgggggaactgttggtatctgatgtcgaaagcaattcgtttgttttcttcatcaaaaaatatttaggcgaaaaaatgggcttcgtgatcggctggacctattggatgtgttggatcgccattgcgatggcagaagtgacagcctctggattatacgtccagttttggttcccggacattccaatctggctgacaggtctggtcctcttattgatcctatttatcatcaatatcgtcgctgtatcagcattcggtgaaaccgagttttggctggcaattgtaaaaatcgtcgcaattgttgcactgattgtcattggaatcgtcctggtggcaatccattttaaaacaccatacggacacgcatcattgatgaatgtggtggatggcggtttctttgccaacggtgcgaagggttttgttttgtcctttcaaatggtgctcttcagtttcgccggaatcgaaatgattgggatgacggcttctgaaacccaggatcctttggtgacaattccaaagagtatcaacgaagtgccaacccgggttctcttgttttacattgggtcgctgttggcactcatgagcattttcccatggcagcacgtttcgccaacttccagtccttttgtccaggtttttgccggtgtgggcatccagtccgcagctttgattattaattttgtcgtcttaactgcggcaatttcagcttgtaacagttcgttatttaccactggtcgaatgctgttttcattgacctacaacggtaaatcaaaattcagtcgaaaagtcggccgtctttctgcccgtcaaattccgtttaacgcaattcttttttcgaccttggtgatcgcggttatcgtgctcttgagtattatgatgcccggcgacgtcttctctttcatttccagtgttgctacaacttgtttcctgtttgtctggggaatgattgtgttggctcatatcaagtatcgaaagcaggttaaaaaaactggcagtcagaaatcgctcaaatttaagatgccgctttttccaatcagcgattactttgtactgattttcatggcttttgtggcagttgttttgaccatgaagacggatacgctgattgctttaatcggctcggtggtttggctaattggactgtttattttcaaaagtctgacagataaggttaaagaagttgaaaaatgatgattggccaaggcatcggcgccttggcttttttcattggtattatcagctttgtttgaatactttttcattactaaacggctgctgggtggtatcattaatggtataacttatgtacgaaagaggacctgttcatgcaattttttactgctgatacacatttctttcatgaacgtttacttggcgttagcgagttcgcaccacgaccatttctgactgtcgaggatatgaatgaaaccatcattaacaattggaatcgtcgggtgggcaagaacgatgtggtgtatcatcttggtgacattgcgattttgcatacccgacctgagaaagtggcactggaaaaaatttttgaagtgctggatcaattgaatggccgcttggttttgatcaagggaaatcacgattcccgtgctttgttcaaatatctgcagcagcataatcatcccgtgggcaatcatcaaaagtttgagtttcacgatgttggtgttctcatcaagatgaatcatcgtcagtattatatgactcactatccgatgatgatgggcatcgttaaacaaattattaatttacatggacacattcatcattatgcagttccgattaaagaaaatatcaatgtcggtgtggatacgccggaaactgattatttgaaaaagaagccaccgtttggaacgccattttcccaagctgaaattgaagaaatggtcgccggaaaagctgaagactttgccaagcggcactaatttagaaaagattggatggtttgatgactgagaagctaacaattttacacacaaacgatctgcactcccatttcgaaaattggccacgtattcgtcaatttatcaccacgcgacgcgcagaacttcagcgagccgattcttccgttatcactgtcgacttgggggatgcggttgatcgcgttcacccgctcactgaggtaaccaacggcaaggccaatgtggagttgctcaaccaaattcattatgatgccgtcacaattggcaataacgagggcttgaccaatagtcatgagcaattggacgagttgtacaatgatgccaatttcgacgtcattttgggaaaccttttggatcagcagaccaaatcaattcccaaatgggctcatcccagcaaaattattaccaccccgcagcatacacgcgtgcttctgattgggctgacagcgccttatttactgacatatccgatcttggggtgggagcctctcaaaccggaaacggtcctgcctaaaattctcgccgacaatgccggcaaatatgatatctgtgtgttactatcacatttggggctgccaaccgaccgtctattggcacgtcagtttcctcagctggatgtgatcatcggctcgcatacgcatcacttacttgttcacggtgaaaaagtgaatcattcactactggcagctgccgaaaaatggggccattatattggtgagattacactgactatcgatggttcccatcggattgtagccagtcaagccaaagtgattaaaaccgctgatttgcccagcgaacctgaagatgatgctgaaattcaggaatatcaagaacacggtgaaaaactgctggcacgcaacaaacttgccagaatcaaagcccccatgacaactaatctcatcggccattcgcgcttggtaaacgaaggtttgcatgcgataatggaaaaagccgatactcgcgctgccattttaagttcgggcctatttttaaccgacctgcctcaagggattgttgatcgaaatcaattgcatcagatgttgccccacgcgatgcatgtcatgcgggtcactttggacggttataatctctggcgcctcatcaaagaaatggaaaagaacaagaactttttgaccaaattcccacaaaaagggatgggctttcgtggcaaatattttggccagctacattatggcggattgcggtatgatcaagatgccggccagctctttttccatgaagagttggtttcaccggcgaaaacataccagattgccatgccggaccactatttgtttattccgttcttcccgacattggagattatcggccacaacgaaattttatacgatgaaaatttaagggatgtgtttggggattatctcgccaaacattatccacttaatcagtgaaaggagggttactttggacagaaaaaccttagatgaactcgttgcgaaacaagacgagaatcgaaagccattggcacgaatcaaccgagtcagtgaaacagaattcttaatcaatgatcataagtatgaattggataccaatcacacggatggttttgactttgacgaattcgttcgtcggtacaatccggcttttagtcagtatgattacattgttggtgactggggatacggcaaattacgtttgcggggattctttaatgatgaccgaactgaaacttccggcccgtttatttctgcactcaacgactggattttggaggacgtcaacttcggtgccgcttattttgtcgttcataatcttgaggcccgaccggtgatcagaaaatcccggaataatcgaggtaaccatcgatcaaaccggtctcataattcccgcaaccggagtaatcatcgcaatcatcggaaccacgcctttgaagaaaagaaggttaccgcccataagccagttgaaaagcgccataatatggtcgtgaagactgaagaaaaatcaaaaaagcaccactttattattcgtgagagtaaaaaataattagaaggattgacttgatgacaaactataagggctattttattgatcttgatgggactgtgtatgccggtaaaaaacgcattccggccgccaaacgatttattgagcgcctgcagaaggccaatattccatttttatttgtgacgaataattccactcagctccccagagacgtggttaagaacctggctgataaccatgatattcacgtcaaaccggaaaatgtctatacatcagggatggcgacggttgattacatgaatgagcatcgtagtggggatgcttcatctgtttacatcgttggtgaaatgggcttgaaacaagttatcttagccaacgattatcgtttggaagccgatcatccggattacgtggtcgtggggctggattcagacctaacctatgaaaagctttcagaggccgtcttagccattcgaagcggttcgacgttcattggtaccaaccccgatacaaacattcccaaagagcgtggaatgatgcctggagccggttcggttgtgaagtttgtcgagtatgccacccaagttgaaccgatcatgattggcaagcccaaagccagaattattgaaagtgccattaaaaaaattggccttgaacagtctgacgtcgtgatggtcggggataattacaacacggatattaaagctgggattaatgccggagtcgatacgctcttggtttataccggactttcgacaaagcaacaggttgccaaagaatcggttcagccgactcaccagattgactcacttgatgattggcggttataaatgtgaaaatgcttggaaaacaaattggctatggcactttaatcatattggggtgccttgccctcgccatctttttgactgtcaacagtgtttggctgtttgacctcaatattaatccgctcaaattagctgcggctaccggtcgcactgctagccagatgcatcatgattatgtcaggattatcgcctatttacagttgccgtggattccttctttaaagctggattacttcttcagttctgcaaagggactgcagcactttcgggacgttaaagggttgatcctgttcaacaattttgttgggcttattttagtgccgactggtgcctacctactgcatcggctcaacaaaaaatcactaacttggctgttgatgacgccaattaaggtcgtcaccacagtttcgttagtgattatcgcgttgatgtttgttaattttgaccaggtatttgtggcatttcatgaagtattatttagaaaccaggactggatttttgacccgaacaccgatccggtgattaacatgctgccggatacgtttttcttggaatgctttctactgttctttgtcctattttttggtgggttggcagtcatctactggcttggccgcagatcactgaaacagcactaattattctggtgctttcatcaaaatccaaagcagtaggtatgcgatgattcccgggaagaatggggtaaatgccagaatgacaaatacgacccgtgccaaagtgggatcccattgaaagtgctcagccaagccaccaatgacgccggcaagcaccttgtttgttgcggaacgatggatattaattttcataatcatcatctccatattttaatttaagtataagcttactataaccaattcgcatttgcattgcaattatgctatattattatgttgtataaaggaaataactaggagaattttaatgttaactattaatgtcaatggaaatctaggaaaccaacaagttgttctttctgataattcggttgggacgttgactggtgccagagttttcggctcagccttgagcggtaatcaagttgttcaatggacctttatctcaaccggccatcagcatgaaggctttgtctatgcgggtccattactggaaggcttagtgatccagtcgatgaacggcaatgacacctaccaaattcattttacgaataaataatcattaacaatcagcggcatacataatgagactggatattgcacctaaaatattcggtctcattctttcttaaaggagagtattatgacaattggaatcgacaaaatgggtttctttacttctgattactatttggatatggcagatttggcaaatgcccgcggggaagatcccaataaatatttgattgggattggacagaagaaccaggcggtaatcccgccaacacaagacgtggtcacgatggctgccaatgctgccgccaagattttaagcgatgacgataaacaagcaattgatatggtgatctttggaactgaaaccggtgttgacaactccaagtcagcggccatctatgttcagtcgttgcttggaatatccaactccgccagatcgtttgaaattaagcaagcctgttatggtggtacggccggcgttcagatggctttcgatcatattgcaatgcatcctgaaagtaaagtgttggtcttggcagcagacattgcccgatatgggattggaacagctggtgaggtcacccaaggcggtggggcaattgccatgctgatgagtcaggatccaaaaattttagctttggacaatcaaagtgcgttttactcagaaaatattatggatttttggcggccgttttaccgtcgtgatgcaattgtcgacgggcattactcaacggatatttatatcgatttcttcaaccaaacatttaaagattactctgcgaaatatcaacggacgctgagtgatttttccgcgatggcttttcatctgccattcaccaagatgggcctaaaagcgcttcggacggttatcgatgatggtgctcactcacaacagctgctcaaagaattcgatcattctaaaaagtataatgccctcgtcggtaatctctataccgggtcactctacttaagcttgttatcactactggccaactccaaaacgcttcagccaggtgatcgaattggtttgtttagttatggatcgggagctcaaggggaattttacagtggtacaattgcccctgaaatccaaccgcagagccttgccggccaggttgaacaagtgattgccaaccgaacgaggctgtctgttcctgagtatgaagcgatgtatgcaaatggattgccaaacgccggtggagatgttacatttgatgctgccgatgatgacagtcgattcgtgttgcttggcagacaggccgaccagctggtttatcgagatcaacaggcataatattgatggtagaagggctcgttgggcattgccgaaaagtcctggaccagaactcagggtaaaagaaagggactgttagcagaacagtccttaggtagaaataattatgaaatatcgctgcggtacaaactgaccacttttcccaaaatgctgaccttggtcaaaataatgggcgccatggtatcgttttctggctgtagtcggtaatgatcgctttccttgaagaaccgtttgcaggttgcttcattttcatcggtcatcgcaatgacaatgtcaccgttatcggcgctttcctgtttgcggacaaccacatagtccccatcgagaatgccggcgttaatcatactttcgccccgaatttgcagcataaataatggttgatcactgtgtgccagagcaggcgggagcgggaagtagtcggtggcttcctgaacagctaagatcggttcaccggcagtcacagttcctaaaaccggaatctgtttttgctgcggctgcatacccaggacatccaagccactactggtgacttccagcgcgcggggtttggctggatctttcacgatatagcctttccgctcaagtcgagcaatatggccatgtaccgtggaggttgaggatagatgaacggcttcaccaatttctctgaccgttggtggatagccctgctcattaacccgttcccagatgaagtgaaggatctggtattgtttactttggggatcattggtcgtttttgacattttagacacctcataagtctttgtttaatacctaaatcatatcataacccgggtcacatttcaaaacacacgttcgcgtaactatcaataattgtgttattatagtcgatatggaggaattttaatgaacgaacaagagaaaaaagaattgcaatcaaaaatcggtgacgatgttttcaaagaactcatcccaagaattaatgaactggcccacaaagcaaaaaatgagggcttatctgaagttgaaaagttggaacaggctgatttgcgtaaaaaatacgttgctcacttccgtgaaaacttcaaaaaacagattgaaatgatgaaagtttatgataagaatggcaaggaagtgacgcccggaaaagtcagggaagtccaacgtcacaaaggtcttcgggacgattagggggcagttttcccctaagaatcgggattttgttgattagccctttaattctatggcataattgtgtaaaattacttagtgatatgataaaggaggccttgtcttggcaacttggatttggatattaatcgttgtgttagccttgatcttgggcttggttggtggcttttacggtgctcggaagtatatggaaaagtacctcaaagaaaacccaccattcagcgaagatcaattgcgccaactgatgatacaaatgggtcaaaaaccttcccaaaagaaattaaatcaaatgatgcattcgatgcaaaaccaaactggtaaaaattagaatgtttcaatgacaaaaagtccccaccaacttggtgagggctttttgtggttcttcgtcaactgttgttggtgaacaaaatattggagttctaatcacttggtgattagggctctttttgtatgaactcgaaaagcgaacagcactcttagccggaatctgaagaagtttcggtaaccaaatccagtgcgcttaatgactttaatcttgttgtttgaaccttctaatggcccgttggtgtagtggtgggtgaaagtgttgccaatttcatcatgatgagccgccaaggtttggagggctgccaacatctcttccgagcacccctgcaggtgatgaaaggcttgattatagttgggccagtcgcggtttttgatggtttcacgtaaccgattcatcacgtcgtaagtttgcttgagctcgggatcaatgtccagtaaagcatcaaccacatccgtggcagttgccggataagggaagtttgtccacttacggaaagcctcgtagttaaggtgattggccggcgttaataatagtttccaatagcgtttcaaggcgtgatactggcgtgaggaagtggccagggttttcatgagacgcactcgcgtcttattaaaagcccggtttaaagcgttaaccaggtggaagggatcgatgacaacgatggcgttcgggaagatctgcccaaccaatttgggataggtatagttcatatcggtgacgataattttcacattttctcgcgcggcttggtcataatgttggaagtacttttgaagctgatagatggttctaaagggcaacaggtcaatcaattcgtgggtttccgcgtccataaattcaaagctcatcgcgtcggtggcgctcttagtacttttaacttcgtccatgaggagaactttgggtaagtagtgccagttggtttgaaagtcgtgttcagcgcgcaagagctgccgaccaacgaatgaatccgaagtggacaattcattggcaatgtgtttgaggctcactggttccgttaacttctctaaacattgtttccgggttgtatttgaaatcgtgcagtgcttcggcactgcactcgtctgcgccaggaagttggtatgacaagccttacagtgaaagtttcgccgattgaggcataggataaccgtgctgcccaatgttttagcgaatctaatggtggtcttccgccaaccatagccaatgatctggtgatcattaataaccccacaattgcggcaggccttgggagaatagttcagtgatccatttaatctgattaccccatcatcacctattttgccattctcaatttttaagtgttcatcatctattcctaacaacattttcgtagtatcatttgacatagggcatttccttctttctctaaaatcttcgtggttgttggttttgatgaacggacaggaaatgtccgctttttttattctaatgaaaaacaaaaaatctgtcatcagtaatagataaaaatctattaccaacaacagatattgtagagccctttttgtcatttcacttactcttctttttttgatacatcaacgtatttaaaatccggattaacggcataatccaaggcgtcgaacgcgctttgcatttccgtttcaatttgtttttgaaaatcatccgttaatttttgtttacggtcaattgtaatgggttctccaaaggcaatcgtgacccgttttcgagtaaaaagctgtttgaatgtcagtggtccttgataaacggccgggaccagcggcacacctgacagctgggcaataaaggcggcgccgctttttaattggctggaatgccgggtgcctgatgggaataagatcaaagacaaatctgattttctgagaattcggactggtttcttgatggcagaaggaccggggttatcacggtcaaccgaaaaagcattggcatgaaccaaaatccaacgcaaaattggatttttgaatagttcttttttcgccatgaaactaaactttttcggactgcccgccagtgcaaagtaaattggatcaaaccaggtgcgatgggggccaaccaggatatagttgccttttggcagtcgctccttgtgctcataacgggcattgccattgataataaacaccaggattcggacaaggactctcatgaatgaataaaacaattcatttccttctttcatatctgatagaattatattaacttaaaatagaagcgtttggcaaactaatttgtgaaggaacataacgatatgcaagtaaacttacatgaagacgaacgaattgaccaattatacagcaaaggcatccaaattattcaaagcaaagacgttttttcgttttcattggacgcggttttgctggccgactttgttcggaccacgcaacacagaaccaaacaaattgtcgacatgtgcgccggcaatggggcagtcggactgtttttaagtgaaaaaacggctgctcacatcaccatgatcgagattcagacaaggctggcggatatggcacatcggagcgttgaactcaatgacttgggtcagcagatatcagtggtcaacgacgacctcaaaaatgccgaccaatatattccaaaagattctgttgacgttgttgcctgcaatccgccgtatttcgtcaactacaagaccagcgaaaagaatccgaatcgatacttggccatcgcgcggcatgaaatcaccactaatttaaatgaaattgtcagctcagcagccggactgttgaaaatgaacgccaaacttttcatggtgtaccggcccgatcggctgacggatttgatcgtggcgttacgaagtcaccgattggagccaaaacggcttcaatttgtcagaccccgaatcaaagaggatgccaacatggtcctggttgaggcgattaaagacggcaagccaaacggtctcaaagtcaaccgcgatattattacttatgacggcgatgactatactgatgaagtaaagaagatgctttatggaacaaacagataagtattatatgtacgtgcttttatgtgccgatgacactttgtacaccggcttttccacgaatgttgaaagaagatttcaacagcatgtgaaaggcttgggtgccaaatacacccgctctcaccgaccaatcaaaattttgttcaagcaacaatttgacaccaaacacgctgccttgagcgctgaatacgcctttaaacaattgagtcgggctcaaaaaattgcccatttagctcaagcggggataaaattagagtgaattattgaacaaactacgaaaagtagtgaaaattattatcaaaaagtgttatactttaagtattctgttaggaggtaatattcgtgaaaattattgcatatggcattcgtgacgatgagaaaccttatttagacaagtggagtgaagaaaatcccgacgttgaagttgcttcaaccggtgaattacttgacgactcaactgttgaccaagcaaaaggtgctgatggtgtggttacataccaacaaaagccttacactgcatctgtattagataagctgggcagctttggtatcaagtacctttcacttcgtaacgtaggtgttgataatattgatgccgacgctgccaagcgtaacggtattcaagttaccaatgttcctgcatattctccagaagcaattgccgaatttactgtaactcagttaatgagattacttcgtcggaccaacacattcgaccgcaaacaagcaaatggtgaccttcgttgggcaccagatattgctgacgaattgaaccaaatgactgttggtgtctttgcaactggtcggattggccgggctgcaatgcgcatttacaaaggctttggtgccaaagtaattgcttatgatatttatcataatccagagcttgaaaaagaaggggtttatgttgatactcctgaagaactctatgctcaatcagatgttctttcattgcatgcgcctgcaaccaaggaaaacgaacatatgattaacgataagacaatcgctcaaatgaaagacggtgtcttcatccttaacccagctcgtggtgcccttgttgacactgatgctttaattcgcggccttgattcaggtaaaattggcggtgctgcccttgatacttatgaaaacgaagttggtattttcaataccgactttggcagctttgacaagatccctgacgaacgactcaagaacttgatgaaacgtgaaaacgttttggtaagtccacatattgccttctacacaaaacgggccgctcgtaacatggtctacttcgccatggacgcaaacaaatcattaattaatactggtaaatcagacaagttggttgaactttaatttaaccggcttgatatacaaaaaaggtttcagtcagaggatatctgattgaaacctttttaggttcttcgtcaactgttgttggtgaacaaaatattggagttctaatcacttggtgattagagctctttttgtatgaactcgaaaagcgaacagcactcttagccggaatctgaagaagtttcggtaaccaaatccagtgcgtttaatgactttaatcttgttgtttgaaccttctaagggcccgttggtgtaatggtgagtaaaggtattgccaatttcatcatgatgagtcgctagggtctggagggttgccaacatctcttccgagcagccctctaagtgatggaatacttgattatagttgggccaatcacggtttttgatggtttcacgtaaccgattcatcacgttgtaagtttgcttgagctcgggatcaatgtccaataaagcatcaaccacatcagtggcagtcgctggataagggaagtttgtccacttacggaaagcttcgtagttgaggtgattttccggcgttaataatagcttccaatagcgtttcaaggcgtgatactcgcgtgatgaggtcgccagggttttcatgaggcgcacccgcgtcttattaaaagctcgatttaaagcgttaaccaagtggaacggatcgatgacaacgatggcgttcggaaagatctgccccaccaatttgggataggtatagttcatatcggtgacaataattttcacattttctcgcgcagcctggtcgtaatgctggaaatacttttgaagctgatagatggtcctaaagggtaacaggtcgatcaattcgtgggtttccgcgtccataaattcaaagctcatcgcgtcggtggcgctcttagtgcttttaacttcgtccatgaggagaactttgggtaaatagtgccagttggtttcaaagtcccgttcagcgcgcaagagctgccgaccaacgaatgaatccgaagtggataactcatcggcaatgtgtttgagcgaaaccggttcggtcagtttttctaagcattgtttgcgggtcgtatttgaaatcgtgcagtgtttcggcaccgcattcgtctgcgccaggaagttggtatgacaagccttacagtgaaagtttcgccgattgaggcagaggataacggtgctgcccaaggttttagcgaatctaatggtggtcttccgccaaccatagccaatgatctgatggtcattaataaccccacagttgtggcaggccttgggggaatagttcagcgatccatttaatcggatcaccccatcatcacctattttgccattctcaattattaagtgttcatcatctattcctaacaacattttcgtagtatcatttgacatagggcatttcctttcttgacttaattctgtggtgggagcaagttaacggacgggagatgtccgcttttttactctaatgataaacaaaaaactgtcatcagtaatagacaaaaatctattaccaacaacagatattgtagaacccctttttattttaaattaggttagtctatttgagcagccaaatccatgagtaagtcttttaattcttccggtgttttgactgtctggtcgggaatgatttgaggatctgcgattggactttgatggctgttataccacacggtttcccagccggctttttttgcgggcacaatgtcttcaaaataggagctgccgatgtacatcatctcattgccccgtaaattgaattttcggttcatcaaggtaaaaataagcgggtccggttttttagccttcgcatcttctgaggtaatgatttgttcgcggctaaaccaatgatgaagtttgagcttcatgattttggcaagttgaacatcattgcttccgttggtgatgatgcctaacttgaacttggtggtcagggtattaaagacagtggtcaatccatcaaatagatgaatggagctgctggccgtttcaaaggcctccgaaaaggctttcgcagattcttgtgtcagtccgggcaaatcatactttttaaacgtgtggtgtaatgaatgatagttgatttcttcgtcagataatttcaaatcggagtctgagttggattctgcaattgccaactgttcctgctcattgtagttggcaaagatctgattcatctgttcttctggtaaatttagattaaatgtttcttcgaaagcctgtacaaatgcgggctttgtatcatacaaagtatcgtcgatatcgaaaacgatggctttaatcatgtataaattcctcctcgccacgaaatatcattctaacatgattcatcgaaatttaacaattttgacaaaaaattaatctgttccgggtatttgtgcttgcgcttccgcggcttttcttatatacttttaaaggtgttttaaatacacacctgacgtaatgggttgagagttgccagggatggttcttaattcaaatgatcgttggggaggaaaaaaacaatatggaggctacatcatggctgttatttctatgaaacaattactggaagccggagtacatttcggtcaccaaactcgtcgttggaatccaaagatgaaggactatatctttactgaacgtaatggtatttacatcattgacttacagaagactgttaagttaatcgatgttgcttacaacttcatgaaggacgaagctgccaagggcgccgttgtcttgtttgttggtactaagaagcaggctcaggattcaattgctgaagaagcaacccgtgccggtcaatactacgtcaacaatcgttggcttggtggtactttaaccaactgggaaaccattcaatcacgtgttaagcgtttgaaggacttgaagaagatgtcaactgacggtacttttgacattcttcctaagaaggaagtttctcttttaatcaagcaggaacagaaattggaacgattcttgggcggtattgaagacatgcctaagatcccagacgttatgtttatcgttgatcctcgtaaagagcaaattgctgttcacgaagcaatgaaattgaacattccgatcgtggcaatggttgataccaacactgacccagatcaaatcgacgttgttatcccatcaaacgatgatgctattcgtgccgttcgtttgatcacttcaaagatggctgacgcaatcattgaaggtcgccaaggcgaagatgacgttaacgaaaagacctttgaaggtaaagatggcgccaaagcagacaaaaaagaagattcaattgaagacattgcagacgccgtagaaggcagcaacgattctaacaaataaatattagcactcgggctgactctaccgctttggaccaatttggccttggtgtggagtcagtttttagtcacaattattagtcacaattaaagggaggccactaagatggcaaaaatttcagcatctcaagtaatggatttacgtaagaagaccggtgtcggtatgatggacgctaagaaggccttggttgcaactgaaggcgatttcgacaaagcaattgaagttttgcgcgaaaaaggagttgctaaagctgagaagaagagtgatcgcgttgccgccaatggtttggcaaccatcgcagttaagggtaataccgctgcaatcgttgaaatcaactccgaaaccgactttgttgcgtcaagtgatccattcaaagaattagttaaacgtgttagtgacgcaatcgttgccaacaagcctgcagacgttgatgcagcaatggcattgcagaccgacaaaggaactgttaaggacgatttaattgaaacgactcaagtgactggtgaaaaagttactttacgtcgttttgaagttgtcgaaaaaaatgatgacgaagtctttggttcatacctgcacaatggtggactgattggtgctttggttcaattaaaaggcgctgacgaagaaactgccaaggatgttgccatgcatgttgctgcaactaatccggaatatttgaatcaagcagaagttcctgctgaccgtttagctcatgagaaggaagttttgactcaagaagctttaaatgaaggcaagcctgaaaagatcgttgaaaaaatggttgaaggccgtctccacaaattcttggccgaaatttgcctggaagatcaagacttcgtcaaagacccagacgtcacggtttccaaatacgttgcttccaagggcggttcaattgttaaattcgttcgttacgaagtcggtgaaggcatcgaaaagaagacccaaagcttcgaagatgaagttcgcgatcaattgaagtaagctgagcgaatttagtttataaatcatttttccaaagatactgatgtaaccaaataataggggttaggacagagcattccgcttttcctaactctttttatttaccatcatgaataactcaaccctgttttctgaaacatctctgtgaactggctgagaatatttgataagaattcttgaatatccctgttttcttgttgattgcaacgttaatatgctaaaattggtagtaacgattaactatgggaggcacttggatgtctgaagtaaaatacaaccgaattattttaaaattaagtggagaagcattggccggagaccgcggctttggtattaatccacctgttatcaaaaacgtcgcccaagaaataaaagatatctttaacctgggtgtccagatcggaatcgttgttggcggcggcaatatgtggcgtggtgaagccggtgccgagatgggtatggaacgtgctcaagcagactatattggcatgcttggaacaacaatgaacgggctggccctccaagacaaccttgaacatttgggagttccgaccagggttcaaacttcaattgaaatgcggcagattgccgagccttatattcgtcggaaggctgttcgccatctggagaagggccgggtcgtgatttttgctgccggcaccggtaatccttatttttcaacggataccactgcagcgttgcgagctgccgaaattggtgctgacgccatcttgatggctaaaaacggtgtggatggcatttattcatccgatccccgaactcacaaagatgcagttaaatttgataccctttcatatatggatattttggaaaaaggccttaaagtgatggactctacggctagttctctgtcgatggataatcacattccattggtggtcttcaatttgaacaagcccggcaatatccgtaaggtcgtgactggtgataatatcggaacaactgtgaaggagaaataatttatggcagatgcacaatcagtattaactgaagcgaaagaaaaaatgaagaatacccgtgaggtattggaacatgatgtgggcagtatccgtgccggtcatgccaacgccagcttgttgagtggggtcatggtggattactatggtgcaccaacgcccttaaaccaaatcgcttcgattaccattccagaagcacgggtgattttgattaccccttacgataaaagtgccttggaaggcatcgaaaaaggcatttatgaagcagacttgggcatcagtccggctaatgatggaacggcaattcgattggctgttcccgcattaactgaagatcggcgtaaggaaattgcgaagcaggtcaaggcaaccggtgaaaagagtaaggttgccatcagaaatgtccgtcgagaggcaatggacacactcaagcgtagcaataagagtgaagatatcactgacgacgaactgcatcgctatgaagatcaagttcagaaattgactgatgatgcaattaaaggtgtcgacggaattgtcgccgacaaagaacaagaagtcatgaacggctagaaagaggtcaatacgatggcagataatcataataataacaataataattcagataacgatgaaattgcggttgtccctggaaccgatgaatttggcaagatgctctttaaactgaatacgcctgttactgaggacaatttgggcgtcttggattataacggcggccacttgcagccggttcaagatggtttatatgcaatgcctgcatatgtaaacgacgactttaacttattcttcatcgtttcgcaactggttgaaaacgactgggtaattgccttttctacagcaactattgaaaacgaccatgaaatcacggacctttcagaaccctatacaaccggcaaaggcttaaacctgctgggccaaaagagtccggaagatgccaataagctgttgaagtatttcaacacattggctgaggcaaaccgcggtgaatggcgaatggttgaacgtccagacggcgaatccgactaatacgaatagcattttatggctgggaaaaaactttggttttgttccagccatttggtgtttaacgatatgtcgcgaggatcccatgctgtttttgaatctgacagccaagccaacattcagtttttaaggagcgtaaaatgtttaagaacacacaagacaatcaacaagcaaccccgcaactcaaaacagacaacattccggcacacgttgccatcattatggacggtaacggtcgatgggcacagaaacgccatttaccaaggattgctggtcataaacgcgggatggaaaccgttaaaacgattaccaaagtcgctagtgatcttggtgttaaggttctgacgttatacgcgttttcgaccgaaaattggaaacggccccatgacgaggtcatttatttaatgggcttgccggttaagttcttcaacgatttcgtgccagacttggttaaaaataatgttcaagttcgtgtgatgggtatcaaggatcaattgcccgttcaaactcaaaaggcggttaatgacgctattaaagacaccgctgactgtactgggatgattctgaactttgccttgaattatggcagccgtttggatatcagaatggcagtccagcaaattggtcgtcaggttgccagcggtcaactggatccagagcagatcacggatcaaaccatcgatgcaaatttaatgaccggatttctcggcgatttagccgatcccgatctgctgatccgcaccagtggagaagagcgcatatccaatttcttgctgtggcagattgcttacagtgaacttgtttttactgatgttttgtggcctgattttgatcgaacggtttttgaacaaatgatcatggaatatcagcagcgtgaccgtcggtttggcggaattaaaactagtaaatagaggagaaacaaattgagacaacgtgtgataacagccgtagtagctttattaatctttattccaatcatcgtaatgggtggaatctgggttgatattgccgctttggcacttgggattgtagccatctctgaaatattggtgatgaagaagaaattattgatttcacctgaatcaattattgcttatttgggagtctgttcactcattctgccagatgcatggacgagctttttacccggacacatcagtcaaaactttgtcttctttttgtttgttttgatgctgcttctccaaacggttctgagtcgaaacctgttctcatttgatgatgccggagtaattgtcctgggcatgctgtatatcggtatgggatttcactacttcgttgccgcgcggggagttggactgacggtattgctatatgctttgtttatcgtttgggtaactgacagtggcgcgtacatttttggtagaatgtttggcaaacacaagttggcaccaagaattagccccaataaaacttgggagggttcaatcggcggttcacttgcagccaccattttatgtaccgcatttatcgcattttacccaattgccggacactcactcttgcaaatgttcatcttcacgattattctctctatagctggtcaatttggcgacctcattgaatctgcattgaagcgttattatggcgtcaaagactcggggaagattctgcctggacatggtggaatcttggaccgctttgatagcttactttttgttttaccaatgcttcatttgttagctgttatttagtttttaggaggaaagtgtcacttgataactacaattattgttttcattatcgtctttggtattcttgtgatctttcatgagtttggccattatattaccgctaaacgctcgggcattcttgtccgggagttttctgtcgggatggggccaaaagtattttattatcgaaaaaatagtacaacttttatcctaagattattgccgctgggtggttatgttcggatggccggtgaggccgatgacggtgaggacgaattaaaaccagggacaccggtgacccttcaattgaatgacagtggtgtggtaacatcaattaacaccagcaataaacactcgcttttccagggcattcccttaaccatcaccgataccaatcttgacgataatttgtatgtcaaaggatatgaaaatggtgatgagtcccaagttaagtcgtatccggttgatcatgacgcaactattatcgaaaaagacgggaccgagttacaaattgctcctcgagatgttcaatttcagtcggcatcgttgcctaatcgaatgctgacaaacgttgctggtgtgtttaataacttattacttgccatcttggtatatacaattttaggttttgttcaaggtggtgttgcatccaataccaataaagtcaatgtcatgcccactgattcagtcgcccggactgccggtgtcaaatccggtgatcgaatcgttgaggttgacggacacaagaccactgattggcaggatcttactgttcagatccgatcaaaagctgataagcaaatttctgtgaaggtccagcgggatggccaggataaagtcttaaccatgaaacccaaagcccagacttctggcggtcaaaagacaggcttcattggcattactcaaacaatggataccagctttaaagccaagatcctttcaggcttcacgacgacttggacagtcgccaagcagctgtttggcgccctgtggagcatggttagcggccactttagtctcaacgatttgggtgggccggtggcaatttttgcgacaacttcccaagcagccaagatgggactttcaggagtcttgaacttcctcgcatttctctcactcaacctggcaattatcaacctcattccaattcctggtttggacggtggtaaactgattttaaacattttggaagctatcagaagaaagccggtttctcaaacaacggaaactgttatcacattgatcggcttcgcgttcttgatgctgttgatgattctggttacttggaatgatattgagagatactttttacattaaacaagttaattttgaaggagaaccttataaatgaaacaatcacagatgctgatcccaacgttaaaagaaacccccaaaggcgccgaagctttaagtcatcaaatgttagttcgtggtggctatatccgccagatttctgcaggtatgtacgcatatttgccattggcctatcgcgttttaaacaaaattgaaaccatcattcgccaggaaatggaaaaaacatcagctcatgaaatgctgatgcccgacattttgccggctgatctttggaaagagtcagggcgctatgatacatatggcccagagctattcaaatttaaaaatcgccatgaaaccgattttattttgggaccaactcacgaagagacgtttacggcgttaattcgcgattccattaaatcatacaaacagctgccactggttctttatcaaattcaaaataagtaccgcgatgaaaatcgtccgcggtatggattactgcgaagccgtgaatttattatgaaggatgcttactcatttgccactaacgatgaggatctggataaaacgtacaatgcaatggagcaggcttatcgcaatatttttgatcgaattggtttgaagtacaaagtgatcatcggtgatggcggtgcaatggggggatctgattccaaagaattctctgctatggctgctgtcggcgaagatacaattgtttattccgatgaaagtgactattttgccaacttggaaatggccaaatcaaaagtcgacgaccagccttcaactgaacctgaagcagaccttaagaaggttgaaacgcccaacgcgaaaaccattgccgaggtggctgctttcctaaaagtctcagataagcaaaccatcaaatcgatgctgtacattgccgatgagaagccggtgatggtccttgtccgcggtgactacgatgtcaatgacgttaaattaaagaactatctgggggctgactttctggagttggccactgacaaacaagccaagacctatttgggggcagactttggttctttagggcccgttggcgttggtgaggatgttcgaatcgtcgctgatcaacgggttgccaacatgaagaatgccgttgttggtgccgatgaaaatggttaccattatgtcaatgccaattctgatcgtgatttccggattgatgacgtggacgattttgtagttgtcaaagaaggcgagaaaacacctgatggtaagggaacactgaaatttacccgtggcattgaaattggccatatcttcaagctgggtacgcgctattcgaagagtctcaaagccaacgtcttggatgaaaatgggcgcgctgtgccggtcatcatgggatcgtatggaattggtgtcagccgcctactttcagcaatttctgaacaaaatgccgatgaaaatgggttggtatggcccaaagcggttgccccatttgatgttcacgtcatccctattaatgccaaaaaagccgttcaaatggatttagctcatcaaattgaagcccaattaacagctgatcaattacaggttcttgtcgatgaccgcaaagaacgggccggggttaaatttgcagattctgacttgatgggaattccactgagagtaacaatcgggaaaaaggctgaagagggaattgttgaaatcaaaatccgaaaaactggcgaaaccgttgaggttaacgtcaccgaattgagtgacacaatcaaaaaaatgttgaagaatcttgactaatgatgtcgtaactaattaatatagacgtatgttttcgtcacttctaaactggttggaccaaaacttgggttttgtgtccagccagttgttgttaaaccgttatttttagaagaggtattgtgatgagtttggatcgaaatcaattatttgaaaagttgcttgaacagcttcaatggacacaggcaaatgaattgccttattttgaggatgctaaaattgatcgcctggaagttcataaacaaagccagcggtggcaatttgacatttcacttccacgaatcctgccatttgaggtttttaacgattttaatgccagactacagtctgcgtttaaagaaatcgctgatgtttcactgaatatttctgcaaaaaatgatacctttactgaacaactgcttcggcaatactggcaatgggtcgttccacatagtggggttacctcaccgttaatgaaggaattatgtgcagacaagtttccctccattgtcgattcgcgggtggagtttgtcgctgaaaatgacatcgtcaaggactttatgaccaacactgccttggggccaattgaagatgcctttcagcgggcaggctttcctgactttacaattcacacgatcgtcgatgaaagttcttctcagcaaaacattcaagccctcaagaagaaaaacgatgctgccaatgcggaattagtcaagaaggctaaccaagcgatcaaggagaatgctcaagctcatcccaggagtggtaacggtgggggcaagtcaaccattggtcggcgaatcaaagatgatttacccgtaatgaagatggaagaaattgtagaagaggaacgctctgtggttgtctctggctacattttcgataaagaaatccgggcattgcgttccggccgccagcttttgatgctgaagattactgactatacatcatccattcaagtaaagaaattttccaataaaggtgaagaagcgctctttgaaggcgttaacgaaggcgattgggtgaaggttcgtggtagcgtccaagaggataactactctcatgaactaactttgaatgcctatgatattaaccccattaagacggttagccgtcaagatactgcagatgatgataagaaacgggttgaactacacctgcacaccacaatgagccaaatggatgccactaataacattgctgactttgccaagcaggccaagcactttggccaaaaagccctggcaatcaccgatcatgcgggtgtccaaggatttccagacgcctttcatgccggccaaaaaaatgacatcaagatgctctatggtgttgaaattaacctggtcgatgacggcgttccgattacttacaatgataagcacgttccgttaaaggatgcgacttacgtcgtttttgatactgaaacaaccggcttatcagccatttatgaccgcgtcatcgagctttcagccgttaaaatgcagaacagtaacgtgattgatcaatttgaagaatttattgacccgggtttccatttgtcggaacgaacgacgaatctgacgtcaattaccgatgagatggttcacggctcaaagtctgaggaagaagtcttcaaacttttccgggaattttgtggcgatgcgattgtcgtcggccataacgtgacgtttgatatggggttcatgaacaccggctacgttcgtcatggcatgcatgagatgcaaaacccaatcatcgatactttgactttggccagatttttgtaccctaatttacggggttatcgactgaataccttggctaagaaatttgatgtcagtttggaacaccaccatcgagcaatctatgatgctgaaaccaccggccacttaaactatctatttttaaaggatgctgaagatcgatacggcattgtctatcacgatcagcttaatgatcacatgactgataacgatgcgtaccgccatgctcggccgtctcacgccattttattggccaaaacccaggccggcctcaaaaacatgtttaaaatcgtttccttgtcaaacgtcaagtacttctaccgggttccacgggtcccccggacgcaactggagaagtaccgggatggcttgattgtcggctctgcctgttcatcgggtgaggtctttacagccatgatgcaaaagggattggatgaggcccgccaaaaagctggcttttatgattatcttgaagttcagcccaaacgtgcttacgcgccactgattgaatccggtttgatcgccgatgatgagaatcttgagcaaatcttaaccaatatggtcaaacttggcgatgagctggacaagccggtcgtggcaaccggggacgttcactatctcaatccgcaagattacatttatcgaaaaatcttgattaattcgcaaggtggcgccaatcctctgaaccgtcaagaattacccgaccttcatttcctcacaactgatgaaatgttgagtgacttcaacttcttgggcccagaaaaggccgaagaaattgttgtggacaacaccaatcaaattgctgatgaaattgaggacgtccatccattgaaggataagttgtacaccccaagaatggaaggggccgaagacgagattaagtcacggacgatggacaccgcccacgcttggtatggtgatccactgcctaagattgtttctgatcgtttggataaagaattaaagagtatcatcggaaacgggttctcggtgatttacttgattgcccaacgactggttgccaaaagtaacaaggacggatacttggtaggttcccgtgggtcggttggttccagtttggttgcgaccctcaccggaattactgaggtcaatccactgccgccacattatcgttgtccgaactgtcaacacactgaattctttaccaagggtgaatacagctccgggtatgatttgccacacaaaaagtgtcccaagtgcggcaccatgatgattggtgacggccacaacattccgtttgaaaccttcttaggcttcaccggaaataaggttcctgatattgatttgaacttttctggtgattatcagccaattgcccataactacaccaaagttttgtttggcgaaaagaacgtttttcgtgccggaacgattggtaccgtggccgataagaccgcatatgggtacgttaaggcttacgaacgcgataagggtgaagtctaccgacaagccgaggaagatcgactggcaaagggcgcaaccggcgtcaaacggaccactggccaacatccggctggaatcatcgttgtcccggattacatggacatctatgatttcacgccgatccagtatccagccgacgatcaggatgccgcttggcaaacaacccacttcgatttccactcgattcatgataatattttgaaaattgatatcttgggtcatgatgatccaacgatgatccggatgctccaagatttgtcaggcatcgatccaaaaacgattccaatggatgatcccggtgtgatgtcgattttctccagcccaaaaatcttgggggttactgaagatcagattcaatctaagactggaacactgggagtcccggaatttggaactcgatttgtccgtggaatgcttgaacagacgcatccaagtaactattccgagttgcttcagatttccggtttgtcccatggaaccgatgtttggatgggtaacgccgatgagctgattaagaacggaacggcaaccattgccaacgtgattgggtgccgggataacatcatgaccgacttaatcaattggggactggactctgaattgtctttccagattatggaaagtgttcgtcatggtcgtggaattcctgacgactggcaagccgaaatgaagaaagccaagatacctgattggtatattcaatcgtgtctgaagattaagtatatgttcccccgcgcccatgcggctgcttacattttgatggcccttcggattgcctatttcaaagtctacttcccaatggtttactatgcttcatacttctccgttcgtgccgatgattttgatattgtctcgatgtgcagaggtaaagaagcggtcaaaaatgccatgcggatgattaatgataagggaatggaagcttcgaccaaagagaagaacctgctgacagttttggaactggccaatgagatgctcgaacgcgggtatcattttcaaatggtggatttggacaagtctgatgccagtcaatggctgatcgatggtgatacgttaattgcaccatttaattcagttccaggattgggattgaacgtggctaagcaaattgttgctgccagagaggacaagccgtttatttccaaagaagacttagccaaacgcggtaaagtttccaaaactttgattgacttcatgactgagaacaatgtgctggcgggattgccagatgaaaatcagttgaacttgtttgatttgatgtaaggcgagcataattgatttgcacatcggcgttaaaacgcgccagccttgtaatgaatcatcgaatatgttatagttaatttactaaataacttgtaagggagtgagcagagatgctcgctctttttaatggataatttttaggaggcctatttttgagcaatgttgttgaaacggtcaaacaagttgttgaaccaattctggaaaaacactcattttacttattcgatgttgagtttgtaaaagagaacaaaagctggtatttacgggtttatattgataaaaaaggcggcattaccattgatgactgcgtcttggtcagcgatgaattaagcgaaaagctggatgcaatggatcccgacccgatcccccaggcctatttcctggaagtttcgtctccgggtgctgagcgaccacttagaaacgacgccgaactcaaacaggcaattggcgagtatattcacgtttccctctatcaaaatcttaacggcaataaaacatttgaaggcatcctgaagtcgttggatgacgacaaactggtgcttcaaaatgataagtggggtaagcaggatacgttggaagtaccgcggaacttaattgccaaagcacggcttgcaattcaattttagttaaaggagacacaataatgagtaaagaacttttaggagcgctgtctgctctggaagaagaaaagggcatcaaaaaagaggttgtcattgaagccttggaagccgcgttggtttctgcatacaaacgaaactacggtcaggcccaaaacgttgaagtgtcattcgacgacaaaaaaggcgagatgcacgtttacgccgttaaaacggtggtcgacgatgttgttgatgaccagcttcaggtatctcttgatgaggcccttgaaattaacaaaggttacgaactgggagacgaaatcaaatttgaagtgacccccaagaactttggccgaattgctgctcaaactgctaagcaggtaatcatgcagcgggttcgggaagctgaacgggaaaacgtttttgatgaatattccaagtatgaagatgaattggtgaccggaactgtcgagcgtcaagacacccgatttgtttacgttaatctggggaaagttgaagccgttatgggttcaaaagaccagatgcccaacgaagtctatcgtccacaggatcgtatcaaggtctatgtcaccaaagttgagaatgcgaccaagggccctcaggtgtttgtcagccgaacggctacagggatgctcaaacgtttatttgaacaagaagttcccgagatttatgatggaactgtggaaattgtctcaattgccagagaggccggcgaccgggccaaagttgccgttcgctcaaacaactccgacattgacccggttggaaccgccgttggcccaagaggtcaacgggttcaaaccattgttaacgaactccacggcgaaaacatggatatcgttgaatgggatgaagacgatgcatcttacatcgccaactccttgaatcccgcagaggtcattgatgttatctttgatgatgacaacgagcgggcctgcacggtcattgtgcctgactaccagttgtcattagcaattggtaagaaggggcaaaatgctcggttggcagctaagctaacgggcttcaagattgacatcaaatcagaaactgaagccaaggaaattcttgccgacaaagccgctgccgctagcgatgatacagaagctgatgaggcttccgaccaaggcgatcaaacagaggattcaactgaggatgccccgacagacggtgcggatgttaataccaatcccgatgagtcgaatgaggacactcaagactaatttttaggaggcgattttttgaaaaaacgaaaaattccaatgcgtaaagatatcgttactggtgaaatggcgccgaaaaaggaattagtcagaattgtccgtgactcagacggccacgtttcaatcgatgagactggaaagaaatccggccgtggtgcctacatctcaattaacgttgagattgcccgcaaaactaaagcggaacacacttttgaaaaagtcttttcaacaactttggatgacaacttttatgacgatctaattgcctatgttgaccataagcaagcccgaaaagagttgtttgaagatggacaatgatcaggcaattttgaattttttaggtctggcacggcgggcaagcaaaattgtctccggtcaagatatgcttttgtctcaaatccgcagcggcaagatttttttcttgtttatcgcagaagacaccggcaaggcaactcaaaagaagtttaatgataagtcaaattactatcatatacccgtgaataacagttacactaaagcagtgcttagtgaagcaattggaatgaaacgaaccattattggcatttccgatcggggtatggcaaaaaaattggttgaattaaccgataacaataaaggagagtgattatatggggaaaaagcgaatttacgaattagctaaagaactgaatgtctccagtaagcaaatcgttgaccgtggtaataaacagggcttcgatatcaaaaatcacatgtcaaccgttgacgctaaccaagagcgtcaaattcgggcgatgtttagtaaaggcggcaatcaatcgactggaaacagtcaatcaagccataagagcagcaataacaatgttcattcagcaagctcaaagccaaaagaacatgccactgctcatgcacaaagtcgaccggctgctcaccatgacagcaacgggtcccatccggtgagccgaaacacacagcaggctaaccgaaatgcagagagcaaccgtagtaacaacggccactcaagtgttgctcgcaacacaaataatactgctcaaagaaatcattccaacaataataaccattcgaatagtcaaaatcattccaacaattcgaaccagtccaataatcaccggaccaaccagaataatgatcgacgcaatcaccaagcttcaaacaattcatccaatacgtcgacccgtaatacaaacagtcattcaactggcagcaatacaactgcaagcaatcataccagttcgaataataacagtaatacaaaccgtagttccaacaatttctcaaatcacaataccggcagtggtcgttttggcggcagcttgaaccggaataataatcgtggcggctcccgcaaagccaagaagaagcgcaacaagaaacaacgtaagcaaaagaatcaacgattgcgtgaagttgaacaccatggtgcaccggaacgaaagaatcgtccattaccaaaggtgcttgaatatcaagatggtatgaacgcccaggaattgggtaaattgttgcatcgtgagccagcagaaattgttaagaagctatttatgctcggcgtcatggtgaaccaaaaccaatcacttgataaggatacgattgagattttggcagccgactatggtattgaagcaaaagaaaaagtccacgaagatttgtccgatttggataagatctttgaaaaagaaatggagaataccgatcacttggtatcccgaccaccagttgtgacgatcatgggacacgttgaccatggtaaaaccactttgctggatcacttgcggcattcacacattactgctggtgaagcagggggaattactcaagcaatcggtgcttatcaagttcgtcacggtgacaacctgatcactttcttggatactcctggacatgccgcttttactgaaatgcgtgctcgtggtgccaatattaccgatatcacgattttggtggttgctgccgacgatggcgtaatgcctcaaactattgaggctatcaaccatgccaaagctgccaagacgccaatcattgtggctatcaacaagatcgataaaccggatgccaatccacaacatgttaccgatcaattgatgcagtatggtctggttcctgaaaaacttggtggtgataccatcttcgttgatatttcagccaaatttggtaagaatattgacgaattgcttgatatgatcatcttggaagcagaagtgatggaattgaaggctgatccggatcaacccgctgccggatcggtaattgaagctcgtctggatcaaggtaaggggccggtttccactttactggttcaacaaggcactttacacgtcggtgacccaatcgttgttggtcatacattcggccgagtgcggaccatgacgaacgaacgtggccgcgatgttaagaaagcgacgccatcaagcccagtatcaatcactggtttgaatgaagtaccagaagccggcgatcgttacgtcgtctttgatgatgaaaagaccgctcgtgccgttggtgaagaacgtgccaaggaagctcaagttgaggaacgacgaaagaccacccgggttaccttggacagcttgtttgattcgcttaaagaaggcgaaatgaaggaagttgacatcgtaatcaaagctgacgtgcaaggctcagttgaggctttggctaacagtctgcaaaagattgaagttgaaggcgtcaaggtcaacatcattcattccggagttggtgcgattaatgaaagtgatgttgccttggccgaagccagcaacgccattatcattggtttcaacgttcgaccgacaccacaagccaagtcacaggctgacagcgaccacgttgacattcgtcttcaccaagttatttacaacgccattgatgaagttgaatcagcaatgaaggggatgcttgctccgacctacactgaacaagttactggtgaggttgaagtgcgtgacatcttcaaggcttctaaagtcggaacgattgctggtggtatggtggttgacggtgtcgttcagaagaatagtaaagttcgtttgattcgtgacggagtcgttgtctataccggcgaattaaacagtttgaaacgcttcaaagatgacgtcaatgaagttaaacaaggctttgaattaggtttaactatcaaagattataacgatatcaaagtcggcgatgtgattgaggcatatgtcatgaaacaagtgcctgtcaagtaatttggaggtgttttgatggctcattatcgggttggccgattagaacaggaaattcaaaaagaagttaacgacattctgttaaagcgggtccgcgatcctcgagttcagggcgtcactttaactggtgtcgaagtcacaggtgatctccagcaggcgaccatttattacagtattttgtccgataaaaaagaggacgaagaaacaactgcaaagggattggaaaaagccagcggactaatccgcggcgaacttggtcatcggttaagcatttataaaacaccggaaatcaagttcgagctggacacatcagttcagtatggtgacaagattgaccgattaattaataaattaaatcaagatggtgaataatcatctcaactgcccacgcctgaatggctgggcagtttttttgtgatataattttcttacatgaaaaaattaggagaattcgaatggatggcgtaattgcactatataaagaacgtggcatgacaagtcacgactgcatcagcaagttaagaaaaattttgcacaccaaaaaagttggccataccggcaccttggatccaaatgtcgatggggtgctgccaatttgtatcggccaggcgaccaagatcagtgaactgttaatgcagtccggaaaagtatatcgcggtgcgattaccctgggagttgcttatgatagtgaggatctggacggtcacttgattgaacaggtgccggttaaaacgccgctgacggatgaacagattaacgccgctctggctcaattgaccggtgacattctgcagacgccgccgatgtattcggccgtcaaagtcaatggccacaagctctatgaatatgcgcgcaaggggatcaccattgaccgggatccacgtccgattcatattgattattttaagcaaattaagccggcaacgtatgatgacgctgcccacacgcagacaatctattttgaagtcggctgttcaaaggggacttacgttagaacgctggcagtagattttggaaaacgggttggcttgccgtctgtcatgtctgatctgaccagaattaaaagcggtggttttgatatttcacagacatccactttggctcaagtcaaagaagccgttgctgcggaagacctgagtatcgtccttcatccgttatctgaagcactggcggaatatcccggttatcaattggacgacagccgctggtcaatcgtttctcatggtggcttcttggaccaatcaatcagtcccacccacgcgccggtggttcgattagattatcaacaacaggtgaaagcgttataccgattggatgaacaaatcggtcaatacagaccgtttagaatgtttttagcttaatgaaggtggtttttaacaatgcaaatttcaagattacactatccgttgtctgatgattttaaggtcgatggcccgactgtcgttgcaatgggattttttgatggctttcataaaggtcaccaagcagttttacaacgggcaaaaaccgaggctgaaaagcgcggtgccaagttggcggtgttgacatacgatcatcatccggcaattgtctaccgaaaaatgtcgccccatgaacagcgatatttgacgctgaatgattataaaatgcagctgctaagagattttggtgttgaccaagtctttctggtgaattattcgtatgattttcaaagtcaaactccggaagaatttatcaacaactttctcaagcggttcaatgcagtggcagtcgtggctggttttgatcacacctatggtgataaaaaagtggccacgatggccaatttccccaaatttgttaaaggggcttttgacgtcatcacagtgccgtctgtcgacattaatgataaaaaggtcagttcgacccggattcggattgaattggattcaggtgacgttgatagtgttaccaaattgttggggcgcccatttcaaacccgtggcgtcattgtccacggcgaggagcgggggcgactgttgggctatccaactgccaacgttgaacactcagaatatcaatggctgccaacgattggaatctacgtggttaccgtcgaaattgccgacaaaaagtacttgggaatggcttcaatcggcaagaatgtgaccttctcggatgttcatccgatgacggtggaaatcaatttgatggattttgaccgcaacatctatggtgaagtcgtcaacgtgaactggctttcatacttaagagctgagatcaaatttcagactcctgaagatttaattgatcagttggataaagacaaagttgcgacccgtgagtacttagagcagcatcctgagatcttgaattagcactattagcactctacacaaaataatgctaaaataaggctatattcccttgacttataacagacggtttgttaaattataaatgtgccttagcactcggttatattgagtgctaaaaagaggtgatttgggtgctaacggataggcaaaaagatattcttcaaataatcattcgtgattacacaagaacgggaatgccagttggttccaaggcattggctgaggagtttccgacccacgttagttccgcgacggtcagaaatgatatggctgcacttgaatcaaagggcttaattacgaagactcacttttcttccggacgggttccatcgatcgaaggttatcgttactatgttgataacctcgttcagccggacccgctggacgaaggtgcggaagacttaatcaaaacttcttttaacagtgagttcaatcggattgacgagattgtccaggagtcagccaaagtattgtcagatttgacaaattacatggcgctgacttttaatccagagtctggcgataacttgaaacttggcggtttccggttggtcaagttggatgatcgtcaggtaatggccatcatcgttaccaacacaggtcacgtcattgataagattttcaggctggccaacgtctcgtccgagcaacttgaaaccattgtgaatatcattaacagcgaactggtcggcaagccgctcaaggatgtcatggacaagttaaaatttgatattccaatgttgatgaccaaatatattcagacccccgaaggcttcttgaagatcttcggggacatgctggacgaagcgggccgagataaagttcacgttgatggtgaactgaatctattgaagtttgcggaacggcaaaatgttgaccggcttaagccactctacaatttactgggcaccgaggactcggtttcaaagattattgatcccaactctaaagatgttcaggtcagaattggcggcgagctgcgcaacgacctgttaaaagattatagtattatcacaggaacttatgatttgaaagagtatggtcatggcgtgattgcagtcattggaccaaccagaatgccttactcaaaggtcatcggaattgttggtgctttgcgggaagaattgaccaagaagttacttggctactacgatgacgataatcaataatttaaggaggcgattgtttggcagaaaacaaagatgattcggttaagaagaatccaagtgggccaacacaggaccaatcaactcaaccagccaaggcagccaaaaaggcagctaagccggaaaaaaaggctgatcaggccaaaagcccagacgcaaatgatattaaaaagttgaaacaaacggtagtcgatttacaaaagaaacttgatgcaatggaagataagttccttcgtgcggaagccgatatgcgaaatattgaaacccatgccaagaaggaacaggctgatttaatcaagtatgacggccagcagctggcccatgatatcctgcccattgttgataacctgcagcgagcacttaaagttgatgtcactaacgaaagcggcaagcaacttaagcagggggtttcaatggtttacgagcatttcaccaaggctttgtctgataatggcgttgaggtgattgatgcgttgaacaaaccatttgatcccaaattcgatcaggctgttcaaacggcgccggcagatgatgatcatccagctgacacggttgttcaggtcctccaagacggatatcgtttgaaggaccgagtgcttcgaccagcgatggttgttgtagcaaaataaaactttaaaagaaaaagaggattatttatggcaagtaataaaattattggtattgatttaggaactactaactctgccgttgctgttcttgaaggcagcgcgcctaaaattattccaaacccggaaggtgcccgtacgacaccatcagttgttgcatttaaagatggtcagccacaagttggtgaagttgccaagcgacaagaaatcaccaaccctaacacggttcgctcaatcaagagtcacatgggtgaacaaggttacactgttgacattgaaggcaagaaatacacccctcaacaaatttctgcgatgattttacagtacatcaaggactttgctgaagattatttaggtgacaaggttgaaaatgccgttatcactgttcctgcctacttcaatgatgcacagcgtcaagcgactaaagatgctggtaaaattgccggtttaaacgttaagcgaatcatcaacgaaccaactgccgctgcattggcatatggtttggacaaacaggagaaagatgaaaagattctggtttacgatttaggtggtgggacgtttgatgtttccatccttgaattgggtgacggtgtcttccaagttctctcaaccaatggtgatacacatcttggtggtgatgactttgaccaacgaattattgactggttggttgacggtttcaagaaggataatggcgttgacttatccaaagataagatggctttgcaacgtttgaaggatgccgctgaaaaggccaagaaggatctctctggtgttactgaatcagaaatcagtttgccatttatttcggccggtgacaacggtccattgcatctgcaaacaaccttgactcgtgccaagtttaacgaattgactgccgacttggttgccaagaccaaggtcccatttgataatgccttgaaagatgccaaattaagtacttcagacattgatcaagtgatcttaaacggtggttcaactcgaattcctgccgtccaagaagccgtcaaatcatggactggtaaagattcaaaccactcaatcaaccctgatgaagccgttgctttgggtgccgctgttcaaggtggtgtgatcaccggtgatgttaaagacgttgtcttgcttgatgttaccccattgtcattgggtattgaaaccatgggtggtgtcttcaccaagctgatcgatcgcaacacgaccattcctaccagcaagtcacaagtcttctcaacggctgctgataaccaacctgccgtagacattcacgttcttcaaggtgaacgtccaatggctgctgacgacaagacgttgggtcaattccagttgactgacattccggctgctcctcgtggggttcctcaaatcgaagttaagtttgatattgacaagaacggcattgtgaacgtttctgccaaggataagggaaccggtaaagagcagaagatcaccatcaaagattcatcaggcctttccgatgaagagattcaaaagatgatgaaggaagctaaagaaaacgaagaggctgataagcaacgtaaggaatcagctgatttgaacaacgaagtcgaccaattgatcttccagactgacaagactctcaaagacgtcaagggtaaggtttccgatgacgaaatcaagaaggctgaagatgcacgtgatgccctcaagaaagctaaggaagacaataacgttgacgaaatgaagtctaagaaggacgatttgaacaagattgttcaagatttggctgtcaagctgtatcaacaacaggctcctaaagacggcggtgctgctgccggcgaaggtgccaagggtggttcaactgatgacaaatccgacggcaaaggtgacgacggcaccgttgacggcgacttccacgaagttcacgatgatgataaaaagtaatttataatcagatattgtaatgagaagtcaaggccggctggctttggctttttgttaaaatatggtatattatcatggttaatgaattgaatgaggatgggagtttctaatggcagaaaaagattattatgatattcttggagtttccaaggacgccagcgatgacgaaatcaaacacgcctatcgtaagctttctaaaaagtggcatccagatatcaataaagcgccggatgctgaagcaaaatttaaggaaatcaatgaagcatatgagacattgagtgacccacaaaagcgcgccaactatgaccaatacggttcagctgatggtgccggtgccggctttggcggcggtagccaaggcgggggctttggtaactttggcggtagcgctggtggatttggttttgatgacattttcagtcagttctttggtggcggccaacagcgggcagatccgtccgcaccccaacagggccgtgatcttcaataccagatgacccttgaatttgaggaagccattttcggtaagaagaccgtgatcaagtacaaccgtgaagcccagtgtaagacttgtggcgggacgggtgccaagcctggtacttcaccagtcacttgttccaactgtggcggccgtggttacgttaccactgagaccaacaccccacttggcagaatgcaatcccgtcaagtttgcccggtttgtcatgggactggtaaagaaatcaaggaaaagtgcccaacctgtggcggtagtggtaaaactgatgagcgtcacgaacttgaagtcaacgtaccagccggaattgatgacggtcagcaaatgcgtcttcaaggccaaggtgaagccggggacaatggtggtccttacggtgacttatacattgtcttccgagtcaaacccagcaaagactttacgcgtgatgggtcaacaatctacgttgaccagcccatcacttttgccagagcagcacttggtggcaagatcaaagtcaaaacggttcatggcgatgttgagttaaaggtaccagccggaacccagaccgggacaactttccgtctcaaaggtaagggtgcgcctcgccttcgtggtaacggtaatggcgacgagcgggtgaccgttaatgtggttacacccaagtcgcttaataagaatcaaaagattgccttggaagcattcgccaaggccagtggtgacaacattgctggcaagggcggtagtaatttttttgacaagatgaaagatgcttttgataaataacatgatcatgtggaggggtcagccggctgttttgccgttgcttgacctctttttatgtcaaggcaaccctgctggttccgtttaactttggataaactggaatggctggtataattattatcagtaaacaaatgaaagtgagaatacaacatggatttagataaaatgaagaatcaccaaaaatatattcgaaacttttccatcgttgctcacatcgaccatgggaaatcgaccttagccgatcgaattctggaaatgacggataccgttgccaagcgggatatgaaagatcaattactggataacatggacctcgaacgtgagcggggcattacgatcaaattaaacgccgtggaattgacgtatcatgccaaagacggccacgactatgagtttcatttgattgataccccaggacacgttgacttctcctatgaagtttctcgaagtctggctgcctgtgagggtgccgtcctggttgtcgatgcagcacagggagtcgaagctcagacactggcgaacgtttatctggcgattgatgacaatttggaaattgtgccagtcattaataagattgatttgccctcggctgaaccggaaaaggtccgagaagaaatcgaaaacgtgattggcttggatgcctctgatgccgttctggccagcgcaaaaaaggggatcggtgtaccagaattgttggaacaaattgtccacaaaattcccgcgcccgacggagacgttgaaggacccctaaaggccctggtctttgactcggtttatgatgattaccgtggagtcgttttaagtgtccgtttattcgaaggcactgttaaacccggtgacaagatcaaaatgatgaacagcggcagtgaatatgaagtcactgaagtgggggttaactcgcctaaacctgttaaacgcgactatctgatgtctggagacgttggttacatcaccgccagcatcaaagatattacccaaacccgagttggtgataccgtcaccaatgcccttgatcctgcagatgaagcactcccgggttatcgggaaatgcacccgatggtttatgccggactttatccaactgacaatgccaagtttgacgatttacgtgaagcattggaaaaattgaagttgaatgatgcagcactggagtttgaaccggaaatttccaaggcgctgggatttggttttcgttgcggattcttgggcctgctgcatatggacgtggttcaggaacgtttggaacgggaatttaatctggagctgatcaccacggcaccatcagtaacctatgaggtcaagctaacggatggcgagtccaaagaagttgaaaatccatctgaaatgccggatgtttctgctatcaagcaaatttctgagccatacgtcaaagcaaccattatggtacccaatgattatgtcggcccagttatggaactttgtcaaagacgacggggtgaatttgacacaatggaataccttgatgagtatcgggtcaacgtgatttatcacatgcctttatccgaaattatctttgatttctttgacaaattaaaatccagcaccaaaggctatgcatcccttgactacgagttggaggactacaaacccagcgacctggtcaaaattgatattttgctgaatggtgaaaaggtggatgctttaagcttcatttctcaccgtcaatttgccgcaccaagagctcgggacatcgttggtaaactcaagaatatcattccccgacagaactttgaaattcccgtccaagcagccattggcgccaaaattattgccagaaccaatattaaggcctatcgcaaggatgtgaccgccaagttatatggtggtgatcgaacccggcggatgaaactcttggagaagcaaaaggttggtaaaaagcggatgaaggctgttggaaaagtggatattcctcaggaggcctttatggctgttttgcagactgatgaggaagaaaaaggcgacaaataggtacttttactggaccattggtcttaacgacaattatttattcaggtcaataacccttgcccatgcccgttacctgaggaaccgtagtacagctagaaatttcataaaaaagcaagcaacagccagtgatattgaggaaatcaaatcactgattcgtttcaggcaggcgatgcttgttagcaacgacacttcgtttgagtaaacgggagcgttggttgatggttgcgacactaaattaagataattttggtatttaaaagacgtcttactaggcgccttttctattgagacagcctttatgacgtcaaaaaagaccgcagcgaaataactcgttgcgatcagatgtcttcaaactattttgttggactcgttaattgtgtactatcagataacgcgcggctgtaaatggtctctaagtgttccagctccagcttgttggcgataacatcgttaaataactgttcaatggccgctgtcatagctttttcgtccggcagggcatttgtggcctcagccttggcctgttgcatttggtataactcctgcaggagattaatgagtcgatgacgaaaatgggataactgtaccgaatgaggcaggtcatcattttcgtgtttgacatggtaatcaaaataccgttccagtttttcaaccgtccccagtgataagttatccaccagtcgcgtgtgatttctgagtcggatgataattgatgagttcaccccggtcaacttctggatctgataggcactgtcttcactgtcgaggacagcttgaaccttttgtcttgcatccatattcattcccccggaaatttagaatttgatgataaaaaggttgcttcggcgtatgtatatcttgtcacatttaccatatgacaagtgacatataattgtcaaatttttcgctatctcaatagcggtgtgtctgctaaccaatccgcaattcggtgactaatttggtatcgataaccggcttgccgtcctctccctggtggtgaacgacgcgacccaacatgccattatcgatgacgtattgatcaaagaactgcttggttgggacctgcaggaggcttcggtcatgcgactgttcaaaagccacttgatccaagaccaagtcttttggagtggcagaaaaaatattataaattgctttaagggcgacttcacctgatttcaaaatggtggtatccaaataacttcttaggaataactgatggccctcaaaaaccgtatcacttgaatgtgattccaacactgcccggtagcgaatctcaatcgtgtcgggtcgaatcttattgataaatcgaatgcggaataattccattattctcagctcctttcctacatcatatgctaaacttgttaaggagtgcaactttgattcattatgagaaaatgtttgcgtttcttctcacattcaattattatatatattaattgtttttttattcgattcgaaaaattaaaatttaataagctgggaggtgttaatgattctaagtcgaacaaaacaatatttaagaaaaaacggttacttctataaaaaagaatatattcggcccttactgacaccggataatatttatattttcagatttggccgcgaccgcttggataaccggcttattattcgctacagtcataagtggactggcagacagcgaatcaacgaaattgatttacggctgcataagcaaaagcatccccggattttcgagaacgaatccgaactattgaactacttggaaggacacctattgaagcacgaggcaaaggtccgtgcgcgtgagaaagaaaaacaacatgaaatatcagatggtgcatctaagtgatatggattcgaaatcaaagctggtttttgcctcattgtggggtgaagccagctttcattttagaatcaaccgacaaaggagaattccatggactggacagaattatcaattatgacgacaagtgaagcggttgaggccgttgccaacattttgatggcatacggggcgaccggggtttcaatcgaagatgccaaagattttgagaaattaaaacccggccgctacggagatcatggtgaaattgtcgatcctaaagacctgactcacgttaggcagggggcgattgtatccgcttattatcccaacaatcagcatattgatgcccaagcagaccaaattgccaccaaggtccgaggtttggcgaagtttgatttgaatcccggaccagcagaagttcacctgacgccagtcgtgaatcaagattggcaaactgcctgggagaagtattaccatccagtatcaatttcgcgattcatcaccattgttcccagttgggaagactatcagccaaaatccgctcaggaaaaaattgtccgcttggatcctggaatggcctttggaactggaacccatccaactacccgactatcacttcaggctttggaaatggtcatgcagggcggcgaatcaattctggatgtcggcactggttccggtgttttaagcatcgccgccaagttgatgggcgcgggggaaatccacgcgttcgacgttgacgacatcgctgttgaatctgcagaaaagaacattcaactcaatccaggtgctaaaggaatccacgtcgcggcaaacgacctgctggccggaattcacactcaagttgatatcgtggttgccaacattttggccgaaattatcgtgccgctggttccccaagcatgggataatctcgttcctggtggctttttcctcacatccgggattatcaaggacaaatttgcaaccgttgaaaatgcgatgacctcacaagaatttcaaatcattgaaaccttgagaatgaaagattggtatggggtcatcgcccaaaagccaaaggatgaggacaaataatgcaacactattttgtaagtgaacatttaactgtgggacagtcgattgaacttcccaaaacaatttctcatcatttatgcagagttttgcgtgccgaagttggtgaccggtttgaactggttggcgatgaccaccaggtgtacgaggctgaaattggtcgactggagggaaaccaagtcgccgccaatattatcaagccacttgatcacaacgttgaattgccggtcgatgtcacgattgtcagtggtctgtccaagggcaacaagcccgaatggattgttcaaaaggctactgaacttggtgtggctcacgtgattttcctgccgatggactggtcgattgttaaatgggatcaaaaagcaactaaaaaaattacccggctgaatgaagttgcgttgagcgctgctgagcagtctcatcgaaacgtcgtgccaacagtggcttatttaagcggattagatgctttattccaattagattttgatacccaattggtcgcttatgaggagtccgccaagcaaggcgaggaaaccaatttggtgaaggccgtcaggcaaactgcttcaggcggcaccatggcggctgtcttcggtccggaaggcggcgttagtccggctgaagttacccaattagtcgatcacgactttgtgttagctggtcttgggccacggattttgcggactgaaacagccccactgtactttctcagtgccgtttcaacgctgaccgaactgatttagtttgctgaataactttgacaacaatgatattattatgataaagatgatttgatgatgcctttgggcaaatgagagaagagttgatacaatggcgactaaaatttggacaccggacgatgtcattaataaggtttctgagtatatgaacaaggaacatgttgatgagattcgaaaagcttaccaatttgcaaaaattgctcaccagtaccaaaaacggcagtctggtgagccctatattacccatccgactcaggtggctggtattttagctgacctgcatatggatcctgagaccgtctcagccggttttcttcatgatgtagtcgaagataccggggctaccttaggcgacatccaagagctgtttggccacgatatcgccttgattgtcgacggggttaccaaactgtccaagattaaatataaatccagcgaagaacgattggctgagaaccaccgtaagcttttgctggcaatgtgtaaagacatcagagtgatgattgtcaagctggctgatcgcctgcacaacatgcggacattaaaatcactgcggcctgacaagcagcggcggattgccagtgaaaccttggagatttacgccccgattgccgatcgattaggtattggaaccatcaaatgggaactggaagacatttcacttcggtatctcaatccccagcaatactaccgcattgtgcacttgatgaattcacgtcgtgatcaacgggtggattatattgaaaaagccatcaaagaggtcaaaaaggcgatttctgcattgggcgtcaaggctgagatttatggccgacccaagcacatctattccgtttaccgaaaaatggttgaaaagcacaaacaatttagtcaaatttatgacctgttggccattcgggtaattgttgattcaattaaagactgttacgccgttttgggcgccatccattcagagtggaaacccatgcctggccggtttaaagactatattgcaatgcccaaagccaacatgtatcaatcgctgcatacgaccgttattggcccggaaggcaagcctttggaagtccagattcgaaccgaagagatgcaccgcgtggctgaatttggtattgctgctcactgggcctacaaagagggaatcacaaacggggtcaaaacctcgcaggataacaataaactcaactggtttaagcaaattatcgaactccaggaagataccgacgatgccgccgatttcatggatagtgtcaaaggtgaattgtttggcgaccacgtctatgtctttacccctaagggcgacgtttatgagctgccaaaaggagccggtccgcttgatatggcctacatgattcataccgaggttggtaatcacaccactggtgcccgggtcaacggcaagattgtccctctggatcaccaagttaaaaatggtgacattgtcgatattattactgccactggttcagccggcccgagtcgtgattggctgaagctggttcacaccaggcgggcacgaaataagattaaacagtacttcagacaagaagaccgtgagaaaaacattgaggacggtaagaacctgatttccagaagactacgggaagccgggtttgagcccaaccggatcatggtaccggataaattgaccaaggcagccgttaacatgcattaccaacacgctgatgatttgttggctgcggtcggctttggggatttgcagccgaccggggtggttaaccgattgacagaggatgcccgggcccaactcaaaaaagagcgtcaggaccaagctgaacgagaagttttggaaggccatcagaccatttctgaagattccgacagcgctaagaagcagaaaaaacgcaagtcctcaaatggtatcgtgatcgaaggcgtcgataatctcctagtgcgattgagtcactgctgtaccccggttcccggcgatgaaattgtcggttacatcaccaagggacgcggcgtgtcaatccaccgggttgactgcccgaacattaaaactgcggaagaaaacggtgagcggctgattgaggtcgcctgggctgacaatcctgaggaacggacgatttatgatgccagtttggccgtccaaggatataatcgggccggcctgctgacgaatgtcttgaccgccgttaatagtgtcacgaagaacgtttcgtcagttaatggtcaggtcgataataataagatggccaccatctccctttcagttggcgtccgcaatttggagcagctggagcggttgattggggcaattaagaacgttcacgatgtttatttagttgaacgaaaattcagataggagttttgctggatgaaagtggttttgcaacgagtcaaggaagcgtcggtcagtattgacggtcagattcatggcaaaattggcaggggattcgttctgctggttggtgtcagcgatgccgacggtgaggcagaagttgactatttaacccataagattagtaaactgcgggtatttgaagatgatgccggtaaactcaatttggacatcaatgccgtgaatggcgcaattttgtcgatttcgcagttcaccttatatgcagataccaaaaaggggaatcgccccagctttaccaaggcaggcgaaccgcaagacgctgatcgggtgtatgagcaactcaatgaacgtctgcggcagaccggtttggaagttcaaacgggcgtttttggagccgatatgctggtgaatattcaaaatgatggtccagtgacgattatctttgatacggataacaaataaaaaatgatcagataaaaataaagtcgaatcgtgtggttcggcttttttaaggagtaacgaaatgattaatcaattattttgggattttgacggcacgttgttcgatacctatccaaaaatggtttccgcgtttgtccaagcattgggtgatttaggaattgacgatgttgaaatcgatcaagaccagatttatgtcaccatgcgccaacacgacgttgggacagccattcgaaagttctcggccttttatgggattgatgaaaaacagcttcgaaaattgaatcgcacccatcaaaccaaattggtcgaagatgccctgccgtttcccagtgttaaagaggttttggaattggctaaatcaatgaagggacgcaactttttgctgacacacagggatgaccaggctaaaagcatgctgagaaagtttgatctgctggacgatttcagcggctttgtcacatcggatcagaattttccgcggaaaccacagcctgattcaattaactggttaattaagaccaatcaggtagacagaaaaaaagcgatcatgattggtgaccgcaagttggatgttgctgcgggccacaatgcaaatatcgcttcgtgtttgtttgatcctgatggcacaatcattgattccggcaatcccgagattcgggtcaccgaaatcaatgaactcgtcccatggttgaccaacaaataattaatgattgtttttaaaatagtttgcgatgccgtcgacaacgtctttcgcaagctttttttgataggccggcttttgaatttggttaaagtcttttttggtattgatgtagccgccctcaatcaaaatagctggaaccgagttgtcccggattaccaagaagttaccgaattccacgccccgcgaacttaacggcagatttttcatctgctggttgactgattctgccaaatgtttggagtcgccgctatggtaaaagtaacaggtgtagccagacgcaacgttgttctcatccgaagagtcaaagtggaaactgacgaagaggttggccgatgatgaattggcaatttccggcctggccgctagtgggacggttttatcggaactgcgcgtcatgacgacccgggcacctctcgcctggagcagtcgttcgactcgtttggcaacttccaaagtgtaccgtttttcgggttgcccggtcattgacagtgcccccgtatccgatccgccgtggcccggatccaaaacaattgtcgcttccgataagctgctgacattttgaacgttgctgttttgaaccagccaggacgctacccagccaatggtgcgatgcttatagatgaccttgatccagttactttttcgactaatcacctgcaatcgctgtccatgctgaactttggcttttaccgagtaggtaacgtctggcccgcttcgaatatttaattgattgaccttaacagtcactgaattggattccagcgagacgatcaacaccaaaaatgtgatgatgatcgtcagggtggcaacaatccagcttttgttttcccaaatttttttcacagttcaatcgttccctcactcaaataatcatattatagttgaaataagcctgagaggccagtctgaatggaaataacgccgatgttcccttgacattttctggctggtacactagtcttatagacagttaaatatccaaccgataaaaagaactatcgaaataagcggcatacagagagcattcatttggtggaaggatgcgtcgattattttgaagtgacactttttgcttatgatggttaatagcgaaatgctattcgtgcgagcgttatccttgagaattaattaaggtggtaccgtgcgaatgcacccttgtctatggacaggggtcttttttttcggaatttaagtgggaggaaacaattatgcgatatcaacgaccaaaaggaacggccgatattttgccaggtgaagctcaaaaatggaactatgtcgaagagactgcccggatgctgtttgacgattatcgttatcaggagattcggacaccaatgtttgaaaattttgatgtcttttccagaacgtctggtgatacttccgacgttgtcacaaaagaaatgtatgatttcaatgataagggcgaccggcacatgagtttacgccctgaagggaccgccggtgttgtgcgggcatttgtcgaaaataagctttacggtcctgaacatccccgcccagtcaaagtcttttatatggggtcgatgtttcgctatgaacggccacagtccggccgccagcgtgaatttcaccaaattggggtagaagcttttggtagtaatgagcccgaattggacgtcgaagtgattgccatggggatggatttgctgaaacactttggcttgtctggcctccggttggaaattaatagtctgggtgataaagcctcccgtgacgcatatcgtcaagcgttgattgactatcttgacccgcactttgatgagttgagtgatgattccaaggttcgtctgcacaagaacccgttgcgggtattggacagcaaagacaaacgcgaccaggaaatcgtcaagggtgcgccatcaattttggactacttgaatgaagattcccaaaagcactttgataaggtcaaacaccttttggaatcactcaacattccgtatgtcgttgaccctgatatggttcggggcctggattactacaaccacacgatttttgaaatcatggttgattccaaggccttgggcgaaggctatacaaccatttgtgccggcggtcgatacaatggcttggttgagcagcttggcggccctgaaatgcccggaatcggttttggtcttgggatggaacggctgatgcttttgatggaagcccaaggggttaaattcccggttcttgaccaattggatgcttacgtagttgggattggcgaacagaccagtgttttgaccttacaaatcgttcaagcattgcgggcagacggtttcgcagctgaccgtgattaccttgaccgcaaaccaaaagcgcagtttaaaactgccaataagctgaatgctcagtacacaattaccattggtgaaagtgaactggaaaaaaagaccgcgaacgtcaaacagatgcggaccgggaccgaggtttcagtaccgctggctgagattttcaaagattttgatgagatcattaccaaatattttacagatgatgaggagattgattagacatgaagagaactacttatgctggccttgttgatgaacagctcatcggccaagaagttgtcttaaaaggctgggtccaaaaacgtcgtgacctcggcggcttaatttttattgaactgcgtgatcgtgaaggaattgttcagttagtattcagtgaggaatttggccaagatgctttagcagttgccgataaactgcgcagtgagtacgttgtggaagccaagggtaaagttgttgcccgggatcctaaagaaatcaaccctaagatgaaaaccggtaagattgaagttgacatcaccgatgccaagattttggccaccgctaagacaccgccattttatatccaagacggcattaacgtttccgaggacctgaagctcaagtaccgttacttggatcttcgccgccctgagatgcaaaaaaacattttgctgcgaaaccggattattcagtcgattcacagttacttcgaccaaaatgatttcattgatatcgaaaccccaacactgacgaagtcaactcctgaaggggctcgagattatctggttccttcacgggtctatcctggttccttttacgctttgccacaatcaccccagcaatttaagcagttattgatgggtgccggttttgataaatactatcaaattgcgcgttgttatcgtgatgaggacttgcgtggtgatcgtcaaccagaatttacccaaattgatatggaaatgtcatttgccgatcaagaagaaatcgaagatgtcactgaaggattcattgccaaggtcatgaaagacgccatgggcatcgacgttcagctgccattcaaacgaatggattgggacgagtcaatggctcgttatggaaccgatcaacccgatgttcgctttggcatggaattaaaagatctttcagacattatgaaggatgttgatttcaaggttttctccggtgctgtcaaagatggcggccaagtcaaggcaattgccgttcccggcggagctgagaagtattcccgaaaagatttggacaaatttgccgattacgttgtacgtttcggagccaagggcttggcctggttgaaggtgaccgatgatggctttaacggcccgatcgccaaattcttcaaggatgccgatctgcgtgaaaagattttagccaaggctgaagcaaagcctggcgatctattgctgtttgctgcagataacagccgggttgttgccaacacgctggcctatctgcgagttgagattgccaaagaacagaacatgattgacgaatccaaatttgccttcttgtggattgttaactggccattattcgactgggatgtcgacttaaaacgttacgtggctgcccatcatccatttacgatgccaaatgaagacgatgttcattacttaatgaatgaaggcgaagacccacacaaagcctacgctcaaagttatgacattattttgaacggccttgaattaggcggtggatcaatccgtatccatacccgggcacttcaagaaaaaatgtttgaagcacttggatttaccaaagagagcgccgaagctcaatttggttacttcctgaacgctttggattacggtttcccgcctcatggtggtctcgccattggcctggatcgctttgtccgtttgcttgctgatcgcgataacatccgtgatgtgattgccttccctaagaactccaaagcagttgagccactgaccagtgcaccacaacctgttgctaccaaacagcttgaagatcttggcttgttcgttgccaaacctgatggtgaaaagtagtttcgagtttcaaatgaactgatttcaataaaatcctgtaatctagtcactgattacaggatttttaatgtaatttttgtcatttacgtttatcattaggcaagacgttcaaaaagttttcgaaggggatttattttatggatgacgtttcaaaattaatgcgtaggcacacctacgtcaccaaaatttcaacttcatttatttacgcaattttagtgtcgattgcggttaattttttctggacacctggacatatttattcatcggggattaccgggttcgctcagttgttgaacaccatcagtacgcgggcgtttccgtttgaaatttcaactgggctggctttattcctgctgaacttgccattatttgtcttgtcgtggcgggcaattggccacgaatttaccattttcacaattattaccgtctttttatccagttttatgattcaattactcaaaccaattccgctcacccatgatccgattatctgtgcaatctttggtggggccgtcaatggatttgggaccgggttggcgcttcgaaacgggatttcgactggtgggctggacattctgggcattgttattcgtcaccgaaccggtaactcgattgggacgattaacattgcctttaactcgttaatcatcgtttcagctgccgtcatgtatggatggccatacgccttttactctgtcctcagtctaatcgttaatgcgcgcatcatggatatgacctataccagacagcagcgaatgcaggtgatgattattaccacccgccccaacacggtgatcgatagtgttcaaaaccatcttcgtcggggaatcacgatcgttcataatgccgaaggggcttatcaacacgatgccaaaacaatcttgttcacggtcatttcacgatatgaaatgggggagttggaggaagctttattggagtccgaccccaacgcgtttgccagcatttcagattcggtcaagattttggggaggttttacgagccgaaaccctgagggcatttttaaagatttcctaagaaacaagttctccaagtggattatgttataatattttttgtgtgtgatcacaaaatattgaaatacggtgaaaattttgaaagttgtttacttatggttaatcaaattattctcagtcctgaatatttggcggccaaagaacaaagttgtttatgtgatgtgctttgatgataatgttgacttcattaagcaattggcacaacgactgcctcagaagtacgttttatatgttctttatcgagccaataccgaagcggctgcgacggatttagcagcctttggtattaaaacgcggccgtttcgcgatggcattaaattcgtgatggacgatgtttcgcttttgatgtcagcaaagctgattatttgcgataactactacgcttttttgggtggcctggttaagctgccattcgtcaaaattgtccagatatggcatgctgacggggcgattaagaagtttggctgggaagatccgaccaccgacaaacgcagccgttctgataagcgccgttttcagaaagtttatgatcactttgatgaatacattgtcgcatcaaaagcaatgggacaggtgtttgtgcacagttatcacgaaaattttgacaagatgcagttactgggataccccagatccgacaagtatctcagtcaagattggcagcacaaggcccgtgagcgaatttatcgatcagctcctgaactgaaaaatcaccgggtcattttgtatgccccaacttatcgggagcatcaggactttaagctgcccaagggactgggcagtgctttggcagcagatccaactgccttggtggttgtcaaactgcaccctgttttgcgggataaagaagtgccgatgcgccgtattggtaatcccaagattaagttttatcacgaattggagaccagtgatttattagctgtggctgacacactggtcactgattattcgtcggtggcatttgattttagtttattgccaaatgccaaatcgatcatctttttcatgtttgatcttgatcgataccgaagcgatccaggaattcaggatgattttctcaactggctaccggtagagccggtttataaggtcgagcagctcagaaacgaaatcctggcagcgacaagcgttaacttcgacaaatttaacgcccattggaacacctataacgacggtcaggcgactgacagagtcattgcgcgttatgtcaaattcttagggtctaattaaggagtgcctcaaattgaaagaagtcagtactttaattaaagaacaatttcaaaatatcggcattatcttccgaatctcaaagtatgaagataaagccgagtatcaaagccattatctgggcctaatttgggaatacttatatccattgattcaaattggtatttattggctggttttcggtatcggcctgaaacacggtaattccacccatggtgtcgattatctggtttggatggttatcggaattacaccttggttctttatgaaccgggccagcctggatgcttccaagagtatctaccaacgggttggtatggtttctaaaatgaaatttcccgtcagtattttgccaaccattaagattgtcagcaacttaagtgccttttggaccatgctggtcttttcaattgtgattggcttcttatatggggtgacgccgtcaatttactggattcagtggatttattacttcatttgtatgattgcctggctgattgcttttggtatttttaattcaacaatttccgtcctggttcgcgattatcggatcttgttgcagtcactcatgcggatgctgttttatatgtcgggcgttctcttcaatttccagacggatgcctttccagcaccgtttgttcatattctgcagttaaatccattcttctacgtcgtttccggtttccgtgacgggatgctgggcagtgcctggttctggcagaaaccaactttgacgattgtcttttggggcatgattctcttcttcttattggttggttctcatctgcattacaaattccgttctcgatttgttgatttaatctagttttgagggtgagcttttgaaacgttcaatgatcaatcttattaaactcatagcccgcattgtactcatcgtgatgaacgatgggtttatttgtatgcccgtcaaaaaggggacggtgttatttgaaagttttaacggcaaagatgtcagtgacaatccatttgctatctacaatcaattaatccaagatgacccggctgcccgaaagcggtgctatttcagtgtcaaacccagtgagtacggcaggctggttaaacagtatccaaatattcaatttgtcaaacggttcacgccgggatgggtgaaatacattgccaaggctgattattgggtgatgaattcgcggatgccaaagtggtggcgcaaaaataagcgaaccactttcattcaaacctggcatggaacaccgttaaagaagcttggaatcgatcttgaaaacgttgagattcctggcagccagacagctgaatatcatcaggaatttattgatgaggctgcccggtgggattatttaattgcgccaaatcaatattcacacgatatttttaaatccgcttttggctattcaggccaattcttagatattggctatcccagaaacgatattttatatactgaaaataacgctgatgacattcgaaaaatcaagcaaaccctatttggctatcagcctaaacaggtgatgatgtacgcacccacctggcgggatgacgatttttccgagaaagggaaataccaattcacgctgccgtttgatctggcacaatttttcgaaaatgtcgatccccaaacgcttctggtcattcggccacactacttggttaaagacaatattgatattagcgggtttgaagaccgggtcaaaatactcgctgatgtcgacattaaccaactatacttaataaccgatctactcattactgattattcatcagtgatgtttgattttgccaacctcaagcggccaatgctgttttatccttatgatctggctcattatcgtgatcagctgcggggcttttactttcagtacgatcaagctaatctgccgggaccaatggttgaaaatcaaactgacttttatcaaaagttaagtgaataccgtcaaactggtgcttttactgatttcagtgacaatttgacccggtttaaccaaaaattctgtgcctgggaagatggtcaggcttcccaaaaagtcagtcaattaattttacaagggggatatacaaatgagtgaaacaccatttttaatcggttctcatgtcagtatgaacggcaaggacatgttcctcgggtctgccaaagaggcggcttcctacggtgaaaccgtctttatggtttataccggagcgccgcaaaatacggttcgtaaacccattgagaagttgaatgccgatgccggcaagcagtatatgtccgatcatggcctccaagcggttgtggtccatgcgccttatatcatcaacctggggaacactttcaaaccggaaaatttcagttttggtgttgattttttgcggcaggaaattcaacgtgcacaagccattggggctaaagaaattgtgcttcatcccggcgctcacgttggtgccggtccgcaaaaagcgatcgatcaaattgccaagggcttaaatgaagtgattgagaaggaccagcacgtccaaattgctttggaaaccatggctggcaaaggcaccgaagttgggacgtcatttgagcagttggctgaaattatcgataaggtcagtgacaacgacaaactctccgtgaccttcgacacctgtcataccagcgatgccggttatgatattaaaaatgactttgatggggtcttgaatcaatttgaccacatcatcggccttgaccggctcaaagttattcacctgaacgattccaaaaatccgcagggcagccataaagaccgccatcaaattcttgggttgggaacaattggttttgataccttgaactacattgcccatcacgcacaattaaaaagcgttcccaaaattatggaaacgccaattttgaaggatcctgacaataaaaacgttaagtggaatcctcatggttatgaagttgcaatgctgaaaaaacagcagtttaatcccaatattattgaagatatgaaagctggaagaccttactagtcaggccaaatcaatcttcgaattcagtggtatttaaattgaggctttccaagataatggtggccgtttcctcaatggacttgttggccacgttgattgttaaacagccaatttgacgatataattttttcgcgtacgccaattcagttttgatatgggccggatccgagtagggtgtatcagcgtccaagccgtaagaaatcatccgttgtttacggattttgctcagtttctcaggggtgttcagcaggccaaacattttatctttatcgatgtcgttgacttcttcagggagttgcaggtccggcccgattggcagattggcaacccgttgattttggttggccaaataaagcgacagcggcgtctttgacgtcctggaaaccccaagcaacacaatgtcagcttccagcagtcccttgggatttttgccgtcgtcattttctacagcaaattcaatcgcagagatccgttcaaagtaattttgatttaaatcatgaatcaacccagggacgtgagccggttgttggccagtaacctgactgagcattgccattggcgtttggacgcagtcaaagtcataaatgccattttgacggcagaaatcttgaaccatctggctgagctccgtacttaccagcgtgtgaaaaatcatcgcctgtttgttgagagcaatttttaagatgcctttgagaattgagtcggtttgaataaacgggaaccggcgaatttcggctttcacatctggaaattgtgacaaagccgtctgggcaattgtctgggcggtggcgccgcttgaatccgatataataaaaatgttttgagttttcatgataaataactcctaaaattatatttgttaagtaaatattaacatgacacatcaattttatcttaaatcattgacgatgtattgattaatatgtataatttacttcgaaccgttttagaaggcacttaaagtgttgattaaacagttacatttaagctcggagggagggaatttcatatggcaaagacagtcgttcgtaaaaacgagtctcttgatgatgctcttcgacgcttcaaacgtacagtttctaaaagcggtacattacaggaatatcgtaaacgagagttttatgaaaaaccaagtgttaagcgtaaattaaagtctgaagcagcacgtaagcgtaacaacaagaagaaacgtcgtttttaataaatgatgactaaaggtcggagctaatgtttattagtctctgatcttttttaatgttaaaatttaagtattaagcgaaaagaggttactttgatgagtgtatatgataaattgctttctgacatgaaggacgccatgaaggctcgtgataaggtccgcttgggtgtcattcggggcattaaggctcaggtgatgaatgccaaagttgccgatggcaatcatgatttaactgaagatcaaattaacgatatcattatgaaagaaattaagcagcaaaaggaatccttggaagaattccaaaaagctgaccgaaaagatttggcagaagaacaggaagccaaactaaagattgccgaggaatatgcaccagaacagctttccgaagctgaagttgaaaaaatcgttcaagaaactatttcacaggttggtgctgaatcaatggccgactttggtaaagtgatgggtgccatcatgccaaaggttaaaggtcaagctgacggcagtgttatcaacaaattggttaagcagcagctgcaaagctagtatactttagataaccacaactttgtggtaatatctgaaccaatatgactaataaaaaaggagctcacttacttggctgatactcaacaagttacaagagagtttattgtatccgaccccaacgaattattacaaattgtcgggactcaagacgagttcattacaattatcgaagagggaatggatgtctccatcaatgtctttggtaattcacttcgagtgactggtcaggatgaacccgttagcattaccttacacattttggagaatattctctctttaattcaaaagggaattaatattaacagcagcgacttcatcagtgcgatgaatatggctcaaaacggcacgctggagtactttaaagatttatacaatgaagtgctcatcaaagacgcaaagggcaaggcggtccgcgttaagacctttggtcagcggcagtatattcaggcaatcaagcatcatgatgtcgcttttggcattggcccagccggtaccgggaaaacttacttggctgtcgtcatggcgatcgcggctttgaagaagggcaccgttgacaaaattgtccttacccgaccagcggttgaagctggtgaaagtttgggctttttgcctggtgacctgaaagaaaaggttgatccttatctgcgaccaatttacgatgccctgcacgccattttgggtgccgagcacactgaacgattgatggaccgggggacgattgaaatcgcgccgctggcttacatgcgtggtcggactttggacaatgcctttgtgatcttggatgaggcccaaaacaccaccaacatgcagatgaagatgttcttaacccgattgggatttggctcgaagatgatcgttaacggtgatatttcacaaattgatttgccaaagcattcgaccagcggattgattaccgctcaaaagatcttgaaggatattgatcaaattgaatttgtaaccttcacggctaaggatgtcgtccgtcacccagttgttgctaaaatcattaccgcttacgaaaaaagtggcaattaatctcgaatagacttgaggaactaaattaatggatttagaaatttacgataaaactgaaaaaggggtttcggaaaaggatcaaaaattgattcgggatgttttggaatttgccggatcttacattcatttggccgacaataccgaaatgtccatgaccctggtcaataatgatgaaattcaccaaatcaacaagaagtatcggggcgtcgatcgggcaaccgacgtcattagtttcgccattgaagatgacgatgatgacgatgatttccccattgtgatggatgaagaattgaaagagtcaattcctgaaaatattggtgacatcttcgtttccgttgataaagttgccgaacaggccgattatcttggccactcgtttgaacgggaattgggtttcctgtgcgttcatgggttcttacacctgaacggttacgatcatatgaagaaagctgatgcggatgtcatgtttccgcttcaaaaagagattttaaatgcttatggactcaaaagataaccgcaagccacaattggataagaataagtcgtttcttcaatcagtcggccacgctcttgaaggcattaaacgactgctgttggaagagcgaaattttcggattgacttggttgtggcaatcattgtattaactttcgccattgtcatgaagattagcatcaacgagtggctctggctgttcgcggcttttttctcagtgattgggtcggaagtcttaaacaccgttgttgaaaacgtcgttgacctcattgttggtcaccactttgacgctttggccaaaagagcgaaagatgttgctgctggtggtgtgttactatcagcgttgtttgctgtgatcatcgggatgttgatctttgtcccgagattcattgcattattaaattaagaggagtaagaaatggataatccagattttcattcaggctttattgccattgttggtcggccaaacgttggtaaatcaacttttttaaaccgggtcattggtcaaaagattgcgattatgagcgacaagccgcaaaccaccagaaacaagattcaaggggtttacacgacgaaagaagctcaaattgtctttattgacacccccggtattcataaaccacagaacaaacttggtgatttcatgatggaatcagctttgtctgctttaaaagaggttgatgcggtgttgtttatggtcaacgccactgaacatcgcggtgcaggggataatttcattatcgaccagctgaaaaacgttgataagccaatttatctactgatcaacaagattgacgaaatttctcccgatgacattatgccgatcatcgagcaatacaagaacgccttggaattcaaggatgtttatccaatctcggcgcttcagggcaataatgtgcccgaattgatcgacaccttaattaaagaattgcccaacggacctcaatattatccagctgatgaggtaaccgatcatcccgaacgatttgtgatttcagaattgatccgagaaaaagtgcttgaattaacccgccaggaaattcctcattcaactgcggtcgtgattgaaagtatcaagacagaagacagtcttttgagaattcgggccacaattattgtggaacgtgatggccaaaagggaattgtcattggtaaaggcggctcgatgttaaagaaaattgggacacttgccagaaaagacatcgaaaatatgatgggcaacaaagtctttctcgaactgtgggtcaaagttgaacctcactggcgcgataaggccaacctgctcaattcttacggttaccgcaaagataattattagaggtgaatcagtttgtcaaaaggtcagcgaacggattttaatggcattttgctttatacaaaagcctatcgggaacatgacctgctgataaaatttctcaccagagaattcggcaaaaaaatgttcctggttagaggcgccaaacgcccacggttcaagatgcgttcagcaattttgccgtttacctacgggctatatggcggcgatattaaagaatcaggattgtcgtatattctcaacgataaacagttagtgcacttccaaaacattagtgaagatatcactaagaatgcctatgccacttatatcatgtcattgattgatatggcttatccggatggtgagccgattgccacttggtatgacaagctgttgaccggcctgcaactgattgaccaaggctttgatgaacagatcatcacgaatatctttgaggtccagctgctgaatgcttacggcgttgcaccaaattgggtggattgcacgatctgtcaccgaacggatctgccttttgattattctgaggcctacggtgggctgttgtgtcagaatcattggaacaaggatccataccggatgcacttggatgcccgcacaatttactatcttcggctgttttcggtagttgacttatccaaactaacccatatcaaggttaacgatcggaccaaaaaagctttgcgggaagttctcgaccagatttattcaagaagtgtcggtgtcgttccaaaaagtaaacactttattgatcagttgggaaaattcaaattataactgataacggcgttgacaatattttgattgtcaactatgattatttttgaaataaataattcaatgatgacaaaagaaatgacaggatggacccttgtagcgaaatcaggatagtgggagctgattatcgtcggtactgtcaatggcgcttttcgagttgaacaattaagtgctggtagtaataccagaagtagggtggaaccgcgatttcatcgtccctatgttgagtggcttagtctataagtcgttgaacatagggactttttttatgcgtttgaataattaggaggaaaatttatgactgaaaaattatcagttcaagagattatcctgcggctgcagcaatattggtcagcccagggatgtatgttaatgcaagcttacgataccgaaaagggtgccggaaccatgagcccctatactttcttacgggcaatcggtccggaaccgtggaatgccgcttacgtggaaccttctcgtcgtccggctgacggtcgttatggtgagaaccccaaccgtttgtatcaacatcatcaattccaagtgattatgaagccttctccggaaaacatccaagagttatatctgaacagtttaaaagaattgggaatcaatcccttggagcatgatattcggtttgttgaagacaactgggaaaacccatctatgggctgtgccggtgttggttgggaagtttggctggacggaatggaaatcactcagttcacctacttccaaatcgttggtggcctggaaatggatccggtcgcttcagaaattacttacggattggaacgcctttcttcatacgttcaagacgttaattcggtctttgatttgaactggtctgacgatgttaaatacggtgatattttcaaagagcctgaatatgagcattccaaatacagttttgaagtttccaaccaagagatgttgttgaccctgtttaatgattatgaacgtgaggccaaacgcctgttggaccaagatttggttcacccggcctatgattacatcctcaagtgcagccatacttttaatctgttggatgccagaggggctgtttcagtgactgaacgagccggctatctgtccagaattcgcaacttagcccgttcggttgccaaagagtttgtggaagcacgcaaacgactcggcttcccactcattaaagacgaaaagaaacgccaagcactattaaaagacgacaaggaggagaaataatggctaataatttcttattagaaatcggattggaagaaattccggcgcacgtggtcaccccaagcatcaagcaactaaagaagcgtgccagtgatttcttgaaggatcaacggatttcatttgctgagattaaaacgttcagtactccccgtcgtttggcactttacattactgatttagctgacaaacagcctgatattgacaaatctgttaagggtccggccaaaaaaattgcccaggatagtgacggtaattggaccaaagcggcgattggcttctcacgcgggcagggtgcaactcctgatgacatcacctttaaggatgttaagggcgttgagtacgtcttcgttgaaaaacacattgccggtaaatcacttaaagaaattttgccggggatgaaggatgtcattaccgccatgactttcccaaccatgatgaaatgggggacgtattcgtttgaatatgtccgcccaatcaaatggctggtggccttgttgaacgataaggtgattcccttcaagattttggatgtcgacacggatcggatgacatctggtcaccgtttcttaggcaaggatattgaacttgccaatgccgacgaatacgaagaaaaactgactgaacagtatgtcgtcgccgacgccgtcaaacgcaaggaattaattaccaagcagattaacaagattgctgccgacaacaattggcagatcaacctggatcccgatttattggaagaagtcaataacttggttgaatggccaaccgcgttctttggcaactttgatgaaaaataccttgccatccctgatgaagtcctaatcacttccatgaaggatcatcaacgcttcttctacgtgaccgatcaagacggcaaacttttgccgcacttcatctcagttcgtaacggtaatgattatgatattcaaaatgtggttgccggaaacgaaaaagtcttgactgccagactcgatgatgcaatgttcttctaccaagaagatcaaaagaaatcgattgccgattacgttgagcggctgaagaaagtcagcttccacgataagatttcaacaatgtatgagaagatgcaacgagtccaagtgatttcaaaacaccttgggaatctcgccggcctatccgagcaggagctcaaggaccttgagcgggccgcttcgatttacaaatttgatttggttaccggaatggttggtgaatttgcagaactccaaggggtcatgggcgacaaatatgccttgttaaagggtgaagatcaagctgttgccaccgcgatttctgaacattacatgccaatttcggcaaatggtgagctgccaaagaccaacgtcggttcaattttggcaattgctgacaaactggacagtattttgacgttctttgctgccgggatgatcccaagtggctcaaacgatccgtatgcactccgtcgccaagcaaccggagtggttcgaattgtggctgataagcagttaaactttgatttggaccagactttgaatctgttaattgatcgagaagatcaagcgtcagttgcaccaaaactggatatgaaagcccaagttcctgccgtcagtgactttgtcaaagatcggatcaaacagtacttggacgacttgggagttcgttacgacattgccgatgcggtgacctctggttcccacaccaatatcctgttcaacattgccagtgccaaaacactgcaggatcataaagacgaccccgacttcaaggacattatcgaatcgctgacccgagttcagcggattgccaagaagggcgccttcaaggctgatgatttaacggttgatccggcattgtttgaaaatgattccgagaaggctttgaatcaggctgtagcagctgctgccaaggattacactcaccaaagcgccgaagaagactttggtcgtttagctcagctcaaagataaaattaatgactatttcgatgccaccatggtcatggccaaagatgaaaagctgaagaacaatcacttgcgccaactcacaatgattgccaacatgattatgtatctcggtgatctcgataaattagttgtcaaaggttaattttgagggctaatatttgtactaattaatgttttatgataatatttaaatacgtatcgccagtaaaacaagtcgcacttttgggtgcggctttttacaggtattgattcagttttgaagatgggaggcgaagtaatggcgaagatcccagaagatgtgattgaagaaatcaggtcacaggttaacattgttgacgttgtctcccagtttgttcaattgaaacagtccggaaagaatttatttggcctttgtccgtttcatgaagagcggaccccatctttttccgtctcggaagataaacagatttttcattgttttagctgtggcaggggcggtaacgtctttaagttcattatggagctgcagaatgtttcctttcctgaggcagttaaaaaggtcgctgagatggaaaatatttctgttgatgagaagtatttccgtgaaagcggcagttcccaatcaagtcccgaaaacacacaacaaaaagcattaattgatctgcacgagcaaagcgtcaagctgtatcaccatattttgaccaataccaagatgggccagccagcgctcgattatctgcataaacgtggattgaccgaccagacgattaccacttatcagttgggatatgccccggcacagcggttgctgaagccatttttcgacgagcgcaaagttgattttcaactgctgcgaaaatctggtctgttttctgaagaccaggatggcaatttgcgagaccgtttcgtcgaccgggtgatgtatccgattcgaaacggttccggtcaaacgattgctttttctgggcgattgttaaccactgattccgacatgccgaagtacctgaacagtcctgagactgacattttcaacaaacgaaaagtgttattcaacctagatttggccaggtcaaatattcgcaccggtgagccggcaattttatttgaaggattcatggatgttattactgcctttcaagcagggatcaagtccggaatcgcgtcgatgggaaccagtttaaccgagcagcagatctatgacatcaaacggattacgcgcgaagtcgtgatttcctatgatggcgatacgcctggccaaaaggcgatcaaacgcgccattgattcattcaatgaacagaagagcaatttggtgatgaaaatcatctcgatacctgatggaatggatcctgatgagttcattcgcaaaaaaggtgccgacgattttaaacagttgattgaccatgctcaggctccagttgagtttgaattgaattatctcaaaaaacaatacaatttggattctgagattgaccaaactaattacattgctgaagctttaaagctgattagccgagtggattccggcatttcacgggatctttaccttaaccggttggcggatgaattttcagtggccaagcaactgctgcaacagcagttagcaccattgatcagacaacccgccccggcggctgaaccgcatcaataccacaagcaggttcaggtcgttaaacagcaaaagcatttctcgttagttgagaaagccgaaatgcagctgatgaaccgcatgctgcactaccatgatatttggttaaaggtaagtaatgtttcggggttcgcatttgttgatgaacagtaccaaatgttgtaccttttagccgaggggtattttaccaaattcgatgattataatgttgccacgttcagcaacctgatttcggaagactcactgcaaagtctattagttgatattgacatgctcgagcttccagataatccgaccaatgctgaaatcgatagctacttaaacattttaatgcatcgagccccggtagaggaaaagttaaagaaaaagcgggcagaactcaagcaagccgttaagattggtgatgttgacaagcaacgtgcgttaacgattgagattgttaagcttgaacaacagaagagaatgaagcaacaagtataacttcaggaggcgttttgatggctactaaaaaaaccgacgataaagtaacagaaacaaagactgccacagctaagaaggcaactgcagctaagaaaacgactgcatcaaagaccagtaccaaggccaagtcaaccaaagcgaagacaactaaggccaagactaccaaaaaagctgacaagccatacaagaaggaatttgacgccattgttaaggctaataagccaattggccatattacctatgacgaattggaaaagaagattgaaaagccttattctctgagtgaaaaggatatggaaggcctcttggagagtatcgaggactccgggatcagtgtcgttgatgaaaacggcgatccggatccgcgagccatcggtgcggctaagaaagtgaccaagaaggaactttctgatgtttccgcgcccactggtgtgaaaattaacgatcctgtccgaatgtacctgaaagaaattggtcgagtttcacttctgagtgctgaccaggaaatttcattggccaagcgaattgaagccggtgacgaagaagccaagcaggaacttgccgaagccaacttacggttggtggtttcaattgccaagcggtatgttggtcgagggatgcaattccttgatctgattcaggaaggtaatatgggcttgatgaaggccgttgaaaagtttgattaccgtaaaggattcaagttctcgacttatgcaacttggtggattagacaggctatcacccgtgcgattgctgatcaggctcggacaattcgaattccagttcatatggttgaaacgattaacaagttgattcgaattcaacgacaattactgcaggatcttggccgtgagccattacctgaagaaattggtgccgagatggacatgccaactgaaaaggttcgagaaattctaaagattgctcaagaaccggtttcccttgaaaccccaattggtgaagaggacgacagtcaccttggtgatttcattgaagatcaggatgcaacttctcctgctgaccatgcggcttatgaattactcaaagaacagctcgagagcgtccttgatacgttaaccgaccgtgaggaaaatgtgttacgattgcgatttggtcttgacgacggtcgtacccgcacgcttgaagaagtgggtaaagtctttggtgtgactcgcgaacgaattcgtcagattgaagccaaggcattaagaaagctgcgtcacccatcacgaagcaagcagcttaaagatttcttggattaatttaatatgatcattaatcgagttggggcacttcggtgttccaactttttttgtccgctaaaatggcccttccaagtaaaatgcctctcggaatctgtcattttccattaggataatttataatgaatttatacacaaaatgaggagcaaaatatgaatagcacgcatttatcgaaacgactacaaacggtcagtgaccacgttgaacctggcagccggctggcagatattggctcggatcatgcctacctgccgattcacttggctcaaaatcatattatcgactatggcgtcgtcggtgaggttgccaaaggaccgcttgccaacgcgacatcagaaattactaaggaccatttgttggatatccttcatccccgacttgccgatggcttggcagccattgaacccggcgacgacattgatgccatcaccatcgccggcatgggtggcaacctgattacccacattttggaagctggtaaggctaaattaaccggaaaagaaaagttgattctccaacccaacgtcggcgaaccggtcgtcagaaactggctgatggccaatcaatatcgaatctttgctgagcagatcctaaaagaagacggccatatctatgaaatcattacggctaaaaaggccgccaaacccgtcacttattcaaaattggcccttcagtttggtccatttttattacaagaaaaatcgccggtgttcgttgaaaaatggcaggaagaaattggcctgctaaagcgggtgattaagaatatgcgtcaggccaccactcccgatacggcaaaaatggcggccgttcaggcagaaattaaactaatcaatgaggtgatcaaggttgaaagctaagcagttaattgaaagatttgagcaatttgcccccaaaaagttggcaatggaaaatgatccggtcggcttacaaatcggttcactcaatcaggaaattcacaaagtcatgaccactttggatgttcgcccggaagtcgtcgatgaggcgattgccaaccacgttgactttatttttgctcatcacccggtgatgtttcatccagctcataatcttgatctcgatgacccgcaaaatgcgatgtacgctaaaataattgccaaccacatcactgtttacgctgcccacactaatttggacgctgctgacggtgggatgaatgattggcttgccgaagcacttcagttaaacaatctaagtgggatggtccctgcctatgatgaatcggtctttcgattaaccgtgcaagtgcctaaagtctatgcgacggctgttagaatgtcgcttgtcgatgccggtgcgcaagccagtgccgctcagtacagtggatacacctacgaaattgacgggacagtctactatgttcccaaggccggcgccgatccaaccatggggactgccggtgaaccaaatgaaatcgaagactcgcgattggaatttgaagttcccgaaagaaatcttcatcaagttctgaagactttgtcagatgttcatccgctggaaaaaccactttacaatttgattcgcctggaagacaagaagcaccattttacgatgggtcgaatcggtgatttgccgcacagcatgtctgtccaggaattggctgaagactgtaagcagacctttggggtttccggccttcgggtaatcgcttctgacctggctcagccgatcaaacgagttgccattcttggtggcgatggcggcaagttcttccacttggctcagcagaagggcgccgacgcatatgtcaccggggatgtttattatcataccggccacgacatgttggctgccaatttcccggtgatcgaccctggccaccacattgaaagtatttgtattcccaaattggccgagctgttcaaacagtggtccgaccagtatcactggcagctggctatttatcagtcaaccatcaataccgatccattcacatttatgtagataaaaggagataactgtcatggcaaaatacgccgaattaattcccaactttttaacgtttgtaaagattaatacccgttctgatcctcaatcaacgagcattccgtcctctgatagagagacagagtttttgaatcaactaaaggatcgtctgactaaaatgggcttaaaagacgttcacaccaacgagcaaagtgcctatgtctttgcgacgcttccaggaaacgtcgacaaatccgttccaaccgttggcttcatttcacatattgatacggctgattttaatgctgaaaatattcaaccacaaattgttgagaattatgatggccattctgtcattaaacttgatgagaagggtgaatatacgctggaccccaaagtctttccaagtttgaagaagtatgcaggccaaaccctgattaccacggacgggtcaacgttgttgggtgctgatgacaaagccggcgtagcagagattattgctgcaatcacttatttacaagcccatccggaagtcaaacatggcgacattaagattgcctttggtccggatgaagaaattggtaccggcgccgaccattttgacgttaaagatttcggcgcagatgttgcttacaccgtcgatggcggcccacttggggatttgaattacgaaacctttaatgccgccgatgcaaaagtcgtgatcaaaggaaccgatgttcatccagctgaggccaagggtattatggtcaatgccatccaagttggaatggatttccacgccgccttacctgactttgaccgtcctgaaaagacccaggatcgggagggattcttccatctgtatgatttccagggaaccgtcgaccacaccgaaatgggctacatcatccgtgaccatgatcgagatcgctttgaagctcgaaaacgacttttcaaggggattgccaaccagatgaacagtgactttggtgaggaccgggttaaggtgaccatcaaggaccagtattacaacatgggagaaattatcaaaaaggatccaacaccggtaaaaattgctgaacaggcgatgaagaacgttgacgttacaccgcatgttttcccggttcgtggcggaacggacgggtctaagatttcttacatgggactgccgacgccgaatattttcgctggcggtgagaatatgcatggccgttttgaatacgtgtctgagcaaaccatggaaaaagcggttgacgtggtactggaaatcgccaaattatacgctgaaaagtaataggtcaaaaaaggtcaaattattgttcagggcattcaaaatttgatagtatagcgttagtggtttggaatgaaaagaatgatttttgtttcgaacctttttattagaacgaattcttgaaacaatagtcaactaaaatacattaataaggtgataatttaatgaatcctgataatttaacggaagccgtcacgcaggcaatttctcaggcccaacagattgcggctactcgaaaacagcaaaacattaccgtggcccatttattcaaattcttggttcaacccggcgagttggcccgagagatttattctcaactcggattgaatttgggagatctgaatgatgaactggatgctgaaattgatgccatcgcgacggttgaaggcagcaacattaattatggtcagtcactctcttccaatttatacgaactgttgcagaatgctgaacagattaaaaatgaatttggcgatacctacatcgctgttgacaccttaacgattgctgtgatgcagttacacggtgacaaatttgccgattatctttctcaacaaggtattaccgagcaaaaggtgcgcaacgttgtggaaaaaattcgtggcggccaaaaggtgacgaccaagaatcaagaggacagttatcaatcacttgaaaaatatgggacggatttagtccaggctgcccgtgacaataagctcggtccaattatcggtcgggacgaggaaattctcgatgtgattcggattctttcccgaaagactaagaataacccggtcctgatcggggcgcccggtgtcggcaaaacggcggtcgttgaaggcttggcaatgcgaattgcctctaacgacgtgccggaaaacttgaagaataaaaccatttttcaattggatatgggatcattaatcgccggcgccaagtaccggggcgaatttgaagagcgattgcaggcggtgttaaaagaggtcaaaaaagccgagggccaaatcatcatgttcatcgatgagattcataacatcgtcggtgctggtaaagctgaggggagtatggatgccggcaatatcctaaagccgatgttagctcgtggcgaattgcatttaattggggccaccacgattgacgaataccggaagtacatggaaaaagacaaggctcttgagcgtcgtttccaacgggtcatggtccacgaaccctccgttggagatacggtgacaattctgcgtggcttgtccgaaagtttggaaattcaccacggcgtcagaatccatgacaacgcgttggtggctgctgccaaactatctgaccgttatattaccgatcgctatttgccggataaagccattgatttggttgacgaagcctccgctgaaattcgggtcgaaatgaactccagtccaactgaacttgaccaatcaaagcgccagatgatgcgcctggaagttgaagaagctgctctcaagcaggaaaccgatgaggcatccaagaagcggctgaaagaagtcgaagaagaactggccaatattaaggaaaaagtcaaccagttaaatgcccgttggtcgcaggaaaaggaagctattaagaaaatttccgacaaaaagaaacaactcgatcaggccaagaatgaattgaaacaggcggaaaacacctatgatttaaatcaggctgccgtgttgcagcacggaaccattccgcagttggaagccgatttgaagaagcttgaagataacgatcagcattccgattggctggtcagcgaatctgttaccgccaatgaaattgcggcggtagtgagccgagagaccggcattccggtcaccaaattagtcgagggtgaacgaaagaaattgctgcacttggcagacaatctgcacaaacgggtaattggccaagatgctgcagtcacagctgtctcagatgccgttattcgctcacgtgctggccttcaagacccaagcaagccactgggttcattcttgttcctggggcctaccggagtcggtaagaccgaattagccaaagctttagccgaagacttgtttgattcggaaaatcacatggttcgaattgatatgtctgagtatatggaaaaggaatcggtttcccgcttggtcggcgctgctccggggtacgtcggctatgaagaaggcggtcagttaactgaagccgtgcggcgcaatccatacacgattgtcttatttgacgaaattgaaaaggcacatccagatgtctttaatattttgctgcaggtcttggatgacggccgtttgacggatagtcagggacggacgatcgattttaaaaacaccattttaatcatgacttctaacttaggttcagacattttgcttgaaggcaccgatgagaacggggttatttcccaaaaagcccaacagcaggttaaccaattattaaaagcttcgttcaaaccggaatttctgaatcgaatcgatgatgtgatcacctttacaccgttgacgaaggccgatattgaacagattgtccagaagctgattaatcagttatctggccgtaccaaggctcaagacatcaaattgtcaatttctgacgaggccaaacgctggattgccaataacggctatgaaccgcaatatggggctcgaccgcttcagcgttatgtgaccaacgtcgtggaaactccgctggcacgaatgatcgtggctgatcagatcaagcctcatagcgtagttcacattaaccttgataacgatcagttaagctttgttcctgaacaattacctgctgacgcacagatttaaaccaagctacctggggaggaattcggtgtgccgattaattaccagcttccaactgaaaatcaaactcaattagccgtggcgtattttcccgctgatcatccaaagggaattgtccaacttattcatggcgccttggagcataaggaacggtattatgaattttgccggtttttgagtgaccatggctatgttgcggtgatctcagataatcgcggccacggccaatcagtttccgacgatgacccttgggggatgatgcgcagtctgccgcaattaatccatgatcagctgttggttacccaattcatcaaagcccggtatcccaatctgccagtcagtctgtttggtcattcttttggttctatcttggcgagattgtatttacagcaccacgaccaggaagtcaatgcggttgcgttaaccgggaccaccaactatattccggtggtgccgcttggcttattcattggttgggtctttttgaaatgccattctgaagatgctaaatggtccttgctatctaaaatttccggcctaactccgggggatcattcctggttgagctataatcaggcaaacattcaccgggtcagtacagatccgttaatgatggatgaatatccggttaaaagtttggtaacactgtggcagggcgattattccctgaaacgccttcaaaaatttgactgtcacaatccacaactgctaattctgagtttggtcggcagtgaagataagttcagtggtggtcagaagggcttggcagacacggttgcaacgctgcataggatcggctatcgaaatgtgatcagtctgcaagagccgcatatgaagcatgaggttcttcaagaaacgcatcggaaagttgtttttgaacgtctgctgcagttctttgacacacaccagtaaagttgattgagacaacaaaaaggctatggcaaaatctgccatagccttttaacgtttcgaaaaactattcttttgatttacttgatgttgctgaatccttgctgatcagatagataccgtttacggcaataaatgcagtaattgcggcagcaattccgatttgggaaggatcccacgttcgaacttcgagggcggaacctatgtaaccaatgatttctccaaagatgtatgcccacaaaacagctacaatatttgaactaataagtttcatgtctaatgccacctcacaatcaatagcattttagcatatattttgtgaaaaatcatcatttatttaatttgccaatttgaatgtgggcttgatatatttggtataattttaattaagaaagaagggcaatcctgtgagttatgttccgttgcaagtcataagttcatacagtttactgcagagtccgattcgcattgcggacttgattgctgaagccaaggatcgcggttatcaggcgttagcgttaactgacctcaacgtgatgtatggggccgtggaattctacgacgcttgtttaaaggccgccattaagccactgatcggtctgactttgcagctgcccggcttgattttgaccgataaagaatatgggtgggtgctgattgccaaaaaccagcaaggatatgccaatcttctcaaattatcaacattaaagatgaccatgcccgaattgacagcttctcagttaggtgactatttgagtgatttagttctgattttgccgccggcagcagaaatgaatgacctgcttctacaagggcgggctgatgacgctgctgatttgattgatcaggtcaaatccctcgggattgatcctaatgcccttaaaatcggtgtcgactaccattcctcggacagcttaaatgacatgttaagtaagctggcggctgacaagcaagttgctttggtggcggattcgccagttgaatacttaaacgccaccgactatttttccatgcaggttctaaaaaatatcggcgcgggagaaaaaatcgccaacgtggcccaattcagtaagcaagtggggccctactggctgcgtccggcgacacaaattgaggctcaataccgtcaggttcacctcgctgacgcgctgacgcaagtcgaccaaattgtcgctgattgcaatgtcgagattaagaaacagcagcccaaattgccccaattcgacacaccaaacggtatcgattccggaacttacctgcgccagctttgcgaaacgggactggcggatcgactaaagaaaaatcagattacagatgcgaccccttatcatcgccggctggatcaagagttatcagtgattcattcgatgggctttgataattacttcttgattgtttgggatgtgattaatttcgctcaccagactgacatcattaccggccctgggcgtggatcggccgctgggtcattagtggcgtataccttaacgattaccgacgtcgatccaattaaatatgatttgctgtttgaacgtttcttgaatcctgaacgggttcagatgccggatattgatttggatattccagacgacaaacgcgatgaagtcatccaatatgtccatcaaaaatacggtcacaaacgggttgcccaaatcatcacatttggcactttggcagcgaagcaatcgatcagagatgtcggccgggtgtttggcttgaatactgcccagcaagatcagtggagtaaggccattcccaacgcatttcacgtgaccctcaaagacgctttggcgaattcccagcgactgaagaatctggtggctgacagtccgctcaatgaagcactctaccaaaccgcccaagcgctggaaggcttgccaagacactattcgacccacgctgccggactggtattaagcgacgatcccctggtgaatttagtgccgcttcaaaatggcaacgaagggctgttgatgactcagtattccaaagattatgttgaatcggttgggttgttgaaaatggattttctgggactccggaatctgtcaattttgggtgatgccctggagcaggttcaactaaccaccggaaaggttctggacatttctgctgtgcccttggatgacgccaagacgattcaattattcgccgacggggacacgactggcattttccaatttgagtccaacggcattcgaaatgtcctgaggcgtctgcatcccgaacggttcgaagacattgccctggtcaacgcgctttatcgaccgggacccatgcagaacattgatgaggtggttaagcgaaaaaccaatcatgaagcgttaacctacccggacgactcgctcaaagatattctccagccgacttatggcgtaattgtctatcaggagcaagtgatgctggtcgcttccaaaatggccggtttctctctaggtcaagctgatattttacggcgggcgatgagtaagaaaaagcttggcgtgatggaacaaatgaaggctcagttcatgaccggcgccaaacagcggggatattcagattcagtcgccaataaggtctttgactatatcgagcggtttgccaactacggcttcaacaaatcccatgcggttgcctatagcaagatggcttatgaattagcctacttgaaagtttattacccaggcgaatttcacgttgccctgttaaattcggtcaacaataattcggttaaggtcaaggaatacatccaagctgccaaatcaatgggggtcaaggttgttggcccaaatattaatcatagtgaagcccggtttacctttcaagatcaacaaattgtgtttggccttgattcaatcaaaggcgtgcgtcacgacatggtagtggatttattggctgagcgacaacaaaacgggccatttaagtcgtttccggactttttgagccgcctgcccggcaagtaccgcaaagttgaattgatcaatgccttgatttatgccggcgcattggatgtttttccatttaaccgttccgaattaatcgctgccgcccctgaatttatcagctccgttgaattaagcggcaattcgatgagcttgttcaaagcattggagcccaaaatgccaaagatgcccgagatgcctctgatggacaagctggaaaaagaaaatgcttatttaggggcttacttatctggtcatccgacagaacgatttgcccccttggcacagcgattaaatgctgagacaaccgctacgttgagttcaggtatgaaaaatatttacttgattctctacattaccaaggttaagattattcggaccaaaaccggcaaacaaatggcctttttagacggtaatgatcaggtggggcagacttcggtgactgtttttcccaacttatttaccaagacccagtcatggcttcacaaagatttggtgattttgatcaaaggtaacgtcgagaaagtcaacgatcttcaggtggtcgccaatgacatccagccggcggctaacgccctgatgaacctcaagcgatcaaaacagcaatctaaatggtatttgcgaattgatcgcgaacatgacaaaaatacaatgtttcacaaactggccgacctgagcagccaatatcacggccaggtcccggtcatcgtttttgaaacagaaaccaaaaaaacttggcagctcgaggacaagctgtggctaaatccaagttctgaaaccaaagagcaattaatcacaatctttggcaggaataatgtggtttataagtaaatttttggaataatttttcagaagtcaggttcattacgtaaaggctttcatttgcggtagacctaacttttgccattccaagtcggtgctggaaagcccgcttacccccaaaaggtgggcgacaacccgcttaaaaagtgataaaatacgattgaaatctaaaaggataccgatgcgttatttaaattgttttgcgacattttaataaggtgttgcgtgcccaaaaaccgaaggagagattttacttatgaagaaaactaagatcgtaagtacattaggcccagcaagtactgatgtagacacaattactaagctgattgaagctggagctaatgttttccgatttaacttttcacatggtgaccaccctgaacatcttgatcgtatgaacaaggttcacgaagctgaaaagaagactggcaagactgttggaattatgcttgataccaaaggtgctgaaattcggacaactgttcaaaaagacggcaagatcgaattccacactggcgatgttttccgtatttcaatggacgcaagtcttgagggtactaaagacaagatcgcggttacttaccctggactctttgacgatgttcacgaaggcggccatgttcttttcgatgatggtttgttggacactgttgtcactaaaaaagacgatgctaacaaagaattagttgtcactgttcaaaacgacagcactcttggttcacgtaaaggtgttaacgcacccggcgtttcaatcaacctgcctggtatcactgaaaaagattcagatgatattcgttttggtttggacaatgacattgacttcatttctgcttcattcgttcgtaaagcccaagatgttttggacatccgtgaattgcttgaagaaaagcatatggaacatgttcaaatcttccctaagattgaatcacaagaaggtatcaacaactttgacgatatcatcaaggtatctgatggtttaatggttgcccgtggtgatatgggtgttgaaattccagcagaaaacgttccgttggtccaaaagactttgatcaagaaatgtaaccaacttggcaagccggttatcaccgctactcaaatgcttgattcaatgcaggaaaacccacgtcctactcgtgccgaagcttctgatgttgccaatgccgtctttgatggtactgatgcaacgatgctttctggtgaaagtgctaatggtgattaccctgttgaatcagttcaaacgatggctcgtatcgatgttaaggctgaaaatgcctttagcgaatttggtaccccacgtccagaatttgactcaagtgatgttactgaatcaattggtgactcagttgcccgtgttgccaaagaattaggcgttcactgcatcgttgcagctacccgttctggttacactgcacgaatgatctccaagtatcatccagatgctgacatcctggccattactttcgacgaacgtactcgtcgcggtttgatggttaactggggtgttcacccaatcttggttgacgaagttaagagcactgatgaaatctttgaattagcttcaaagaaggctctcgaaactggtttagctaaggaaggcgatttgattatcgttactgccggagttcctgttggtgagagtggtaccaccaacttgatgagaatccaactgatcggttcaaagctggttcaaggtcaaggagttggtgacaagactgttattggtaaagcggttgttgctaaaaacgctgctgatgccaagagcaaagtaactgaaggcagtatcttggttactaagtcaactgacaaagaatacttaccagctattgaaaaggcaagcgccgtagttgttgaaaccggcggcttgacttcacacgcagctgttgttggtatttcaatgggaatccccgttgttgttggtgcagctgatgctaccagcaagatttctgacggtgaattgattaccgttgattcacatcggggcgttatttaccatggtgcttcatcatcaatctaaatttaacttgtgagtaatcacaattaatcatgacaggtccgggcggttaatccgttcggacctgtttcctgttatgataagggcggtcgaattttcactgaaaaacgtgtaaaataagattaagctcgattagatcggagataagcatgaataatattattgcgcaagttgtaaccggtaagatcatcgatgaaaatgacaaggactattacgttcagattgaaggagaaacatttctccttgataagactgagctcaagaaacccttgcgaatcggtgcgtctttcactggttttacgtatgaaaatgaacagcataaaatgcaaataaccagaaacattccggatatccgtcgtgatcattacggttttgcgaccgttgtgaaggaaaaatttggtttaggggtctttgtcgacattggcctgcccaataaagacgtcgttgtctcaattgatgaactgccgacagtccggtcattgtggccgcaagacggtgatcaactgctgattgatttgacggtggataacaagaaccgaatttggggtcacttagctgacgaagaaatctttgcggcaattgccaagccggccaaggatgatctgcagaacaaaaatcttaaggctcgggcataccgcctgaagatttccgggacgcgcttgttgaccgaggattacaatttggcttttctgcatcctgacgaacgactcatggaaccacgtttgggacaggaagttgaagccagagtgattggcatgctccgggatggcagtgtcaatatttccaccaagccacgggcttaccaagaaattggtgaagacgctcagatgattttggcggccattgaacataccgacgacaaacaactggcgttcagtgataaaagtacgccggattccatcaaagattactttggtatcagtaaaggcgcattcaaacgggcgttgggacatctgctgaaggaaaacctgatcgaacaagctgatggccacatttccttgaaaaagtaggcttttatgatgcacgaacaaattgaggactatcttcattatttacgggtcgaacgcggcctttcagataatacaattaaaagttatcggcaggatctgcaggaggccggtgctttttttgacaaacacgccaaatcaattgctgacattgaccagtttgtcatcttggattatttagaaacccttcaacggcagcataaagcccggaacacggttatcagggtggtctcgacattacggcggttcttccagtacttggttcaattccacgtgattgttgacgatccgatgctcaaggttgattcgcctaaaaaggcccagacactgccggacgttttgactgtggcccaagttaatcagttactatcgatgccggatactcataaaaaattaggtctgcgcgaccgcgcgatcttagagacgctgtatgccaccggcctgcgggtcagtgaactggttaacttgaagttgggtgatttgcatttgccgatgaacttgctgcagacaattgggaagggcgacaaagagcggatcatccccatcagcgacgtggcgatcgactggttgaatcaatacattcaatcgacgcgtgtccaactactttcgggaaggcccaactcagagttcctatttttaaatgcccacggtcaccaactgacccgccaggcaatctggcagatgattaaaaaatatgtcaaccaggccggcatcaaacgccatgtcacaccacatacactgcggcattcatttgcgacccacctgcttgaaaacggggccgacttaagaatcgttcaggaactgttggggcattccgatatttcgacgactcaaatctacacccacgtttctcataagcatttaacggaagtttataataaatatcatccgcgagcataacgaaagaggttgaatacatgttatatcaataccgaaaagattatgaaaagatcaccatgggcctcttttcgttggtttccgaactgcagaacatggatctggttgcccaagaaatgagctggtacgccgccaaagacgaccgactgatttatttatggcgggacccatccaataattggtcgggcttagtcggaattgaacttcaaggaaaccagctgttggttcatcaattggtgttaaccccgcaaagcgtcagtcaggggaactataaccggatttttgacgacctccaggatttatatccaaaatatcaaattgtggtcggctttgaaaatcgagccgcctgggaaaaatgggagaatacgattaatcatgcctgaagtcaagcagccggaattacatttgaatgattttgacgggccactggaagtcctccttcatttgattcaggaatccaagatggatatttatgatattcagatttcaaagattaccgagcaatacatgcagtatatctatgatgcccagcaattgaatttggaaattgttggcgaatactttgtgatggctgccaagctgatggtcatcaaatcaaagatgctgctgccgacgattactgacgatcaaccggatgaacagcaggccgatccccgtgaggaattagtgtcccagttgttgaattataagcggtacaaactggtggcggccagcatgaaaaagcgggaaatgaaacggcgggagagttttacccgctccgagttgagcgtcccgccgaccaaagcggaattgattcagccatctccgttcaacagcggcgacatcatggccagctacgtggatgccttgaaacacttcaagtataatcaacacatgtcgacggtgattcatgagtggtcctttacgatcgaaggccagagtcaacgggtgcgcgagctgttaaaccaaactgataaccggatttcctttgataaattggttgccaattcaactcaaacagaagaggtcgtcactgattttctggcgattttggaaatggccaagtataacgaagtccagctcaatcaaccaaccgtacaatcgaccattgaaattcgaaaggggcctggataccttgatcagtaatctggcaaaaattgaagcactgctttacgcctcgggggaccaaggcatcacgttgcggcaaatgtcccagcggaccgcgttaacggtggccgcctgccggcagctgctggaaaaaattgtccaaaaatatagccaagatcaagacagcggcttgaaggtgttcgtcagcgacaatgtgtatcggctgggaaccaaggaagaattgtcagaactagtgggcgattatgtcaacgatgccaaaccgcgggttctgtcggaagcggcattggaaaccatttcaattattatgtataaccaaccgattaccagaattgaaattgatcagatcagaggggtcaatagctcggcgattctccaccggctggtcaatcaagatttgattgaagtgactggggtcaaagaagaggtcggcaaccccaaacaatacgggatcactaattttggcctggattattttgggttgaagtcgttgaaagatttgccgccattgccaaaggatgaagtcttggatgatgataccagtgattcactattaacccgttttaacaaagagattgataaagaaaattaggaggtggatgtatgaacgaagaacgtttacaaaaagtgattgcacacgcgggagttgcgtcccgacggaaggctgaagagttgattgccaaaggacacgttaaggtcaatggcgaggtggttaaagaactaggaaccaaagtcaccccaaacgatgaggtgaaagtcgatgaagtgccgatttcaaaagaagccccagtctattacctgctttacaagcccagaggggtcatcaccgcggtaaccgatgacaagcatcgaaagaccgtggttgatattttagaagaggttcccgaacgaatttatccggtcggccgcttggactatgacacgtctggcctgttattattgaccaacgatggcgacctggacaacaaattaacccacccaaagtacgaggttgaaaaaacctatgtcgccaaggtcaagggaattgtgaccaatgacgacctcaaacacttgcggacgggtgtggtaatcgagcatcgaaaaacggccaaggccaagaccaagctgattcgcaccaacaaggactcgtcgattgtccaattgacgattcatgagggtcggaatcaccaagtcaaaaacatgtttgaaaaaattggttacccagttgaaaaattaagccgggaaacctatggctttttgacattgaaaggcttgcagccgggggattatcggccgttgaaaccacatgaagtcgaagaattaaaggaattgacgggcaagacaaatcgttgacatttgccttggttctgctatatttgaattaaataaattggtttatcttcagggcagggtgtgattcccgaccggcggtcatagtccgcgactcacgagtgatcgtgctgagctggtgaaattccagtgccgacagtaaagtctggtatgtagaagattaaattttacattttttgtaatgccctgacaaattctttttgtcagggcattattttgaagattgaccattggaggagaggttttttcaatggaaaatagtggtaagcatacgcagtttgcaacaacgcgtttggttgagatgtccgtgtttgcgggactctcatatgttttgatgtttttgtcagtgccgattattccaatcgtgccttacatgcggttggatttggcagacatgccgattttactgggaaccgtcttgtttggaccggttggcggcatgacgattgctggtttgaaggccttgctttactgggtaacgactggtgccgacgtgattaacttcattggtgtcggttcatccctggtttcatctttggtgctcatttgggcatactacctggctgaccggcttttctcatttaccaaggggtggaagaaagcagggctggtaattttgaccatggccattgccttgacaattatcatgtcattgaccaactggctgggagttattcccctatacatgaacctgattggcatgaaattaggctttccactggcaaccgtcattttgtccggtgttgtaccatttaacttcatcaaaggaattgtcgtcggtggtgtgttctacctaatcaagaacagtttcctgccacgcttaaaacttcgctaaatgtggatagaaccattcaaaatttgtttgatatagtataattgaatagtgagtaatcttagaggctgggacaaacttgcgggtttggactggctttttgtttcggaggtagttcatggacttaggcattctcatgttaatttttggtagtgatcggcaatttcggcgggtgaaggcgattaaaaacaccttacgggggcgccgcactgtttccaatttatactgggcactggaatatgggatgcttgattttatcgacgttctccacggtgccgacttcggtgaagaccagccagtcttggcccagttgtctgccaacgggttggctcaagccgatgatgacttcagaatccaattgactgcaaagggggtcgaacagcagcaagcttatttgaatcagctgctgcctctcgaatccctggcagtttcgtcgcgctatgatgtggccaaattcatgcggcggttcagttttgccacccaaattgtttcagaattcagctatggtaacaatcaatactatccccagtcaattaattattttgaagatcagctgttaaaacgctggtttattgatcataagcaggaccatctaccggaacatttccgccaattgttaaacagctttttgagtgacctccaccaggatgaactggctgatctcttcgttcaaagcctggttggacatgacttctcaggattgacagctgagcaggtggcagtcaaacgccacgtgccgaccacaattatcgaattgcagtggctgcagttgtatgggatgctcctggaaaaagtcatgcgcgcaggaaagacgagtttatttgcaccattgactgccggattggccaaaccaattatctccaacagtgctcaaaccacctttaagatgtttgtccggcaagcggatcgaaatccccacgccatcgcaactcaacgtcacatcaagctgacaacggtttatgaacatctcttggaggcagctatcctgaccccggtggcgaagtttccatataggaacctgatttcagaagatttgatgaatcaactagtagctcatcagccagcaaacgtgggcgagtggtctttccaagatgccagtcaggtggttaatcaattggcatttttccaatttcgactttttcagatatacaggagtaaaacgacagatggtcattgatctcaaacgtgaattaaaaaaatattttggctttgacaccttccggccgggccaagaaaaaatcttacagaatctgttggcccatcaggataccttggcgattctgccgacaggcggcggcaaaactttactttatcagatgtatggggcaatcacccatcaacgggtcatgattgtgtcaccgctgatttctctgatgcaggatcaggtcagtcgactgcaatttctgggatccaaacgggtggttgcgttgacttccgcgttagattttcaagagaaaatggcgattttaaatcatttgaatcgttaccagtttatttatgtttctccggaaatgctggcaaatgaccaggttcaacagcggttgaggcggctgagcatcggcctgtttgtcgtcgatgaagcccactgcatttctgaatgggggcctgattttcgcccggattacctcaaattagggacggtgcgggagatgctggggcggccactgacgttaatgatgacagccactgctacccaaccggttcggcgagatattattcggcatatgaattttcgattcgaggacgttcaccaaattgtcttgcctgtcaatcgagccaacatatttttaagtgcgaaaatttttgccaatcaacatgataaagacgctgctctgattgaactggtcaagcagctcaatggacctggaatcatttatttttccagtaagagtaaagccgagcaggctgccaacacgttgacgaatgaaaccaatcgccgggtgatggcttatcatggggggatggacagtcagccgcggtttcacattcaacagcagtttttggcagggaatttggacattgtctgtgccaccagtgcctttggaatgggcattgacaaggataacatccgctttgtcattcattaccacctgccggcgaacattcaaagctacgttcaagaaattggtcgctgcgggagagatcaacaaccggggttggcaattttgatgtatgaacccaatgaccgcggcctacaaatgggtctgatcgaccatacgatcccggatgaaagcctattgcgttatttgtatcagcatcctaaggcattagccaccgatgatcagtttcgggtggtcaagtattatcatgacagcggcgactcgtttgagcaggccaaatcgatctttgatcatgctcgtactcggcgggtgaaggaactgggggcgatggtccaatacgtctacacggaaaaatgtcggcgtgatgagttgctgaagtattttgatgaaacagtcccggatggcgagcggaacccggcattttgctgcgatcacgatgtcgatttttggaatcgctggcaggattttaaccggcaatatttgattcaaccggaaaaatccggccaaaacgaaaccaaaggctggcagcaagtcattgaccagctgtttttatcaaaaaattaaggtaaatttaagtgaattaatgataaaataagtttgtctatatcctgatcaagaggggggtcaatatgaattcgaatgatgaacataaaaaaactgacgaagatcagccctggaatcaaacattttctgaggatcgtgatgaaaatggtaatctttcgcgagtcaaacttagaaagcagagccaaaatcaccatctgattacgatggtcttagcggcgttaatcattatcgttgcggtggttgcgctggtttacggcctggttcgccaaagtgcgatgggcaatgattcaaagagtgccgcgtcttcgtctgtcagggtcgtccgacaggataacgcaaaaaaaaaatcttcttcagcggccaaagccaaatcgaattcagctaaagccaagccagctgtaaagaaagagcagccaaagtcggccagtaaagccgcttcaacccaaccgaaagcctcgagctcgacatcgtctgcttccagtgtgcaatctagtaacgcccagtcggcaaccagcagttcaacgactaacaagacgactgctgccagcggccatcaatacgccactgtcaaggccggccaggggatgtttcgggttgcttataataacggtttgaccactgaacagctgatgcggatgaacgggctaaatgccaattccaagctgtatccggggcaacggcttcgggtgcggtagctttaaagaatcactcaaaaataatgtcaggtaaggaatgttagaatgcgaaaaaatggattacaagtagcaattgatgggccggcctccgctggtaaaagtactgtcgccaagcgggtagcaaagcaatttcactatatctactgcgataccggtgccatgtatcgggcaattacactgcaggcaattcgtcagggcgtctcctttgacgacgttgacgagatcggcaaaattgtccatgcctcaaaaattacttttgaacccagtgatgacggacaaaaggtcttcattgacggcaaagaaattaccgaggcaattcgtcaagaagatgtcaccaattcagtttcggcagtcgctgccattggcgaagttcgaaagcagctcagtgctcaacaacaggaaatcgctaaagacggtggcattgtcatggacggaagagatatcgggacggccgttttacctgacgccgaagttaaaatcttcctgattgccagtgttgccgaacgggcacagcgccgatataaagaaaacattcaaaaaggcattaatacccctttggatgaactacaattggaaattgaagccagagattataaagattctcatagaaagatttcaccactaaccaaagcaaaagacgctgtagaaattgatacaacgtcactttctatcgatcaggtggtttcaaagattgccgatgtgataaataaaacactgaaataacaactaattagtcaattgactggtaatattgttcaatttaagataaaattatgattagagttgtttcaaggaggaattgtttgatgagtgaaaatgcaaataatgataaaaatgatttattaaacgctttaaacagcgttaatgaagtaaaggttggcgatgttgtcaccggtgaagtattggccaaagatgacagtcaacaattaatcgtgggtattgaaggctccggtgttgaaggcgttgttcccccacgtgaactttcgtctgaccaaaatgttgacgatatcaagcagggtgacaagctcaagttggttgttacttctcgaatcggcagcgacaaggaaggcggcagtttcctgctttcttcaaagcgtttggaaacccgcaaagtttgggatgaattggctgaaaagtcaaagaatgatgaaacgattactgccaaagtcagccaagctgttaaaggcggcttggttgttgatgccggtgtccgtggattcgtgccagcttcaatgatttctgaccattacgttgatgatttaaaccaattcaagggtcaagaacttgaattgaagattattgaaattgatccagttgaaaatcgcctgatcttgtctcacaaggcaattgttcaagctgaaaaagctgaagaacgtgaaaagttaatgcaaactcttcacgaaggtgacgttgttgaaggaaccgttgctcgtcttaccaacttcggtgctttcgtagatctcggcggcatggacggattggttcatgtttctcaaattgcttacgaacgtgttgacaagccttcagatgtattaaaggttggccaaacagttaaagttaaggtattatccgttgacttcgaccgtaaccgaatctcactttcaatcaaacaaactcttccagaaccttgggacggaatcgaagaaaaagctccagttggcagtgttcttgaaggaacagttaagcgcctggttgatttcggtgcctttgttgaagtgttcccaggtgttgagggattagttcacatttcccaaattgcccatgagcacattgatacacctgctgatgttttgaaggttggcgagaagattaaggttaaggttcttgatgttgacactgaccgaaagcgtttggcattatcaatcaaagctttgaccgatgctcctgaagaagaagccaagccaaagaagtcaaacaaccgaccatcacgctcacggaagtctaacgaccgttccatcagtaatgcaccggaagaagaaaccggctttactttgggcgatatcattggagacgaattgaagaagtccggcaacaatgatgacgatgataacaaataatcaattattttaatcatgaaaaggggctggaaacaaaacgcaagttttgtcccagctcctttctttctgaattaaccaagcaaaggagggatttacatggcattgccaacagtggcttttattggccgcccaaacgtgggaaaatcgactatctttaaccgcattgccggtgatcgaatttcaatcgttgaagataccccgggtgttacccgggaccgtatttattctcatggtgaatggctggcaactaaatttgcaatgatcgatactggtggaattcaaatcagtgatgcaccatttgcaacccagattaagagtcaggccgaaattgccatcgacgaagcggacgtgattgtctttatcgtcagcggtaaggaaggggttaccgcagaagatgaacaagtcgccaaaattctttatcgaagtgacaaaccggttgttttagcggttaacaaggtcgataatcctgagagccgtgaagatatctatgagttttattcactgggatttggcgatccaatgccgatttccggagtgcatggtctgggattgggagatctactcgacaaggttgttgaaaaattcccaaagaccgatgaaaagacggataacgatgatattcggttcagtattattggccggcccaatgtgggcaagtcgtcactggttaacgccattttgggtgaagaccgggtcattgtttcagatattgccggaaccactcgagacgcaatcgatacccgctttgaggcggatggtatcaagttcacgatggtcgatacggctggaatcagaaaacgcgggaaggtttacgaaaacactgaacgatatagtgtcatgcgggcgatgaaagccattgaccaaagtgatgtgatcttattcgtcatgaacgccgaagaaggcattcgtgagcaggataagaaagttgccggatacgctcatgaagctggaaaagcaatcatcacggtggtgaataagtgggatacgctcaaaaagaccaaccacacgcaacaggactttgaaaccctgatcagaaatgaattccagtacatgtcatattcgcccatcattttcgtttcagccgttactaagcaaagaatcgaaaaactaccggcattaatcaaacaggtttatgacaatcatgagaagcgtgttcaatcctcagcactcaacgatgtcattatgggggcggtcgctgttcatccaaccccaacggttaatggcaaacgactgcgaatttattatgcgacccaagtcgtgaccgggccaccaacatttgtggtgtttgtgaataatccggacttgatgcatttttcttatgtccggttccttgaaaaccaaattcgtgataattttgactttaccggaacaccaatcagaatcatcaaacgcagccgaaaatagcccaaaaatcagcaattcttaacaaaatcttgatttttcggcgtttatcgacactaaattgggcaaaaccattgcaatgacggcattcttatgctatctttgaaaaagaaatgatgttggcaaacggcgttatttcagcattccggatttgtgagaattcgacttgcaatggtttacatacctatctttgagggaggtgaatacactcatggcaaataaagcagaattagtaaccaatgttgcagcagcaactggtttgactaagaaagacgctacatcagctgtggatgcagtatttgaatcaatccaagctagtttagcaaaaggtgacaaggttcaattaatcggtttcggtaactttgaagtacgtcaacgtgccgctcgtaagggccgtaacccacaaacaggtcaagaaattcaaattcctgcaagcaaggtaccagctttcaaacctggtaaggcgctcaaggatgctgttaaatagtattcatctgttaagccagaacggcatttgtcgggctggctttttttatacactttggaggacaaatatgagctattcaaaaactgctttagaccaacttgaaggcggccaaattgatgattttaagaaatcatttcagcaagctttggatcacgattcggatgatttgctgtactcattggccgaagagctgtattcactcggcttttcaaattactcaaatactatttacgaaaaattatttaaaaaatatcccaacgatgacggtctaaaaatcaatctcgccgaacttgccattgatgatgatcaagacgacaaagctctcaattatctgtcacaggtttcgccgcagtcggacgaatacgtccgttccttgatggttgcggccgatctgtaccaaacccagggaatgttcgagattagtgaacaaaagctcttagaagcccaaaaattggctcctgatgaggatgtgatcaagtttgctctggcagaattttatttcacgactagaaactaccgcaaagcgattaatttatatttagcactaatcacctctggtacgttggaaatgtcttcagtcaacctggttgaacgtctgggtgtttcctatgccgaaattggtaagtttgaacaagcgatgggttatctggaacagatcaagccgattaatatgaacgccgatgttaaatttgaactggcattcacctactttaatttgaaagagtatcaaaaggcaattaaagccttcgaggatttgcgtgattcagatccccagtacagttcactgtatccatacttggccgatgcctatgttaacctcaaacgggttgatgaagcattaaaggcgatccaagaaggaatttccattgaccaatttaacgaaaaaatctggcagaaggccggccaaatcgcggaaatggcgaacgaagacgatttagccttgacctatttccaaaagggccatgagatcgcccctgacgacatggaaatcctgaccttactatcagactggtacgttgcccacgaacgctacagcgataatctgaagcttttagaaggggtttttgaagaccacgtcgtcgatgcccatcttgcatataatttggcactgtcttatcaaaataccggtgaaatcaaaaaagccgccaacaattacgaattggccgccaatgaactttccgataatcccgattttcttaaacacgccacgctgttttaccgcgaaatcggcaaaccggatctcgaaaaacagtccttgaaaaaatacttggatttggtccccgatgacatggaaatggcagaattgtgggatgaaatgtgattcacgatctgcaattaaacatcagaaaaaggtcaccagttagggatctcgccaaagttaaagtaaaccttagtgggatagcccaaatgggtgaccttttatcatacatataaactattgcagttctctagttctatagcagtttgaatcgctttggccgtttataagtgaagccttcaccgatcgcctcgttaacttcaataattgaaataaaggcctcttcatcgattgattcgaccagcttttttaaagtgtgcagttcgcttggggagaccacacaatagatgatctgtttggagcggtgggaataacctccttcggcattcaaaaaagtgacgccgcgattgagctcgtcttggatggcattggatattttttctgattcgttactaatgattaagatccctcgagccgtgtaagcgccgcgttgggtgaagttgacgatcattgaaaaaatccagacgtaaatcaacgtatatgccatctggcggacgtttaaataaatgagtgatgacagcaaaaccaagacatcaattgtgagcagcgtttggcccatttgaacacctttaaaccgctcgaacaagcgggcgacaatatcaacaccaccggttgtcccgccaaaacggtaaacaattccacagccaaagccaccaaataagccggcaccaattgccgacaacaacaggtcatgatcgatattaatcacgattgggacccgctgccaaatccataaaaagattgccagggcaattgttccgtataaggtataaaacatatctttctttcctaagtagcgataaccgatcgcgaacaggggcacgttgaccaagatggtcgaataggccgggtcaatgtgaaacagggcccggagaatcagtgtgataccggtcacgccaccatcggctaaatgattgtaaatgttgaagaagacgattccaaatgaataaatggcggttccagccgcgattaccagtaaatcaattaacgaaatatctaatttgaagcgactttgcttttgtgccatcgtttttcctccctgaatgatctgacaactcatcatagcaattctaattgacaattggcaatcatttcaccgaactttttgtttcaagcggaaattctgttaaaattacaacaggataaatattaaatggatggcgattattgtgcggatggtagaaattccaaaagaattccacgaagcattaccaattttacaaaagattgaatcagcgggctatgaagcctattttgtcggcggttcggttcgagatacgattttaaagcggccgattcacgatgtcgacattgcgaccagcgcttatcccagtgaggttaaggcgttgtttaaacgaacggttgacacaggaattgagcacggcaccgtcatgattcttgatcacgggactgggtatgaagtcaccacttttcggactgagtccggctaccaagattaccggagaccggatcacgtgacgtttgtgcgctcactgaaagaggatctcaaacggcgggatttcacgattaacgctttggcattggctgagaacggacaggtcactgatttgtttgggggccttagcgacatgcgaaaacacataattcgcgcggtcggcgatcccaatgagcgattcaatgaagatgccttgcgcatgatgcgggcggttcggtttgccagccaattggacttcaagattgaggatgccacactggctggcattgcccgccatagccagttattggcaaaaattgccgtggaacgctcccacaccgagtttgtcaaaatgatgctgggatcagacgccaaccacggcctcaagatcatgattcagacgaatttatatcaacacgtcccgatactaggtgaacatttagttcaactcagacaaatcgccgacactgatttcaccctgaccaatgaagttcaggtttgggcccttctggcttttaaattcggattcaacagccaacaaattacccgctttttaaaaagatggaagactgccaataaaataattaatgatgttatacttacggttgaattacttttcgcaattcaacgtggtcaagtgactaatttaaccctttatcatgccggaagtgaaaacgtcgacaacgcaatcgcagtgtttgcggaccagtcgaaaactactggactatctgaacgttataaccgacttgccattaaaaataagcaccagttgaagataaccggtggtgaattaattaaaagaggggttttaaaacccagtccacagcttggccaggttttgaattatcttgaacaaaatgtggttgccgataagatcaacaatgaacctgaagatcttgttcaggcagctatcgactttttaaatgaggactgataattgaatggaaacaatgcgcgttgagaacttagcaaaaacatacggtgagaagacgctttttgataagctgaattttattattaatgaacacgaccgaattggcttaattgggactaatgggactggaaagacatcgttattgaatgccattgccggcattgaccatgactcgacaggtgacattattacctcgaaatcttacaccatcggttatttaaagcaggatccagaactggacgagagtctgtcaattatggatgccgttttttccggatcgcaaacggtctatcgaacaattcgccattacgaagctgctttgaaagattattcaacgcatccagaggacccagaagcagccaaacgatataccaaggctgaagcccgaatgaatgaagaagacgcctggaacgcgcaaagtgacgttaaaacgattttgacccagttgaagattaccgattataaccagaagatttccgaattatccggtggtcaaagacgacgagtggggttggcacaagttctgattcaagcgcccaacttactgttgttggatgagccgaccaaccacttggattttgattccatcgactggctggaaaattatctggcggcttataagggatccctgattgtggttacccatgaccgttattttctggaccatgttgctaacaaaatctgggaactgtcatttggcaaactttaccagtatgatggcaactatcaagattatgtccagcaaaaagcgacccgggttcaaggtaaaattcaagccgagcataagactcagcagctctacaaacaggaattggcgtggatgaagaccggtgcgaaggcccgttcaaccaagcagcaggcccgcattaatcggtttaatgacttaaaggaaaacgtcggtaccttacagcttgatcaggatgtcaatatttcccttggccagacccgattgggtaaggaagttcttaagatgaaagatgccaatttaaccattgacggcaaaacaattctcaaggatttcaatattctcgtccagccgaatgaacggatcggaatcagtggcgagaacggtgccggtaagaccagcctgctcaacgtcattgccggtcggctgaaattggattctggaattatcaaagtcggcgaaaccgtcaaaatcgcctactatacgcaactgaccgagccgattcctgaagataagcgggtcattagttatttgagtgagattggccaacaggtcaccgataataccggcaacaagattagtgttgccgaattgcttgaagaatttctgtttccccgtttcatgcacggcacgttaatccgtaaactttccggtggtgaaaaacgacgcctgtatctgttgaaattattgatgcagcaaccaaatgttttactcttggatgagccgaccaacgacttggatattgcgactttgaccgttttggaagattacatttccaaattccaagggaccgtcattaccgtttcccatgaccgttacttcttggacaaagttgctgatcgattgctgatttttaaaggcaacggtgtgattgaagaacaccgcggtcggttcaccgattacctggcctcattgaaaaagacgtcgaaatcgtctgccaagtcagacagcgggcagtcaacttctcaatcggattcggcaatctcaagtcaagacgcaaccgcttcaaatgccaaagccaagaaaaaactgacatattctgaaaagattgaatatgatcacatcgaagatgaaattgaaaagctcgaatctcaagttgaagacattgataagcagatgcaaaacaatggctcggattatgataagctggcggatcttcaagcacaaaaggaccagttgtctgccgaagccgataaaaagatgaaacgctgggaatatttaagcgaatacgctgaataattaaaaacagtcacgttctgataaaaaggagaattgccatgttagaagacgcctatttagatcttgcacgttatgttttggaaaatggccacaaaaaaactgatcgaacccataccggaaccatcagtacgtttggctatcagatgcgatttgatttatccaagggatttcctttattaaccactaagaaagtgccatttggattaatcaaaagtgaactcttatggttcttgaagggtgacaccaacatccaatttttattgaagcataagaatcacatttgggacgagtgggcttttgaaaagtttgtcgcttcaaatgactataccggcccggatatgactgacttttctcatcgggcacaaaaagatcccgaattcaacaaagtttatcaggagcaaaaaatgttattctgtgatcgaattgtcaacgacgatgattttgccaaaaagtatggcgacttaggtctggtttacggtagccaatggcgggcctggaagacttccactggtggaacgatcgaccaaatccaaaatgtgattgatttaattaaaactcaccctgattcaagacggatgatcgtttcggcatggaatccagaggatgtgccaacaatggccttgccgccttgccacaccttattccaattctatgtcaacgatggcaagttaagctgccaattgtatcaacgttcaggagatattttcctcggcgtgccttataatatcgccagttacgccttattgacctccatgatcgccagagagtgtggattggaagttggtgattttgtgcacacctttggggatgcccacatttaccttaaccacattgaccaagtcgaggaactcctttcccgtaaacctcgtcaggcacccgaattgtggctgaatcctgaaaagaaacatttggacgaattcgaaatggctgatatcaaggtcaaaaattacgacccatacccagtcattaaagcgccggttgcggtttaggaggaagtcgatgttagcttttatctgggctgaagacgccaacggtttaattggtgccaatggtcaacttccttggcatctgccggacgatatgcattacttcaaagaaaccacgatgggcaatacgattatttccggatcgaaaaccttccgcagttataatcggccactgccgggtcgtgagaatattgtggtttcacaccaaactgattttccaacgggcatcaaagttatcccttcgattgaacaactgtgtgacttgattgctcaaaatcccgataaacaatatattgtgaccggtggtgccaatctatttgcccaattacgttcaaaagtcgaccggctttatcgcacgaagattgaagctgaattttccggtgacacctatatgccagccattgactattctttatttgaattgagcaaatcggtcgttggtgttgttgacgccaaaaataagtatccccacacttttgaagttttcgatagaaaataacgccggcataaatgcttatgaatctttggcagaactttgatataattgtcgttggactatcaattaattattaattttgtaaagaaacgagtggcgtaaatggcaaaagtaaaaattgtgacggactcatctgcccagttgacagatgaagaactcaaacaatacggcattacaattgttccattaacagtgatgattgatgatacggtctacgttgatcgtgatacgatcaccaatgaaacctttgttcctcaaatgttggcggctcacgatctgccaaagaccagtcaaccaccagttggtaaatttgttgaagcatttgaccggttgggtgaagacggcagccaaattctctgtttgaatatgttggccgccatcagcggcactgttcacgcagccgaacaagcagccacaatcagcaaatccgatgtgaccgtggttgacagtcaaagtaccgaccgcggcttgggctttcaagtgctcgaagcggctaagctggcccagcaaggtgccgacatggataccattttagccagagtcaatcaggttcgtaataacaccaagctttatttatgtgtcatgactctggataatattgtcaagggcggtcgattgcatccgattgccggggcaatcaccaactttttaaacattaagttggggcttcaagtcactgacggcaaacttaaaattatttctaaaggtcgcggcgataaatcgcttaaaaagtttttcaatggtattattgatgaaatgaaaaacaccgccgctgttaagtcgattggcgtttcatacgtcactgaaactgaagtattaaaggacactgttcaaaagcttaaggctgactttcccgatgcatcatttcttgaacgggtgacgtcaccgaccatttccacgcataccggtaaaggggctttcgcgttgatttattacagtgatcccgagtaattgcagatctgaaatattgcttaaaggggcgaggcaaagcggctgttttgttgtcaccccttttagatttgatcaccatttgagaggttgtttttgtgagtcaaaataaacatgttaaacagacacagcatcattttcgttggattatcggattgatcggcctgatcgtgattggggcagccgcatttttcggctaccattatttcaactcggccaaagaaacactgccaagagaagttaaattaacggctgttggggattcactgactcaaggggttggcgatccgaccaacaaaggcggctatacccacttgattcgccaaaaagtgattcaaaaaaatcccaatgttcacctgtccactgccaactatggcatttcaggggaaactactaaccaaattaatcatcgggtggtttattcaaaacggctgcagcacagcatacgagaagccgatgtgatcacgattaccactggtggaaacgatttactgaagtttttgaaggcgaacgttgttggcttgaacaaacatcagttgaaccagaaattgaccagttattgtcaaacatatcaagctagggttacccggctattccgaaatatccgccacttaaaccgtcgggcaccgatttttgtttttggcatttacaatcctgtctacgtttacttcccccaggtcaactacatcaacgacaccgtggctcataccaaccagattaccaataaagtgatccaccaacagcacaggatgtactttgtctcgattaacaaaccgcttacagacggtcagtttaccactgccaaatccagaaaagctttggaagaaaaggccgctgccagcattatcgccgaaaatcatgattcgcctgccgacattgagcagttattgagtggccaacctgcccagtcaaataaatatctctcaaatgatgaccatttccacccgaatttgaaggggtatcaaattatgaccaatcgcttgtattcccaaatggccaagcacatatcctggttaaaggagtgatccaaaatgagaaaagcctccaagcagacgaaatcccgcaatccttggaaaatcgccttcatatcgttaatcggcctcctggttgttttagttgccggcatgtttttggcggtttatttatcgtcatctacaacgaaattggtaaatcaaaagtcgaccaaccagtcggagccaatttccgccactatcaataaagctcaactcaatcaactatccaattattatttagataagctgcagaagggccgaccttcgcaatatcactttgaagtcgccaacgaagggattgtctatggctcactgactttattaggttccaacgtcgattattcactgaccttcgacccgaaagtgatgcccaatggtaatattgaacttcacgctaataagctggcactggggaagttcccggtcccaatcagttttgttttaatgtatgtcaaacaaaactataaactgccaaagtgggtccaactgattcctaaagataaaacaatcaaacttgatataattcacatgaacggtaagaatgggattaattatcgggcccggaccatcgatttgaaaggccaaggaaaatttgcctttgagattcttttgccgaccactgacaaggaggactaatatgcacaaaacgttctaccaatatttaatgaccaaacgcaaccccggaagtactgatccagaggctgaatttgccaacaacgcattttatgatcagtcatttcccaaacaagaagatgagtttgacgcgttatccaagtatttagaagaaaatgcttcataccttccgaccatggaaatttttgattccgtgtggaaggaatatcaagaaagcttttaggaagtgaaacaatggcagtaacaattcaatggtttccaggacacatggccaaggcaattcgtcagtttgaagaaaatctttctttagttgacgtggtatttgaagtgattgacgctagaattccgctgacttctcaaaaccctgaaattcgacgaatcagtgccgataagccgcatctttatatcatgacaaagcgtgatttggctgatcctcaattaaccaatgcctggctgcagtattttgctgaacacaaccaaccggcaatcgccattgatgccaaaaccaaatttggcatcaataatgtgatttcggtgatttcacccattttgcgtgacaaattgcagcgggaacaggataaaggcatgaagaaacgaccgatccgagccattagtgttggggtaccgaatgtcgggaaatcaactgttttgaaccgattggtcaaccgtcgagccgctcaggttggcaaccgtcccggtgtgaccaaggggcaacagtggcttaaatcgactgataagttggaattactggatacaccgggaattctgtggccaaaattttccagtcaagaagttgccgacaagctggcattgaccggtgcaattaaagagagcgtttatgccagtgacgacattgccttgtttggcttaaagcagatcagacagcttcacccggaaggcctcaaagaccgttatcacttaactgacgacgatttggatttgtccgacgttgacctgctgttacaaattactaagaaagtcggcatgcgcgatgattatgaacgtggctccaatcggattattcaagatttccgtgccggcaaaattggtcgttttactttggatgatcctgaaacggtgagtgacgatgaccaagctaacaattaaagacgttaaacagcttttatcccagatgtctgatctcaccgatccgcggttgattgagttaaaggctgacccgcgaaaaggggttcaattggcaattcagtcaacagaaaaccgcctgcaaaagcaggccagagccctggatgaatttgaacagcggtttaaatatgaacggtctttttggcatcaggggctgcaatatgttgccggtgtggatgaagtcggcagaggtcctctggcggggccagtggtggctgctgcagtgattctgccgcacgactttgacctggtttccgtcaatgattccaagcagctgacaccgacccaacgcgcagagttggccccgctcatttcagctgaagccctgagcgtggggattggatcggtggataatcatgggatcgatgagttaaacatttaccaagccactcgtgttgccatgaaacaagctgtggaatctttaaccccacagccggatgaaatcattgttgatgccatgcagattcccgttccgattcggcaaaccagactgatcaaaggtgatgccaagagcatcagtgtttctgcagccagcattgtcgccaaagtctatcgggaccatttgatggacgagtacgccaagcagtacccggaatacgattttccacacaacgccggctatggaacggccaagcatttagcagctctcaaggaactgggaccaacgccgattcatcgaatgagttttgccccggtgaaaaagtttagccaaaaataaatatgttttacgtagataactcttaaaaggatgatgacaatgcttttaagagattttttgttaagaatacatttatgtaagggaatcggcatgattggtaagtcaaaaatttatacttgggtaaatcaggtcgactggcgggatgatcaactgccgacctcaggattcttggctgccgtcgctcaactaaacgttaagaacaccgctaacttcaaaatcagctatcaacagttaatgcgaaacgacgacaaagtggaccagctggtcgatggtgaacagtggctgagcattgcagatgctgaatatccacttcaattgcgagaatcgtttgcgccgccgttagtgctgttttatcgcggagatttgtcgcttttatcccagccacttttaggaatcgttggggcgcgggactgcacctcatattcagttgaaatcctaaaaaatttgattcctggaagagtttccaatacaatggctattgtgtcggggctggctaaaggggttgatacgttggcccaccaatgtgtcatcgccaaccaaggtaaaaccattgccgtgattgggacagggttggacgtgtgttatccatataccaatcaggaactacaagcaacgattgccgccgaccatctgttaatcagtgaatatcccaatcataccaagggctatcgaaatcactttccggaacgtaaccgcatcattgccggattggttcaaagtgttctggtcactgaagccaaaaaacattccggtagtttgatcacggccaatttagccctgcaaaataatcgcaatgtcttagccgtcccggggtcaattatgatgccgctttccgttggtaccaatgaattaatcgctgctggcgcaaaaccggttttacgtgagttggacatcttggaggactactttcagacgcggatttaagggtagtgagttgacactttaaaattcctgcaatatgatgtggtagatttgtaataaaaattcctacaataatgtaactaaaaataagcagttttgaggggagaaaatatggcaacttctacaaaaacgaaaccaaaagccaaagcaaaatcaaaaactaagcgaaaatcgcctaaaaaaaatctagtcattgtggagtcacctgccaaagccaagaccatagaaaaatatcttggccgttcatataaggtggtcgccagtaaaggacacgtgcgggatttgcccaagagtaagatgggcgttgatatcgaccatgattatgaaccgcactacatttccattcggggtaagggtgacacaattaaagaattacggtcagccgctaaaaaggccaaaaaagtgtatctggcagccgatccggatcgtgaaggggaatcgattgcctggcatcttcagcacattttggatttagatcctaacgaagataaccgagtggtatttaatgaaatcaccaaggatgccgtcaaagaatcattcaagcatccccgaaatatcgatatgaatctcgttgatgctcaacaggcccgacggattttagaccggttggtgggatattcaatttcaccgcttctctggcaaaaggttaaaaaggggctcagtgccgggcgggttcaatcgatcgccctttggctgattattcaacgcgaaaaggccatcaaagactttaccccagaagagtactggtcaattgattctgaatttaagaagggccgcagtaagttcaaagctgccttttacggcttaaacggtaagaaaaaggaactgccaaataacgaggcggttcaaaaggttctgcagcagttggatcccaaaggtgactttgatattaccaaggtaacccgtcgtgaacggaagcgccaaccgcagccgccatttaccaccagtacaatgcagcaggaagccaaccgaaagctcaacttcagaacacgaaagacgatgatggctgcccaacagctctatgaaggaattaatattggtaaagagggtagtcaaggtctgattacctatatgcggaccgattcaacccgaatttcagtcattgccaaacacgaagcgtcccaatttctacatgagaaatacggcgccgaatatgcggcaaccaaaccaattaaaggcaaattgcccgagggtgcccaagatgcccatgaggccattcgtccgacttccgttttcagaacgccggccagtttgaaacaatatctgacccgcgaccaatttagactctatcaaatggtttggtcaagatttgtggccagccaaatgactccggcaatcatggataccatggcagtgacaattgaacaaaataacgtgacctttaaagccaatgggtccaagatgaagtttgatggattcttgaaggtttatggtgatagtaaagaaaaggacaacttgttacccgatttggagagtagcgatgttgttaagttggtcaagaataatccggaccagcattttactcagccaccggcacgatacagtgaagcaacgctgattaaagcccttgaagaaaagggtgttggccggccatcaacgtactcaccaaccattgatacgattcagcgccggtattacgttaaggaagttggccgtcgatttgagccgactgaattgggggaaattgtcaacaagattattgttgaatacttcccagacgtggtaaacattgacttcactgcaaatttagaaggcaaactggatcaggttgaagaaggtaaagagaactggatcaaattagtcgatacgttctataaaccattttccgacgaggttgatgctgcaaccaaaaatatggaaaaggtccaaattaaagatgaacccgcaggtattaactgtgaaatctgtggcgctccaatggtcatcaaaatgggccgttacggtaaattctatgcctgttcaagattcccggattgtcgcaataccaaagcaattgttaaggaaatcggtgtgatttgtcccaagtgtcataaagggcaggtcattgagcgaaaatcaagaaagaaccggatcttctatggttgctcaagatacccggattgtgatttcgtttcttgggacaagccaatcggcagagattgtccaaaggatggtcacttcttagttgaaaaacgggtcaagggcggcacacaagtagtttgtccaaacggcgactatgaggaaccggcacaaaaataagcatgcgacgagccctgtttaggacccggagcataagtgaggagcaccaataatgaacgaattttgttcattgttggtgctcctcacttatgtagtagggtcctggggcgtaggagctgaactcaaaggccgaaggaagcacggaataaactaactgctgtatccctgtaaaagcaatcttgaatgagtcctgatgaacgttttttgttcatcgctggttgtttttgtttgtgcagtaggggtcaggggcgtcggagctgaactcaaaggcagaaggaagcacgaggtaaactaactgctgtatccctgtaaaagcaatcttgaataaatttcggggcacgaattttgttcattgttggtgctcctcactcaggcagtgtcccttggccgtcggaatcatttctgttaaattgatccctttgacagaaagcgggcctcgccgcaatccccatttttgcattcaacggtcttttgttccacaatgcacaaaagggtgtaaaatcaaggtgatagaaagacaaggggaggcttcaaaatgttttcatcaaaacacagtagttgtacaactattctagtcggcaagaaggccagctatgacgggtcaaccatcatcgccagaaatgaggatgccggagatgccgttaatccaaagaagtttgtggttgttgaaccagaagaccaaccacgcaattatcagtcaaaattaaccaagtttagtgttaaactgccagacaatccattgagatatacctcagtgcccgatgctgtccctgacaagggcgtttggggcgaggcgggcatcaatgcccataatgtggcaatgagtgccacagagacgattacaaccaattctcgggtgatcggtgccgacccatttgaaaaagacggccttggcgaagaagatctgttaacaattaccctgccatatatcaattctgcccgagaaggggttcaacgagtgggtaaactgcttgagaaatacggcacatacgagtccaacggaatcctgttttcagatgtcaacgaaatttggtacatggaaactgccggcggccatcactgggtagcccaacggattccagatgatgcctatgtcatcgcgcccaaccagacaggcatccaagagatcgatttcgatgatccagacagctttatgttctcaaaagacttgcgtaaatttgcccaggagcaccatctcaacccaaccagtcactttaacttcaggaaggtctttggctctgatacccagctggaccgtcactacaacacgccgcgtgcttggtatggtcaacgatatttcgatccggaatcagtgaaggataagacgccaatgagcaatgatttgccgtttatctgccacgccaaccgcaagattacgattgaagatatcaaattcgttctgagctcccattatcaggacacgccttacgatccatttgcgccgggagctgattataagaccgttccatatcgaccaattggcatcaaccgcaaccaagagctgtcaatcttgcagttgcgtccaggaattccttcggcttattcagcaattcagtggctgacatttgcctccaatccgttcaacacgttgacgccattctttaccaacgtcgtcaatacaccggactgctaccgtgataccaccgagacgctggacagccacaacgcctattgggcaaaccgcctgatttcattgattgctgctgatcattatcaggccttgatgcaagacattgaagactatcagcttaaagaaatgggttatgctcacgagcgaattgcgcaagttgataagcagatggccgaaaaagaggcttccggctcacacgtcgttcgagcccttggtcaagccaatgcccggactgctgatcacgtcatgaaagcgaccgaggatctgctgacaaaattggttgttaaagccagtcaggatcttccaggctcatttacgcgggaacattactaaactaaatcagtcatcataacgaaatgaagccggctcacaaaattgaatttgtggccggcttcatttcgttattcaatttttaagacagattatcttactgttggaggcgagtcgttataggttcgtatcttgggtaaaattgattggtgagaggtctgttgaattggtgatgatgtcactaatcaattggttgtaagcatccaggcccatcttggcattggcaaagttgactttggtcagataattggcgagttcgacattggacaaaccttgaagtgaggcatcagcttgtttgactgcttgttggaaattcactcgcagtttggctttggtgtcatttaatttgggcccgaatttgacgtaatgcgggtcaactaagacaccggcaagcttgtaagtccaataggcttgattgggggcatagctgcctgaagcattctgataggattttggcgtggtgtttgcgccggcataaaatggcacaaaagaactttgagcagcgacgcccattgccaaccattgaatccctgcagcaggagtgggcatatttggccgaatttggaggatgtgggcctcttgcgtcttggcgagactaattggtcgatagaggtgcttgtcgtgctcagagccctcgccaatggggtcaaacggtgtgccttgataatgagagcttaagaaatcttcaacgtcaaacaagctcagtttgcggttggcatgattgatgaacggcatttcctgactggttggttcaaaatttagttccggtgagaacatttttaagccgtaccatacgcggggtgtgttataaaccgtgtccgacaagtcagcggtaccaaagattttacggaagttgaaggttttcccggatggatccgggttcaagtgattttcggagacaaaccggcgaatcttgggtgaccacatgaagttgtcagggtcgttaaaatcaacgtcttgaatggcgctttgattggcaatcaccgcgtaaccgtcgtctggaatgcgttgggcagcccagttgtggccgccgccggtttccatataccaagcttcattcttatcggcaaacaaaatgccgttggattccgatgtcccgaagtattccacaatttggcccaatcgagcaattccttcacgcgcggttttgacgtaggggaggacaaccgtaatcattgcttcttctccaatgccatcttcgttgagcggatcggcccccaaagccagctgattggtataggtgctctcggtggcactcatggcaactccaaactcattaaaaccattttcttcaaacaggccgaacttgtcagtccattcaggggtggcagaatattgaaagcgcactttaggcagggttaacttgaagccgttgtctttggatgagaaaaccggggcttcactaaattcttgatgctcgtggatgacataattctttggccacgaggatttactatcttcgtttcgggcaatcataattgacccgtcaatgctggccttcttgccaacaatcatactggtacaggcggaaaagtttttgtatggtatcattttaaaatctcctattcgcagttaaatgttactccaattattgtatcatctttgatccataaacggtcctgacacgtccaaagtgccatcaagatattgcaggcaaaaataatttaaggtatacttttgccattcgaaacaaatggaggaatcaaaatatgccaattgtagatattcatttaattgccggccgttctcaagatcaattgaagggcttggtggaagacgttaccgcagccgttgttaaaaataccggtgcccctgcagaacatgttcacgtaattttaagtgaaatggaaaagaaccgttatagcgttggcggtgtgctcaagagtgacgaaaaatagtcgcaaataatttggaagtccgccaggcaactgttgcgggctttttgtttgcgtttaattcggggatcaatcatcaaattcttttactttgataaagtttatctcaaggttggtttgccagtcgatattattgtatacttaacaaagaaaaagcgtttaaacgcacgaataataggaatggagacctttacatgaatgatcagcaatacataatgtccattgatgaggggacaacaagtacccgggcaatattgtttaataatgatggtgatatcgttggtaaagcacaacgggagttccaccagtattttccaaaatctggttgggttgaacacgatgccaatgagatttggaatgccgttcaatcagtgatctcagaagccttgattaatgcggatgtccaaccatacaaggttcggggaattggtgtgaccaaccagcgggaaaccacggtcatttgggataaaaataccggcgagccgatttatcatgccattgtttggcagtccaaacaaaccgctgcgttagccgatcagctcaagcacgatggttatgatcacgatggttatgatgatatgatccatgaaaaaaccggcttgatcattgattcctacttttccgcaactaagattcaatggattttggatcatgtagacggcgctcgccaaaaggccgaaaatggcgatttattgtttggaaccattgatacctgggtcctttggaagttgaccggcggcaaggttcatgcgactgattataccaatgccagtcggacgatgctgtttaacattcacacgttgacttgggacaaagatattttggacctgctgcacattcctgaaagcatgctgccggaagtccgctcatcgtcagaaatttatggttatacagctggttattccttctcgggtgttcaggttccgattgctggaattgccggtgaccaacaagcagctttgtttggccaaatggcgctgcagcgcgggatgatcaaaaacacttatggaaccggtgcctttatcgtcatgaataccggtgaggagccgacactttccaagcggggactgttgacgaccattgcatatggaatcaacggcaaagtcaattatgccttggaaggaagtattttcgtcgccggttctgccattcaatggcttcgagacggaatggaaatggttaagtcatcccctgactcggaacaaatggcgattgatgctaaaagtaccgatggcgtctacgtcgtcccagcctttaccgggttgggtgcgccctactgggatcaggatgccagaggggcggtctttggcctgactcgtggcacgaccaaaaatcagtttgttcgagctacgcttgagtcattagcttatcaaaccagggatgttgttgacaccatggcagctgaaaccggaatcgatttgaagtcgctggcagttgacggtggggcagctaataacaattatctcatgcaattccaagctgatattttgggaacgccaattcagcgggcctcaatttcagaaaccaccgcgctgggtgcagcctacctagcaggcttggcagtcggcttttgggattctatcgaagaaattcgcctgaccgttaaatcacgcgatgcttttgaaccgcaaatggacgagcagacacgcacaaaactgtataccggttggcagaaggccgtccaggcaacgattcagtatcatcccgacgaagactaatcatttatcattttttcgttgtgagttcactgaccacttttgattgctcaaacttacgacaattgaccattaacaaagaaacgcagtcactccaacatttggaatgactgcgtttctgcattaaattatgggattaaatcgctgttcgtctcgatggttggtttttagttctcagttaagcaccaaccgcaatgtccagtcgatcttggagataatgggcaacaccatcttcgtcattggtgaatttcgtgacctcatcggactggcccttgattttatcaatggcgtttttcatcgcgacaccggtgcctgcgtattgcatcatggtcaaatcgttgccttcatcaccaaaggcaataatgtctttttgcaggatgccatagtaatcggccaaaaatttaaggccggtggatttatggacacctttcgtggcgatttccacaattggattggggccgccccaaggggagacttcaacctcgtcgccaaattgatgttcaacgaagtcaatcaacccctgcttgagttcgggttccacttgaactgtgatactaatagggttttcttttaggcttttgcgactcagtacctgattggtggccaaggtgctggggaagaagccgaaaccactgcttaatccctggttggccagaaacatattccggccttcaacggcaatcaacgacaggccgagcggtttgctttttgcgagtaattcagtcacaatttctttatcaattgtgtactggtattcacgattccactgttgatgtggtaaaatgccaaggttgccattgaaattaatcattggcgtcgttagctttaaatcgtcataaaaattttcagagagtctattgggacggccggttacgatactgactatgtatccttgctcagcagctgcccgaattgtttcggcagttttggcgctgattagactatcgttatttaaggttgtgccgtccaagtcgagggcgattaatttctttgtaattgtgatcactccttactaacatatccacttataatatccaaaaacacctaccacgtcaattattagtaccaaaaagggagattagaatgaacttaccaactgattttgtgaataagtatcagcaattaatgggcaaatcagaagccgcccagttcattgccagctttgacgaaccgacaaccccgggttttcggcttaatccattgaaagccagtcaaccaattgatttggacctgagtgagcccacggaacactgccaatttggctatcatggtcaggtcagcggcaaaaccgtcgatcatcaaagtggggcggtttacagtcaggaacccagtgcgatgtatgtgggtgaagttgcccaccccaacctgggagaaagggtattggatttgtgtgcggcgcctggtggtaaaacgacccatcttggcagctatctgcaaaataccggcctgctaatcgctaacgagattgacagcaagcgtgccaaagcgttggttgaaaacgttgagcgatttggcatgaccaatacgattgtcaccaacacggatccggaccatttagcagcccaattaccggaattcttcgatcggattttggtggatgctccgtgttcgggagaagggatgtttcgaaaagacccggacgccgtccaatactggtctgtcgattacccaattgaatgtgcggcccgtcagcggacaattttgacccaggcggttaagaatctaaaacctggcggagaattgatttactccacctgtacctttgcccctgaagaggatgagcagatcattgcctggctggttgacacttacggatttgaaattcaaccgattaaaaaatttgccggaatggatgacggtcaaccagattgggctgatggcaatcaggatttaaccaactgtgtgcgtatctttccacatcattttaacggagaaggccattttattgccaaattgaaaaagcctgccaacgcagaaaacgcaaaaggaccgcgtcgcttccgcggcatcagtcgaaatattgaaatgccctccaaagatcagaatcaattgttcaaccagtttgccaaagcaaccttaaagaacgttcactttgacaaattggtggttttcaaagatcatctttactcagtaccggaaaatacgccgaacttgtctggcattaaaattgtccgacttgggttggaaattggcactttcaaaaagaaccgctttgaacctagttatggcttagccttggcactgcatcccgatcaagtcagtcaaaaaatcactatagacttagcggattggcaaaagtacgtgcatggcgatacattccaagtctcaccagatctgaaaaaggggtggtacctcctggtttgccagcaacagccagtcggctttgccaaagttgtgaatggtacggccaagaatttcttccccaaggggctgagatttgcgatgtaaaaaagagttaaatcaccatcagaagattgtggcttctgatttttgatttaactcttttttaataggctaattttctttgctttaaatagctcaataattgtggatcaaggatcaacctttgccgttgtaagtcagcaacggttcggcagttcagcattaacatgattgtttttagtccgtactgccattctctgacatcgtcaataatttcattgtcacttttatggatgatctcatgaagccagtaacctgcaacgccaactgctgaggcacccagtgtgaggcatttagccacgtccagcggtgatttcacaccgccggcagcaataatgcccaaccgatcagaaaaggcgcgggcttcgaatagagactcaacggtgctcagtccccaatccgtcaaataagccatgtcttttgaggaacggcggaagttctcgatggcagcgaaattggtcccgccatgcccgccgacgttgacatacttcactcccaggtcaaccagttgtgaaatagttgcttggctcatgccaaagccaacttctttcacaatgaccgggacaccgacgttggcaataattgcttgaatattgtcaataaagtgaaatccccgatctccttcaggcatgacgagctcttgggcgacgttgatgtgcaactccaaagcatcggcggcgatcatctcgacggctttttgggcatcttcaacgctgtggttggcaccgatatttgccaagacaattccgtttggattggtttgacggacaatactgaaggaatcgcgcacctcaggatcacttaacccaacgctttgagagccgaccgccatcgccaatccacaggcttttgccaccacagcaagtcgccggttgatctctttggtgcgggggctgccaccagacatcgcttcaatataaaaaggggtcgtcagcgacagggagccaagctgagtggttaaatcaatatcatctaatcgatatttgggcagactggcattcacaaagcgaacgccggcaaacgagttgtcgacaggttggtagaacttttcagccagggacacatgttcatctttacgatgggaatgttgtgaagtcataagctactccttgtcaagatcgatgacgggatggactttaagggccagctgctggatgccattttcctgccaatgggcgatcattgaatcaacatcggtatctttgtcggcaaccacgatcccgcagtcaccgccaccagctccggaagatttggcagctgcagcatggtcgacggcaatgtcgcacatcttcttgagaattggggtttcaatcggcactttggtaaaagcggccaaatgttgaaggatttcccggttacgggcgatgccctctttgatgaccgacaggctgccatttttgaaaccgtcaatcaattcgtccaggcaggctttgctttcggccagaaaatggatgtaagtctcatgttgattgctcttttgaactgcaaccttgtcaaccaaatgcgaagttgaggccggagaaccggtccagccgataatcagcttcaacccgtcaggtggcgttaattgcgtaatttttaaatgcggccaaggcttgttgactaaggaaatcaggtcttcctgcattcgagcagccatgagccagctgcggtcaaatgaacggtaagcgatccagccgccgtatacactggcagcgatatctcccaaagaaccgtttccttggacgtccaaatgggcaattgccgatagtttgaagagtttactcttagtcagcggtaagttatagaactgacagagagctttgacggtcgccaccgtcacggcagctgaagaacccaatccatacttttttccgttggggctatccaaatcactattgatccgcagatcatagagctccatctgccggccgagggactgggcatattcctcggtgagctgaatggctgaaattatgtagttaaaagtattgtcacggttatccagaatcatttgatcaccgcgacgacgccaatagaccgaatcttctcggtattgttttgaaacgatactgccataggacttgcttcgagaaatttcgacagttacgaattggtccaaagccacaataatagaagggtagccagtttcgactaccgcgtattcaccggcgatatataattttcccggagctttaaccttaatcaacggatcatttcctttctagtttataaatatttgacacccgggccaggcttggcaacggtcactttggttgggccaaacaggtttgagaaggtatcggtgatggtttgaacattggcttgttgacaaatgactttaatattggggccggcatcgattgtatagtaacattcaatcccggaatgcctgagccgtttaacttcgttcatggcggtcaaggtgtcgccgttgaagtagagaaaatccggatcggcactcagtgttagggcgtgcatccgcatggcatttaactcactaattgtgccaaaacgcgtgaagtcatcatcttggatggcggctttgatattctccagatcggcttcgacgaccttaacccacgttggatagtaaggggaggtggtgactgaaagggccatgccttcccgactggaaatgggtttttgatgcttttcaatggttaatgcaacgatgcagatgtcgttcaaatgagtcgtctcaactggaatggcgtacgaattggtatcgtctgaccctttttgccattccacaaagccgccaaagattgaccggcaggctgaaccggatccccggcgggccaatcgggacaagtccgttaaactcagattcatgccggcggctttgctggcagcggcggccaatgcagcaaacgccgaggcagaggatgccaagccagctgccgttggcacatgattagtcgatttgacttgggcgtttaaatcaattcccgattctcggcggacaatgcttaagaagttgtgaacccgttgaccgctttttccggttaccggctggccatcaattgtaatctggtctttatccaggttggcgttaaatgtcacgctggtttgagtataaaattgatccagcgtcaaagagagactgccagtgtaggggatgatgagttcaggattttgtttgccccaatatttaattaaggcaatattcgtgtgagcaactgctgtaacggtcttatctgacgaggttgtcatgagcttctcctgttgaaaattgataattcttaaatgattgaatccaagtctgagtggcaccggcttttcgaagggcagtcgaaatctgttgagcatcacgttggttcttggctagagcgatgacacagccgcccaaaccactgccggttagtttggcacctaaagcgtgattgtcacaagcaacttgacagaatgtgtccagagtgtggttgctgacgccgagttgggccaggtcacgttgggattgtgtcattagtttgcccagtagcacatcgtcggtggttgccaaagcattgcgagccgtttcggcaatcttgctaagctcgtcaattaatggttgagaactttccggttcgtcgaccaggttatcatgaaccaacgaaacggcctcactggtttttcctttaatcccactatcggcaatgaccaatgatgaggttggcaaattaaagtcaatctgctcgttgatttcgtttcggataaaccaaatcggcatgttggagctggcggtcgcagagtccaggccgctgggattgccgtgggtaatcttttcttcaatacccgctaacttcagcaattggcttctggtcaaattgacctcaaaaaaatcaaaaaaagcccgcacaattgcgattgccgttgccgctgaggatcccattccgcgttcggcaggcagtttgctttggatgtcgagatcaaaagcaagcctttgagcgccaaataaactaacgagatgagtgattaatgttttaacaccccgcagattctccgccatttcactaattgggccgtcaaagtaacgacagtgaatttgttggccggctggaattctttgaatggtcgcaaccacatcaacggagtagattgggatggcgatggcgggcttttcgtaaacgacactatgctcaccaaaccaaataatttttgcgtaactttttccagttgctttatctttcaactttatccgctcactttcaaacattccaattttatcatagttcgctgattcgagaacgttttaacgatatttttagagattcataaataattctacttctttccatggtagattatcacatcttgcttgtagtatgattaaagttagtgaatatttaagaaaagtcagctcataaacagattggtgaatgacaatgaattcaaaaaccacctttgccgtggttgatattgaaacgaccggaacagacatttctgccgataatcggacaattcagttcagctgctgcttggtttccaacaataaaattataaaaaccttcgtgaccgatatcaatccacaacgagaagtccctaaccgaattgtgcagttaaccggaatcaccaacgaacggctgcaaaaggccaaaacttttgaccaggttgccgctcagctgtattccttactcaataatacggtttttgtggcccacaatgtgaattttgattttccgtttctgaactcggaatttcaacgcgtcggctaccccgaattacaaattgaagcaattgacacagtcactttaagtcaaatcctgctgccaacgttatccagttatcggctgcaggatctcagcagttatttcaatatcgaacatgaccatccccatacagccgatagtgatgctttggcaaccgccaagctcctgcttattttactacgacaaattaagatgctgccgaaaatgaccttggaacagatcatcagtgttaatccgtctctgcctcaagacacgatgcaggtttttttggatgccgatgaaaccaacaaaaggcaggtgcacgctgccaaattgcctgatcacctgagaatctcatcaggactggttttacgaaaacaggacccaatcgtcgtgactgatgagtctgataaacagcgtcttcactatccaaaaacaaaaaaggccaagcaaaaactgcttccagacaacttggagtcgcgacttgagcagaataaaatgatgaacttgatctataacaattatgccgatcaacagcatcacgcagccaagaccctcttaattgaggccccaaccgggattggcaagagtttggggtattgtctgccattgagttatttggtgtccgcccacaaaccggcagtcatcagtacttcgacaacttatctgcagtttcagctgcaaaatcagacgttgccaatgctcaacgaggggctgcctttcaaagtcaatagtgtcattttgaagggggccagtcactacattgacctctacaagttccgcaatttattaaacgttcctgataactcgacccaaaccgcgtttattaaagcgcagatcttggtctggctgacggttaccactacgggtgatttggacgaactccacttaaacgtcgaccaaacaccatttgtctggaaaattcagcataccggcgtgaaatggctggatccaaacgaaccgttttatgacgacgactttttgcgttacaacttgaaaaaagcacaaaatgctgacttcttgattgtcaatcatagctatttaattaaaaattggcagtatttcaaggatctgccgaccaaaccctacttactgattgatgaaacccaacagtttgccgaaaccgccattcgtaacaatcaggagcggattaatccgttatcactgacaaccgcaattaacaaaatcttggcagatattaatggaactcacgaagataatatcaaagaaattgtggaagacgacgccatcttggaccacgcgatcgaagcccttgacggcaaactccgacaagctaaggccttggtctcgaccgttacgacgaccctctttgaaatggtcgtcaagggcaaacgactccaccgcaacgccgagttcttcgagcgcttaattccaattaatgagatgaaggcagccaccgctgccaatcaagagccgatcaaccgtctccgcgcgctccacgaaagcttggacggactgctggccactttaaatgcccaaattgaccataatgccggcgcatataccaaccacgatttcttaagcatttattctttttttgaaaactacaatgagttcaatcatcaactacgcttgctcttagcaatcgttgatgttgacgaccagtcaattgagcagcatgtgacgtgggtcaccgtcaataatgtcaaagacgtcaatagcctgacacttaaccgggggattttgaaaacagaagattatctccgcgaccatgtctattctgcctttgaaccggcaacttttaccggggcgacaattttctcttcacgacgttcacagttcatttacaacttattggggattagtcgcgatgattcttcgattaaacgactcaaaagcgacttcaatccaaaagatcaagcccgactctatttggttaccgatcaagacgaccggcaattcgcaaccaattccgataattatcttcaaaaggttgccgacaatatcgaagttatttataagaatgaaccgcggcagaccttggtactgtttaactcactcaatgcgattgaacggacgtatcggctgcttcaggaaagtggcttcacagcgacccattttgttttggcccaaggcgttcatggaacagctgccaaaatcagcaagcagttcatccatcatgaacccgctattctgttaggggccaatactttctggcagggagtcgatttcccaagaaatctactggaaaacctgattgttgcccagctgccatttgatacgccatcagacccttataatcacgccctgtactcgattgagcgcagtaagggtaagaacccattttatagtattacgctccccaaagcgactctcaggctgcgtcagggcatgggacgcctgttgagaaccaaagatgacttcggaaccatttttattttggatcccaggttattatccaagcggtatggcagcaccattctagccaatttacgcaacgatattcctgttgtgaagggttcaattgatgaatgtgtattagacatggttaagttttttgaaagcagaaattaatctgcggttgagcagtccgatatttgctataattagaaataacgaaatttgagaggaagttaccatgcaacggcatcgaagagttaaaaaacaatcatacgttaaaatttcctggatcgttatctcgatcattttgattctctgcttttcgttcttcattatcctgcacacggcggagcggccgatgacaattgcccgcggccagaccgaaacgattgctaaaaagtacgccgggttaacgaaagtcgactcgttttacacctctaatttggggaagacttattattccgtttccggtgttgataacaagaacaaaaatgtttacgtcatcgtcgctaaaaaaggcggcacggtcaacgttatcaatagcagcagcggtattagcgagcagcaggccaaaaatgtgattcaacggcaaaaacacccatcaaaattaaacgggattggcctgacgatgattaagaaccagccatactgggtggtcagctatatgaacgccaagaatcatttgtgctttacgacaatcagcttcaaaaacggcaccatttacaaatcgattgaaaacatctagaaatgaaaggacacttcaatgaaattttcaaaacgggcgatgcaggtcacgccttcagcaaccgtcaaagtttccaatactgccaaggcgatgatcagaaagggcatcgatgtcattaatttgggcatcggtgagcccgattttccaaccccaaaaatcattgccgatgcagcaattgacgctattcgatcgggcaaaaccagtttttacaccccggccagtggtttacctcatttaaaagaagccatcgccgaacgcattaaggaggactacggcgttgtctacccagctgatcaaattagtgtgaccaacggtgccaagatggcactgtacgtgttaatgcaggtattggtcgatgacggcacggaagtcttgctgccacggccaagctgggtcagttaccgccagcgggtcaatcttgcaggtggcaagccggtgattgttgagacggggacggacttcaagattaccactcaaagcttggatgcagctgtaactaaaaatgctaaggtattggtgatcaattcaccgcaaaaccccactggaaccgtgtattccagggatgaactggcggcaattggtcaatgggcggtcttgcataatgtgaccttaatcgctgacgatatttatggcaaattggtctataatcaaaaccagttcgtttcattggttcaaatcagcgatgaggttgctgcttcaactgttttggtcaacggcgtttccaaagcctattccatgacggggtggcgaattggctatttagccggggcgccggaattaatcggcaaggtaaattcgattctatctcattcaaccggtaatccagctacggtaagtcaatatgccgcgattgctgcctttcagtcggaccaatcagccgttgagacaatgcgagaggcctttgaacaacggttaaatcaaatttatccgctggtgcaacaaattccggggtttaagttggcagctaaaccgcaaggggcgttttatttattcccaaatgttgaagcggctgttgacctggcaggtcttaatgactcaggggaattggtcgatcagctgctggctaaagcccacgttgcggtggttgacggagctgcttttggcatgcccggctacctcaggttgagttatgctactagtttggaagacctggtaaccgccgttgagcggatcactgaatttatgaatcagtttttagaaaaacaagtatctggaggaatcggaattgaaacaaattaacatggttgacgcacctaagtacgttaacgaaaaagttaaaattggtgtttggttaaccaacaaacgttcaagtggtaagatcgcctttctgcaattacgtgacggaacggcatttttccaaggcgtcgtcgtgaagagtaatgttaccccggaagttttcgagttggcgaaggaagtcaagcaggaaaccagcatgtgggtaaccgggatcattcatgaagatgctcgttccaaatttggctacgagatcgaaattgaaaccatcgaggtcctttctgaaacccatgactatccaattacgcccaaggaacatggtgttgacttcttaatggatcatcgtcatctttggctgagatccagccggccccacgctgttatgcggattcgtaatgaggtcattaaggcgacttatgatttctttaacgatgaaggtttcatcaaaatcgatgcgcccatcctgactggaagtgcgcctgaagggacaacgacgcttttccatacggaatacttcgatcgcgacgcttatttgtctcaaagtggtcagttgtatgaagaagccggtgccgaagcgtttggcaaagtgttctcatttggccctacctttagagctgaaaaatcaaaaacccgtcgtcatttgatcgagttttggatgattgaaccggaaatggcattcatgcatcaagaagagagtcttgaaatccaagagcgttatattgcttacttggtgactcgagtgcttgaaaattgccaaatggaactgaagacactgggacgcgacccagaagttctcaagaagtacactgttttaccttatccacgaatcagttatgatgaagccattacgatgctcaaaaagggtggctttgatttggagtggggagtcgactttggttctcctgaagaaacctaccttgctgatcaatttaaccaaccggtctttgtgatcaactaccctaaagcaattaaaccgttttatatgaagccacatccaactcgtgatgacgtggtgatttgtgctgatctcttggcacccgaaggatatggagaaattatcggtggttcagaaagagcaacagattacgactatctctatgatcaaattgtcaaggctggtttggatcctaaagaatactcatggtacttggatttgcgtaaatacggcagtgtgccgcattccggctttggcttgggacttgaacgggctttgacctggttaacaggtgaagaccacgttcgtgaggcaattccattcccaagactgcttaaccgaatttacccataaattgaaattaaacactggtttggtggattcgaggtgaattggatggaagattatgcacgcaatctactaaatgaggggcaaactactgtcagcaactacctgttaaaacattatcatcagattggaattaccaatcaggagcttttcatttacctgctgattaagggaaatcatgacctggtagttccaatgccggaaatggcagatctgcaagcccagacgaattattctgaacagcagctgttcaatttatttcatcaaatgattgaaaagaagctgaccaaaattacgcaagtagtgattgaaggtcagcaggtcgatgcctacgatttcacgccgatgtatgaaaaattggcattggtcaagcccacgggaacctctcctgaggcgtcggcaaacgaaaagcccaagactgtcagcagcaccgaccgccaagcagtctttcaaagtattgaacaagaatttggtcgaactttgtcgccgattgagatggagtctatcagtcagtggttggatattgatcattattcaccggaattaattcagctggcgttgaaggaagccgttttaagtcaggtttataatttaaattatatggaccgaatcattagtacttggtacaagaaaaatttaaagaccccacaacaagttgaagccgccaaaaagaaccggaatagtccacattcggatgatatttcaaccggttacgacggtccggaaattccgtttatcaacttgtcaggtaattcagataaataaacaattaggaaatcggctaaacttttagccgattttttcgtacatagtcaaagggacaatcggttcttcaatgtggcattcagaaacccgtgataaggaagtccacaggaaatattggtaaacgaaaagagaccctcgacaaatgatgtgtttgtcgaaagtctctgatggactgtgctgattttattgggtttcgtcagtaccaccgttattgtcattgttattggtattgccgccaccattgtctggcgtcgtaccgccattgtcagtggaactcgatgatgcggcactactgtttgaatcatcgttaccaccatcgccactcggtttttgctcagatggcgttgatgcggatgactcgttggaactttctgtactgctggaactctcattttcccgtggttgcgtgacaactgccgagctggaacttgaaccaccttcagttgtgtagccactggtcgtttgatttgaactattatcggtgactgtcccaggataaccggcaacataatactcagtggtcccgccacggttggttgcgacaacgtcacttggctgggcccaatcggtgttgggtttatcttcagaaatatagcccatcacgtttttatagatttcctgggcgatcgatgtttgtgccgaggtgacataggaatttgctttgaattgatggtcgtatccagtccagatggctaatgaatagttcttggtataaccggagaaccaggaatccatcgtcgacatcgccggcactttgttcaaataatcgtcgggatactgtgtcgtaccagttttaccggcttcataaagaccagccaccttggctgcagtcccggaacctgcagaatctgtcatcacgcccttgagcatattagtgatcataaatgcggtcgccggcgacatggcgcgtttgccttgctggtgatacttgtgggtcacaccgttaacttgaacaatcttgttgattaagtacggtttgtaataggttccgccattcgcgaaggctgcgtaagatgcggccagctgttcagaggaaatgtagagcccaatcccattttgaatctcgagtggtttgctaaacgacatccccaggtttttcaaaaagccggttgctttaggaaccccaacattttcaagtgttcgaattgccgggatatttcgcgactcaaccagtgcttttcgcatcgtgatcgtgccttggtatttgttatcaaagtcatagaccgatttgtcggttccaggataaacgtacggcgtatctttgaccggctggtaggtcgggtatttaagatattgaatggctggaccgtaatccataattggtttagctgttgatccagaagacctgccggtttggacagccctgttcaaaccgaacgccactttggttttgcggccgccctgcatggcaacgactttaccattattgacatcgacaatggttgcgccgacttggaaacggttgttggggtaggcaatggtcggatcgttattacttacctgataaagtttcttttgcgcactcatgtccaaattggtgtaaacttttaggccgctatttggtttgtagcctttgtcctcgagttcttcgatggtctgctttaaataagaatcaatgtatttagaagtcttttcagaggttcgcgccttcgcgtgggtcgctgaaagatgggctttgacactggtatttttggcagcttgggcttgcgattcagtaatgtctttggttttgaccatcgcatcaaggacttcatttcgccgtttagtcgcatactgaggatacttataagggttgtagagcgtaggtgactgtggcatacctgccaataaagcgaactcaggtaacgttaagtgattaagcgtcttatcgtaataatattctgccgccgtctgcatgccatagacgccgttgcccatatagaccttgttgatgtaaaattccaaaatttgactcttactgtaatgattttcaactttgattgccagccaagcttcctgagcctttcgcttaaaggttcgatcactggcagccgttgaaaagaccgacagtttgactaactgctgagtgagggtacttccaccctgaagacctaaagaagatccggtcaaattcgagatggctgctccggcgattcggatggggtcaacgccatggtgtttatagaaacgccgatcttcaatggaaacgacggcccgtttgagggttcttggaatgtttttagatttgacgtagtcccgattctggcttcccagacgtgaaattactgtgccgttggcatcatagaatttagtggagttatcactggtcagcgcagaccgggtgattcgtggtgcactggaagcgtagtacgtgaataggccggcgccaaacagaaataggacaccaaccaggattaaagcccatttgaagattcgccgaaaggggccttttttatgggtattgctaaactgtcgtccgcgccgaacttcagcgcgtgagtttttcggattgttctgtgacatagccttctccttcgtaacttattcgatgaaagaatcaaccgcgcgaagatagggtagtaatgggttaattctgtattgaatcaaaaagccttccttttcaatgacttttctgggaatggatttgcgaccgccacttttttgggcgtcccaataggtaatcaggtcggtggctttcaaaacaaacacggcctgatccgaaatgaatttgataatcgcaaagcagattccttgctgttgtaagcattgtcgcatatgttcaacttgatgttcatgaaaatttttgagtgggaaagactgtttattcttggtctcttttgcatcaaagtcaatgtattttccgcgatatacgccattataatctgtagtggaagcacgacgaaaataagcttccttaattctggcggcacttctcttgggatagtcaacagaaacgatctgaattggagtcggcttcttatgaataactgcaattcctgcacgaagataatactgattgctcttgttgatttcgtcctccaaggtcattcctcgatttgagaagttaatcgaatcattgtgggtaccggaagaagtcggctgctcatgaaactggtttccattcgggtatctgatagtcattgaacgttagcttcctttttgtgaatagttatattgtacttcatttaacttaataataaccacaataatgttattataccaagtagagtcttcatttaaaatatttaatcgttagggtgatatcatgagccgcttgtgggtaaccggctatcgaagctatgaattaggaatttttaaagatgacgatccaaaacgaaaagtcattgatttggtcttaaaaaatgaaattgatcaggcaattgttgacggcatggattggttaatttccggcggacagttgggaattgagcagtggtcgttggaaatggccctgaatttgaaaaagacctatccagacgaatttcagacgtcaatgatgctgccgttcgctgacttcggcagtaattggaacgaaaacaatcaaaccaagctgcagacgctaaaggcacgggtcgatttttcggcgtcagtttctcaaaagccgtatcagtcgccccaacagttaagaaattaccaagaattcatgctgagtcataccgatcaggcattattgatatatgatttagataatccagggaaatcgcaatacgattatgatcaaataaaaagatttgctgacaaccatccatatccgtataaactaattactttcgacgatttacagagtgctgcggatgaatatcaggaaaacttgaataatagtgttcaagatgactaatttatgatattattttagttggtttgttgcaaatagtgaggtgtaacccatacatggaaaacattaattatactccgaaggatattcttcaaaaggaattcaagcaaaagatgcgtggctatgatcccaatgatgttgacggctttttagacgacatcatcaaggattatgaaactttcaacaaagaactccagtccctcagtgatgagaatgagcgattaaaagttcaagtcgatgaattgaataagcagattgcggtatccggttcgcagccaatgccatcagctggtggcactgctccaaccagaagtgttccgagtcagccaatgtcaagtgcgactaatatggacattttaaagcgcctttcccaccttgaaagacgagtattcggatcacaacttgataataataccaatgattcacacaggctttaaagcttgcatataactaatatggtgtaaatcctgagtaattgcggtcgtatcattacggctgaggaaagtccattctcgcacgggctgcgatgcccgtagtgttcgtgctcggtgaaaaaataagccgggggactctttgtgagttacggcggatattaaagctaaggcttgctatgctttaattccctaaggtgccacagtgacgaacagtattggaaacggtactgatggaacgcggtaaacccctcgagcgggaaacccaaacttttggtaggggagcttcacacacggtaaatgaaccaagtgtgggggagaagtatttcgatatttctcagatagatgattactacttgttatgtcgtcctgggatataataagcacaaaacatggcttatagggatttacaccaaacaggttgagtgggagcttgctcccacttttttgttacccagaaaatgcaggagatagataaaatgaaatttaatttaatggctacttgtgccgccggtatcgaagccttagttggcaaagaaatgcgtgacttgggatatgacgtccaggtcgaaaatggtcgggtccgattcaccggtaatgaagaagatattattaaaaccaatctgtggttgagaacggcagatcggatcaaaattgttgttgatgaatttgacgcccaaacgtttgatgaattgtttgaacaaacgactgcaattgcctgggacaagttgttgccaatggatgccgcctttccagttgagggccgttcgcgaaactcaaaattgcacagcgttcctgattctcaagcaattgtcaaaaaagcgattgtcaatgaattgagcactgcctatcatcgccacacccggttaccagaaaccggtgccgaatttccactggaagtggcaattaataaggatcatgtgatgctgaccatggacaccaccggttcaagcctcttcaaacgtggctatcgaatcgaaaaagggtctgctccccttaaggaaaacatggctgccgccctggtgatgttaaccagctggtatcccgacatgccatttctagatccgttttgtggttcgggaacgattccaatcgaggcagccatgatcggccgcaacattgctccaggctttaatcgtgacttcatctgtgagcagtggccttggattgatcatgatatggcccaaaaagttcgcgatgaggcagattcgaaggctgactatgacattgaacttgatatttctgccagcgatattgacggcaatatgatcgaaatttccaaacgaaatgccgaagaggccggcctgctggctgatattcagtttaaacaattggcagttgccgatttcaaaactgataaggtcaacggcgtgattgtcggcaatccaccctatggacaacgaatgagtgacgaagaacatgcccatgagttatacaaacaaatggggaaagtcttcaatccgctcacgagttggtcaaaatactttttaacctcggaccttgactttgaaaagtattatggggaaaaagcaaccaaacgacgaaagctctacaacggatcaataaggacggactattttcagttctggggaaagaaagttcgagatttacgtaaattagaccaaattaagagcaaataagccggaatatatgctaaaataagaacaacttggtgaaaagaagtgggtaaatggttaaacaagtcgcgataattggcggcggaattattggtgcaacagccgcattttatttgagctttctacaaggtaatgacaatattcaagtgacactatttgacgacgacacggggcaagccacgaaggcagcctccggcatcatctcgccatggctctcaaagcgcagaaataagcgctggtacgctttggccaaacgtggtgcagaattatacccatccctcgtttctgacgctcagttgagcaaccaagcctatcagcagacaggtacgatcgtgactcgcaagaaccacggtgacttattggcgctttatcaggaggccaagatcaaagagcagcatacaactgcgatgggccgggtcgaattgctggacgccaaagaggtaaaacgccggatgccgttgctcaccgatgctccggaaggtgtttttgtcagtggtggcgcacggattgacggcggccactttgtttccgagctgctggaacgggcggctgccaataacctggatgtcaaaaatgaacgggtttccttgacggctaatggcgccattaacacgacagcggggcccaaacattttgatattgtgattattgccaccggtgcttggatgcatgagtcgcttcggccattggggttgaacgtgaaggtccggccgcagaaaggacaattaatcgatttaactgtcaagatgccccataaatggcgaaatatgccagttatgatgccagagggcagtagtgacgttatcccgttcaatggcggtaaattggtgattggtgcgactcacgagaatgacgagggattcgatttaacgcctcagccagctgctcgccgacagttactcaacaatgccaaagtatttatcaacacgctaacggacgcccaagtaagtgacatgcgggtcgcaccagagcctacacggaagattttgcgcctttctttggagcagtcccgacattgcccaactctttgattggtggcggtctggggtcttcaggtttaactaccggaccgatgattggctatcttcttgctcaggcagtgtttgaacgggaaatcgatcattggcaggattacacaaagccggtcagccagtatattgactagattgaatgcagtgcttgaagtgccagtgtatgggcgcccatgttttgtttgtctggaatccaggtgttgaccaccgttgcgaattgattttgcagtcccagtagtttgtccagatgtttttcgaaatgtttggcatattgtttattgagactgtcaatgacgattttgctgtcagtatagaaaaaaatcagttcgctgggattaatttgtaagtcgatcaatttttggaatccggcaattgctgcgctaaactctgcatcatgattgtccgttggcgtaatcacttgattaagttgaatttgtttgccattgttgacaatgagaatgccgatggcggtgtgtccggtatgctgattgacggctgcgtctgtatatagtttaatcatgttatctacactttctttaaggagtttatttatgataagccaaaagcgtcacttcttttatcaaccaagcccattgagcagtattatttgttggagttggacttttgtcgtctttttcattggcgtgattatctggctggaaattactcattttcagtggattacgttatttttctttgtgttgtttgccgtgattgtctgggcggaaattcattttcgcagtattcacgtctacgatcacaaatttgtcgtcagtcgcatcacgaatcctcactggttaaccgttgatctggaccagatttcacacgttcagacctcgaaataccaactggcctttgtcgccaacaccaagatctacagcttcattttacccgccaactccgttattgagatcaaagaattgatttccaacaaataattgctgctccgttgtcagtcgatagttatttaggagggtcataatcattatgaagagcgatgttgaaatttctcaagaaactgttatggaaccaattaccaagatagctgaaaaaattgggattgctgaagaccaaattgaacaatatggtcagtataaagcaaaaatcaattttgacccaaccactgaaaaggcaaatggcaagcttattttagttacttcgatcaatccaactgctgccggcgagggtaaaaccaccgtaacagttggattgggagatgctttcaacgaattacataaaaaggtggttctggcattgcgggaaccatctctgggaccggtcatgggtatgaaaggcggcgcaaccggcggcggctacgctcaagttgtcccaatggatgatatcaatctgcatttcaccggggactttgatgctttgactgaggctaataacacattagccgccttaatcgacaaccatattcagcacggcaatcaattaaacattgatccgcgccaaattacttggaaacgggtgatggacgtcaacgatcgggaattgcgccaggtcgtcatcggtcttggtgggagaacctccggtgtgccgcgtcaagatggttttgatattactgttgccagtgagttgatggccattttgtgcctggcaaccagtctgcctgacctgaagcaacggatcagtcggatgttgattggctatacttacgaccggcaaccagtgaccgtggctgatttgcacgttcaaggagcactcactttattgcttaaagatgcgattaaacccaacctggtccaaaccatcgaacatacaccagcatttatccacggcggtccgtttgccaatattgcccatggctgtaacagtatcttggcgacccaagcggctttgcattttggtgattatgcgatcactgaggctggtttcgggtccgatttgggtgctgaaaaattcatggatattgtcaccccacggctgaagcagagtcctgattgcgtcgtagtcgttgccacagttcgtgcgttgaagctgaatggcggtgctgataagcatgaattgaacacagaaaatcttgaggcccttaaaaaaggcgttgtcaatttgaaacgtcacgttgaagggatgcagcagtacggcaaaccggtggttgtcgcaattaataagtttgccactgataccgaagacgaattaacttatttacaaaactatgtcaccaatgatttgaaggttactgggacgatcatcaacagctgggctgaaggtggtaaaggggcagtcgaccttgccaaggatgtcattgaagcttgtgaacggccagccgaattccacgaattatatagcgatgatgattcaatagaggacaaaatggccaaaatcgtcacccaaatttatgggggtgatgggattgaattttcaaataaagccaaaactgctttaaagcgaattaaaaagttgggttacgatcaattacctgtctgcatggcgaaaacccagtattcatttactgatgacgccaagcagcttggggcacctgagaatttcaaaatccatgtttcagatctgcaactaaaactgggggccggcttcatcgtcgccttaaccggaaaaattttaaccatgccagggctgccgactcatcctgcagcactcgacatggatattgatgaacagggtcggattaccgggctgttctaaagggagcgtttattttgccagtactttatgttatcggaatcattgccttaattgcgattgatcagattgttaaacacttggtggttgccagtttggcattaggtgattcattttctgtgatcaacggtgttttgtcgattaccagaattaacaataccggggctgcttggagcattttatccggccaccaatttattttcgtgatcatcgcgattttagcggcaatcttagtgacttactttattgtgaggtactggtcaaatatgccgtatcgaattggtctggggctgttgctagccggtacgctggggaacgtcattgatcgcatcatgaacaatcacgtggtcgacatgtttcaactcgactttatcaattttccgatttttaactgtgctgacatgtacttgacgtttggaattttgattttggccattgcaatcatccgtgaaagttgattaaggggaacaattattttgaaagagtatattattaccaaccagactggacgtttggataaagtcatctcggaacttgattcttcaatcagccggtcacgggcaaaaaatttaattgacgatcaacatctcaaaatcaatggtgagccagtcaaaccaaagtatcaagttaagtcgggggataaaattcaggtcgattcggtgcaaccgactccgatcagtcttgaaccggagaacatgccacttgatattgtttatgaagatgatgatgtgattgtcgtcaataaaccacaggggatggtggttcatccttccccgggtcatccggaccatacgttagtaaacgctctgttgtaccatagcccgctgtcaacgattaatggcgagtttcggccgggcattgttcaccgaatcgataaggatacttcaggattgttgatggttgccaaaaatgacaaagcacatcagtttttgtcacagcagttgcaagcccaaaaaaatctgcgaaaatatgttgctctcgtccatggacgcattaaggaagattcaggagtcgtcaacgcgcccattggccggtcaccaaaggatcgaaaaaagcaggcagttgtttcggacggcagaagtgccgtgacgcattttgaggtgttggagcgatttgctgactacactttggttgcctgccgactggaaaccggtagaacccaccagattcgagttcatatgaaatacatcgggcatccgatcgttggggatcctttatatgggccaagaaaaaccattcgtggcaatggacagtttctgcacgcccaggagttgggatttgaacacccccggacgcatcaattgatgatcttttcggcgcccctgccaccaatatttgaacaaacacttaataatttacgattaaacaacgctcttggatcttgacaatccggcgctgttttcatattctgaagtggtatagcatttttatgcaatcatcaggtacaaacgttactcaattaaggagcttttactaatgggaaagataatactagataaaatggctatgcagcgggccttaacgagaattacgtatgaaatcgttgaaaaaaacaagggtgttgaagatttagtcttaattggtatcaagacccgaggaatctttttggcaaaccgaattgccgatcggctccaacaattggaaaatgtttcgattcctgtcggtgaattggatattaccaactaccgtgatgatatcgaacacgatgccatgagcagtgatgtcaaaatgtccaataacaagattaacttttctatcgaaggtaaacgggttattttggtagatgatgttttatacacgggccgaactgttcgggctgccctttccgcggtcatggacttgggtcgtcccaagagtatcaatctggcagttttggttgaccgtggacaccgcgaattaccaattcgggccgattttgtcggcaagaatatcccaagttctcaaaaggaaaagattaaggtttatgtttcagaaattgatgacaaggatgctgttgaactcatcaaataattctcattgcgaggagtcagcatgacggaaagatatttaattttagaagatggatccgcgtatgctggaaaggcattcggatcactggcaacaacgacgggtgaaattgttgccaattcaacaatgaacggttatcaagagattatctcaaatcagatttaccataatcagattatcgtttttacccaatcatctatagggaataccggactcgaccagaatgcgtacgagtccattttgccgtccgcaaaaggtgtcattgtcagggagtacgaaaatctggcaactgaccactttaagcggatttctttggataaatatttaaaacaacacaaaatccccggaatttatgacgtcgacacccgagaaatcagacatcatctacagaagcgcggcaatatgaaagcaagcattgtcgacgtcgcggatgatcatgcttttgatcagctgcacgcgacggttttgacaaatcaacaagttgctcaagtggcaactcccaagccgtttcccaaccctgatgaaggcgccaacgtggtcgtagtcgattttggcttaaaaagcggcattttaagggagttatcccatcgtgactgtaacgtgacggtggtcccttggaacttttccgccgcccaaattttggatttggatccggatggcattgttttatcgactggtccaggttcgccggagaatttaccaaagtctgtattagacatgattacagaggttcagtcgcaggcgccattgtttgcgatgggcttaggccatgaactgtttgcgcttgccaatggtgctaaagtttcccaactaaccgttgagcatcacggcagtaatcatcccattcgggaaattatcaccaatgagatctttttctcaggtcaagaacaggggtatgcagttgatccaaaatcaattgaccatgccaaactgtttatcacccatatcgatttggtgaatggcactgttcagggcttacggcacagagattaccccgcattttcggttcaattttctccagatggggcaccagggcccaaagacagtgttggcttgttcgacgactttatggaaatcatggcaagaagaagggacagcaatgacgatagatattaacaaggtcctcctgcttggcggtggcccaaccaacattggccatgaaaatgaacttgatgcagccgcttttgaacgcttgatggcgctcaaaaaaaccggtgcgaaaataatttatgtggataacaatccattttccgttactactgaagaaattcaaccagctaacgtgtatgttcaagaggccaattttcaaaatatcgtcaacattattgataaagaaaatccggacgccattatggcaaccactggcggacttaacggcatgcaaattgcttggcagctggctgaaagtggcattttggcctctaacaacatttcactcttgggcatcaaaccggctgatttgcggaaggttatggacaatcagaaacttcgtgatactttaaccgaaattaatgaaagagtcattgcctcgaaaattgtggccgatgacgacgaagccatggactttgtccgtgaggttggtttcccagtgattgtcaaaccgatgtcatcaagtcatgataccagtcggtttatttgtaataatactgacgaattagaagatgctttggatgtgagtttcaagcgaacctacattaagcgctgctcgattgaacagagtattgtgggttacaaggaaattgaaatggtcggtatccgcgatgaaagcggcaataagctgctggtttcgggaatggaagatatggatccaattgggattcattctggggattcaatcatttttgcaccaacgcagactttgattaatgaagaatatcaagcgctcagatcggcaacttttcgcattatggatgctctgaatgtgacgggaacttgtcacgttcaattcgcccagtctagaaccgatgccaattattttgtgaccaaggtgagtccgttctttaccagaaacaccatcttggctgctaaagcaactgggtaccccttaacgtacgtctcaagctttcttgaaatggggtacaatctgactgaaatcaagttaccgagtaaatataacaagtttctgccgttcatggagccaaccatggatcatgtggtcgttaagattccattatggccgtttagagacattacggacgttgaccagcatttgaacactttaatgaaatcggttggatctaccattggaattggccggacagtggaagaagcgattattaaatccatgcatagttcccagttttcaccacgggatattttgcccagcgtgtcgacggttaatgatgacgaggtcattaatcaactcattcatccattggccagtcgaatattaattttgatggaggcattgcggcgaggcttttcaattgatgagctatctgaactgactcaaattgatcgtttctatttctacaagttgaatcaattattgagagctcaggattttgttgtcaataacccaatgtcaccgcaatccattgaaattggacacaaatacggttttggtgacggcatgctggctgaattatggcaagtcaacatttcaaagattcagcagttgaacgaaaactaccagaatcacgtcacttacaaggcagttgagccgagcgccggtgagatgctggaatcaaccaatattttttacagcagttatgaattggaaaatgaaagccggccatttgaagaaaagagtgctttggtgattggtcggggtgggaaccaactcggccccaattcggcagcggattattacacctcacagattctcagggcgcttcacaagtcaggctataaaacaattatcatgaacacaaatccgaatgccgtctcactaacgccacagttaagtgacaaacaatacattgagccgatccaactcggaaatattctcaacattattaatttggagaaaccagatgtcgtcattctcccagggaaccgacactacttgtctaaacagttaaaacaatttcaaaatcttaatatcatcgttttgccgccggatcaaaaagttgccacatacaatcaaaagtatgcgacaacagctgtcgatctgttcatcgaaggcgatgaaattttaccagttacgaccatttcttttgtggggaaagatcaacggactgacctgcggtttattaacgactataaagaaccgatggataactggaagtctgacgaagcaaaattgattgccgatgccactaacaaggtagatccaaaagaatggcaggggctggttcaagtcttgtataatacaactggtgattctaaatatgagatgaccggcattcggcctgtacgaattactgagaccgcctttctcaccaaaacgaccgggattaattggattaacgttttggtccgtaaatacctgcacacattggatatggaagccttgcgggaagacttgaagccaacggagcacaaacgtgcatcgattatgactgctcatttccccttcagagaactccaatccagtcgcactgagggaaccactaagcaagaagtcggttcatcactatcatttaagaattttgaataagattacaacaaaaaggtcggggcaaaagttgatattttgccccgaccctttgtgtattctacatattatcaagctaaatagtgtgactgacaatgtgagaaagacgctcctaaatgcaactgatgtatatctatggcgcgcattttttgtatgccagaaattgaaagcagattactcacccgcttattttcgcatctgatcaattagattttcatccggggtgacgaacaatgtcgtttgattgtcataaatcacataccccggtttagtaccattgggtttgcgaatatttttgacttttgtgtaatcgacttgtactttggcggatccgcgcgctttcgagaaataggcagctagattggcagcttccgccagggttttctcagacgggtcaaagctgcggataatgacgtgtgatccaggaatatttttggtatgcagccaggtatcacgtttgtcggcggtatgcatagttaatttttcattctgcagattattcttaccgactaaaatttctgtcccatcacttgcgacaaacttttctggtttgttaatcttttgtcgcttatttttcttctttttgttctgctcatgatcacggagataatgaccttgttccaattcgtacttgatgtcgatcaggtcttggggatcagccagttcaatttgggattgaatattttcgaagtaatcaacctcctgcttggtcagttgaatttgttcgccaacaaatttaacagcgttcttcaatttttggtatttcttgaaatatcgttgggcgttttgggaaggggattgttgattggaaagctgaatggtaatcaatttattttcatcatagtagttgggcagttcaatgctggtcattccacgttgaactttgttgagataagttgttaaaatctctcccttgacccgataatcatccgcattttcagtttctttcatatcccgctggagtttcttaagtttcgtgcgattctttttaagctgttttttaacgacttgaatcagcaccgcgccttgttctctgacccggtctctttgggctttgctggcgtaaaaagcatccagcaattcgctcaatgttgagaaagtttgatttttagttgtacccggatagggaaatgcggtaaaattaatcttgttacctgcaacatggctaaaggttggctctggtgagtcgaatttttggaagaaatccttgaaattagtctcaactttctcgtccttatgcaaactagttgctaatgccaaagatgtgtcgttgcccaatccttgaattgttttccgcagattttcagctaaaacgtccacgtttggaaaatctttgatcaattggcggacccggtcaaagtcagtcatcgtaaatgggttttccaagtcctgcttcggcggtttgatataagttgctccaggcagcaacaagcgatatcggttaacgtcagaaccaacgtgtttaatagcgtcaataatttttcccgtggcttgctcaaccaggatgatgttactatgacgggccataatttcgacaatcagatctaattttgtctggtcacccagttcattgcgcgccgtgaaggtgaacgtcaacacgcgatcattttcctgttgggaaatctcactgagaattccaccgctgagatgcttacggacaatcattgtaaagtttgtcggcacactggggttgacatatggaactttggtaatctgtacccgggcatacgtcgggttggcagacagcagcagctgttgattctttccgtgagctcggattgttaatatgagttcattcggatagggttgattaattttgctgatccgacccgtttgcagcagatcggttaattcatttttcatagaatgggtaaaagaaccatcaaatgacatcttatcactcactttcgtataagtagcatgtactagtatagcgcactttcttgactgatgctaaggaaggcacatgttatttgtatgtcattatcaaatagcgtatactaatttttcggaggtcttttcatcatgaaagatattcttgtggcacttaattctgctgccaaaaatcatcgatctcaaatattcaatattactaaggcaatgaacctgacaatttctgaatggaagttgttaaatcaagtcattgccggcaataccacccaggaattattgtccgaaagtaccaaattggatatttcaaccttgtcgcggcagttgaagcgactattagaaaaagatatgatcgaaaagaccgcggttggtagggacaagcgacaattgatttataaggtgactgacaagggaactcaggccagtcaatatgttgccgccgaaattcaaaagctgactgaccgggtatttaatcattggactgatgaagagaaaaatcttttaaagatattgatcaatcgtcttgaaaagagtttggatagaatttaattacgagcaggtgaatttaatgaaaattgcgatcgtgactgatagcacggcgtatttaaccaaggaagaacaagcgaaatacaacattatcgaagtgccaatccctgttattatcgatggccgtgagtacaaggaaggtgtcgatttgacgacggcagaattttacgataagttaaagaattctcaggcctttcccagtacatctcagccgccaatcggtgagatgattgatctctacaattctttggctaaacaaggctatgacaccgtgattagtattcatcttgccagcacgatttctggcttctatagttctctgactcaaattgcaccaacgatcgaagggatcaaagtcatcccatatgattccaaaatcaccgttaagttaatgggctatatggccatccaagccagcaaaatggcacgacttgggcgcacgcccgaccagatccttacatatcttgatgggcttcggcagacaattgacgaactgtttgtcgttgatgatctgcaaaacctggttcgcggaggccgcctttcaaacgcctcggcattcattggcggaattcttaaaattaaaccgttattgacatttgatgataaaagtaatgaaattgtcgcctttgaaaagatccggtcgcgtaaaaaagccctcaaacgagtggaggaactctttgctgctgccaaacaaaaagctgattatcctctgcgggcattggtcattaacggcaatgatcctaaagccggaaatgaatgggcaaataaaattcacgaactttatcctgatatgacaatcgaacaaagttattttggtcccaccattggtacccatttaggcgaccaagcattagctcttgcgtggcttcgagactttgatcaggataacatttaaaatgaactattttaacttgcgatcgcttattgttcagtaaaacacgaactaagcgattgcattttttagtgcatgtgataaactttaatagttacataaaataaatatggggtaggattcaatgcgttaagtgtcggaggaacggaatgtgaacttcgaacgaaaaatgatcgacttcgacttgtcgaccatttgcggtgttgtttccgcattcgctatgttatttagttctctaaataatggtgagctcctttataaggagatgctgcatcatgaagtcattgtcattgggttttcgtaagctgcgggttgtggatattgttgtcttgggaattttcatgtcgttattgttaattctcggtcgatttactgtcggtgttcagtcctggcggttaagcttcggcttcgttgtcactgcgattgccagtatgctgtatgggccactgtggtcatccacaatcgctgcattaacggatatcatcggcactttgatgtctggaagtgtttatttccctgggtttactatctctgcaattttaggcgctgccatttatggctattttttctatggcaaagagatcacatggaaacgcgtgatcattgcccaattaatcattgcggttgtcgtcaacgcaattttgaatacctattggttgacaattttatataagacaccgttttgggcatttttaccggttagagcgttaaaagaattggtcatgacaccgattcaaatggcaattctttactatatgctgaattcccagacaatgagtaatattcagagtcggttgtttaaataaaatgagaagcgacgcaccgtaccaacatattggtcggcgggccgctttttgtcgtatacaaaggagtgaatcatgatgtattacatctcattacacaacatgcggtttcacagtcatattggcgttttgcccgaggaaaaagtcgttggtcaaaatattcaaattgatttaaaagtgaaagtcgatgccgatccgactgatgatgatttgaagtcgacggtgtcatacgcagatttctatccaaccatcgccaaggtgatcgacaataatcaggtcgacttagttgagaccttggcccagacagtgattgccgctattaaaaatattgattcgcggattatgactgtcaatgtccggatccgcaaacaaggaacgccgattgatggtgttttggacgacgtcgaaatagaaatggagcattagtatggaagatgtatatttaagtttaggcagtaatattgggaaccgcgaggcatttttgcaacaggccatcgaggcattgggtagtgacccacggattatgattgaaaagcaggccagtctgtacgaaacgtccccggttggtggggtcaagcaacgggcatttgtcaacacagctgtcaagattgggacgacctatgaacccctggcactcttaaaggtgattcatgaaatcgaaagtggtctccatcgaactcgccaggttcactggggtccaaggaccgtggatattgatattatcttctttggcaatgaacaaattgatcaaccagggctgtcgattccacatcccgaagcgtttaatcgattatttgtgttgattccgattcaagaattgattgatggacaatttccagacgctgataagattgccacggccattaagtctctccaacaagatgatcaatcaatcaaaaaaatcagtccggctaataacttctacaccgaaatcaccaataacgttactaacatattggctgcaattggtgacgacccgactagaaagggacttattgaaaccccggatcgggttgccagaatgtatgccaacatctttgattctatcggactggaagattttcaagactataaactgtttgattcaccggagtcagatgactcaaagacggttatggtgaaagggattccattttattcgatgtgtgagcatcacatgatgccattctggggcaaagtcagtgtcgcctatgttcctgataacgggaaaattatcggtctaagtaaaatcctgcgactggttgattttgtatcacacaagttaagtctgcaggaaaaaattacggatgatgttctcagccaaatggaaaaaattctccatcccaaaggcgtggcggtaattgttgatgcccgccatatgtgtatcgaaatgcggggcgtcaaaaaaaccggcaccgtgacccgaaccactaaatttaccggtgtcttccagcaaaacgatgagctgagaagtgagtttttgaattcaatccaggtgggacaaatatgaacgatgatttaaccagtcactttgccgaatttttatataatcaaggtgatcgcattggtttgttaaagcaagttctgcgccaattgggcaacccggatgctgactatccaatcatccatatctgcggtaccaacggcaaggggtcaacggcaacgatgattgccgcaatactccagcagatgggaaaacgagttggtttatttaccagcccgtttatcggtgatgttaccaatagtattcagattaatcgccaggcaatccaaactgatcaatttgataagtatctcaatcgcctcaagcagctgatgacttcatttggtgatggacagcaggaactctctgaatttgaggctatgtttgttgcggccatgcagtacttttctgatcaacaagttgactatgtggttttggaatgcggtctgggtggggagctcgacgcaaccaatgcagtgaaaacaaccatgtattcaatctttactaaaattggcatggatcatattggcattctgggaaataccattgaagaaattgcgacgacaaagtcaaaaattattcgaccaggaaacacaaccattgtggcccccaaccaacggccggaagtcctggcagtcttgaaaggtgaagcgagtcacaaagccgccaacttccttgatgccaacacagttcaaattgatcggcagtcaactaaagcaactcatttcgtttatcaagtcggtcatcaatctggtcattttcaatttggactgccgggcgattaccagttggaaaatgtccgaaccgtgttgttgtggttggatgattttcaaaaaaagcagcacttatcactggacgccagtcaattattaacccaagcgctggggaagctggatgtccccggacggtttgaaaccattcacgctcaaccgacgatcatcatcgatggtgctcataatgttgatgcgatcacagctttcgctgaatccgtgaaacattcattttccagccaatccaaaatgattattaccgggtttctgaaggataaagattatgtcgataatgtgcgattgctggcagagattcccaatgcaactttcaaattaacgcaacctgctaatcctgagcgcaagctggacgaacgtcgtcttcaaacggtcttccaaaacattactggcaagatttacccgattttttccgacccgatagctgcccttaaggcaagcctcaaggaatcagccaatcaccccgatcagctcattttggtggtgggttcattttatctcatcaacccaattcgagattatttaataaagacaaggagcaattcaaatgactaattctaatgaagtccatttcaaagggaaaaattttgatttcaatctgactaaaacgccaattatctattccattctcaatttaaccccggattcattttacgatggtggggtcaataccagtattgatcaagttttggaccgcatcgaaactgaaatgggctatggtgccaaaatctttgaactgggtggcaaatcgtccaaaccccattttgatgacattagtccagatgaagagtggcagcgggtagaaccttatcttaaagcgattcaaaaacggtttccaaatattgtattggcaatcgattcgaataccaactcagtgattgaacgggcgttgcaatctggaattcagatcattaatgatattgatggctttaattctcaagccaaactggatttggttcaacaatatcaaccctcagtcgtcacgatgtttaatggtcgcaattttgacgaacaaccaacgacacttgaagacacgatgcattcatttttcactgactcgattaatcgtttagaacaagctggtcttcaaagagagaacattgttattgatcccggggttggcttctctgatagcaatacgcttgaatttgatttgattaaaatgcgttacacaaaacaaatgcgccagtttgcagcaccgatcatgatcgcaatttctcagaaaagttttgccaaacgactgtttgatgcaggctcagatgagcgactgatcccaacattactgtttgaagcatacatgacccaactgggtgggcgaattatccgtgtccataacgtcaaagaaacccaagaactgattaaaacctatcagatcttcaaggacatattaagtgattaagaagctgtccaagatctatgatttttgatatacttctatgtaaaaagcgagtttaagctatgaaaaattatcccagcaatattactcggcaacaatttgaattaattcgaccagctttagaaaattttcgtaagcgaactaagcctcgaaaatatgacctctacgaggtcctctgtgcggtcctatatgtcttgaaaaccggttgccaatggcgtcaagtccccggtgatttcccagaatggcggtcagtttacaactattacaaaatttggtcaactaaagctgagcctacggctgattctttattggaacaagttttaaaaaaattgtcattgctcggcgaacttaccaaggacgttcagctttaacttcctttattatcgttgacgctcagagcgtcaaaaacaccgctactgctgaaaacaaaggttacgacgctggtaagaaaatctcggggattaagcgccatctggcagttgatatcaatggctttccgcaggccattcacatgacgcgagcgaacgtctctgatcgagacggggccagtgcaatgatcgctttacatgccatgcatttacgccaggttcaaaatgtcttagttgatggtggttattcaggcgttaattttcagctcgatgtagccagtaatttaaacgcaaccgtgcaggttgcgaagcgcaatgagttgcatcgattcgaagtcatgccccaacgttgggtagtcgaacgatcttttagttggctagagaattgtcggcgactttggaaaaattgtgagcgtcaattaaccaccagtctgcaaatggtcgttttagcgtttttagcactattacttaagagattttagacagcttctaaggaagtgatcaaccatcttagttgaacaattaatcgcccaaatcgtaacgctaaaaagtcagccatatccctggataaatacccaaaaagtgcagacagctatcgagttgctgagggcaaactcccaaggacttcgcgaccggaaatcgccatttcatctgtctgcaagtgcgatggtctttgaaggaggtaaggggatctttatccggcacccatacctgcatacaattctattgcctgccggtcacgttgagccaaacgaaatgccgattgattgtgccatcagagaatttaccgaagagaccggtttggttttaaaaactagtcccaattcgttaatcgacgtcaacatcattgatattccggctaatccgcaaaaaggcgagggtgctcatcaacatctggacttccgctactggttctcctcgattgaaccacataccaaatatcatgctgagctgccaatatttcagttgaccaggcaggaggccccggtggagtttcaaccatattttacactaatatgattggcaaaaataagagatcatgattattgccatatacaattagccgattcaaatcaaggaaaagtttctgtaaaaccggttattggtatatacaattatttaaaaagaaggttcaacacaatggacaatcaaattatcaccagaaaaatgcaggcagaagattatccaaatgcttatgcattgtggcaacaagttcccggcatgaatctgcgggaatttgacgatagttttgaagaaatcagtcgattattgcgattcaatcccaatttctgttttgtagcggagaccaagactgacaaacagatcatcggcagcattctgggtgcaactgatggtcggcgcgggacgatttatcatttggcagttgctccgggttatcagaatcaaggtttgggaactcaactggtcaataaagtgattgaacagctccaagctgtcggtattcataaaatctttgtcaatgtcatgaaagataatcttgcaggccaatcattttggcagcatctaaaatttgttaaacgaagtgacgtgattcgttttaataaaattatttagatacgtatcagagaagcggggtgcagactcatttttcttgatacggattctactttacataatatatattatacgaagtagagaaaaggtaaaaagaaccagctaccaaagccaacactctcggcaatggtaactggttctttactttaatttcgtgaacaattaaccaacggcttcctccagaggatttccggattcaacttgagtgttcgtttggtaattatccactcgtacttttaaaacgtgacgctgaatgcgtttatttaacggtggcagtttcatatagtcaccgtacaagcgtgttaagtatgcatcataatctgctaggactggcacccgtaaattttcaaaggccattgggattaaatgatggatctctgtcggcttgattaattcttttccgtactgatacggtgatgacatgttaatcaacgataattccgagtgaccgttatattgggtcattgtgctgagtcgaatatcgtatagctcactcaaattataatccgcatacttagattgtgtgatactttgctgatacaggtcaggataaaatcgctttcgaatctcttctaacagcattgccaattttgcttgctgtttttcctgttgcggacgtttatttggcattcgatcgaacggaaatacatcaataaagatgccattcttggcttttgtcaactcacggccatgttccaagatccgcgtgccatcagccatcactttagcgaaatcgtattcgtattgtggatcaaggcgattctcttcaacgaagtatcctcgatgtgacaactctgccggtgcaacttgtagaaacctttcaaaatcagtgcgcggcaaaccaatatcaatatcgtcgtcccatggaataaagccgtgatgacgcacggcaccaattgctgaaccaccagttagaaaatattccagatggtatttagaattgattgctgccacatttgccagaatacccagttgaacttgatgaattaattttaaatcaaccatatttagaacctccttaatcagaaatccgatctcatatctaaacctctttcaaattggattgttcacttattaatattaatcgattccaacattgggtcaattaatatgcttatttatgatatacttaacttaataaaatacagattttattaagttatacgccaaaaaataaacagccccaccaaatttactgcgatttgctgggatatgattaactgaattaaggagcttaaaaatgaaatcatctcaatatattcaacacaatcaacagctggttcaaaccctgccaacttatattaatgaatattatcttgacaaatcaacggttccattatcccccgccacgctatatcagtatctaaatgagttttaccgcttcttcacttggatgatcgacgttgggattactgacgtgaaaactgtcaaagaaattccactctccgcgctggaacacttcaaaaaacaggatatggaactgtataagtcttacctgctgaaccgtggcaagcaaacggcttcccatccgcaagcaccaatttctcatcggacagtcaatcgttccctgaacgcgctctcagccttattccgatacttatcggaggaaaatgaaactgccgatggtgagccttatttttaccggaatgtgatgaagaaaattgccttggttcccgacagcgaaacctatcaaacccgtgccaacaacattaaggatcaactcatgttgggtgacgcggatgtgaaatacattgaattcatccagaatgactatcccaagacactgaccaataaacgaacgctgtcattatatcaacgcgatcgtgaacgtgacgtggcaatcaatgcgctgatgcttggcactggcattcgggtgtccgagctgaccaatgcaaatgtctctgatttaaatttgagcaaagcggcaattgtcgtccggcgaaaaggcggcaagtacgattccgtgcccattgccagctgggtgcttccctatctggcaacctatttaaacgtccgtaagcaacggtatttggccaccaagactacccctgccctctttttgacgaaaggggcaagccaacccagaagaatttccaccgcgactgttgaactattggtggcgaaatactcccaagttttcaaccacgtgcggattacaccccacaagttacggcatacattggcttcgaagctctatttggaaaccaacaatgagcacttggtggccactcagcttggccagagttcaaccaatgcgactggcttatacacgcacatcattgacaccaagcaacgccaagcccttgataaacttcatcgtgacaaacagcgtcactaaaaaaattcgtgggtagattgccacaaaattcctcagcgatttgttttttgatccacagctgacccctcaactgattgagttgattttacagctttctgataggcagaccacatttttgattgaactttcgaaaatgtcatctgatcaaattcactggagtggatccatttacccggaaaatagcttaaatcaatatcttccgctatttggccttccagtaacttaattttccattgctgatgggtaaaggtgtgaacaaccgttggcgtagatactggatgcaacgcgacacttagttggtaatcggtctttagtcgggtttcgattatgtcaattaacgttgattctgtcgccagttggtcatcagttaaatttttgcggtcaaataacggaaacatccaaaaattggccagaatgccatgactcgggcgtttttcaaataagtaccccgccttggaatggatgaccactccaaagtaatcgtggcgaaccggccgcttctttttggtcttcactgggtaatggtcttcaatcccatccagatatgactggttgaaatccttgaccggtgattggctggtatcataattggtggctgtcatgtagctggcacccaaatccataattgcttgattaaagtcgcctggtcgatcctttgaaacgattgggttgattattttttcaaatacctgacgagtgtgtggtttagcaacatcatcgtcgatttctaacagcctggcaaaaacgcgaaaggcatttccatccactgccgccactggttggccaaaagcaatactggcaatggcaccggccgtatagggcccgataccgctcaattcctgaagctcttttgcagtcgttggccattggccctgataatcgaaaacaatctgttgagccgccttttgaaggttcctggcccgagaatagtagcccagtccttcccaagctttcatcagcttgtcctccggggctgcagccagatcttcaatcgttggaaattcgttcataaaccgtaaataatacggaatgactgtttccacctgagtttgctgaagcataatttctgacacccacacatggtaaggatcctgatcctgccgccatggcaaatcccgcttattttggtcataccaggctagtagcgtctcctgaaatgctttgattgtcttatgtgaccatttgatcatctgacgatttctccttacagtttaattcaaaataataaagggctgttggcaaaatttgcgttttgtcacagccctttatgtgaatggtcattaatagctgaaatatccttggctaactaatttttctgccagttcttcttgataaagttttcgcgtccgcccatttcttccatttgataacggagcggatttttcttgtagaattcttgatgttcttcttctgccggatagaatggtttggcatcctcaatttgggtcacgattggactgtcaaattgttcactctcggcgagggctttctttgaagcttcggcaatttttctttgctgctcatccttcacgtaaattaccggacgataattatcaccgcgatcttggaattgtcccatggcgtccgttgggtcagtttgatgccaatagatttccactaacttatcatacgagattacctcagggtcaaagaaaattttgaccgcttcagtgtggccagtggtgtggctggcaacttgttcataagttgggttgggaacatggccgccagtatagccggaaacgaccttgttaataccgggaatagtgtcaaatggcttgaccatgcaccagaaacatccacctgcaaaaattgctgtatcttccatgcattgcacctcaatttcatttattcaaataattgtttgtatttactgtatccctttgcgtccaattcggcaaccggaataaattttaaggctgctgaattaatgcaaaatcggtgaccaccagcatctttgggaccgtctgggaacacgtgcccaagatgtgaacccgcctgcttacttttgacttcttcgcgaatcatgccaaaagaagtgtccaagtgcttatcaatattggctgggtcaatcggtttcgtaaatgatggccaaccacagccggcatcatatttatcggtcgatgagaacagcggttctccgctcacgacatccacgtaaataccggcttggtaaaagtcatcatactgaccgctaaatggcgcctcagtccctttgttttgggtaacatcgtattgttccggggttagtttgtttttgagttcctgcttgtccatgataaccctccattaaattaggttgtgtacaactaaactaaattcattatagtggccaaccaacccaaagtaaacaaaaacggccaaactaaccattcagattagccggaccgtttgaaagagttgatgaattagcttaatgcatctgttaatggcggaacaacttgcttcttacgtgaaacaacacctggtaatgacattgtgtcgtcactgagtttgctgttaaatgctttttcaactgcagatgatggttcgccgacaacaatcatctttgaatcgctgttcaaaacgttagtaatcagaactaagaacaagtcgtagcccttatcagcagcttcagccttcatggcattctcaatgtcatttttacgcttgtcaatttcgctgaattcaacgacgttgatttggtcaatccgaacactcttaccgcccattgtaaatgacttggcatcagaatcaatgagttcttggtccgtctttgctgaaacgttggtcccagctttaagcatctcgatgccgtacttttcgtaatcgatgtcagcaatttcagctaaagtcttgacagcaattttatcttcttcagtggtcgttggtgacttcagtaacaacgtatctgaaataattgctgaaagcattaagccggctaattgagcagggatttcaactttgttttcgtcaaacatcttaacgataatcgtactgcagcagccaactggttcggcgcggtagtatagtggctgatcagtctggaaattagaaattcggtggtgatcaaccacatgagtgatggttaaatctttgatgtcactgacactttgttggaattcattgtggtcaaccaacatgacggagtcaacttcatttttagcagttttgataattcgtggagtcggctcgtcaaaataatttaacacaaatgcggtttctgaattaggttcacccaaagcaacggcttcagtatcataccctaatttgttctgcagatatgaataggcttttgcagcaacgattgcatctgtatcaggactttgatgaccaaaaactaattctttactcatttacataatctcctttgataatcaaaatttatttccctaaacgggctaaataatcttctttagcaaggaactcatcgaacttctgtaagaaacgttcaatccgcgggatttcgttcttgcggttccggtagacgaaattcagatcaaacttgactttaggatccaattcagtgacccaaatgtcatcgtcagtcaacttcttaaggtcgatattgagcatatatgactttggtaatgccgtgttggtgtgggaattaatggcgaacttcaaaatctgctcgggcatggtatatcgtgccgctacctttggccagtccaccatttggttcttaaaggattcccgcaaagtttggttgagataataatcttgtggatacatcacccatggcctgtcgttgacatctttcaagtggacccgtttacgtttggccaaacttgggttgtggtggataaacaataagtcatccgagataatcttcttggagctgtatggcttccagttcttaatcgattcatccggcaggtacatgattgccaaatcgattcggttgttctccaagctttcccaaatctcttttctggtcagcatgtggaaattgacttccaaatccggattttcctggtaaagtgccagggcaaaatcttcaaagactttggtttcaacggaagcgaggattcccagattaatttgaccagtcgttgagctggtagcttgttgaatctggtcgttggcatcatttaacagatcgtatatctgccgggttgtcttcaacatgatcacacctgcatcggtcagccttaatttcttgccaaccgagtagaataattcagttcccattgtcttttcaagcttcttgatttgttgggtcagcgctggttgcgtaattcccaagatctgggcagcttgtgtgtagttcatcgtttctgacaactggagaaaatacgataaagtctttgatgcaaaaatattttcctgagtggttttcattcagactctccttatcggtccgtgcgaccattatataattaacaggatactgctattatgataattcttattgttaatacaatcaattaatatggtaaaaatttaatcaattgataagccgacaaactttggtctgattgaaaccggggtgccttcactgtcaacatcaattacaaatgagccgttggaataacgcccacccaatgaataatctgctggtaaaatatcgtgaacccggcgatgatcggtccgcacttcaagcggctggtcttcgctttcgattcgacaaaagtccacaattctgtgcggattatttttaagttcccgcaggatcataacgccctttcgagcccttgaagtggcaggaatttctttaacagctaatttcttgaaagacccacgttgggtcacaattgccaagacatcgtcttcagagaccagttggaggttggtgactttatcaacacctcgaagccccatggattttacgccggtagttctggcgccattaaccggtacctcatcgatcccatagcgtaaggctaagccattattagagataagaagcatttgtccagcagttgcgggcgtcttcaaataatgaatggccactacccgctcatcagcagttttgagcttctcataggtgtaggcatggctcttgtaggtccgtcccggcttcatatccgcaaaaccagtttgtttgacatgcccttggtcagttgcaatcaagaaggttcctggttgcttgagtgaatcaaaagcataggtgccaatgatttcctcgtcagcatccaacccgatggtctgagaaatatgctcaccggtatccttccacttcacatctgccaattcaaagactggccgatagatcagattacctttattggtgaacataaacagatgatcgcgggcatttaattcggccataaagattggataatcttcatcttttaaaccagtgtcggttgtcgaagctttatatgaccgaatgctgcttcgcttgatgtagccgtcatggctgaccatcacgatcacatcctcgtcagggatcaagacatctgtattaatcttgatatctgaaacctcagcttgaatctcggttctccgagcgctgcgataagttttcgccaatgcgcgtaactcgttggccaaaacccgattgagttcttttggactattcaaaattttgttgtctttggtaatttcgtcggccaggtgctggtgttcgttctccaactctgtcacgtcagtattggtcaaacgatacagctgcaaagcgacgatggcatcagcctgtttttctgaaaaatcgtaggttttgaccagattgtcacgggcatctttacggttcttacttgctcggatggttttgatgaccttgtccaaaattgataaggcatgaatcaatccctcaacgatatgctgacggtcctgagccttctttaaattgtatttggtccgcttctcaatgacttcttgttggaattcgagataggccaccaagatctttttcagtgacaaacgttccggccgcatatgggaaatggcaaccatattgaaattgtaggaaacctgcaagtcggtattcttgaacaggtagttcaaaattccttttgagtcaacatcacgctttaattcgacaacaatgctgagtccgttacgatcactttgatcacgaacctccgaaatgccttcgatcttcttgttcaagcgaatttcatcaatccgtttgactagttgggccttattaacctcgtaaggaatttctgtgatgacaatttgtgatttgttgcctttcagtggctcaatggaagtcttcgagcggacgataatcttgccgtgaccggtttcgtatgcttttttgatgccgtcaattccttgaacaattgcgccagttgggaaatcgggtcccttcacaaactgcatcaaatcatccagagttgcatccgggtgcttctgcaggtaaagaatcgcgtcaatcacttctccgaggttatgcggtggaatatcggtcgcatagccggcagaaattccagtagaaccgttcacaagcaaattggggaatcgggatggcaaaacagttggttcgtactcggtgtcatcaaaattgaggacccagtcgaccgtgtccttttcgatatcccgcagcatttcgctggcgattttgctcaaacgcgcttcggtataccgcattgcggcaggcggatcaccgtccattgaaccattgttgccgtgcatttcaatcagcggctcgcgaaccttccagtcttggctcattcgattcaatgcttcataaatcgaactgtcgccatggggatgaaaattacccatgacatttcccacggattttgctgatttacgaaacggtttgtcgtacgtattgccgtctttgttcatggcataaaggattcgtcgttgaaccggctttaaaccatcccgaatgtcaggcaaggcccgttcctgaatgattgatttggaatatctgctgaaccgttcgcccatgacatcttcgagggtcaaactttcaattttactcattttttagacgcgccccctaatcacttgtattatccaagatgctgccatcttcttctaaattaaatttgacgttatgttcaatccattttcttcggggttcaactttatcgcccatcaaagtggtcacccgtttttcagcgagagcggcatcatcgatccgaacccgaatcaaagtccgagtgtcaggattcatggttgtttcccacagttggtcagcgttcatctcacccaaacctttgaaccgctggaggctgtagcccttgccaaagtcctttgataccttatttaattcttcattggtccaagcatattggactttcaacttcttgccggcacccttctgtagcttgtaaagaggtggtaaggcgatgaagactctgccattatcgatcattggccgcatgtatttgtagaagaacgtcaacaagagaatctgaatatgagcaccgtcatcatcggcatcggtcataatgataatcttatcgtagttggcatcatcaatgttaaaatcggcaccaacgccggcaccaattgtataaatcatagtattgatttcttcgtttttcataatttccgggagctttgcccgttcggtgttcaagaccttccctcgaaggggcaaaattgcctgatatcttcggtctcggccctgtttggcagaaccgccggctgaatccccttcgaccagaaacagctcatttcggctgtaatcctttgattgagccggggtcaattttcctgacagcaggcgttcttgttttttatgccgtttgccggttcgggtttcatcccgggcttttcttgccgcctgtcgggcttgtctggcacgcaaggctttatgaaccagagtctgggcaaattcaccattttccatcaaatagtagcccagcttctcactgacaacgttatcaacgattgagcgggcttcaggggtgcctagtttttctttggtctgaccttcaaattggagaatttcttctggaattcgtaacgataatacgacggacagtccctcgcggacatcgctgccttcaaggttcttatccttttccttgagcatccccacttttcgggcatagtcattaaaggctttcgtccaagcatttctcagacccgcctcgtgcgtgccgccgtccttggttcgaacgttgttaacaaatgacagcatggtttcagaataaccatcgttatactgcgcagccacttcgacttccacgccgtcttttttgccgtcgaaatacatcacgtcgcccagggtatgcttatcttcattcaaatattgaacgaattccttaataccctcttcgtaatggaaaacgtcttcctgctcctgatcggttcgttcgtcagtcagggtaattttggttcctttaagtagaaaggcggattcccgtaatcgctcggaaagaaccgagaaattgtaaaccgtgctggtgaaaatagttggatccggtttaaaggttaccgttgtcccactatgagcgcgggtcttgcccaattttttcagtgtgcccaccggatggccgccgtttttgaaatcttcttcgtaacggtaaccgtcacggacaatcacaactttcagccaagtagaaagtgcgttgacaacgctggcgccgacgccgtgcagtccaccggatgttttgtagccgccctgaccgaatttaccgccggcatgaagcatcgttaaaatcacttcaggagttggtttccctgaagcgtgcataccagttggcatcccccggccgtgatcgaccaccgtgatactgttgtccttatgaattgagacgtcaatttcgtccccataaccggccaaaacttcgtccacggcattatcaacaatttcgtagaccaaatgatgcaggccgcgtgaatcagtggaaccgatgtacattccaggacgctttctaaccgcgtcgagtccctcaagaatttgaatcgaggaatcatcatatttttgcttttgctttaccattcgttatgactcctttttttgcaatctacttcataataacctaaatttacgccgatggaaacgaaattttattggctgaactcaaattacatgctaaaatgagaaacgctattaagtttattaattgcgactattgtgaggtttgagatgaattctaatattgaacaaattataatgctgttagtgctagcttatttgctgggatcaattcccagcggtgtctggattggtaaaattttctttcacattgatattcgccgacacggttccggcaatatcgggactaccaatacctaccgggttttagggccgattgccggctcgattgtcatggcgctggatatttctaaaggagcggtagcgacattactgccgacattttttcatatcaccgcgatcagtccgttgatctttggattcatggcgattttggggcacaccttttcaatctttgataaattcaaaggcggcaaggcggtggcaaccagtgcagggatgctgctggcatacaagccggctttcttctttttggcagccgggatttggattctggtgattttgttaaccagcatggtcagtcttgccagcatgatcggttttaccttaacgaccatcgcaattttctttacccacgacattttattgagtgtcatggcggtgatcctgacctttttcattttttaccggcatcgggccaatatcagccgaattaaaaatggcaccgaaagtatggtgccatttggccttggcaatcggctgcgaaaacgtaaagatccgaatgaataaccaatcaaaaacgagtgatttctgaaataaggaatcactcgtttttagtttggattttaatcggccggacaattgatgcgacagctactatcaattagaagaaactgattgaatatcggccggcaaaggcgtggcggccagccaactgattaatcgcaaatttatcttccagcttgccgtcggcattcactgtatcagccagtccccaccacggttcaatgcaggcaaatggggctttttttgggtacggtgaccagataccgacatatggtgcattctcaaccgtgagtgaaacaccatgatcattttgggcattggccagcatcacagtcgtttcctggcgatcaaggctcaaaacgatggcatcgctgttaaacagctcgtggttcaacggcagcggcttggtcaggtcaattgcctggggatcgtttggatcgctatacggcggttttaaggggatttgaacgtatgacttctttggtgctacccgaataaaggaatcctcgaagttaccttcccctttgaccaaaggaatgttaaagccgggatgagatccaattgaaaataacagtgtgtcttgacttggattgatgacgtttagactcacattcaattgatgatcgaccagttcgtaaatgattcgcagttcgaatttaaacggatatttggccaacgtttcctcagtgggccgcaaaaccattgagactttggttggtaattgggattcaacttcaaactgattgtcccgggcaaacccgtgttgggtcatttcataagtatggccagcataggtgtattggttgtccttaagtcgaccgacgatcgggaacagaattggcgcatgccgtttccaaaatgctggatccgcctgccaaatatattctaatccgtcagtatctttcacggaggtgagttcggcaccctgctcgttgatgagcacggtcaaatactgatttttcaaggtaatcatttaatctcttcctcccaattttacagaatgtaacgtgaaagatctttattttgagccagtttgccaactttatcatcgacgtatttttcagtgatcgtaatatcgcccatctgcatatccggtccttcgtaaaggatatcttcaagcagtttctcaagaatcgtgtgcagacgacgggcaccgatattatcagtattgtggttgacgtcagtagcaatctcggcaattcgattaatcgcctcaatggtgaaggttactttgatattatcagtcccgatcaacgcaatgtattgtttggtcaatgagttggttggttctgtcaaaatgcggacaaagtcttctttggttaaatcatttaactcaactctgattgggaaacgtccttggagttctggaattaaatcagagggcttgttttcggcaaaggcacccgaaccaatgaagagcatgtgatccgtgttgacggtcccatatttggtattcacctgagagccttcaacgattggcaaaatgtcgcgttgaaccccttcacgggaaacttcgccactgttttgagactttcccggagcaatcttatcaatttcatcaataaagatgattccggtattttcggcgcgaacgatcgcattatggtaaagatcggccttgttgatcaattcctcagaagcctggcgggttagaatttcacgcgcttcgcttacagggacggtgcgcttgattttctttttgggcatcagtccggctaaggtatcattcaaatcgatccccatttggttcatcatcgtgctttgaccagcgggttgttgggatggatcatccatttcaatttcaacctggtcgttttccagcaaaccggccttgagtttttctgcgatcgacatccgtttttcacggatatcatcagttacttcttcttgatcgtcctgattttcagacggcatctggccattttgcatctgagtaaacatattcatcaggttctgcatctcattttggcggttctcttttttctttgccggtgccaaaagtttgaccaagcgattgttggcctgcttttctgcctcgacatggacctgtttgtactgatcagcccgttccaattggatggcattttcgaccaggtcacgaaccattgattcaacatcgccacccacgtaaccgacttcggtaaatttggtagcctcaaccttcacaaacggtgcgttaactattttagccaaacggcgggcaatttcagttttcccaactccggtcggtccaatcatcaaaaggttttttggtgaaatttcatcctgcatgtcttttgacagctgcattctgcggtatcggttccgcaaggccacagcaaccgcttttttggcctcgttttggccaacaatatattggtcaagcacggaaacaatttcttttggtgtttgagtagactcagtcaatttaagttcctcctataattcttcagaaatcacgttttgattcgtgaaaatatcgatgttgccggcaatgtgaatggcggcttcagcaatttctctggcgctcatgtcttgggcatgatgtttcatggcagttgccgcagctaaggcaaagttaccgccggaaccaattgctaaaatatcatcgtccggttcgatcacttcaccttgaccggataccagcaataaatctttgtcgttcatcacgattaacaaagcctcgagcttctgtaactgttggtcgccacgccactcttgggccagttcaacggcggaacgtttcaggtcaccgtcaaactggtttaatttcttctcaaatcgttcttcgaggttaaaggcgtcagcgacacttccggcaaagccgacaacgacttggttgtcataaatcagacgaactttgtgggcggttcccttcataatgactttttcacccatggtaacctgaccgtctccagccattgcgagatggccattgtggcgaacagcgacgatagtagttgcttcaaatttgattggcataatatacccctttgttagtttgattttaatgaatcattatttcgaggaaaatactttttataatcattcattaaatgtgatttggtaacgtgtgtgtagatttgagttgtcgacaggctgctgtgtcccagcaactcttgaaccgaccgcatatcggcaccattattgagcatttcggtcgcaaacgtgtgtcgcagcatgtggggatgaatcttcgtcgtcagactactttgtttgacgatttgatccatcagatattcgatgccccgacttgtcagcggtcggccgtaatgattcacaaataaaaatggatggtcttgatggtacttggccatgattgggcttctggcgtcgctgagataagtttcaatcgcctcttgagcatattccccaaagggcacgtatctttgcttgttgcccttcccagtgactaagatggttcggttgtccaaatcgatgtcattgagctgaattccggcgcactcgctgacccgaatgccagtcgcatataaagtttccagaacagccgtatcgcgcaatcccagttggtgattgggattttgtctggctccctgaaaaagcgcccgcatctcattttgatacaaaaatctgggcaaacgccgatgattgctcttcaagtggacatattcgaatggattgttggcgatcacagtattcttcaccaggaaagcatagaacgactttaatgccgacaccttttgggcgatggaattcctggcgtactttcgctcgtaaagatcgctcaaaaatgcttcaacatcaaacgagtccacttgggtcaatggtttgcgttcactgggaatttcggccagaaagcgggtgaattcggcaatggcctgctgataagcctggatggtatcagtagaatagtgacggtcactctgtaaatacttcagaaaccattgaatatttttttgatcttcatctgattcagccataactatcaccttcaacgatgtaatcgtgttcatgtcctaatatctatgatagcaaataaacgccgtttgtgcgcagtttgctatgaaattaaccaaaactaaatccgatcataatcatcgaataagcgtcattttaccgacctgattagcagtcatcaatcgattgtgctagtcttaaccagaacttaagcattgtggtagcctggaacctaaaaacgagaatacaaaaaaactgaatcgaataattcgatccagtctaattgattcattatccacgtgaacgaagggaagctcgaatacgagcagccttaccttgtaagtcacgcaggtagtaaagcttggcacgacgaacgtgaccttgtcttactacttcgattttatcaactcgtggtgaatgaagtgggaaaattcgttcaaccccaacaccgttacttactttacgaacggtataagtggcttgaatgcctgaacccttgcgtttgataacaacaccttcgaacaactgaatacgttctctggtaccttcaacaaccttaacgtaaactcttacagaatctccggcacggaaatcaggaatgtcattacgtagttgcttctcgttgatcttgtcaatcaattgattttgtcgcataaacaaatcttcctttcactaacattcattatcttgtctgacagcggaatgttgttttgcggcttgcgccaaaaattagtgtaacacaattattcatcgtctgtaaaggtatttttcttgtcagtatcttctgcggcttgcttttcttcttcctcaatccggacgtcagccaacaatttcttttgggtgctggttaaattgtgatggtcgatcagatcgggtcgccggaggtaagttcgtctcaatgcctccttttgattccataaggcgatttttttatggtcgccgttcatgagaacttcagggaccttcattccccggaactctgccggccgggtatactggggctcttccaagagacccgttgaaaaggattcctcaacgctggattgatgattgcccaaaacaccgggaattagccgggtaatagcgtcgatcatgaccatcgcaggcaattccccgccagtcaggacaaagtcccccaatgaatactcatcggtcacgatggaacgaatgcgttcatcatacccttcataatgaccgcagataaaggttaaatggtcatcatgtgacaactcttcagcatcatgctgtttgaatggctttccggccggatccatgagaatcactttgcccttaggatagccggcagcttcagcagtttgtttggtgtggtcgtacgcatccaaaatgggttgcgcctgcagcagcattcccgcaccaccgccaaagggataatcatccacgtgacggtgcttgtcggtggtaaattcacgaaaattggtgacatctaaatcaataatgtgattttcaattgcttttccaataatcgaatcgtgcatcgggactgaaaacatttctggaaataaactcagtacgtcgattctcattcgtccaagccctccggaacatctgcggttatcttaccggcatcaaggtcaacattcgtaatgacagaatcgatctttggcagcagtaaatctttttgctgatcgcgttcaaccaaccaaacatcattggcgccgggtgagaggatctccttcacttggccaattgggttaccatttggatcaacaacgtccaggccgatgatttggtggtagtaatactcaccaggcttaagatcatcacttgagaggctttcctcatcaattttaagttctgatggctttaagtactcaacgtcattgatcgagggatgattcttgaagtgcaataggataaatcctttgtgcttgcggacaccgtcaattgtcagcgccacttgttcgtgcttgttaggcaatttggcaaaaaccgtgttgccgactttgaaccgtttttctggaaaatcagtaatcgaaatcactctgacttcgcctttcaagccttgggtattgacaattttgccaatattataataattcattcactcactcctccagctctaatgaatctcattttgaataaagaaaaagggcctaaacaaaaccttcgtttcgcttaagaaccctattgtttcccatcgtcgacaatcagacgagctttcttttgaccctcaaccggaacactgtaaacaatggtccggatggtctgaatcacatggccatgctttccaatgattctgccaatatcttcttcgttcaacttcagatgatattccataaatcgatcggattcattatgcgaaatctcgatatccttaggatagtctaccaacggtgagataatcttattaattaaaccatcaatacttgtcatgatgataatcactcacttacttttttgagtatttagcttcgtgatatttcttcataataccggcatctgataagatgttacgaacagtatcagatggttgggcaccattgttcaaccagttcatgattgactcttcttcaagagtaatcttggcaggctgagttaatggactgtaagtaccaacgttttcgatgaaacgaccatcacgaggactacgtgaatcggcaacaacgatacggtaatatgggcgcttctttgaacccatgcgctttaaacgaatcttaactgacatgcttttacctcctgtaatgttttaacgattaataatataccagtaattcgaatgcttgtaaaggtttttttctttacaccatcaaaagaactgacggattgacttgttttggccaaactgaccaaattaatggcgtgtcaatgctgataacttgtcagaattaacggcgcttcttattctttttcttcaaacggcgtttcttattctttttcattttacgactgaactgtttcattgccagtttggacattttaccgcccatgccggtactgttcatcatattttccatgccggacatgttgcctttggaaaccttgttcatcatggttttcatttggccaaattgtttaatcattcgattgacttcttggattggtcgaccggaaccgcgggcaattcgtcggcgccttgatgggtttaatacatcagggtcagtccgttcttgatcggtcattgaatagacaatcgccttcaggtggtccatgtctttagggtccatgttggcgttttttaattggggattattagccatccccggaatcattttcatgatttcatccaagggtcccatcttttgaatttgatttaactggtcaacaaaatcgttgaaatcaaaggtattctcttggattttctcagataattcctgagcctgcttttcatcatactctttttgagtcttctcaatgagtgaaagcatatcacccattccaagaattcgcgaagccattcgatcaggatagaagacgtccaaatcagacattttctcaccctgaccaacgaatttgattggcttttgagtgacggcccgaattgaaagtgcggcaccaccacgggtgtcaccatccaacttggttaagacaactccggttacgtccaaggtcttattaaatccttcggcggtcgccacggcgttttgaccagtcatggcatcaatgaccaacagaatttcgttgggttcaacggcatccttgatatgacttaattcgtccatcaacttttcgtcgatttgcagacgaccggccgtatcaatgatcacgtagtcattatggtcttgcttggcctgttcgacaccccgtttggcgatttcgaccgggtcaacatccgttcccagtgaaaacacggggacgtcgatttgctgaccaaccgtctgcagctgatcaatggcagccggccggtagatatcatcggcaattaataacggtcgggcgttctgctcattctttaattttaaagccaacttcccggcagttgtggttttaccggcaccttggagaccagacatcatgataatggtggggattttttctgctttattcaggggaacagcttcttcccccatcgttttagttaactcttcgtcaacaattttgacaatttgttgcgagggatttagcccttccaacaccttggcaccgttggcacgctcctcaacggttttgacaaagtcacggacgacttggaaattaacatcggcttccagtaaagccagtctgatttcccgcatggttgcccgcagatcggactgggaaacttttcctttgccacgtaaagttttcatggcgttttgtaaacgctcggttaatccttcaaaagccaattaattcaccccttattgttcttcggttgtttccaaatttttgatcattgaattcagtttgtcatcgtgtggatattttttttgaatataagcttgaatgtggtctagtttgtcgttccggtcaacaaagctgtgatacaaattcagcttgtcttcatattgctgaagaatcttctcggaacggcgaatattatcatagacggcctgccgactgacgttatattcaccggcaatttcccccagcgagtagtcgtcagcataatacagttcaatatagttggcctgctttttggtgagcagtggctcgtaaaattcaaacaaagaattgatgtagttatttttttccagttccatattgaaactcctttgacggccaatacgtcatctagcgtacagatttatataacgtcagtcaacgttaaaatacctgactattcggaaatgaggcctttgaataaaccgtaaacaaagtcgtttggatcaaacggcttcaaatcgccgacctgctcacctaaaccaacgtacttgaccggcagatgtaattcactgcgaatagcgaggacaatcccaccacgagctgtgccgtcaagcttggtcaaaacaattccggaaacatcagtggtttccttaaacattttggcttgagtcatggcattttggccggtggtggcgtcaagtaccagcaagacttcgtgtggggcttcaggaatctcacgagttagaattttcttcattttacttaattcgttcatgaggttgaccttattctgcagccgaccggcggtatcaaccattaagatgtcatagtcttcttttctggctttaacaaccgcatcgtagaccacagatgccggatcacttttcgctttgcctttgacgatatccacaccatctcgttctgcccaaacattgagttgttcaattgcgccggctctaaaggtatcggcagcggctaaaacgacctttttgccttggtctttatacatcttagccatcttaccaatcgtggttgtcttaccaaccccgttgacaccgacaaacatgataactgtcggaccggattttgccatgttaatggccgaattttcaccattgccggcttgatcgtacatgtcaatcaattttttaacgattacgttttgaacatctttgggattcttggcattttgcagcttgacttcatcgcgcaactcatcggcaattcgcatcgaggtttcaaaaccgacgtcggattcaatcagcatgtcttccaagtcgtcaaaaaatgattcatcaacgtgacggaagtttgctaaaagggcattcagtttttgaccaaacgaggaccgcgacttttccaatcctttttcgtattgctgagtatttgaatctgtggctgattctgccggttctggactttcagctgatttttcaggctcagctggcatatgcgactcttctgtcgaagattcctgctcagccgatgaatttggttcactaacagttggtgctggtttttgagcatcgtccggctgctttgtggtttgttggccatttgattcttcaggctgttctgtcggttgttcttcggtcttttcagctggttcatcagccggcctcttagtggctttggcggactcttcaacatctgtggttgtttgatttgaagtggcggcgctttggtcgtctttggcaggtgcttctggtttgggttcggtttgttcagttgattcagtcggctttttttcatcgtcttttttggaacgacgtttaaatatatcaaaaagtcccaatcaactcacctccgtttttaaattatctaaattaacagtaacaacttttgaaacgcctgattcctgcatcgttaccccatacagttgatcggcgtaaatcatggtttcttttcgatgagtgatgaccacaaactgggtctcatcaccaaaacgctttaagtattttgcaaagcggtctgcgttaaacgggtcaagggcggcttcggcctcatccaagatgcaaaatggcaccggtcgaaccttaatgatcgcaaacagcaaggtgatcgctgttaaggctttctcgccaccggacaagagatttaagttgcgatagttcttgccaggcggcttaaccataatctcaattccagtatccaacatatcatcaggatcggtcaagaccagtttggcttcaccgccgccaaacatatcaacgaagacttttgaaaaggcttggctgacttgtttgaacgccgtggcaaatttagtcgtgatggtgtcatccatgtcgcgcatggtggcggttaaatgatccttggcatccaagagatcttgtttttgactggtcaaaaattcaaaacgtttggaaacttccttgaattcctggatggcaccgatattcaccggcccaatttcgtcaatcccggtccgcagcattttaatttggctggcaacctgcttttcatcccaattccagtcgggattcgctaaatcatgttgatcgatctgataagtcgtttccagagtcgcaaagttggtatccagattctggtggtttttagcagcagctgtctgggcactggtaagttcatatttggcgttattcaagttaatctgctcatcttgaatcttttgatttaactgatccaaatgatcctgcgcttcgccaacggtggctttcaacttgttttgcgtcaggttaagtgcgtgttggctggcttcggcagtcttaatttgctcgttcaacgtccccgcgtccacttgacgactgagttcagcctttaagtggtctcgctgtttgatcaggcggtcccgattctgccgatgagtcgcaatctgctttttgattcctgtttgatcaacttcaagctgattcaacttttgctgctcaacaacaatcgcctctcggacttgttgcttttccgtggtaaatttttgagccgattgtttaacgtttgccagttgaacccgtttgttatccaagtcgtcattgactgcccgcaattgtttgtcgatggcatcctgacggttgaccagctggtcggtgtcagttgttccatcggactgggcagcgttcttcaaagcgagctggagggtcttaaattcacgctgcttttcctgaacagcctcttcaagtgaatgacactggtcctccaaggttgcggtctgttggcgaatttcgaacgcttttcgttgaccacgctcatgtgacgcagtgattttagccagctcatccttggcatgctggagccgacgttcattttccgtcagcttttggtccatttgagcggtcgattgattgagagcggccaactcggatttttgaaccaacaccccttggttatcatgacgactggcaccaccggttaaggatccaccggcattgacgacttggccatccaaagtgacaatgcgcgtgcgctgattaatttgcttggaaatgttaattgcgtggtcaagcgtatcggcgataatcgtggtccccaaaaggaagcctttaatctggttgagattatccggcatggataccaaatcggctgctacaccaatgaatccaagaacttcttgtgactcgtggacgattgtcgaacttagccgccgacttttaatggttgaaattggcagcagggtcacccgccccaaacgctctttggtcagcaaaccaatggcggaggaagcggcccggttatcctcgacaatgacgtgttgggcttgagatcctaatgcggtctcgatggccttcacatatcgttgatcaatcgttaaatagtcactgaccggccccaaaatcccggttaattggtttttccgtttgagaagattcgccacgccccgataaaagccacgataagagtcatggagattcttcaaagactcggcttttgctttggcctgctcggcaattttgagtgctgccagccaattggcttgggaactgtcgacagcctgctggtgagtattcattaattgagttaaatcagccagctgcttggaaacatccgtcaattcagattggctggatgctagagcggtttgtttgttagccaattctgcctgggtttggccaaggtcttcgcgcactttattaatccgctgtcgctgtgaccccagttgctgctcaagttgggcttcatcatgagttttcatggtaatttgatttttaatgtcggttttttgctgcagtaagtcgacatattgattacgcaattggtcgatttcagattcaattaccgaaacgctattcgctttttgggcttctgccagtttgtcgaaatcggcttgtttggcagcaattttttccgatagccgtttgccggcatccaccgattgggtaagtttgacctgaaaatcgtcaatttgcttgtcagtcagtttgatttgttccgaaatccggtttaaatcggcgtccttaaaagacttctcttgggcggacaactgatgcttgctcttcagcgactgaatttgttcggttgctgtcagaatttgctcgttgatttggtcgatttgggcccggttttgagttaaattggctttcagtttgtcgcggtcattttcatcccggcgaacttgagcgtaaattttattaaccaagtcagacttttcactaacggtgtgtttgagctgctggccggctgcgatcaatttctgagttgccaaaattaactgctgcttttcaaactgatctaaacgctttttttgatccagataatccgttgccagactactttgctcttcaagcggtgccattcgactttgaagttcagaaatgatgtcttccactcgattgagattatcggaagtctcatcgatttctttttgggcagtattcttgtgctgcttgtatttgtagacgccggcgacattttcaataattgatcgtcgctcctcaggtttactgttgaagatttgttccacattaccctgagaaatgatcgacaatgacccttgaccgatgccggtatccatgaacaaatcggtaatgtccttaagacgacactgtttttcgtttaaataataggaactatcgccgttccgaaagagtttccgggaaagcttgagctcatcgaagggagacttaatgaaatggtcggagttgtccaaggttaaagtcaccgaggccatgcctaaagaccgtcgatcggcggagcctgaaaaaataacatcaggcatccgcgacccacggagatttttggcagattgttcccccattacccaacggattgattcggcaatattactcttaccgcttccattgggaccaacaattccagtcattccacccggaaacttgatgagggttttgtctgcaaatgatttaaaaccgataatttcaatggatttaagttgcacactcattctccagtctaaactagattgtcgccctcggtatcaaactgttccagggcttgttgggcggccttttgctcggcgcctttcttggaatggccaattccaacaccgtaaagtttgccgtcaattgagacgttgaccttaaacgaacggtcgttgtcgggtccgtattcgtccactaattcatagtcgatggccaccggaccgtctgcttgggcgagttcttgtaactcggtcttatgatcaaagaattcggcaaacatgccttcatcgagctttggaaaaatcactttggtcacaaaccgtgttacctcggcctgcccttggtccaaataaaggcagccgacgaatgattcaaaaatatcacataacagcgagtcccgatcacgagcccccgccttttcttcgcccttaccgagacggatatactgattaaaatgacattctctggcaaaggtgctgaaactttgctcattaaccattgctgctcgaagtcgcgtgagccgtccttgaggcatctttggataacgtttgaaaatgtagtcggagacgatcagctgtaaaactgcatcccccaaaaactccagacgctcataaaattttaagccttcaccgcgatgctcattgacgtaagaagcctgtgtgaatgcttcatcaagcaaatcctgatcgtcgatatggatgccaaaatcttgctttagcatctcatttaaaccctttatcaatcttttacctccacataaaatccagataacagtaaaaaattgaaattatatcaaacttgagataattccaatttaagattacttttattatttttgatgagccatgacaaaatcaacggcctcgttaatggtattcagcttttcagcatcctcatcggaaatttctgcgttaaaagtatcttccatatccaatacgaattcaacaaaatcaattgaatcagcatcaagatcgtttttgaaatttaagtcaccggtaattttacttcggtcgacatcaaactggtcagccaccaaatcggcaattttattaaacacttcatctttgtccattttgataaacacctatttcataaaattaatttgctaatgattattatatcaactatttactgcttttgatactatcttttatctgctgcagttcatcagcatggtcgacgacgtattgattcagatcaggaatcatatttgaggcaataatctggcggatttggccaatcgtattcttcaccgtgtctgctttgctgctgccatgtgtcttgacgaccggcgcattaacgccgagtaaaactgcgccgccatattgtgaatagtccattgaaccaccaattttgtggaaagcttcttttaacatcaaagccccaaattttgccttagtgccgctatccatgatggtcgtcttaattaagctgagcatcgacaaagcagttccctcaatgctctttaatacggcgtttccggtaaagccgtcggtcacaaccacgtcggcggccccgttgagtaattcacgggattcaacgttgccgacaaaattgatatctttgtcggctgccaaaagatcatgcactttccggtgattcatatcacctttatccgcttcggtcccgttgttcaagagaccaattcgtggattttcaacttggttgacgttttgggcgtaatattttcccatcaaggcatactggtaaatatttaaaaccttggtgtcggcattggctcccacgtcaatcatcacaaatttatcttgattcttaacgccgatgaccggcaaagtggtggtcaatccgggacgatcgattcctttgatgcggccaacgataaacaaaccagcggctaaaatggcaccagtgttccctgccgagaagaatgcatccgcagttccttctttaacggcggttgctgccagaacgatgctggattgttttttggtacgaacggctttaaccggttcatcacccatttcgatgacttcatcggcttggacaatctgaattcgatcatcatttttaagatattttttaatttggtcggtttgaccaaatagttggaattcaacatcggcataagcatcccgtgccaattcaattccttcaacaacttctttaggggcgtaatcgccgcccatggcgtcaactgcaattttcatatttaactcctatttaatccgtagtaatagtttcattatattttaaatactgtgataattgtacattttctggctgcttttgccagtcttgatgaaccgtaatactctgggcctcctgattggcaacttgtaaaatattcaaatcaccaaccggatcggccactttgaaatcaggcatccctgattgtttactgccggtgatgtcaccttggccacgcaattccaaatccttttgggagaggaaaaagccgtcggtgctgctggcaaccgccgtcatccgctttttacccaactcgtttttggggtcggcaatcaaaatgcagtaggactgcgtgtcgccacggccaacgcgaccgcgaagttggtggagttgtgccaaaccgaaatgatcggcatcaaatatcagcatggtattggcattcgtcacgtcaacgccaacttcaatcaccgttgtcgccaccagaacttggaattgattgttcttaaaatcggccatggccgtatccttttcttcatcggacattcgcccatgtaggagaccaaccgaatactgcggttcaaaaatcgctttgaaacggtcgaaaatcgccatggcgttcttcatatcgacagcttccgattcctctatcaacggtgtgacgacgtacacttgatttccggcatccaattgtttcttaacgaatcggatggcactatccgttttagcggaggtaatccaagttgtcttaattggcttgcggccctttggcagttcgtcgatcacagaaacgtccatatcaccgtacatcgtaatcgccagtgtccgcggaatcggcgtggcagtcattgccagcatgttggtactatttcccttcagtcgtaaggcctggcgctggttgaccccgaagcgatgctgttcgtcaatgaccgccaaaccaagatcgtgatagtcaacttgatcttggaataaggcgtgggtgccgacaatcagattgacttcgccgtcagcaatccgtggcagcatcgccttacgggctaggccagtggtcgccccggtcaacagggcaatgttgatatcaaatttttcaaacaacttggcaaacgtgttggcatgctgctcggctagaatttcagttggggccataattgcggcttgtttgccggcactaatcgctgccaaaatagcaattgcagcaaccacagttttgccactaccaacatccccttggagcaagcgattcatttccaatggtttgcccaagtctgtcaagatttcattgacaactttgttttgggaatcggtcagtttgaattttagttgactggtgaactgcccaaccagatcgggatcgtaggtgactttggctgccggatccggttttctgtggcgctgttttaaaatttgaattttcatggcaaataagaaaaattccatgaacttggcagttcgaaaagctttttgggcagcgaccggtgatgttggaaaatggatattttgaatggtatcgtggaaagattccaatcgatacttggtgcgaattgattctggaataacgtcaactagctgatcctggtattcatcaaatccaagcttgatcaattgcttaatggtattttgtttgacttctttgttacttggatagattgaatcataggtatcgcttttttcgccgtttaaaattttcatcccttgaatctggttacgattgcggtcaaaggtaccaaaaataatcacttgggcttccaactcaagctgctttttcagccacggctgattaaaaaaagtgacgttatagatttcatcattaatttttaaatgaaaaccaagccgacttttgcgccgaccaaaaaaacgaacagttggctcgctaatcacgatccctttgacggtgactttttggccatcgacggcagttcttaaatcttttagcgataaatcatcatatcggcggggataataagtcagtaagtcgttgatggtattgattccgagcttattaaaagcagtcaggcgcttttcgccgactcctttgagaaccccaaccgaatcacttaagctggccaatgttatccctcctttgtcattgatataaataaaagcttggccagtgttgaccaaacttttaggaattgtttattcaaccgaaattaagaatgggtagactggttgatcaccttcgtgaatctcaacttccagttcgtcatccaatttcaaaatgccggcctggactttttcggcagccgcctgatcagcgccttcaccgtaaatgatcgtaatggcttcactatcgtcatccagcatcttcttaaccatctggatggccgtgtcaatcagtttatcaccaatggtggcaatatcgccgtcaacgatgcccataaattgatcttttttaatatccaaatcatcaatcttagtgtcacgaatggcggtcgtcacttggccggacttaaccgttggcaaattatcttccattgccttttggttatcttcgagcgaattttccggattaaagccaagcatggcggtaatcccttgtgagatcgtctttgaatgaacaatgaccgtcggaatatcaaccaccttggcagcttgttcagccgccaggaaaatgtttttgttattcggcaagacgattgcctgtttggcttttgtattttgaattgcgttgacaatgtcttcggtactaggattcatcgtctgtccgccgctgacaatgtagttgacgcccaaactttcaaacagttggttcagccccttgcctgaagaaacagaaataatggcagtatctgaagttggctgttgggtgctgatactttcagctttttgaattggtgaagcatcctcttggctgtcctcatcttcttcaatgatggtttcttgttgaagtcgcatgttatcgactttaacagttgccaaatctccaaactcctgaccccaggcaagcactttgccgggatgttcagtgtgaacatggactttgacaatatcatcatcgttgatcaccagcaatgaatcgccaagtttggcgagataatcataaaaggtctgatagtcaaactgatgatcgacttcgcggcctttgccgattcggaccataatttgcgtacagtagccatacacgatatcttctggatttaatttactttgaacactttgatcggccactttaatcatctgattcatttccgcatcgttaggttgatattcaccagattcagcttcgtttctgccattcaagacatcatcgaaagcttccaaaacgaataccaatccttgtccacccgagtcgacgacgccaacctgcttcagaaccggcaataaatccggtgttttctccaaagcggattgtgaggcctggtagatggcatccatgacagcgacaacatcattggtcgtagcggctgctttcttaccagcagtagcggccattcgcacaacggtcaaaatggttccctcggttggcttcataacggacttataggcgatttccgtcccggcaacgaaggcatcagaaatatcttgggcactcaaagtttctttaccctccgtggacttcgaaaagccccggaaaatctgcgataaaataacccctgagttgcctcgggctcccattagaagtcccttagccaaagcagcggttaaatcgccaacgtttgtcttgacatctttattcacatatttataacccgaagccatggataggctcatattggttccggtatctccatccggaaccgggaatacgttcagtgaattgataaaatcagaatttttatttagtttagttgcggctgcttgaaccattgccgtaaattcggtgttggtaatttctgtaactttcaacaacttgtcctccttggtcacttgcataatcagtcattcattacctgaacgccttgaatgatgacattgaccgaatttgcagataccccaagcatactttgtaggttatacttaacctttgcttgaacgtttttagaaacctctgaaattttgttgccataagcaacgataatataaacgttaacttcaatttcattatcgtgttgtttaaccacaacacctttgaaataattctcgcggtttaaaatcgtgttgacattgtctctgagctgattgcgacttgccatacccacgactccgtaattatcggtggcagccccaccaacaacatttgcgatgacgttgttgtcgatgtcaactgttccaaatctggttttgattttgacggccatgtgcagcagcctccttaattttctattaacctattaacgatagttaatattaccacaataacgctaaaaaccaaagtaatcttgatgcccccaagaagactgtcaagtataattacttgaaagaaaagtattgcaatatcaatgtatgtatgataaattattctagtgtaatgaaacagactttaacactaaaatcaaagagaagggagatttgttacccatggcaaaggattttattaacggtaagcgtacccactttggtaacaaacgttcacacgctttaaactcaagccgtcgcagctggaagccaaatttgcaaaaagttcgcattcttgttgatggcaagcctaagaaggtttggatttctgcccgaacacttaaatcaggtaaagtaacccgtgtatagtaataacttggatcgatgttaatcggtcttttttattaccttcaaaaatagaggcaactctcagcagccgttttcggtgagctgagggttgcccctttttttagttataacgattaatatctttgctttgaataacacacatcaccccactgccaaatttaaacctggcagtttcaccaacaaattcgttgctggcaagcgacattgggtgtttaacctgataatcattcagctgatatttttcatcaaacaaagttaaatgatccatcggcgttaacgccacaaaggccaaatattttttatcaggttctttttcaatctgataagtccctggcaaaaagaaagtaatcgtattttgcttgtcaatcattcgaattttcggtgcgtagggcttgaaccggggctccaaaaccatccacagattggctagaaaatgatccagccgaccacccgtcgcaccgtaaatgtcaagtcgatcggcgtgatgttcctgcaaggcgaccttcaaccccaattgggtatcagtatcgtctttttcaggaattgattggcggatatccttaatgtggtcacgaaccaattgaagttctgccggttttaaggaatcaaagtcaccaatcgcgacaagtgggtcgattccccgttcaatcaaatggagattgcctctatcgatgccgatccaatcacctttaatctgtccatttttcaattcgtctggccagaggtcaatggggccgccaaccaatagatttaagatcttcatttatttggtcgcatcctttattgctttgattcggctaacaggatcatcggcgtcaaaaacgtatgatccggcaactgccaccgttgcaccggcttgataggcacccacaaccgtgtggtcattaacgccaccatcaatttcgatgtcaaagttcaagccttcactttttttcaactcatcgagttctgcgatctttttaaccgtttcaggcaggaacttctgaccgccaaatccaggattaaccgtcattaccaagacctggtcaaccatgtatagtactggcttgatggctgataccggcgtacctgggttgatgacaacttcagccttgacccctttgttcttgatcatctgcaaagcccggtgaatatgaggggttgcctcaacgtgaactccgatgatatcggctcctgcatccgcgaattggtcaatgaaacgttccggttgttcaaccatcatatggacatccaagatcatcttggtgatcggacgaatggctttgacccacccaggtccataagataaagcggggacaaactgaccgtccatgatgtcgatgtggagcacttctgccccaccctggtcgactttttcaatatctttttgtaaattgacataatccgcgctcaaaattgaaggtgcaactttaatcataactaacttcctcactttttataatttggtttccggtttttaatgtcggtgtacaactgcagataattctcataccgactctgcatgatctcaccgctggccacttcttttttcacttcgcagtccggctcattgacgtgcacacatccccgaaagcggcacttcacagatgcccgcttgaactctgggaaataattggcaagctggcggtaatcgatctccaaggtatcatacgaggaaaatccgggagtgtctgcgatatacccatcgttgacccgcaataaagcaacttttcgggttgtgtgttttccacgatttaatgccgtagaaatctcaccggtagcgagctgcaaatccggtgccaagtgattgagaagtgtcgatttgccggcacccgtctgtcccattatcacattttcttttcctgaaaacaattgccgtaaatggttcaacgaattttcatcaaacgcggcttccggcagaataacgtcataaggaatgttagcgtaggcaactgctaaatctttaaaataattcagttgtttttcagataacagatccgtcttggtgaaataaatgatcggcttgatattggcaatttccaatgcaatcaactgacggtccaataagttactggaaaactccggctgagtggttgccgtcgtcacaatcgcctgatcaatattggcaatcggtggccgaaccagagaattctttcgtggcagcatcttcaatatgtatcctttgtcgccatcttcaacttggaactcaacgtcatcgccgaccaacggtgtaatttgacgctttcgaaaattccccctggcgcgtgttcgataaaccttgccttctgagtgaacatcataaaagccactcaaagactgaaaaatctttccctgtttcaattgatcacctcgataaaaaatcacttcccttacattataagagaagtgactttgttttgcagtaattattaatgtgaatcgtaggtcacgttgttatcacgcatgatcgtccgaccatcgcggaccactttgtattgaccgacttcattgccagacaatttaaatggcaaggtgacttgcgtatcctttgtgatcaccatctgcttgtaaaccgtcgacaaactatgatcatggtctttgagataaatcaagaccacgttctcgttggaaccactggaactatctgtggaagcagcatcactggagatgccactttcattcaatgtggagtcagatgatgccgccgaactgttgtcgaggtacgggatgataattttaacattgaaactcttcaattcatccgaactgtctttcttaggcccacgagaaatccaaaccgcgacgttgccgccctgttgaatcgattcgttggcatttggtgattggcggacaactcgccccttgggctgatcgtcagagtagacataatcaaaagttgggttaatttccaccttgttagaatatgagaccacttgagccttggtcatgccggttaagtctttcagcgtaatccgtttaacaccggttgaaaccacaaaggtcagtgtcttggtagccggattgaaccgtttgccggactcaaagtcctgttggagaattctgcctgagccaaatgaacttgaaggagcgttacgccgatgaaccgtaaacccttcgtcttccaatttctgtttgacaacatcatattcttgaccgacatagttgccgacccgaacgcgacgaggcccggaactcacgaccaaattgaccttggtgccctttttgactttggtttcttccttgggactggaactgatgacgcgatgacgatcaatcttatcactactttgatatttgacactgccaacggtcaaattagcggctttaatcttggcttccgcctcagtttccaacgtcccggagacaattggcaccgtggttttcccgttagctgaaacaatcatgatgaaggccagaataattaacagcaggccaacaatcccaccgataatccaccatcttcgtcgccgttttttcttcggcggctttggtttgtcgttcgaggtaccggcaggcttttcctcgcgtttagccggattggcatccgctgaggcagtcgtatcatccaatggtgaaaatggcatcacccgggttgcttcatcaaccgggttttgtggcggctgaaccgtaaatttaggttcattagcccgtgacttgtccaatgatgtattcaaatcagcagccatttcattaactgtttgataacgatcatcgggattcttagcggtggctttcaagacaacattttccattgcctggggaatgcgcggatcgaaatccctgactgaaggcattggcgtttgtgaatgtttaatggcaattgaaacggcggtatcaccgttaaatggcactttgccggtcaagatttcatagagaataatccctaatgagtaaatgtccgatctggcagtcgccatctggcccttaatttgttcaggggacaaatagtgaatcgagccaataatcgaacgagtctgagtcatcgtatcttctgtaccggcccgggaaattccaaagtcggtaatcttaatataaccgttcttatcgaccaaaatgttttgaggctttaaatcacggtgaataatattatgccggtgggcttcactgacagctgagcaaatttgctccataatattgacaacttcggcatagggaatgggaaagttgtccttgatgtatttctttaaatcttcaccgtcaacaaattccatgaccaaatactgcatcccctcaacctcgtcaacatcataaatgccaacaatgtgaggattatccagttgggtcgccgccattgcttcatgctgaaagcgcttcttagctttggggttgtctcggaaatcaagtcgcaacagtttaacggcaacttttcgcttcaaaatgaggtcttcggccaggtatacgtcggccattccaccctcgcccaagcgaccgataatttcatagcgaccgtttaatacatagcctttattcatcggcggtcacctccgaatcgtattgggcgatcaagacagtaatgttgtccaagccgccattttgattggccaaggacaccaacatgtcacacttagtctgtaattcttcatccattgacaaaattttttcgatgtcggcatcgtcgaccatattggtcaaaccgtcggtacagagtaaaatttgatctccaggttgggcggtatacggtttgaagtcggcggccgaatcgttgttgattcccagactcttggtaataatatttttgtatgggttggttttggcctggtctggagtgatatcaccgtgtttgaccaattcattcacataggaatggtcttccgtgatctgagtgaattgcccgttggaatagacataacctcgactatcgccaatgttggcgatcagactctgtttgccatcaataagtgtcgccacgatggtcgtccccataccatggagtcgtgtgtccgtgttggattcatcgataatcgcggtattttcttttgccaactggttttcaaaccaagtttcaattttatccaggctggaaatactggtcgtttcaaaagcggctcccatgtgggtgacaaccatttgagaagcgacttcgccagcattattgccgccgattccgtcggtaattaatgccaaaatgaggccggtttgatttttgaacgcgccgaccgcatcttcatttttgtcgcgaacttttccagttgaggattgatatgcaatttgcaaattgatcaactccgttatgatttccgaatgagggagcaaacaaagaagccgtctgaatcatagtcatcggggtagatttgaaccatcttgctatccggattcaaatgattggcagtctttgtcttcgtgatttcaaaattagggttctcgctgataaacttggcgatcacgtcttgattttcctgtttaacaatcgtacaggtactatatgtaatagtaccaccagttttaactttagcggaaacggcattcaaaatttgtaactgaatctcacttagacgattgatatcagcaattgttttgtcataacgaatctccggctttcttctgaggagtcccagcccagaacacggtgcatcaactaaaattgaatcaaacaagccgtcttcaaatttggtatcgactttgcgggcatccaattcaaaagtttcaacttgcttgtagactccgagacgagtggcatttcgctggacggtctttagtttgtttttatgaatatctaatgcaaagactttgccggccttcaaacggctggcaatttgggtagttttgccgcccggggcactgcaggcatccaaaacgttgttatcaggggaaatctgcattgattcaactggcagcatggcactttcatcctgaatggttaacaggccgtcagtgaaaaagtcactgtgaatgatttggccatcgttaataataatcccttcactggaaacttggctgggttcggcatcatagccgtccttggccaaatctgccagcaaatctttttgagagattttggctaaattggcacgaaccgattgttttggcgctttattcagggatgctaagattgaagccgtttttggcttgccaagttgttcgtcaagcatttctaccaaccaggttggcacactatattcaatcgatagtcgggtcttttcgtcctgaatgtcatccaagtttggcatcccctgccgatccatttgatgcaaaataccggtcacaaatcggcgggtgccgtcatggcccatctgcttggcaattttaattgtttcatcaaagattgcccgcttgggaacccgatccagatactccaactggtacatcgcggtatagagcaactctttgacccaggcttcagtcttttccggttcacgcaaaaacggccggagttgatattccagcgttaatcgatgctgaatgaccccgtacacaatgttggtgaacagtcccttatcagctgggcccattgaagtggattgaatcacggcattaatctgcagatttgaatatgaaccattactggtgcgaaccaacgtcatgactgcaagttggcgtggattatttgttgtatatttcatttatttaatcacctgttggccaactttaagtgactgaccaatcccatttaagtaatctgttatttgttgttttggtttgccggcgggctgaagctcctgaatggataaaacagtgccttttcctgctgacaataataattgatgcttggttttctcaaccactgatcctggcgccatttcagtggtttgatcgacgacttgtgcccgccaaattttggttcgtttaccgttgataaccgtataagcgaccggatccggccgcagggcacgaactttggcgttaaccataaacgcggtttgattgaagtccagttgctcttcttccggtttgatgttgggtgaaaagacgacttgatcctgatcttgaggcactggggagatatcgccggtgatcacttttggcaaagtggctaacagcaggtcgcggcccacgatactgagtttgtcaaacatcgtctcggtatcatcatctggctgaattggaaccgctttttgtgccaaaatgtcgccggcatccatctttttaaccatgtagatgagactgatgccggtttctgaatcaccattcataatcgcgtactgaacaggcgcgccaccacggtacttaggcaaaagtgagccatgaacattgacggccgcaattttgacggcgtttaacatcttcgtcggtaaaaattgaccgtaggctgccgtgacaatcaagtctggatgaaagtcaatgacccgctgcatttccgggctcccactaagtttttcaggttgaaacaccggcagatgattggcaacggcggcttgtttaaccgggctttgtgaaatccggtgtttccggccgactggtcgatccggttgggtgacaacacataaaatatcgtatttttgatcaagtaatccttgtagaattgggaccgcgaactgtggcgttcccatgaacacaactgtcgtcaaatttatcgtttcctttcgtgattcaaattacataaagtccagcggttcattatcaattgcaatttggaggccttgacgttgctttttttgtgactggactaaaatctcgtctaaagtggcctttaactgaggttcctttcgatacttgataatgatttggtaatagtaacggttgtcaattcgggtaatcgtttttggcgttgggccgagaatgattgcctgtggggatagctgcttttttaaaaagttcataatcccaaacatctccgaagccgtttgattctcactgggagaattgccggttaacttaactgtatagtagtacggtgggtatttgccatcgtggcggacacgcatttcggtggcgtaaaacttctcgtaatcctgcgttttggccaattgaatcgcataatgatcagggttaaaggtctggatgatgacctccccggttttgtcggctctccccgagcggcccgagacttgcgtgaggagttcaaaagtccgttcacttgatcgaaaatctggaaactgcaacgctgaatctgcgtttaagacgccgaccaaggtgacttcaggaaaatccaatcctttggcaatcatttgcgttcccagcaaaatatccgccttgtgggcgccaaattgatcaataattgcttcatgagacccctttttacgagtggtatcaacatccattcgcagaactctggcagttggaaacatgtctttgacctgttcctcaagctgctcactgcccatgccataaaagcgaatccgtttactgtggcattgtgggcagacagttggcaccggttctttgtggccgcaataatgacaattaagggtatgtgtatttttgtgcatcgtcagcgaaatatcgcagttggggcatcgaggaacgtacccgcagtctcgacacatcaaaaaggcagaataaccgcggcgattcagcaataaaatcacctgctcatgtttgtcgaggcgaacctggatcgcatcggccaattttgtcgatagtgcactgtggtgttttgccagttcagttttcatatcaataatcgaaacgtgcggtaaagcatgctgattgatgcgatgcggcagctttaacagtgtatagacgcccttcattgcccgtgcacgggattccagcgatggagtggcacttcccagtaccacggggcaattattataggcagcccgccatttagcaacatctcgggtttggtagcgagggttgtcggcttgtttgtagctgctgtcatgctcctcgtccataatgattaagccaatattgctgagcggcgcgaacacagctgagcgaaccccaacgaccactttggctttcccttggttaatccgctgccattcatcgtagcgttcgccggaagacatcgcactatgaagcatcgccacttgatcaccaaatcggctgcgaatgcggccaacaatttgaggggtcaaggtgatttcgggcaccagcatcaacgccgtccgcccaagttccagcgcgtgggcaattgactgcaggtaaacttcggtttttccagaaccggtgacgccttccaataaaaagacctgatcttttttgtggacgaccgcctgttcaatcgaatcgactgctgcttgttgatcaggttgtaacttaaacggctgactgggggcgacatctctgagaaatgggttgcgaacatggcgcttcaatgttgaagccacccaccccttcttttcggcagctttcaaagtggcgctggtcactccaagggatgcccatttggaaaccagaagtgtttcgttttgatgggtcttgagcaggtttaacaattgaatttgtccacgagcatttttccgtacggttttgagggcgtcatcaatctggacgtcatttaattgacctcgataagcttttcgcataattggccgggcgcggttggtgagatcatactcaacttgaatatcgccggctttctgcagatttaaaatctctgctaaaacctgattattatatttctggcggtcatattcgacttctggctgtccttggaagatttccggatactgctggcaaacttgttcatttttggcaattagtttcttttggttcttagtccgcattccacctggaagcatggtttgtaaacagctgattttaaaggaataggtttgatcagccagccactcagccaatttaagtaactcagaattaacgactgggtataaatcaatcaggtcggcaatcggtttgagtttgccgttgaagctggaactgtcggaaagaccaaccacaaacccagtaattttgcggttgccaaaaggaacctggacgcgcatgccaggttgaatttgatccgctaaatgatctggaatcgaatagctgaacggactgttggtttggcgtgctgggacgtcaacaataacttgagcaacctgcaaggcagattctcctttcactgattttgcatttgtgtggcaataatatcgattaactgatcggcaacctttgccttactctcgacattcgtcttaatttgcttaccgtcagcaaataaaaatgtcacttggttgttatcggcgttaaagccaatcccgctttgggaaacatcgttagccacaatcatgtccaaattctttgattgaatttttttggtggcgttgctgattaaatcattggtttcggcagcgaagccgatcactaattggccaggctgtttgatagtggcaatttcttttaagatatcgggatttctaacgagttccagggtcatggtttgattatcagctgtttttttgatttttttatcggctaccttggccggtcgataatcggcaacagcggcggccattaccaaaatatcagcgtgaacaaaggcttgtttgacatctgctaacaattcagccgccgtttcaactcgaatgaaattgacgccggatggcggggtaatcaacggattagccgcgatcaacgtgacattggcaccggcatttttgaaagcgttggccactgcgaagcccatttttccagatgaatggttggttaaatagcgaaccgggtcaagtggttcacgggttcctccggcagtgacgacgacagattttccggctaaggatccacctttcagctttaagcttccatcaacccacgttaaaatttcgctgggttccggcatccggcccttcccggaatagccctcggcaaggaagccttcagccggttccatgatttgaataccggcttgttttaagttggcgatattttgttgggtggcaaaattggcgagcatgtgagtattcatggcaggcacaacaaataccggcactgccatcgttaataatgtggaagtgacaatattatccgcaatgccattcgccattttggcaatcgtattcgcggatgccggggcaacaattgccaaatcagcatcatcagcagtcttgacgtggggaatgattgtcggatctttactgtcaaaatcgctggtcaatacggtattcttactgacagtttgaaatgccagcggtgtcacaaacttttgggctgcttcactcataatgacgtgaacatcgttgtggttcttcactaataggcgtaccagtgacagtgatttgtagacggcaatgctgcccgtcacaaatacggcaacgtttttgttttgaaacattcttccaccccgtttcagatttcattctttattgtaccaaatctaagacggataaaaacagtcggcgtcttaaaagttggctgcaccccagtggaaaaggcgattaacttcaaaatgatccccccggattgctaacgccgagtttcggccgggatcacaagataagctgacaacaggattggctggtatcatcttgtccaacaaagacaaagggactgccagcaaaacagtcgttttgccgcagtcccttaatgatcaatcttattcaaaatcttttgctttaggatcgattttcaatacaccagcagcaatttcttccaaagctttgccgactgatttttgtgatttgtagtgatccaataatggcttggcaccggcatccaattcatgggcccgcttgctggaaagcgcaattaatgaataacgggaatcaattttatctaacaatttatcaacagatgggtaaagtaacataattatttatctcctaacattgactcataatcgggcatcacccgagcaacttttaatcgttcacttctaataatcgacttgattcggtcaacagccaaaggaacctggtcgtttaagacggcgtaatcataattacgcatcatgctgatctcgccgacggcctttttgatgcgcttattaataacatccatcttgtcagttccacgaccaaccagacggtgttttaattccattagatctggcggagtcaaaaagacgaagaccgcatcaggaacattggcgcgaacctgcatggcaccattgacttcaatttccaagaaaacatccttgccggattccaaggtctcgttaacatattttaatggggtcccatagtagttgtcaacatacttggcgtactcgagcatttcaccattctgaatattctcttcgaactgctctttggaaacaaaataataatcgacaccgttcttttcaccgggacgcggctttctggttgtcattgaagttgaatattcaaaatcaacatcaggctcctcaaacaaggccttacgcaccgttcccttaccaactccggacggtcctgataaaacaatcaacattcctcttttagccatcgaaaaaatcccttcaattatttgtaatacctgctattatcgccctttttgccccatttgacaagtcccagggcactgattaagaaatttgcatttgggggttgcgttttagaacgaacgttcgtataatgaagctacaaacaaatgttcggggtgaacaaaatgcaaaacaaacaatcatatctctcagaaattaccaagacctttcgaaccaactatgatcgcttcttcgaaattgtccgtaacactcaccaaatcaaacaaatgccgactttccagctgcattatttcattcaacagacactcgaaaacaactttcccatcacgatcgaatttaacgatcaggataatgaacagaccggctacttaaccaaactttccgcagaccgttacctattgacttcagatgataatcatttcactcgaattgtgaagttgtcagaaattaaagcgattcgtaaatactaagattatatcagattatattttagggcttgagacaaaactgaatgttttgtcccaagcccttttgcatttttaggattaatctgggtaaacagtgcgttcaacagcagcttccaagtggatagcggaaattaatcatttatttttcgacggcacttaagatgctttgatcttttgtttttcctcatccgccaatttcaacagctcactagcatgttccttggttaacttggtaattgccgttccggaaagcattcgcgagatttcagcgacactttgggcggttgtcagttccgtaatcgtcgtggttgtccgattgtcagcaatctttttttcaataaagtcgtgatgatcactcatcgcagccacttgtggtaaatgggtaatacataaaacttgagatttttgtgaaatcgtataaatcttattgccaatcgcctgggcaacccgtccagaaacgccggtatcgacttcatcgaaaataattgatgtgacaccagcagccttggcaaacatggtctttaaagccaacataatccgggacaattcgcctccagaagctgacttgaccaatggcagcattttctcaccaggattggtctgaatataaaattcaactcgatctgcacccagccggtttaaagcacgattttgctggatattgacctcaaagaccgctttatccatgtaaaggtcggataactgctggtgaacggctttttcaagctttttagcccaccggtggcgaatgtctgagatcttagttgcctgctgaatcaaatcggatttgagcgtggctaattgcttatccaaatcgtcgctggcttcggcatcccccgacatttgtttcagttcctgtttgattttggcaagatagtccaaaatttgactgactgaatcaccatatttgtgcttgagttgatagatggtgttgagacgctgctcaacttgatccaaacggtcctgatcaaattctaaattactcaattgatcggaaatctgactggcaacatcttgaagcgcgaagaaagctccggatagattatccgaaatttgtttatattcaggatccaaatcttcaatgtcctgcatcgaactcattgccgatccgattgaatcaattgacccgctggcctcctcgtcgccgttaatgccttcataactagccaagagcgcatcatgaatcttttgaaaattgttcaaccggtctctttcagcgactaaatctgtgtcctcattctcatggagatcggcagcttcaatctctttaatttgaaatttgagcatatcaacccgttgagcccactgcttctcattttgatgtttcttttgatttagatcgcgcagcttaataaattgatcgtattggtcttgataagattgcaaaacacttgccagttcatcttcggcatagtcatctaataattgaatgtgccgttccggccgcattaactcctgatgatcattttgaccctgaatatcgacgatcgtttcgccgattcgtttgagggtggcaatattgaccatgattccgtttacccgacagctgttgcgaccattggcaaaaatgacccgctcgataatcacgttaccgtcactgtgatcaattccaaggtcatcaaggacgttgtaggtggggttatcatcatgaaggatgaagtttccctgaataacggctttggaagccccggtccgaatgagatcatgggatcccctgccgccaaccaagaggccgacagcatcaatgatgatcgactttccagccccggtttcaccggttaacacggtcattcctgcctgaaaatcaatatctaagtgttcaatgattgcaaaatcggtaattgatagttcgagtaacatgttttcaacctctcaataattctattcagttcccaacatactattgatctgattgcgcatattaatcgcatcggcttcggttttgccgataatcaagaccgtgttgtcatcgccgagggtgccgaaaatcccgctgtagttcatctggtacatcaaactagaaatgaccggtccactaccaggtaagactttcataaagaccaacttgtcttgagagtcaaccgacacaaacgaatctcgaatcgattgaaccagtttcttttcagtatcaatatttttttgcgtcggcaaactgtatcgatacccaccggtaactgaaggtactttgacgagctgcatatctttaatgtctctggaaacagtggcctgagtaacttttatcccctgcttatccagtagcgagacaaaatcttcctgtctttgaatattattacttgtcagtaattgtttgattagcctttggcgttctttcttacgcatcattacacccccaacaataaaattgaataaaaatacaggtttacgaaccctttaattcagaataagcgttctcgatgactttttcaatcgaaacatttggtgacatgactggttgatcatcagattctaactcaactaaaaattcaatattgccagcgccacccttgatcggcgagaaatcaaggttttgaactgaataaccgttggccacagcgaagttcagaattttttccaagaccattttatgcacagcgggatccttaacgataccatgcttgccaacattggccttaccagcttcgaattgaggcttaatcaaagccaccacatgaccatttttagtgatgatctgtttcagcggtggcaggattaactctaaagaaatgaatgaaacgtcaattgaggcaaactcaggctgtccatgggtgaaatcggccaacttactgtacctgaaattggtgtgttccatgaccacaacccggggatcctcccgcagtttccagaccaattgattactgccgacgtccagtgcgtagcttaatttggcaccgttttgcagcatcacatccgtaaacccgccagttgaggagccgatatccaacacggtcagccctttaacattcagatgaaatactttgagggctttttcgagttttaacccgccacgactgacatacggcattggcttgcctttaaggtgcaggtcggtatccacagggattttggttcccggtttgtccaaccgttcttcgttatcaccaagaatctctcccgccatgacggcacgtttggccttttccctggtatcaaacagtccttgggttactagtagtacatcgactcgttgcttttccatattacttttcgtccttatttttaaaatagcttgtgaaatcatttaacagactggtatcaatcgatagcgcttctctggcagttgcgagggcctgctgggcatcggcgaccgtctgattcagcatttcatatgatttggccaaaccaagcaaattgggatacgtatttttattagcgtcctggtgaaccggtttgccgatttctgcttctgtcccaacaacgtctaagatgtcatcgtaaatttggtaagcttcgccaaacttctcagcaaacgttaacagtgacttgcgtttttccggaataacccggcccataatcaggccagcttcaacggcatagcgaatcaaggcaccggttttgttgcggtcaagtttttgaagccctgacaacgatagccgggtgccttcaaattcgatatcgtcggcctgacctgaaaccatcccatgggggccggcagctttggcaagtgccaaagtcagttcagcttgggtttgactgtccaaatcattatccaccagccactgaaatgccagtggttggaggccatcacctgcaagagttgccatcccagcgccaaattttacgtgattggtaggctttccccgtctgaggtcatcattgtccatagccggcaaatcatcatgaattaaagaatacgaatgcattagttccagtgcacagctggtttttaagacggtctggtcgattgggtcgcccaaactcgccaataccgcaagcgtcaacaagggtcgtaagcgtttccctccagcgttgactgaataaatcatcgctgcttccagagtcgtctgatccgtatccggtttgatgtcattttccaaaatctgattgatttttggaacccacaaccgttcaaaatcagttaggttggttgccatcgctatcatccttttcatctttaggtgcttcgaattccacttcattgccatctttgtccatcattttggccatggtgtgttcggccttggttaaggtgtcttgaagctgttcactcagttgaattccggttttaaatttggccatcgactcttccaaggaaacgtttccctgttccaattgattgacgatggtttccagttggtccattttttcctcaaaggtttgattgtcttgtttatcaggcatattatttctccttctttgcatttatctgattgacagaagcgttgacgataccgtcactgaaatggacatcaattgttttgctgctcaagtcggcaacccgtttgataaaatgtccctgttcgtctgtggtgtacgtataacctcgactgagaatcttcaacgggctcaagtggtcaagtgagccgaccaacatctgataatgttgggaaacatttttcaggttctgagttgttgcccggttgagtcgacctttgagtgttgccagtttttgctgctcttctctaatcgtatatgttggcgcgaccaaacgcaggcgcaatttaagatcagaaaaacgatcctttcgtttaccggtaatcttgtcagattgattatagagtcgctgcgtcagtagatccaaacgttgagcaaaagtttcgtaaatccgttgaggtgtcgtgaaaacagtggactgccggagtcgcttcaatcgctgtttgtcttgctgaacaacctggtaagtcgcattaatgatgcggttttgggtcgtcctgaggtcaactaacacttgatccaacctgggaactgccagttcggcagctgccgttggtgtcgcggcccgaacatcggcaactaaatcagcaattgtggtgtcggtttcatgaccaactgaggaaatgactggaattttactggcaacaatcgctctggcgacgttttcttcattaaacggccacaaatcttcgatcgatccgccaccacgcccgacaatgagggtatcaaaattgccaatttgattgactcgctcaatttgtcggacaatgtctgcactggcctcggttccttgaaccagggcaggaaacaggacaatttgggcaatcggatatcgacggcggacagtggtaataatatcgcggataaccgcgccgcttggcgaagtgacgaccgcaattcgtttgggaaattttgccagcggctgcttgggcaaattgaataacccttcggtggacagtttttgtttgagctgttcgtaagcttggtacagctgaccaacgccgtcaggttccatctgttccacatagatttgataacttccactgggttcatagaccgaaatatggcccacaactaaaactttcatgccttcttcagggatgaattttagccggttgaaagccgatttaaacatgatcgcactaattttcgcgtgatcatccttcaagctaaagtattggtgggcattcgggcgcaatcgaaagttggagatttccccagtgaggtataccttagttaaatacggatcaacatcaaattttcttttaatatattttgttaaggcgctaacggttaaataatcattcgccacgttcaaggctccattctgctaaatcaacagtttgctgcatcaaagttgcaattgtcattggaccaacaccaccgggaacgggtgtgatgtaagaaactttgtcaaataaatcatcatagtcggtgtctcccactaggtgcccttcttcattaatattttgaccaacatcaataatgacggctcccggtttaacatcgtttttagtaacggtatgaagactcccggttgctgaaacaatcacatcagcgttcttagtatattcagtaatatcttttgttaaaagatggagaattgaaaccgaagcaccagcatttaacattaaagcagccattggtttaccgacaatggcacttcggccgatcatcaccgcgtttttccccttcaaatcaatgtgatattcatcaaacattgtcatcacacctttgggcgtacatgcaaccggatacttggttgaatcatttaagtataattttccaacgttaattggatgaaaaccatcgacatctttttcaggcaaaatggaacgggtgatttgtttttcattgatttgctttggcagtgggtcctgcactaaaatccccgtaatcttgggatcctgattgtactcctgaacaactttcagcaactcatcttgggtaatggtatctggtaattccctgacaattgaatagattcccaatctaacggccgtccgatgcttatttctgacatatcgctggctggcaggatctgtgccgacaatgatcacaactaacccgggagtgattccgtgttggtcttggagttgttttacccgttcgctcgtctgtgcgtttaacttctttgccaatgcttttccatcaataatcgttgccatctagaaaccgctcctttatattttcatcgtgagaaatcatatgtacaaaaaaatagatttacacatgtgtaaatctattttaccagttcttctaaagcatgtgacaaaatcccgttaacaaattttcgtgaacggtcgtcactaaatttttttgcaagttcgattgcttcattgattgataccttggcaggcatgtcatccacataaaccatctcgtagatagcaatctccaagatgattaaatcggttcgggcaattcgctcaagtgaccaactggaagctaaatacttttcaattgtatgatcgatttcagacttgtgttccaaaacgccagaaataagttgatgcaggtattctgggtagtcgtcgccatatttaccgctcgtcaaaacttggaagaaatccttccaatcagtttgatcgttggtatttagggcaaacagtgtttgaaacgcaatttctctgatctggtgtcgtgttaattccactattcctcaccattttcttcattgtcagcgaacggattatccggatcaatcgtactggtggttttttccggaatcacgccttgaacatgcacgttaacttcggtgactttcaagccggtcataaacaacagctgctgttcgacttgactttgaatttccaatgcaacttttggaactgaaacgccatagttcaagtatacatagacgtcgatcgttaattcctcatctgtgtatgtcaaattaacgcccttaccgtgttcttttcttcttccaagtaattcattgacactcgttgaaaatgagccacgcatccggttaacgccgtcaatttgcgatgcggctaccccagcaataatttccaggacattgggtgcaatctcaattttgccaagttcgggatcatttgaatgaagaatgatattcgtgtcttcagccattataaagcctccgtttcagatcaatcggctactatgcccgtgaaatgtaagttccatcggtggtattgatagtcaacttgtcaccctggttaacaaagaatggaacttgcaatgttaatccagtcgtcatagttgcgggttttgaaccacccgaagcagtatcacctttgataccaggttcagtggaagctacttcaagaacaacggtattaggtaattcaattcctaaggtttcgttgccgtattgaataacttgaacttccatgttttcttgtaaataattcagttcgcttttaatttgttcagcaggaattgaaatttgatcgtaagtatccatatccatgaagacatgttgatcaccatcagcatacagatattgcattttgcgcgtatcgatttgagcctgttccatcttagcgcctgaacggaaagttttttcttgaacagcaccggtccgcaagttcttcagctttgaacgaacaaatgcgccacccttaccaggcttaacgtgttggaagcttaaaatccgccaaattgcgttatcgacctcgatggttaaaccatttttaaaatcagcagttgaaattgccattgttgttcctcctaaatgtaatgtaacataaatagattatataatactttcggtcaaaatagccaatgaaaatggcattctaatcctgagcaattaaaaagccgggatgcaaaacacgcgttttgtcccagcctctttaattaaactattgtgcttactttgcagcttcagcaactggataaactgaaacctgacgcttgtcgcgtccttttctttcgaaacgaataactccatcaacgactgcaaacaatgtatcatcgttaccacgcttaacattgttccctgggtaaatatgagttccacgttgacgatagatgattgatccactgtgaactgatgagccatcagcagcctttgtacccaaacgacgaccagctgagttacgaccgttggcagttgatccaccacctttatggtgagagaagaattgtaaattcattgctaacataggtttacacctccagattaattgatttatttcgctgtgtttaacttaatatacttactataactttcggctatatcagccattccgttcgcaaaagtattcaaaactgcatcagcttgaatgcgcttttttgaatcgctaacaactggtacattgactgataaatagccaccattgtcatcgtcactgtcgacatcgacatccagtccaacaacctcttgaagaccgttaaccgttgtgatgcttaacacagaaacagcagaacagacaatgtcttgcccatattcacccgcatcggcatggccggtgatggtgaacccacttacatgaccgcgataacgcttaatggtcgccttaatcatatcagtcacctcaaagtaaattatgccttgattgaatcaataacaaccttggtatatggttgacgatggcccttctttgaacgtgagcccttctttggtttgtaacggaagatgataatcttcttttgacgaccctgtttttcaacagttccagttactgatgcgccatcaactaatggtgtaccaactttaactgaatcgccaccaaccataacaacttgatcaaaagtaaccttttcgccttcttctgcgtctaatttttcaacgtagattgcgtcgccttcggaaaccttgtattgcttaccgcctgtagtaataactgcgtacatatcttgtgcacctccttataagtttgcttagactcgccgagaacaagcgctccgatcactatcgaagacttatcagcttgaatcgagcggttgtagctgtggaagccacaattacaacgttactagtatacataattggcaggtgttcgtcaatagaaacctgatcccataaaaaaacaaccgctacccacggctgttttatttacgttgagctaaatgtctgccattggctcgcgtggtggttgaagaattggtaaaatactgaataatgccactaacgatgaaaatgaagacaataaagattacaaatcccacaacgtccacctcctaattgttgtgacagcagattgctgcacaactacattatccagttttgtcaacgaacgttcaaatttttgaattcaaccaactcaaattttaataaaaatgcaactttcttaaggaattcataatcatattgacatctttgccctaaaagactgattaaacattgactaccctgttaatatttcatataattgttattgttgatttgtcgcaatagctcagctggatagagcaacggtcttctaaaccgtaggtcgagagttcgaatctctcttgcgacattctgacgtcacatcaggcatttcgagatgtttgctaaataccttcaattcctattttaacgggattgaaggtattttttatttacaccactatttacgccgcactctaggaaatgtcaaaatatcagtccgcttacttagtgttatcaaaacggccgaaccgaagctgaatctcttcgtttcgaccgtttcttattatcttcaattaataatcctgatcctgccgatcttcattaatcttgtttttatctttgaaggcctgttcaatctcctgctcagtataaccgaaatcaaccaagccaaatttaagaaacagtcgccaggaatggctaaagctgtcaccgctgtgatcaaagtaagcgtcaaacaacatgcgttttaaggctaaatattgcttatctaggttatcttcttttttgaactgtttgattttgtccagatcatcctgcgagtttaaaatcacgtgattccaatttttgaggttggaaatcaataggtagaaatccattgcgtcaacgtactcatatagcaacgtttcccgcggcgttttgttgggatcgtgcttaccacgatgcgtcttccagaccttgaaccactcggaagtgttggccatttcagccagttccacatccagggccacaaaggcatttttcactctgccgtcatttgaccagtggagttgcttctttgattcgatctggcgattcaaatacaccgatgaagcaatcaatgattgtaaatccatttcaaactcctatccaaaaataaacttgttcgataaaatctcgagttgctttttgttatccaaataccagtctttgatgaacgggtaatccaataatagattcagccagctttctttttgatcctgatcgtggatggttgctccccacttgggccgatcttcatcaccggcgttataaacgttcagctgggtatcgttatccaaggtcaaggaggccccaccattttcaccagacatcaaaatatattggttatcagccgacttaacaaatagctcgtccaaaatcggctctggaattgcgccggcagcgaattcatagaactcaccgttaacgccgtccaagacgttaaagtcaatcttaaaaccgaagctttctttgagcacttcagcagcccgcataatcacgttcatcgcatctttaagagccgaaacgtccaagccctccaaatcaacgacaaagtaatcgatcaaggccgacccatgaaacatcatttccttactcttcagattcaagtagaatagcggtcggttatgggccgtggggccaaagaagaatccggcagcattcttggtcgatttagtaaaagtaaaggtattatcaccaagtgatgaaaatttagccagcagcttttgaacgtgttcagagttgctaattgaaagtccatcggcgtggtcagacaacttcaataaccgttcaaagaataccagctgaacatcttcatcagaaaattggtgtggaaattccacaaaatctgaattgagttgataattggtcaacgaaacagctgcagtcaacaattcatcgaggtcctgggtctgatttaggctggtaaatgcattgacatacttggacccattgtccaatccggcttgaattgactgagtatagtgattcaaaagctcagtcgtcgttaaaacattcttttctgtttcagtattttcattactcaccgtcagtcacctgcgattctttgctcaagctttgcaagtatttggcgtataagttgttattgttctcaataaatgcttcaaaactgccaaatgaagctcgaatattttgtttttccaaattgtaaatggtctcttctttggacagcgccaaaatttggttttcattctttttgatttcggaccgggcacctgaagcttgttcatcaatattcgtcaactcaagcagatcgttttgtaattgctgatgctcttccttaaccttgccggcttcccaaggcattggcgacttctcttcattttccttaatctgcttgcgaatctcttccttacgctgatcacgtttggtttgatcttcaatcaattgagtcagtttttcgttcttttgacccagttcacgcatctgatcgtcgtttacccgtttgttttgagcttcaagttcaaatgatttggccaaggtattatattcgtcttcagcaaaattgaatcgaacgttaattgtatccaactccccaaacatccgatggtcccaccagttaccaaagtaaatgttgaatttccccaagtcatattcgtggtaatagaaaaatggataggtggttcctaaataatcaatgagtttgtcactcaaatgatgacttaactgagccttcagatcagcggccaggccaaagaaattagtctccggctgatcgggctgttcacccttgacttctgttgcaaagcggttgggatccatcaattcgtatacttttaaatcattgccatttttgatcgagtcattcaaatccgacagatattttaccttttcgcttaacgcggaagctaaaatcgagtcgttttggctgaatggatcgttttcaattttgttatccataatattgcctcgtattccccttatttatacatttaatgttatctgaaaaacgtacataaataaagggctaatcgcattatttatgaaagatttgtcaaaatgatgagaaaacaatccattcttttgaaaattaggtgaaatgacaaaaacgaccagaccatcataatgggttaatgatgacctggccgcctctgtattcgattgttttcagttgaaagtttgactctctttttccatttgcctatatggagttgtcaaacagtcccccgtcgctgcatgataacttatttgacaatgtaggcatttttataattgtacgttgccccggctgtattgtaaataatgcctttgaccttactgctcaacaggtttttacttgctgattgatatagcggtgtaatgccctggttgtccagtaagatattttgtgccttggtcatgtcctcaaatcgcttgtcagcgttcccagcatcggtggttgaagatgccttaatcaacttgtcatactgcttgttcgaccactgtgggacgttgcttgggttgccagacgttaggatgtttaagaaggtaatcggatcggcaaaatctgcgtaccaatcacccatcgtgacttggtaattatgtgatttctgtcgtgacagcaacgtttggaaaggaatatttcttaggttcaccttgagcccaggcagattcttttctagttgcgactgtagatactcactgacttgtttttgcgcgaattcgtccgaactgagcagtgtaaaactcattttggtgatccccagttctttgaggccggctttccaaagcgccttggccttggttggattataggttaaagaatccggtttggcagtggtggctgtaaaatctttgccggtcttaggattaattgacagtcctttggaaacaaaactttgtgaattaaaggaaccgtctcccaaaatcttcttggttaactggccgcgatcgatggccatcgaaattgcttctctaatttttaaatttttgaacagtttcttcttttggttgaatgccaggtagtaacaactcgaagtttctctggtcaccaaattcttattgttcttcagatttttggccaaaacaccagataagccaacgtattgcagcttgtcggtcttaaattggttatagccggtcgaagggtccttagtcacttgatagtggagtttgtccagtttgacagctttcttgtcccaataattttgattcttggcaagcgtccaagtcatcccggttccgttccagctggttagcttgaacggtccattgtagaccatatccgcactcttcgtcccgtaattgtcgccaaacttctcaacgaccttttggttctgcgggaagaacaatgggaagcccattaacagtttgaagtatggaattttcttttccaaggttacgactagtttataattgccgtcagctttgattcccagtgaattgggtgactttttgttagcttggatggcatccgcattttgaatccctgaaaaaagataaccgtactgggaggccgtttttggattgacagttcttcgccaggaatacacgaaatctttggcagtaaccggatccccattgctccatttggtgcctttacgcaaattgaaagtatattttaacccgtcatttgaaatgttagttttggtggccagtgcattttcaattttgctgtccttacccagacgataaaggccttcatcaatgttgtttaacacttcaaatgtttgaaccgacgtcgttttggaaaggtcaacagttgagagttctgaatcgactgcagtggtaaattcctgtttggccgccagtttccccgaaccgctcttttgcgatgaacagccggtgagaattaaggctgcggagatcactaaccccacttttaagccaacttgaatatttgacataacagacaccccttcatgaatctatatgagactgaaatacattcaattataaacacattatattttaatgagagataatcggtataaaaagggctcacagcagtacaccatcgtgcaccaccatgagctctttcaataatcgatcacgctcttatcaagtgcggcaaagttattttaatacactaatacttttcaagatactggtcacgttcccaaccggaaacttgtgtgcggtatgaatcatattcaaggttcttagcttcaataaagctactgtagagatgttcgccgagggcctttttcatcgtttcatcagctgaaagatccttcaatgcattatgcaaggtatcaggcaggttagtgatgtggctcttctgacgttcttcagcatccattcgataaatgtttcggtcaatgctgtgttctggttcgatcttgttgcgtaagccatccaagccggcttccaagacacaagcgattgccaagtatgggttagcagttggatcaactgagcgaagttccaaacgagtggaattaccacgagcacttggaattcgaatgagcggcgaacggtttgaaccggaccatgcaacgtagacaggggcttcgtaaccaggaaccaaacgtttgtaagagttaacgattgggttacatacagcagtaaaggaacgggcatgcttcaagagaccgcctaagaagtaataggcttcttgagaaatttccaactcgccatccttgtcgtagaaagtattgcctttatcgttgaataatgacatattcaaatgcatccctgaaccattaataccactcaaaggttttggcatgaaggttgcgtacaagccgtacttgcgggcaacggtcttaacaaccaacttgaatgtttgaatattgtcagcagcagccaaggcatcagcgtacttgaaatcaatttcgtgttgaccaggagcaacttcatgatgggcagcttcaacatcaaagcccatttcttcaagggtcaagacaatttcacgacggcaattttcacccaaatccattggggccatatcgaagtaacttcccttatcgttcagatgaagggttggttcaccattttcatccatcttgaacaagaagaattccggttcaggtccaatgttaaatgaagtaaagccggctttcttcatgtcgccaagaacacgaatcaggttattgcggggatcggctgcgtatggctcgccgtttggacggtagacctggcagattactcgagcgattttcccacgatcagtactccatgggaaaatcatccaagttgataaatcaggatacaaatacatatcactttcttcaattcggacaaagccttcgattgaagaaccatcaaacatcaatttgttatcgaggagtttctccaactgagtgattggaacttcaacgttcttaattgtcccaaataaatctgtgaacatcagacgtaaaaatttgatgtcctcgtcttttaccatcttgcgaatatcatcttttgaataatcatgctttgtggccatctatccatcgctcctatcaatgatttagtttgtttaaattgttcaaattattcggatcatcaaatgacgaagaaggcggcttcaatccaccaatgttaagaaactcgtcttgaagaatttttctcacatcactgtcagtcaaacccttctcgagattacgcttccgctcgtcttccaattgattctgcttcttgtacacctctttgataccagagatattcagaccgtcatcaagataatctttgatttccaaaagccgatcgacatcattcaatgaatacatccgtcgattgccttcattacgaagcggcttaatcaattcctgctgttcataatatctgatttgtcgtgctgtcaagtcagttagcttcatcacagttccgatcggcagaactgacattgaacgccgtaattccttctctcgcattgttcacctcctaaatcttgtacccataataccattcccataatcaaagtcaagactaaatgtcacattttataacatgaatttattgattgttgtcatccagccatttttcaacgtcactttcaatctccgttaactgatttggtcgctgaaccaggttataccaatttggttgcgggtcagttttgttcctaaaccaagttaattggcgcttggcgtaatggcgtgaatccttcttgatcagctcaattgcttcttccaaggtcgattggccctgaaaatacgggaataattcacgatagccgatccctttgccggcttgaaattgctgtccgtcatggtcatacaaccagcgaccctcggacagcagtccctgcgccatcatttgatcgacccgctgattgattcgctggtataacaacgcccgatccgtcgttaatccaatgacgaaggcatcgtattttgatccggcattatgctgatcagaaaatcggtgaccggtgtttatgtagacttccaaagcccggacaacccgcctgacgttgtgaaccggaatggcccttgctgcggcaggatccactttggcgagtcgttggtgtagcgccaaatcccctttttctttggcttcagccagcaattgtcttctcaagtcatcattttgatactggtcgccaccaagttccagcccagataaaagtgcctgaaggtaaaaaccggttccaccgacgattattggcagcttgccgacttcgtgaatggcttcaatcagtttcgaagcatcctgaacgaaatcggcaacagaaaaacgttcgtcaatatttctaacatcaattaagtggtgtttgacccctgccatttcttccggagtaattttagctgtcccaatgtccaagtgtcgatatacctgcattgaatctccggaaataatctcggcgttaaatttttgagcgagtttgatcgacaaatccgttttcccaacggcagtcggtccgacgattgctaaaagtttgatcattccagtccctcccgcatctctgacctgatctgaacagctctggcaggatagtcggtgatgatagcagctaggttgcgttcaaaacagtactgcatatcctctgtggaattgacggtccaaggacgcagattttgagcaggggcaaaaaagggatgtcgtttaagccaacgaatgtccggatggaaatcggcaattaaatggtccttcttgagggttttggcctgcttagcggcagttttgaacaatttggcaccggctaatttagggtccagccggttgagaatttcaagggaccgggcattaaagctggagtaaatcagctgaaatgggtagtcgattgacgcaaaatagtcaaaaaccgctttttcaatccctggatactgaatcttgttggtcttcaactctaagttaaaaattcccgtgaagttgtctttaattaataattccaccacctcttggagcgtggggaccgtggttcccttaaattcactgctgaatcgaacaccagcatccaaatgtttaatctcagccagatttttgtcaacaattctgccagaaccgttggtggttcgatcaactgtttcatcatgcataataattaactgatggtcttttgaaaaatgaacgtcggtttccaggccgtctgccccatcgtcaatggcggtttgaaaagaaatcagtgtattttccggtcgggttcctttactgccgcgatgagcaataattttggtattgattttcacaataaactcctttttgaacgattaattaatcaattaactagatatctatgaaaaaataaagcataatgaaagtataaacgagtattggagggtttagatatgaaacagtttactaatgggctcattgttggtgttctcggaaccgttgctgctggggttggtgctttactaacattcaaaaagtcagttgtggatccaatcgaagatgaagagcaaaaattcgaggataaccgaaaaaaggcaatgcgtaaaagccgagctgcccaccacggataaaacattatccaatccattacactaatatcgattataaaaataggactatgaacaaaacgactgctttgttcatagtcatattttatcaataattactctttttttccttaccattccaaccttgataaccactttttaagatataaagatctttataaccctttttgcttaaaaagagtgcggctcgtttgctgatcgttttgccttgatcatacatataaaccggcaagtctggacgaagctgactgtaaaagtttttgatggttgagtaaggcatgttgcgagcacctaaaacatgaccatctttaaaacttttttgttctcgcaagtcaatgacctgagcttttctcatgcctttttgaaactcatcatttttcaaatacgttgcaacctgtttaacacgcatattttgaaaaatggtatagccaccccatgcaagtaaaataacgatcaaaatgatggttgtcaccagattggcggtgattgcaccgattatcaacaaaaacatccctctttctctcaaataatttgattatttagttccaaatggttgattatttctaaattgcaaggctaatgatgcggcaccaataattccggcatcattcccgagttgagccaacttcaaccgtgttgagtcacgaacagaaggaaaggcgttctcttggaaataacgagtcgttggttgaagcaaggtgttaccggcgttggaaacaccgcctccaataatgatgttttccgggttcaacgtgttaccaatgtgtgaaagtgccaatcccaagtatgagcagacccgatcaacaatttggttcgccaagatatcaccgttatcagctaggaagaagaccatcttcgatgacaaatcttcgtcgccatcaatcaattctttaatccgtgaatggccggtaaacttcttggccatatctttagcaatatggacaaccccggttgctgaagcgtattgttccaaacagccacgctttccacaggtacattgatatccattagggacaaccgtgatatgaccgacttccccggcaccaccgttaataccatgaaccagcttgccattggcgataacaccaccaccaacgccagttcctaaagtaatgaagacaacatcttttgccttgtcgccggcacctttccaatattcaccgagagcggcgctattcgcatcgttgtcgatcagaattggtaaattgagattggctgaaatggttgctccaaccggttgcacgatatcccagttcaagttatatgctccaacaactgttcccttttcgcggttcacagcaccgggagttcccatgccgataccataaaaatcacttgcgttatagtcgtcttttctcatttgatcactaattgatttgatcatgtcaggcacaatgtgactgccgtgttcactaatgttggttgggattcgccacttcgtcaggacgtttccttttgtatcaatgaatgcaaatttaactgtcgttccacccaaatcaattccgattaatttcttagccaatgtattttcccctactttcttgtttttcttcaattcgatgttcccgcgttaaaatcagtttggcatgaataaactcatcatgactgatcagcttggcatcatggagatggtccaactccaacgccatgacttcaatgtcccaaagtcgtttgccgacatatacataaatatcgaattttttcagcagctgctgaacatcatacagcgttttcattatctcacatcctcatgtaaatttctttcattttcaaaaaatttaaaattttgcccgcatacctattgtaaacaaaacgaaagcgattacaaccagcataattgccgaaataattcgtttggtttggctggtcttggaaaaaccgacgcccgtcacgtacgccacaaggaatccaccaaccagtccccccagatgcccagcaatatcaatgccggaaacaaaaatatcggttccgatatttaggataataaacaacaggaatgttttggccatcgaaacaattgccgggtttttggaaaaactttcccccagcatcataaaagcaccaaacagtccaaagatcgcagtactggcaccggcagacaagctgtcggtaaaagcaaaactgcccaggttgcccatgatgccggaaacaaagaagataaccgcaaaccgccagtgtccaaacaattgctcaacatactggccgataaagtataaggtgatgccgttcattaagatatgggtgaagccaatgtgaataaacattggcgtgatcaatcgccaatactcgccggcacggatgagtgggttgtatttagcgccgaattcgaccaaggtgacggggttttcagttccgcccattactgacatgatcgcaaaaaccactaccatgatgattaatagtccatatgtgatataaggctgatttcgtaaattactcatgaacccctcctgttatccgtttagtaaatgagtttgtcgactttaacgtcaaaatcttccacgttccagacgggttcgtcaaatagttgaaccggcgtcaccaaagcgatacttgtgccggtaaagcccttcaaaaagcgatcgtaaaagccgccgccaaacccaactcgaaagtgatttttagaaaatgccaatcccggtaccagtaaaacatccagctggctttttgccagcacttgaccgccaacgggctcaatcgtgccaaatttggtctcactgagtaccgtatcaggttccagcagcacaaaggtcatctggcggtgcggaagtgttcggggaactgctacttgtttatcatgggttaacgcccagtgaataattggctgggtatcaagctcatcatccatactgagggtgatccccagcgtctcactattcgcaaagtgtggctcagcgaataactgctgatacaagcgttgaatttccggtttttcttgtggatcttgtaaaaagtcatgaagccgagcgatctgctgatctcgcagggcggcttttaattggttacttttggccatttacctcacctgattcttcagtcaaatctaattgacagactctgttgtatataaaaaaggtttgggtatttacccaagccttatttggtttctcgatgtaatgtaactttacgctcgcgtgggcaatactttttaagctccaaacggtcgggattgtttcgacggttcttgctggacaagtaagtacgttcgtggcattcagtacattccattgtaatgtgtactcgcatggaatacgacctccaaacttttatagagtagctagtctaatagcctcaacttaaaatattttatcatcaatcctgataaattactaggacaaaatcgataaatgttaagtgtttttacttaacagtcgaagttgattggaccgtcttccagtaagcagagtagatttgtttggccagcgccatgttattactttcagcgttaacccccaggttaggcattgccaaagcaaccaccacctgtggatgagtcgatggcgcatatgaagctaaactcagggtaactgtttcgttaccattataaaatgtctgagcagttccagttttggcagaaatttccggtttgatggaatccaacatcccaccggtcttgtaggtgttggttccatgaaccacccgatacaagccggttgtgaccacgtttcgttgcgcttgagtcatatcaatatgattgagcacctttggcatcactgtcgctttaaccgttcctaatttaccatcttggctggtgccgcgaattgcttgaacgacatgcggttcaattcgattaccaccgttggcaatggtagacatgtactgagcaacctgcatcgttgtgtaggcgtcgtagttaccaaatgaaagatccaaggcacttccaatgtgcttatagccgctggcaccctgtaacccggtagattcaccagggatatcaatcccagtcttgacccccaagccaaattggttgaagtaaccgcgcatcgtgttgaagacgttgggactcatggttaatgcgccaccttcaacatagttgaagtggccttctttcatcgctaactgcatcatataagagttggaagaaacttgcagcgcatcactggcatcaacagcaatatttgcatgaccgttgtggttgaaccaagacgactttttaacaccaccggtcgtaattggctgatcggttaaggtactgttggttggtgtaatgacatgatccatcaatgcaccggaaaccatcgcacccttgacaacagaacccataacaattgagctgttaatggttcctaaaatattatcagtgatcttggatgtcttcggattgcggtcaacccccgccattccgatgatggcaccgttattcggattcatgacgaccgcataagttccggttgaattaccaccggcaccggactcggcagaacggactaaggattggagctgcttttggaatttggcattgattgtcaattgaaggttgtcacctttttgaccgccatatttcttaatttcctttttgatctgattatcgctattcaaaatgatttgggtctgggatttggttccccgaagaaccggttcatactggcgctccagataactttgaccgacactgtcgtttcgtgagtagccttgtgccaataattcattgacccgatcacttggcagaccgctcttttcattcgagacagttccggtgattccctgaattgaacggccatttggataattacgactccaactggttccaacattaaccccaggcatatcggccagatgttcccccaccatggcaacttctttggtggagacgttgtcatccttaatattaacggtggataattggtaggcaccactcatcttggcgaatatggttgcagcatttttgagtgctgatgaaaaagtggcatttggataactttcaaccttattgacagccttgtcgtatttggcatcctcagaataaccggaaatcccagggattgacttttcgactttggctagattatctgtgtttgccaaatagtaatcagccagctggcgcttggttaaactgccggtaggaacggtcacatattgggctaatcggttggcggtcttgtacatgtccgaggacaacacattcacgcccttggtatagataattgcttggtgcgcggaattgccgactaaaacgtgtccggttgaatcaaaaatcattccccgctgaacattcccgttgaccactgaggtatccgaacggttcacttcggctttaaatttagaaccgtacatcacctgtaaataggccaactgggtcagtaatgcgacaaataaaattccgacaataataaaaataatattaattcgaaaaggcagtgaaacagcctttgctttgttcgttttcttggtgcgctttttaaaaattttcacgatattaactccttgccatgaaacttattctatcaaattttccaactaaaaactacaaccggtagtcaatctttaacttattatgatattctatatgttgttaatcacttttaaaaaggatgtagattatgaattcaaagaagacaacgaaaatttccatattagtgctgtgctttttggtaccggtgctaatttccaccagttactttattttccgccactttgctccgtttggcggctcgtcagtcatgaccgttgacctgggccaacagtatattgacttttataccaatttccacgacaccctcctacatagtccaagcggctttttcttttcattttcaaaggctcttggaggcgacatgatgggaacttgggcttactacttaatgagcccgctgaacttgattatgttgcttttcccactttctaaattacccagtgtcttgggcatcatcacgattatcaagtatggtctggctggtttaagttttggctatttcttgatgaaagttaccaaacacgttggctggtcaatcattggtttctctgcttcgtatgcgatgatgggctggatggttgccaaccaattcaacatgctttggacagatgtgttgttcgttttgccaatgattttctatgggctcttcaagatcttgaaaaatcagtcgagtgccatctacatcatcagtttaacggccatgttgattatgaattactacatgagttacatgatcgccatctttttaaccctcttcatgttcatttactgggctgccaaggcattgccggtggaaaaccaaacatcgaccaaagccgttctcaaatggcttaaggcgtcaattctgagcggtattttagctgcctggctgctgctgccgacctttttctcgcttctgggaagcaaaacccaatattcaaagggccaatacaaaatcaagtttgaatataacccactggacatgttgggcaagttctttaatggatcagttaatttcaatgaactgcctgccggaacagccaacgtctttgtcgccagtgtcgttttgatcctatttgtttactacttctttattccaaccatcaaacgaaacgtcaaaattgccaatctttcgttgacagcatttatgattctatcaatgtgtttccaaccactggatctgttctggcacggtatgcagctgccggtttggtacactttccgtttctcctacctcttctcgttttggatgattctgaccgcctttcaagcctttctgcatatcttggatgaaggcatcaactggaaaggttatctggtcattgccggtatcatggctttgggcgttctttacgtcgaactccgctggaagcatctcgaatacatgcgccacttcgactttctctggggctgtgtttatttggtcgtttcccttgggatcgttgtcttcttaggcatttatcgcagaaacattgttctggcgatgaccttggccgtgctgatgagtggtgaaatggcccttaacatggtcacctcactgaatcatcttgattatttgaaggccagcaattacacccagtttgagcgggtgatgcgcaaacatgtcaataagattaagcaaaaagataagggattctatcgattgggaaccactttctcgcggaccaagaatgacgctttcactggtaattacaatggcggctcaatcttctcgtcaaccctagaatccgatacgtctcaattcttcaaaaatatcggtcagccaaatggggattcatttgtcctttactcaaacggaaccatgtttactgattcattgttgaacatgaagtattacatgagccaccagattccggaagctaatccgaacaagaaaccaaagaagcagctgttgactactttgacaagaaaaccagattacaacaattacaccttgttgtcacaggacgccttgattggtacctaccggaatccgtatgcggtcccgattggtttcctggcgcctaaatccggaatggaacataattcaatcgccaagagcccgatcacttaccaaaaccaaattgcccatcgtctggatccaaacatcaagaacttgtttgaaccagcaacctacactgacatgcggtataacaacattcaaccgatttctcaattagataatgctgtcttgaagaaaaagaacctcttggaaatgtcctacatcattttctctgtcccaattgagaagaacacgtcttactacatgacgttgggaaccgaaatcaataaaggcaacatttcaatttcggttgatggtcaagcgcagactcaatttacaccatctgaaaaaaccatcattgctaacattgccacaggtaccagcatcaataccactgcaaatgttcaaatctttgtcaacaagaataacgccctcttacaagacgtgaaattgtacaaagtgcataattcaaagattgctcagttctctaaggacttaaacgccaagccgtataaagttacgaagtggaaccaccatcagttaaccggaacggtggacgtcaagtccaacaatcaagcattgaccacgaccattccatttgagaatggctggactgctaaggttgatggtaaatcagttaaaccaaaacgctgggcaaagatgttcctgtatatcccaatcaacaagggtcaccataaggttgtctttacttactggcctgaagggctgagagtcggcctactaatcactgcttttggcttagcatttatcggcaccgaggcaacgttaaaacatcgtaagaaacaaaaagccaagcacactgagacaccaacaaataccaaataaattgcatgattaaagggatgaaaaccattttggcttccatccctttttggttggttacgtttatttatcaagatccccattaggtgtgtacgtgtacacaacattttcaggatctttttctggattaaaatcgactttcaaatcaaagccgacaaagaaccagcgatcatcctcgtcaacgaaataagtaattccgtccttttcagttttggtataagtctcacctggatgatcatcgcgggttaacgctaacgagaagccttcatggacgggagtcttcccataaacctttccatagaagcgcacaccattgccttggcttaaccccatttcagattggaaccatttgcttgcggaatcagttacatcaattttcattattatgccacactcctaaaatctgtgtttgtattcgcttacaatcgattataacatcattaaggtatttcacaaacgatatgcaagccgattagacactgacattgttcatcaaggggctcttcacctttcaaaacgtgacgattgcgggcttaatttaacttatcaaaaaagaacggttctacaatatctgttgttggtaatagatttttgtctattactgatgacagttttttgtttatcattagagtaaaaaagcggacatctcccgtccgttaacttgctcccaccacagaattaagtcaagaaaggaaatgccctatgtcaaatgatactacgaaaatgttgttaggaatagatgatgaacacttaataattgagaatggcaaaataggtgatgatggggtgatccgattaaatggatcgctgaactattcccccaaggcctgccacaactgtggggttattaatgaccatcagatcattggctatggttggcggaagaccaccattagattcgctaaaaccttgggcagcaccgttatcctctgcctcaatcggcgaaactttcactgtaaggcttgtcataccaacttcctggcgcagacgaatgcggtgccgaaacactgcacgatttcaaatacgacccgcaaacaatgcttagaaaaactgaccgaaccggtttcgctcaaacacattgccgatgagttatccacttcggattcattcgttggtcggcagctcttgcgcgctgaacgggactttgaaaccaactggcactatttacccaaagttctcctcatggacgaagttaaaagcactaagagcgccaccgacgcgatgagctttgaatttatggacgcggaaacccacgaattgatcgacctgttaccctttaggaccatctatcagcttcaaaagtatttccagcattacgaccaggctgcgcgagaaaatgtgaaaattattgtcaccgatatgaactatacctatcccaaattggtggggcagatctttccgaacgccatcgttgtcatcgatccgttccacttggttaacgctttaaatcgagcttttaataagacgcgggtgcgcctcatgaaaaccctggcgacctcatcacgcgagtatcacgccttgaaacgctattggaagctattattaacgccggaaaatcacctcaactacgaagctttccgtaagtggacaaacttcccttatccagcgactgccactgatgtggttgatgctttattggacattgatcccgagctcaagcaaacttacaacgtgatgaatcggttacgtgaaaccatcaaaaaccgtgattggcccaactataatcaagtattccatcacttagagggctgctcggaagagatgttggcaaccctccagaccctagcgactcatcatgatgaaattggcaatacctttactcaccattacaccaacgggcccttagaaggttcaaacaacaagattaaagtcattaaacgcactggatttggttaccgaaacttcttcagattccggctaagagtgctgttcgcttttcgagttcatacaaaaagagctctaatcaccaagtgattagaactccaatattttgttcaccaacaacagttgacgaagaaccaaaagaactaaccgttgagcaaagatgctcacagttagctcttttcacatactaggttatttgtaatatgcaagttgctctattcaaccttagtgattttaactttcatggttccggccggaatgggaatattaacttcttcattgagacggtgaccaatgagccccttggcaattggtgaatcattggaaattttacctgacattggatcagcttcggccgccccgacaatttgatacgtttcgggatcttcatcaggcagttcttggaaggtcactttcttaccaaccgtcacctcatccttatcactatcatttgaatcaatgatttgggcatattgaagcatgtgctcaatcgttgtaattcgactttcaagcatactttgttcatctttagcagactcatactctgagttctcagataagtccccataacttcttgcaattttgatacgttcaaccacttttggtcgttggtttactttcaagtcttctaattctgccttgagtttatcgcgaccatcggcagtcattggatatgtgtcttcagccatttggtaatttcccctttttatctttatattgttgaatcaaggttattcttaatttctttgttgccacgccgcatcaaaatggaacgcattttggttgtcagcaaatcaatcgcgacttggttctccccaccttcggggacgatcaaatctgcgtaacgtttggttggctcgacaaactggtgatacattggcttaaccgtcatcaaatactgatgaataatgttatccagtgaacgaccacgttctttggtatcccgttcaattcgccgaattaaccgaatgtcattgtctgtgtcaacaaatactttaatatccattaaatcacgtaatcgcttatcgtcaaggattaaaattccttccaagatgataacttcgcgcggttcttggtgaatggtctgctgactgcgggtaaattgaccatagtcatagaccggtttttcaatcggttcatattgcagcagttgcttgagctgctcaatcaacagatcaaaatcaaatgccatcgggtgatcataattcacctttttgcgatcgtccatcttcatgtcagcttggtcattataatatgaatcctgttgaatgatcgtgatcgaataattggataattggtcaaaaatcttgcgtgcaaccgtggtcttgccactaccggatcctccggtaataccaataactactggccgtgttttgtgatttaccatgtaaatagatgccctctcaattagttgttatcggaagtatgcgctgcaatttgctgctgatgttcagcatacgtctttgagtaatatacttttttcgtcttggtattggcaacgaagtacagatagttctttgaacgatccaaaggatgcaggacagcactcattgaactaatgcttgggctgtcaaatggtcccggaccaaatccggtatacttataaagattgtatggcgaatcactctgcagatccttgttcgtcaaaactttgttatttcggtgaatggcatacaaaaccgcgacgtctgattgtaatggcatgttgatatcgatccgattcaacaataccccagccatcttccgtcgatcggtctggttgacaccttcccgttcaatcaatgacgacaaggtcatgaactgctgcatgttcatcccggattttttaatggcggcaaagtgcggcgaaaccatctgattggtcttggcaaccatttggttaaccagtgacttcagcgacgtattcttttccacctcataagttgcaggatacaaatagccttcaagacggtagcgaacgtttttggctttcatcgccggattaagcagcttcggataacgactggccagttgttcaaggtatgtctggttcttcattaatttcaagaaatctccacgatcgaaatcagttgtcactgaaatctgggtcgcaatttggtcaatgttggcgccttctcgaatcaaaactttccccttggtgctttggatcggttgatcagtcccgccgcgttgaagccgtttggcaattgttttgaggctcatcgagggttttagttgataatacccagctctaaagttggccatgttgttggatttgacatagtaatcaaagaccatgccacttttaacaatttttttattttgcaggatcgaaccaatttgcttgttcgaagcgccaagcggaatgtgaacctgagtgacgttagtgttctgtgggttcagtggctttaaggcatcttgaaaataccggtagcccatcagcccgattgttgcagctaaaataaccagtaaggtaatgacagaaataataattcttcgcccgaggcttttattgggtttggggtttcgtcgacttgagtcatcgctcatgagaagctcctcctatctgttcaatttaattatagtttccaaattatctaatttctgcatttaaatcagctgttaaccgttttttaatcttttcaaaggcggtgttgaccacttcgtccttcagggtttcgcggggatccacataagtcagggagtaagccattgatttcttgccgtcgggaacattgtcaccttcatagacatcgaataaacgcacatcgttcaagaaggcaccaccacgtttattcataaccgccaaaatttgactgttggtaacatcctgatccacaactaatgaaatatcccgtttgattgatggatatttggagatagcttggtattggttgtcatcttttggcaaatcaatcaactcctgcatattgagttcaaatccataagtttccttgattttgaactgcttggcaattcgtggatggatttggcccaagaaaccgacgtaatggccgtggatcgaaatgttggctgtccttcccggatgcatttcaggatattgatcagtggcagtgtactcaatgtcacctttgacgcccaaattaaccaagaactggttaacaatgccttttaactggaaaaagtcgaccggcttgacatggttattccacagaggatcagtgaaattgcccgtgacaactccggcaatgtgttcaacttcttcaggccgaatttggtccgcactatctttgtaaaagacccgtccagactcgtaaagggccacatcgtcaactttgtgggcatggttataggcaacgtcatcaagtaatcctgacaacatgttcattctcagcaccgcatgatcctgggtcataggccagagcagcttcgtttcttgactatcacgcatcaaaaacatttttgcttttttagcagtagtcaaagaataagagatcgcctgagtcaggcccaagccttccaaggcagttctggaagcgcgctgcagtttttgaatcggcgtcaaaacaccaatactttgccgtccggtcggcagcgttgccgggagattatcataaccgtaaattctggcaacttcttcatacaagtcagcatcgcggaaaatatcccaacgacgagccgggatggtcacatttaaaccgtcatcgtgggcttcgcttgaaaagccaagccgatcaaaaatacttttaatttctgcggtggttaatgaagttccaagaacatgattggttcgttcagcggtaatataaatcgttggcagtttaggatgatattcactggcagtcaccgtgcctttggcgagcttgcctccagcaagctgcttaatcatgctgacagcttcgtcaacagcatcttggacaccgtctggattaattccccgttcgaagcgttgggaggcctcagagtgcaaattatgccgttgggcagtcttacgaatcttgaaggaatcaaaaatcgcagattcaatcaccacgttgctggtattgtcatcgatttgggtgttgaagccccccatgacaccagctagggcaatcggtttgtcgtcatcggcaatcacaatatcgtctgcggaaagctcgtgttcatcctcatcaagcgtggttaatttttcacccttttgagccaggcgaacattgacgttaccgttaattttatctttatcaaatgaatgcaatggctgaccgtacttgagcaaaatatagttggtaacgtcgacgacattgttgatcggtcggatgccggcgttccaaagaacaatctgcagccaagaaggactcggcgcaattttgactccttcaacaacccgcagcttgtaggttttggcaagttgatcgtcagcttttgcctgaatttcttgattggcatccaatgaactgtcttcatcaaccactggttttttaatttctggttgctggttatagattgcagccaggtcgtgaacagtgcccaaaatgcttaacatatcaccacgattgggagtgacatcaaggtcaataatgggatcatccattcccaagtacttgtaaattggttcaccaacaggcacatcgtcatcaaaaacgtaaataccgtcggcccattccttagggatgacgtctttgctgaacccaatttcatccaaggcacagatcatgccggatgattcaattccgcgcatcttggaacgcttgattttaacgttgccaccaattcgtgagttgggcagcgccacgataactttttggtcaacgtccacatttggagccccacacacaatttgtaagggttcgtcttctccgacatccacttggcaaacgtggaggtggtccgattccggatgtttggtcattgataaaatgtggccgacaacaagctttttcaagccgtcttcggcaacggtgacagaatccacctcaaccgctgttcgttcgatcttttcagccagatctttagcgggcatattcagatctaaatattgtttgagccatttatatgaaactttcattctctaattacccctcttactgaattgatttaagaagcgaacgtcatccaaatagaaatcacggatatcgtcaacaccatatttaagcattgcgaaacgatccggaccgactccgaaggcaaaaccaccatacttcttggagtcaacaccggccatgtccaaaacatttggatgaaccattccggcacctaaaacctcaatccaaccagtgtgtttgcagacatcacaacccttacccatgcagttaaagcaagtgacgtcaacctccacagacggttccgtaaatgggaaataacttggacgaagacgaatatcgaatttatcaccaaaaatattttgggccatcgtgatcaaagtacctttcaaatcggccatagtgacgtgttcatcgataaacagcccttcaacttggtggaattgatgagaatgcgttggatcatcagtatcccgacggtaaacgattccaggtgagatcatcttcagcggtccctttgaaaaatcatgtttctccagtgcccgtgcttgcattggtgaagtttgggttcgcattaggatttccttacttatgtagaatgtatcctgcatatcccgggctggatgattcttcggtaagttcatcatttcaaagttgtacttatcttcttcaacttctggaccggaaaggacttcatagcccatccccaaaaacaaatcgacaatttggtcaatgatttgttgaatcacgtgcggctggccttgtgcgaccggccttccaggcattgtcacatcaatcttttcagctgcaagttgtgcattgagggcagcatcttccaatttttcacgatgatcagaaacggcttcggtgatggcatcccgaatcttattggcataactgccgacttccggccgttcttcaggggttaattctttgattccccgcaacgcagcggtaatcgggccctttttgccgagtaaatgcactcgaatttcatttaatgtttttaaatcactggtttgctgaatatcagcaagccctttttctttgatctctgtcaattgatctcgcagtgacatagtatccctccagttcaaattttaaacacaaaaaaactccgcccgataagggacgaagcaacgcggtaccaccctaatttgctgtcaaaagacaacacacttaagacatcgctaacggtgattaaccggaaattttttgttaaataacgcccaatttcagctcgaaaaatgaattcgtgaagatttcctacttcgttctcaccaaccacgaagtctctcagataggttatcaacctactacttttttctcaaacgctttacattagtgaataataagctaaaacaaaaaaatggtcaagctacttttcaacgcttggataccatttttctgaccatgtatgaatttcatgcatgattggagctaattctttgccttgttcagtcaatgaatactcaattaaagatgaatcatcgtgttcggttctgacaacgacaccatcgtcttccagttcgcgcaggcgctctaccagtacacgatcgctgcacttggggatttgtcgggcaatctccctgaatctcaaaacaccttcctgaaggaggacgtcaatgattaagccattccatttttttccaaggaatgaaaatgtcttctcgaacttgggacacaaataataattaatggcatcttgcagaccaactacttgtcgcatataaattcccccctctcatcggacaaccgctatttaacagcagttgttcgcttaacttgcttctttaacgtttcaaactttgatttaagtggactcacgaattcgtgaacagcttcgtagtcatcgactaaggagacgatgacactttcttcgtacttgggccgtgccaaagttaatccccacatgtgcttaagaataatatctttttccattggggataacttggtgatccgttcggcattccgcagggcgacccgtgggtgaataaatgcgtgagaacccaaatcaaacttggtggttctccagtcatagaaaaacagatcatgcagcagaccagcacgcgcaacggcacgataatctaagccccttcttttggcaatcttataactgtcaaaagaaacagcaattgaatgttcaagtcgagttgagtgatggtgctgagtatagttagccaatttcttaaccatgtcagtcgccatcaggtcagaaactatttcacgatactcggaatcgtttttccattcatccttttgcatgtaatacccctttgtctttatttacaaatatgatacatggtatcgccccaaatatcaatgaaaacgaccgttatttaacaaacttgaaaagtaatatgccggtcgctacggcaacatttagcgattccgcctcaccattcattggaatgtaaaggttttgatcggtcttttccaaaatctttgggtcaaccccattaccttcatttcccataatcagtgcaaattgcttggtaggtgttatatcatagtaggaaatggcctgatcatttaattcggtgccataagtcttaacgccagcttctttaaaggctgccatccattccaagatatctccggtaaacagcttcatgtgaaattggctgccctgcattgaccggacaactttcgggttataaagatcagccgatcccttgccaaagacaatgccgtttaagcccgccgcatccgctgttcggaccatggtgccaatattgcccgggtcttgaatgttatccaataacagccaggcaccctttaagtcatcgggaatctgttcatggtagtcctcggtattgagcacagcaaacacaccctggggcgtctctgtggacgagatatgtttggcaatttctggtgtgattaagaaaatttcggtatcatcgtcaaccggcagatcgcccaaatagctttcgtcgacaaccatcagttgtttgatggtctggcgatggcgaatcgcttcatcaacaatgtgccagccttcaataacgtattcgccggacttaacccgtcccttcttggactgcatcttggtccattcttttacccggttattctgattcgatgtaattctttcaatatccataaaatatccctctttcattattaattgtaggtggtgatcatttgaacgacaaaattcaaacagtcaaaatgaacgcttccggccgagtccaaggcgttggctttagatggtcaaccatccagctggcagaaagcctcaatatttccggctgggtcaaaaatgaaatcgacggcagcgtttcaattcttgcaagcggcgaaagtgaaagtctggcgcaatttatccaaaaaatcaaaaattcaccaacccgatttgccaaagtcaaaagtctccaagtcaattatatcgcgaaaagggtaaataaagggtttaatgtgaaatattaaattgaaaagcaggcaataatctagtaagattgttttgtttacgtactaacttaagaaaggtcttactcatgaaaaaatttaaacacctcaccacgctgggattgctttccggcatggcccttcttttgagtggctgtgtccgaacaaccaagtccggtaagccttacggagccgtctatgactatctggcccgccctgctcaggcaattatggaatggattgcccaatttgtcggtagttacggctgggccatcatcgtcctgaccgtggttgttcgcctattcctcttgccaatcatggttcgccagatgaaggcttcaactattcaacaggaaaaaatgcagttgattagaccacaaatggctgaattacagaagcgtcaaaaagcagccagtacccctgaagaacagaccgctgccagccaagcaatgatggcattgtacaaacaaaacggcatttcgatgaccggtgggatcggttgtttaccattattgattcagatgccgatctttactgctttgtacgccgcaatccgttactcgccagagctgtctcacacagttttcatgggcattcgactcggccaatcaagttggctgttagccgttttgtcatttgcttcctatctactacagggctacattgccatgctgggcacccctgcagcgcaaaagaagcaaatgggcgccatgatgctgctcagtccaatcatgatcctggtgttcacgctgagtgccccagccggtctgggaatttacttcttcattggcggcctattcgcatgtttgcagacgttgatcatcaatatgtaccgaccaagaattcgaaagcggatcgccaaagaaaatgaaggcaaaaaagcagtgacggttgaggatctgatgccggatccaacgccgagtaccagtgggacaaaatcgaccggttccgatattcaccaaagaaatcgtcaacgaaataccggcaagcagcaatccgggcatcagcctcaggctcgtccagctgctcagccaaccaaaaagacggtggataagcaagctgaaaaaccagcggctaagcgtcctcgaaacgctggtaaacaacaaagacatcataaataatcacactcaatcacatcttttggtgtgatttttttatttctgcaagattttgagtgatatgacacccaaactcaggataagaatggtaggatattcatgtatatttttcaggaaaagagttgttttcgtttatgaatcaaatttcgctattgatcattctcctggcggcccttgtcatcccattggcaatggcccgttttaaaatcacctttctaccaacagcggttgttgaaattattgttggtatcctgctgggaccgtcactgttcaactggatcaccaactcggaaaccttggagattctccaaaatgtcggggtcatcttcctgttgttcttaagcgggatggagattgatttcagcctctttaaaaagaagcccaccactctttcaccgctcgagaagaaaagccagcatgatcagccgaagtactcagtattacaagtggctacaatcgcttacgcctcaatagtcggcatgtcatttgtgatcgcttatctgcttcaactcagcggcttgttcaccgatatttggctggccgcgattctgttcatgacgatttcactcggcattgtcattgccgggttaaaagaaaaggagctgcttagcaagccgttcggtcaggcaatcctcttaatcgccgccctgggagaagttgtcccgatggttgggttgactttttacgcttcagcctacagtccccattccaaatccttatggctgatcttgttgattctggttgcagctgcgctcttgttctggcggttcaaagcctttttccgcttctttgatcggatcaacaagtcgaccacccagctggatattcggctttcattttttatcatcgtggccctggtaaccgtcgctgaatcggttggcgctgagggaatccttggtgcatttcttgccggaatcgtcatcaaattacttgaaccgcatgaagaaaccaaagttcgtttggactcaattgggtatggcttcttcatcccaattttcttcatcatgagtggcgttaatttgaacttaaaagaattaattacgaatccacaaacgctggtgttgattcccgtgatttttgtcggctacgttttggcaaagagcttggtattcagtgctttaaaattgcgcttcaagaacttaaacgcagttgctggaactgcgatgactgccaccaccattaccgttgtcttggcagtgctgcaggtagccagccacttacacagaattaccagccaacagtcaggtgcattcttgctgtcagccgtcatcacttgtgtctttgggccactgatttttaataagctgtattcatcagaagccgaggatctcaaaaaaacgaccgtgcactttatcggcaccaatttgacgactgttcctgtagcgcaacaattagccaagggctggtatgatgtgaccatgtataccaacaaccagcacaattatcgggccttcaacagtgaaacgaccatccatcggctggacagtttggaaccggaggtcatgattaaaaacggtgtttttgatgctgatgtcgtggtgtttggtcagattaattccgaaaagaattatgaattggcgaaaatcgccaagcaatatggtgtccggcgggtaatcgtccgattcgaagaccgcaatattttagacgatcgcagagatgagttggatcgactgggagtggagctttataataccccagatgttaatatcagcatgttaagagcgttgatcgaagcgccatcaacaatgcgcttaatgacgtccacagattccagtgtctacgaagttgccctgagaaaccggctgtatgctgacattcaggtccgcaacattccatttatcgacaaagttaccattacccaaatttaccgtgacaagcggtttatccggccaaccggtggcacatcgttaaagctaaatgatcggattatttttaccagcagcaaagccgaggcaccagaagttcgtagggaactcggaaaacttaattagtcataatgactcttacccattagaagctgtctaaaatctcttaagtaatagtgctaaaaacgctaaaacgaccatttgcagactggtggttaattgacgctcacaatttttccaaagtcgccgacaattctctagccaactaaaagatcgttcgactacccaatgttgaggcatgacttcgaatcgatgcaactcattgcgcttcgcaacctgcacggttgcgtttaaattactggctacatcgagctgaaaattaacgcctgaataaccaccatcaactaagacattttgaacctggcgtaaatgcatggcatgtaaagcgatcattgcactggccccgtctcgatcagagacgttcgctcgcgtcatgtgaatggcctgcggaaagccattgatatcaactgccagatggcgcttaatccccgagattttcttaccagcgtcgtaacctttgttttcagcagtagcggtgtttttgacgctctgagcgtcaacgataataaaggaagttaaagctgaacgtccttggtaagttcgccgagcaatgacaatttttttaaaacttgttccaataaagaatcagccgtaggctcagctttagttgaccaaattttgtaatagttgtaaactgaccgccattctgggaaatcaccggggacttgacgccattggcaaccggttttcaagacatataggaccgcacagaagacctcgtagaggtcatattttcgaggcttagttcgcttacgaaaattttctaaagctggtcgaattaattcaaattgtttgccgagtaatattgctgggataatttttcatagcttaaactcgctttttacatagaagtatatcaaaaatcatagatcttggacagcttctaagtatcaggccgaaagtgaacgtaagcgaatcattgagcgccagcagcaagggattgccttagctaagcagcagggtaaatatcatgggcgcaaaccccaatacacccaagacgatccccgcttgcaacatgcttttaagctttatcgagctggcatgagtgacattgatgtgtcccgaaatacaggtattaaacggacgacttcaatccattctttgtcgtaacgagttggcatgtaaaaattccttccttttgagagacgatttattcattataccctctcttaaaagttgtctcaggaatcagcttacatccagagattattcttgatttaattggagcaacgggtattgatatacaagaatttgatgaattagctatgaagctttagttgtactaattgcaaatgggactacggaaacttttaatagatttatcgaaaagttcagctaatcactgtttttttgcatatggtcaggaggtggcgatatcatgattaattcatagtaaatacgggtatgagtttccggagtgggcacaggcgggtgctcggatcgataagatggtgtaaggataatagacgtcgtgctaaatagcgtggcgtttttattttgcccaaaatttggaggtggccggcatgggccagatggtaaatagcagatttggccttgtcagtcgcatagagacacgttgcttgggtgacttagaatatcagcttaaatatggacggtggtaacgtaaacagccgcagcgaccacataagccgcgtattacagtgtggagaaaaaacagggtaacaagcgtgaaaaaataaaagaagaccagattttggtcttcttaaaaatgataatttatttatcgtctttatctaacttttcctttacgttatcaaccgtatctttaacagcatctttggcatctgacagtttatctttagccttacctagaataccttgacccttaccttcagcttcgcgggccttgtcgttcgtaaccttgccttcaacttctttagtttttccacttaccttatctttggtgctatcaatcttgtcatctagactcataatataacctcccataatgtatttgttacaacagtattattccacattttaatttgcttgtctaataaggagatcctacaagagatagtgtgaatgacacttataaggtagattgcaaatttaatccgaatttttggacaaatttgtcagcataacctgatacggtgttttccagtcaagtattttaagcggtcgctggttaatttggagtaacgtcgtcgttaaatcttgagcactaatgtgctcaaaacgagtccccttaggataaaaataacgtaaattccgattaaagcgttcattactaccacgttcagctggcgtataagcatgacagtaataggtcttaataccatattgtgattcaaatgatactagcccactaaactcagtaccacggtccacagtaaaactgtgcaccggtccattaaaagttgttaggaacttagtcagtgcttcattaacactcgctgtcgttcggtcctttaaccgatatgcccaaaggaaccgtggtttgcgatcgattaaagttaataaaactgccttactatgcccacgaggaccaacgactgtatctagttcaaaatcgccgatgcgcttacgttgattaatcatcatgggacgctgttcaattgatcgccccaaagattgattatatttggatcgttggtcaacgttacgccgttggcgtacgccatgttcaggtagatcattcaaggggaaatcaattttcccctgatttagccaattataaatagatttagtagctagtttaaattcgtgagcaatcattcctggtgaccagcttagacgtaaatggttgagaattttttgctttaactcatcgctcagcttagttttccgaccacatcgtgatcgcttgtattcggcatctgtttgtgctaattcagcctgataaggttgacatcgagataattcataagaaattgttgacggtgatcggttcagccgaacgcccatttggatattggacagccctagttcacaaaaggtttcgattttaattcgttcggaatagattatactagacaaaagatcagctcctaaaagatgggtttgtggtaaacaccattttaaaggaagctgatcttttttgtccgaacagcgttcggattaaatttgcaatctacctcttacataaagttatttatgaacactgatttaagctaagctgccgatatcacaatctcaccatccactaaatcagccttcaagtttttgacatctaagtggtcaaggtagaaatccgttaccttatcacgaatttgttgttcaattactcgccgtaatggccgcgcacccattgcttcatcatagccttgttccatcagccaatctttggccgctttagttacctcaagtttgatggattttttggctaacgttttttgtacatccgccaacatcaaatcgacaatttgacttaagtcttgcttagtcagatgtgaaaattccacgattccattaaaacggttcagaaattctgggcggaaaaatggtgctaacttatccattaatgactgatctcgttgcttgtcaccacttaatgcttcattaccaaagccagcattagaagtagcaataataatcgtatttttgaaactaatgacattgccttgtccatccgttaagcgcccatcatccatcacttgtaatagtaacgttaatacttgtggatcagccttttcaatttcatctaataatacaatggaatatggattacgccgaacccgttcagttagagtattagcattatcttcatagcctacgtatccagccgaggtaccaattaatttcgacacagctgtacgatcagcatattcactcatatctagccgaataatcgcattttcatttccaaacatatctaaggctaattgcttagctaattcagtctttcctacgccagttgggcccacaaacagaaaacttccaatcggctgatcaccctctgaaaagcccgcacggttacgccgaattgcttttgctaccatttcaaccgcttcatcttgaccgattaccttacttttcagacgcttatcaagatttttcaaatgctcaatatcattagcgcccatatcagaaactggtataccagttaaacgttcaaccgattgtgccacatcatcaatcgtggcagtgattttttctttttgatccgtttctttaattttttgcttggtttcctcgatcgacttcttgatatcagcggcttttttaaagtcctccgatttaacggcggcctccttagctgcctctaattttttaacgcgttgatccaatgtctcaacatcagtttgcgaatttttagccgctaaatgagccgcagtcatgtcgatcaaatcgatagctttatctggcaaagtgcgttgtggtatatattggattgaataatccacagccgccttcaaaacatcatctggtaatacaacatgatgatgcttttcgtacagctttttaacaccttgtaatatacgtaaagtgtcagcggccgtcggttcattaatcacaacctcattgaatcgccgtgccaaagccgcatttttcaaaatagtattgcgatattcatcttgagtcgtagccccgattacagtcagctcgccacgtgacaaagcaggtttaatgatatcagccaatcccttgccaccgtcttcaccaccagtggcacccgtgccgataatctgatgaatttcatcgaagaatagaataatattaccagctgctttaacttcctttaccagctgtttaatattctcttcaaaagaaccgcgatattgagttcctgcttccaaagacgataaatcaatcgaatagatttctttatcttgaatcgtttctggaactttaccagccacaattgcttgtgccagaccttcgacgactgcagttttacctacaccggcatcaccaactaagattggattatttttcgttctacgactcaaaatttctgcagtttcttgaatctcattctcacgtccaatcactggatctagtaatccatcacgagcctgttccgtcaaattagtccctaacttttctaaaatccctccttttttaacagcctgtttaccatctttagatacttctattgttttattattttggggtagcttaccagttgctcggtattgagcaaactcatctggtgtcaacgattttccattaactaagtaccgtgcacgctccgaattttgattatccatgcgccgaaataattgattgaaaacatcatccatatcattgttgaaaaaaggatcattttcgtagaaattcgccatagtacaacacctccataaaaatttacacgtgtaacttagtgaccataatatcctttcaaacttcagctaattgtatcacgatttttatgtatcattaagtaaagtgcttatcggtgtattaaacgagatactttgaaataccattacaacaaaccctttcaggataaattgccgttaattagtatatcaaaatataatatgtggtagattgcaaatttaatccgaatttttggacaaatttgtcagcataacctgatacggtgtttgccagtcgagtattttaagcggtcgctggttaatttggagtaacgtcgtcgttaaatcttgagcactaatgtgctcaaaacgagtccctttaggataaaaataacgtaaattccgattaaagcgttcattactaccacgttcagctggagtataagcatggcagtaataggtcttaataccatattgtgattcaagtgatactagcccactaaactcagtgccacggtccacagtaaagctgtgcaccggaccattaaaagtggttaggaacttagttagtgcttcattaacagtcgctgtcgtccgatcttttaaccggtatgcccaaaggaaccgtgatttgcgatcgattaaagttaataaaactgccttactatgcccacgaggaccaacgactgtatctagttcaaaatcaccgatgcgcttacgttgattaatcatcatgggacgctgttcaattgattgccccaaagattgattatatttggatcgttggtcaacgttacgccgttggcgtacgccatgttcaggtagatcattcaaggagaaaccaattctcccctgatttagccaattataaatagatttagtagctagtttaaattcgtgagcaatcattcctggtgaccagcttagacgtaaatggttgagaattttttgctttaactcatcgctcagcttagttttccgaccacatcgtgatcgcttgtattcggcatctgtttgtgctaattcagcctgataaggttgacatcgagataattcataagatactaaacagtttctcacaccagttttgatctttgccatttactatcatggcaatgaggctaagattgaaggattactgacggcatcacaagtgttcctgagtattgctttaccgtttgccatcatcccactggtcatgttcaccagtaacaagaagttgatgggtgagttcgccaatcatacttgggtcaagtacgctgcttggtttgccaccattgtgctggtaaccttgaacatctacttgattctccagacggttggcttgctgaaataaccgtttaaagacctttataaaaaataagtaggtttccgttatattctttataaaagtgtttagcagttgggagtcgttgacaatttaaaaatttgtctgcggcttcttttcttttagtctaaaatagaggttaataactaacagggggattactaaatgatcaaacccgaaaagacaatcaatggaaccaaatggattgaaacgattcaaatcaatgccgaagaacgggcaaccctcgaagatcagtatggcatcgatgaagatattattgagtacgtcactgataatgatgaaagtactaattatgtttatgatatcaatgaggacgaccaattattcatctttctggcgccgtatgccctcgacaaagatgcgctgagatacattacccagccatttggcatgttgctccataagggcgttttattcacgtttaatcaaagccacatacctgaagtcaacacggcactttactcggcattggataatcccgaggttaagagcgtcgatgcatttattctggaaacactgtttacagttgttgacagctttatcccaatttctcgcggcattaccaagaaacgcaactatttggataaaatgttgaaccgaaagacgaagaacagtgacttggtttcactttcatatcttcaacagacgttgacctttttgtccagcgcggtccaaaccaatctcagtgaactcgatcgtttgccaaagacccattttggtgtcggtgctgaccaagataaaattgatttattcgaagacgtgcaaattgaaggagaacaggtccaacggatgtttgagattgaaacccaagtcgttgaccgaatcgatcataccttcaacagccttgctaataacaacctgaacgatacaatgaaatttttgacaatttggtcactgaccatggctgtgccaacgatcattaccggattctatgggatgaacgtgaaactcccgttagccgggatgcaatatgcttggatgctgactttggggatttctgtcgccttgattgtggcgatgctgattatgctgaaggtctggcggaagatgtgatgggtgagtgacttgctgctgggtgggggacttttttggaatgtgtatagttgagcagttatgctattttgagcacccttcggcttctgaaatacgctccgacgaccctgaccccggccacataagacaaaaaatccagtaacgaacaaaaaccgttcgctactggattttctgccttatgctctggggtcaacccgggtcttgtcacgctcttattttttaccatttctttacccaatcaataccaagcaaaaacattacccttctatactaaaagtgttagaagctgtctaaaatctcttaagtaatagtgctaaaaacgctaaaacgaccatttgcagactggtggttaattgacgctcacaatttttccaaagtcgccgacaattctctagccaactaaaagatcgttcgactacccaacgttggggcatgacttcgaatcgatgcaactcattgcgcttcgcaacctgcacggttgcgtttaaattactggctacatcgagctgaaaattaacgcctgaataaccaccatcaactaagacattttgaacctggcgtaaatgcatggcatgtaaagcgatcatggcactggccccgtctcgatcagagacgttcgctcgcgtcatgtgaatggcctgcggaaagccattgatatcaactgccagatggcgcttaatccccgagattttcttaccagcgtcgtaacctttgttttcagcagtagcggtgtttttgacgctctgagcgtcaacgataataaaggaagttaaagctgaacgtccttggtaagttcgccgagcaatgacaatttttttaaaacttgttccaataaagaatcagccgtaggctcagctttagttgaccaaattttgtaatagttgtaaactgaccgccattctgggaaatcaccggggacttgacgccattggcaaccggttttcaagacatataggaccgcacagaagacctcgtagaggtcatattttcgaggcttagttcgcttacgaaaattttctaaagctggtcgaattaattcaaattgttgccgagtaatattgctgggataatttttcatagcttaaactcgctttttacatagaagtatatcaaaaatcatagatcttggacagcttcttaaaaaggcgtcacattcattgcagtttgcaacggatgtgacgcctatttaaacttatttttcatgatgttcatcgtcatttaaaggacgatcatcatgtttggaagtatccaagattccttctgggagtcctgaatcttttgattgttctttggaggttgatgaagtctttttctccatctcttcttcgcttggcagatgctgcaagattggcagattgatttggaaaatcgaaccggaaccaagtgaactttcaatcgaaatgttaccatggtaagcttcgatcagcctgtgggcaattgaaagtcccagtccgttaccgcctttgtcacgactgcgggctttatcgacccgatagaagcggttgaagaccttttgcttatcctcttcagaaatcccctcaccaaagtcctgaacggcaatgttaaccatggccatcgatgtagacaatgacaggtggacttcttttcgcttggttgaatatttaatggcattatccaaaagaatcaccaatacttgttcgagatgattccgataaatcttaacgtaaacgtcgtgatcggtgtcatcatcaaacgtaaaggtaaaatctggatgaatcattttgaaatcattataaacctgttcaaacacttgattgacatcagtaatttcttcgccgtaattaatttcaatctgttcggcacgggaaagatctaacatttcagaaaccagactcttcattcgattggtttcctgcagtgaagctttcaaagattcttccaagacttcgggatcatctttcccccaccgcagcagcatatcaatatgaccctgaataacggcaaccggtgtccgtaactcatgggaaacgtcctccacgaattgctgctgctggtcaatatagcgctgagtttgatccaacatgccgttcaacagctgagccaagtcggttaattcatcgttggatcgaaaggccggtacccgtgcatctgagtcgggatcgcttttaacttcattaatcgttttttgaatatcattaattggccgcaataattcctgagctagaatataggcaaaaatcatcgtcaaaagaacggaaatcagcaccagaataattaagataaccagcagcttgttagccgtcgctcggtaattgtccaattggtcagtgacctgtgcgtacccaatcaatgagccattcttctttgaaagcagcggttctgagccaaccagaatttgatggccattatgtctggtggtaaaaattttccgcttgctggcagaataaaacttggccgtactcttccgtgattcaaataattccttgccattgacactgtagacattgactaaaatattatcgcgggaaaaattaacgatcaacgaattggaatacaaatcgttgccatcggcttgtgtcacctgatcgttactgtcggtgatctttggcttcaaatagtgtcccacatcgcttttggtcaatggtgaggcataattggtcaaccttgaagaaacggtactcaaggtattgtcaatgtgcgaacgttcctgttgaaataagacgttggtaaatcgattaaaaattaagcatgagaaaataacaacaatcgctaaaacaccaatggacgtaaaaaaagcccacttccattttagcgatgtctttcttctctttggttttgtgttgggttggttcatgaccgcatcacgtaccccgtacctctaactgtttgaatataactgttctcacctggacgatcaatcttgtttcggagatatctgatataaacatcgaccacgttggtttcaacttcggaatcatagccccatactttggtaagcagaacatctcgagccaggacaacgtcaacgttttccatcaaagtcagcaacaattcatattcacgctttgtgaggttaatcacttcatcgccacgacgaacaattcgactttccttttcaatggttaagtctttgaacgtaactgatttcttgttgttcttttgttgatcattttcgatttgaattcggcgaagcaaagcccggattcgagctaagagttcctcaatcgcaaagggtttgacaatgtaatcatcagcgccatgatcaaagcccgaaactcggtcaataacagagtcccgcgcggtcatcatgataattggtgtgttcttcttttcacgtaggcggcgggcaacttccattccgttcaattcaggcaacatcaaatcaagcaaaatgacatcgaagttctcatccaatgcagcctgcaaaccagttctgccgttaagctcaacttgggtatcgtagccttcgtgctttaactccagttcgacgaaacgtgctaagttcttttcgtcttcaataatcaaaattcgactcataaatgatcagctctcccataaaatatcttaatttgtttattagtaacgtagaaaccttttaacataactctcattttaccataattatgagagttttagtcttttactttaataaaacttagaaaaacggctaaaattgcttggaaatatttttcatttaaactaattttgtgtagaaattcacttgataatgcccaaggggacgtttataatgaacttgtttgaaaatatattacaaaaaggatgattaaccctatgaaagctgctgttgtaagagacccagttgatggatatgttgatattaaagatgttactttacgccccattcaccaaggtgaagccttagttcaagttgaatattgtggattatgtcacacagatttacacgttgctgaaggtgactttggtaaggttcctggccgaatcatcggtcacgaaggtgtcggaaaagtcattcaagttgccgacgatgtcactaacttaaagattggcgaccgtgtttcaatcgcttggttctacagaggctgtggtcactgtgagtactgtatcactggccgtgagacactctgccgtaacgttcaaaattccggctacacagttgatggtgctatggctgaacaagtcattgtccctgcagactacgccgttaaagtaccagaaggacttgatccaatcgaagcgacttcattaacctgtgccggcgttacgatgtataaggcactcaaagttggcgacactcgtcccggccaatgggttgaagtcgttggttgtggtggcttgggtaacctcgctgttcaatatgcccataacgtctttggtgcccatgtggtagccgttgatggtaacgagcaaaaacttcaagcagctaaggacaacggtgcagatatcaccatcaaccgtcatgatccagatgttgccgatcaaattcaaaagaaggttggcggcgtgcacaatgctcaaattactgccgttacaactgaggccttcactacatctgttaacgctttgcgtccagatggcaagttggttgctgttgcccttcctaagggtgatatggcacttaacatcgataagacggttctcgatggcattcaagttgccggttcactggttggtaccagacaggacctcgctgaaacattccagttcggcgctgaaggcaaagtaaagccaatcgtacaaactcgtcgacttgatgaggtcaatgacattatcgatgaaatgaaagccaataagattgttggccgaatggttgttgattttactaaataaatataatattgatccaaatgaattaagggccaccagcgaaacgcatctcgctggcggccctatttttatgtcttgaattgtcaaattaagtgcaacacgacattaaagaatatttcataaggcgttttccatccgagacatttacggggacgattattcatttgttctgcatatgcttgtatccggcggtcagtaattgaatcaaggtcagttccttttggcaaatattcgcgaagcaagccgttagtattttcgttagttcctcgttgccaaggagagtgaggatcgggaaagtagaagggcgtactaaacttatcagttaaacattgaactttggcaaactctttacccctattcggggtaatcgttaacgatctaccaggccatagcttcattaagtcgctcaaagtatccgtgactgcttctgaagttcttttagcagctttaccaataagcaggtaacgagattttcgatcaaccaatgtaacaacacaagcctttccgcttttgcctaacacggtatcaccttcccagtgaccaatttctacacggttgtcagcttctcgcggacgatcatgaatcttgtttgggattggaatcttgcctcgcttttcttgataagctttattgtggcgagacttgccgtgatgccttagatggcgcacggcactagagctgccagatttaaacaaattatcaaataagccattgaaaatcccacggtaaatagtcgtggtactgatctgcaccggatacttttcgactgccaagcgattcgatatttcctccggagaccaaaggtcttcgcagaagtgttctctcaccacttcaaacacctgaggattactcaagagagagactctgccacagttgcctttgcgctgtttgtacttctcctgagccttcgaaggtgaataggatttaccagtagaattacggcttaattctcgagaaatggttgagtaacttttcttgatatggctggcaatctcacgaagtgagtttccatgattcctcattaaaaagatagtttcccgttcatctatggtaatatgcttgtagtgatccatggttaaattcctttcatgattgttttcgcaaacatcattttacagaaatttggccatgggccattctttatttaattagtgttgcacttaaagtgtaaattcaaggtatataaaaaccaatttagaatccatggcgttctaaattggttattaattacttgttatctttgataactttacggcctttgtaaaagcctgatggtgatacgtgatgtggcatggtgtattcaccggtctttgggtcgaggctcaaattaggagtcgtcaacttgatgtgaccgcgacgcatgcgctttcttgctttagaagttctacgtgctggtgtagccattctttttccctcctcgtcaaaataaaatatccactagtgaaattttaagtccagctatttcgaatctcgattcttaaaaaagtccttcaattcggccagacgtggatcaacggttttcaattctgccttctgcttgctgtagtcatcgacggacataacatcccaatcgtcaccacttggcatctctttgcctgcaagttcttcaggagacaggacgtgcataggaatatgcaaaatcacattatcaacaactgccctttgcatatcaaccatatcatcttcatctaaaacaaagacaacgtcatcttttccataccgtgattcagcagccttggaaggaacataaaactcctcaactgtaaaatcaagcggtaggtcaacgggtgtcaatgaacgggatgacgggacgaccaacttcccaacaatatgggagtcaataatcacatcaccacgatcggcaaaagcagttccttcaacgtgaaagtcggatgcatcgatcacttcatcagcgtagcgatcaagcaaatcggctttgatttgaaggttctcgttgaatgtgaaaggatcagtatccgagtacttttgcaagtctctaaagtaccatttcaatataattcctccaatgcaacaaaacttattataccggcaacaaataggcttgtcaaggcaatttccttgataggagtttacggattattccaggatgattggatgtcgataataatcttgagacaagccgttaatcatctgggttaacatcccaccccgaaaatccatttggattgtgtcggcaacaacgtcgtcagtaattttggtaatcaatggaacgtcaaggtctcctttgatttgattcaagtatctttgacctaccgcgttaaagcccaacagccggacatatccggccgcctgaagcatatcacttggaactgcatgtaacaagacataggtacacagtcgctggattcttgtatacgtataacgcttggttttgaccaaatgtaggaactcggtgaagctttctgccttgattgcggcccgttttaaacggtactcaattccctcggtcatttgataaatctggtaaagcttttcaatcggactctcaaccaattcaaacctgagaaacggccaaaaatcttgccaggtgagcattcggtcatgctcaagcatccccattgtccccttgggaaccactcgatcagcagccttcaagtcatgtttaaggaccccttggcgaatcgctgtcgcactggcaatagggctggcatcgtcaatttgagtcgcatcatgttggctgccctttcgcttgattggtaccagcgaaagcggcctgcctgtttcaacattggcttttgcgtatccaaatcctaagacatcattgggttgattcaaccgaatgccggttttctcaaatagataatcctggaagacggaggcatatggacgatcaaatcgtttaaagtcggcaggattttttggctgatggtcaatcagcttttgataatccatttcaggatgctcagcaccaaaggccaaccaccgacacttcattttggcagccaaatcaaccgccccttttgagaataggtgggaaggctgaaccgccgaaaataatggcagttcaatgaccaggtcaactccacccagcagggcagcgtgagcccgttgccatttgtcatacgcagccggttcaccccgctgcagccaattgccgctcataatggcgacagtaacatctgcgccggttgcctgctttgcctgttcgagcatatataaatgtccattatgaaagggattgtattctgaaacaatcccaacagcttgaagcatattctccgacttccttaatcttttcccgtactaaagaaccagcgcttggtttcccgtacgaaggggttgtccccaaaatcggtgcttgccagagttaccaagaaaccagtctgtgacagcagatctttaatcaccgtgtcatcgtaagcgcgctcacgatggacttcattatacgcatcataagcatccttctcctcattgtattggaagaagttcaactcgtgttcaacagccattggcgcgaagtcaccttcgtagctggtccacataaaagcggcatcttcactccgatagttgtacatataaccaggataaacctcggttgcctgataaggtgaaatcacgtcaaagagaaactgaccgtccgaattgagatgatcatacactgctttgaaagttgtctccaaatcattttgatcaatcagataattcaaggaatcatcaaaacagcagatcaaatcatactgatcaaggccgtccagattgcgcatatcagtttgaataaagggcacgtcaacacttgcctcgcgtgctctttgctcggcaattgtcagcatgtcctctgatagatccgccccagtcacctgaaaccctttttgggctaatttaatcgccaagcgaccagttccgcaggccagatccaaaattttaatttctgaaggcggtttttggatcccttttgtcttgttcacaacaaaatgggcccaacgatcatagagagttgcgtcaaataaatcatcataaaatttggcgaattctgtatagatcattatgcctccacccacgaatcggtattaacgattggggcatccgaccataatttttccaaattgtaaaaatcacggacatctttctggaaaatgtgaacgaccacgtcaccgaggtcaattaaaatccagcgggcagaatctttaccagaaacactgtagacattgacgtcatcggcttcaacctgatcaacaatttcatcggcaatcgccttcacctgtcgactggaagctgcgtcagcgatgacaaaatagtcagccatcagactaaccttttgcatatcgagaaccacaatatcgttggcacgtttactgtctgccgcacgaacaacgacttctgaaatttctttactgttcatatttactccttaatctattcctgaacttggtacccaactattataagtcatgattgtctgtggaaaaacgggcttattgtgggcaaccaagtatcccaacgtttgtttggtttggtaggcaacgccatcttgcagattattcttggtcatcttgcgtgcctcatcgacacctggaaaatcccgacctggttcaatataatcggccatatagacaatttgttccaacggcgtcatatactggtgcccaactgtatggtacctgacggcgtttaaaatatcaatatcggtgatttgtaactcatttttgacaaacaaccaaccaacaacaccgtgccaaattgcgttgccataattcagcagttcagggtctaattgatagtccttgattgcttgaataaaatcgtcatccggacgttgctttgcatagtcgtggaccaatccaccaatcgccgccttttcaacatcaaccccgttttgttctgcgaggtccatagccgtctgctcaacacgcagacaatgctgaaagcggtgatcactgagagcggcgcgtagtttgccaaccaactcgtcacgagtgtatggaacgaaatggccttgatagattagttgatcatttttcatataaatggttctcctttatataacgttcaacagcggccggaaccaagtacttaattgactggtgctgtcgcatttttgagcgaatcagcgatgatgaaatatcgatgaacggcacgtcaacccaaattaccgggtatttggaagctggtgtgtagccgtcacgtttgacaccgacaaacgaaaccaatttgaccagatcatcgattcgataccattttggcaggtaatcgaccatatcaccaccgataataaagtaatattgattctcgggatgctgttgggtcaactgtttcattgtgtcgtaggaataactgacgccgccacgcataatctcagtcatttcaatggcaaacttgggattgtcccgaatggcgcagttaatcatggccacccgatctttggcatcaatcgcaaatttccggtcaacgtgcggtggattggcatcaggcataaagtaaactttgtcgagccctagttgatccaagacctgttcggcaataattaaatgcccgttatgaattggattgaaggtcccacctaagattccgatgcgtttaccgttttgttttgtaattgttttcgtctgggttaatgtttcgacatgattcatgacgttgctcatccttcattacctctaaatcgccaaaacttcgttggataatttttgcttatttggatcttttgacggcttgaagagaaccaaagtcttcccaatcgtctgaaccaccgtcacatcacttttggtttcaatatagtccttgatgtcatcgacggttgctgttgagttttgtaaaacattgattttaatcagttcacgcgtatcaagtgccttttgaatctcttcaagccaaactggtgaaagaccgtttttaccaacttcaaagattggccgcatgcgattggcattggctcttaaaaatcgtttttgttttcctgttaatttcataagtccctctttatttaaatcattgctgggcgcatcaaaacggatacgcctttaggagcccatccagtgacggaaacgccctctggaacagttacccaacccaagccctcaatcactaaatcacttttttcggtggacttaaatgcatgaggttccaatgctggaaaatcagccttttgatcttcggttggcggtgttagaaatgaacccacatgagtagcgtaaaactcatcggcattttctaatttcgttcgatgaatgaataaattattctcagcatagactgtgaatccatgacgcttctcaccagagttgtaatcaaaacgggcaacgcccccaaagaagagtgtttgacccggatttaactggtaacctttcggcttgattgttttttgtggcgtcaccaaattcaattctttaccggacagatggtgggccatttgctcaggctggatgatccctggggtatccactaagttatgaccgtcattgagcggaatgtcaatccgatccaatgtcgtccctgggaatcgagaagttgtgattaactccttgatgccagttgactggcggacaattgagttgatcagagttgatttaccaacattagtaaccccaacgacataaacatcttttccctgacggtacttttcaatttgatccaacaaacgatcaatatcaaaattcgtcttagcagaaatcagctcaacatcaattggccgaataccggccgcgttagcctgttgtcgcaaccaatccttcaccttgttatgcttcaaggctttgggcaaaatatcgagtttattaccaaccaacaggaccggattgttgccgacaaatcgatggagaccgggaatgaggcttccgttcacatcaaaaatatcaaccacgtacacgatcaaagagtcagtatcagaaatactggttaacagctttaagaagtcatcatccgataaactgacgggagcaatttcattatagtggcgaagtctaaaacaacgctgacaatagacctccccattttcaagccccttcttcaaagcagattcaggggtgtatccgagtgcgttcttgtcagtcgtctggacagctgccccacaacccacacaatgaacgacttcaccgtcaacaacaacttcattatttgccataattcctcctatttccaatgtaaatcaggatattttttcgataatttattccagacaatcttttcaaagtaacgatttatcgtggtattccaagcatcgtcacgcaccagtggcttcaccaaaatgctgcgaacaccgcaactgttggcagccaccacatcagtcatcaattggtcgccaatcataacagtgttgcgcttttgtaaattaaattccttgagagcgtgccggataccgatagtgagcggcttcattgccctgggaacaaacggcagctcgtaatcttgaaccgcgcgttgaattcgcttgtgactgttattggacacaacaatcaccttaatgccaaatttcttattttctgacaaccagttgcgtaacgcttgagaacccttcttggagttccaaggtaccaaggtattgtctaaatcggttagaacacagttgatattatgatcccgcaggaattggggagaaatcgtgtaaatatccccaatcatccatgttggtttaaatcgagacaacatatgtcgctccttaaattatagtaaatttatttaaaaaaacttccaccaaactatcggtgaaagtcattttagcacatcaaaattacttaagtgcttttttagcttcgtcagttaaagctttgaaagcttcagtatcactaactgctaaatcagcaagcattttacggttcatgtcgatgttggcaagcttcagaccgtgcataaattggctgtagctgaggtcattaagacgagcagcagcgttaatccgtgcaatccaaagtttacggaagttacctttgttgttacgacggtcacggaatgcatatacctgtgacttcataacttggtctttggcagtcttgaataaacgagactttccaccgcgataacccttagctaattttaaaacacgcttacgacgtgcatgtgtgactgttccaccttttactcgtggcattttgaattcctcctatattttgaaaagtaataattgaatgtatagttgattttatagatgtggcaataacttcttataagttttgatattagtcttgtccatcatactagtaccacgaagttggcggcgttgcttctttgtcttaccgtggaaacggtgactggtataagcattggcactcttaaatccaccgttggcagttctcttaaaacgttttgctgcagcacggtttgttttttgtttaggcattggtaaaaatcctcctcaagtatttaacaactattatttttgatcttggtcttttggtgaaagcattaagaacatgcttcttccgtccatcttaggtcgttgggtaacggtggcaacatccgccgtttcagcagccattcggtcaagaactttccggccgatatccttatgcgtaatggcacggcccttaaatcgaattgagacccgaaccttttcgccctttgccaaaaacttcttagcattcttcaatttggtgttaaaatcgttcacatcaattgttgggcttaatcgaacttccttgacactgatgactttttgtttcttacgggattcacgttccttcttctgcaactcgaaacgatacttcccataatcaagaatctttgcaaccggtggcttggctttcggtgcaaccaggacaagatccaagtcggcatcttcagctaactgaagagcttctgacttagtcttaacaccaagttgatcaccattagcaccaatcaaacgaacctcacgagcacggattccatcattaaccatcatatcttttgctatggtacttcacctccgaataatttgaaaaagcagaaagagagcgggcacacatttgcgcccgctctcaattaaagaacttggctgaccaagctcttactcgatatcatgcccagcaaattcagaaatttactcaggcgagaagcgggtagctcctgctttcatttgaacaactattacagaatatcatctaatcacttatgtgtcaactatgaaccgttaagcacattaataagtgactcagtaattcgttaatcttcttcgcgtgaatatgaagcaatgtctttagatacttcatcaatgaagtccggaactgactctgattgggtatcctgctcaccatacttacgaactgaaacgctgttgccactcacttcttcatcaccgacaactaacgtatatggaatcttgtgagtctgtgcatcgcggatcaggtaacccatcttttcggcacgagtatcaactgacgaacgaatcttcaatgcccgaagttggtcgttaatcttcttagcgtaatccaggtgcttgtcttggctgacaggaataatcttaacttgatgtggtgctaaccaggttgggaaggcacccttgtagatttcagtcaggtaagcaacaaatcgttccatggtagaaaccaggccacggtgaatcatgactgggcgatgttgtttgccatcttcgccgatgtagtgaagatcgaagcgttcaggaagcataaagtctaattgaatcgttgacaaagtttcttcatttcccagagcggtcttggtctgaacatccagctttggaccatagaaggcagcttcaccttcggcttcaacataatccaagcccatttcatccatggcacctttcaacatggtctgagcacgggtccacatttcatcgtcatcgaagtacttttcggtgttcttcgggtcacggtagctcaaacggaaggtgtaatcgttaatatcaaaatcgtgataaacctcaaccatcaagttcaagatattcttgaattcttcttgaatctggtccaaggcgacaaatgtatgaccatcattcaaagtcatttcacgaactcgttgaagtccggacaaagcacctgatttttcgtaacggtgcatcattccgagttcagcgatccgaagtggcagttcacgatatgaacggatatggtggttataaatttgaatatgacttgggcagttcattggccgcagttcaagctcttcaccgtctcccatgtccattggcgggaacatgtcctcacggtagtgatcccagtgtcctgattgtttatacagatcaaggttggctaaaaccggtgtgtaaacgtgttggtatccgttggcaacttccttgtcaacaatgtagcgttcaatggttcttctgatcgttgcaccgtttggcatccagtaaggcaagccggcaccgacttttggatcaacaaagaacagatccagttcgttcccgatgactcggtgatcacgttcatgggcttccttgcgcttctcaaggtcggcatccaaatctttttgcttgttaaaagcagttgcataaatccgttgaagcattgggttggatgacttgccctgccagtaagctccggcaactgagagcagcttgaagatcttaactttgccggttgatggtaaaacagctccttcggcgattgactggaagtcaccgatttggaagaatttaacttggccgttaacttcgtttgctttgaccaattctttttgataaggatcgtcgccggcaacctttgcagcgtcatcagcgcttaagaagaccaccttgattggcagatcctgtttgataatcttatgcattgaatcttcaagtgcactcaattgatcaacactgatttgagtgtcaggtttatcggtatcaacgaagaagccgtcttcatcggcatcgctttcaccaaagtggatattatcaaaatcattggcaattgccattttcaaaatctgggcggcagttgcgcgtaatacactgaggccttcgtcactatctgacgtaacaatttcaatcttgccgcccttatgtaggggctcgtcattgttgacccattttccgtcaaccttggcggcaacggcttttttacctaaactgacggcaattgatttggcaatggcttctgaggtaacgccgtcatcaaattgtttaacactaccatctggaaattcaaatgaaagttgtgacatatttcttactccctttatatttttattggagccacaaaaaaagcccctgacatacttatacaagtacatcagggacgcaattagcgcggttccacccaaattggatttttggatacaattatccaaaaagctctcaagtggctgctaacggtaccaaccgggaaagcattatccgcaatccattctcaaagagtggtaacaaacaatttctcaacaaacggtcttccaggctggaaccattctccctgtgatgagtcatcactgtcatgtctctttgattcattgacatttagtatagagttgccgttcaaaaatgtcaattcaatttgtaaattaaactggtcgccgatttttaccagtcatctcgacctcacgagacaagaatcgaattcgctgcatgagtcgtttggctttcaatggttcatcgtcgcctttttgattgatacgcaaatgttcctgttcgagttgggccattgaaaaattagacgtaaaaaacgtcggtagctgctgttgcatccggtattccaaaataacgcccaatacttcatcacgaacccacgaggacattgagtcagccccaatatcatcaatcatcagcaccggcgactttttgatcacatcaattttttcggtgaccgagttatcggtgatcgccgatttcatttcgacagcaaaacttggaaaatggaccatagtggtttgaatcccgttatcggcaagttcgttggcaattgcacctgtcaggtatgttttaccgacaccaaacggcccatatatgtacagacccggatggaaagtctttttgtcggccttcatttgagcaataaaatccaatgccattgaaagggccgtataacgattggggtctggattatcgggatcagccccgtcgaattcggcgatccgggcatccttgatatctttaggcattgaaaccgtcttgattcgacgcgccaaggactgactgcgctgcttttcgatgacctctggagaggccgaatacgcaatatcaatcaagtgatcgttaatgaccaattggggcaaatacccaggcgcaaatgattgtttcttggccttaatctgatttttgacattcacatactcatacagtttggcagcagaacggtcaaccgcatcaggagccagttcaccttgatgatcctgaagaaatttggcgatctcagggtcatttttgatctgttcgataattttttggaaacctgatgcgacattgccacccttaaattgacggtcttccattagtttcttgacgaaatcacttactttttccattcaatctcacctactccccggcttttttaacttatcaagctgtgctttaagctgcttcttttgggcatcagtcaactgtgaggttggctggctggcagaggaaggttgatcatccttcgcccaatccggcagggtctctttgacattaacccgtcgctgtttgtacttggcagcccgcttatcagcttttttctgtttgtcgattgttcgattcttaatggcatcgattgcatgctcggcatcaaaaatcccgtgttgtgaccaatcatcggcaatcgttgacatcaggtttttattgagagtcgaacgattttcatcaactaataaatagtaaatcaaaatattgatgacttcattcggcaacacgcgcaggttgacaagctcgcgcaaggttcgctgctcaccgctggtcacaataccgtgcttttgtttcttgatttgttccaaaaacacgacaggagccgtctttttactaattgaaatcagttgagtggttgccgtgtcgaattttgcagaagaaggcgtgatctcggcagtaggtgctgccttctccacgttctctgcttgatgccggctgaaattgtcagtaataattgccttcaactgtgattgattcaattcattggtgctgagattagttgccttttgaatgagtttagccatttggatctcatcaattccatagagcaaattctctgacaaaatcaaatcacgagcggctttaacagagttaagatcgacgtatgaattttccaacatgcttaataggagtttgaagttaaactggtgactatccggttcgaaactgttctcactgacatttgcagctgatcgaacaatggtctgcttggcgtcgttgactgcgcccggaatgtttttaatcaggttctggggcacagcaaataaatccagcagtgaagccgaaatattggtcgtctccccgagatccggaagtggcagcactagtcggtcgacaatctgcttgtaggttgtttcgcccactttgctcaataaaataatcgacaaaatatcggttcgtaaaaactgttcagcagttagcggcagattcaacgagtagatcaagacatccggtttgttttgggaaaccaaagtattgatcagtttaacgccttccaattgctttcgaatcgccaccagctggtcaattttgcaatttaacatgctctgaatttcgtaatgcttatgcaaaaccaactgattatgatcatttaagctcatcgaccacaacaaattgtataatcccaatgctttttcaccaatgattggtagatacaaattggttagaacactgtgatcaaggctccgattaatatgggcattggtcgtgagatattttgtatcgggtgttaatttatcgaacgactctgccattatttgtcccccgagtgatcctgaccctttttcttatccttttccataatttccttaagctctttataaaagaccgacatatccttgaattgacggtaaacactggcaaaccggatataggcaatttcatccaaattggccaaatcttccatgacgtattcaccaatttgttggctggaaacttcattctcgcctagtgaccgcaatttattttcaacccgatccaccaaattggtaatggcatccatcgaaaccggccgtttttcagcggacctgacgatcccctttaacagtttttcacggttaaattcttcgcggttaccatttttcttcaccactaataacggtgttacttcgacccgctcaaatgtggtaaatcgaaaaccgcagtgttcacattctcttcttcgtctgatcacccgaccgtcatcagttggccggctgtcgacaaccttggaaccattgtatccgcaatgaggacattgcatggtgttcacctcgtctatttcgtttccttcgccaaccatctgtcgacttgtgtcagcgttgttgtcattgttcctgagttataaataattgtatcagccaaatcgcattttgtctgcaatggccattgatttccgattcttttaattgcacttacaatactcagtttattgcgttttatcaatctctgcaactgagtgaccggatcacagtaaaccaccaccacctcgtcgactaagtggacatagccattttcaaataaagttggtgcgtccaagacggtcatttcagtatcccgataacgtttcaactgagaaagaatctcttcgcgaatgaatgggtcaatgattcgaaccagttgtttgagatcagctggattgttaaacacaatccggccgagtgcctggcggtcaagtgcgccgtcagccagcaaaatccgctgtccaaatgcgtccaccagtgcttggagcccaggagtcccggtttgttcaacttgatgggtcacgatgtcagcgtcaatcacaggaatcccctgctgatgaaggtaatcgctgaccactgattttccggtggcaatcccgccggttaagccaattaatttagtcattttttacaccacgtaaaggttggcattttgggcaaaagtgggtgccccgctgagccaacttgattttaacaatctttgtgccgcatctcgagcagggttcgccttcacggccgtaaacattcaattgattttgaaaactgccggcttccccatatgcagttgaatatgagtggacggtcgttccatgaccggcaatcgccttggctaattcggcgataatattttttcgcaactctttaatttgtctcaacgtcaacgtgttggcaggctgttgaggattaattttgcttagccataagacctcatcggcgtaaatattacccaacccggcaatattactctggtctagtaaaaatggtttgatcactttgcggctcttaccaaaaattttctgcatgtaatcgacggtcaaatcatcttcggtgggctccggtccaatcgttttcagaccggcaacctgcatttcagtgccagtatcaaccaaattcattcggccaaattttcgcgtatcattgtaacgcaactggcgcccatcggtcagatgaaaaatgatatgggtatgcttaccgaccggtgcatcttcaggctccacatcgtacttgccttccattctcagatgagaaacaatcgtcagattatcgctcagtcgaatcagaaggtatttaccacgtcgatcaattttttcaatcgttttgccacggagggcttttttgaaatcgtttggtggtaaattaatcattttggcatacaacacatccaccgattggatggtgcttcctttaaccaattgggtcaggccgcgtctaacggtctcaacttcaggtaattcaggcattgagatcccccatttgcttcaacttattttgcatcataccaggtcttaccccagtggctttcaacttttaatggcacattcaagtggatcgctgaatccatgacgcttggaatcagttgtttgacggtgtccaattcctcgtcaggaacttcaaaaattaattcatcgtgaacctgcagcagcatgcgggttttcatatccttgattgcatcggccatattaatcatcgcaattttgatgatgtcggccgcactgccttggattggtgtgttcatggcagtccgttcagcgaatgaacgcagattaaagctcttggaattaatatccggcaaataacggcgtcgatgggcaatcgtctcaacgtagcggtggttacgggcaaattcaacgatgtcttcggtatattttttaacgccgggatattcttcaaaataacgttcaataaactgatgcgcctgttttctggtaatgccggtattggacgctaaaccaaaatcgctaatcccataaacaatcccaaagttaactgccttggcctgacgccgaagttccggggtgacttcttcatttgacggcagtccaaaaattctccgtgccgtggtggcatgaatatcctcgccatttttaaaggcgtcctgcatattttggtcgtcggtaattgacgccaacacccgcagttcaatttgagaataatcagaggagaaaatctgccagcctggatgtgatggaataaaggcctggcgaataagtcggccttcctcggagcgaaccggaatattctgcagattgggatcgactgaagacaatcgaccagtctgggttaacgtctgcagatatctggtgtgaactttggaatcatctggatgaatgacctttaatagcccatcaacatatgtcgactgtagtttggaaatctgacggtagtccaacacattttgaacaattggtgcatccggagccagtttctccaaaacatcaaccgaggtcgaatagccggttttggtcttctttagaatcggcaggcggagcttttcaaacagaatctttcccagttgtttgggagaaccaatgttaaattcttcaccagcttcttggaaaatggtctgttcaatttcagcgagccgctctttaaacttactgcccatgccctccaaagtggctgcatcaactttgatgccattgatttccatgtgggcaaggacaaaggcaatcttgatttcgatatcccagtacagtttggattgattatgggcatccagatccttaaacatcccgtcgtgaagagcatcaatcgctttgaccttatgaaccaaatgggccaaaaaggcaggtgattgcgggtcaatgtgtcgcttggcaccctttccatagacttcttcatcggttttaacattatagaatccgtgtaaatgggcaacggtgccgacgtcgttgctattattagttgtattaagcaaatatgataccagcagcatatcgaagtccacgttggcaagctcaatcccttgtcgataaagaccgacataggttcgtttggcatcaaaaaggttctttttgatggtcttgctggtcaggaggtcactgacatgctgattgtgaagcaattcaggatcgttggtcacataccatttgttaccctgtccaatcgcaaagccaaccaatggcgatgtgtggtagttttcttctgacatttccaggtgaaaagtcacttcatctgtgaactgatccagctcagccgcattcttggcggacaagacagtgtattgaatatctgcttgatcgtcggcatgatcctgatcatcaacagataacttggccagaaacgatttgaagcccattctctcgtaaaaatcggtcagtttatcgatattgtctccctgatacttcaactgatccaaagagactgttaccggcgcgtcgcggttgattgttgccaacgtgtgggcgcgctcggcctgggcttggtcatgaatcaaatgttcctttaattttttaccggaaacctggtcgatattttgatagagattgtcaatcgtgccaaattgttgaaccagcttgacagctgtcttgtcaccgactttttcaacgccgggatagttgtcggagttgtcgcctttcagacccttaatttcaataatctggctcggtttaacacccagcttttcttcgacgtgtttgggggtatatgtttccagttcggtgacaccctttttagaaacctgaaccgtggtcttatctgaagttaactgggtcaaatctcgatcgccggtgacaatcacaacttggtagtcaccagcttcttcagcctttttggcgagcgttccaataatatcatcggcctcataatccggtaattcataggtggaaatgccgcgggcgttgatcaattcttttaagaagggaaattgctcggaaagttcagttggtgtcttagctcgaccgcctttataatcagcgtacattttcgttcgaaaagtggttttgccggcatcaaatgcgaccagcacatcggtgggcttctcgtctgctaatactttgtccaacatccggttaaagccataaatggcgctggtatgtaggccagatggattggtaaatttgtccatggccgtgtataaagcataaaacgctttgaaggcaatactattaccatcaattaataataattttttagtcattaacttctcctctggtgaaaactgttactttaattttaccacgacagataacaaaaaacgatcaaccaaatcaatggccaatcgttgtgacgaagtgtgaattaacggtcgttgttgccgaaaatcgagagtaattggagaaacaggttcacaaagtccaagtacaattgtaaagcaccaaagactgccaaaccggtcatggaaacatcaccattaccagaatattggttatacatctgcttcatcttttgggtgtcataggcggttaagaccgtgaagattaacactgcgatgatcgagaaaacaaatgaaatcactgaactgcgcaggaagatgttaataatcatggcaatgattaacgcaattaaagcagcagttgcttgggcaccccaacgatcaaggttcttgtgggtgactaatccaacggttgtcattgtgatgaaaattgccgaagcggaaacaaaagctgccgcaattgaggcacctgtatacgcccacgcaatcgtggcgaaaacaaaaccacttagaattgaatacaacatcagtactgtaaacgcgagggtcggccgtttcaacgcttgaagtgagatgacaaatggcaaaacaaaccacaaaatcattgatccccacatcacaccttggtgacctgcaatgtaagccgccattccaccagcaacagacccactaactaaaaatgctgttgctgcagaaactaaaacggccaaactcatccagccatacattttagttaaaaaagcattcaacccggctgcgttgttgacgactcgtcgagcttcctgttgttcatttggataattgttcattaaatccgctcccttttgtttgtaagttcaaatattgcctcaaacaatttgcagtatttatacttatactgttaagtaattctaccaaataaaagccattaatcaagtatttaggactcaactaacagcttttataagatatcttaattaatttttttgcttaaatggcttagcagatcttcgtaagatttttcatacttttgaatgtcgccagcacccatgaaaataaccacgtcgttatcgtagtccaatagtggcgacatattgtcaacggacaaaatgcggccacccttagtgatcttcttagacaggtcctcgctggaaacttttccgtgactttctcgcggcgaactgtaaatcgaggtcaggaaaacttcatcggccaagttcaaactcttggcaaaatcatccattaaagcgatcgttcggctgaaagtatgcggctggaagaccacggcaatctttttgcttggatattcctgacgggcagcatcgatggttgccttaatttcagttggatgatgggcataatcgtcaatgatcgtcatcccggcaatcttacgttcggcgaaccgacgcttaacgccttggaaagtcttcaattctttgcgaatttcatccaaatcaacatcttcaaagtaagccacggcaatcacagccagtgaattgaaaatgttatgctcaccaaacaatggcactgaaaagtttcccagatttttacctttataagtgacatcaaagctcgaaccactggtcgtccgcttaacatccaccgcttggaaatcatcagtatccttgaggccataataatagattggtaccttggcttttagttgacggagacgtttatcatcaccccaggcaaagatgcccttcttcgtctggttcgcaaacgtttgaaatgcatcggcaacatcgtcgatgctcttgtagtaatccggatgatcaaagtcaatgttagtcataatggcgtaatccggttcggttgccaaaaagtgacgacggtattcatcagcttcgtagacgaagaaccgggcattgggaacacctttcccagaaccatcaccgattaaataatcggttggtgcaattcctgaaagcacgtgggctaacaggccagtcgtactggtcttcccatgggcaccagaaaccccgatgctggtcttacccttgatgatcttgccaagaaactcgtgataacgataaaccgtcaaccccatgtctctggctttcttaatttctggatgatcatcagtaaaggagttaccggcaatcaccgttaatccttcgtgaatgttgttttcatcgaaaggtaaaattttaataccagccttttcaagcccgcgttgtgtaaacgtgtactggtcaatgtctgacccctgcactttctcaccacggtcatgcaagattaaggccatggcggccatcccggttcctttaattcctacaaaataatataccgtatctgaattcattagacatcctacctatccattatgttatttttgatgattctgctgtgattcccgagcggattcatctgccgccggcttgtaatacactgtccgcggcttggacccctgctgctctgaaaccaagttcttttcctgcaaatgatcaataatgtttgcagctctattatacccgattgaaaatacccgttgaagctttgaagtggaaattgtctcttcattgccaatatattttaaaacctggggcatcaaccgatcctcagaactggtttcagtactggctcgtttcaagctatcaggagtaaataagtatttaggttctccctgttggcggacataatcaacaattccgtcaagctcctgattggtgacaaaagcaccttggagtcggaccggctgatttgcaccactccctagatatagcatatctccgcggccaagtaaacgttctgctccggcggaatccaaaatcgttctggaatcgacttggctggataccatgaaagcaatccgagtcggaatgttattcttgatggtcccggtcacaatatcaacacttggacgctgcgtagcaacaatcaaatggatgccggctgcgcgggctttttgagtgatgcggacaatgtaatcttcaacttcactggaagcgaccatcatcaggtcagccaattcatcaatgatcaccagaatataaggcattttcagcccatactcgtgagcctcacttgcctgtcgattgaactgttcaatatttttagcaccagcagctgcgagcttttcataacgccggtccatttcctcagtgacccatttaagggaagctgcggccgtcttaggatcggaaataacaggtgataacaagtgaggaatcccgtcataaggtgccagttcaactgcctttggatcgattaacagtaatcgtaaatccgccggggtcgctttgtacagcaaagaaaccaacaaactgttgatgaaaacacttttgccggatccagttgccccagcaatcaaaccatgaggcatctttttaatgtctgtcgttctgggaactcccgacaaatcaacacccaaggcagtggtgagtggcgattgactgtcttgaaaatgcttggttgaaatcacttctgaaaggaccaccggcctcggattgggattagggatctcaattccgactgtcgttttaccaggaattggcgcttcaattcgaatatccttggctgccaacgccagctttaagtcatcggttaagttggtaatccggctgactttgacgcccagtgccaatttgacttgaaattgcgtgaccgttgggccatttgtccagtcaaccacttgcgcattgaccttgaaggctgagaaagtttgattcaggatttcagattggtgaataatccagtcatcaattgaatctgattcagcttgctgcggcttggccaacaaagacagcggcggaaattggtaacctctgtcttcagtcggcttctctgagacgtttggttcagccgatgaatgttgaacacccttcgtgggttgattaacgtgattcacttttttaacctgggcattgtgactcagttgttgagcgttaaacaaagaaaggtcagattcgctggccctttggttatgcataattgaattgaatgactgtcccaacccatggtgattcaaagccttccgcggttgacgatttaaatgccgaaccccttggtctgagctgatctgtggttgatctgtcactgatgatttctcaaaggatttcacagatgaattttgaggttgaccttcagtcggcttgacgggctttgttgattgaacggggtgctttagatgctgctcacgaggctgatcaattgttggttgcttattggcaatcacaatgagatcatcatatgtaatcctcagccggcgtgtcaattcatcgtacagacggtgacgacgatgctcttggctgagaaaataattcgtttgaatttgctgtttccgtttatcggattttgaccgcttttgcggcttgaaatttttaatttctttcaaaaaagccggggtctcatcccgacgatcaaacttggaatcagggaccttgcttaaccttgtagcttggattttcggtgccaccggctgattattctgttttgtttcccgctcttgatgaggctttcgggtaatgcccttccgccgaaaaaatgcgggtccatcataatgcttcattactcatccacccaaagtcctttaatcaaataaatgctgtgccttgtgaaaatcaaaggcatcccctacctggtaatcatcaggtaaaatcagtgccccgggaacttgcggtgcgttgggcagccccaactcgcggccggaacaaatcatgccatcgctttcaacaccacgtaatttaccaggccaaataatttggccgtcaggcatcatggctccacttaacgcaacaaccactctaatgtcctcacgcatgtttggcgagccgctgacaatttggacgtccttaccggtgccaatgtcagttttggtaatctgtaaatgatttgccttggggtggtcttccactgatttgacatagccgacaacaaatttgggttgattatcataacggatatctgccggaaaaccgtgatcgcccaaatattggttcaagcgagtaacctggtcttcggttaaatgaacttggccattttcatggacaatttctggaaggactttacttgcttctaaaaagttgtaccccaacgtctgattgctatcagcggcaaaaatccgggcaaccttatcatgaattgtcacactttgttcacccacatccgggttcataatgaggaccattgtgtcacctgtgctgtttgggttataactggttattaacatttcaaaattccttccaacaattaattattttgctacggtacttgctaacgagttaataaagttttcaacttcggctttagtcttgcggtcgccattattgaagcggccgatttcttgaccgtctgaataggcaacaaaacttggaatgcccataatgcccattttaccggcaagatcgatattttcatcacgatcaacctgtaagaatgtgtactctggatattcggcttcaattgcaggcattgccggcttgatgaagcggcagtccgggcaccagtcagcggtgaagaacagcatatacttgccgttctcaagttgtttggttaaatcttttaaattggttttaggtaaattttgcaaaattatcatcctttcacttactaatgtaaagtacatcatagcacaaatttccgaccagccaaatcagtttgctcatccgctgctaatagtctaaagtatacatatcatatacaaaaaaggtgaaatgatgaaaaaacaaaccgtcttctatggcctggcactcgcagcctttgccggcagtgcctatttcgtggccaagtccgatcgcaaacacgaaaagtttttagcagctatcgtcaaggataccaaacaatcagccgcattaaaaggcttcaaatatattggcagttggagcattctaccgaccactgattccacgccgctttttcactttggcttcaattatttgaaccctgaaggtgatcgcaaaacagaagaattctgggtcgaccaaacctcacaacaagtggttaagcatcaagtcatgacgctgtaaaatgcacaatcagcttataaatgggtcccttgggactgaacttttgctcatactccgtttcgatattcgattcattttcaggagaatgatgtaaatccaacgaaacataatcgaacttcatcgggaaattattcatggtgaccagggtgtattcgaataaaccgcgattatcagttttgaattcgatatccccgtcctgatccagcacatgattataagtcttcaaaaacagtggtgatgtcaaacgacgtttggcatgccgcctttttggccaaggatcggagaagttcaagaaaatctttttaatttcattttcataaaacaattcatcaagattggcaccatcagtcagaacaaactgcacgtttggcaacggatccgccataaacgaccgtagtgccgtggcaatgactgaagtctgcagttcaatgccaatatagttgatgtcggggttggctcgagcagtctcaataatgaaccggcccttaccaatcccaacctcaacgtttaagggttggactttggcaaaccggtcctgccatttacccaaccaattctttggatcggtcacaatatagtcgccgtggtttttgatatatttatcagcccacggcttttttcttacacgcatatcattctcctattattcaacgatttatctggttcgctcgcttcgagccaaacgtctgggtaaatacagatagacaaatgcccagatttcgagtgcttcgccgacaatcacgtcaatgatcgtgaccggcgtggccaaattaacggtcagaactgccaccgcaaaaacgacgccaaccgtagtcaacaagtacagcagaaccctttgaaaactcttcaattggtactgattggtaattggataaatgtggacgaaggcgttatccgagaaatgaaaataaaacggaatcatttggaacccaattaagtagacaaacagcaggctcaaaaagatgggtaacagctcgcctttgacgaataccagaaataaggttccgatcaccagcagacgaacgtatagcccactcatctcattgtcacggacaattccgtgagcgtagagatataagtaggtgttttttggaatcagcttgattcggttcaagaccccgtccacgtaacggcggcgtttgacagacccttgcagagttggcacatccgtaaacaaattaaagaattgatagacggtgtgcatccgactgttttcatcggtaatcatcgtcgtccagtcaagtgatcggctgacccaattccggcgggaaaaataactgacgaaaagcgcagccacagcaatgcccaacccaagccaatagttgatgtagatagacgatcccaatgcaatcactgggacaagcaatcgaaagatgagccgactggccaaccaggattgctgcaaatggtatttgcgggcaaagtctgtatttagccacgttattttcaagattaaaatggttgccaaaagcagatacaactccgtcgatgtggcgcgcatggtaacttgaacaaacggcatcaacaagatccaaaacagaacttgaattgcgacagcaatcgaaaaactataccgaaagccgcttcgaagatagttataaagttcagcttctttgggcaacaaaaaaacatagtctggggcttcaatcaaggtcgcaaacctgcccagctgaacgctaaccaacaaaataccgataatcacaattggtgcccaccacagaccggtgtgcagctgcttaagtgcattggaatagtagtatcccaacccaccaataacaaacaacaaagccaggacaaagtagtcgttaaaaaccaatctgagatagcgcatcatttcctttagatgcgtcgttaaacgctgcctgaataactgcttcatgaggcatcgccttcccttgccagagtcaggtaaatatcattgagagaatcgccggcatctgggaataatttccgcagctcttcaatcgttccttcggtgcgaacttgaccgtcatgaagtaaaacgaaccgatcacaataacgttgcgcggtatccagcacgtgagtcgacatcaaaatgctggctccctgttgctttctttcagagatcaggttcaataagtcgttaacggccagcggatccaagccaagaaacggctcgtcaataataaagagtttggcgttagtcaaaaaggcacagacaatcatcaccttttggcgcatcccttttgaaaagttgtccgggaaccagtctaatttattatccagccggaaaagtttgagcaggtcatgtgctcgtttccaagattcgtcttgatcaagtccataggccagcatggtcatttccaaatgttcctttagcgtcaattccttgtagacaattggctgctcgggaatataagcaatctgctctttatattgtttaacgtcatcgtttaagccgacgccgttgattttgattgagcctttaaatggcgttaataaaccgataatatgattgatggtcgttgacttgccggcaccgttcaagccgatcaacccaaccaactcgccatccttaacgtcaaaattgacgtcctttaacactggtacttgggaatagcccccaaccagattcgaaacttgtaaggtcattgtttacctccgtatcatgataaatgtacaaacaagattataccatacaaaattagcctttgagctgggtcaaaaacgcaataatggtataatatcattagtattcacagaaagaaggtagaaattttgaaagattgtattttttgtaaaatcgtaagaaatgagatccccagctacaccgtgtatgaggacgacattgtcaaagcattcctggatatttctcaagggactcctggacatacgctggtgattccaaagaagcacatcgccaatatctttgaatatgatgaagaattagccagtgaagtttttgccagaatcccaaagattgctcgggcagtcaaagcttcaaatcccgacatcaaaggcatgaacattttaaataataacggccaagtcgcttatcagtccgtctttcattcacacttccacctggttccccgatataccagtaacgacgactttaagatgatcttcaaggataactccaacaaatattcaccggaacagttaaaggcgattcaagaatccattgaacaacatatgggtgattaatcatgaaaaccgtttttaaaattgttggtgcaactgccgttgtcgccggagtttatttatacagccgaaaagaaactccccaagagttcgttgaacaagccaagtcgacatttaatgatcgaaagcaaaaggccgctgactggaaagctgcttatgatgactttaagaagttgatgaatgctttcacagcacagatgccggcccttgagaagaccattaacgacatctcacgggatgtggataaagcgatgttcaaaattcagccacggcttgacgaaatcaacaagtataccgacaaattaaagtaagtaaaatatgaatatttgtttaaattcttgaggtcattatataaacgacgcagattatgttattattatcgggaacgtttgctttgcagacgaatacttttaggaatggatgtgtttttgtatgaaaaaatggctaatcgttttagccggcattatgatgagttttacccttgcagcttgtggcagcaaaactgttgcaacaaccaatggtggtaagattactgaaagtgcttattacagcagtttgaagagtacttcaagcggtaaacaagtattgcagcaaatgatcttgaacaaggtcttggaaaagcaatacggcaaagatgttaaggactctcaagttaatagtgaattcgctaaatacaagaaacaatacggttcatcattcaactcagttctccaacaaaacggtatgactgcttcacaattgaaagattcaattcgttccaatctcttattgaagcaagccgttaaggacaacgtcaagattaccgacgcacaacttgaaactcaattcaagtcttaccaaccaaaagtaactgttaaccaaatcttggtttcaaagaaatcaactgctgaaaaagttatcagtgaacttaaagacggtaagagcttctcaagcttagctaaaaagtattcaactgatacagcaactaagaacaagggcggccgaatcgcagcattcgacaacaccaacacatcacttgatgccaacttcaagaaagctgccttcaagctgaagaacggtgaatataccaagacccctgttaagactcagtatggttaccaagtaatccaaatggtcaaccatccatcaaagggaacttggaagcaacacgaatctgaattaaaggatcaaatcgttaccagcaagatgtctgatagcaataccttacattcagttgtttctaaggttcttaagaagggtaaagttaccatccaagataaagacctgcaaaacgtcttatcagactacctttcaaccagctcatcagctaagaagtaatttttaaatcattcatacaaaaaaggattggacaattaaggttcttcgtcaactgttgttggtgaacaaaatattggagttctaatcacttggtgattagggctctttttgtatgaactcgaaaagcgaacagcactcttagccggaatctgaagaagtttcggtaaccaaatccagtacgcttaatgactttaatcttgttgtttgaaccttctaatggcccgttggtgtagtggtgggtgaaagtgttgccaatttcatcatgatgagccgccaaggtttggagggctgccaacatctcttccgagcacccctgcaggtggtgaaaggcttgattatagttgggccagtcgcggtttttgatggtttcacgtaaccgattcatcacgtcgtaagtttgcttgagctcgggatcaatgtccagtaaagcatcaaccacatccgtggcagttgccggataagggaagtttgtccacttacggaaagcctcgtagttaaggtgattggccggcgttaataatagtttccaatagcgtttcaaggcgtgatactggcgtgaggaagtggccagggttttcatgagacgcactcgcgtcttattaaaagcccggtttaaagcgttaaccaggtggaagggatcgatgacaacgatggcgttcgggaagatctgcccaaccaatttgggataggtatagttcatatcggtgacgataattttcacattttctcgcgcggcttggtcataatgttggaagtacttttgaagctgatagatggttctaaagggcaacaggtcaatcaattcgtgggtttccgcgtccataaattcaaagctcatcgcgtcggtggcgctcttagtacttttaacttcgtccatgaggagaactttgggtaagtagtgccagttggtttgaaagtcgtgttcagcgcgcaagagctgccgaccaacgaatgaatccgaagtggacaattcattggcaatgtgtttgaggctcactggttccgttaacttctctaaacattgtttccgggttgtatttgaaatcgtgcagtgcttcggcactgcactcgtctgcgccaggaagttggtatgacaagccttacagtgaaagtttcgccgattgaggcataggataaccgtgctgcccaatgttttagcgaatctaatggtggtcttccgccaaccatagccaatgatctggtgatcattaataaccccacaattgcggcaggccttgggagaatagttcagtgatccatttaatctgattaccccatcatcacctattttgccattctcaatttttaagtgttcatcatctattcctaacaacattttcgtagtatcatttgacatagggcatttccttctttctctaaaatcttcgtggttgttggttttgatgaacggacaggaaatgtccgctttttttattctaatgaaaaacaaaaaatctgtcatcagtaatagataaaaatctattaccaacaacagatattgtagagccacaattaattgtccaatcctttttgtatctcgtcaattataacaattccccttgcgtcggtttttgtttggggtcaattgaattctcaggtttgtagaatcgtcgattatccaatccaaagacccgatcactgaattggccgggttcaatattcttagtggcgctttgaatcatcataatcgtcgcatctaactcatccaaatgatgcagaatttctgcctccaatatcttcggccgttccggtgaaccatactccagtaatccgtggtgcgacagaatcatatgccgcaataaaatcagatcctgggatttgggatcaattcccaatttatcggccgcttcaacgatctcggcatccataatgctgagatgccctaacagattccctgctaaggtgtactctgtggcaattgggccggacagctcaatggttttaccgagatcatgtaaaatggcccctgcgtacaataatggggcattaatgccctcatactgattcacgatcgaatgggccagtttgagaattgaaatggtatgaaaagctaaccctccagcaaaatcatggtgattggattttgcggctggaaaggtataaaacgcgttggcgtgcttggaaatcaagctgcggacgattcgattatagattgcgttggtaatctcaaagatggtttggtcaatgtattcttccatctgatcgcgagacatccccgcccgtttgacaaaattaaccggatcgtggggctcactttggttggccagccgcattgccagaatcttgatttgaggagaattcatgtagttctcccgcttacctttcaacagaacgactttgcctgaaacaaactgctctacatctgttggcgaggcatcccagtatttgcctgagatttggccggattgatcttgaaaaaccaacgacagaaatggcttaccatttttagccacccgcttggaggcgtcttttaataaaacatacatctcaaattcttcatccaacttgatatccatcaattgttttgccataaaatcgcctcctaaagcgttttaagatctaagacgagcttggaatcagtatttgcattgagattagcggtgaagtaaagcacttgggtcttctcactcacctgttgaagcattgtcagagctgccgcttttcgacgctggtcaaagttcacaaagccatcgtcaatgataattggcattggatattgactgctgaagccaaccgccatcgaaaagatcagtgccaaataaagctgttccaacgtcccggttgacaattcgttgattggaaaggagacatcatcttttcgaacgacagaaatttcttttttaaaaataatctccttgtaggcatcattcgtcaaagtggcgaaatattgctttgccaatgccagtgtctttggcagtcgacccttgctggcaatgtccaacactgattggatccactgggaactgagcttcaaagccaggtacttctgaacattctcaacaatttcagtttgttgattggccagctcctgccgcaaatcgtagtattggccattcttgattaaaccggcaatttcagtctgaacccgggtcatttcccggctcaaatcattcagttgatcttgtaaggactgcactttttcggtagcttcacgaacgtcggtgttcaaggcatcttggtcaatattttctggaattgaaattttggttgccttaatttgactttcaagcgtggccttttgatccagttgcttggccagttcagcctgaaaggcaacacctttttgaaatgcttcgtcgttttcaacatgtcgatccttcaagaaggtttgtttttgctgggtcagttcgaccagcttggcctttgcggcagccagtgtcttcttctcctgagtgagtactgcttgttggtgctgataatcggtagacaactgctgccaatgagcaacggtcttgccgatggtttcaatggcggtcgaatgctttgtttgatcaaatttcagccaatcactggcaaattgccattggtcaaggtaatcctggtacttggcctgctgttcattgagtgctgttttttgctgttgataactctgttgcaggcgctgaatttctcgaagcgaactttgcatcggcagccatctggcttcatcaattccttgcagtccaaattgctgttgaacagctgtcaactctgttcgaatttgctcaagtttctgatcgatctcaactggatcttcatgacttgggcttggctgggactttgaactccctttggcactataccatccccaaacggcagcagcgaccgccagaatatatccaatccatccaaacgaactagagcctaataagaaccctaataccaccagagcggctgccacaccataccagattagcccaccattaccatgaggctgttcggcagactgggttttctttcgagttacctccgcccgtttctcttggagattctgttgctcccgcagcagttcgttcacccgagaaaaggtctggtcatcaaatgcttggggcagattcccctgtgcatttttcgcaattgaggcagactgggtctggacttgtcgttgaacgtcctgcagctgagaatcgcctaattcgatggccaaagcaacctttctggcgtctggcagctcttggtataaccgttcgatcgtgtcgctatgagcctcatagaaagtttgaaccggttttctggatgactggcgggccgcttcatcgacagctgtttgagcctttttaacatccgcgctttcagctgtcagtgacatgtttaatttattaagctcattgagatcagcactaccgaattgtggcttcacctgagatgaatcgaccgtgttgagatcgtttagcctgttaaccagcggcaagaccgtctgcagacggcgtttgttatccaactgctgattagcagtttttaagtcagcctggaggtcccttgatttcacctggtcctgcttcaattgaacctgcagatcctggtagtgtgggaagtggtccttggcagcgccaacctgatcttcgagttttttatattccgcaatctgaatattaatcttttttgtacgaccgcggggcgcatacatttttgccgactgcttatccaaattggcctggaggtccatccaatcgcctgccccggcgacaccaagtgattggattcgcagccgtaattcgtctcgacctattttgtagaaggccgtctgatcaacgctgccaaagtaaaacaattggtcataagcggtccggtcaattggcgcaatgagctgctggtagtcatcagcggtaagctcagtatcgttatccaaatcgtagaattttaccgtcccgccgtattttaaaccagttcggacaaccttatagttatgttgatcagctgaaaaaataatttcaccgccatatggggcactgcccttgggctggtactgaccgtggatggaatgctttttatcagtgaatccaaacaggatccctttgataaacgcgatgatggtactcttgccggcttcgttaggaccataaatcatctgaagtggatttttgatatcaattttttgatcaatccagcggccaaaaccataaatgttgagttgtttgattatcacttggatttatcctcctcagtatcttcatgaacgacattttcctgaagaattgccccggcttgatcaaagatctcctgtttggattcttcagatccgacttcgtccttgatgaaagttggctgcttattaaagtccttgagaatttgatcaaaaacttcgtcattcaaggttgccgccttggcttgattaaaataatcctggtcaatgctgctatagaccagactttttacttgtggcgcttcaattgaagtaatccagcagttgagctgctgccacttgtcggcattaatgtcctgcaggtcatccaagagatcaccattattaattttggccagtaagtcggcatcgatcgccgtttggctggccaattggatccgaatgaaatgtaatttgtcgtagtgcaggtcggcaactttttccaaaattgattcaacaatctggtctgcagagatttcatcaagagaaatggcgacccggtcccaaacgatcggtgcggttggcacaaatttggttcgaaggtgctgatcgtcactttgaaccagcaaatagcccttctcacccgattcattaatatggcggccttgggtgttcccagaataattgatggtttgctgctcatttaacgactggcgcttatgaatgtgccctaatgcccaatagtcataacctttttcctcaagttcagacagtgtgaacggtgcgtaattggcctccggagaattgagtgaacttaagcttccgtgtaacatgccaatattccaattcacatcactaaccgccgttgggtagtcttgaatcatgggttgggtaatccactgcttatcaaagctaaaaccgctgacggccactactttcccatcattcaaggtatactgcttggtttcaacctggttgccaaaaaccagtgtattcgctgggtagccaaatgaagccggatccgccgtagagtaatcatggttgccaaagctgataaaggcttcaattccatgttcgttcaatcgattaagctgagcgatcaggaacgcgtcggcggcgacgcttcgttcttctcggtcaaataagtcaccggccagcaaaacaaagtccacttgctgcgcaatcgcgttatcgataattctttgaaaggaatcaaaagttgattgatgaactttctcccagagttcactgggtaaaacatgacttttgagccccaagaacgggctgtcaagatgtaaatctgctgtgtgaataaatttcatgatagatcccttcttcaacttatgtataaaggaaaggccgaggcaaaagtgcacacactttttgtctcggccccttttgtcccgtgcttgatctgcttatgatttgtacaagtcgctgattggttttgtcacggtctcattaatatctgataataactggctcagtgccttttctttggtcattaatgcggaaattaattgactctcgcgcattttcccagcaatcgcctggatgttctgaatctcgtcttgggttggttgaacgccctgcatttgtttttgctgaagattctgttgagcatcttgaaaatcattgaataatttgtagtcatccaaactcttcttgagtgcgtcataggcagctttgatttccgtaaattcatcggatgcaatcaattcggcttgaagctggttggttgttgcggtcattttttcattcattaaatagggtcccctaacaattttatttacttaattctaacacattactgaaatggcttcctgccaaagttagtgtttgaaccagcttttggcatcatcaattaaatctttggctttttgttcgatttgattaccatattggttcgttttcttttgaatggtatcccaaagattgtcattactgctttcaccttgaacaatggattgggcatccttggtgttaaagctggaattcttggtatatggcaacatggtctgcatttcgtttttgaacagtggcccgacaccagtcccactcaagttttccaaatggtgggcctgactggtattatcaaatccttcccaagtcgccaccaccaaatctggcgtatagccaatgatccatttatcttttgtggcgtcagcagagccggtattatcggcttcggtacttccggtcttacccgcaacctgatacccatacggcttggcgtcagcaccggttccattgttaaataccccaagcatcatgctggtcatctgtttggcaaccgaactggacataatttgacggccttcctgcttggccgtgttatcaaccaccactttacccgtagaatcaacaatcttgcgaatgtaaaatggtttaacaatctttccgccgttggcaaaggccgtataggctccggccatttgttgaggcgagacgccgccggacattccgcccaaagcgagcgccaggttcttgtccttcttggtgaccggaatgttaaagtctttgactgattgataaccgcggttgacgccaatctgattcagcagccaaaccgccggtgcgttcatactttgcgctaaggcttcatacatcggcacttttccttgataaacattgttatagttcttcggtgtgtaatgattggtgccataagatttcttcttatcaaccagctccgaatcgaacttgtagccggcttcaagtgccggcgtgtagacagccagcggtttcattgtcgatccaggctggcgggtaatctgagtggcccggttgtaaccccgaaagacgtgcttaccacgaccaccgacaacggcagtcacgccaccagtggtcggtgaaacgccaattgatgctgcttgaacttcggtgccatcagccgcgttggccggaaacatagcattgttattaaagttgttctgcatcgcctgctgctgagcctggttcaaattggtgtaaatccgatagccacggttcatgatctcagattccgtcatcccatacttactgatggcttcatcaatgacggcatcaaagtaatatggatacttgtaaccgtcttttcgaacataggtatcccgcagtgtgattggcgttttcttgtagtaatttgcttgcgcctgggtcagcttattattttcaaccatcagctgtaagacgacgtttcgtcgccacttggcggcctttggatgatcaatcgggttaaaggcacttggtgatgtcagcatccccgccaagacggaagagtcaggcacagataaattgacagcattttcaccaaaatattttctggcagcatcctgaaccccccaaacgccgttaccaaagtaggcattgttcaggtacatggtcaggatttcgttcttcgagtatacattttcgacttgaattgagaggaataattctttcagttttcgagtcatcgtctgctcttgagacaggtaagcattcttgaccagttgttgggtcaaggtacttccaccaccactaatataattgcgatgaagcagcttgttcttaacaagtaaaaacattgcccgggcgattcccttgaacgagaaaccgtattcatgataaaagttacggtcttcggtggatagcacggcctttggaatgtttgccgagacttgatttaaatgaacataagtccccttttgagcgtataattcgccggcttttttattattaacgtcaaaaatttcagttgtcttcgagagcgaggattccaagttctggacgtgggcggttttggcaaggaacaccaaataggtgctggtcacaagtgaaatactcagaaaaatgaccacaagccacttaaccaagtggaatcttcgacaaaatcggttgaaacgtttcaaaaaggtcccgaccgattttctaaatgagttggtagaattcttattcatgcgatactccttttgtgaatacctcaatattgtatcatatctgaaaagtggcgaaattcagggtggaaaaatttaacgaggatttaaaaaagagtgcccgccacaagctattgatcaatctgaaatttttcgaaataaaaagaccccctacctggttggtagagagccttggtttcaaatacaattagattacattgcgtccggtgctttgacgcccaataagttcaatgattctttgagaacaattgaaaccgccttgaccagtgacaaacgagctgccaattgatcgtcttccaccaagatctttgagtgcgcataatacttgttaaaggatttagcaagtctcaaggcatacttggcaatttctgatggctcaaagtccttgcaggcactcttaacgacgtctgggaagtccttcaaagcggtgaccgtttcccaagccgctggatcatcaagctgcttgttggcaccgtggagatcaatgtccccggcttttctcaaaatactttcggcacgggcgtgtgaatattgaacgtaaggaccggtttcgccttcaaagcgaagttggtcttcaagcacaaagtcaatgttgttagttcgctcattcttcaaatcaccgaagataattgcgccaaccccgacttctttggcaacttcatccttgttaggcaaatcagggttcttcgcttcgatttgcttcttggccaagtcaatcgcatcatccagcacttcatccaacaagatgatccggccggaacgagttgacagtttcttaccattaaccgtaatcagaccaaatggaatatgatgcaggttttcggcagatggtaagcccatttcaagtaaaacggccttcaactgctggaagtaataagtctgttcggcacccacaacgtataagttcatggctggtttgtaagttcgatcacggtaaatggcagtggcgatatcacgggtaatatacaatgtggcgccatcactcttcaagataagggctggattcaaattatatttatcgagcttaacgacttgagcaccctgggattctacgagcagacccttgtctttgagaatttgaattccttcgtccatcttatcgttatagaaggcttcaccgttgtaggtatcaaaagtcacgcctaatttttcgtagatcttgttaaatgattccagggaaactttacggaaccacttccacagaaagacttcttcttcattgccgtcttccagcttcttgaaagtttcacgggcttcatcatccaattcaggatgttctttatcttcattatggaacttaacgtaatacttcaccaggttgttgatgggatctttcttgacgtcttcttcgttaccccacttcttgtaggcaacgatcagcttaccaaattgggttccccagtcacctaaatggttatctttgattggatgatagccgtttttaaccaataacttggcaattgagttcccgatcacagttgaacgcaggtgtcccattgaaattggcttggcaatgttaggtgatgacatgtcgattgggacattgccacccttaccactgtcgttttgaccataggctgagccttcttccaaaacctcattcaaaatttcattactgaagtttcctttatccaagaagaagttcagataggcgccctttgcctcaaccttctcataagaggattgatcgattttctcaaccaattcttgcgcaatggcgtttggtgccttatggaaaactttagccaatgagaatgctggaaatgccaaatcacccattgctaaggtcttaggcttttcgagcttttcataaacctcagctgacgacaattcgtcatttaaaacacttaaaattgagttcgtaacctgtgctttgtagtccattaatgttccctccatctataaatatacaaaaaaactcttacaaaaataattgtaagagacgagtaaacccgcggtaccactctatttgataaaaatatccgctcaaagtattaaattgatattctaaaaagcgcgcttcgctgactcaatttttcggctcccaccatcccgaaatcgctgacaattcagtgaccagctactgttcttttattgttgaatatttataacgttcaatgtgtataataacttgttgacccggtatatgtcaacatttatcaccacaccggagtgctgagacaaccaacactaagcgggtaacgggaatcggacccgcgacgcaagcttgggaagcttgtgttttaccactaaactatacccgcataacaaaaacaattatatcattttaaattatctttgtcataaagatttgaaatctctaaagaattttggaaaagattgctttttcgtcccaaaatacagatacttaacttaagaggtgatttgaatgtggatcatattgaactacagctgttgggcaattctattcgtcaattttatctggggattgacccgatccatgaaaaagcacgtcatcgattcgatgatgatcgcccgcgtcttctactggctcatcatgattagccaagtcgtcatttcacttcgttcatttcaccgtcatccactgctggttatcattggtgcagtggtgacgctggcagtgattgcattaaccgaaaccgcttatggccgaaagcaagacgtcaactacagccccaaactgctgtggttattgatgctcgccacgctaatcgccgtatgcctacaaactttggtcaactattaagttagttggctatttattttgcccgatttgcctcggccaactcaatacacttatcagccaaaaccgtctgggcgtcaatcactggataatcgtgattacccgcccgctgctgggcaactgacagttcagtacagcctaaaataacgatgtcacattttaacgattcaaccatttgagaaagaatcaggtgatacaatccctcatcgacctcgtttttggccttgatatcatcatagattaaggtcatcgtctgatcagcaatcttgtcggttggcttaactaattcatagccggcattaataatttcatgatcataaatttgatcatgtaaggtgccttctgtggcgattaaaccgacccgtttggcattcggcgcgtaatccttaatggctgcaacggtttcctttggcatatgcaagatcggcacatccgtgagtttctggagctcatcatagaagtaatgagcagtattgcaaggaatcgcaaaaaaatcgggatgtagggcactctgctgcttgacgtcttctgccagcggaatcaatgggttgggctttgagtgatccaaaatgtagtctgtccgatcgggaacggtcgaatgattgaccaaaatatagttcagatagtcctgatccttggttgcctgagtccgctcatttaaaatatgaatgaaggtttcagttgcttcggtgcccataccaccaataattgtaaagaaatttttcaactaaatcagtcccttatttttcgacaaagtatgtcttaaagctcttggcataattgtgcatcatccacttatataatgcaaaacgtttgatatttttgtccttggcgtaccagaaagtgtcgccataacggccttcgttgatcatttccatggcttgctttttggcagcattgtctttggcgtacttttcaaagatctttggcgtgacaccaagccacaggaaatattggcgtgggtccttgttggcatacaaggtcgactggtccttcagtgaatcgaagacgtaatcttgaatcacccaatcagctaaatgatggccgttcaaggttacgaagaaactgctccggccagtccgcaaattgatttcaaacaatttgtaagaattgtctcggtggtcaaatttcaaatcaaaattggcataaccgtggaaattaattttttcgaggaacgcctgaactttgttgtagatttcctgattaaattcaggaatgattgcgacataattcccaatcgctgccggcgctggatcttccagtagtggatgacccagacacatcaatttaacttgatgattcttatcgacatagacgtttaaagtgcgcatattactgtcgtcaccagggatgaagtcttggagaatgaagtcggatgtataaccgttatcataactcttggcaacaatctcctgaaattctgcttcactcttaatgataaacgcctttttgcgtccttcaaagtgaatatcaagccactcaacactattggccggcttcagcgcaaccggatagccaaatggctgttcaatcggctcgcccgaagcatacatggctttggaaatgatcttcgttttcgggtatggcaggtcgtattgatcacacatcttgtagaagttttccttgtcgttgagcttcttaagtaaatcatagtcaatgtatggacaaatgaagacatcttctaattctgctttatgtttggcaatgagttccgcatagccatccccacaaccaattaaaatcaccggttcttgatgattggcataacgtttcttaagctgcttcatcgtatcaatccagactggatcctcactaaaaccgggaatcagttccaaatcaacaattttggtgaagcgcgtcggtgccaactgggtttgggcaaatgctttgaccggcttgccataaatttcgtataaacttctggccatcccgtaggcgttaaagtcactgcctaacagaacgggcgtaaaatcaagctgcttatttttcattactagagtcctttcacaagatttttaacaattgccgcatcgccttcatacggaacgtttttgccattaatcttttgatattgatcatgacctttaccggcaaccactaccaagtcacccttctgactttcggaaacggccttggtaatggcttgcttgcggtcggggatgtaggttgtagccacttttgaggtatcgatatgagcagcaatttctttggcgatttgttgcggatcctcggttgccgggtcatcggtcgttaaataagcctgatcggcagcctcgttgattgctttgccaaggccctcgcgacgatcaattcccttatcacccgtgctgccggtgataaccgtcactttaccgttaggagcctgttttttcaagaaatcgagaacggaatgtaaactgccatagttgtgggcatagtcaacgtaaaccgttccgtgatcatgggtctgataaatttccattcgcccgggaaccgtggtattggccagaccataagcgatctcggtcggtttggcccccatcaaggcgctggtaatcgcagcggcaactgcattgccttcgttataatctccaggaattccaatccggtatacaccgtcaatgttcaattgcttcgccttggcggttcgggcagtcacttggatttgattttccgtcagcgaatcctttaacgatcgatactcgacatctactggaaattcagtttcctgattctgcccagcccgtccataaataaagatattttcaggttgggtggttgctttagccgcgtaaaagatgtcggttaaatgtgtcccgtcagcgttaagcacacaaacgtcggaattaaccaacaactgttctttgcagtgcaaatagtcggcaaaagttgggtgctcgttgcgaccaatatggtcaggtgaaatgttgagaaaaaccccaacatcgtaatgcagaccataaacccgattcttcttgtaggcttgagatgaaacttccatcactaaatgactcatgccattatcagcggcttttcgcatcatggtaaacaaatccaacgattcaggagtcgttaaatttgatttaacaacatcttcgggctttaatccgacaaccgtattgatggttgaggataaagcaacctttcgctgataagtttgatccagaattgctttggtaaagtaagcagatgtcgttttcccctttgtcccagtgtaggcaatcgttggcaattgatcttgtggaaacccaaaaaatgccgcacttacgagcgacattgctttttggatattcttaacaataatgcctggaatgccggcattttggtatgtcttttcggacatgtacgcggtggcgccattctgtctggcatcatccagatacgcagatttgaagttccccttacagaagaacaaacagttgtcagtgaccgatttagagttatatgaaatctggtcaaagggatgacttgagctgctcaattgactttcaagcaataaattatgttctttgagtaaaactaaaacctcagcaacagtaatttgtgccaatatgtgcaccttccattctttgcatatttctaaatctgggtacgatgaaccaagctgaccgtgttctcagttgtatcttctgggaagtaaacttgataccagaggataaaggtatagatggtgaaaatcttctgcatgttggacttaccttcagcatgctccttcaacagacgatccaattcgttggtattgaagaactttttacctgtatcagaatggaaagcattcacaattcgttcgtgatacttaggatcattaatccagctggcaattggagatgggaatccgagcttctctttaagagcagtcttcttaggcatttcccgttctgctgaagttctcaacgcaattttggtctcatccggtgtaattcgtgtcttgactggcatggtttcagcaaatttggcaacttccttatcaacgaatggcacccgaacttccaatgaattacacatactcatccggtctgccttgtggagaatgtcgaatggcagccaagtgttaatatcaaagtactccatttgggtcatttcgtctttgcccttgacatcatcaaagatgtgcttggtgtaggcgcctgaatctgtgttaattgaaggatcttttaacacgcgattgcggtcgtcgtaattaaagacgtagttcacacgatagtaccgttcactcaacggctgggcaccacgaaccaagaagcgtttaccgtggaaacgaggcagccgtttggcaactgcagccagccccttacgaaccggctttggcacatacttctgataacaatcgaatgggatagcttccagataggtgttgtagccaccaaagaattcgtcggccccttcaccggacaaagcaaccttgacgtgcttggaagtgtcctttgataaataatacagctgaatggccgctggattagaaagcggctcatccatgtagtacatcatagttggcaggaaattgaagtaatcatcgccattcatgtagattggcgtattcttttggttaatggtcttggcaaactcagtcgaccaagccaactcactatatttggagtggtggaaaccaatcgagaaggactggatcggctttaatttggcagcttcgtttaatacgtagcttgaatcaattccactggacagaaaactaccaacttcgacatcggcaatcatgtgggccttaacagaatcatcaatcaacttaccaattttgtcggcgtctccttcaatggtttggctattgtcaatatgatcgtagttgaatttgtagtaacgatgggtttcagttttgccgtttttatgaaggaaatattggcctggcaaaagtttgtagacgtgcttgaacatggtttctctggaaggaataaattcaaagctcaagtgaattggcagtaagcgcaaattcagttcctttttgaagttgggatgctccagaaatgctttgatttcagatccccaaaggaacgtatcaccatcatcgtaatagtacagtggcttaattccgaagtgatcccgggcaccgaagacctcattgttcttcttatcataaatcacaaatgcaaacatgccgcgaagcttgtctaataaggctgggccccattcttcgtagccgtataccaaaacttctgaatcaacatcagtcttgaaaacatatcccaaatcgcgaagttcttcacgaatttctttataattgtaaatttcaccattaaaagtcagtactttagtttggtcagcgttgaacattggctgacggccatgtgctaaatcaatgattgaaagtcgacgaaatcccattgaaacattgtcgtcggagaaataagcttcgtcatcggggccacgatgcttgatccgatcagccatgctgttaatggtaccttctggaacatctttttggttaacgtaaccaacaaatccgcacatattttatacccctttatcaaatcttcttggttagtctgaaattaataacgttttatattttatcagattacatagattgctaccagtagtataaacctttcttaaagaacggcttgcctaaaggaaattaaaacactttcgaatttcattttaccattcttttaagttatactttagatagagtatcaaattgtttttgaagggagagatacaaatggacgagatcgtatttttcaacccgggagattctatcggcaacttccatgatcacaatgaagctgtcaaaaccgctcaaatttacaaggaaaaagaacacaacaaaaaggttttagttgtgcatggtgtcgacaacaagaacttcgatatttttatggccgacgacatcattagtcacgacaatgaaagaaacgcgattcaaaagccttataagatttctgatcggatttagtaattatgtaaatttcatcagaaaaagggattcaaaattgcttccaacaattttgaatcccttttagtttatagataaatttatctttagcctttagtattaacaaccaaaactttcgttgttgcgtttcgaacaacaaaggccgtggtagaaccaatcaacagtcggttaatcgcatcgacacctgacttaccaatcacaatcaaatctacatcgtgctcatccgggtaaacgtgcgcgataatgttctttgggttgccgatatcaatggctgtttcatatttaacaccttgtgaatcagcatacttcttggcttcgtcaataatgttctcggcgatcttgtgctggtcgtcatacatgcttggcggcatgccggctgcccctgcaccatagtagaagttggtgttgttaataaccgttaccaactggagctttgaatcaaattgtttggccaacttgcaagcttcttccagtgcctgttgagaatttttacttccatcaagtggtaccaaaatgttgtcatacataaatatcacccttctttcttgtaagcggacacattactgtctacaccactataatgctacgtttatatccgaaaagcaattaataagtctgaagatatatttttaatcacaagcaggtacaattttccggtatgaccgctttccaattcagtcaatggactaattaatgttataatttaaatgttatcaaattatggaggaagtggttttcatgaggggcaaaagattagttgtgggcatattgagcgggatttttgtgattgctggcagtgtgtcgaccagtgcaaaatccaacacgtacacgatgccaaaagtttcactatcgaaaacagttgtggcaaatattgctttaaaaccacaaagctcatcccaactgacggattatgtctatgacaccgtcgatccaagttcaccaaattatcatcaatacttaacgccgggcgaatttgccagtcaatttggccgcccgacgacagacatcaacgattttaaaagttacttagggaaatatcatctcaaggcatccgtctatccgggaaacttggccatcaaagtcgttggcactcggaagaatttgattcgggcatttaacgccaaacaagtgaaggtcagtaaaaaagattatcgaaccaaagttaaattaccggcaaagctttcggcccaaacagtcagtgtcatcggtgtgtacgcaacgaaaccaaaaagtaagaagacaagtcttgcagtaacaccatctctcccacaaaacccgactcctccaaataccgatttgagtaaaaccagttttgctaaaaagtatggtgctttaaaatttgctgatcattatcaggttagtgatttatataaacaaggtttgaccggtcaaggacagcgaattggcattattgccatggacgactttaatgccaaagacgtgctcaaatattggcagcaaaccggtgtcaacgccgaccccagccggattaataaaatttattcaattgacggtgccaagactggtcacttgatcctgtcgatgggattgaacccagctcaaattgaatcaacgctggatgttaaccagcctggggccgtcgcacccgatgccaaaatcgatgcttatatcggcctatcattaaaaaacgtcacttcaacgacatcatcttattacaccgcctttatgcaggccgtttcggatgatcgtgataaacaaatttcaaccagcttttcacccaacacggagcttgccagtcaatgggaacaaggtgccagtgcctctttgggtgagtacaacgacgcctttaatctgctgttggaacaagcagctgttcagggcatctcagtctttcgggcaagtggcgactatggtccgcgtgaattggcccttaaacaattcaaccacgttttctcaacttcgccatatcaagtcattaccggcggcaccacattaccctatactagaattaccgatggccgcttaatcaccattgataaggaacgggcttggggcgacacatacagcaatccacaaaccaaaccggcgaattatggcggcagcggcggcggattttcaattttgaacccgactccccgctaccagcaaggattttccggcgttaacaccttccgggcaatcgatctgctcaaatataagcgcggtggtttcttagtgaataaagatccgcaaattatcattggcaaggggtctggtcgaaacgttcccgatgtttcagccaatgccgacagttacactggttacgcgacctacgtctccgggcaagacctcgcctatgccaaggatggcaaaacggtcatcagcgttccagtcaaacaatggacagtcaacggcggcaccagctttgtatcgccacaaatggctggtgccaacgcggtgatgaacagcgggacaacttcgccaatcggcttttggaacccacaaatctatcaatttgcggtgcaagctgattcaccctttactgtgcttgacgatgctgacaacaataataacctgtattacaccggccaacctggtaaactttacaatcaagccactggactaggaaccgtcaacttcgccaaattgtataccaagttctcgtcagagggtgcccattaagacaatcgttgttttaactcgagattcgccaacgaaacactcaagctttaacatgttgataacttaaaattagtcggccaatcctgcttatggataatcggccgactaatttttaaaaaaaatggatcaaaaaagaggttgagatcgctatcgtgcaatagtgatctcaacctcttaactttatatgatgccctcggcaggattcgaacctgtacttgattgctcaaacagcgacctgaacgctgcgcgtctgccagttccgccacgagggcaacaacatgttttattttacactaaaagtagtaacttgaaaagaagttttgtcgttttgttttgaaaaccagatatcgactggaacttggatcatgtttcatcatcaggtaaccaatcaaagccatgaggaaagcccccgccaaatcggcgatcaggtcagtcatcgtgtccatcaaggctgctcggccgagcaacaacttgccagcttcttcgtaccgttgcaggttcaaaccacccagcccatcagcggtaaactcatacatttcccagaaaacaccacaagtcgttccaaacgtaaaggcaaacagactcatcaaaaatggtttgtgggttgcattatctctggcactcatcaatccttgaaaaattgaaaaccccagtccagccaacatcattgcggaaaaaacgtgttcatacttatcccaaaacggtacactgtaaaattgcaatccggatccaaggaaaatggacatgtataggaaaatatagaagaaaaccaattcaatctgtggaaaataaaaccggcccaacttctcgattaaaaatggcaagctggcaatgaggatcccaataaagacctccaccaagagcaacgtctgcccgtgaaattttggttgtcctttcattaaccaataaccatagtaaccaagataagcagccattgagaccaccgtaatccaaaataaccaagtactaaatctaagtttaccaattttcatatgtaacaatccccttttatgtcaaattaattgtccgcaattaaattgactccctgtgttaagtcttgcttttaaatataaatacattacaataataacataaagtatttaaattgattcgactagtgctgtccgtgtttcacggcagtatgtgcaaaaataataggagttgaaattatgcctcaaacccaaccaattcgcttggacagccaattgtgtttccaagtctactcagcgaacaaaaaatttaatcatttttatcagcaggcactgaagccttttgatttaacttacccacagtatattgcgatgctgactctgtggcaatatgcaccgctctcagtgaagcaattgggcgaatacctccacctggacagcggcacgttaaccccattactcaagcggctggaaaatcatggctggatcacccgctcccgttgcgaagcagacgagcgaaccgttgtcatccagttaaccgataaagccaaagagcaacaggacaatgtcttcagtcgtgtgaacagctgctttgatgttttgggattaaccccagctgaaaaagaaacttgttctcagacgatggcgaccattgaacaaaagcttgatttgtacaatcaaacacagatctaaacgctctgaccaaaatgttaagattttggtgcagagtataatctaatcataaatccaatttaaaatcgaggctgggacaaaatgaaagattttgtcccagcctcgatttgtgtttgaatgttacctagtataattgtgggccaataagcagcttccgaccgtataagggggattatcgaaatatccaactggaattcgggtaatccccttatagagccaaaccacttattggttcacgctcactttttgttcatgccaaccaatcaaccactgactggccaacttgattaaatttttggatcgtttccattcggttcaaggatccagcagtcaacatggcaatgtcaacagaatggttgttatatacaatttgagcgacatcatggtcaatcaaattgccctcaccagtcttattgtatacagcaacattctcgcctgattcatcaaaattacctggtagtttgtatcggaactgctgattggcgaaccagctctggacttcggaaccattatgaagtgcttgctgaagcagccgcaaactttcagcagcactggtatagttatttttgccactggcaagtgcccgaccgtccatcagataacgttccagcccggtctcgtggaaatcatgggtttgaagataatgctgaatatgattcattcccatcaaggagatcaccacattagtagccgaattatcggacacactaatcatcaacgccaacaagtcccgaagcttccatggccgaacagacatcaattgtaagattccggcaccgcctaccaactcatccgtcgaaacatcaacggattgatccagatcaacgttgctgtccaaaacatcgtttaagatggccaatttgatcaaagaagccgatgggaaggcctcgtggctatcatggtccaccaaggtctgaccgttgctttgaattaacaagccatacttaaacgaactgtcagccatcacccgttcaattgtttcagaaagctcactcatcgccaatatctcctaaagccggcgaactcggccgcaaattttggttcagtcagttctgcaatatcgactttggcgcctggcgttcttgattcaatcatctttccattaccaatgtacatgccaacgtgatgcacgtagcccttgccgtgatcatacgcgaaaaataccaagtcacccggtaggatttcttccggtgctaaaggtaaaccgttttcttgttgatcgtcagcgtcccggggaatatcaaatccaagtacccgatgaagcgtgtacgcaaatccagagcagtcaaaaccataggaactggttccgccccagagataacgctcgcctaaaaattggcgtcccatctcaaccatcgtttcaccagcattgctaccaacgaatggcagtactgctgctgatttgtcaatgaaaccctttccaagcggggtcacgacggcaatgtagtcaccactggtgcctgtttgtggcagcacagttcccaagctgatttcgaggaccggctttttgttttcatcatacaaattggctgtccgaacagcaattctcacaattgaggtaaccggtggataactaatctgctgatcgcttaataatttacttggcacccaaccaggatagccccttgaatcagaatcatctcgttgactgggaatatagactttggcccagtcaccgtcgaaatgatcaataatgacttcatcgttaaacaaagcctgcgtttctaataagtcatcatcggaaagcgcaactgattgctcatcactcatttgttcaacccattttttaccatcgccgtctaaggctggttgatcaacttttcttggtgattctttagacttccaaatagttgccactggaactttgactcgtcttgtttccatctgggcacctccattcgttaaattttagtatacatatattatacctcattagccaccaactacctgccagatagcataaaaagcattgctggcttgttcaccctactcaaaaaaggccggaacatgaggaatccttatgtccgagcctcttgggttacttaaatcctaatcccggtaaatctggaaaagagatttcgtttttttgattgatgatcccaccggcaattgggttgctggagaacatcatcgatgcgtccaaatctacatactgaatatttcgtttggcagcggccaagtgagccgcagcagtaacggaaaccgacgattcaatcatactacccaccatgcagggaattccggcagcctcggcaagggtattgattttaaccgcattatcaatcccgcccgccttcatcaacttaaggttgataatatcacaaccacgcatactaatgatgcgagcggcatcttcaattgaaaagatgctctcatcagccataatcatcgtcgtggtgttggcggtcacgtaagccagaccatcaaagtcagtggctttaaccggctgttcaaccagttgaacgttcagattcagttcccgcatccgattaataacggccacagcctgttttggatgccagccctggttggcatccaaacgaatttgaatggctggcccaactgcttttctgatggccacaattttatcgaggtcggcttcttcagaatcatcccccaccttgattttcaaagtggtaaatcctttggtaatcaagtcttgagcttgggtgatcatatcctcaatcgtcccgacactgacagtataatcggtcgtgatgtgatccgagtggccacccaacagttgatatagtggcaccccatacgattgagccagtaaatcgttaacggcaatattcaaagcagccttcggactcgaattatggaccattgactgatcgatagtcgccttaatatccgctgagtcaaacaatggtttgccaatcaatttcgggccaatcacatcgttaacggcactttcaatgcttgggagggtatctccggtaatcaccggcgtcggtgctgcctcgccataaccgactttaccatcactggcagttattttaacaatcagcgtctgggcagtggtgacagttcttaatgcagttttgaacggccgtttgagtggcacagcagcttcctggacatcaatctttttaatcacgggttccaataagtgtcactcctcattaattatttaacgtaagactctttgaaattgtagttggcaccagcagtgttgtaaacaattcccttaacttttgaattaaccatccatttttcaccagattggtaaagtggaatgattgcttgatctttcaaggccaaattctgagccttaaccatgtcatcccaacgagcgttggcattgctgccatcgtcagcgttgctggctttgattaacgaatcatactctgaattcttccaaccggaaatgttgcttgggttattggaagtcaaaatgttcaagaatgtgattggatcggagaagtcggcaaaccaattggcaacggtcacagtaaattgaccatcagcttgtcgagataaaattgaacgaccaggaatgttgttcaaagtaaccgttaagccaggtaacttttgtaaggcactttgcagatactcactcaattgcttttggtcactgccatcagagttcaacaaagtaaagtgtaatgacgaacgaccaacttcttgaaggccttccttaaagagctgtttagccttggttgggttataagtcattgatgcgggagcggttgtgtctttcgtaaagtcagttccgttcttcggtgaaacggccaatccctctgaaacaaagctattgttatcgattgcgccgccacccatgactttgttggctaatgtctttcgattaatgatcattgacattgcttggcgaattttcaggtttttgaagaccttgttcttttggttaacagcaatgtagtagttggaagactgctttcgtgaaatcatatctttcttgttacccatttgtttggcctgggtagctgacagttgcgacatatcaagtttaccttggttgtaaaggttcaacgacgttgaagaatctggttggacactaaacttgatgtcatcaagcttaacagccttcttgtcccaataatcggtgttcttcttcaaagtccacttgttattggttccagtccagccagtcagcgtaaacggtccgttataaacttgggtcttggccgaagtgccgtaatcgttgccgtatttattgactgccttggcatcttgtgggaagaagacaggaaagcccatcagcaaattaaagtatgggattcgctgttccaaggtcacagtcagtttataattaccacctgctttaattcccaatgaagaaactttggcttttttgttttgaatcttgtcagcgttcttaattcctgagaacaggtaaccatactgtgaagccgtcttaggatttaaggttcgctgccatgaataaacgaagtctttggcagtcaccggatcgccattactccatttggcacctttacgcaagttgtaagtgtaagtcttaccatcctttgaaaccgtccatgacttggcgattcccggttcaactttactattcttgcctagacgaaccaacccttcatcgacgttgtttaaaacgttgaaagttccaacagccgtggtcttcgatggatcaacagtcgtcagttcagaatcggttgaagtcttaatcgtcttgttagcttgaccagacttttgaccacaacctgccagaattaatgcaatgcttgctacacctgcgagtgcagccactcctcgagataaatgcatgatataatcctcctctaatatgtaagacgcgtaacaaactcatcttggttctaatttagcataaaagtgtcaaaaaaacaggccttttctaatattgagttcagaaagcctgttagaatatgcgattttgctgtgaattttacttagtaattgcgattgccatcttacgagacaaataaatcggctcaaatttggtttttggcagccagtattgaccgtcaatcggatcactcacgtggacctggtggtcatcgatcccgtccaacagaaccgcgtgattattagccggaacctgaccaaatggatacgaatcccactcaggttgttcaaaatgaacggtcacagaggttaacaccggctccccttttgccacaaagtcatacaaccactggggatctgccccactcagttcttgcagattaccataacgatttccccaccacatcaggggtcgggtaaagattgcctcaaacttgccgggccgattggtgaaaggtgaaccaccaaagccgtggtaaggattgctatctggtgaaattggcatctgaaggagaaattggccataattcaggtctaaagctcggccctgataatggagcccctccagcaagctggctgcctcacagccgttaatggcaccccaagcaagttggcgaatgttttcagcacctaataaaatcttcgcactcatttaaccaccccaagctgtgaaaagacctgctcaaccatatcggtataatcaggttgctgagaaatcaacttcttgcatgcatcaactaaatttaaccgaagccgtccctttcgatcaacgactgattcggcatggaccattgaacttaagatcgactcatcgacaacggctgccgtagctctgaagaataaatcaatttggttatcgttaaaccgagtaacagtatcaaactcgctggtttcgaaatggtccacctgattggcggttgaaaatgccaaaacgatttctccgctgccgttgccaatgtagccaccggaacgattaatcccaaccgttgcccgcttagccattcgtttgagttggcgggcattcaatggcgcatcggtggccaggatcgtgataatggaccccttttcttctttttgcttatccttggccaacattttggccaagggggctccaataggcatcccattgacaataaagtcggttaaataaccatagttggtcatgacgagtgcaccaacagtgtattggtgcttcttatcaacggtcacaatccgcgaggaagagccaataccgcccttgaggtcatagcacatcatcccccggccactaccgacggcaccttcttcaaagtcatcgttaacagctgccaaagcatcggacacattctgttcagtaatcgccattttgcggatattggacacgtcgccatcgttacactcagcaacaatcggattaactgtactggtggtatccccaatttcgggattagcagccagcatttgtttggtgagggcatttagggccgtgcccacgccaaaggtattcgtcatcacaatcggagtttcaatggttcccaattcatcaatttggacgaggccgacgcttttaccgaagccgttaagcacacaagaggcagctggtaccttgtgccggaaaaggttgccggtatggggcagaattgcggtcacaccactatgaacgtcaccatcatcaatagtcacctgcccgaccttgacgccgccaacatctgtaatcagatttcgccgacccttgacgccatccgaaagatcattcatcaattcaaccgataatcccatgattaacacctctcacaattaattacacggcaaaaatcatcgcaatcattccgccgactgcgattaaattattcaaaaaatggaggccaattgataccttcaaatttttagttgttacatacaaataggccaaaatacaacccaagatcgcatacgtcaaaaaactgatgatattaaaatgggaaagatcaggatccatatgcggcagggcaaaagccatcccactgacaataatcggtgcccatttttcggtcgaccgaaagaacgcagtcatcaaatatccccgaaaaatggtttcctcaagaatcggcgaacagaagattgccgtaaatcccatcaaaatcagggtaagatgattgctggacaacaatgattgaatttcctgattgttgtccgtttgagtgacgtggtagaccagtttattaaggtttcccaataagaactcaattaccaaaaaggcaatccaagcaatgacaattgttttgacattttgccaggtcatttttttgacttcgtagcggccatacttccggtaggcatactgtgccagccaaatggcgattagaaagcccaacaaatacaaggctccaacagcgtaattggcaactgctgacagcttgccttggacaatgaacatcagtggcagctgaactgagccgaccaaaataatcagcccaaaaaagatcattaatcgttcaaagtagtcaccaaaagttaactttctttgctcttccatgcagcgtctccttaactattaaaagctttgttcaaagctgtaaaatcaacggttccaagtccggtcgcctggttataaatcttccccggttgtccggtatagtacaagttggtgttatttgtccgactgtccaacggtttgaacggcgaagttgatcgtttggcaaatcgatagatctgtggattccaaaagcccaagcggccattggtagtgaaatcagacattaaaacactggctgcggccatctgtggggcgacgacactggtcccaccggtaatcagccattgccccttggaatttcgattgttcttcggcgtaatgaacatgctgtaaccggtattggggtcggcattcgctgaaatgtcgggcaggtttctgccgctggatttgccgctaagattaatcggctttttcaacaattccggccgaccatatttaaatttccacagattagtcgcatcatacgtcccgacaccactgatccctttttgataggcgggtctggcattatatttactaaaaccgccgccacctccggcaaagaagctttgaagcatgtccaaagttccgaaaaatcgttggtgtttatagttggggtataaaaagtcagccccccaggtgcgttcctggtgaatggtgacttttttcttattgacagtataggttttcggcagtgtcgtgccgccgactgcggtcacatatggagaattagacggcgtatcaacggacaatcctgacgttaacccggtggtaatcccatcataggcaccattatcaccagtcgcggtgaagacactcattccttgggcagctgcctgctcaaataataagttcatgatttgattatattttttcggggtaatcccctgtttcatttcataggccacttgggcttcactttggccccaactgagtgacaaactatcggccacgttttgaccaactgcggcagcaattgaattcaccattcccaaaatgtttggacgggcaatgtaggtccgaatgttgctgtccggtgcgattgcgccggcctgttcaacatcgatagtcgtttcatcatagccatcccaggtacccttaaagccgttagtccgataaacgcttagtcgattagatttcacattgatgccctcatcatcccagtagcggtacacatcattaggatggaagttggcaaatgaaatgatcccaatggttttactgcggccagtcgacccattatcgtatagggactgcagattgtagcgacggacaaatcgcgtcggcgaatactttttggtggttgtcgtcccgctggcagttctggtatgcagcgatgagggctgaaatttggttttgtatgaggaaaacggtgagtaatttgataacccaaagacggtataaacgaccttggaaagtttcttgggtagttgaggatttcggctggccttttgatatttgacctcaccgttatttacgttcaccaggttaactttaaacgccttctcgacgtttttggttgatcccttgaccaccataatcaaattacctttgtaagtctgagccctcaaatgatggtgtctgagatatgtctgcaaagctttaatctgctttgggctctgactgaatcgtttggcaaaagtacttggggaaacaaatttgcgataagtcggcgaactcggcgtcactgtgttgtaaacaaattggtgaagcgccgactgactttttggccgcagcacaatatcaaccaattgctgtttggaatcagcgacgttggtcgtcttggcagctgcctgtccgctggttgccgcaaagccaccaatggcaagcaagatcaatcctgcggttatgaaaatcctgtggagccaatccttgttcatacaatccccttcaaacaatcttatttgtcacgactattgtcgtctgcttctcgttgggcttttctttcatcgcgttggcgaacaatcatcaccaccaacggcgtcaaaatcaggcgaatgacaataattgcaatcagccaaatcagcgcgaacgacagaactgacaaatgccagaactttgtgatgaaaaacgccactgctaacactaatacgacggcgccgacgattaagaataatttagactttttcaaatgaattctcctgtaaaatttcttatttcatactatcatactttgccaatggagttcacgtttgaattgggaaagttagagtttgtcttcgggtatttaaagtcgatataataaatacatcatggaaataagatagttgaaaggagaaaaatcatgctcaaagaatttaaggcttttattgccagaggaaatgtcatcgacctggctgtcggggtgattattggtggcgcctttactggaattgtcacctccctcacaaataatttgatcaacccgttaattgggatcttcttaggaaaaattgacttgtcaaacctgattttcaaagtcggtgatgcgacttttcgttacggggcctttatcaattcactgatcaattttctaattgttgcctttgtcgtttttatcttaatcaaactcattaacaaggtcctcaagcgtcagccgacaaagcctgcaatcgataacaaagaagtactactttccgagatccgggatctgttaaaaaataaacaatgaaccgtcaatgacgcaccgcagaccattccaaaacggtaattgattgcgattgcatgatgtctgggctagaattaaaagtgtgaaggtttaatttatttcccaaaaattgagaagaggttttgttatgagaacgtttgctattagggcccgcgatggggtcatggaattaaattattcagaagattccaacaaaccgccgtttcgaaagtttatgatcacatataaccccaaattttcaattggcgataatcttgaaaatatcaaagcagcgctgaccggcctgccgatcgacgccgccattatcgaaaattcgttaaactatgagttttcagatacgattattggcattaatcaccaaaagattgatatcggattggcaattgccaacatgatgaatattccggttgttaatctgcaaaagatcaaagaagttgggctgaaaaaagccgttgccgataaggaagaataccttaagtggcatctggattactatggtgaatatgccggtaaacggaactacggccaagaagccatgctgacaatcgggaacggttactttggtctccggggggcctacgttgagtcccacgctgatcaggataattacccgggtatgtacgttgccggtgtttacaaccaattgacgactaagattaatgaccgcgacgttgtgaacgaggatttggtgaacttaccgaatgcccaatacattagtttcggtgttgaccatcaactgccatttaccattaagaaagccgatattcaagatatttaccgaagcttggatctgaagaccggtactttgacaaccaccctgcacgttcagctttcaaccggccatatcatccaagtccgggctacgaaagttgccaacatggatcagtggcaccgttacgcaatcaaatatgaattaaagcccatcaatttctccggcagtttacaaatctatgccggcattgatggcaacgttattaacggcaacgtggaacgttatcaagactttgatcagcaccacattgatgtcatcggcatgtcagctcatgacaatcaagtctcgatgaccggtcaaaccaagacctcacacgttcaatttgtgatcaactccaaactcagcagtccagatttcgataccaaaaaattgatcgataccacgactgaggaaggtaaagtccaacaggctttgagcattaacgttgagcccggcaaggaatacgaattcaaaaagaatgtcaccgtctttacttcccaagacgaaaataaccatttggaagccgatgcacaaaaagaacttgatgactcctcatttgaagatacgttaagcgatagtgaaaaattctggagcaatgtttggcaacactccgacattattatcgataatgatcttaccagccaaaagttgaccagggtcaatattttccacatgttagttaccagtgctgctttgtcgtccggtaaattggatgcatccgttggtgctcgtgggctgcatggtgaagcttaccgtggacacattttttgggatgtcacgtttgatttgccattctatgcaattcattaccctgcgattgccaaacagtgcctactttaccgttacaaccggttagctgaggcgcgaaagtatgctgcctcagaggacaaacaaggtgcaatgtacccttggcagtcagggatgtatggcgatgagcaatcacaatttgttcacttgaatccggttagcggcaaatgggatcccgataacagccgcctacaacggcacgtttccatttcagttgcctatgacattatcaattatgtccacatcacgggcgataaagaattcatggatcaatacggattggaaatgctgctgtcgatttccaagttctgggtcagcatgaccgactacgatcaatcaaccgaccgttatgacatccatcatgtcatggggcctgacgaatttcacgaagagtaccctaactccaacgatcatggcttaaccaataatgcctatacgaatatcatggtttcctggctgtttgacaaggtcaataccctggtatcgcaggaagacagcgccgttttaaagcaagccagtgaaaaagccggctttgacgacgcacttctcgccaagatgaacgatatcgcccataaactgcgattggacatcaacgaagaaggtattatcggccagttctcagggtacttcaacctatccaaactgaatttcgattcataccggaagaagtatggtgatatttccagaatagatcgactgctcaaaggcgaaggcaagtcaccggacgcctaccaagttgccaaacaggctgatacattgatggcctactatgaactgccgtttgacgaagtgcaagaagtcatcaaccgtctggggtacaagctgcccgccaacttctttaccagcaacttacggttctatcttgaccggacgactcatggatcaactctttccagaattgtttattcggttctggacgaaattgacggcaacatggaccagtcatggcagctgttttcaactgccctgttctcagattactacgacattcaaggcgggacgactgccgaaggaatccacctgggtgtaatgggtgcgacccttcaaattgaaacgaaatgctatggcggtgtccgatttgataccgacgaggtcacgattaatcctcacctgccaagcacttggtctaaaatttcatttaaagaaacttaccaaggaatcaattaccacttcgtcatcggtcatcatcggatcgatgtgaccgcagatgccgatactcacgtcagtgttgcgaaaaaggcttattcactgactaagaacaagatggcaacaattacctataaataataaggagtgaatgataatggcaaaattttccgatattaaaggcttcgtgttcgatttagatggtgtgattaccgatacctcggtttttcacagccaggcatggcatcaagttgccgataaagtcggcgctccatggtccaaagaacttgaagacggtctaaaaggcatcagtcgaatggactcattggaaatgattttgaaagctggaaatcttcaagataaatacactgatgagcaaaaggttgatttggcaactgaaaaaaataccaactacttgaagttggttgatcaaatgacccctgacaatatcttaccggggattaaagcattcttggacgaaatcaaaaatggcggctacctattgtcattggcttcagcatctaaaaacgcgcccaaagtcttgcaaaagctgaatttaaccgattatttcccaaagattgttgatccaaaaacattgagtaaaggcaagcccgacccagaaatttatttaaagggtgctgaattgattgatctcaagccggaacagtgcatcggcgttgaagacgcggcagctggtgttgaatcaattaacgcagctggcgaaacctcgattggcatcggcgacaaaaatatcttaaaggatgccgacattaattttgccgatacttcagaaatgacgttggctaatattgaaaagcaaatgaattaagggttcgtttcaccccctaattctgatgattaacgacgaaaggcaactacctctgtttcggggtagttgcctttcgtcgttaaatggtcgagaacaacctttgacgagatattaatcaatcagcccataatgtttaaggccgttcacaatcccaccgttaatatttgatttagtgacaaaggacgccttttccttaacttctgggacaccattacccatggcaattggaaatttaacttcggaaaacatttgcaaatcattcatttgatccccaaacgcgtatgatggaacgtcaccgaggttcagtttcttcatcaaagcctgaattcccgtttgtttggaaacaccccacttcatggtatccaaacaacgcgggttgttacggaccaaagacaacttccctttgaacttgtcttggtagagcttatccttatcgtaattaaagacgtttaagaaattaacttcatgatgcttgtaaaattctgggtcaacatgtggtgttaatcgcaacagacgatagttcactttcgtcatgtcattttcaaaagtcaacgcaaattccttattgttgtaaaaggaaatgacatccccctgctgttttgcaaaggcaaggatttcctcaatcacatcatcactaatttgttctgctttgagttttttgccttcatactgaacataactcccattagcgctgactaacgagttaatcccagtggcatcaatcacatactgaatttcaaaaatatttcgaccagtggagatcaccggtaaaatattattggcacgtaattcattgattgccgctacattttcgtcggacacgtttttttcattatcaaaaagtgtcccgtctaagtcaaagaacacaaccgctttatacattaaattccctccatttaacttattaactatattgtactacttaatatgtgcggcattcccaattttaacttccgaatcgggaaattatatatattgtgttaccacattttgtggtacactatatattgtcattttattataaagaggggctaccatggtgataataactgcaggaatgattggggtcggaaagaccactttaaccggaaaaattgcggaacatctcgggacaaaagcgttttttgaacccgttggcgataatcccgttttaccgctttactactccaatccaaaacaatacggatttctacttcaaatttactttttaaacaagcgtttctcaatgatcaaacaagcattgagtgatgataataacgtcttggatcgctcaatctatgaagatgcactgttcacccgggaaaataatgctcagggaaacatcaccgacactgaattggcggtttacctcaagttattgaataacatgatggcagaactcgacgagttgccaaaaaaggctcctgatttgctggtgtatgctgatagtgactttgacaccatcaagcaccggatcaaaaaacgcggtcgcgactatgaacagtttgacgacaaccctggccttcaggaatactacttcaagatgtgggcagcatataagaaatggttccaagaatacgatgtcagtcccaagatcaaaatcgacttgcagaagtatgacttgtccgatcccaagaatgtcacaatcgttctcggacagattgatgatgctttggctaaaattcgccaaccacaaagtgagacactctaacagacagtcataagtttcaggtctaccagatacgatgaaaaggccacggagttaaaaggagatgttcagctgataatttcacagctaaacagcccctttttattttgccaatttaattttcccaacgattgcgtccggatccgccttataatcgacgcttccctttgacaccaagtaatcaatccggtggcggtaccaccagtcagccgtgaacggataatcgcccaaagtctcaccaattacccgcagaatatttctaaaccgccgttgactgagattggcaaggacaaaacgatcgtaaaagtcaatcgattgactgacaacggtgccgttaatcaccgttctgatcggattattttcactccttaagtcatgccaatagtaactgaaggctctccgggaattagcagacaggtccctttgtagtgatgccaattgaaattcatcaatggcgtcttcactgatttcacctaatttggaaataatcattaaactgtcttctcggaccaaggtcattggaaccttgacactcatcgtttgaactgaaaaatcctttaaataatcgcaaatccacaaaaagccgcagtagtcgtcagccgtctcactccaccaaatacgaaacgattcgccagcctgagcactttgactcagttgatcaagcccctgccgtaaagcatttaccgcttcgacagttaattgttcagaggcttgataatgagcgtattcgattttataaatggtttgacggctttccataaacgagcgttgactgatgtcccccaagctcagatacattggcaatgccaaaacctgcccgtcaagatgtcttttctgatagtaatacttcaatgttgatgcaaaactatcactgaatacgatgtcaatcatgaccaaacctcacccttcgaaattgtcatttctcaatgacgtgcttcgaaaagtataacttttttggtggcctggatgcaacttttatttgactgaatcaggccactcttggtaggcttgatataaacaatattgggggagatgtagatttgcaaaatacaaaacaacataaattatctgccgctcaaatttgcggctggatcgtctggtgggtgatcaccattgtcgttttggcgctggcaatctttatgctgaccagaacgacggatgctgcaggcgttcataactcatggaactatcacatgatcgccatttttcttttgctggtgtatggaatccagcaaatcattgcgttctttggtattaaacgacttcactacaatgaaagatacgtgtggccgattgttttaatcgtgctgggcgtcttgggcagtttcttgtacgtgattcccggaatctggggattaattgttaacaatccgcagaagaatcagccaaccaaaattgaatgatggacggcaaaagaggtgaaccaggtattctcgaaataccggctcacctcttttttcaggttctacaatatctgttgttggtaatagatttttgtctattactgatgacagttttttgtttatcattagagtaaaaaagcggacatctcccgtccgttaacttgctcccaccacagaattaagtcaagaaaggaaatgccctatgtcaaatgatactacgaaaatgttgttaggaatagatgatgaacacttaataattgagaatggcaaaataggtgatgatggggtgatccgattaaatggatcgctgaactattcccccaaggcctgccacaactgtggggttattaatgaccatcagatcattggctatggttggcggaagaccaccattagattcgctaaaaccttgggcagcaccgttatcctctgcctcaatcggcgaaactttcactgtaaggcttgtcataccaacttcctggcgcagacgaatgcggtgccgaaacactgcacgatttcaaatacgacccgcaaacaatgcttagaaaaactgaccgaaccggtttcgctcaaacacattgccgatgagttatccacttcggattcattcgttggtcggcagctcttgcgcgctgaacgggactttgaaaccaactggcactatttacccaaagttctcctcatggacgaagttaaaagcactaagagcgccaccgacgcgatgagctttgaatttatggacgcggaaacccacgaattgatcgacctgttaccctttaggaccatctatcagcttcaaaagtatttccagcattacgaccaggctgcgcgagaaaatgtgaaaattattgtcaccgatatgaactatacctatcccaaattggtggggcagatctttccgaacgccatcgttgtcatcgatccgttccacttggttaacgctttaaatcgagcttttaataagacgcgggtgcgcctcatgaaaaccctggcgacctcatcacgcgagtatcacgccttgaaacgctattggaagctattattaacgccggaaaatcacctcaactacgaagctttccgtaagtggacaaacttcccttatccagcgactgccactgatgtggttgatgctttattggacattgatcccgagctcaagcaaacttacaacgtgatgaatcggttacgtgaaaccatcaaaaaccgtgattggcccaactataatcaagtattccatcacttagagggctgctcggaagagatgttggcaaccctccagaccctagcgactcatcatgatgaaattggcaatacctttactcaccattacaccaacgggcccttagaaggttcaaacaacaagattaaagtcattaaacgcactggatttggttaccgaaacttcttcagattccggctaagagtgctgttcgcttttcgagttcatacaaaaagagctctaatcaccaagtgattagaactccaatattttgttcaccaacaacagttgacgaagaaccttttttcatttcagttgttctaaccgacttgaaaccggctagtcgcgatggaccacaaacacatcacagggggcttgagcaataacaaaagctgctgttgaccccattgtcatccggtcaacaaaatttgccccggtggccccgacaacgattgcatccacatgttcgtcatccaccaactcgtgagccaattgatttttgggatcgcctgaagttacaaaggcactgacagcaagtcctcggtcttttgccatcaattcgtatttatgaacgagccgttgaaatctggatttgacctcatcgatcgttgattgattgacgttgccaaaaccgatcaaggcggcttttgacacccccagaatttcacggtcgttgataattgccacaattgtcagcttggcatggttgtgctcggcaatcgtgattgcctgtctaacggccttggcggcagtttttgaaccatcaatcccaaccagaatattcgaataattaaagtccaacatactaaccacctcaatgtttttacttggctgtcaactcataaattgattgcccataaattgccattgccttgattaaattggcaaccggctgaaactcatttgcctgatgcatggtatcttgggcgtttgggaacaatgcgccaaacgccaccccacgtttcatcaaacgggcataagtaccgccgccgacgacttccggtttggaatccatatcgcccgtctgttcctggtaaacgtgcatcaaggtactgacaatcggatcacttggatcaacgtagtgggtgtccatattgttgatttccttaacggttccatggcgtttatcggcagcctgttgcaagtgagccaaaatttcttgatcatcagttcctttcgggtaacggaagttggtgttgacgctgccgccgtgctgcgtgtcaaatttcataatcccaacgttcatggttaactctcccatgatgtcgtcgacgtgcgcagcaccgattttggttgcccgggaatcgtcatgcaggtcttcagccaggtaggaaataaattccttagcggccccgtcaaatggatagtcattcaaaaacttggcgagatacgtgccggcattgacgccgttcttgggttccatcgcgtgggcagctttaccggtaatgtgcaaagcaacgccctgaccggttgatttgacatcaccggcaatcgggttttgatccaaaaattcggtaaagccatcgacaaatttttcgttatcaccgacttcgaccagcgcatccgcagatccgggaaccatgttcaatcgcaatccggaatcaaatcgcttcaaagtgaattcggaaccatttgtatggccaaaggtcgtgacataagtggcattgcccttctcaccattaatcagaggaaattcagcatctggggaaaaaccaaaggtcggttgcggttcaacttggaaataatgcttcatcccggtccagtcactttcctcgtcagttccaataatcaaacgaatcttcattttgggcataatcccattgtccttcagcattctcaacccataataagcggctaacgcaggtcccttatcatctgacgttccacgtccatagacgttgccatttttttccaccatttcaaatggattggtttcccagccgtctccagcaggcataacgtccgcatgggcctgcatcgccattgtctgatcgccggaaccatactcaatatagccaacaatgttgtcgatattttgcgtcttaaagccgtcgcgctccccaaatgataaaaatttgagcatcgcttgggttggcccctcgcccagtggaaattcatcagtcttgtgctcatcgtcacgaacactgttaatactgatcaattcctttaaatcgttcaaatactcgtcttgataactttgtgcgcgctttttccaatcaactgtcatttttctcgctcctgtccatttcttatagttcaattttatcacactattcaattggcgttggcaatctgtccactccagaaatgctataattagggtgaaaaacagattcggatgggagatctgatgatggtaaatgtcaaaaaaatcacaagtcaaattttaacagatgtcattcgtaagcgaccggcagatagttttaaaggcacttacggcaaaatcgctttgattggcggcagccaaaactttggcggtgcgattatcatggcctcactggcagcagtttattccggagccggcttggtcaccacgattacggaccccagtaatcaaaccagtctgcatgactggctgcccgaagcaatgtttgtggattggaacaattttgatcaggcagaaccaatcattaaaagtgccgacgtggtggtcattgggcctggcctgggaaccgatcccagtgcgttgaccctgttgacaaaagtctttcggattgccggcagcgaacaaaagttagtcattgatggttcggcactgacattgcttgctgccaacaacttgccgctgccacaggattcgatcaatattttgacgccgcatcaaatggaatggcagcgagtatccggcattaagattgccgaccagacgccagagaaaaaccaggcagccgccaaacagctccacgcaattgtggtggttaaatcacatcgaacgcaagtttatgcggacaaccacgtctacgaaaacactggcggcactcctgcccaggcaacgggcggaatgggtgacaccttggccggaatggtcgggggctttgccgcccagttcaaagatccgcaaaaagctgtgttggcggcggtttattctcatagtgccattgctgataaattggctgaaaagcaatatgtcgtcctgccccaccaaatcagtgaggctctgccgaaatttatgtataagcatcaagctaaataactaaattgaatcacaaaagtctccatcagctgaattgtcagtgatggagacttgtttattttatcttggctaaatatgaatgaaaacagctggttattggattttaagcaaccgtcgcaacttgtcacttcgcgggcccagaatcatatcggcaattcgactcttcaaggctaagtataggtaaatcaccccaccaaccaaaacggccgccaaggtcacgatcagactgacaacccgtccaaatggattaccaaccaattgaacaacaaaattcaatccataaaccgtcaacaatgcagcagcatacataaacaatgaatatttcgaaatcttccgaaaagcaatgtccaacatccgtttttcaaaaccgaaatggcgattcaaatatataagaatcaaccagttggcaacggtcaagccaatcccggtggaaagcagtggcccaaacgaacccaaaaaataggtacaaggccactgaagcacaaacttaaccactgttccaacagcaaagaacttaactgcccgtctgttttgagacaatccctgcatcacggcagaaataacgacaaacaatcccatcggaatggaaataatggatgaaaacgttagaatattagcgccgagtgcctgatgagtggtgccatagaagacccggttaagcggtccggcaattgcggccattcccagggcagcgggaatcatgacaaacatgaataatgccatcacattggagttttgtttgcgaatttcgacgttgtccccgctggtcagcgcttctgagagcatcggcacggcggtaatcgccaaagcagaggaaagcgacacagtaatcataatcaatttatttgagttaacggcaaacattgcatatagatcggagagggtcgcgtagttgtaatcagttgccatccgcataatcttgaagaaagtaaactggtcaatcagcataaaaatcgtgattccggcacccaatataataaagggcactgcctgcgcaataatttcctgatataattgttttgcttcaacgtggatctcattattgctggacaaaaccagctgtcgaaaatcttcgcggcggcggaagtaataaacgccaagggtcgccaggccggcaaccgcaccaatgaaagcagcaaaagttgattgagaaacagcattgacccaactgccatgcagcacccgcatcataatgaaggctgtcaaaagcatgtaggcaactcgagccaactgttccacgaattgggaaatcgctgatggcgccatttgttggtaaccttggaaataaccacgggtgaggctcatcgtcggaataatcaaaattgcccatgccaatgaatgcaaaaccggaatgacgttgggattgccgccgtcaattaagggcgcaccaaaatacaggatcaccgcacagataactcctgtagcaatggccaacaccaagccccgtttataaagccgaacgccgacaccatactcatttaaggcattgtaatgagccacttgtttggcgatcgccgagggaatcccggcaatggcggcaatcaagaagaaactgtaaatgttatacccgagtccgtacagcgcgttggcttggaagaaataattgccaaaccaaatcccccagggaataatatagactgcaccgagaaatcgactcaaaatactaccggccgtcatccacgctgacccggataacatctggtcacgcgacttttccgtcaggttttgatgattatcaatcatgattgttcctactttcgtatactttgacactcgcttcattttaatcaagttgctaatgaatagcaataacggggtgatatattaaaaattacttaagcatcaattgttttatagagatgtaatgaaaaagtattgtcatgaacaccctaaatgcactagaatatttttatatgtggtcttaataattttcgaggtgaaacacttgtgagtaaaaaaagaatcgagtggattgacgttgccaaagcggtcggaattgtcgccgttgttttcggtcacgccatgacacgacacggcaccatgttccattttctttattggtggcacatgccgatcttcttcatcatggggggctttttcttaaagccaatcgtcaataacaattggatcggttttttcaagaaacggattttaccactgctaatttcatatttaatctgtggtggctttttgattttactgtcacacttcatcagaggtgaaagttggtcgtacacgatcttctactttgcccgattactgtatggtggacggacactgaaccactacctcagtgttttttggtacattaatgtttacctgttggccctggttttcacatcgattgtcattacatacgtcaaaagccgggaagcacagattattgtggcctttgcttcattaatcatttccaccagttacaagcacatttacttcctaagttataaatacgttccctgggacttcgatgttgcttttatcgccatgttcttcatgttatttggctatctttatttccacaaaattcagcaattcgttaaggacctgtgggtgattattccagcagccatgcttaccgtctggttgttttggatgcagcacatggaccggttcaacttcgcgttcttcctgaagtccaaaatcattcacgcttcctatcatcacattccaatttctcgggtttcctacattacttttatcccgattattgtttgtttagtcgttttcagcgccagttactatttctgcaaattcatgccccagttcctcattaagccggttcaattattgggccaacagacattgggaattatgtatctgcacaaggccgtcatcgatatcatcgatgaagctggctacaatggtgccattatggaaacaattctggcggttttaatttcgtttatcctgtcacttggctacggctatgtcaaacaaaaaataaagaattcacgtataaggcggtcaattagttgataaattatcggcgctcaagaaacttgcgaatactttactttgtaatcggcgggctcatcatcttgggcttcggttttaacatttggcaggatcagcgtgcttcggatcagctcaaggccaactatattgactccagtacgccgactatctttgtccacggctggggggccacccttcgttccgaaaaagatatgatctccgcggcagaggtcagtggcgccgcttcaaggcgaatgattgtccgcgtgagagccaacggaaaattgtcagtcactggaaccgttaagtcatggatggtgaatccaatcattatggtccgaatggacaataaccgcgccggcgaggttcagtatgctcgctggctgaccaaggtctgcaagttactcaagcagaaataccatgtcaatcaattaaactttgtcggccattccatgggggcttacgcggtaatctactataaccttttgaacggcaaccggtctgatttgccgcgaaccaataagttatgtgtgattgccgggccttatgatgggataatggataatcacaaatctaatcagccgacatcaggtccactgatgcagttatgggatgatgcgcccaacaaaaatcgcattttgccgactggtaaacccaagatcatccatcctgaatacaagttactctatcggctgagaaaaaattttcctcgtcaaaccagggttttgaatatctatggtaacttgggcgatggttcaaattcagatggcgtggtcactaacgcttctgccctatcattgggttatattttgcgagatcatgtcagtttttatcaaacatttcaagcttttggtccaaaggcgcaacacagtgccctgcacaataacaacattgccgtcaataaaattctaacggaattcctgtggaataaaaattaccaggatagttctgcgagtgaattaatgcaatagcaactcaaaaacagccaaaatccatttcggattttggctgtttttcattcatgtagttgattatttaaaggcactcactaatttacgattagctgtgatatatgaaccatcagctaagacaaaacgcgttgtcaagtgataatgaaccatgcgtttgacattgacagtctggcccattttgtaggtggcaactctaccagtcaaattcttaccttgatagccatgaatgccggtcgggttgatcactttgatttttgggtgacgactggcgtaatagactggtctcacataggtccagtttgccgttaggtagcctgttttgccatgggaagggctttgatgattgacatcccgtacccggtaccgcaacttaccagtagctgaacgagcgtagccggttactacaaacatgggtcgggcatagcgcttttgagctggatatcggaaaagtcgattgacggccttaaaattgggggaactgtatagcccgaccgttttgatggcgtagacggccatcccttttacggcgacttttttgtttggagtcggttgggttattgtagcttggcctacatgcgtcgagttgttcaaaattgcgaccccggttgctcccaggtgggaatcagtcgctggccgggatgacgtgcggacactctctgttggccgactaacagagatttgactttttcccgccacattaaccctcgtcgaattcgttggttttgacgggaccactggccattgttgtgcaacctgggacaaatctgacggaagacttgcagctttcgtctcgacaggtttagccgcctgaaacaccggttctttagttattaaagttggttgaggaaccgtgggccgttgttgcttaacttcaacttggggagcacttttttgcacctgatcagttgagttgactggtaataccggcgctacattcgaactggctggctttgtgtcgccactgtcttgtgtcaccggtttggcagcttccacaagttttgaatcggtgcctgcgtgagaattcgtagacccctcagcatggttctgctttggccgggtttctttgacctgctcggcctgatctggctgagaagcattcactggctggtaccagaattttaccaggcaagtcagatcccttaattctctaaaacaaaagtttaccgattgatcgttatttttagtgaaatatgggctttcaaaggttgcctcaaccggctgatatccctgaattttcttcggcttaatggttacttggtcagcgtaatgcaacgttttggtggcactgtccagtgtgttactatcttgacgattcatatagttaatattcaccgttgcggtatagaggccggtactttcctgactgtatttgagcagcaacgggtgctgcaagtctgcacgaaaatctggaactgtatgagaaatcgttgtggttggaacaaagttcttataaaccggtacttgaaaggatccccctacattgccgaccatcttaattggcttgactccgggaatcacctgccagtcaccactgggatcggattggtacaccggctgaacataaaatgtcacccgctgtcccaactcagtcgtgcgcatgttcgctgctggggaatccgcgtgagctaacggtgcctgcagcatgattaacccactggcagccatgagcactaaactgctccaaaatttaagactattagctttcccccaagtcactttatcaaatttatccatcatctttctccttcaacatttttcaagacgacttaactcgtcccgttcgtaatatatatacggagaaaatggcggaatgtttttatttttttgaaaataattcaactgttcaaatcaaaaacagctgaggacaattccccagctgtttgcttgatcacgttaaccgacaacaatattaacgatcttgtttggaatgacaatcactttgcgaacagtcttgccttccagatagcgttcaacattctcatcacttttggcagtttgttcaactttgtctttatcaagatcacgggctaccttaatgtgtgaacgaactttcccgttgacttgaacgaccatctgaacagtattttcaactaacttggaagcatcatacgttggccatttttcataggtaatcgtgccgtcatgacccaatagactccacaattcttctgcaatatgtggggcaaccggtgacaggagtttgacgaagccttccatgtaatcaattggcagtgaatctgccttgtaggcgtcgttaacaaagaccatcatttgagaaatgccgacgttaaaccgcatatgttcaaaatcatctgaaacgattttaaccgtctggttataaatcttgtccagcttgccgtcgttgatcgtggtgacgcggtcacgaagatggttgttatcgtcgatcagcaatcgccatacccggtcaagccaatggtaggccccgtgaatgccttccgtgctccaaggcttggcagcatcgattgggcccatgaacatttcatatacccgaagtgtatctgcaccatattcatcaacaatatcatccgggttgatcacgttaccctttgacttcgacatcttttcgtggttggttccaagaatcatcccctggttaaccagtttctggaacggttccttggttggcacaacccccaaatcgtaaaggaacttgtgccagaatcttgcatatagcaaatgtagaacggcatgttcagccccgccgacgtataagtcgactggtgaccagtacttcaacttttcaggcgaagcgatcgcctggtcgttatggggatccatgtaacgcatccagtaccatgaactaccggcccactgtggcatcgtgttggtttcacgtttgcctttacggccgtttttatcaaccacgttgacccagtcatccaagttagcgagtgggctttccttgccaccagaggtttgaatatctttggcctttggcaatcgaagcggcagctcatcttcaggaaccagcgtcgtttcgccatcttcccaatgaattactggaattggttcaccccagtatcgttgacggctgaaaatccagtcacgcagccggtagttgaccttttcatgaccggctttatgatcagttaaccaatcgatggctgccttaatggcgtcatctttgcccatgccatccatgaagccggagttgaagtgagaaccgtcacccgtataggcagcttcgtcggtattaccaccttcaatgacaggaacaatcggcagtccaaatttcttggcaaagtcataatcacgatcatcatgggctggaacggccatgatggcaccggttccgtatgattcaagaacgtaatcgccaatccagattggcacttctttaccagtcattggattaatcccataggcaccagtgaagaccccactcttatctttgttcaaatcggttcgttcaagatcggatttgcgggaaacttcttcttgataagctttgacttcagctgcttgttcaggggtggtaatctttgaaaccagctcgtgttccggagccagcaccatgtaagttgccccaaacagggtgtcaggacgggtggtgaacacttcaaccttgtcatcaggatgacctttgacctcaaagaacacgctggcaccacgcgagcggccgatccagttgcgttgttgttccttaatactttcaggccaatccaggtcgtccaagtcatcaatcaatcgatcagcgtaagccgtgatcttgaggacccattggcgcatcggcacccgataaaccggatagccgccacgttcagtcttaccgtcaacgacttcctcgttggcaacaacggtcccacccataaaatcaggggcccagttaacttcaatattgtcttcataagccaatccgcgtttgtataattcttcaaaaatccattgggtccatttgtaataacttgggtcggtggtgttaatttcacgatcccaatcatatgagaatccaagtgaacgaatttggcgtttgaaagttttgatgttcttagctgtaaagtcccgcgggttatgccccgtcttcaatgcatactgttctgcaggtaatccaaaagcatcccatcccattgggtgaagaacatttttcccctgcatccgcttcattctagccataatatccgtagctgtgtagccttcaggatgcccaacgtgcaggccctgacccgatggataagggaacatatccaagacatagtatttgtctttgtcagcaacttcttcagtcttaaatgtcttgtgttctttccagtaatgctgccatttgcgctcaattacctcatgattgtatgccattttgcaacttccacctttcatatttctcaatcaatgaaaaaagtcccataagaaaccagactgggcttcttataggacgatttatcgcggtaccacctatattctcaattacttgagctctcgaatcaataacggcgacaaaccggcttgatttacttcgttcgaccaagcattcgacgatgagttcgccacgacctgttctgagttcacagcagccactcagtttctggaaaacaggcagttggttactaattcgtctctgcattttcacaaattgaaattattgcttattatcataccaaaacaggtcttaaaaaacaactgctcagcgtgctataattttattattggagttgaaaacatgaaaaaacaatcacaaaaaatttcaagcaccgttagtttggtttcactggtcatctttttggttctgacttacggcgtcgtcttacataaagaatggatcaatacctttgacacctacttcggccacatggtcagaagctttcaaacgccctcgctaaccagcttcatgattcattttaccgagctgggaaattatcagtcactattggggttcacaatcggtgccggtttgattttatttttggttcgcaaaatcaagtcagccttattcctgttgattaacggcgtcgtcttggcagccccaattgataccctggtcaaacacatggttaaccggccgcgaccatccctgacccatctggtggctgttcacagcagtagtttccccagtggtcactcaatgagtatcatggtggttgccggcagcctgattttgctggccaaccgcatgcttaaaggaagtagccaacggctgatcgttgatctgattttgatcatcatgattgtcggtatcggtatcagccggatatatgttggcgttcattatgccagtgacgttctgggtggctggagtcttggcctagtgaccttaatggtgtcacaatgggtatttaatcgattcgcaggaggtatctcatgaaaatcaaatcagcattggaatatagccatgaactgttatcagaaactgtcgattccggagataccgtcgttgactgtaccatgggtaacggtcacgacaccctgtttttagccaatttagttggcaaacaaggcaccgtgtatggatttgatattcaagcccaggcagttgaaaataccaaagcacttctaaaaaccaatcacgttcgcaccaaaaatgtctacctgtacaatatcagtcatgccaaagttgatgaaattttaccatacgagaccatgatttccggcgccatcttcaatctcggctatctgccgggcggcgattaaaggctgcctcaaccatttgtgccataatgacgtgatcgtcgtggttgcctactacggtcacccaggcggcgaacgcgaaaaaaacaccgtcctcgaatttggcagtcaactcgaccaaaaacgatacagtgttttgaaatacagcttcttaaatcagcagcattttccaccaatattgatggcgattcagcggatcgattaattgattcgctgttttttatttttgcggtcaaacaaattgcagatataggcaatgataatcagaatcaggccgaccacaaagacattatgcagggaattgtacaaaatatttcgcaactgcggcaaaattttgtcacttaactgattggcagtcaatgggttaatcagtttgtccatcattttcaaggacgtatgttccgtttgccgaaccccacgcagcatggtggtgttcatgacgataccaaagattgaaatcatcagtgtctgacccagcgttcggcacaaagtattaaaggaagttgccacaccaatctgagttggtttaacctcattttgaacgctaataatcgacgttgtcaccgttaagccaaagccggtcccacagatcattgaaatccccaagaaggccacaaacggcgtatatgccggaatcagcaccataataatggccccaaccaagataaagaagagactgaggttaataatgcggtaaggtgacgtcctggccagcaatttaccggccaaaaatgagccgacaatccacatcagggaactcggcgtcaccgcaaacccggccatcgatgcccgcaggcccaaaattccctgggtccagtccggcagataaacttcgtagccgatcagaaagccactgaccaaaaaaaccacgatattttgaacgacgaaggtccgattatcaaatagttccatcggaattaacggatcggccgccagtctttctgtccgaataaacatgacggtggcgatcactgtaaccaagaagcagaccgcaacgatctgccagttgatcggatcctggccgaccaactggaacgcatacataactgccaacagcatcatcgtcagccaagtcgtcccggcaatgtccattttagtggtactgtggtgtttgtcttcatgcagaaaaatttggaccatgaacatgacaatcagcccaattggtaaattgataaagaaaatccagtgccagctcaagtgatcaacaatgaaaccacctaatagtggcgcgatcacagaagcaattccccaagcagacgagttcaggcccaacacctgagcgcgcttttccaggggataaatatcggcgataatcgtattggaaatcggcatgatggagccggctccaaccccttgaaccgcccgccaaaagatcaaaaccaccatcgagtgcgataacccggacatcaccgacccaaagacaaagatcaaaatcccgccaataaacattggctttcggccaatactgtcggccaatttaccatagattggcgtcgcaattgcattggttaacagaaaaatggaaaagacccaattcattagggaaactccccgcaggtcaccgacaatcgtcggcatggcagtcgaaacaattgtcccttcaattgcggccataaaggtggccacaaagagggcaatcgttactaaggttacattacttttggttgctgttttcgtcatgaaatgacctcttttctttaaaattaaacaaaaaaatgcccttgaattttcaagggcgttttgcttgtcagctgtttataacttgaaatagtcttttaacgcatcaaccttatcggtatgctcccatggaagatcaatatcggttcttccaaagtgaccatacgctgcggtctgttcataaattggtcgttttaagtccagcattttgataattcctgccgggcgaagatcaaataatgctcgcgtggcatcaatcaattgatcttcaggcactttaccggtaccaaatgtattaatgtcgattgaaacgggcttggcaaccccgatggcatatgccaactggatttcagcttcgcttgccaaaccggcggcaacaatgttcttagcaatgtatcgcgccgcataactcgccgaacggtcaactttggtagcatcctttcctgaaaaggcaccgccaccatggtgggcgtaaccaccataggtatcaacgataatcttacgtccggttaacccggcatccccttgaggaccaccaatgacaaaccggccggttggattaaccagataacgggtcttgtcgtcaagatacttggcaggaatcacctgtttgatgatttggttgatcacatcggtccgaacttgatccaatcggacaccatcgtcatgctgagtgcttaagacgaccgtgtcaactcggaccggcttggcgttgtcatcatactcaacggtgacttcagccttggcatccggtcccagataaccaatctcgccactcttacgcaagtctgcctgctttctcatcagcttgtgggctaatgaaatcggcaacggcattaactcgggtgtctcatcaatggcatagccaaacatgaggccttggtcaccggcaccgatttgatccaacgggtcggtattgccttcacgttgctccaaagcgtcatcaacacctaaggcaatatcaggtgattgaccatcaagggcaacgataacaccacatgaatcaccatcaaagccgtaacggccatcggcatagccgattcgcttaatcgtgttgcgaacgactttttgaatatccacataagcagtcgtggaaatttcaccgaaaacaaacaccagtccggtggtgactgaggtttcgcatgctacccgagcatccgggtcttttgctaacaaggcatccagaattgcatcactaatctgatccgcaattttatccggatggccttctgaaactgattccgaagtaaataaatgtttttcgcgcattctattttccccctattattttttaaggttacaaggcttcttcacgcatcacgtgaatcctatcgggaactcataactctacaatcttatcatatttgatttgcttttcaagccttattttcagctgtccattgaccatctgacagaaaaccagtaggattatttttataattagctattaaaaatgtgaggaagttgaggatttgttaaaatttgaccgctccattttaattcaatcaggactgcgcgccgtcagcatggtctttatctggatgctatttgccaatatctcgttaaagggatttttcgtcaatccgcgtcttctgcatctcttggtgatcgggttcgtgtttgccgttttattgaccgttgttagccgaccacgcaaaaatgccgtcatgatcatcttaaccgatattttgctgggtatcttattggcgtcgctgtacctcgatacgccaagcattaacgtctggctgattctgatcggctttttgctcgccaacctgctgttagtctctaatttaatcgatgaacctcactgtcgttggattatttatgggttcatttccggaaccggaattgtcttgttgttcacaacgacctaccatcactatttttcgctggtctcactgatgtatatcaccctgatgattttcgcgaatattttcttttcctactacgcctttatgaagcaaaacaatcagctgtccataatgatcgtgtcggtgctgattttaatgttgtgtctcacactcaacatctcatttgttaaaatcattcttatcgctggcattctggcattctacgcttattttgaatcccgggttaatttccgtaattttgaaaaacgggccaatgtttcgacggtttccttcctgttgttttcaatgctggtctgtttttaaggttcatttattataattttgttaatatggttaattttaagaaaagaatcaccaactttgtcacccaccttcattcaatcgtgtagtatggcgttgattgataaattcgacaaggacggtaacaagcgtgaacattaaagtagttggtgatatccgagtaggcaaaatacaaccctcattaactgggaatcccattgttgacgatgtcctcattcaacatttttgtgatcgactcaaagaaaaattaaattcactgcaaccatccgttgatattattcccgaccatttcttcgatgctaccaagccatgtgccgacatcattttgatggacaggcgcatcatcgatgatctccccgacgaactgctgatgaactttaaaataatcgacattgaccataatgatattttacgaggtaacattactgaggctgtgaacgcactcaaacgatatgattccggcaagcacgtttttgcgatgtagtcgtgaaacttacccgtcggtatttgcaaattgcatcatacaaaaagcccgtcatcttgaatgacgagctttttgtataccgaaaaatccacgaagcggctttcagctatgttctatttcttgaagcggcgatccttcttaatatacacaatcatcaataagaccattaccatcgttaaaacgactgtatagaaccaagcttccccacgacctgcaaatggtagtttaacgttcatcccataaaacccggaaacaatcggcggaatggctagaatcagtgaccaaatcgtcagaaactgcatcgtttggttcaatttattattcaaaatattcccaaatgccgactcggtttcccgaaccacgtcgccgaccacatcaaacatggtttgacactgtttgtattcaattaacaggtcaccaatggattcattggttttgctggcaagttcgggggacatcttcaagttatccttgatggtggcttgtaactcctgcagggcgatcaagttgcctgccgtggccgagcgcagatagaccagactggtctttagtgctgccaattcatccaaactgtggttgcttattgcccggttgtgcatcccttccaacttctcggctttctgactgatctcgtccaatttgtcaaagaacggcgaaatcaatgcaaacaggattgccaaaatgtgctcggcaacactgtcatatgccaacttggaatggtctgaaaccagcttagcctgctcttgggcgtgacacaccgtaatcagcagggaattactgaatcccagaaaaatcggcgatgtgagcattcggctttgcttaggatccgcaattgccctgaccaccagtgcactaaaccctgacagatcatcaaaagtggcccgtggctgctcatgacgatccagcatatagcctttgaacttggctggtgcccgatagtcaatcgtaatgtcatttaattcgtcttcagttggtgaaattgcctcgacccaggtgtaagtgtcaaacttatgaattttaatcatggaattgcctcttcaatcgtcattttatgaataactaaagtctaattttttccgaaagcaatttcaatccccaactacctgccgccatgacgccgttggatcacctggtaaattaccagcatcgagccaattgaaatcaaggaaatgaccatcgccacccgcgttgagctgttcaccaataggaatccaagaatgaagacaaagaatgccagtgtcaaataatcactcaacggatacccaggcattttaaagacctcactgcccttcggatgagctcggcgatatttaatgtggacaatgattaaaaccacccacaccacgacaaagttaatggttgaaacacttgaaaccaggttgaagacccctgctggaataaagtagttcaaaacaacgatgattaacagaaaggcggttgagaagttcagggcaatgtttggaacgccgttgcgccccaatttggttaaaaatgacgaagcattcccacccatactcaacgcgtacatcgtccggctggtactgaataaacaactgttagtggcggagactgcggcagtcaaaacaacaaaattcaaaatcccggcagcccccacaattcccactcccgagaacacctgaacgaatgggctggcggtcgtggtgattttattccaagggtaaacactcatgaccgcaatcatcgagccaatataaaataaaccaattctaattggtaagctgttaatcgcctttggcagattggctttgggatcgtcagtttcgccggccgtcaatccaaccatttcaatgccgacaaaggcaaacaccaccatttgaaatgacatcaagaacccgtgggcgccagttgggaaaaagccgccatggctgaccagctggctgaacgaagccgtcgagccgtcaacatttacatggaacacggcgagtcctactccgaccacgactaggagaataattgccacgactttaatcatcgaaaaccaggattccatctcaccaaacaatccgacattgaccagattggcggcgaacagacataagagaataatcagcggtggaatccattggggaactccgggaaaccaaaacttgatataaattccggtggcagtcaaatcggccattgccaaactaatccagcagaaccagtaagtccagccggtcacaaactcccagcggtcacccaaatacatttttacaaaatcaagaaatgaatgtttgctggtatctgacagcagcaattcaccaatcccccgcatcagcaggaaacaaaagatcccgacaatcaagtaggataaaatgattgatggccctgaagtgtgaatggccgaaccggaccccaagaacagcccggttccaattgccccgccaatcgcaatcatctgaatgtgtcggctttttagtgaacgcgatagtgaatttgtttgatccttcgtttccatagtgtcctccttaaaaatgtccattaaaaacgcccccagtacctattacagtaccaggggcgttcttcaacgcggttccacccaagttccacaatacaatatgtattgcctcttattgcagataaggctgccgccattaagtattgccattttagttgctggctttcagcaaatgccagctctctgtgaatatttaccagtatacggttcatattttaaatgtcaaccccaaatcgtcaacacatgttcacagatgaagaacaaagacgaaattaaatcagcaaattagttgatttttcggccaatatcgagtatctttgagccaataaaagttaatcagacttttaatcgagtctttatggagggatacatttatggaatctcatacagctttactgattattgattataccaacgattttgtggccgataaaggggcgctgagctgtggcggccctggacaggtacttgaaccgcatatcttaaaattagctgacgaatttgtggccaatggcgactgggtgattttaccgaccgatgtgcatacaccaaatgatccataccatcctgaaaccaagttattcccacctcacaacgtccgaggtacttggggccgtgaattttatggtggcttatcaccttggtttaaagagcatcaagcagatgataaggtgtatatgtatgacaaaacccgctacagtgcctttgccggcaccgacctggatatccggctgcgtgaacgccacgttgacaccgttcatctagtcggtgtctgcagcgatatctgcgttttacacactgccgtcgacgcttataatctctgctacaacattgtcgttcacaaaagcggcgttgccggattgacccaagccggcaatgactgggcattggatcacttcgaacatgttctgggagcgactgtggaagattaatggcgagttgctttgcaaaatttcccgatttagtgtttaatgttcttcagtagacaaaatatattttcgatcgaagatgggatgaaacgattgttttgtgaccatcttcttagtgtttgtgaatttattttggactagggaggaacgacaatggctaataaagtgtccagatacaataatgaccagtgggaaaccgctaaagaatctgttttgcaagagtatgaagattataaacaaaccctgcgggatcaaggggtcgactatacaatcaagaatgcccggaaattattgatctaccaggacctggttgccgagtggcagcacaaattgggaaccgttatcaccgaccttgaagataacctgtttgcattaacgatttttgatgaccttaaaaaacgaaagcaaagctcgcttttggcgcgcggatatgaacatatttccagttggccggacttcaacccaacggcgctggccctttggttggagcttgaggaagacgaggccatggcttagtaagtgaggtggcaaaatgtctcattttgatatttccatgttgatcaccatcgcgattggttttattttgatgaccgtaaccaacaaccgtccgttcgcaatcactttggcggtgttagcaattggcttaaccatcatgctgacaatcaaaaagatcctgaatcgaaaacaatcgcatagttaagacgacaaccacaaggggctgcgacaaatctgtcgcagcccctttgctgtctggttgatcaaaatggtctttaattattttttcttctcacccttatcttttttctggttcttttttagaaattcatcccgtgtctgtaaatccttcacgtgaattttaatttcggttggcttcaaatcggtcatttcggtgattgtctgagttaatttagtggtaattttgttaaagaccgttgggatgcatttgccatattccaagactgcatccattgccaatttaacttctttatcatcgttgtctaaatctactttcaccccagttgagggatccgtctcgtcactgaaacgatcagtgaccgaatcaatcaggttcccctctaaagacagcaccccatccacatcacgaacggtattaccggcaatcttggttaacacactgtcatcataagttaatacggttgctacactgctgttttcttgtgtcatggtttttccctccattggctattccaccctgtcatcattgacagtgtttgcgatatcgtctttctttcgggtactttgctgttcccattcttttttggtcagaacatcgttaatatttaaattaatttcaacaacgtccaaactggtataattcttgatggctttttgggtccggctgcaaatttcatcaaagatctgccgggcgtcggcgccatattcaatcgtagtttccatgtccaaggcaacctgtttttcaccaacctcggcgtcaatcccctttgtcggatcagtggtttttgagaaccgatccgctaattcactcatcatcccgccatcaagcgacaggaccccgtccacatttctggaaaccagtccggcaattttttcaattaccgagttttcaaaggttaacttcttgtttaaatctgatttttgaatcgttgcatccatcacagtcatctcactttccttccgttatttaatcatcactcactaattggctgattaagcgcttgagcccgccaaacttccagataacggtcccgatcaaggcaccaatcaaggtcagtgccaacaccgtcagcatgccgctgaggccgccaaagacccacacgacgcctgcgaccattccgaagacggctccgtacataattgcattcatcgacatcctcctcctaaactactcgtgggcgactggctttttcgcgtctgcttgaagcttcaaacggggtcactttgacccgcactttcttgacttcaacatccatcaactgctggatctcatccacgacattgttctgaatttcctcacccagtttgaccagatcttggttgagtttatcaacggcgttgacgctaacgcgaaccacccgattccgagtcctcaatcgcaatttgacagtcacatgattgacgttgttttgcgtcataattcgattctgcaaaatcttttcaaccgctgacttggaaatactcagtctgccgtgtggggactcaaatcgcagctggtcggccttccttggcgcaaagattgccattatcaacatcatcagactgactagggcgacgaccgcggatacaatcgcggcaccaatcatcatccaaggagtatccgtttgaattgtctgagtcacgactggtgacaaatagtcgattggaatgactaacccaaccagccaaactgattgggcaatcccaatcagactgacaatccagatcattaatcttgagaacttattcaatttgcaacctcctttcttaaaagaggtaaccttaacgtgccattccccgagtcaccattgaaacgaccaggactaaaataacagctccgacaatggccggtaaaattgccatcccagctaattgaggcccccaggaaccaaaaattgcttctccgagccaggcgccaatcaggccaccaacaatgttgccgatccagcccatgggcatgtcacgactggcaatcgctcctgcaagtgcgccaatgatgccaccaatgataagtgtccagagtaaactaaacatgataatcatcctttctacaaatagtattgtggaaattatagctcccttgctatagttatattttataataattaatatcttattgtgtgaataaggtgtgaagaaaagatgaaaagagtgtgaggcaagctgattagctactaggcactaatgccgtcggagcattagggtgataacagtagttaacgctggttttgcgttgactgctgttatcggactaagcggagaaagctggcttgtcgaacacgtttagagtgtgagtccgagcggttagcaaccggagcataagctgacttgcggggaaatcgagtttgatttcgccggaagttggcttatgtgcaggttgctgcttgggggaacacgtttgcctgaaccaacaaaaaaggcgtcaaccaaacggtcaactcctcaatccaaacattaagcaattccaagccctgccagcacccccacaatcactgaggcgaccaacatcaagccgagcatcaccaaatgaaatttcttatgcatgacaaccagggccaggtattcacgaatgactgcgttcggcaggtaataaaatggggttttcgacccgatcccaaaagcatgcataccaacttcccgagaaaggataccggctctcaaagtatgataattgctggtaacgaagacaattctatgattagtcgaaccggcatctttatcaatcaaggcttttgaaaacttcatattttgaaaagtattcactgactggtcttcaatcaaagtgtctgcccctctggcaccatgttccaaggcgtagtcacgcatggcgacactttcagggagtaactcgtcaccaccctggccgcccgaaaagaccaatttggcgcgcttgttggttcgatggatttgttgattataaaatgcgattcctttattaatgcgaccaccaagcaggcgaccgactttgtgtccatcaaccaatccagctcccaaaacgatgatgtaatctttattgctccggggaaaatataattgatacaacagcatcgaagacaacgtattccacacagtcagcaaaatataagcaatcagcatcgtcaaaaaagtcatgacaaacgcttgaatcggcgttggcaggtcaattgggttaaagaaaatcaaaatatcaatgaggacaacgccgatcccgacgattaacgtcaacgacccgctgagactataaccttcttttcgccaaacgacgattgcgttgataaaccagaaaataaaactcaaaattaatcccaaaataacggccagaccaacgattgcgacggccacggcaatcaccaacgcattatatttttcgccaaacacctcaaataattgaaccaggagggccaataatgccagtaaatccaaattggccagccaaccaagaaccgacgtgtttcggttcttgatcaaatatgtacctaaagccaccgtcaaaacggcaaaaacgacgcctgtcaaagccaccatccacatactcgttcccccttttgaattcaactaattcaacaaataaaaggccggcagcaaagcctcagttttgccccggtccagatggatcccagaatgctatttgttggtgtaatccttgctattcatttcttctgcagcgaattccttaataaatttcaaaatggctctgaccttgtcgtccccataacggctgatccagctgtcaaagcgtttggtgatcaaatcgttgacgtgcttttcggtttgctcaccggttggagttaaatgtaaataaagtcggcggcgatcactttccgctggtttttggaaaatataatcatgctgtaatagaactttgatttggcgcgagattgcgcttcgggttactcgccgttcactggcaatatccatcaatgagacgttttgtttttcagcgattgtatgcaaaattaagtattgttcaaacgacaatccgtacttagttgcgggttcagaaacaaagttatctaagtatttaagtgacgacaaataaacgtcgattgcttcttttaatagatcctgatttgttttactcatatctgtcaccattcccctttaattattaaaccttatatcaccttaattatatattttagtaaccagtgtcgcaactaaatggattaactttatcgttttatggcattatgctttataattatgacataacaaaaaaggattgatatttatggctgatgatgcaatttcactaattcaccaagtagaactggatcttttcaaacaatttgccaaaatcacccaccaacaccacatccattacattgctttgggtgggacaatgctgggggctgttcgccatcaggggttcattccctgggacgatgatatggacgtcggcatgctgcgggtagattacgagcaatttttgaaagtggctgagaaagaccttaaagggactcactattttcttcaaaccccatggacggacgagaattacgctctgagctattccaaactattggataggaataccttcattgaggagaagaacaacgttaacaacgcccggaaaggcgttttcctggacatcttccccttggatcgaattccagactctcctgcccgtcaacggcggcaaattttggacatgcgaagactcgacagccgaatttatttgaaactgcgttataacgtgatcgataatccaattcgcaagtttcatgcctccctttctgccgagcaggcagagacggcagaagatttcaaaaaacaacgcgaaagcgtcatgaccatgtataacgacaaagcggcgttaatgaacgtcaagaatctcgcctcacaatatgcctatgaaaaagaaattctgagcctggaccaactaaatgatacgattgtgttgccatttgaggacacttatattcgggtcccagctgactacgatggcatcttgaccaagatctatggcgattatatgacgctgccgccggaaaatgcccgaactgaaaagcacattgtccgtttaatcactgataatcaagagtttgaactctaactaattacttgcgttgacttgattaatttggtaggttacatatgacaagcaatgcagaaatgaaggtgttatgaatgtttaatcccaatgaatcccgattcgccagctacacgatcgtttcatcattacccgatgaggcaattgataacgtttggtacatcatctataacgacctgcaaggcgttttccaattatcaaatctgatcacatttaatttagttaataacgatggcaatttgtcctatgatttcattcaaggaaatgaattggtggcaacttttgattcaccatatccttacgacaatggttatccaaaatccctggtcgtctatgacagtggtgaccggcaaatcattgcgaccccatctgaaatcaacttataaagttactttgcgtgttgtaagacctgaccggaagttttttcggttaggtctttttgaatgccctgagaaaatcattccacttaagggacattggttagattaaagattaaataaccagacttccaaatgaaaaaatgataaaaagaaaagagcaggcaaattgcctactctttgtgtaactgctccggctgggttcgaaccagcgacctcttgattaacagtcaattattctaccactgaactacggagcaaaaatatttacttaacgaccacttagataatatatcatatctaagagtgactgacaactacaaaattgcataaaaaaagattttgggggatcaacagaccccggaagatctttactgctccggctgggttcgaaccagcgacctcttgattaacagtcaattattctaccactgaactacggagcaaaaatattttctttaaaaacgacatatatatttatatcatatccagcgaaaatatgcaaactattttatcatctaaatttcatcaatccactaactaatgtgattttctttaagaatgatgtcgactcctttctgcatttccggggttttgtgccattcttcaaagtgatccatatcttcagtcggcatcgtataattttcgttaatatattgctcatatttggccacgtgaggagaatgtgggatattaagctgtaagatcctgacctgcttaataaaacctcgctcagctgccaattctgcccgaccattctgcaccatattgctgatctcaatatacttgctgccatcgtttctggtaatttcttcaattagtgtcaatacttcatgactcttcaacgtgtgacctccccttatttactcacgaagaacattatacataaaaaaactgacgttataaagacgtcagttttttaagagagaaagagaattgattagaaggtatttatttagtacccgaacataatatactcaatattgaaagcgctgtcaactaaatttcgaaaaaaggttgccaaacaatcgtctggcaacctgaaagtcattctttacccggcagatgaagcgtgtgcgatggatgaacaatcgcagaaggattattaatcacgtgctcgactgaatggccggaaacgttaaccaagcagaagaagaccaccacaatcaacacagcccaggtcaataattgattccaaactgacattttttcgctaatgaccgagccgtaaaaacgtttatgaatcttagcgggaacatccttctcatccgggtgagcattttgttcctgttcagtgatttgcttttggtaatttttaatgctgaaatttttctgaacactcttgcgttcagtttcaaacttatgtttttcttttttgcttaacttcttaaaccactgcgtgaactcgcgatacttctgggtgacttctttagtgtcaccaaccattttgagttcaccatagttgatccaagcaaccttgtcacacaacatttcaatctgtttgagagaatggctgacaaagataatcgtcttgccttcctgcttaaattcggtaattttatcgacacacttttggtagaatgtatcatcaccaacggataaggcttcatcaatgatcaaaatgtccgggttaatgtggacggcaatcgcaaacccaagccgggagcgcataccacttgaataactcttaaccggctggtcaacaaaatcgccgatatcggcaaacgcaatgatatcaggcattaattcgtcaatttcttcattggttaacccttgcatcaaggatttcagacggatgttttcacggcctgtcaaactgctcctcaagccggcgtgaattgccacaatcgaagtttccccgcgaacgtcaacataaccggtggtttgggggataattccggaaatgatattggaaatcgtcgattttccggacccgttaactccgatgaggccaagggtttctcctggtttaaccgtcagagagacccccattaatgaccaaaaatgaggaacctgttttttggtaatcgaaaagaatgagcgtaatttttcagactgcgtcttgaataattcatactctttggtaacattttcaacttttactttataatcgttttccattgctccgctcctaatttaagagagactaaattcacgagtaacattataacaaactttgcaactgaaaaaaggattcccaaataaactttgcgaacccttaaacatctaacggcgaacaacgtgctgcaaaggcaaactattaaattggatcacggcgtcgccttgattgatggcgactgctcccttgtcgttaaaaacaaagttgggaataatccgctttggaatactgttaattttggaacgtgaattttctgctcgaattaaagctgattttttggagtcaccagctaattgcttgttgaaagaggcatcaattttagaaccaatgtccccggtgctgacagatccatcaagtttgtttaaatcatacttggtgataattgcatttaatttattaccgtaattcatatcagtggcataagttaatgacagtgccatggcggcatcactggaagaaatggcgttcgtcgtccaggtgccctcataataatttggatcggacaatgtcccgtggcgtaacagataagcattatctttgattgaggcttcaacgcttggatattttttaaaagccgccgcagtcatataatgctttcccttggaggtatattccccggtactcatagtcacagattggccattataagcgcctttaaccccgaagtaattgttggcgtccaatgatagctcggaacggccaaagtcgctctcaacgattgcctgggccatcatcacggatggatagagatggttagccttactaatcttcaccaccggcgttttcagctgattaatgaagtcggtttccacgctggcatgcgagtggtttgcttggacaaaacaaaagccggtaaccgcaaccgtggcgattagggctttcatcatgacatgtttgaattgcttaatgatgctaaaaacctcccaataccgatgttacgacgaatggtcaacaacatcggctgtttccatattcaattatgataaaaaggcactggaaacccaatatttggttgaagaattaggcgttgagattcgataccaaagtgaatggtcgctgaccttatagccaattttatcgactgtcaccttagtgccaacttgtaaatcaacctgattgagcttgtaatgcttctgcaaattccccgtcgagtttgcatgatcgtacaaataagtcgaattggcattcttagaaatcgacttggtctccttgtggttcacaaccgcaaccgatccaggatatgatactacatctgaagctttaatccaaccctttgtcttgccgtccgcaatccgataccagagaaccagccccttggtggtcttttgaagcgcggttttgttaacgttgtaacctttgttggcggccgcaatcgtctttacctttttaaccggttttgacagatagctggaacccacaatgtggttatagatgtaccccgaggaagttttacttggcgttaacgcaccagttgccgttccagaataggtcgtggcaaatgacaatgccggagcactaacccagaactttttggctttggcattgctatagaagcgtagacggtaccagttagttgagctgttagtcttgactccgcgcatatccaggtagacttgaacccgactgttaacacccagctgtgaccaagtataacgtttctcagaggtggttgaccccttcacatgattatatacgtaatatttcttgtatttactggaaagtggtaccaaatctttgcctgaggctttgtagtatttaactttggcaagttttggtgctgtaggcgtcgaagtcgtggcagacgaagcagttgttgagctggcacttgaactgcttgctgttgaactcgatgctgcagatgatgacgaagcagaggtcgacgatgatgctgacgacccatccccggtctcgccaaacagctgatccaaattataggtttggataactgtaatcaacgactgaccatatcccggcgctgtcgcatatttaccagtcaaggcatttgcagcgtcctgatacgttgccgcgttctctttccaagaaccggaataatacttggggttccagctggtgccgtttcttaaagtggacccattgtcggcaaaagaagcgtacgcggttggatactttttaaaattggcagtggtattaatcatctgaccattgctattatattcggtcgtcggcatcgaaaccgaggcaccgttgtaagcgcctttaattccaaagaaattattggcttcgatcgtcagctgactttgcccccagccgctttccaatccggcctgagccatcatgaccgacccgtataagttgtacttcgatgaagctttggtaacgtcatttttatattttgagataaaactgcttgctgtggaagcataagcttgttggtatgtactttgggcagaaaatgctgtgaataaaacccccatccccgtaacaagtaaggcagttagtccatgcttaattattttattcaatgatccacacctccgtttaggccacatccctatcatattagataacagagaaaaaatgaagccctaaatagaattaattagccaaagaagctttagactttcttaataactttaacaactcttataatatatcattttctgtttgaaaacaaaaaaagaaactaccattttgagatatcaagaaagtttttggacaatgtctggatttgtccagtatgtgtctgtttcatggcatgcctcatcaaaaaatgattgataaacaaaaaggacaagcattctctgcctgtcctctatagaaacgctattcaaatttactcaacagtgacactcttagccaagttacgtggacgatcaacatccagtcccttgttcaaacttgtataataagcaatcagttgtgcagggaccacgctgagcagcggtgtgatcaactcattgacgtctggaatgatcaaagtatcatcttcctcggccaaacccttacgaacgatggtaaaggttgccgcaccccgtgattcagtttcctgcaaattgctgcgggttaaattagcggttcgtttttgcgtaatgattccgacaaccggcgtcccttcttcaatcagggcaatcgtgccgtgcttcaattcaccggatgcaaagccttctgcctgaacatatgaaatttctttcagcttcaaggcagactccaatgaaacggtttggtcaattccccgcccaatatagaaggcccggttagctggaacaaaatactttttagcgagatcatcgatgacatctttctcatcaataattgcctgcatcccggttgcgaccaatcctaattgctggcgaatatcaaactcttcggcgatcgtttgctctttggcttcacccaacgccttggcaagaatcgcttcaaccccaatttgcgcggtgtaagccttcgttgaggccacagagatctcagggccggcgtgcagtagcatcgtgtaagttgcttcgcggaagagcgttgaattttcaacgttggtaatcgtcaagctctcatagttattggcattgacgttcactaaaacttcacgactgtcggcagtttcaccactttgtgacaggaagataaagaatggcttcttggacaacagcggattgtcataggcaaattcagaagcaatgtgaacttcggttggcacatgggctaacttttcgaataatttctttccgacgagtccggcatggtaactggttccggcacccacaatgtacaaacgatcggcttccttcattgcattgatcaattgtgaatcaacgtttggcttgccggattcttcagtgtaaagggaggccaatttccgcatcacgtttggctgctcgtcaatttcttttaacatatagtaaggatatggtcctttatcagtctcttgagcatccatgtcaacatggaaagtgtcccgctgaaccttgtggccgtcacggtcttcaatgtcaactgaatcaggcttaattgtcaccacttcaccgtcatgtaattcaaggaagtcatgggtcacattcagcatggccaaagcgtccgagcagaccacgttgcagccgtcaccaaccccgatcaaaagtgggctcttgttcttggcaacgtacaaagtttcaggatctgtgctgtcaatcaataagaaggcatatgaagatccctcaagtaaactcaaagtcttcaagaaggcttccttagtcgtcatcccctctgtttgaacaaatcgatcaaccaattgaacaaccacttcagtatcggtttgactggtaaaggtggtgttgctcaagtacttggcttttaattccttgtagttttcgatgaccccattgtgaaccaagtaaaaacggtggtcttcagaatattgtggatgggcattgtcaacgctcacaaccccatgggtagcccagcgggtgtggccgattccgacagaaccgtgaacttccggtccaacggcagcttcgagttcggagatgcggcccttacgcttcaccagatagtcgttgccatttaaatcgttgacataaataccagcggaatcataaccacgatattcaagtttttcaagcccttccaataaaattgaaacagcattatcatttccagttactccaactattccacacattttagtattctcctcaaatttcataaattggtatatacagaatatgaactctatatatttatataacacgtataatctacctaacttcgagataaaagtcaacaaaagatgtcaaatggtataccaaatcttaaaaattgatatatcaactttggcagttgagaagagaccaaaataaaaagatgttgcagtaaactttcgttttacttacaacatctgcttaaaatcatatttaaataaatgattctctgaaaaaatgtctaaactattcaattcccatttcgtcacgaacaacatctgcaatccgtttggtgtaatcatcaaccaaatcttgtgttggtgcttcggtcatgactcgaagtaggggttcggtcccactgggacgaaccaagacgcggccatcaccatgcatttcttcttcaacttgggcgatcacgtctttaaccttgtcattgtccaaagcgtgtttcttatcggctactttaacgttaatcaagcgttgcggatattttttgatctcgccggccagttcagacaatttcttaccggtggctttcatgactgataatagttgcaaactggtcagcatgccgtctccggtggtgttgaaatccaagaagatgatgtgaccggactgctcgccacccaaattgtagccgtcctgattcattttttcgacgacgtaacggtccccaacctgggtcttcacgctggtcatcccttcacgttccatcgccttatacatccccatattactcatgacggtcgtcacaatggtattcttcttcaagcggccacgttcagccatgtatttaccgcaaatgtacatgatagcatcaccatcaaccaacttaccgttctcatcaactgcgatacaacggtcaccgtcgccatcaaaggcaattccagcggaaacccctttatccaagacaaacttctgcagctgctccggatgagttgatccaacatgatcgttgatattaaggccgtctggattagtggctagcgtttcaaattcaatgcccaaatcggcgtacaatgtggtgaccagcttgctggtggaaccattggcagcgtccacggcaaccttcatgccggaaaggtcctcagaaattgtctgctcaaggaaatgaatatacttttgactaccttcaagataatccccaacgactcccaagccatcggcggctgggcggggcagaatgtcttctggcctttccaggatgccctcaatctcttcttccagttcgtcggacaatttgtaaccatcggcaccgaagaacttgataccattatattcaaccgggttgtgtgaagccgtaatcatgacaccagcatcagcttcctgatttctaaccaggtaagcaactccgggtgtcgtgacgattcccaggttcaacacttcaattccgaccgaaagcaggccggcaaccaaggcttcttcaagcatctgcccggaaattcgggtgtctcgtgcaaccaaaacctgaggctgtttacgttctgaatggtgggtcagcacataaccgccggctcggccgcacttaaaggccaactcaggggttaattctttgttcgcgataccgcgaacgccgtcagtaccaaaatacttcatgttaaaaattcctcatttcagtttaaatattttaaatatttgttagttatttctggtgattttgaccgaaatccgctctggatcaaatcctttaacgtcgtttaatttaggatccaacgtcacctgcttggtcttagtcttggtgacatcgctggtgtcgacttcgactttgacagaggccagcttggccaactccgccttggtcccaaatacccgaacccgcttggttgccgaagtcagcgtaaagctctcgttgtcatcagtgacaccctttggttccagtttgatcggcaattctttactattgcccggcgtgattggtaacgtgacatctgcggtagccggggtaatcaccacgttaaccgtgttttgtttggcgtcgagggcttcaataattgcctgactggaaattgatgacttggcattttgcggaacgttaagctgagcgacaaccgacttaatccggttaatctgatctgacgcaccggtaatcttgacgttcttcacatcagcgttggcctcgcctgcctgatatcccgaagcaatatttcgttgagagtatttaacggtcaatggatacgaaacagtttcccgcggctgaatatcaaccttaattgtagctggttcgaagcgatatctcaaatcattatttaaaccgtcctgctgaatcctgacggtatgtgtccccactcccaatttggagaggtccgcgtaggctttaaagttttgtgtattcgcagtggtggtcaccaacgcggatgggccggtgagatgaactttgaccttctgcggataaccggtcacaaaatatttgttactattcacggttaaagaaagcggaactgaaaatgtctgggtccggtttgaggtcagtgaggttgaattggtgttgccggactgattgctggttgtgctggattgggtactgccaacatacatgaataacaggatggcaaagaacagcgacagcaaacgatatgcccagttttttaagagccattgtcgcatattaccgtccccctttgaaatgcttgtcaataaagccggataccgtactaagaaatgtccggtgggtctgatcatcttcatcggtaaacaattgatctttgaagtatttcaggtagtcatcccgtgtcatcccacggagtaattcgttattttgagtgattgacacctcaccggtctcttctgaaataaccactgtcatcgcatctgtcaactccgagattccaacggccgcccggtgacgcgtccctaattccttggggatcaggttactttgagaaagcggtaagtaagctgcggcagcggccacccggttattcttaatgatgacagccccatcgtggagtggggtgttcgggatgaaaatgttgattaacaattcaccactcacatcagcgtccaacgcaattccagtctcaatatattcttccagacctgtattcatctgtaaggtaatcaaggccccaattcgccgtttggacatatattgaattgcccgatccaaagcggtgatcatcttttgagcatcttcgttttccttgcgccctttgacaaaaatggacccacggccaaggtgttccaggccccgacgaatttccggttggaaaatgacgatcagcccaataacaccccaattaatcacctgatccatgatccaagacaaagtggagagcccagtataagcactaataattttaaccaccaagatcaggacaatcccgcgcaaaagctggactgccttggtatctcggacaatcaaaagtaaattataaattagaaaccaaacggccaaaatatcaatcaggctcgtcaagttatgtatcgtaaaaatatctgaccagttcattacgctctcccctaattagttttcagaaatattatatcattgtcgcctgtcaaactgataatcgattaaaatttgtgacgatgtttaaataaaacattaaaaatgaccggatcgatcaagtattgatggtatttcttcgcgaaaaatagtttaattatatattgatagggggttttaacgtgaacgcaaaaacaaaatggctggtccgggcactctttctggtctggatcgccctactatattcatatttaaaacaacccccgtttaactttttagtgttaaatacgtttctggcatttattccaattgaactcagcttccacattgacgttggcaaacccaaaaacggcctgctgttttgggtgctgatcatcgtctggctgttgttttatccaaataccccctacctgctgacagatttattccacttatcgctattgaatccttatggtgtcaacggattgctaagacttgacgatgtgatgtggttcaagtttgcgctgctattgatttcaaccattttctcaactttggtcgggctttggggcttggataaggttggcgatgcgattacagccaggttccatgcccacaatctgttggtcaaacacgccgtcattgtggcgctcaccattctggcatcaatcgggatcttcattggccgtttcttgcggattcacacgatttacttgttcttaaccccggaattatttatcagaccgttattgaacatgtggagccgaccggcaattgtgtttattgttttattaacggcagttcaactggtattctactacacactcaaactcattcaaaaaccacaatcaaaataaatgggatgctaccgtaattcgacggttcatccctttttatttgcctcaatatcaatccgtcacgaacttttctctaaaccgcgcaacataatcgctgggcagatccaacccatttttcaaatacccatcaaacgagccaaagtgttccagcaaaacatcgttggcgtggcgtaaataatcggcatcaaccagcaaggctgtgtgcaggttgtccaattgctgctgattcatttcatttttgaaccggttgagcaaatcttcattggccttgacccgcagttgattagtcagcagataatcatccataatttgttgatcgtcagcgccagccacctttaaaatcacggccgctgcaaagccggttcggtcttttccagcgaagcaatgaaataggatcggtgcatcatctgccagcaagtccgtcatgaaatcatgatacccctgttgggcagactgacttaaaacaattgattcataagttttaagcatattctcatgaaccttgttgccgtcggtaatcatcgcccccagactagccccattggacgttttatcagacaaaatatcaatatggtaatatttggcaccagaaatcgcactatccggtgcttgtttgacttcatccgtacttctaaagtcgtaaacatcccggatccggcactggtcttgcaggaaggccgtttgttcctggctgatcccagcaatttgaccgcttctaaaaaagtatcctgactgcaatttccctgaaggaactctgattccgccgatgtctctgaagttcactaaccctttgtcattcatttgaagtccccctactcgttttgataatccataatcaaaactgtttcagaatagttaatatattgtcttaagtgggcagccatcgaccagtcaatattgccttgttcgaggagcacctgcacgccttcacgttcggcagccaaggccttaattctcaagctctggtagttcatcgcctgatcattgatctgctttttggaatgatccttggccagctcaatctgatttcgataatgcacaattaaatgataaaccgactgactgtcaaaccgttgattgtcaatatcgtcacgggcaaagtagtcggataatgctgagatagccgccttcgcctgttcccgttgaatcagggccagctcatcggaaatatcttcattcgttttgcgccgaatcaaccacaaggagacgcgattccgcagtttaatgaaattccgcgcggtcccatgcccaagtttgactttccgaccaaccgagcggatcatccgattttctaaacgctgcagtttggcactggcaatcaagaaggcctgtttggaaattttttggtcgtcgaataatttctgcactgcggcccgttcaccacgaagcgcaacccttcgaagtgccaattcatcagcaatgatggagtccatttcttttttatcttggagttttaattccagccttcgaatcagaaactgataatcgagaattaagtcaaaagcctctttttgattattgggccgccgttcttcttcaattcgttgaactgccaatttcatgatatagacgcgggcctcatcttcagaaatgtattccgcatcgctgtcggccgaactggtatcaatttcatccggatcatcggttgagttggctcgggtcaacagtggtgccttatcttcagaaatcagtggcaaggtgacggtggccacgaccagtgaaatgatgatcactcccgcagcaacgaataacgccagtgatctggacggaaacggactgccattatcaatcgtcatgggaatcgataaaactccggccatggtaacggccccccgaacgccagacaatcctgccaacagcgccgccttaaaggtgggcatttgcttggtttgaattgatttgatttttcgggagcgaatactgctgaccgcttggtaggcgtagatccagacaactcgaatggccaagagaatcagccaggctagaaaagaaattcccagtgcagcaaaggtattaatcttgttattttgaatcacattggtggttgctaacggcagttcaatccccagaattaagaagacaatcccgtttaaggtatagataataatgtcccaggttttttcactgaccaatttgagctcaggttgactgcgatccggtgccgttccgtaaaagtggaagatgatcccggcggcaaccaccgcaattacaccagaagcatgcaagaattcttcggtcaccaggtacaccacgaaaggcgttgtgacctgcaggaccgtgctaaaaatgacatcgttgattccctgtcgatacagccagttttcaatcatcaaaatcagccccataatgaccagaccgctgacgaagcccataatactgatataaacaaagtcaatggcggccgttttaatggagaaaacgccggtgaccgtggctgcaattgcatatttaaaggcaatcaggccgctggcatcattgatcaggctttcgccactgacaatgtgtaaaattccttccggaagctttgcccgtttggaaatcgactgcacggcaaccgggtcggtcggcgacaggatcgctgccagcgcaaaactgaccgaaaacggcatagttggaataattaagtgaaacagcaagccgcctaaaattgtcgtcaaaaaaaccaatacaattgcattggccaatattggtccccgcaacttccacaactcctgcttggggaacctgcgcccgtcgttaaacagcaacggcgcgataaataataacaggaaccaatcagtttcaagcggaatggtcacccgcatcattaaagcggctcccagtcccaaaacaacttgaattaaactaaccggaaccgctggaacaaaatggtcaacaacgttggaaaaaacaaccaacgtcattaacagaatgaccgcttcaagaatgtgcacgcattaccaactcctagtttgacttggggtcttcaccaataattctgacttccgtctccagatgcacgccgaatttgtcgtaaacggtcttttgaacatgggcgatgacgtttaaataatcagtggcagtggcaccatcgacattaacgataaagccggcatgtttcattgaaacctgagcgccgccgatctggaagccttgaagtccggcatcatgaatcagtttaccagcaaaatagccggttggccgtttgaagacacttccacaggacggcagttccaacggctgtttagaggcccgcagagcattgagatgatccatccgcttttgaattttgtcggcaatgccgacttccaaagagaaggtcgccgaaatgacgatttgctggttttcttggacgctgcaatgccgataaccgaaatccagttcttgatgattcaagtgaataatgtggttgtcgggtgtcaagacttcagccccactgacaacgttggcgatctcaccgccataagcaccggcgttcatgaacaccgctccaccaacgcttccggggatccccgctgcgaactccaagtgagttaacgaatgggcttgggcagccttggtcacgtcaatcaaggcagctccggcatccgcgacgacctcattttcatgtgacgaaatccggttcattttggtcagaatcattgtcaggccacgaatgccgccgtctttgacgattaagttgctggcattgccaaccacagtgaccgggagcgattgctcgttggcataatccagcatttcttgacattctttaatcgatttaggaaaggcaagaatatctgccggaccgccagtcaatgtgtgggtgtatttggataaaggttcatttatcaaaatctcaattttgggatataaatctacaacagtttttgattgcatcatttttcaattcctcggtttcaaaacatatacattaattttaccacgaaacaagttatctatggggcggaatagccggaaagcactccggttgcgttttcacggggttctttgtacaatgtgattaacttgaggtgaaaaatatgaattttgttgcgatggattttgaaaccgcaaacgcaaaaagagccagcgcatgttcaattgccctggccatcgttcgggataatcaaattaccaatgaattttattcattaatcaatccggaaatggactttagttggcgaaatatcaacgtccatggcattcatgaacgtgatgttgtcgatgccccgacctttccggaagtttggcgccacattcagccgctgttttcagccaataaattggtgattgcccacaatgcatcatttgataacagcgtcttgaaacgaacactggaacgttatgaagttcaaccgccgcactacctgacactggacacgttaaggacctccaagcaattctacccgacgttggaaaatcacaaacttaacaccctttgcgataagctcaacatcgttttgaaacatcaccataacgcgctggacgatagtgttgcctgtgccaatattctattaaccgaacaggcccaatttggcagtgaaatgctgcggccatttgtcaaagcaatctaaagagattggaacgaacttagtttcatcccagcattcaacaaaataacgcaaccattccaagattagggatggttgcgttatttcattaagtgcctgagatcaaccagtcatcacgtccgtttaataaaaaagtggcggtcttagttgcaataagcaaccacgtcactcaaggcttcaatccttttttgggacatccaaggccattctcacaacttcacgaccgtcttgaaagtacacgtcggtatcgtgaaagccaactttgtaataaacatgaatggccggctcattcttcgagaaaacagtcagcaccagttgatcaagcgagctaaaatctgttgcccagtcaatggccagttccatcaagttggtgccaatcgagtaaccttggtaacccgccagcacagccacgccgacttcaccggccccattatcgatactgtcaacggtcacaatcccaatcaattcggagccataggtggcaaccgccatcaaattggtccgagagtgattgatcaaattaatttgttgggcttcgtcggctgcggtaatgtcatccaaatcagaatcgaccaaaaacgtatcggactcgccttgaagaaccttcaacaaatccaaaattgcctgaccgtcactcggttctgctaaccgaaagtctacttcttctgccacatcattgctcgctttccactgttattctgaaaatatatcatcaattagttgttcaaaacggtgcccggtggcttcaaaagtcagcgttctcacgttgtcgccctcagaatcatcccgccgaaaaataatccgaagatagtcatccggtagttcgtcggcaacaaactttgaccattcgaccacgttgaccccgtcgccattaaaatattcttccaagcccagatcatcgccaccgccttcttcaagtcggtacacatccatgtgatacagcggaattcggccgtcttgatattcgcgaataatggtaaatgtgggactcttgattggtcgcgtaatccccaatcctttggcaagtcctttggtaaaggtggtcttcccagctcccaaatcaccatcgagcaaaatcaaatcttgtggcgccaagtatgcggacaatttttcaccgatcgccatggtttgatctgctgagtgaacagttatcgtcttcgtcaattaatcacctcattcaaaaaggaaggattgcgacgcaacaaccaccgcaatcctaccctgtttaattatttctattataatgcttgagccgctgtgatgatagcaactttataaacgtcttcttcattgctgcctcgtgacaggtcggaaaccggtttgttcaatccttgaagaattggaccaatggcttcaaaaccaccgaagcgttgggcaatcttgtagccaatgttgcctgattgtaattcagggaaaacaaagaccgtagctttaccggcaacttttgaacccggtgccttcttctcggcaaccgttgggacaaatgcggcatcaaactgcatttcaccatcgattgccatatcaggtgcctgttcttgagctaatttggttgcctcttgaactttggtgaccatatcacccttggcagagcctttggtcgagaagctcaacagcgccactttagggtcaatatcgaaggtcttggcaaccttgccgctttcaacggcaatttctgccagggcattggcatctgggtccaagttgatagcacaatcggcaaataagtatcgttcgtcacccttttgcataatgaaagcaccactgattaatttaacgccgggcttggtcttaatgatttgtagagctggacgaaccgtgtcgccagttggatgattggcacctgaaaccatcccgttgattttgttcatgtagaccaatgtggttccaaagtaatttggatccttcagccaatcgcgcgccttggcctcatcggtcttgcccttacgacgttccacgatagctgcaaccatttcatcgatttgatccgctggttggttcaggtagtcgataatttcaacgttccccaaatcaatgtcagcgtctttagcaactttttcaacggtgtctttagcccccagaatcactggattaaccagtccgtcctttgccagacggctggcggcaccaaggattcggacatcgtcaccctctgggaaaacgatactaatgtttttgcccttgatcttttgcttaagactttcaaataattccatgataaatcctccaattctacaaaatcagtctaagatgtttgcgataccttttccggcagctgccagttaatcggctcctcgcccattgcttccagtgcttcattggtctttgaaaatggttttgaaccaaagaatcctcgatgagcagacaacggactgggatgggccgattgaatcaccacgttggttttcgtatcaatcaacgcaattttatcccgggcagctctcccccacagaataaagacaacgggcttctcacgagcggacagtttttggatcgccgcatcagtcagttgctcccaacccttccctttgtgggaaaaggcctgaccattgcgaacggtcaaaactgaattcagcagtaatacgccctgtttggcccagctttccaaatcaccgtgttcaaccggtttgattccgaggtcagactgaagctccttataaatattctgaagtgacggcggaattttaacgcccggcatgacagaaaaactcaatccctgggcttgatgaggctcatgatagggatcctgtcccaaaatcacgaccttcaccttgctgaaaggagtcagctgaaacgcctcaaaaatgtgattcatatcaggatgaatatattgcgtcttgtattctgatatcaaaaattggcgtaactgctgataataagttttctcgaattcgggctttaaaacatcccaccagtcattttttataaacggtttcattcccaacacctcacgttttattctaccataccatttttaaaataacaccagcgtaaataatttcagaacgtgttaaaatgaaaataatacaagtaaaggaaatgcgtctatgagtcgaaaattacagttgaatttaaccgaactggatcacacccgttcgactaaggtcaccgatcaatatcgagacacaaaatatttaattgtcggcaagtggggcttgattgacgacactttttcaatttactcaatttcaggtgaagtcgtggcaaccgtccgtcaacaatctctgggcatgacgcctaaatttgatttgtattacctggaccaatttgtgggcggttccgtgatccattttacgatgcactacacaacgatttttatcaacggcattaattggttggttgccggtaaccaggacaaacaaacttaccgaatcatgcacggacgccagcggattgcgacaatcaagtcatacagtcagtccgatcaagtcattcggatcatggatgtagacaataccaatcatgaaccattggtgcttgccattgcggctattctcaatcatccctcgttggcacatgcttcccgattgaagttgggtgttttgaataaagcacccgtcaaaccaaatcttgaaagtgaaaacatttcgaccctccacaatgaaaataagcgatgaatcagtcggcagcttgccaattgatttcatcgctttttgtttgagcttgattaataatgtttcataactcgttcaatttgacgcttttgatcacgtcgcttgatggtttcacgcttatcgtactcatgcttaccggttgctaccccaattaaaactttggcaaaaccatttttgaggtagacctttaaaggaacgattgtgacccctttgtcttgggtaatttgagccaatttgcgaatttgctttttgtgcagcaacaactttcgattgcgcagcggatcatgattaaattggttcccctcagcgtactcactgatgtgaacgttcatcatgtaggcctcatcgtttcgaatttgaacaaagccatcctttaggttaattcgccgagcacgaatcgatttaatttcggtacctgtcagcacaattccagcttcgtaggtttcggaaatcgaataatcatgacgagcttttttattttgcgccatcaaattatcgttattatgctgctttttgcctttggccatcaaatcacctcgcttacagcttaatgtttattatggttccgatgtccgttgttgccatggttgtttctcccacggttgttgttggcgtgattggaacgggaattgttattcgaattgccgtggcgctcattattgccatggtagttattattatgataagtccgctttggcaacatgttactttgtggcgtcttttcaggatcaacaatatcaaagtcaacggcactctgcttgacgtcaacattgaccactttaactcggattgcctgacccatcttgtaggttcgccgagtatttcgaccaaccaaggccataaattgttccacgtattgatagtagtcatcattcattcggctgatgtgaaccaagccttcaaccgtatttggcaactcaatgaacagaccaaatttcataactgaactgacaaccccatcgaattcttcgccgatgtgatcgttcatatattcagctttcttcattgaatcggtatcacgttcggcatcaacggcccgacgttcgtattgagaagtcgtcgtcgcaatttcatccaacacgttggcataacgtttcttggtctcatcgttaatcccgttatcttgataataatgaatcaatcgatgaaccattgtatctggataacgccgaattggcgatgtgaaatgggtatagaacggtgctgccaacccaaagtgtcccaaagactgatcggcgtaacgagcctgcttcaaactccgcagcagcatcactgaaaccatcatttcttcaggcttgccggcaacttttttcaagacattttgtaaagtctttggggtcacatgctctggatcacccttcacattaatcccgaatgcagtcaacgtctcaaagaaggttctgatccgatcggcatccggcgtttcatggacccggtaaataaagggaacgtgtttttcatagtagtgcttggcaaccgtttcgttcgcggccagcatgaatgattcaatcatccgctcggcagtaccacgaacccgcagcttaatatcgattgggtggcctttgtcatccacgataatttctgcttcgttatcgtcgaagtcaattgccccacgcgcttttcgatgcttgtataaaattttgtgcagctcacccatggtttcaaacatgggaaccaatttatcgtaacggtccatggttttttgatcgtgggattccaaaatgttgttaaccgctgtgtaggtcattcgggcggttgaacgcatcaaactcgggtgaatccgatgcttgatgatattgccggatggatcaatctccatttcacaactcatacataatcgtaattcgccttcgttcagcgaacagattccgttggataaacgtcttggcagcattggaatcacacggtcagtcagataaacggaagtcccacgacggaatgcttctttgtcaatggcgctgccgggttgaacataatggctcacgtcagcgatatgaacccctaaatgataattgccattggggagtttccaagcggtaaccgcatcgtccaaatctttagaagattccccgtcgatggtcaccaaatcctgatcagtaatatcttctcggccaatcttctcggcttcagtcacgtgatctgggatggcatctgcagcctgaatgacatcttcagggaactcagcgggaatatcatgggcataaacaatctgtaaaatgtcaattcctgggtcatcaactgatccaataacttcatcggcaatccccaccatgtaatcagggtgcttggtagatgggtattcggtgatttgagcagtgatcacttcaccaggtgttggcttcagcccgacgtcgttgatataaaatttgtacttggcaattttcttatcgttgagggttaattgaccaatgtatcctttgtcatcatcagtcttttcaaacggtccaaccacgcgggtatatttgtgttcggcaattttagtgactttgccttccgggccccgatcggatcccggttgtgcaggccggacgatttccatttccacagtatcaccattcagtgcattcatggtgttatcgggcgcaatgtaagcatctggagcattttcatcataagtgacgaaaccaaaccctttgtcattagcgtggaaaataccacttaattgttgtttatcaggattcaattgaaacttgccgtcttcagtcacaacggcgactttatcgcgttccaaagaagccaattcttgaacaatcagcttaaaggctgctgaaccatgcgatctcaggacgtcagcaattttctcgacagtaaacacgttatccggataggttcggagaacgttttctatttgatttttcaaatcattatcttgcaatctatattcctcttattattcataaagttgtgttaaaaattcggttaaatcagcctcaagctgcttgtgagcaggattaacggtaatcatgtgactggcgttggggtattcgtggtaactgacccgactgttcaccaatccatccctcaaagacttggcactttcaggattcacgatctcatcgcttaacccctgaccgatgaagtatggttgggtgattttaggtaaatcctgcgccacaccaactgtgaaatcagcaatcttacctaatagtatatcaatattttcgtcaagccacttgagttttgaattcataatcgcttcattggtatcatactgaacaaaattggctttggccatttgcataaaggtattatgaacactaaactgacgctttcgaacaattggtgatccaaacgaaccgccgccgagtaaagtcggatcattctccagcgttttagcggcaaaaataccgcccagcgagatgccaaagatactgatttgggtatatcccctgtcctttagaaactggacggcccgtttggcatcgttccaccaacgctcgggcgttccctgaatcaggatatcggtaaaatcagccgtcccatggccagtaaacattggcgcatacacggtataattctgacgctccaaatacctcgcgagcattcgaacgtcaaccgggccactggcaaaagcatgcaacagaataattgctctcggtccgtgttcaaaataaaaagatttgactggtgtttgcatagcacccatcctttcatgtccacccattcaattataataaaaatccccctgcatttaaacaggaggattgaatactaatgagatgatatccaaactaatgcaagtgctaagagaaagaaaattatccctaaaacaagtgtagttttttgcatgaatgcttcaaagccacgtggcttctgctttgcaaacaagtcatcggccccaccagttaaggcggacatggcatcattagtctttgatggttgcattaacactgcgattgtaattaaaacacagtcgatcagcaataatgttaacaaaaagttgtacacgttgatagcctcctaccgttaaatcggcttaatactactcttactaaactaacacattatagcagaattcgctaccttttgggattaagtttctgttgttaaggtaataatttgctgggtgatcgcgtgctgatttttagttgagacgttgatgaacaatgtatcgccccatcgaatcaaggtgccgccagcaggcacaatttcgacaccgtttcgttgaatcttggtcagcagtgaccccattggccatttgatctgacgcaccattttgccatccatctgtgaaccggcatacacggtttccataatttcagcagttcgacccaaattcatcttggtctgaactttcaggagctgctgaagcatcgagtaatagaccggtttgccgtttaacaggtctaagacgccgtatgcgattaaagacacgaccgccaggccaaggagatgggtcagagtcccaaccatctctgtaatcaaaagaattgccgtgaaaggggccttactgattgccgcaaagtatccggccatccccataataatgaaactcgagaaatacagtggattcatcaacccaagattgacagcgatactgccgacaatcgcgccgattaaaccaccaaggcaaagaattggcaggaaaatgccgccgggaaggccactcccgtatgaaagcatcgagaaaacaaaccgaattatgaaataaagacataaaatcagagttggataatttgccgaactcaacctcagaataatgtcactcccgccacccaacaagtgcgggaaaaacgctcccattgggatcaccaacaacagcggaataattccgttgaagtaccagggaatatgagtatgccgataccactttcccatccgaagaataaccatctgatataaccggcccaacacgccaaggacaattcctaaaatgacaacccacaaaaaatatttgagtggcagtggcgtacttcgcatgtataaaaccggcttgaggccaaaaacatacgtcgcaaccatgtcagaagtgaccgcagatgtgagcgaaacaatccaaatattggtggaaaagttatgataaatctcttccaaaacaaacagcgtactggcaattggggcgttaaaagccgcacttaagccagcagcggcaccactggaaatgagcacttggcgatcaaacccaacttgtttggtgaaatgggcaactccctgccccaaagttgaccccaactgaattgagggaccttcgcgaccgagatataaaccacttccaatcgccaaaatgccaccaacaaatttccgccacagaatcgcccaccagccgtaatcaacctcacctaacaattgaccttcaacttgtggaatgccggatcctttaatatccggctgctgctttagaaaccagccaaccaataagccaatggcaacattaatgacaattgtcgtcagtagaaacgacagatgatggatcgaattgatataaagatagcgcatgaaatccgtcatatggccaattgaccaccgaaacatcgagactgccgatccggcgagtacaccaatgacgatcccgttaacgattgtttttacttgagacagcttgtaacttcctcttacctgcaattttgctcatcctttaatgatttctgatatccatcatatcataatcaaatgagtcgtttgaaaagttttttgccgattaacgcgccaagaagcaccacccccgacaaaacaccgacaacggactgcgattcaccggtttggggaagcttttctgaaacatccgaagcgtctttggcttcgttgtgtcgctttgctttggtttcagacggattccggccactgatagctgactgacgcccttttttgtggccagtctttgagctgagtgcagtcggttcagctaatggcttgtttgatttatcggctaatttgatgtaagtgaattgtacatcttcaggcatcagattgtcagccttcagttcctgggttggttgctgaacccgataacctgaaataaacttggccgtgtaagtcttggtttggccatattcaagttccactgagtctttagagatggttttgccatcctgatccacgttgataatattaaaggtgacttttttagcagtataatgcaatgtcagggttttcgaacttgcatccaggtcggtggactgtaattcatagccataaaattcgacgttctttgaccggaatgcccgggcctcttctgaagtgagatgcagggctttattgaagagtaagtggccgtgagtgtcgatcccatggagttgataggttgtggtcattggttgcttttcctgatgatcggttgatttttcgggtacctttgtctggttgatttccggaattttgggttttgtttgaacgaccggtttttctgagtcttttgaatcagattcggaagtcttaactgtgttctttgtggagccggattgatctgtggttttaccaggaaggtcggctggcttttcagacggcttcgcagacgtttttgaaattcctgcactttttcatcggggttgagtgattcggctgtggtttctaccggcttggatgatctggattttttgccggtttcggactgaacggatgatgtcgactttgcattagtcgacgaatctgcaactgcgccttcctttttgctttcaggtttagtggcaccagtctctttatcagatgatgatgacgccccattggttttagtggcgggctgggttttgggttcaggatccggcaatttggttcccggcgccgccactggtgagtttaattggccgttttcagcccctgtggcacccactaccttcacttttttatcatcatgtttggggccggacttggaagtggtagcgtccttgacttctttatcgggcgtttcggctggtttgacatccggttggtgcactggttctgtttgggtaacggatggaacgacacgattgccagcctcgctcggtgtacttggtgatggttgcatgtcagttgtcgcagtcgttgaaaccaccggcgttgaagcagactcgctcatgggcttttcactaacgagctgaattggttcgcttgtctgcccagtttcaccagacttggaattaccaggttctggctggtctggtacaaccacattagccaacttatccgcagcaatcaatggattaaggctcttatatttgagggtcacatcccagttggtctctttgatttttccgttgatatcctttgaattgagcagttcataacctgaaacgtcaaattcgtttttattaaggcggtaggtaccaaagatagttgcttgattgaaaaccttgttgtcctgaattggttggttattttcatcaaggtacttgatggtcaccacagcatcttctgccatatagttaaccaccattccgggagaataatgcacttcggaaacgaccggatggtaatgtggaacgttgtccggggcactaaaggttgacgacttactcttatcaatgtacatcttgactgtggcttgtttgtcaagcaccgacttgtcaccacggatgtttctaacttgaaactgttggtggatggtaattttgtcaggaaactcctgggtagctgtttgactggtttcagcaccaacaatctgctcatgcaccagtgggctggcgaatcccagcacgcctaacgaaactgataataaaagtgtttttttcaaaataatacctccattatttgtgatctaagagttagatacgcaaaaatggaggcgttttatgtacaaaaaaagtcgctttcacgacttttttcaaattacttgtttaagatgtcttgacgtgcttgttctgacaagttgtagaatgagtgaattcctttgtaatcggcaacgtcaccgagttggtcttcaattctcatcaattggttgtacttggcaattcgttcgccacggctcattgaaccagtcttgatttgaccggcattgaggccaacaaccaagtcagcaatcgtggtatcttcagtttcaccagaacggtgtgaaatgattgcagtgtagcctgcttctttggccatttcaacagcttcgacagtttcagtcaaagtaccaatttggttaagcttgattaagatagcattggcaacgcccatgttgatacctttcttaaggtaatcagtgttggtaacaaacaaatcatcaccaacgatttgaactttcttaccaaggcgtttagtagccatttgccaatcagcccattcgttttcatcaagaggatcctcgattgaaataactgggtatttgtcaacgatgctttcaagcaaagtcacaaattcatcagcagtgtatgacttaccgtcaccctttaaatcatatttcttagtatcggtgttgtagaattctgatgctgcacagtcaaaggcaatggcaatgtctttacctggcttgtagcctgcacgttgaatagcttcaacaaggatttcaaatggttcctcgttgttcttcaagtcaggagcaaatccaccttcatcaccaacggcagttgagtatccgcgttcattcaacaagttcttcaagttgtggaatgtttcagaactccaacgaatagcttctttgatggttggagcaccaacaggcatgatcatgaattcttggaaatcaaccttgttgttggcatgcttaccaccattgataacgttcaacattggtgttgggagcaagtgaccattgaaaccaccaaggtagttgtacaatggaacttccaattcgtcagcagcagcacgagcagcagctaatgaaacacccaagatcgcattggcacctaacttacccttgttgggggtaccgtccaattcgatcatagccttatcaatagccaattggtcagtaacatcgtagccaacaatttctttagcgatgatgttattaacgttgtcaacggctttggtaacgcccttgcccatgtaacgatccttgtcaccatcacggagttcaacagcttcgtgttcaccagttgaagcacctgaaggaacgattccacggcccattgcacctgcttcagtatacaattcaacttcaacagttgggttaccacgagagtctagaacctcacgagcataaatatcagaaataattgacatgtttttttctctccttagcgaaagttgtgaccttttgtacaaggttcaacttcaattctattagtttctcgccgaagtttcaacataaatcagcgaatttaactatttttgtaaaaagtttgcaagctttaagaatgaatccggttttaagctggcaccaccggccaaaacaccgtcgatatcagtctgtgacagaatgtcatcggcgttttcgtcgtttacactgccgccatacaaaactcggacttgatcggcaatatcatcgccatacaaatcagcaatggtttgacgaattaaataacaaccctcttcggcttcatcgctgctggcggttttgccgctgccgattgcccaactgggttcgtaagcaacaatgatcttctcagcttgttgcggggtaatcgatttaagggcgttggtcacttgactgaccacccaggaaattcgatcagcggattcacgccggctcatcgtttcatcacagcagatgattggtgttaattggttgcgaaaagcagcgtgaacctttttattaataatgtcgtcggtttcgttaaagtacttacgacgctctgaatgaccaataataacgtgggtcacgcccatttcggcaagcgctttggggctggtctccccggtgtatgcgccctcgtcttcataaaaacaattttcagcggagataatcagtggtgaatcaccattttcttcgaccatgctctccaaaaagagtggcgaagccgcaatacaggtctcagttatcttaggatcgggtaatttaccctcgatggcttgaagaaatttgactgcttcagcgactgataaattcattttccagttacccgcaacgaacggaattctcataagaatcatcctttacattttttagcttaatgccattgtaaccaaaagagaatttaaaagccacatttttctcctataccaatttttagtaaaagaaaaagagctcgctaaatagcaagctcttcgtcaattatttgttgtcaattgctgcaataccagggagtgttttaccttcaagatattgaagtgaagcaccaccaccagttgaaatgtgggtcaatttgtcagcaacgcctaattgtttgacagcggcagttgaatcaccaccaccaacaattgtagtcgcatcgtttaacgttccaaggaacttaccaatgcgaagggttccttgggcgtagttaggcatttcaaagacacccatcggtccgttccaaacaacggtcttagcatctttaagaacattttcaaagtcttcaattgacttaggaccaatgtccaaagccatccagccgtcatcaatgtcaccggcaacaactttgtgttctgcgtcgttcttaaattctttagcaaccacgttgtcagttgggagaacgatcttgtcgccacccttttcaaggatcttcttggcaacatcaatcttgtctttttcgatcaatgagtcaccaatcttgattcctttggctgcatagaatgtgtaagtcattccaccaccgatgatgatcttgtctgccttatcgagcagattgtcaatcacaccgatcttatcagaaactttggcaccaccgagaatagcaacaaatgggcgctttggattgttaacagcttcgcctaagaactgaatttctttttccatcaagaaaccagcagcaactggcttgccgtctttgtgcattgcttcggcgattccagcgtttgaggcgtgggatctgtgagcagtaccaaaagcatcgttaatgaattcgtcggcaagtgaagcccagtattcacctaatttaggatcattaccggattcacgcttgacgtattcaccattaacgacatcttcataacgagtgttttcaaataagagaacactgccgtcttccattttgttgatagcgtcttcaagctgtttaccttcagtaacgggaacgaaaataaccggcttgttcaataagttggaaagacgttctgcaactgggcgtaatgaaaggcccttcttgtcgtcttcttttttgattcggccaagatgtgagcaaagaattgctttgcctttgtggtccaaaacgtacttaatggttggtaaagcagcttggatacggttatcgtcaccaataacgccgtctttgatcggaacgttaaagtcgacacgcatcaaaactttctttccttcgagatttaaatcagaaactgttaattttgccaatttggaaacctcccaaaatcgatttgatttgtgatctagagaacatagcgagatagtaaaagacggagaaggccaccctcctccgccaattacaattaattattaaagtgaagcgaacttcaacaaggtacgaaccatgttgcaagtgaagccccattcgttatcgtaccaagcaacagtcttaacaagttggctgtcaccggcagtagtaacttcagtttgagttgggtcaaatactgaaccatgtgaatcatcaatgatatctgatgaaacaatttcgtcagcgttgtaaccaaatgcagggttgtcagcggtgtgcttcttcatagcatcgttaacttcgtcagcagtaaccttcttgtcaaggactgcaactaattcagttaatgaaccatcaacgacagcaacacgttgtgcgtgtccttggagtttgccggcaagatctgggataaccaaaccaatagccttggcagcaccagttgaatgaggaatcgtgttagcactggcagtacggttgttacgcttcttcttagtcttaggaccatcaagaatttgttgtgaagcagtgaatgcgtgaacagtcgtcatagtaccaactttgataccaaagtctttgttcatgaagtaagccattggtgccaagcagttagtggtacatgaaccagctgaaacgatgacatcgtttgagttcaattcatccaagttaacaccaggaacaacagtcttaatttgaccagcaggtgctgaaatcaagacacgctttgcaccagctttgatatgagcttgtgatttttcttctgaagtgtagaaaccagtacattcaagtacgtagtcaacaccgtcatttttaacccaaggaaggttagaagcatctttttctgcgtaaacaggaatttctttaccgtcaacgacgatacccttgtcagttgctgaaacatcaccagggaaacgtccatgggttgaatcatacttcaataaataagccaacattgatggagtggtcaaatcgttaattgcagccacttcaatctcgtcggagtgtaattcgtggatccgcttgaaagccaaacgaccaattcggccaaaaccgttaataccaatctttacagtcatactaagttttcctcctttaggaaataagaaaatattaagacacagtacacgttaatcgtaccatgaaatgaaaacaaagtcagcacccttgtgaacgaaagttcaaagtatgcatcgagtaaccataaaatattacccaaattcgagtatagcagaccgcgggagaattgcaatgcaaatggatttagtaagcgttttcacaatcaatttttctttgttcttgaaaaagttctcactttctagtatattggtataggaagttgcgcccgtagtgtaatggatcgcacgtaagattccggttcttgaaatgagggttcgattccccccgggcgcatcagatttcactgacccatcgcaagcaaggattcatgtttcattaggtcatttttgacacataggtaattgtgttagtggtgaaactaggttcagtggacacaaagcaattttaatcagcgaaacagtgaggcagatgccccgctgtttttttgtaagcaatcagcttgatcgtcattccgcttttttcatatacagaattggaaagtgattgccctgttcatcaaattccgtgcgcttgtaaacttcaaatcccatgtgctcataaaatccgcgcgcaagtgggttttgttcgttcacaccaagctggtcgatcgaatactgctccatcccataatccaatagtcgtttgcccaaacccttaccacggtattgatttgagataaacaacatttcaagcattcggtcattaattcccatgaagccaaccggatccccattgtcgttttcaatcacgattaaatgctggacgccgccaatagcttccggaatgaccttcttaatcttttgaatctcgttatctgtcaaaaataaatgggtcgccttgacggaactctcccaaaccgtcaacaagtccttcaccaatttgggactgaccttggtttcttcgacaattttcattctctttctcactttcatgcaaactgactagggtgtctgttcctatgccaaacaattccatttatcgcttctggagtgccaaatcaagtcccaaaatatctcaggtaagtcatgggatgtttcttgacggtttggtcctttcaatggtcggcttgatttcacaaacaacaaagaggtccaagcttaatccttgaacctctttttttgatggttaatcttttcttcgcaattcaacaacccctggttaatccgggacggacgttggctctcgaacaccttcggtaaaatcaacgccttctttagcatagaagtccatgatctcttgacgttgggactcaaatttcggtggcaatgacagtccctgccccatcgtcaaaatgggttcttcgagactgaaccccggagtcgtcgtggcaatttcaacccggttatcaccaggatcgcggacgtacagactcttgaaccagccacgatcggcatactcttcaatgtttaagtgctgttctttggcaatatcccaaaatttgaacaaggccgcgttagttggggcttgaatcgcaaaatgatcgatactgccccggccaaaccgggtccggacatcttgctggtcactttcaaataattcaatggactggccgtcctccaattggacaacattattttctaccggaatgcccaaccagttatggaaaaaggcactggtagcttcaggatccggcacgtggagttctgttcccattaaatgcgtaatttgtttttcagcggggatcccattatcaggaaccacccgcatatcggttaaaacttctgacgtctccaataatttaacttccacatcatcagggtcggcgaataccagaccatggtcaatatcttgaacggtcactgaatggtcggttaaccgtttcttccaaaaatcagtgctcccggttggaatcgaaagtttgatattattgaagaaatgcttaccgtcagtccgatggcctaataatggcaccacaaaaaatgtcaccactgaccccggtgttccgagatagtcaccgtagaataagtgacgaatgcggatattttcctgattgacggtgttttttaccaggcgcatccccaaaacccgggtataaaaatcaatgttttgttgagcatctctggttaacagtgaaatatgatgagttctcatagtatatcctcccgactcggtatttgctgattactgttattgtatcacgaatgaatccgctttcttattataagcatttctttatcaaagactgatgaagattgaccgtaaaaattaatgatttgatgtgagcaaaacatttgaccttttttgaccaataaactatcatattaacatgaacttggcgtaagccatctttcataaaacctataaggaggcatcttgaatgaatttagtgccaaccgtcattgaacaatccgcaggcggtgaacgtgcgtatgatatttattcacgtttgctaaaagaccgaattatcatgttatcaggccctatcgaagacgacatggctaatgcgattatcgcccaattacttttcttggatgctcaagactcagaaaaagatatttacctctacatcaactcacctggtggtgtgatcacctcaggcatggccatttacgataccatgaactttgttaagtcagacgttcaaacgatcgtaatgggaatggccgcatcaatggcttctgtccttgcttcttctggagcaaagggtaagcgatttgctctgccacatgcccaagtcttgattcaccaaccttctggtggtgctcaaggtcaacaaactgaaattgaaattgctgctgaagaaattctcaaagctcgtaagatgatcaacaatctcttagctgagaattccggtcaaccaattgagaagatcaacaaagacaccgagcgtgataattacctcactgcccaggaagctgttgattatggccttttggatggcattatgaccagcagttccgaaaagcagtaattcaattcgttaattgaattgtgtgatgcctttcaaagcagtcctcattttatgagggctgctttttttacataatccacctgattgataatcggttgatgaccgactagaatataggtgaagttagttaaaaaattaacatgatgaatgatgaatcgaggccattaatatggatgttaatcaaacaaaagaacaagttaaacaaactgctgatgaatcaatccccactgagatgaaggcctgggaaattgttaagcctggttcaattaacggtgcggtttctcctttacgttacaccaccaagccggtgccaaaaccaaaacgaggcgaagttttggtcaaggtcatcgcttgcggggtctgccacacggatctccatgtaactgaaggcgatctgccggttcataaggaacatttgacgcccggtcatgaaatcgttggtcgggtcgttcagatgggtgctgaaacccgtcgatttaaattaggcgatcggattgggattccttggttacgttggacttgcggggtttgtgaatattgccggtccgggagagaaaatctctgccccaactcactttataccggctgggatcatgatggcggctatgcagaatacgtcactgttccggaaggcttcgcataccggattccggcccggtttgattcactgacggctgccccactgctttgcgccggaatcatcggctatcgggcatatgaacgggctaacgtccctgcaggcggcaccttgggcctgtatggtttcggtggctcggctcatctaaccgcccaaattgcaatgaaacaaggcatcgaggttcacgttttaacccgtggtgaagatgccaggaaatttgccctgcagctgggagcggcctcagccagaggaacctatgatatgccacccgttaagctggattcggcaatcaactacacaccggtgggtgacgtggttccaaaagccatggaagcgctgaaaccaggtggcacgttggcaatggccggtatccactcaacagatattccgcaaatgagttatccaagtcacattttccatgaaaaaaatctcaccagtgtcgaaagcaacacccgccgggatggtgaagagttcctgacattggctgatcgactcaatatccatccggaggtcactgaatatccgttggccaaagctgacgaggcactgaaatatattgccaaaggtgatattcgtggggcctgtgttttaagagtcagtgagggctaacctctgtcattaacagttaaatgattggattcaaaaaggattctaactatttcacagcgaaataattagaatcttttttaggtttaaaaatgtgttgaaactttactagcttggtcaaaactaaacttcaggggtcagtccctgagccagcttgccggcatattcgttaatctttcgcaatcggtgattaaccccggatttggaaattggtccaccctccaccaagtcgcccaactctttcaaactgacttcgggatgtttcaagcgcgcccgggcaacttgggccagcttagggttcagtttatttaatccgaccatctcgtcaatcagtttgatattttcaatctgcttactggcagcgttggcaaccttgttgaggttggcgttttcacaattaaccagtcgattcacggagttgcgcatgtcgcgaacaatccgaatatcttcaaatttcagcatcgagctggtcgcaccgatcaattgcaaaaagtcggcaattttttcagcctctttcaagtaagtgatgtagccgcttcgccgttgcgtagtccgggctttgaggtgatacttgttcatcatttctgcaaccatttcgttatgattttcatacagggaatagatttccaaatgatacctggaagtttctgggttattaacagagccgctggctaaaaaggctccccgcagatatgagcggatttgcgaatcttctgtcagcatatgacttggaacccgttcaacgattgaagcaccatcaaaaatgcccagatcatccaacagctgggttgccttattttcaactcgtaaaatatataaattattctttttcagcttcattttacgacgaacactgagctcgccagtgatcccgtagaactttgaaagcagcttgtacatccgcctggcaattgccggattttcggatgaaacgtttaacacaaagtgatgattggatattgaaagggagccattaattcgaatcaaggccattaattcagccttggcattatcccggtaaacggtcaaagaggttagttcctttttgacctcacttgcgtatgacatttaatcccctccatttcttgagtgactggcctacttatggtcgtccaatgatcgacccagtaaattgatcaattcgtcagcgacctcttgaccattgtgaaaggcaccgcgatcctttaattccagaaaatcggctgagataacccgacagcccatggcccgcaatccggcaaaatcatgtttaaccggctgggagacttcattccatttttggtggtcaatgtattcagccggcacttctttgatgttcaccaaaacggtattaataaaattcatccctaaatggcgattcaagacccgaacatggtcggcttcggtgaagttctcagtttcacccttttgagtcatgatattacaaatatagacgatgtcggcgctggtttgtcgtaaggcttcacccacgttttcaatcattaagttgggcaaaatactggtgaacagacttccagggcccaagacaatctgatcagcgttcataatcgcatcaatcacttgatgaaccgcctctggtttatgagaatcatcagtcgtctcgacccaaacgcgcttaatcaatttgccggcagccgtaatttcagattcaccgctcattgtcgtgccatcactaaattcggcgtttaattccaggggctcgttggcagccggataaatatggccatccaccttgagcatgtcactcaatatctggacggaatcaaaaataccgcctttcatctctgaaagtgctgcaataatcaaattgcccaaagcgtgaccggcaaagaattggtctgaacttcgaaatcggtattgaaacaaatccaaatacaactcaggcatctccgatagtgccaccataacgttccggatatcgccaggcggaacgacgttaatgtagtttctcaagataccagaagaaccaccatcatcggcgacggtgacaattgcagtaatgtcgacgtgtcgatttcgtaagtttttgaggataactggcagcccagttcccccaccaatcacgacaattcgcggttggtgcgtatgaagtgcgtcaagcatcagttaccctcctttgttttatggcggtcaatatcccgatgggtgatgttcaccggatactgatctttcaagtcatttgccagctgttgggcaattgccacagaacgatgttgcccgccggtacagccgatcgcaatagttaagctggccttgccttccttttggtaaccgggcagtgtgaagaccatcatatccaataatttttgataaaattctttggccccttgggagttcatgacataatcgcgaactggtttatcaaggccggttttgtaacgcattttggcatcataatatgggttgggcaggaatcggacgtccatgacaatgtcagcgtccaacggcagcccatatttgaaaccaaacgacatcacttccacgtggaaagtatgtgtttcatcagttgattcaaaattgtggaaaacttcttcacgtaaccgccggggcgccatattggtggtatcgacaaccaagtcagcagcctgtttgacgttggccaacaattcacgctcttttttaataccgtcaataacgcgtccattacgagccagcggatgagcccgacgcgtttctttgtatcgggaaacgagtttttggtcagatgaatcaagaaaaatgatgtcaacattattgtcatcatttttctttaaatcgttaaacatatcgatgatttcatcgtaaaagacctgtgaccgcaaatccattactaaagcaattttattaatatcccgctccatgcggattaattctttaaattttggcagcaaggttggcggcatattatcgacgcaaaaataccccaaatcttcaaagctttgcatggcaacggtcttaccagcaccactcattccggtgatgatgacgaattggttgttaacagccataatgatttcctttcgtataacgaacttcaaccagtataacataccgggtgtgtcatgtgaatgaaagaaacacccggagatacttgtccccgacccagtgagcattctagcagtaatggggcaacttcagacagcaaaaaagagccacttccaatcagttcattgaaatggctcaaccaaattatttacttgctttgactgcctgcttttcagcctgcttggtcaatttcttatccctttcaaggacgggcttaaggtactgaccagtgtaactctcagggactttggccaactgttcgggagtcccggtcgcaacgaccgttcccccaccatcgccgccttccggtcccaaatcaatcagataatcggcactcttaacgacatccaagttgtgctcaatgatcaaaacggtattgccttgatcaaccagcttttgaaggacgcctaataatcgccgaatatcctcactatgaagaccggtggttggttcatcgagaatgtagaagttttggccattggccttcttatgcagctcagaagccaacttcattcgttgggcttccccaccagataaagttgtggccggctggcccaaatgaacatatcccaaaccaacgtctttaattgtttgaagcttgcgagaaattttagggatggcactgaaaaagtccacggcttcgtcaacggtcatgtccaatacatcggcgatattcttgcctttgtattcaacctcaagggtctcggcattgtaccgcttgccatgacatacttcacaaggaacgtaaacgtctggcagaaagttcatttcaatcttcaagatgccgtcaccatgacaggtttcacagcgaccgcccttaacgttaaaactaaagcggccctttttgaagccccgaagtttggcatcgttggtattggcaaacaagccgcgaatgtcgtcaaacacaccggtataggtggctgggttggaacgcggtgttcgaccgattggcgtttggtcaatatcgataattttttcaatatttttataaccagaaatggacttgtatttacccggcttctcggaattatgattgagtttctgggcaagggcctttttcaaaatatcattgaccaaagtcgacttaccggagccggagacacctgtcatcacaaccatcttgccgagcggaaaatcaaccgtcaaatccttgaggttgttctcagcagcaccagtgactcgaatttccttaccgtttcccttgcggcgcttatctggaaccggaataaaccgcttgcctgagaggtattggccggtgatcgattccggtactttttcaatgtcggcgggtgttccgacggccattacccgaccgccttgctgaccggcacccgggccgatgtcgacgatataatcggcagcccgcatggtatcctcatcatgctcgaccacgatcagggtattgcccaaatcgcgcattttcttgagggaggcaatcagtcggtcattatcccgttgatgcagcccaattgagggctcgtcaagaatataaagaacgccagtcaaatttgaaccaatctgagttgccaagcgaattcgctgagcttccccgcctgataaagtccgagcggaacgtgagagggtcaggtaatccaacccaacatttcttagaaaagtcagtcgatcagtaatttctttgataattgatttggcaatcattgtatcctgttcaccaaatgtcagcgatttaaagaagttcaattctgctgtgacatcaagagctgaaatttgggcaacgttatgcttgccaaccttaacagccaatgcctgacggttcaaacgatagccgtggcaggtctgacaagttaattcggtcatatactgacttaaattgtccctggtaaagtcgctgctggtgttgtgatagcgccggtcgacgttattgacaaccccttcaaacgggccgtcaacatcacggatgccgccaaagtcactttggaggacaaaatggaatgatttggtctttgaaccgtataacacaaaggtttgctgtttcttcggcagtttgttaaatggcacgtccatgtcgatgccttgagcatcacaaacctgcttgagcatattcggataccatttggaactagcagaattccaaggtgccagagccccttcggccaaagtcttggttcgatcaggaaccaccaaatcttcatcgacttccagcttcattcccaaaccatcacagtcgggacaagcgcccagcggtgagttaaaggaaaacagccgtggttcgagttcaccgactgtgaatccgcaaattgggcaggcgtagtgttctgaaaacatcagtggatcgcgctcgcccaaaaaatcagcgacggcataaccgccactaaggcgcaaagcagcttccaatgaatctgacaatcggttattaatgccatctttgacaataattcggtcaataataatattaatgtcatggttcttatttttatcgagttccggtgcttcatcaatatcataggttttgccatcaacctgtacccgaacaaagccttcacgcttgatcttttcaaaaatctttttgtgttgaccttttttcccacgtacgattggtgacagaatctgcaattttgttctctcaggcagtttcatgatctggtcgatcatctggtcaactgattgactggaaatcaccgagccgtcgttgggacagattggtacccccactcgggcccacaacagtcgaaaataatcattgatttcagtgaccgttccaaccgtcgacctagggttcttggaagtggttttttgatcaatcgaaattgctggactcaagccatcaattgaatcgacatccggcttatccatttgccccagaaattgacgcgcgtatgatgacaaactttcaacgtatcggcgctggccttccgcataaagtgtatcgaaggccagcgagcttttccccgagcccgataagccagtcatgacaaccagtttattttttggaattgtcacattcacattttttaagttgtgggcacgtgccccacgaatgacgattttatccattgccaatatgcataatctcctttagattacttactcgtttgaccctttaattcaataattgtatcacgcaaagtagcagcctgctcaaaatcaagctttttggcagcgtcacgcatttcttccgtcaaacgagccagcatatccttttgatctttcttactcatttgttcaaaatcactttcgacaaagtcgtccttttcgccggcatcatccgagcctttggtaatcgaaattaagttacgaattggtttgacgatggtggttggcgtaataccatgtttcttgttataagcaatttgaatggcccgtcgatgagcggtttcgtcaatggccgccttcattgaatcggtcacggtgtccgcgtacataatcacagcgccatgttcattccgggatgcccggccgatagtttggatcaacgaacgctcattacggaggaagccttccttatcggcatccaaaattgcaaccaaggaaacttcgggaacatcaattccttcccgcagcaagttaataccgaccaagacgtcaaacttaccaagccgcaagtcgcgaatgatttgagttcgttcaagagtcttaatatcagaatgcagatacttcactttgatccccaaatctttgagataatcagttaaatcttcggccattttcttggtcaaagtggtcacaaagacccgctcgtgcttgtcaacccgcttattgatttcaccaaccaaatcatccatttgccccataatcggtcggacgtcaattgttggatccagtaaaccggttggtcgaatgacctggttaaccacatctttggtttgatccagctcataaggccccggagtggcagacatgtagaccacctgatgcacgtgctgctcaaattcgctcaatgtcagtggccggttgtccagtgcgcttggcagccggaacccgtagttgaccaactgttgctttcgagcttggtcaccattatacatcccccgaatctgcggcattgtctggtgagattcgtcgacgaccaacaagaaatcgtcagggaagaagtcaagcagcgtaaacggcggctgccccggctttctgcggtccataaaccgtgaataattctcaatcccgctcgtgtagcccatttcacgcatcatttcgatatcgtaagtagttcgttgcttcaaccgttgtgcttccagtaatttgccttctttttcaaacttggcaacctgcttgtccatctcgtctttaatctctggtagtgcaacgttcatcacgtcatcactggttaaaaagtgagtcgccgggaaaatcgcaatatgatcccgatcgccgatgacttcaccagttaaagtatccacttcgcgaatccggtcaatttcatcgccaaaaaactcaattcgaaaggcatgttcatcccaggatgccgggaaaacttcaacaacatccccatgaactcgaaaacgaccacgctgaaaatcaatgtcgttgcggtcatattgaatatcaactaattggcggagaaaatgatcccgttcaattgtctggccaacccgcaatgaaacaacgtgatttcgatattcggatggatcacccaacccaaagatcgatgaaactgaggcaaccacgatgacatcgttacgctccagtaaggaactggttgccgagtggcgtagctggtcaatctcatcattaatcgacgaatccttttcaatgtaagtgtcactggatgggacataggcctccggttgataataatcataataacttacaaaatattcaacggcattgtgggggaagaactctttaaattcaccatacagctggccagctaaggttttattatgcgataagaccaaagttggcttgttgacctgggcaatcacattggaaatggtaaaagtcttcccagttccagtagccccttttaaaatttgggcttttttgccttcgttaatacctgccaccaacttcttgattgcatcaggctgatcaccagttggtttatatttggatactagatcaaattttcgatctgcttcacgttcaatcaatttgaatccccctaacctctataccaaaatgacacaacataaaagggctgcaagcaaaatcatattttgtttcagcccactattcaacgctattttaccatacgaacatactttcgccaatcattattccttggaattgtcttccttttttaaaactttgcgggtgagccgtcttaatttatcctgagtcgtaaagttttcggccagcatatccggaatgactttcgtcaaaacatactgaacacaatgcatatcacggtactccagcatcgttgagaggctctctttatacatctcagggtagacttcctcgggattacctttttgaatttcgccaaaggattcatacaacaggtcaactttatcggccaccgctaaaatacggccttccaaactatcatccttgccttccgacagacgtcttcggtaggcatcttgaaattcatccggaatttcattttggacaaagttttccgtcaatttatcatccacatcagccagcattgaacgcagcttgggtgttgcatacttgaccggcgtcttgatgtcaccaataaaccgctcggtataatcatgattgagggctttttcatacaacccgcgccagtcgactttttcgccggcattttcctcgacgtcacctaaaaattgggcaatttcagttaccttgaatgaatgggcagcaaccgaatgctgttcgaatttaaagtagccaggtgctcgattgatcaattccaactcgtctaaactttccaaatactgatgcattcccattgataattccccgtccttttcctcgcaaaaagagccgtgaacaaaacaactgtttgtacgcggcctccctttgattaatcattaaattagtgttccgaaacactggactttgatgtgtcagccaatgattcaacatacttgaatgcttgttgaccggcaatcccaccttcgccaacagctgttgcaatctgacgaagatccttttgtcgaacgtcaccaatggcataaataccaggaattgacgtttccatctgatcgttggtttgaatccagccatcttcatcagtaatgtccaaatctttaaaagcatcggtcattggcagcagaccaacgtaaataaagaccccagacgtctcaagaactgattcttcatttgtctggttattgactactttaacgccggtaactttgttatcgtcacccaaaacttccgtgacgttggaattccaaacaaaatcaatcttgtcgttggcgaatgcccggtcttggataaccttttgggcacgcagttggtcacggcgatgaataactgtcacatgatcaacgattccagcgaggtaagaggcttcttcaatcgcagaatctccaccgccgacaacgacgacttctttgttcttgaagaaggccccatcgcagacagcgcagtacgaaacccctttgccaccgtattcgtgttctccggggatccctaatttcttatattcggaaccggttgcgatgatgaccactttggcttggatttcgtcttcgtcggtcttgacgatcttatagtcaccgtgatcttccacagcactgacggttccataaacgtattccgcaccaaagttaattgaactgtcgtacatattctgagcgagatctggacccatgattgatttaaaaccaggatagttctcaatggcagctgtgttgttcatctggccgccataaattccccgatcgatcattgcaactgacaggttggctcgtgaagcatatagagcagctgtcatgccgccggggccggcaccaataatcacgacatcatattgtttagccatatggatcctccctttaattaccaaattttacttacacgttaatttactatgaaaaagtaagtctgtccagtagatacacttacttctttttgtcttcttcagttaattgggcgcctaaatctttgagataagttcgcaaaccatcagaaatttccggatggcgcaggccaaagatgatgttggttttgagccagcttaatttgttcccggtatcgaatcgttcacccttaaattcatgagcaaagacccgctgtgtctggttcaaggtgtcaattgcagatgtcagttgaatttcaccagttttatccggtttggcgttttccaaaatgccgaagatttcaggcgtcaacaagtagcggccaataatcgctaaatcgctgggcgctttctctggcgttggcttttcaacgaactttttaacgttgaacaagcctgggcggacctcttcagagggatcgatgaccccatatttggagatatctttgtgggcaactttcttcactgctaatgtggaagctccagtctgctggtagctttccattaattgtttggtcagtggcactttgtcctgcatcacgtcatcaccaagcatgaccacaaacggttcattgctaatgaaactgcgggcggtgtaaattgcatcacccagcccacggggatgagactgacgaatgaagtaaatattcatgtcgttggtcttgcgaatggtttcaagaatatcgttcttgtgccgttcctccaagttcatttccaactcgggattcgagtcaaagtgatcttcgattgagcgtttgcctttaccgatgacaatcacaatgtctttgatccccgcctgtttggcttcttcaacaataaactgaattgtcggtgtatcaacaatcggcagcatttcctttgggagtgccttggtttccggtaaaaatctggttcctaaaccggcagccggaatgactgctttggttacttttctggtcatagtgagcttcaccttctctgagttattcaatttctgaacggccttcacgggtcatcagttggttaatcgtttctttaatatcagcatgatcatataaaacgtggtaaattgccgaagtaattggcatttcaacaccgcgcttcttggaaagttcataggcagcccgagttgtcgcgattccctcaatgaccattcccatattattaatgacttcatccagggaatgacccttgcctaattcgttaccagcccgccagttacgggagttggtactggtggcggttacaataatatcgccaacgcccgacaaaccgataaaggtcaacgggttagccccaaacgacgttccaaggcgggaaatctcggctaacccacgggtcatcaaggccgccttggcgttgtctttgtagcccaacccatacaaggcaccggcgcccaaagcaataatattcttcaaagcagcgccaatttcgacgccaatgacgtcgtcactggtataaacacggaaatagttgttcatgaacaagccttgaatttcagtggcagcttggtcgctatcactggcaacggtgaccaaagtaatgtcatgggtcacgacatcttcagcctggctggggccggacagaactgaaattgatttgcggttcttaggatcaatttcttgagccagaacttgagataatcttaagtaagttttttcttcaattccctttgaagcatggatgatattcactttttgattccggtcggccaaaatttctgcaacttgtttggcaactgaacgggttacctgggtgggaaccacgaataagatgtaatcaacaccatcgatggcgtccttcaaatcattggtagccaccagtgaatctgagaacgtgaaattcttgatgtattttgtgttggtatgctgttcgttaagttccttaacttgtgtcgggttatacgaccataatttgacgtctgacccattctcgtccaataaactggcaagaacactcccccaagaacctgcaccaagcactgcaacttttttagccatgataaatctcctttattagtaaatgatcaattaactgttaatttggaaccctctaaataccaaggattatgtggctggcgtaatcgacgataaatgatgattccgattgcaccaacaaataaaatgattgaaagaatctgcgatacccgaaggccgccaagcatcaaactgtcagtccgcatgccttcgacaaagaatctgccaaaagaataccacatgacataggttaaaaagacttcgccacgtttaaacagatgggaattgtgccgcaaggttatcagcaccaaaaagcctaagaaactccacagcgactcgtagagaaaggtcggctgccgatacgcgccgctaatgtacatctgggtaatgatgaaatgtggcagatgaagcccagtcagaaagctcaaagatgttacctgaccgaaggcctcctgattcataaaattgccccaacggccgattgattgtgccaaaataactgttggtgcggcaacatccaacatcagccaaaccggaatgaagcggtggcggcaaaataggatcaccacaatcatcgcaccaattaaagaaccataaatggcaataccaccgtcccagattttgatgatttcaccagggttatctttgtaataagaccactggaagatgacgtaatacaatcgcgcacaaattagcgcagcgggcaacgcccacaaaatcatatcgtaaatatcgtcggctttaatcccacgtttatcgccttcgcggaccgccaaccaaaccgccagaatcacgccactggcaatgataataccataccagtggacttcaattggacccaggttaaaggcgatcgggttgagggctaagctcaataaatttgtcaaaataacgatctcctattttttatctgaatctttgtcacgaccatcgatgagatctttatttttctcctcaagatgttcctgttcttctttatgcttttcgtcgtttttgctgttgaccttgattaaattattcaagttacggtcaaaggtttcagtcgcgtcatagcccatactttgggcacggaagttcatggcagcggcttcaatgatgatcgccaaatttcggccggttcgaacgggaatcgtgattttcggcacatcgacatcaaaaatatggacattctgagtcccgttgcccaaacgatcaaacttggcttccttggtgtagttggccagatgaataattaaggcgacttttgtctgactgcggacagcaccggcgccaaacaaagtcatcacatcgataatcccaattccccgaatttccagtaagtgacggagaatcgcaggggcggtccccatcaaggtttgttcatcttgttggtaaacctctacccgatcgtcggcaatcagccggtgaccacgtttaaccagttccaacgccgtttcactcttgccgattccactgtcaccggtaatcaggattcccaatccataaacatcgaccaaaacgccgtgaagcgacttgcgttctgctaatttatcgtcgaggtaattagtcatgttactgagaactcgagacgtcgtcaatttggaaccgaggacgggaatgtgctgttcttttgcggcctccagcaattcttccggtggatccagttgggtggacaccacgaacgccggcgtctgtggttgacacatctgctgcatcacatcgaggagctcttcatgagacatccccttggaatatgaaatttcagtaatgcccaacagctgaattcgtttgacagggtaataattaaagaacccggttagctctaggcccggtctggaaatatcagcagtggaaatggtcctttcttcaaggtattccttcccataatagacatccagcctggcgtttttaaccaaatcagcaaccgttacactttcagtcaagaacatccctcctcaattaatcaatataattttatcactttgagcctgacaagtccttatggcttgcggaaatattcagcaatgatccagctgaccgcagacatcagaatggccacgccaattgcgacccaaaatgatgagaatctgaaattagccccaacaatcgtcgccgtcagttcaagcatcaacccattaatgacaaatgtgaataatcccagtgttaaaaggttaatcggcaaagacaagatcgtaataatcggtcggaccaaccagttcaaaacggctaaaaccaccgccgctacaaaagcaatgcccacgctggcaacgtagaagttggcggggaaaaagccgctgatcgcaacaaacaggatcgtatcgaccaagacattggttaaaaatctcaattattgaccccttttcttgtcatcatgaacgtctttttcttcgacgttatgaatgacttttctggatttgtcgttagaagttccgccggataaggtggttttgaattggtcaaaggccgatccactaccaggtgtatcactgggaattgtgaacatcataatgatataaccaataattgcgaccacgttgatcccgggcgtaaacgccaagaccacatacaagattcgaaccaagacagcgttccagtccagatactcggaaattcctccaagcacgccggaaatcacccgattggtactggaacgccgtaattttttatgactattcatcctcatgcctccacaataaaacttctagcttaagattatctaaaaaaggcactgcaatcaagtatgcagtgcaaaatatcaaccattcttaatttaattcaataatttttccggttgccagataaaccgtccactcacaaatattcgtgctgtaatcactcacccggcctaaatctttggcaacgtttagataaataatcgctgaactgacaatctctggatccttggccatcgcttggtaactgggagaagcaatgtcgttataaagctggtcaatttttttatcgtactgttgcgcggtccgcttggctttgtcctgatcggcatcaccgtaggactcaattgaatcggcatactgctcgctgacttcttgagacattgtggcaatgatctcttccactgaagcgatccgctgcttgcctttaatatcaatcaccgatcgagcgacgtttcgggcatggtcaccggctcgttccaaatcagtgacggcttttaaaattccgaccacttcccggaggtcccccgtgaccggctgatacagcgcaatcatttcaaatgaccgcttttcaatatgaatctggaggtgattaatttcgtggtcgttggtgatcaccgtttccgccttttgaatatcatggtcgacaaacgactgcccggcgttggtcacggcttcaccaaccagtgcccccaatttcataaaatccgcctttaacgtaataatctcttcatcaaaaactttccccataagcttctctcctatccgaatcgtccgctaacgtaatcctccgtttgtttttcctcaggattcacgaacatcttagttgtgtcatcatattcaaccactctgccttccataaagaacgctgtcttatcagaaattcgggaagcctgttgcaggttgtgagtaacgattattattgtataatcttttttcaactcaagcaaagtattttcaatcttggcactggaaatcgggtccaatgcactggtcggctcatccatcaaaataactgatggtgaagtggcaagcacccgggcgatacaaattcgctgttgctgcccgccggaaaacgacagggcgttatcgtacagattgtctttgacttcatcccaaacagccgcctgcttcaaacttttttcaacaatttcatctaatttttgtttgtcacgaagtcccgcgatccgcaaaccataggtgatattatcatagactgaaaatggaaacggattgggctgttgaaagaccatcccaatcgactttctcaattctaccagatttgtttgcggagaataaatattttctccgtgaaattgaaccgttccggtaattgtcacgccatcgatcatatcattcatgcgattcaagcaacgcagaaatgttgactttccacagcctgatgggccgatcagcgcagaaatttggttaggcaggaaatccaaatgaattccgtaaagtgcctgaaaatcatcatagaataaatccaaattgtctgctgaaataattggtgttgccatgattgttcctcctaaccaaagtttcctgatacatagtcgtctgtcatctgtactttcggccgcgtgaagacctttctggttttgttgtactcaatggcctcacccatgttgaagaagaccgtgtagtcactcaaacgggctgcctgctgcatgttgtgggtcacaatgataattgtataatcctttttaagttcacgtaaagtcgcttccagttgttgcgttgaaaccgggtccaaggcactggccggttcgtccaacagtaacacatccggttgaaccgccaaggctctggcaatacaaacccgttgtgcctgcccaccggataaggaaagggcacttttattcaaactatctttgacctgatcccagacagccgcttgttttaaagtggtttccaccacttgatccaaggttttcttatcatgaattcctcgtcgctggagcgcgaaagtcacgttgtcatagattgatttggcgaatggattcggtcgttgaaaaaccatcccgattcggcgccggacctcataaacatcgatcttgggctgattaatgttgacgccttgataaagaatctcacctttcacagtggcgacgccatcattcatccgattaagggcccgtaaaaaggttgacttacccgatcctgaaggcccgatcaaggccgtaatggtattttttctaaacttcaaatccgcgttgtgcattgctaaagttttgccataatagatttccaaatccttggtctgcatcgtaatgtcattttcttcgggattaaaatcataaataaaccgcttgggtttgttatttaattcagttgtgttttgcattttcagccacctactttactgaagtcattcgttcaaataccttccggccaatccatctggccgacaaattaaagattaaaattgccaggaccaggacagccgctgaaccggaggaaacctgtgtcaaatcaggcatgattccttctgagttgattttccaaatgtgaacggccaatgtttcagccggccgcaacggcgacaatgggctatcaatgttaaaggggttccaatcggcaaaattcaacgctggggcgctttgaccggcagtatagatcaaggcagccgcctcaccgaaaacccgtcccgaacaaagaatgattccactgataattccaggcagtgaagcgggaacgacaatgtgaataatcgtctcatatttggaaagtcccaagcccaaaccgccttggcgctggtcatcggaaacgttggaaagtgaatcttcaatatttctggttaacagtggtaagttaaaaatcgttaaagtcaacgcacctgaaatgattgagaaaccatagttgaactgaacgacaaacaataagaaaccaaacagtccaaccaccacagaaggcaaggaactcaaaatttcaattgaagtcttgatcgtagcggtaaaccagttatctttggcgtattcgttgaggtaaatcgccgcgccaagtgcaattggcagagaaatcaacattgctaacaccaagaggtaaaatgagttaaatagctgaatgccaattccgccgccggcattaaacgctttggccggggacgttaagaaatgccaactgatattgggcagtccggtgataaaaatatagccgatcaaaaaggctaagatgaccaccacaaagccagcaacggcttttaaacaggcaatggcaaatcggctttgcttttgtgttcgattcatttcttaaacgcccctttccgaccgatcatgtgaactaataaattaaagaacagtgacatgactaacagaaccagtgccagtgaccagagagcgtcattttgaagcgatcccatgacggtgttccccatgccggcggttagaacagaggttaacgtggaagccggtgacgttaaattttgcggcatcaaagctgcatttccaatcaccatttgaacggctaaggcttcaccaaaggctctggccattccaaaaaccacggcagtcaaaatccctggtgtggcggctcttaagacgactttccaaatggtctgccacttggtagcacccaaggccagtgaggcttggcgatagaacttgggaacgcccctgagggaatcgacagtcattgatacaatggttggtagaatcatcacgaacaggacaaaggtcccggataggataccaaacccactgccgccaaacgtatttcgaacgaaaggaacgactactgagaggccaataaatccatagacaaccgagggaattccgaccagtaattcggttaccggctgaagaattttagctccccgtttaggagaaatctcggtcatatacaccgcagtcccgatggcgaacggcgtcgacagtaaagcagccagaatcgtcacaagaaaagagccgacaatcatgggcaacgcgccgacggcttggtgcccgccgggagtcttggtaccgggattccacaacgtaccggtaaagaagtctttgacagaaataccatctttgaagaaggtggccagacccttgctggcaacgaagacaataatgccaagcacaatcgccataatcagcagcagcgccgaaagactgagcagatgcccaaatcgttcgtaacgggccgttttagattttttcatcagttgtttggctaatttttcattttgcacgattattcccccgatccttttgtaattttgccctcccaggttctctggtaatgcatatctttcacagagatgtaacctagtttgttaaagagggtcgtttgaatatgatcgtttttcaagtaagttaagaattttttagtcaatccggtgggtttcccacgggtgtaaatgtgttcataggaccagattttccacttattgtccatcacgttttgttccgtgggcttaatcccatcaacgcttaatggatgaatgctcttgttgaagtagccaaatgagacgtagctgatagcccccggcgttgatgagacaatctggcggacagttcctgaagaatcctgctcctgggcggtggcactttcatggcctttaagaccatattgttcaaaggttacccgggttccgctcccctgagaccggttgatcaaagtaatcggcaggtcgggtccgccaagctgtttccaattggtgtatttcccagtaaaaatcgcaatcaactgggcggtactcaggttgttaatcccgacgcggtcattggtaatcggagcgactcccacaacagcaattttgtgatcgaccaagccggcgggattaatccccgccttttcttcagcaaacaaatccgaatttcccatctgaacggcaccggactcgatttgactcagcccggttccagatccaccaccctggacattaatgaaaatgccagcgtgatcagcagaatattgttcgctggccgcttcaaccagcggctggagcgcagttgaaccaacagcggtgattgattgctgattggttgaggtcttgctgcgggcattgtaagcaccaattccggcaacaattaccaccacacacagtaacagtttaacgatcgtccgttttcgcatctcaattcctccttgaatcttcaagtaccattgtattaaaccaatgtaaatatttgaccggacaaatgtaaatgttttgtaaatagataaccgggtgttgataattaatggctgaaggaacgcaaaaaagccggagatgctcccggattgattgatttgaaaatgtaaatatttggttgaaattcagcaaaaatcagtctgtttgtgtgttgggctggtcacgatccttgacaatcggaaagttcacggtaaaagtcgagccaacaccccgctgacttttaacatcaatcgtgccgccaactgcatcgaccatttccttgacgattgaaaggcctaagccggtcccactgaccttctgcttcgtccgggagtcgtctgcgcgatagaagcgttcaaataatctggaaatgtctttttgggcaatcccaattccggtatcggaaacgtggagctgccaataactgtcgttgtcactataggtaatgttaacctcgccatttgggcgattatatttaaccgcgttgctgaccagattgcgtaaaatccgcgtgagcgtggtggtgtcggcaatgacttcaacgtgttccgggacttgattatgaattgcaacgtggttgccttggatcattgattgatatgaagcaagctccgcatcaatgaaatcatgcaaggccaacggtttgtaatgataattagtaccgttttgaatatgggaaatcgtcagtacgtcttgaaccagcgaggccagctgatcactttgttgatcaataattttcaaaaactccaccaaactcttcttatcgtccatcgccccacccagcagagttttggtaaatccggagatggcagtaatcggcgtcttgagttcgtgactggcatttcgcaaaaagtcaatctgcatctgtttgacgttaataatatctgagatgtcatacataatcaccaggatgtgaaaatcgttttcgagttgattgaacaccacgctggtatcccaggtaacagatgtcgccccgacgctttgaatctcttcttgctgagacttgtgactgtcataaacattctcaattaaagacagtagttgataattgcggatgtcttgggtatagggatgaacctgagtcaaaatatctcgtcccagcatgacggacattttatggttggcgaaaatcacatcgtgagttgaatcaattaccatcaccccgactggaaggctggaaagaatcgtaattagttcagcgttgctgtttcgaatactctttccttcgtcctgctgcctgctttgaagttcgttgagctggtcggcaacgcctttgagtgggttgtcgggttcaacgaaaagcggcaccgccggttggtgatgaacaatgttttccgtcattatctggagttgtttgagcagcttatcatgctggcggtattgaatgatgagaataatcccggcaatggcatcgaccagggccaataacagggccaggtcagcccagcccaaattgccgctcgtaaaaccataaaaaagcacggccagtgtggcaatgcttaagattacaacggttaaaatttgtttatagattttactcagcgtcatcatcccccgtggagaactcataaccaaatccgcgaacggttcgcagatatttcggccgttttggatccggttcgatcttttcacgaagatgggcaatttgaatatcgaccatccggctttgacctgagtagtcaaagccccaaacaccctggagtaattggtcacgactaagcacttgattttcgtgactgaccaagtactccatcaattcaaattccttcggcgttaactttaagtttttcgaatcagcgctcacacggtattttttgtggtcgatggtaaacggcccagtggtttcgacattttcagctgatttagtagctggcgtttcggatgcagcagcactcttctcataccgacgaagtaccgcgttaatccgcgcaatgacctctcgcggactaaatggtttgggaatataatcgtcagcacccatctcgaggccaaagaccttatcaaattcggtatctttggcagttaataaaatcaccggtgtgtcgtttcggtccatccgcagctgcttgaggacttgttccccactcatctgaggcaacatcaaatccaaaagtacgatgtcaaattggccattttcagccattgaaagcgcatcgactccgttagtagcactctgaacttcaaaattggcttgcttcaagttatattccaataaagtaacaattgctggttcgtcgtcaactacaagcacttttttcacgatagccctcctaatgactaagctgtgtatatgttttgaccccaatttcatgaggtgaattcttgaagatcgccgattcggtcatcttcaactgatcgtttcgatcgcgaactttgaaccgacaataagttgagttggtgctgagcgcgcgataaaaagaatcttcatcagtcaccgaaatgccattgacctcaaggatcacatcgccaactttgagatccatcttggcggctggggtttccggttgaatgccaattacccggacaccatccatcacttcactatattcaaacgactgctgattgtcacggtgtttggcaagcccaagaatcaaatagtagcccaacaacaggataaccacagcgggtaaaatgaggtgcggtatgaagtagccggcaattgccaggcagacaccaatccctgccagtaagtaaataccgtgactcattgttttaaataaggccctgggaacacttcttttgacggtaaatttaagtccaatcagaattggcaccaataacaacgcgtagaaatgattgtgtacttgaaatagcggcatcattggtaagctggtatggatccagtctccgggaacaaacagcaggaacggaaaaatcgttaattcgttaaatttataaacggccgttttattgtttcgttggttgcgcaccaaggtcggtgaatcaaatcgaccaccgttaacgttcaagaaaacggcgtttgccaagataatgaccacaaataaaatcaacaaattgagcggggccacagttgttgagttgattcccagtccttcaaaccaatgaagcagcggtcgcaattctgatatatttggcaatcccagcgtcaataaactggcgataccggcaacagtcaccgacagcagccaccaaggaatcagcgtgagcgaaaccagcagtaagccttcataaatgatcaaccattccagtgaaatgcttaaaaagccacctaaaacgacggaggccagtatcccaaagatcagccccattctgacaaaatgtcgaccttcataaaaatcctcataaatggcggagttaaaaatcccccgctctttcttaagccgcctcgtatgaattaaataactgcggataaccccgatccacaaggcgggttgcaatccataaaaaccacaagcaatcaaaaatttcattatgtcttcctcaccaataattataaggctagtatatcatttattgacagctgatttaagctgatttgaaatccgaaaggctaatcaagatggtggcttaaccggcagttgctgactttgggtgcttggtagggttctccaatcatcctgtcgttgataaaaaaaggcccttaacgcaatgtggcgtcaagggcctgatcgtatcattctcgttgattcgcaccgggctaaagcaaacgcggctttaataaccgattagtctggattcttctgacttaattgccattgcagataggcgttgatgaacggatccaaatcaccatccatcacgccgttgacattggcagtttcgtaattggttcggtgatctttgaccatcgaatatgggtgaaagacataggaacgaatttgagagccccagccgatgtctttttgttcaccctcaattttggccttttcttcggcctttttctcttcttcaagttcatacaattttgacttcaacatgttcattgccgtttgccggttttgaagttgtgatcgttgtgcctgactggcagccacgattccagtgggtaaatgggtgattcgaacggcggaggaagtcttgttaatgtgttgcccaccagcaccgctggaccgataaacatcaatccgtaaatcatccgggttaatatcgattgagacgtcatcatttaattcaggcatcacatcaacggatgcaaatgacgtgtgtcgccgaccggctgaatcaaatggcgacagcctgaccaatcgatgaatccccttttcggaccttaaataaccataggcattttcaccgctgattaatagtgaaacactgttcagaccggcaacgtcaccgacctgataatccaaggtctgcacggtgaacccatgggcttctgcccaacgggtatacattcgcagcagcatcgaaccccagtcctgggcttcggttccgccagctccgggatggatttccaaaatggcattattatgatcatatttgccgttaagcaacagattcaactggtagcggtccagtttagttttaagctgcttttcatcagtctcaaattccccctccatcccggaatgagaatcctcttcgatcaattccaaagtaacttttagatcatcgagtttatttttgaggccgacgaaattgtcgcgtttggtttttaattgattggtttgatcaatcaatttctgagcggcttcttggtcatcccaaaagcccggctcagccatcttcgactcattaattgcgatgctttcacttaaggcatcaaggtcaaagtgacctcccaaaaccatcgatggctttttgcatttcagcgatttgtttttttgcttcactcaattcaaatgacatattactctcctctaattttgttccaattcaaagaaagaatccaaacaatcgtcattgccggattctttccaatacatattaacgttgcatgttttgacgaatttcagccttcatgaacagacgggttgcgtcatattcgatatcggcaatcatttcttcaaacatcttgtaaccctctcgctgatattcaaccaatgggttttgttgaccataaccacgaagaccgattgattgacgtaattgatccatgatgtcaatgtgatcagtccagtgggaatcgacaactcgcaagataacaaccttttcgaattcaagcatttgtgattcatcgtagagttgttcttgcttttctttgtattctttgtttgccagatccatcagcatactcttaatttcgtcagctgatttgccttggaaatcttctagagaaatttggtctgggctgaccatcgcactgatggcaaagtccaagatggtttgcagatcccaatcttctttttcgccttgggtatgcaaatcaacgattcgattgatggtccgttcgatcatcggcatgatgacccacttcaaatctttttgctcatcaatgacttcacgacgctcaccgtaaatcacttcacgctgttgtctcataacatcatcgtattgcaaaacgttcttccgtgaatcgtagttgttaccttcaacccgcttttgagctgattcaacttgcttcgtgatcattcttgaacgaataaccgcgtcttcaccttcaacatttaaatgctccaggaagtttttgatcttttcagaaccaaaacgacgcatcaagtcatcttcaagtgacaaatagaactgtgacaaaccaggatcaccctgacgtcctgaacggccacgcagctggttatcaatccgtcgtgactcatgtcgttcggtcccgataacagctaagccgccaagttcaacaactccgggtcctaatttgatatcggttccacgaccagccatgttggtggcaattgtaacggcaccacgttggccggcattggcaacaatttcagcttccttggcgtggtttttggcattcaataccacgtggggaatcttttcttcatcaagtcgttgtgataagtattcagaagtttcaacagcaacagtaccaaccaacattggctgaccctttttgtgaagctccttgatcttgttgacaacggcctcaaatttggcttccaaagttggatacaaaacatctggatgatcaacccggacaaccggtttgttggttggaaccgaaataacttccatgttatagatctcacggaattcttcagcttcagtcttggcagtaccagtcattccggcgagcttcttatacatccggaagaggttttggtaagtaatggtagccattgtcttactttcctcgttgatcgtgacgccttcttttgcttcaagggcttggtgaagaccatctgagaatcgacggccttccatgatccgtccggtaaaggaatcaacaatcttgacctcatcatcttgaaccacgtaatccttatcacgaagcatgataaagttggcccgtaaagcctggtccaaatggtgggtcaaggcagtattgtcggtgtcataaagattctttaagttgaagtacttctcagccttttcgattccctgatcggtcaatgaaacagtcttggtttccagatcaagcttgaaatcatcgccttcgtgcaacgtcttggcaaatctgtcagtccgttggtaaaggtcggaagtgccgcttgattgaccagaaataatcaatggtgttcgggcttcatcaattaaaattgaatcaacctcatcgacaatcgcgaagttcaaaggacgttgaaccatttgttccttataagcaaccatgttgtcacgcagataatcgaaaccgatttctccgttggttgagtaggtgatgtcggcagcgtaggcttcccgcttctcatcggcatccttttcagtggtattaacgccaactgtcaggccgagccaattatataactcgcccatttcagtggcatcacgttgggaaaggtattcgttaacagtaaccacgtgaaccccttcgcctgcaagtgcatttaaataaaccggcatggtggcagttaaagtcttaccttcaccagttttcatttctgcaatatttccttcatgaagaacaattccacccataatttggacatggaatgggtacaagcctaagacacgctttgcgccttcacgggcaacggcaaatgcttccggaagcaaatcatcgagtgtttcgccattttgatagcgtttcttaaatgccggtgtcttggcttgtaattcttcatcactgagttgacgatactcttcagcatacgaaccaactttatcggcaattttactgagccgcttttgttcgcgtgtatcactttcaacccatgttcttaaaatattagccattagtaaattcccttctaaaataaaatactgatcaaattgttcttagtatttgtggactacatacttatttagtgtaacattttaggccgcccatgaaaacacaaaaaacaatgcatcagcggcatttaaccatgataatacattttgaatagatatgaaaggttaaacgatcagattggttcacaaatatttccggaaacgaaaaagaatggggataaattaagctgcaatttatccccattcttttgacggtgcataatacgcatgcccgttaattgattaacttaattattcttcgccggtctcaatcaagccataacggccatcattacgacggtagacgatgttgatgcctgaagtttctgcatcttcatagatgaagaaatcatgccccagcatgtccatttgaagaatggcttcctcgttatccatcggctttaaagccagttgcttggtacgaacaacctggaatttggattcgtcatcagaatctgactcgctggcagaagtatctgcagcaggtgcaaattcaagattcttaaatcctttttcacgagacttgcggttaaccttggtcttgtacttacgaatttgacgttcgagtttgtctgtcaccagatcaacacttgcgtacaaatcgttggacatttcttcggctctcaaagttaagtatggcaaaggaatggttacctcaacttttgcttgcttatctggataaacctttaaattgacatgagcagtatttttcatgtccttttcaaagtatttctccagtttactgatccgtttttcaacataatcccggatcgcctgggttacctcaatgttttcaccacgaatgttaaaaattagcatagcgttctctcccttcaccattaaaggcttaatggtccactaatgaaatcactttcattactggctacaactttagtataattgaaagttcgaattttaacaatcattgggtctggatttctttatcgagcaagggtaaatcctttcacggaagctgccccggcttgttggatcaaagcggccgcatgcctaatggttgtcccggttgtatacacatcgtcaaccaataaaacggcccgatttttaacctgatttttttgtgattcaatcatttcaaacggttgatcaagcaataaccgactctgacggtttttcgccgactggcggatggctttcttgtcgaatctgacgcttaagaggtttaaatagcggtcattttccagcagcccggtcacctgattaaagccccgagtggccacggtgtccttccccaccgggattggcacaatgatcgcagattgcttcttcaactgctcatgaatttgatcggaaaaaactttccgtaatcggtaatcaccggcaaacttgtatcgtttcatgtaatctttcattgccggattatattcgtacatcgccgagttgataaatttgaattggccgtccttctcccagcgcagacaatcatagcagggatcgctcatatcatttgttcgccgtcgaccgcaactggaacaagttggtagcagattaagcgcggaaaaagtggcggaacacgcctcacagatcgcccgtttctgcagtggggttaaccgaatcaagtctgcaagtgggatttcctgtctcagtctggagccacacaataaacaggctttcataattgagccgcctttcgattcatcagcttaatctggcggtcacaggatttgatgttggccgttttagattcacaataaaagaggacctgtcccgtcggccgatcactatttcgacccacccgaccagcgatttggacgagtgcagccgccgaaaaaatttcactgtctgcctttaataccaagacgtcaatgcctgggaaggtcacgccccgttctaaaatcgtcgttgtgatcaaaaaatccagttgttgactgcgcattaaggccactttctcaattcgctcgggatcagcagaatacaccgttttgaatttcgctgctatcccggcagccttgatggcagctgccgcttgacccaagtctttaatgtggggaacgaacagtaagaaccgctgcttttctgctaccaagtcagccaccatccgcaagattttttgaggcagtttgccagattgaagctgctcgttaagatttttgacccgaattaccgagatttccggtaaatagtgtccatgatacctgattggtaaataactgaccgacaactgttttctagaaattgctttaaacagtgcctgatcgggggtcgccgttaaatacagcgttgccccagcgggtttaatcgcattttgaacaccaaaatgaagcattgggttaccagaatatgggaagacatccacctcgtcgacaatcaggacgtcaaaggcatggtaaaatcgtaacagttggtgggtcgtacaaatggtaatctgactgtattggtaccgctgctcactcttgccatgcagtaacacgattgaaacttgattgaacgcggcttgaattcgtgggaacagttcgatgcatacgtccacccgcggcgaagcaatcccgactcgcaaaccatttgaaactgcccagctaatccctttaaacagcatttccgtcttgccggctcccgtcactgcccataacaagtgacgttggcgttgttgaaacacttcaatcactttgtcggcacactcattttgtaattgggtcagctgcccggaccaggataatggatccggattctcagtaaaatgatttggctcttccaaataagccagtggcgacaaggtatccacccgacccatttgaatacaaatgtagcaataaaagtggtgattgggtaaactggcaagtgaatggcgcaattttgacccgcagcgaccacatttcaatccatggtcatcactgatggccggacgtaagcgaatgtccggtgaattttgcagtgtcgcggccagatcacgctgtggcatttggcggccatacaactctgatagatcattaatcatagatcatcacctcaatcactaattacgtaaatactggaggaatcctttttgaaaaatgaatcactgacaattaaatcaaacggtacccatgaaatcgaaattaaaaaatcccgctttctctgcacgatggcacgaattgataacgaggaccaggcaaaaaaaatcattgatcaggtgagtaaagacaataccaaagccaaccacaattgctacgcctacatgttgggtgacgatgaccacattcaacgcgaaagcgacaatggcgagccatccggaaccgccggggtccccatcttggaagttctcaaaatgaacgagttacataatgttttagcagtggtgacccgatatttcggcggcattaagcttggcgccggcggtttgattcgggcttatagcaacgcgacatcgacaacgattgataaattagggatcgtcaaactggtaaataaacagaaaataacgctgacaattgattacaatcaattcgataaactaaagtatttcttggaaagccaatcgattccaatcgaagagacagcctataccgccaaagtccaagtggtcgtggcagtcagtgacgaggattttgattccttgatcactcagattaccaatttgttaagtgatcaatttgcatatcaaaaaggcggacatcaaatctttgaggtcccctattctcgtgaaaaaagacaacatgacgaaaccaaggaggatcattctgactgagttatcaaatcgtgcaacagatgcagctgcctcaaactttccagtgatcgatataaaaaagtctgccaaagatttgggttctacaatatctgttgttggtaatagatttttgtctattactgatgacagttttttgtttatcattagagtaaaaaagcggacatctcccgtccgttaacttgctcccaccacagaattaagtcaagaaaggaaatgccctatgtcaaatgatactacgaaaatgttgttaggaatagatgatgaacacttaataattgagaatggcaaaataggtgatgatggggtgatccgattaaatggatcgctgaactattcccccaaggcctgccacaactgtggggttattaatgaccatcagatcattggctatggttggcggaagaccaccattagattcgctaaaaccttgggcagcaccgttatcctctgcctcaatcggcgaaactttcactgtaaggcttgtcataccaacttcctggcgcagacgaatgcggtgccgaaacactgcacgatttcaaatacgacccgcaaacaatgcttagaaaaactgaccgaaccggtttcgctcaaacacattgccgatgagttatccacttcggattcattcgttggtcggcagctcttgcgcgctgaacgggactttgaaaccaactggcactatttacccaaagttctcctcatggacgaagttaaaagcactaagagcgccaccgacgcgatgagctttgaatttatggacgcggaaacccacgaattgatcgacctgttaccctttaggaccatctatcagcttcaaaagtatttccagcattacgaccaggctgcgcgagaaaatgtgaaaattattgtcaccgatatgaactatacctatcccaaattggtggggcagatctttccgaacgccatcgttgtcatcgatccgttccacttggttaacgctttaaatcgagcttttaataagacgcgggtgcgcctcatgaaaaccctggcgacctcatcacgcgagtatcacgccttgaaacgctattggaagctattattaacgccggaaaatcacctcaactacgaagctttccgtaagtggacaaacttcccttatccagcgactgccactgatgtggttgatgctttattggacattgatcccgagctcaagcaaacttacaacgtgatgaatcggttacgtgaaaccatcaaaaaccgtgattggcccaactataatcaagtattccatcacttagagggctgctcggaagagatgttggcaaccctccagaccctagcgactcatcatgatgaaattggcaatacctttactcaccattacaccaacgggcccttagaaggttcaaacaacaagattaaagtcattaaacgcactggatttggttaccgaaacttcttcagattccggctaagagtgctgttcgcttttcgagttcatacaaaaagagctctaatcaccaagtgattagaactccaatattttgttcaccaacaacagttgacgaagaaccaagatttggcagactttttatgatactaatgattatttttactggtcgtatctttaaccaatttcttaatgccattcaacagcggctgtcgatcttctccaaccaggccaatcgtttccacaaacaattcaaggccgattaacacggaaattgtcagcagaatcgagccccacaaggttgaaatcggataaagcagtgagataaacgaaaaaatcagggcaattccatagatcaccaacaccgtttgccgatgggtcaaaccaatttgcatcaaacggtgatgtaaatgtcgcttatcggcatgcgtaatcggttccttatttaacaaccggcgaaaaatggcaaatacggtatcagtaatcggcacacccaagatcatcactgggattagcagcgtgatgaaggtggcgttctttaagccaaacagcgaaaagaccgacatcataaatccaataaacaacgcaccggtgtcgcccaaataaattcttgccgggaaaaagttataaggcaaaaagccaatgcaagcggcgaccagggtaaaaatcatgatggcaacgaaaatattaccgacgttcaagaagaacatggcggtaattcccatggtggttagggcaataattgcaaccccagtggccaagccgtccaatccatcaatcaagttaaccgcgttagtgattgccaaaatccaaatccaagttaccggcaaactcagccaaccaaggtggattgtgataaacggtaaggtaatggtggtcattttaacgccggctgtaaagtaaacccacagcgcggcaattgaaatccccaaaactttttgccggggctttaagacgaaaatatcatctattatcccagtgagaataatgatgacttccccgccatacaccccccacaaaattttggttgggaactgatcccgcaataaaatcatggtcgtaaaggtgtaggcaataaaaattgccaacccaccaatcgttggcattggaattttattaacccgccgtttgtttggccggtcctctgccccaacagcaaaagcaagtttccgaataaatggggttaagactgcagaaataatcatggtagcaaataaagacacaatgatctcgaatttcaaaattgtaacctcacttatttccttccaaatcaatattaattcaattatacaaatgacaattcataaaaacaaggtatgtctgactcacaaagtaaaggagcttactcaaataattaatacggaccaattgtgtgaattttcacatttttaaattttgccaacgttttcaattgtcatatttcacaaaaacatttatactagagattgtaagacaacaggttcaattattttatatttcacaaacggaaggagtttttatcatggctgacaaaacaaatactacacaagccgagacgaaagatgcgcccattcttattcaaatgggtatcttcgccgcggtattgtttgtttccagtttaatttcagcatggttggtagcagtcgcaccaaagttccctgttccaaccccagttcttggtttaattattctttatctcctattaactttccacatcgtcaaagttgaatgggttgataaatttgccacatttatgatcggaatgatcgcatttctatttgtaccttcaggaattcaattgaccgcatctcttgatatcatgaaggctcaaggtgtacaacttattgttgctattattatttcaacggttgtcttacttgttgttgttgcttacaccacatcattctttatctggatcagaaagaccgttttccatggcgatattacagttagtgaagacgtcgagaaaaagtaattaaaggggtgaatataaatgtctgctacacaaacaactattattgcgtatttagggacaccaatttttggtatctgcttgtcactgttggttttcttgtttggtcaatggctattcaagattggtaaaggattcttcttattccaacctctgtttgttggaatggtacttggaatcttcatcctctggttgatggctaagatgttcggtgttgacgttacttggttctacaccaacgcttacaaaccaggtggagatatcattttctggttcttgaacccagcaaccattgcgtttgccgttcctctgtacaaacgtaacgatattgttaaacgattctggttagagattctgctatcattaattattggtttgttcatctcactgttcatcatctactatgtatcaaagctcatcggcttgaacaacaacggaatcgcttcaatgcttccacaagctgctactaccgctattgcaatgcctatctctggtgctatcggaggtactcctgccgttactgctatggcatgtatcttgaacgccgtcttgatttacgctttggcaacatggctcatcaagatattccacttgactgaaccaattggtcaaggtcttggattaggtactgccggacacactgttggttcagcaaaggccattcagttaagttctgtatctggtgcgatggctgccatcgcggttgttatcatttcaatcgttgttgacatcgttgttccaacatttgccaacttcatgggaatcgctcactaattccttgcgagatcaaaagatcgtccatttgggcgatctttttatttacatatttttctcgaagttaggcgactactcaaacccaattatccctcccctaagcacgtttcgtgtctttcaagataattgcccacaatcctggtgaaaccggaacgaggcggttaaaaacacactaaaacaggccatccgttattgtctaatggatggcctgtatcgtatcgtttcatttaactactcacgcagatggtagttataagtggaaataataatattttgtcgtgaatttaaaattgctcttaatctcaaactagtctggttatgcaggacattttcccaacgatgtcttggcacaaattgtggtaccaggacagtggtcgaatagtttcgatcagctgcccgcttggcaatgacatcacagaaacgtaaggttggttgagcaatggaccgataggatgaatgaatatcaacgaatcggacatccgggaaatctttcttgaactgctcagacgtcttgtgttccttctcagggttggagtcaaaagaaacgtgcattgcgatgacataatcaccaatcgattgggcataactgatagcattggcagtcacccgagtgaccccgcttaccaggacaatgacagtcgaaccgtcaaaatggtgagttgtcgcaatttcagtattctcttcaaccacccgcagctgttcggcaacccgcttgtaatgatgattgatcttgtagaaaatcctcaaaagaatcggcataacaatcaaataaggccaaacatttggaaatcttagtaaaaacaggcaggtaaccaacgtcagtgaaataaaggcgccaacgaagttgataaccgacttcagctgccaattcttgccccgatttctccgccaatggataatcattccggactgtgacaacgtaaatggaatgaacacacctacggcatacaatggaatcagtgaattggtccggccaccaaagatttgaattaagacaatcgcaccaacggctaaggaaataatgccgttagagtaccccaaccgatcccctttgtcgagataggcatgaggtaagaacttgtctttagccaagttataagccaaaattggaaatgctgagaatccagtgttggcagcaaccgccaaaatcatggcagttgataattggaggatatagtagacaatgccatggccgaaaacagtttcaccaatttgtgaaaggactgtttcgtggctgtttggcataatgcccatgtagtaactcaggaaggtaatcccgccaaagaagcaggccaagatggtcgccatgatggctaaggtcgccgcagcatttttactcttgggtttgttaaaattagggacggcattactgatcgcttcaacaccggtcaatgaagatgatccagatgagaaggcccggaagaacaggaccaaagtcatgccttcaacaggtgccccaatatgagcagccgcatgatattcgatgttgccggttacaatgttataaccgccataaatgatcatcgcgataatcatgatgatgaacaaatacactggcaacgtcaaaaacgaagcagattcgcggattcctcgaaggttgaggagcataatgcccacaacgatcaaacaggaaatcaacaccccatgtgaatataatgacggaatagctgatgtaatggcttcagtcgctgaagttgttgatacggccacggtcagcatataatcgaccagcaaagagccgccggcaatcaggccggcctgctcaccccagttggtgctggcaaccacgtaagccccgcccccagagggataagcatggataatttgctggtacgacaaggtaatggcagccaacagaaccaaaacgagggctgcaacccaaatttgatacatcaatgcagctgcagacagcgtaattaaaatggtcgtaatctgctcagtaccatatgcaactgacgagagcgcatcggatgatagtaaagccagtgctttaaatttggttaaagattgaccaccctcatcagtggtctttaatggctttccaataaggagccgtttgagatagcgccacataaatagttactcctttatttaataatctaccattcttgtgaaccataaaatgatagtccttctgacaactaaaaacaagtcttgatatgtacgtctgaatgggctcacagcaaatcaccatccagacaagctaaaatatccgtcagctgtgcactcagagtcaaaatatgatctaagccacatgctaactactttaatattgaattgattaattcgcaagcacaaaataagcaccaatcccgatttggaatcgatgcttattgtacaatactttcattcaaatcaacgatttaacgcttcattacatacccataccaggttgtggcattggagcagctggtgcgtctttcttaggctcatcagcaacaacagcttcggtggtcaacaacaaggctgaaacagaagcagcattttgaagtgctgaacgggtaactttggtaggatcaacgattccgtcactgatcatatcttcaaatttaccattggcagcattgtagccaattccaggcttttcgtccttgagcttttcaacaatcactgagccttcaacaccggcattttcagcgatttgacgaacaggttcttcaagggcacgaagaacaatgcgaataccagtctcttcatcaccgccagcttcggcatccaacttggcaatttctgggatgacgttaatcaaggcagttccaccaccaggaacgaatccttcttcaacggcagcacgggtcgcattcaaggcatcttcaatgcgatacttcttttctttcaattcagtttcggtagcggcaccgacacgaaccacggcaactccacctgataacttggcaagacgttcctttaacttgtcacggtcaaagtctgaagtcgtcttttcgatttgggtcttaatttcagcaactcggttggcaatttcatcgtttgaaccggaaccgtcgacaatcgtggttgaatccttggtaacgttaactttgttagcttgaccaagttgttcaagggttgcatccttcaagttcaaaccaaggtcatcggtaatcaaggttgcaccggtcaaaatggcgatatcttggagttgatccttacgacggtcaccaaatccaggtgccttaacagcaacgacgttgaatgttcctctcatcttgttcaatacaagagttggcagagcttcaccgccaatgtcatcagcaatgatcaagagtgaacgaccttgttcaacaatcttttgcagtaatggcaaaatgtcttgaatgttggtgatcttcttatcagttaccaaaatgtaaggattgtccaagttggcttccatcttgtcattgtcggtaaccatgtattgtgacatgtagccgcgatcaaattgcattccttcaacgacgtccaagctggtatcaacaccacgtgactcttcaatggtaataacaccatcatgaccaactttttccattgcatcggcaatcaatttaccaacttcggtgttggcagatgaaattgaagcaatttgagcaatatcatctttggtcttaacatcatgcgacattttgtgaagggcatcaacagcggctttagtagccttttcaataccacgacgaattccaactgggttggcaccggcagtgacgttcttcataccttcattgacaattgcttgagttaaaactgtggcagtggttgttccgtcaccagcaacgtcattggtctttgaagcaacttcagaaaccaatttggcacccatgttttcaaaatgatccggtaattcaattgatttggcgatggtaacaccatcattggtaattgtcggtgtaccggcactttgttccaaaacaacgttgcggcctttaggtccaatcgttgccttaaccgtatctgctaatttatcaacacccttgagcattgcgctacgggcatcttcagaaaactttacttgtttagccatttcaaatttcacctcaaaaaaatatttttgattattgattcattgaatgattcaaatgattcacttattagcaattatcttgttaaaatataattattcgacaattgcgacgatgtctttttcatgaagaacgagataagtttgatcgttatcctcaatctcggttccggcgtacttatcaaacataaccttgtcgcccttttttacaacaggtgcaaccttggtaccattatcaagtacacggccatcacccacggcaacaactgtaccggcttgcggcttcttttttgcattgtcagcaagaacgataccgccaaccgacttttcttcttctttttcagtttcgataattacgcgatctcctaatggttttaacacgttagtccctccgtttgcaacaatttttagcaacattagcactcacatgataaaagtgctaatcactgtgtataatatattattttttcagaccaattgcaaggatttctgcgcatttcttggtgaatttatctgcagattgccttgccgacggtaaatgagcgcataagaaaagaccggcgttttcaggatcaccggtcttttcttcattaatttgttcgatattttacttgccaaagttttcgatgaaataaatcaaagtttgcaattcattagttaagtcaacattttgaaccaggacatcttcaggaacctgaagccgaattggcgtaaagttcaagacaccctttaccccgccggcgacagcatcgtccgcgatggactgagcgacttttgcgggcacggtcaaaatgatgactttgatctgttgatcatgcagttgatgtgaaagttcctcaatcgggtagacaggaacaccgtcttcaattgtgttcacaatcttgtcgtcggtatcaaaagcagcagagattcgaacgttgccgtctttgtgaaaattaaagttcaagagcgcatggcccaaattgccgactccgatcaaagccacgttggtcagatgctcttgattcaagatcgttttgaaaaacgaaagcaggttatcaacatcgtatccataaccccgcttgcccaaagcaccaaaataggaaaagtcacgacgaatggttgctgaatccacctgcaccgcctcggccaattccgttgatgaaattcgttgctttcctgtatcgtgtaaaatatttaagtatcggtaatatatcggcaatcgtttagcggttgcgcgtggaatattttcagctgtcaagaaaatttcctcctatttgtcattttagttaaaagaactttgtgaattcctatttacatctcattctaccataagatgacatcttgtgaaatatatttcaaatattacttacaaataattcctgaaatcgtgtaaattatgataaaattgattgttggtagttacaaaatgaaaggtggccaaacacttgataatcttacaagcacaagatctaaccaaacgattcaatggcgaaactattttctcaaaagttaatttggccattcaagaaaaaagccgtatcgcactggttggccgtaacggtgccggcaagtcgacactggttaaaatgatcatcggcgaacaatctgtcgacggcggccaaatcagcactaaaaagaatctgtcgattggctatttggcccaggataccggactcaattcagacaaaagcatttatgctgaaatggcatcggtctttgccagtctaaaagagcaggaagcaaagcttcacgctctggaaaaacaaatgggttctttgggcgttgacgccaacaccgaagaatatgaaacgatttcctcacaatatgacaatatccgtgccgactttgaacagcacaatggttatgggtacgacgctgaaattcgtggtgttctccatggatttggattcggggaagctgactacgatcggccaattaatgaattgtcaggcggccagaagactcaacttgccttggccaaattgttactggaaaagcccgaattattaatattagatgaaccaaccaaccatttggatgtggaaacgatcacttggctggaaggttatattcaaaactatagtggtgcccttctgatcatttcacatgaccgttacttcctagacagaattgtcactgaggtttacgagatgtcacaaggtaccctccaccacttcactggtaattacacggactacaccaagaaaaaagaccagttgattgaacaagaatggaaagaatatgacaagcagcaggctaagattcaaaaactgcagaccttcgttgacaaaaatatcgttcgagcatcgaccaccaaacaggcgcaggcccgccgaaaacaactcgaaaaaatggataagctgcaaaaaccgacggctgattcaaaaactgcccgcttctcattttcaccaaaatccaaaagcggcaataacgtcctgaatgttaccaacgcagcggttggctacagcacggttctttgtgagccggttaatctggacgttaaacgtcaccaagcgatcgcaattgttggtccaaacggtgtcggcaaatcgacgctcttaaaaagcatcttgggcatcattccatttttaaagggcaaggcgcagtttggtactggcgtcgataccggttactacgaccaggaacaagcctcactacatgcctctaaaaccgttcttgaggaactatgggatgatcacccaacgaccccggaaggcgatattagaagcattctagggagcttccttttctccggtgacgacgtgagcaagatggtccatgatctgtccggcggtgaaaaggcccggttgctcctaaccaagttggcgatgcagcacaacaactttttaatgttggatgagcccaccaatcacttggatatcgacagccgagaagtgttggaaaaagccctcaatcaattcgacggcacaattctctttgtttcccatgaccgttattttatcaacaaaattgccacggcggtcgttgaattgtcccgacatggcaccaccctttaccttgggaattatgattattatgtcgacaaaaaagatgagcaagaagccatcaaggctcatgaggctgaaaagaaggcagcgggccaaccgactccagttgctgtgccgaccaccgataaaaagaactacgagattaataagcaaacccaaaaagaacatcgcaaacttgaaagagaagtcaaggctctggaaaccaaacttgatgaattgacacaatcaaaggatcaaattgaagcagaaatgacgaagccggacgtctttaacgacctgggaaagttgcaagatcttcaacagcagctcgatcaggtgactgcccaaatcacagaaacagagtccagttgggaaacggccagtttgaagctcgaagataatgagtaacataattcaccaaaggcaaaagatatccgattcacattgtctacttgaacaattggcgacaacccactaaattaaaaagcagcctgagtaaaaggatttttaaagtgaacccctaaggttggacaccaaatctaaccttgggggttttactatgtcaaaatttaatttagaacttcgaataaaggtcgttactgaatacttatctggtaaaggttcaccgtctctagctaagaagtatcgcattagcaatcattcaatcattctggactgggttcatcgatttgagcggcgaggtattgaaggtctaaaagaccggtcaatgtcccaagaatattctagtcagttcaaagtcgatgtattaaactggaagaaacgaaatcaagcttcgcttccagtgactgccttacactttgacttgtcgtcgccaagtacgatttggcagtgggaaaaacacttccaggaatctggaatagcgggacttgagcgcaaacgagggaatcctaagaccatggtcaaacacaagcagaacaaccccaaacctgaaaaaccacagactccagccgcagaattgaagcagctaaaacaagagaatcaaatgttaaaaatagaaaatgaattcttaaaaaaactcgatgccttagcacgaaagaagtcaaaacacacgaactcatcgaactagtagacgagttaaggcagaattttcaagtttccatcaaactagttcttaaggctgttcgtattccccgtagcacgtattattatgctaaggagcatcgtggtcgtaacttagatgattcacaaattattcaggcaattgatgagattcgtcaacaagatccaaaatatactcggaaatacgggtaccgacgaataaccggtgctttacatgacgcttatggctttaaaatcaatcataagcgggtcttacggattatgcgggaacaagactggctatgtggcgcctttaatcggcagaaacgaaagtataattcttacaagggaactgttggcgtcatcgccccaaatcgacttaagcgacgattcaaaacagatcggccttaccagaagttagtcaccgacgtcagtgaattccgatatgggaaccaaagtcaaaatgaacgggtttatttagaaccagtcctcgacctcttcaatggagaggttctggctttcaatatcagtgaccacccgaccgttgaatttgctttaaaacctttgaaagaagccctaaatcgaataccggtgttagattatcggacaaccgtccatactgaccaagggtttcagtatcagcatcgccactggcaagacacgcttaaagagcaccatgtatttcagagtatgtcgcgtaaagccacttgtctcgacaacgccgccatggagtcgttttttcacattatgaaagtcgaggttatggatgaacattttgagaccaaaacagcgcttatcgaagctatgaacgaatggatagacttctacaatcatcggcgcatcaaaacaaaactggacggcaagtccccggtaaaataccgggaacttaccgtccagaaagcagcttaataaagttgtccaattttaagggttcactttatttatccttctgctcaggctgcttttgggttcttcgtcaactgttgttggtgaacaaaatattggagttctaatcacttggtgattagggctctttttgtatgaactcgaaaagcgaacagcactcttagccggaatctgaagaagtttcggtaaccaaatccagtgcgcttaatgactttaatcttgttgtttgaaccttctaatggcccgttggtgtagtggtgggtgaaagtgttgccaatttcatcatgatgagccgccaaggtttggagggctgccaacatctcttccgagcacccctgcaggtggtgaaaggcttgattatagttgggccagtcgcggtttttgatggtttcacgtaaccgattcatcacgtcgtaagtttgcttgagctcgggatcaatgtccagtaaagcatcaaccacatccgtggcagttgccggataagggaagtttgtccacttacggaaagcctcgtagttaaggtgattggccggcgttaataatagtttccaatagcgtttcaaggcgtgatactggcgtgaggaagtggccagggttttcatgagacgcactcgcgtcttattaaaagcccggtttaaagcgttaaccaggtggaagggatcgatgacaacgatggcgttcgggaagatctgcccaaccaatttgggataggtatagttcatatcggtgacgataattttcacattttctcgcgcggcttggtcataatgttggaagtacttttgaagctgatagatggttctaaagggcaacaggtcaatcaattcgtgggtttccgcgtccataaattcaaagctcatcgcgtcggtggcgctcttagtacttttaacttcgtccatgaggagaactttgggtaagtagtgccagttggtttgaaagtcgtgttcagcgcgcaagagctgccgaccaacgaatgaatccgaagtggacaattcattggcaatgtgtttgaggctcactggttccgttaacttctctaaacattgtttccgggttgtatttgaaatcgtgcagtgcttcggcactgcactcgtctgcgccaggaagttggtatgacaagccttacagtgaaagtttcgccgattgaggcataggataaccgtgctgcccaatgttttagcgaatctaatggtggtcttccgccaaccatagccaatgatctggtgatcattaataaccccacaattgcggcaggccttgggagaatagttcagtgatccatttaatctgattaccccatcatcacctattttgccattctcaatttttaagtgttcatcatctattcctaacaacattttcgtagtatcatttgacatagggcatttccttctttctctaaaatcttcgtggttgttggttttgatgaacggacaggaaatgtccgctttttttattctaatgaaaaacaaaaaatctgtcatcagtaatagataaaaatctattaccaacaacagatattgtagagcctgcttttgatctaagtattgaattatccttcatcacaggatcgctgacgatttcataatcacctcaaaaaattggcaattatttagcctcatctgccagccaatcaaactccaaacccggatctgcatttaaagtggcatcaccacgaacaccatgccgatacagcatctcaccggcagcaccgatcatagcagcattatcgccacacaaagacagtggcactagttcaagtttggtatcggcaaacgtggcaacctctttggttaaccgctcccgaagaccttgattggcagcaaccccaccggcaagaattaattgtttgaccggaaattctttgagcgcgcgattggttttgtcagccaagacgtcaacaacggcttgctgaaaactagcggccaagtcttcacgactcaattcctcgttaatttgatcagcatggtgcaccgtattgataaaggcactcttcaacccactgaaactaaagtcaaaattatcgtcagcatccattgctcgtggaaaatgaaaagtatcctgacctttgtgagctaattcatcaactggcttgccagccggatagttaatccccaaaacccggccaattttatcataagcctcaccggctgcgtcatcacgagtttcaccgataatttgaaattggttttcctcaggcatgtaaaccaattctgtgtgcccaccagaaacaaccaaggccattgctggaaactcaatgggttcgaccagccgggcagcgtaaatgtgcccagctaaatgattcactggaacaagcggcaaattgtgcgcccaggcaaccgccttagcggccgtaacaccaattaaaagcgcaccgactaagccaggaccgtatgtaacagccactgaagtcagttcatcataagaaacgtccgcctcacgtaatgcatccccaatacagccggtaatctgctcgatatggtgtctgctggcaacttcaggaacaactccgccaaagcgttgatgactcttgatttgcgttgcaacaatatttgaaagtattcgattgccattctcaatcactgcgaccgacgtttcatcacagctggtttcaaaagcaagtactaaatctctagccacttaattcatcccatcccttttaaccgattttggtgatgtccaaaaccatatttaaagcgtcttcacgatcgttaaagtaataatcttttttaatcccgttatcaacaaatccaatatcccgatataatttttgtgcacgggtgttgctgacgcgcacttcaagcgtcaccttggcatattccaattgacgggcctttttgataattgttgtcaccaaaaaataccccaagccatgattctggaaatttggggcaaccgcaacgttggtaatatgacagtccttagtatgatcgtttagcgagcagccaataaacgctaccagccagtcgtttcgacgcaacactaaatataggcgatccgttttgcgcatcagttcggttcgaaaggcccgatcatcccaaggggtctggccaccgtaaaccgcccgctcaatccccagaatctcgggaatatccggaatcattgccttggccaaaaagtactcagttccattaatttctacatcgtggtttttgatgtcgagatatctctcgcgaagctgaacctctttgttataaaattgttggttaaaccactctttaaactttttcaacatagtcatgcgtatcctcattaggatgtaattttttccaatcagcctcagccttggttaaccgcaaatatcgtgggacaaccgcatcaacgactggtactggtgactgactcaatccatacaagcccagtaaggtcgcactgggaattcccaaataaggattggcaaccaccagacggttatgcagaacgtcgcgcatcgatctttcaaatggatcggtatcccctaaaatgataatccgttgatcgtaacggctaacggtttccaaccattttgttagattggtgtgctgatcctcgatcacggtttgaatccgacgacttcggtagcggtataatcccgtaaacatgttttgattccggccatcaaaaatcgggttgatcagcacatcttcttcttgaacattcaaggcaagatttaacaagctggaaactggtaccagctcgatttccaaggtgcttgcaatggttttcgctgccgtgacagccatccgaatgccggtgtatgatccagggccggcagcgacaaccacccgatccaaatcagttggcttcaaatcggccttttgcaccaagtcttcaataaccggcatcaagaattcggcatgtttgcgatgagtggtgatggttgtttgcgccaacagttggtcattatccaaaacagcaactgaaagtggttggtttgaggtgttaattgctaagattttcattattaatcgttaccctttgctttaatatccttccaaacaattgtggcacttgctgaaagaacatcatttgatttaatttcgtgaactgttttaattttagcattatctgaagaatcaacaagcactgagctggtgacccgattgccatacttaacctcgttctcaaagcggatatcaatgttcgcgggttcgtgttggttcaaaaagtccattggcaatgaatccaacatccactccggatacctggaattattgacgtggccgttaaaatcaatatcgctccaacgaacttggtattcctttgcgctaacatcatcagtcgcttcaattcgttcaggacgtgccaatctgggaacccgtttaaccttctccgactgatatggggcaataatcgtttcgtcaatcggcgtaattttgcgggtctgttcgttcattaacacccagatactctccaccttgaccagctcgttgccagcttgatcgtgcagccagaattcccgaaaggcaaaataacgattatatgacgtgcctcgggttgtcattttgacgactgaatctttgcgtggcaagtgagtgatatgaattgagtaagaagtaaccacccagccaactccataatgatcaattaaataagtttgatcaaggcctaaattttcgttctggtgttcggacgccaaaatcaaaatattgatcaacattggaattgaaatccggttgttgacgttacactcgtaaaacggaatcgtatgcaattcgctaaaactgtgagcaggcatggacattccttctttctatttgatgtcatggtactgattatagatgacctgtttttttaaatgatgatctttggcaacctttttgattgcttcattaacgctcaagccattttcgatgtaaaagtcaacttgttgatcaacgctcatcccggcaagcggatcatcaccctgcgtttgtggatgggcatttcctgacactataataacaaattctccgcgaatttcagttgaattggcccattcattgacctgatcaaggtttccgcgaatgaattcttcgtgctttttggtcaactcacggcagagagctgcctgacgatcccctccgagctgagtcgataaattcttcaaagtttttttcaatcggtgcggggcctcgtaaaaaatcattgtctcttctcggttacggagctcatcaatttctgctcgctgttccttcggctttcttgataagaagccatagaaataaaatggctgcggcaaaagcccggaagcaattaaagcagtgatcccggcgttggcgccaggcagcggcacaacgttaatctgctcacgaatacaggcaaccaccaattcatggcccgggtcgctaatcgacggcatcccggcatcgctcacctgggcaatcgtgattccctgcttgagtttgctaatcaactcgggaatccgctcggcagtattatgctcatgaaaactgatctgcttggtttgaacatcgaaatggttcaacagtttctgtgtgttgcgggtatcttcagccgcaatcaaatctgcagactggagaatcttaaccgcacgaaaagtcatatcatccagattgccaattggcgttggaaccaagtacagcgtgccatattcacttaatgtgtcaaaactcttttgtgtgtccactgtttacctcttaatcgcgtttgccatagataatgtccgtacagaaaatacaatcttcaccgttctcccgtcgcttaccgtaataagaactgcagacatgaaatccttcattgtacagtttttcgagattcttgcgagattttgacaaacgtggcgaattattgtccattttttcggttatttcgttaatccgatcgcgcaaatgctgattttcaatctccagctcagcgtttttttccatcaacccaataagtgattcatgcaggtgagaaaaattttcagcactcgcactgagctgtgtatccatttcttttaattcatcatataagttttgactgtccacgattttatcaccctttagtaaactatgattgcccaattgcgagtatctttagtgtcaaagcttcaattatattttgaaaattgacgttaactgccatccggctattcatatcaagcagctcgtcaagcatggttaacagttgatcgttattccactgattggccgccaatttggtctgtgcaagaatcgccggatacttcacccgatcatccgccaaagtcccgtatttcatttccaagacatcgtcaaacaaactcagcatcatggaaataacaatccgctgacggtccttgttggtaattagaggcatcaaagacatttggatgaaaggcattgccatgttgttttctttgaccaaataggtaaaccatttttccaaaagccgctgcatcgaggcaaaccaatcatctttggacagctctttaatctgatccaaactattggtaatggaaatcattaagttgacttcactcggcttgacaccactattctgtaattcttggaccatctgctttttacttaggctgggaaattccacaacctgagttctggaaataattgtcggcagaaccagattgcgattctgactgatcagaaagctaaccacgtttccggtaggctcttcgataaactttaagagactgttagctgccccagtggtcattttttcggcttctgaaataatgaaaacctttttggatccctccatggcacttttggtaaattcacttttaacgtggcgaatctggtcaaccttaatactttgaccatcaggttcggtgatgacaacatccggatgatcatgattcatgattcgcacacattcggcacattttccacagggcatgccattttgaacattcgtacaaaaaagccgcatggcaactcctattgcgactgaaaattggccggcaccatcttcgccggtaaacaagtatgcgtgtgacaattcattgtttttgattaaattcatgaattgggtaaagatggtcggctgtttagtttgagcaacgttaacaatatcgtgttccataacgttcccttctagaactgtttaaaatcttcgattggcaaaatcataaccgtagcgccaccaacttgaacttcaattggaaaggtatgttctgccgtatcaccgttcaagctgaccggcggtgtcataaattgttgtctagcggaacaggtttctttgattagtttcaaagttatatcaacttttgaatcatcaacggcgaccagataagtggtatttcctgctcgcagaaagctaccggtggtcgagaatcgggttgcgatgatatcgtgagcaacgaaaactgatcgcaacttgttggcatctttgtcttgaacgatcgcaatgactaatttcataatcaactctccttaaaatactcactggcaatttggtggataatcttaattgtatcattaacgacgcgattaatcggttgagttgcatcaatactgataaatcggtcggcattttcgtcacggaccttcatataaccctcatgaacccgtttatgaaattcattggtttcaacatccaaccggtcaattttactgcggtcgcggtgttcggcgatccgatccaggccaacgtcaaccgggatatcaaagtagatcgttttgaacggtaacaacttttccgttgcaaactcattcatcttggcaacttgtgccataccgatctgacggccggccccctgataagctactgaactgtcaacataacgatcacacagaaccaatttattctgtttgagtgcgggtaaaatggtttcaaccagatgctggcgacgagcagccgcataaagcaaggcttccgttcgataatccatctcagtattctcacggtcgagaatgactttgcggatttcttccgagattttattgccaccgggttctcgggtgaccaaaagttgatcgccgatttcctggttaaaaacttcaatcacgcgattcatcacggaagttttgcctgcgccgtccggcccttcaaaggttataaacttaccattcaaaacaattccctcacttttaatttaaattaattgtacttgctgttcgtttgcctgtcgattcagccaacgcttatatggtccggattattcaaaattgtcatgatcataactgataaccgagggctgaatttggtaattcttaatttttcgaattcgtgcctctttatatatgaagaaatatttttgacgggccaacgcagtttcctgctccatctccatatcactgtcagcaaccgcttcttgggtttgagcagcatgatcccactcttctttcaaattgttgattaactccaacaagcgatcgtcgtattcacgtttaacattttgccgtcttaatcgattaaaaaacattcgaaaaatcccaccttgtcaaattaaatttcagtccgtccttggactgccttaaacaacgtgacttcatcagcatattcgatatctgatccaacggataatccgtgagccaaacgagtcactttgatcccagcgggtttaatcaacttgctcaagtacattgcagtggcttcgccttccggggtggcattggtggccacaatcacttctttaacggctttattttgctggagtcgtttgatcagtgaactaatattaaggtcttcaggtcctttgccttcaattggtgacagtaccccatgcaaaacatgataaaggccgtggtactcctggaccttttccattaccatcacgtctttgggttcttccaccactaggatggttgattgatcacgggttttatcacgacaaatttcacagggatcttcatcggttagattaccacaaatcgaacagtaatgaaggtcgttcttggtggcaaccagcgcctttgaaaacgctttgacatcatcttcattcatatcgacggtgtaaaaagcaagtctggtagctgtcttactcccgattcccggtaacttcatataactatcaattaactttgcaattgcttcaggatattgcatactttcccctttttttcgtgcggactacattcccggaatccctttggtgtatttacccatggtgctttcagtcgctttatcaacctttgaaagaccatcattaacagcagctaataccaaatcccccaacatttcggggtcatcgggatcaatggcttccggcttaatctggatatccttcatctttttgtcaccgccaaaggtcacttcaaccatgttatccggggcaacgcccttaaattcctgctgtttaagattctcctgttcttcacccagttgcttttgcatctttttcatttgcttcatcatcttgttcatgttcataccgttcatcattttcttttcctccaattaatcatctttgatatctaaaatgtcggtgccgaaaagttcggcagccttcttaacgactggttgactgtccggctcttcttttgtcggttccggatcgtcatcagccggttcagcttttgggtcgtttgcttctttggattgggagccagccttttttatcttgtctttgtgactggccaaatactcacggcgaatatcgggccactgattttccggaacaaacacaatttgaggggcttttcccacaatacgatccaaattgttttcaagagcatccttcaaatcagtgtcgccttgagccttctgatacaaaaatgggtattcgaaggcaacaattactccgccggcactggcagccaccggcgatgacacgtgcatgacagcccgttgggtcaccgacaaggcatccatcaagtccggccaaactgatttaaattgatttaattgtttccgggtggctttacccaaaattggatagattttagccagctcaatgtgattgtccattgagtgagcctcactgactttggcaggctccggcgtgctgactgttggtgactgaggtgtcgattcccgtttgagatcggcaacttccgccttgagttcggcaacttgctgcgtcaattgttgaatttccgcattaacttccggggccgcggccgttttagccgactgctgtgattgtggtgctgaaacggccttgggctgatttgtggcatccaaatgggtaattttgaccgtcaagacctccagataaacatctggatgagcggtaaaccgcaatgaattagaaatcgcattcaattcattaatcatctgataaatggcttgatcgctgatctggccacttaaggtcttgaactggtcatcaatgatccccagttccatttcttcaacgattccggggtcctgttgatacaacagaatatcctggcagtaactggtcaaatcttcaatgaaccggctggcgtctttaccctcatccaatattttttgaatggtgatcaacgcgctcttggtgtccttgttgaccacctgctgcatataggtggttaataattcattggtcacgctgccggtcacaagtaaggcgttctcataagtaattttattgtcaccataagacatcgcctgatcgaggatactcaaggcatcccgcatcccgccctcagcagctttggcaattaatttcaaggctttgtcgtcgtactcaacctttttttgatcaaggatatatttcattctttccaaaatatcctgaggtttaatccgcttaaagtcaaatttttgtgtcctggagatgatcgttgccggaatcttgtgcggttcagtggttgctaaaataaagattacgttagccggtggttcctccagcgtttttagcagagcattgaaagcccccgttgaaagcatatgaacttcatcgatgatgtagactttgtaatcagcctgagttggggcgtatttcgccttgtcccggatatcccggatttcttcaacaccgttgttggaagcggcatcaatctcaatgacatcatttaaactgccctcattaattgctttacaagtctcgcactggttgcagggctcaccatcttttaagtagtgacagttcactgccttggcaaaaattttggctgccgaagttttacctgttccccgaggaccggtaaacaaataggcatgactcgtttgtttagtaattagcgcattttttaatgttctggtgataatcgactggccgacgatctcatcaaatctttgtggtcgccaaacccgatataatgcttgatagctcattaccaaatcctccaaaatagaatgccaaattcttaaaatcgttcaatgaaacgtctaaataattatatgatgaatccaaccagagtgcaatcaacgaccgtctgactttcaagaaatttctccaaaaaaatgcccccagcaaagttgctgagagcaaaagttctatgtacaagaggcacaaggttgatgatacttagtgctgcttccttccggacctgacacagttcgtaacccgacccttgcctcagggccttgcggcaatatctatcataacttaaatgattcagaattgccagccttattctttcttttcttacgcgcagccttgaagaaatctttcatgatccgcgatgccgcatcggcataaagcccttcaacaacgttgacttgatgattcaatcgggaatcttccaacactgcatataaacttctggttgcgccggctttgggatcacgagagccaaaacaaacattttcaatccgcgaattaataatcgctccggcacacatcaagcacggttcaatcgtcacataaagatcgcaatcaatcagccgccaactccgcagtgttcgacaagcctcttggattgctaaaatttcagcatgggccgtaccgtcatttaaatgttctcttagattgtgaccacgcccgacaattgtcccgtcatggacgaccacggcgccaatcggcacttcaccgattagataggccttgtttgcttcgatcagtgcagctttcataaaacgactatcagcttgaaacatttcgaaccctcacgatttcttgatgctttgaagaatgtagtaacctttgtcccgttttaaaatctgacagtcaccaaataattcggtcatcaatttcttggcagatggtgcgccctgctttttttgaagaaccaccgtcaaggtgccgccatcaactaagtgatcgactgccccggagatcatggcatcgacaactttcttgccggctctcaccggtgggttggtcacgatggcagcatactgatcagtaatcgcttcatatatattactttcaaaaatatgaacgttatcaacccgattagcgtcggcattctttttggcaagcgccaaggccacctcattgacgtcaatcatatcaatctgccgatccggaaatgctttggcaattgaaatgccaattggaccgtacccggttcccatatctaacagtttgccgtcaggaataaggtcataattaatatgattaaccagcacccggctgccgtagtcgaccgtatgtttagagaacacaccgttatctgaagtaaacactaagttgtttccaagcaacgcaaagttccatgtaatcggatcggattcaacgttgggattctttgaataataaaatgattgttctgacataaaattctcctaaaatgatcttttataatcgttatctatatttggtgcttacaattagttttgtcacaatatattgtgttttaatcgttgcatttcacactatttagtgtaaacttgaatcataaattaaattttaacgaaacaggggaagtgttaacaatggctaaaatcacactatattcaaagaacaactgtatgcaatgcaaaatgacaaaacgttacctttcagaacacaacgttcaatttgaggaacacaacatcaacgagcaaccacaatatattgattacctgaaacaacgagggttcatggctgtccccgttgtcgatgttgatggtaagcaagcattcagcggctttcgacctgatcagctccaatcgattgccggctaattgccttcatccattctaacatattgatttcagattagcgggcgaaaccacaaacggtctcgccccttttattcgcaattataagaaagcgtggtactaaatatgtcacttcacaaccttaaggatgttacctactttgatttgaacaacgaaattaacatccccgtcaacgggcagattccactgcaaaaagacaaggaagccctcgaggcctttttaaaagaaaacgttcagccaaacttaatgaagtttgacagtctcagcgatcggtttgattacctgatcaaaaacaactattacgaagccgattttattcataaatatcaactatcctttgtcgaaaaactgtaccagtacttaaacgatcaggatttccactttaaatcatttatggcagcctacaaattctacgcccaatatgctttgaaaaccaacgacaatgatttatatctggaaagcttcctggatcgggtcgccgctaacgccctcttcttcgctgacggtgacgagcagttggcaatggatttggccgacgaaattgtccaccagcgttaccaaccggccacaccaagcttcttgaacgccggccgggaaaatcgtggcgaatttgtatcttgttttctgattcaaaccaccgatgatatgaatacgattggccggacgattaattcggccctgcagctgtcaagaattggcggtggcgttggaattaacctttccaatcttcgtgaagccggtgccccaatcaaacatatcgaaggtgccgcttccggtgtggttccggtcatgaaattacttgaggacagcttttcatactccaaccagttgggtcagcgtcaaggtgccggagtcgtttacctctcagtctttcatccagacattatcgaatttttgggtgccaaaaaggaaaacgccgacgagaaaatccgcctgaagactttatcattgggagtgaccgttcccgataaattctaccaattgattaaagccgatgctgacatgtacttattcagcccctacgatgttgaacgtgaatacggcgtgccattctcttacgtcgacattaccaaggaatatgataatttggttgccaatgacaagatctccaaaaagaagatcaaggctcgtgatttggaaactgaaatcagtaagctgcaacaagaatcaggttacccatacatcattaatattgacactgccaaccgctccaatccgattgccggtcgaattgtgatgagtaacttatgttcagaaatcctccaggttcaaaccccatccactgttgataaccagcagcattacatcaaaatgggcaaggatatttcctgcaatctgggatcaaccaacattaataatatgatcgctggcgatgactttggtcattcagttgaaagcatggtccgcgcattaacatttgtcaccgaccactccaacatcgacgtggttccttcaattcaaaaaggcaataaagaatcacattcaatcggccttggcggcatgggactacacagtttcttagccaagcaccatatgtactacggctcgcctgaatcgattgaatttaccagtgtctacttcatgctattaaactactggagcttagttgcatctaacaagatcgccaaggaacgcaaagaaactttcgtcaacttcgaaaacagcaagtacgctgacggcagctattttgacaaatatctggacggatcatttgcaccaaaatctgccgaagtaaaagctttgttcaaagacgattggattccaactaaggaagattgggaaaacctcaaggaatcagtcatgaaagacggcttataccaccaaaatcggttagcagttgcgccaaacggttctatttcttacattaacgatacgactgccagccttcacccgattatcaaccgaattgaagaacgtcaggaatccaagattggtaagatttattatccagccccatacctttcaaatgacacaatgccttactatacttcagcctatgacatggatatgcgtaaggtgattgacatctatgctgccgcacagcagcatattgaccagggaatggcattaaccctctttatgcgttcaaccatcccagaaggcctgtatgaatggaaaaacggccggacagacaagatgacgacccgggatctcaatatcttgagaaactacgcatacaaaaagggcgtcaaatcaatttactatattcgaactttcactgacgatcaacaagaagttggttccaacgaatgtgaaagctgcgttatttaaaggagaaattcatgactgagaattataaagcaattaattggaacgccatcgatgaccaaatcgacaaggccacttgggaaaaattaaccgagcaattctggctggatacccgaattcccctgtcaaacgacctatcggactggcggacgctggatcaagatcatcagtgggttgtcggtcacgtcttcgggggcttaactttactggatacgctgcagtcccaagaaggaatggcatcgttgcggaaagatgttcagactcaacacgaaaccgccgttttgaacaatattcaatttatggaatcggttcatgccaagagttattcctcgattttttcaaccctcaacacccctgatcaaattgatgagatttttgactggagtgacagtgaggaattcctacagaacaaagcactcaaaattcgcgacatttatgccaatgaaccagacccactcaagaaaaaggttgccagtgtcttcttagagactttcctgttctactctggcttctataccccactttggtaccttggtcacaacaagattccaaatgtggcggaaatcattaaattgattctccgtgacgaatcagtccacggcacctacattggatataaattccaaattggctacaatcaattgccaaaggaaaaacaagaagacatgaagaactggatctacgacttcctgtacaaactgtatggtaacgaagaaaagtacacccatattctgtacgatcaaaccggctggacagaagatgttctcaccttcattcgttacaatgccaataaagcgttgatgaatttgggtcaggatccgctcttcccagacacagcagaagatgttaatccagtggtcatgaacggaatctcaacatcgactgccaaccacgatttcttctcacaagttggtaatggctacctcttggggaacgtggagtcgatgaaagactcagattacgatatttaaataaatacctcacagtaactcaataaggctgatgcatccccgctgggatgcatcagccttatttttgtctaacaatcactaatctactaaatcctttggagtcttcccgttgaccatcgtctcaagattccccagtgagatatcaatcatatttttcacagcttcactggtatggaatgcggaatgtggcgtgaccaagacgtttggcatcaacgccatcttcaatacatccggatcattgacttttttggttgacctggagtcttggagatcagcagattcattttcaattgtatcgatcccggcaccagcgatttcaccgctctggagggcaaaaatcaaatcatcggtatcgacaattgagccgcgagcagtattgatgaggattgctgtatccttcatttgctcaaacacctcatggttaaattgatgataattatcatcagttgccggcatatgaattgagataatatcgctctcctgataaatttgttccaagcttttggcatatacaaacgagttgtcggtatttttcagcggatacttgtcataggcaattacctttgcccccaagcctttgaacagcttgatagctgcctggccaatccgtccggttccaatcaccccgacggtctgttcgctgatcagacggcccatgaagttgggcgaaaaatgaaattcatgcttttgatccaactgctgacgcatatagcccacttttctagagaggtacagtgacatcatcacagcaaattcagcaatactttctggactgtacgccggcacattggtaattttaacgccattggctttagcggctggtaaatcaatgttatcaaccccgacatttctgagcgataagtatttgattcctaagcgtttaaatgactcaaataattcagctgaatattgaatcgtttgaaggcaggaaataccgtcaaagccggctgcttcttcaaccgtctcctgattcaaagttgtggtggtgtatttcacttcaattccgtgatacttcccccacttctcaataaacggtatttcatcatctcggacattgtatacaataaatttcatagttgcctcctagtgatttcagcttaaatttggttccgcttccattttaccaaaaataattgttgaaacaaaatccaagtccacctgcagaggccaaagttgagtgaatccctgttgacaataaaaatagagctggaaatcaaggacacttatttccaaccctatttcaaattattttagttgatcaatgaaacgatcaaaggctgcttgacctttgtcgtcccatttgtaaacgccggcatcttccagaaccctgccaaagactttgccaacttcttcgtcgactacctcttcaacattgtccttggtaaaatggtcacgtttcatcaattcatctgcccaaggcttatgataatcagcaatttgattatcttcacccaagacatacttttcgacttctttcatttcggtcttcagacgagcaggcaaaattgcccggcccatgacttcaatcaagccaatattttccttcttgatgtgttgaacatcttgatgaggatggaaaataccatcaggatacttgtcagaagtttgattgtcccgcaagacaatatccatctcaaactggtcatcattcattcgggcaatcggggttaccgtatgatgtctggttccatccgtgtaggcccgaatatcaactgactcatctgagtagttcttccaagtttcggcaatccgattggcagcattcacaactttattggcatctttgctgaccaggcgaatggttgccattggccatttgacaattcctgccgacaagccatcaatccccaaatcaaccggtcgatcaatcttggctttcatcatcgggaacgtgtggcgaccaccttgatagtgatcttgagccaataaggaaccaccaacgattggtaaatcggcgttgctgccgacaaagtaatgtgggaactgcttgatgatgtcaaccaaattgacaaacgtccgttgatcgattgacattggcacgtgcttttggttaaggaaaatcgcatgctcaccaaagtatgcataaggtgagtattggaatccccacggttcgccgttgatcatcatccgaataacccggtgattgcttcgggctggatagcctaggcggccgagatagccttcattttcaatggctaacgggccaaccggataactggttgactttgcccggccagcggcagcaatcgccttaggatccttctcaggctttgacaggttaatggtaatttccagattgccataatcggttttggtttcatatgaaatatttttggcaatcgcccgagtcttaatataatcattgtcttggctcatatgatagaagtagtcggtggcggcatcaggagattgttgatacttgttccaaaagatctgattcaaagttgatggaattggtgttaacaggtccatcagttgatcttcaagaatctccctgttggtaatcgaatcttcgaccttaccatgttcaatggcgagatccaccagatcgttggctaagtcgacagccgacgaatcctcggtcgactctccaaaaccatcgccgatcagtctaaaaatcaggttggtgacataaatccggtcaacatctgaatatggtgaatcagatttgataattaaatcgacaaacttttcaactgctgattggctcatgattactgatttcctttccgatcgtcataaccctttgggtgggtttctttccaattccaggcggtctttataatttcgtgaacgtcatcaaattgaggcttccagccaagaatcttgcgggctttgtcactcgctgcgatcagcgtgcttggatcacctgcacgacgggggcccattttggcaggaatcggcttgccagtcacatcacgggcagcatccaacatttgtttgttggaaaagccggttgatgagcccaagttaaaggcatcactatcatgaccagcttggagatacttcagtgccaagatatgcgcgtcggccaaatcaagcacgtggacgtagtctctgacgttcgtgccatcaggcgtatcataatcgtcaccaaaaatcgtcaactcatcacgttcgccggcagcaacttgtaaaatgatggggaccaaatgggtttcagggtggtggtcttcaccaattgagccatcaggcttggcacctgcaacgttaaagtagcgaagggcgacaaacttaatgccgtaagccacatcactccagtgcatgatcttttccattgccaacttgctttcaccgtatgggttggttgggacctgcggatcagtttctttaattggaatctgcttgggttccccataggtagcggccgttgacgagaagacaatcttcttaacgttatgggcgttcatcacttcaagtaaactaatcatgccaccagtattattgtcaaagtacttcaatggcttttccatggattcaggaacaactgagaatgctgcgaagtgaatgaccccttcaatctcttctttatcaaagacttgattcataaagtctttgtcacggacatcaccttcatagaaacgggccttgggattgatggctgctttatggccggtaaccaaattatcaaccaccgcaacgtcatagccattttcaattaatcgatcaaccgtgtgcgaaccgatatatcctgctccacctagtactaaaattgccatttaaatatcctccttctaatcaattcgttacttaatctctttaggaccatctgaaatttctgcaatgtagaattctgccggatggccaatctctttctcatagacttcgccaacatttttggtaaaggcatcgacttgatcacggtcaacaatcgcaattgcacaaccaccaaatccggcaccggtcattcgcgcaccgacaacgcctggttgtttccaagcagtttcagctaatgtatccagttccttaccggttacttcgtaatcataatgcagtgaaacgtgagatgcattgactaatttaccaaaggtttccaagtcattattgaccagcgcatcctttgcctgaagggttcgttgattttcgaataccgcgtgacgggcacgacgaatcaaaacatcatcattgatcaggtaactattttcatcgaattcactttcactcaaatcaccaagagatttaattggcaatcccacttggagacgcttcaaagcctcttcacattcagcacggcgttcgttatatttagaatcttgaagctcacgatgtttcttggtattcataatcacaataacccgatctcccaatttggcgggaacgtaatcatatttgagggtattcgtgtccagaagaattgcttgatccttcttccccatcccaatggcaaattggtccatgataccggaattaacaccgatatatttattttcaaccagttgaccatatttaaccaggtcaagttcgtcgatccccagtgaaaagacatcattaacaatctctgcagtcaacagctcaatagatgctgatgaggatagtccggcaccatctggaaggttaccataaacagcgagatcaaagccatggccaatcttatagccgtgttcgagaatctgaacgagcatgccttttggatagtttgtccagccatcttctttgttatatgccaaattgtccaacgatacttcaacaattccagcatcggaaacgttgccggagaacatgcggatcttgttgtcttggcgttctccataagctgcgtagatgcccatgctgattgcacaaggaaatacgtggcccccgttataatcagtgtgttcaccgatgaggttaattcgacctggtgagaaaaatactttgcttgagtcataaccgaacttgtcattaaatagcttttgtacgtcatcagaaatcataaatttcatccctctacatatattttagtaaactttactaaccaaaatttaactcattttggcagcgttgtcaaccttaacttcacaattccctcacttgtaaaatacaattgagaatccttgatatgattgaaccacttggatgttggtgaagacttcgtgaatgtggataaattttatgaaaacgcttcatcagtttccaaacaaagccttttatatcaaggtaaatttcagtaaacattattttgatgaaaaattgttggtatttttacatttaaccgcacaaaaaagccagcagatatctgttaaataccttccggctgctgtttaatgcgattgtctgccaggttacttaaccgacaatcaattaattttcgactcagtccgccttatttgggctgattggcgtccataatgtaccagagagccttggagaggcctgccggctttttattgcgcggttgattaacaaccaggataatctgcagaaccgcgtaaaccagcccgcttcgacgataatacgcaatatattttgactcccacttatcaacgtacttgtccttataagaccggagtccctcaaaactataaagcttataaccgtattgatagatgagatgaacaatccgctcctgagtgaaactgaagcgggaagttcccacatttgagaacggtgacatccccaagtcaaagtacttgtatcctttatcgtgggatatttcataaagattaatcaaaatgccatccatgatgcctgatggggcatcggcggaggaacgcatgagatcaatcgaggtgaccactttattaccatccggcatcagattggcaaacgcaacaattttgccggcatggtctttcatcacagcaatcggtgcctgctgaaggtagtattcgtcaaaaaagccgagtgagaaacccttttctgctttattatccaaccactcgtcagaaatcttccgcagagtggccagcaactcatctgaaaacggtggctgtagaatttcaaactggtagccttcgcgatcgaatttgtgcattaatgcccgttcgccgcgatgtcgtttaccactaagagtgaactgatccaagtcaactaatccatcctcaccggtcttgataaagtcaaacccggtttcgtgaaggctcatggttaattcttcatcaatttcgtagaataccagtttcagatctgatttatcagcttccttgacaaaatcatcaatcgcgtcggcaaattgggcacgattgccgaccggctcgcccataattaacagtttgtcagcaattttcttgaacatgaagaaaacctgatcttcgccgtctttgctgtaaaagtaaatctgcttatcgcgcaagaatgccagatgactatcctcattgccaccgaatttatcaatcacagccttcacccgatcggcatcaaatcgctgtgtcagccattctggatggccggcggtcaagtaggcattcatcccaaccagaaccgccagggcgatcaataagccaacaaaaccgaccagccaggcacccgcagatggaaaaagataagctttatcaaaatggagatgaagatttcgattggcagcaatcccgatgagggtataaattgcaaatgtgatgataaaaattgacccattaaacaggaacacaccccaggaattagccatccggtcccggtataacaccgccttggagagccgcagagtgattaggatgatcacgaacagcaagaccatccgccaggtaaacgcctcgttaaaccatgtgttaaatatcgaaatgatcagcacaaataccgtaggggcatacgctttcttagttcgagtccagataccactcgccaaaccgattaagaggaatgcaacaataatattcatcatatgactgacgaaaaaaatcgaatatggcaatagtttgacatacagtttattaacaaccactacattgggaaccgtggcaaacaacaacatcataattccggaaaaatacataaagccagttaagaagacttgggcaatccgttgaaacagaagtcgtggtaggtcatcgagaaaggtgttgagtttggacccggtatcgtgaatgaacagaccagtgcccacaatgaatggtaacaagtaataaaacagacggtaaagcagaatccagaccagtgcatcacttcgggcaacgccaatgaatcccagtccaatgatgacaaagatatcaaaggaccctaatccacctgggatcatcgagacgaccccggcaacgttggcaaccacaaaaatgggcacaaccaatcggaggtcaacgggtagattcatgagataaccaatcaaaataaagaaccccagggcactcccccattcaaggaacgagccggcggtcatgaccagttcctgtttggttgacaggtcactgaaaaactgtgaattagtcacttgggtaaaaatcatcaccccgggaaaatatacggcaccgcccaatagccaaatccaatagtgggcaaattctgtcccgatcccaaagccaaagatcatgatcagtgaaaccaagcaaagtaaagaaagccctgatatcagaaacaaagcaactttagaaattgcatagaggatctgtttgcgggtggcccctttgccatagaaatgcgcgcgtaaactgccgcccaacaatccgccaaaccccagtaaattcgtaaaggtattcaccacccagccacttttaacgatgtagccgggtgaaaatttagttggtaaaaactgaacaattgaatagtcgtacaccagcatcggcagaattgaaataaagcctgccaccagcattatcaaaagagcgccgcgactttgactggccagaacggttttgaactgttcaccgttgacttcacggataatcttagccaactgtcgaataacaaaaatcaaaacggagaagacaaaaatcagcttgatcatggtcatccgtttgtcgatgaattctttgacacgtgtcattattgttccaccatcatttcattttgaatatgtactcttcgtctattatgccaattaattgaatttcacacaacaaaggtgcacaaaaaaggttctacaatatctgttgttggtaatagatttttgtctattactgatgacagttttttgtttatcattagagtaaaaaagcggacatctcccgtccgttaacttgctcccaccacagaattaagtcaagaaaggaaatgccctatgtcaaatgatactacgaaaatgttgttaggaatagatgatgaacacttaataattgagaatggcaaaataggtgttgatggggtgatccgattaaatggatcgctgaactattcccccaaggcctgccacaactgtggggttattaatgaccatcagatcattggctatggttggcggaagaccaccattagattcgctaaaaccttgggcagcaccgttatcctctgcctcaatcggcgaaactttcactgtaaggcttgtcataccaacttcctggcgcagacgaatgcggtgccgaaacactgcacgatttcaaatacgacccgcaaacaatgcttagaaaaactgaccgaaccggtttcgctcaaacacattgccgatgagttatccacttcggattcattcgttggtcggcagctcttgcgcgctgaacgggactttgaaaccaactggcactatttacccaaagttctcctcatggacgaagttaaaagcactaagagcgccaccgacgcgatgagctttgaatttatggacgcggaaacccacgaattgatcgacctgttaccctttaggaccatctatcagcttcaaaagtatttccagcattacgaccaggctgcgcgagaaaatgtgaaaattattgtcaccgatatgaactatacctatcccaaattggtggggcagatctttccgaacgccatcgttgtcatcgatccgttccacttggttaacgctttaaatcgagcttttaataagacgcgggtgcgcctcatgaaaaccctggcgacctcatcacgcgagtatcacgccttgaaacgctattggaagctattattaacgccggaaaatcacctcaactacgaagctttccgtaagtggacaaacttcccttatccagcgactgccactgatgtggttgatgctttattggacattgatcccgagctcaagcaaacttacaacgtgatgaatcggttacgtgaaaccatcaaaaaccgtgattggcccaactataatcaagtattccatcacttagagggctgctcggaagagatgttggcaaccctccagaccctagcgactcatcatgatgaaattggcaatacctttactcaccattacaccaacgggcccttagaaggttcaaacaacaagattaaagtcattaaacgcactggatttggttaccgaaacttcttcagattccggctaagagtgctgttcgcttttcgagttcatacaaaaagagctctaatcaccaagtgattagaactccaatattttgttcaccaacaacagttgacgaagaaccacaaaaaaactgtgcatcgacaatgtcgatacacagttctgagaacaattatgattaagcaatgaattacttaagggtagtaacgacaaataccactatggtagtgatagaataacgcatttgccataaatctgccacataattctttttttgactcagatttcactatttttcgctttattctcgtatttaatactacgaggtgatgaaactaaatttcacctcacaaaaaaagcctcgcatactggcgtaccagccacattaaatgtggagcgaggggattgatatctatgacttatttatactcttctaaaatcagagtgtcaatgtttatctctttaaatacaaaaagcccaccccgaaattaatcgagatgggcgttaaacaaacatcttttaattaagccgcagtatatgttctatataagaacttgaatgcttcccgatcatttttaggaaacatagccatcacgagagtgttaaacattaaagaatggctgctatttctatgacgctgattaaagattttattcagtttactcgatggcatttgcaaaacctcaagaattttttgtcccttctcaaaatccgttagtttactggattcctgaatttctttaattaaaatcattcgatggttcgagtaatttttgattccattagtaacctgattaaaaaatgaataggttttattgcgtctagaaagccacgccacatcgtcactgctcataatcattttgcttttatcgcgtgccatttgatttaaaaaattcttgaatctctttgcttcttttattgatattcccaaatcttttgaaacatccctatcttttgttgcagataattgaactgctaaataacgatagtaaaaattaattacgtaagcagtattctcattcctatctctttgttcttcttttgaaaatctcactttaattgaatctctaatgagtgaatatgaaatgcgtgaattctcaatgtaaacaaatactgttaaaaataccgacatagcagaaatcagaaacgctaatccagaagcagataacaaaattgcccagaagctattcatcgttttcacttccccattctttaggttttgaatatgtccaaaatatcatatcaaatatttgaacggtaaaagaaagtaataataaaactgccgtaaaaaagcattgccagaaattcaaatctttattatctttcacaattagtatataaccaaatgtaagaaatagaagtgcaaaggtcaaagtaacgatgactatacccaaaaatttgataagcgtatgtccctttacctttgccaaagaattatagaaagataacttgatgagtaatctgaaggcagtcggcatagtaagcgtcaatgctgaaaaatattgcacaaaggaaattttaatatttataagcatatataccgaagctgcaaaggtcaatacatatattcccacattcaaagttaaaagtaatccttctttattgtctttttcacgtattagtgtataaacactattcggatcagcttcgcgtaaatgtttaaaatatgtgtcctttgacaaagcaactatacctacctaatttcatcatttattatacattctaattctgataataaccaatagcaatactcaatatttaaattggccaagagatgttcagcaagggcaccattcgtcactcctggcttagttcttaggcttagacttttttaaaaacttgacgtaccatttatttgatgaaacatagccttggccgttaatgtacagccgtgtaatcttgccatacttaactggtatggcccagaaacgagagccagtaccgtagcgcgtatatcgcttgcctgactttttaaaatccaagccattatataccggcaaccattttaatcgaacttggtaaagcccaggagttacatagtaagatggcttttcactggtcttgctcccagacagtgaaccatcaaagtcgtaactggcatcaacctttagtcctttaaaatcatcggtaaactgccaactatttgcgttggctaccccaggctgcgaaacgccataggcagccacccaaatatgcttgtcaataagttccgatcgcttaattcgtccagaattgaaccaggaaccgctgccgtaggtgatgacatttttataaccggcattgataagatagcgcaaaaagacgttcacttggggagttgtattgtagggcaatccggatgcttcaacatcaattgctagaactgttgacttatccagcccaaacttcctgacccaagccaaaaagtaccgcgcttctgctgtcccatttccatgaaagaagtggtaagcgccaactgcaccaaatactttataggcattcgtcacttgggcggatgctttcggattcaagtagttggtgccctcagttaatttgaccatagcagcatcaactccatgagctttaaaagttttgaagtatgaaactgatgatccttggtaactggcaagatcaattacaattttaggcattctgatcactccccgaatttgctgcaggtttttcagcactttctgcaggcttggcagctaccgatgctgtagtagaaggctctgcactggcacttttctgcgtgctttctgcagaatttgatgcttgtgaggcggttcctgctgaacttgcagcagttgggtcggatacttgcccatcttgtgtgtcagaatccgtcacttctggtgaagttagcggagcatggttgtcatatcccagtttcttaaattgttgatatgctttctcgacaaccgaatcgacaatttctggagttacccaggttagcccaagttttgccgcaaagtcagcgacatctttgtcggccgcctttttccggtcagatttggataatcccgccaatgtggcaaacttggtaacggtcgttagggcgaaatcagtcaactggttgatttgtttatttttgatatgaatctttaagtatggttggacttgcttcacgaccacaataatcagagccaccaatgcggctagaatgccggtactttgaagccagctaaaaatatcactaatctgtttaaaaatttgcataatattctcctcctaatgtaataaatgaatgagttgttgtagaatcaaataaatcacggagcttgagccaatcgcaatggtaaccaccttccacaagttctgacgattgataacttccatctcgtttttatgattttcacttttctcgtctccacggatgacggcttccaagatacggttattttgttcccgcaaatatttgttgctttcatcgacactttttaaagtgtcagtcattttattgttaagatcagtaatccgacgctcgtgatccgataattctttgccatgtttcaataacatttgatgatcctgatcgcttagtggcaacggcctcacttcccttctattttgggtaaaataaaagcacctatcggggggacaggcgctacttcatatatggggatatatgaaattaaatcataaacaataaccgaaaagatatattggagggtaatatcttttaaatatgactagtaaccaatgtaccggttacccagccatcggtatcaagttttacataataattcataaaaattttcctcctatgagattgtgaccgaaccacctgtaaccgcataaatgaaatttccatagccatagactgtacaggtattattcttaaagttgaacgtgattgattcagcatgggatccggttccctccatgttattaaaatagaccgcttcaaagctgccagagatatttttattgcttgacatggtaaagctaccaccatcattttccgtcatatggaatccgccaaccacatagccaacgtgtggattattcttgggcacatagataccaagagaaccttcaacatatccagaagccgtcataggaatgtagtcataatccgagatgttttcaaagaccttattactgccaacataaaccttcttgacgggttttgcatttatctcaatactcattccattaccccctaacttgcgtcatcatcatagatgtagtagtaagtgttcggatccttggtggtaatcgcatcaaactgagcctgggtaccattccaagtcttcggtaacttagctaaagcagcctgtaaatcggccatagtagcggcctgattatcccccttatctttcgaggcgtcatttatgactggcgcaatactgaatgtctgaggagcagtaaatgtgttagtctgtcctgttcgtgctaggtcagacggtaaactgcttgctagtaataacggattattattaaccgttggaacggtatcaaagttgttagcaccagataggtggggtactttggaatcgtcagcaagaagtttccaagtcgtccaagtagtagaatacattgtccgcatatacgtattatttagctgtacaccatatgctatttgaatagttgtggagataccatatccagttttaaaacaatgaacgtaataaaagtcttgaggaagtccccagttagacaggccacttgcagcccagccattaagatacatccatcccataggaatatcattcatatccgtatatcctacgtcaattcttccaataatattttcattagcagggagaatactagctccatttgcagatattgtaccatcgtgattgtcatgaacaactttactatcgtcagcaggtgtgtaaccaattttatcttgtttagcgttaacttcttcgattcctgcgacatcgctagctggtttacgcatatctgaaacgttaacttttttatccagttgctgattaacgtcaaccgtcttggcgtaagcattccactcactccaaacattggttgtagaattgaaatagcgagttgatcgaatgttgttaattgtatcatctaaagtttgcatgattggcaccgtcttatctccactaccaatcgtggtcaaataaccagttcccgaaaaaccacttggagcatttaccactgtggtatctttgataattctggtaatgctgatatctaaaatggtattgaaatcagtacctttcgaagctgtctcatttggataatttaacgcatttcctatcgaatgagaaatcatctgttgaacatcttcacgggatagggtaccactgtttgaaaccataatggttacttgggtaccacgaacgatgtcagtatatagatccagataaatcgaagctgttgtcgcattgttttctttagcaatcattgtcgctccggcagttaatggaataacactgaataatacctcttgattggttgaattttgtttggcatagaggccgacaccatagtaaatatagtcttcattcacatcactgttatcaatggtcactcctagccgagacttgttgtcttgtgttgcaatggctttaggtgttcgcgattgcttatagttaacactagttaatgcttgtaattgtgaaaccgaatcaccggtaatatcatcggtaatcgtcactgctttagtaaaggtaattgcgctgattcctaaagcttggttcatcatggttaatgcttgattggttaatgtatttttaccccaagttgctggcattagttaatccctcgattctgtataataaaacggctttgagtcactgccacatttccaacatataggctttgttcatcaatttgactaaattcagttccattaattcgaattgtcgcttccactgaccttgccagttgctctgtcaggaaccgaacggcatccggatcactggcgtattgaaatggtaatcctgtaatggtaattgttcgcgcttcaccaccagtttgccatgattgaataattcgaacatccgaatactgacaatctaagatataagcaactgctttaatgatagaatctgtcgttccgtcagccgtcgccgctaccattgctgctcgaattttaaatttgtaaaagtcatcgttcgccccagctcggtaaacattaaactgttcgccaaaatagtctaatgatttacccgtcaaatactccaatgaatgaaaaatattcattttttccaacgcggtatcgaaatcattcgagcgctgcagaattgcattcataattttatagaatcgactatcatattgttgattggtcagacgactcattttgctcattaatgttggtgtatcgtccatttcaatcaggttatcatcatgtttgatatcagccattggttgtcgtcacctcaatctcatcagcattaaccactggtgcttgtgtgatgcctaaagtgatatcagtagctgctaacttggctttatctaagcccatttgaacaacaaatgaatcaatgccttgaacttgagctagtgcgccgtatactgcactgatgtaaactggtcgtcccatgtgtaggctattgacataattctgtaaggcatttagtacatcgtcggtaccactatcggcattccagttactattcgccttaacggtaattgcgaagtaaatcggaacttctgttgctcgattaaaatagatcgtttcgggtgtgcccgcaatatcgtaggcaaccgctgataagctgccgaatgtttgagtaccggcgcctttggctttccgcactgcattggcaatgtcctgatcagttccaccatagacaacaatttgaagggcatgtgctggtgtcccattagcatctgtcacgccgctagtattattatcaatgtacttgtctcgaatcccgttcacactatccaaagcggtatagataccgtcaattgttgagccaatgttagcaacgttggtttctagaatccgttggcgtagtgaatcatccgtttcttcatctgcaccccccacagccggttgtggattatctacggtatcaacgccatcaaccggtgtcgcaaactcggttatcgtatgggcttgcacattggtatcactcgaataatcttctgaaaccaccgatgcggtagctgtaaacgtgccatcgccatcatcatcagaaagtacagtatcttcaactagcacaaaataagtgccatcgtcagtcatgaattcggtagtcccaccttcaagtaaaaccgcacttgtacccgtaatatttaccgttgcattcgcctgttgggactggttacgaaaaatcccccgattataagctagataatcgagggaaacaccgctggcaaactgcacgtaggcatttagccaaacttgttgctgcttttggttttgtttccaattattataggcaaccgcccgtataattcgaccatagacggattgaggagcaacattaatgtcatcaccagcattagctttaaaaatggcagtctgtttggcaacttcttcagcataactctcaacataataccctgtttcatcaaatgccactattgtcacctactgtcaatttaatattcccttgatcatcatactggttgccagaatcctgaatttctgaggaatgaatatcgactgaaatagcactcgttcgtttggttatatcgtgagtgatttgaacatcgtcaacggcatcgattcgtgattcttcattagttaaagtatcagagatatcttgcgctgcatagttatcgtcgtatgcttttcccagaatattatccaacggcaaaccacaatcaggggctagttcattcatttcaccttgttcaattcccagcagttcagcacatgattgaaacagttcatctgttccagaaacttctactaaatcatgtgtgagttcgtcttgctgaggatctcccgaactatcaatcattagatcccacatatgatcacctcctaattaattgcgacaataattgcatcgttaagatcatgctcacgtggatcatcttcacgttcaaaataacccttgccaacttgatagccatctaaacaataatcatgaataatcatggtcacctcagtgcccttcaccaatttcttaggtggcggggttactttagtcgttccaggaccatctttgggacaaatgggtgcgagataaccagtgatgtgttcccagacctcgtcaacccaatagacactaaaaggcacttctacgttgttaataattcccattttatcgccagataaatcttgaactagcggctgaacatcagcagtgtgcgcgattttatcgtatttcacaatttttcccaccaggcaattatgattatctctcgaagctgcttgagcaattgcttgggcggcttttttatagggatttgttatcttcgccaaataaaacacctcctatgttttgggaatggctccgtcaatgaccatggttggctgagtgccatcaaaactataagttccactttgagcaactaatgtcttttgaataaagtcaccccgaacttcatacgtactgcgcactccaatttgtggcagaagataagaagtggattcatataatgcgtcaccagagtcagaatcatctgaataggatggttcgcttaacaatccagacgtgtaatctaaaataatatgcgatgttttgctctcttttagatcatcgatttttagctgaccacgatcgtaaaacattttgcttttacattgcttaactagcttggcaatagcatccagcggtttacccgataccgtataaccttttttaaaaggtttatcttgagccaatttcattaccgtaattttaatgcccgattcatgggcaatcttcttaatcgcaatcgacggcttaacaccttttttaaaggataggttcgaataaaccttctttttaacggtgtaacgagtccgcttgattttagtcttaccatcaatatgcacatgtccttccttgtaatggccgaccttcttaccatcctcatcagaatagtaatgaattcgtcgcttaaccgtcttaccttttacattgaccttaactcgtttataatggccgactttctttgtcttttgcttttgaatggtcttggcagaaatactactataatcttccccagaggagaacgtgattggcaacgtagtggttacaccatcatattgaatcgggtcaactgacttaatctccccttcatcaattagtgttttaccaattccttggtacgaaataaaaaaagcgattttatttttcgcttttagataattccgaatatgttgattggtattaatgaacgaggcatctgactctggcggtgttgaatccatgttgaagttaatatcaaaagtgaatagcaaatccgaaccaggtcgcaagttattctctaattccagctttttaccactttgcgttgtgatcgtacagtaaagtacgggaaaacgaatctgattactcattcgtatccccctctaggtcaatatcagtatcatcgtcggtatcggcaccactgctttcattggtgtcggcttctggcgtttcaaaaccggatccatcagctggccgatcatcaaacgttagcttaacggtatcaccaaagttatcaccattacactcgatctcttgtccagattcatccatagggactaaatcttctgttggataatcatttgagttaagagatgcaaataggcgttgattaatcactaacttttcaccatttactaaggcattcccatcagcatcccataaacgtaccgtcaaaaagttagcaaatttgtttaagtcaatttccatctgataggcacggccacctaaaacaacatcaaagggtttcccatagtcttcaggtgtaatctctaaagtatccagtaatgccatttaaccaccttccttatgcaactctgattttgactccgtatggtaaaacattgacggccgacttatattgattcatcgaaaccaatttggcaatcgaagtattatagtcagttgctaaactggcataagtagttccctgcttggttgtcacgtactttttattcacttttttgttcttagtcttgtttttcgtgccactactggcatttgtaccactggtttttaattctgaccaatcaatgaactgaaggctgaaagtaatcgttaaagctgtctcttgcttgttatactctcggtgaagtgcagtaaataaacagtgcttgtagtagatgcgccctttataggtcatttcacaaccttcggccttccatttaagcaattgattgtaagccgttcgttgctgggaatcagttcccataattcgggctgtaatcgaaatgtccttctcagtttgctgcgagtgagtcgctgttggttccccttttggtaatgcgttcggcgttacctgaatcgtattgtcctcggattctggtactgatgacatgaagaccaccgcactgctgtggcggtcggttcggtacaacatggcatgccccacattgaacttactacgattagtcgcaattttttgagcaatcttagatttgttagcggttacctttgccgcagtatttcgcttagccagtgttgatttataagtctttaatcgcttgttagcctttgacttcgcattggtatgtgctttaacggacttatttgccttatcaattctcttcttaaggtttgctttagtagtcccactcgctttttcatatgcttttttatccttagccaagcctttgttcagcttggcaatggctgcagattcatgcgcaacttttccactttctttcttaatgtctgcttttaattgcttatcagttaaggcctttttatttttggacatcacttagttcccccaaactgatcaataatttggcgcgccatattctgtcgttcgcctttgagagcctgtttaatcatcttgttgattgcacgttgatttagttcaacgccactgccaatattaaactcaaatttatcatgcgtttcaatatggacagttggttcagttttagcaacgtgacgataactagaagccgaaaaagccggcttcttgataactcgttcgagttctctcagcattttgccaacgcttaaagaagccttcatcatgttagttgccatcaccgcagtatctttggctgtaaatactcgtccagaaacatttggcaagaagagttcggcacctttttcgccaacaattgaagctttgttagtctgcggaatgccgccccgtgcaaatctacgagtcccatgtggtcctgatcccaaccaatcaaatttacgcttcccccaaatagttgtcataccggttgcatttttgtattgactattatttaaataagctaggacttgatcataaggactattccaattcttatgtccagaaacggcataatttaagaaagtacttttaacaaattgaagtggcccaccagcaggattgcctgaagccgaattactatcgtgaatttgctgagcaatatttctattcccagattctgaaaacgccattctgatgatatcagacataactttcccacgaatgctgctgggaactttcataacactctcggctttttttatcattgctttagttattgaactaccgcccatttggccaccaaagcttccaccggatacttgaagattattctcaacccatttaagttgtggtgcgagctctttggcaactagctttgataatgcactgctatgcttggtgttagttttcttatttcctttggaacttccaccccgtagcttggtaatatcaaaccagccatgagttgaatccggattgtttgaaaatggattactcttagaaacaccaatatggacatgagtaccggaagaaccaagtgcagcaattttctgaccagtttgaacattttgacccatcttggcatacagaggggcgccagaattgtttttaccattaaattcctggtaaataacatagtagccatcacttgatctggtaactaaactttcaccaataccgttagctccaccccaacccgatggagcaccaccttctcgaatgactttaccaccatgaacagcatgaacaacgcgtccgccggagaaatcgacaccatcatgaattgcaaggccgccaggagtagcaccacgatagccaaatccagacgttacagagaatccagaaccgggattatgtgcccagttaccaccggcaccgcttccaccaccattacgagcatttttcatttgtttccaaacttcatcagcccatgggttaccatattttccatacgcacccttagtcgtgttggtagcgccctttgataagtctgtcccatgcagcttaatgttaacggtcatgtttttcttgagccaaccgctagggtctttggcacttgagttaatcagcttcttcaggaatgcattagatacgcctgaacctttggcatagtgagtaataccacgagcctgcgatagacgttgcatttgtgtgccatttagtacggcatccccacgctttagtccgatcacgcgattcttaccctgcggtgcgtatagactgttgccacggatgataccttcttgacgtggtccagactccgcatcgttaaccattgcaatttgatcttcacttagttgaccattcgaaccttgagcataatggatcgggttaataaccgaattattgccgccaaattgtcctaatgacttatcgatacccttaatcccgttattcagctgattaattgtgttagacatcgctttatgagcgtaattatccattcgaccaagtgcatgaccgaatccagtagccgtatcatcagccgcattcgtgacacccttgcgaacttgattcatttgaccttgaacgcccttttgcatagagtcaaagtctttgactgaactcttacgaatattgtttgtataatcgccggttttgttgtagatgtttgaccattgatgcctgttctgtttggataattgtgacaactgactaacactacccttctgagtagcgtcataatcatcaatcgtatttttcttgatcttcttggttgatttagatgtgtcagaataggttttatcccaaatccttttggacttcttactgaacttatcaattgaaccatttgcttttgaagttcctaagccgtttgtgccgttggcatagccaggtagtgattgcccataactaccagacaaaactcttttggtagcttgagcattcaaaatatgttccccaggctttaaatgtgccagttgtggcccattaacacctaataagcgagcttttcgaccacgaaccgtgtaagccagttccagtccaccttcaccaaccagtgcagtttgagcatgggtgattttgccaccagtagcataagaactgtattttgataaatcattagtggggttgtatggtcctttataagacttaggacgcctgcctttagtggttgtcgtaccagcattatttttgccatagttcttagcgatattgtcggtgaagtcgcctgagttaaacttactctgtttggtttgtagaccagccttgatgtttgatgtgatcagagccggaatcgagttgccgatatcctttgccgctttgctaaaggcattgacagccgcaccggcctcttttctggctgcttcaacaatattttttcgctgcttctcagcataggtagtcgtgctcttatattgctgtttagcattggcaatcgtgcctgctcgctgcttttccgcagccttaacagcattcttataacgattgctattaacaccatactcagccttggcagtgcttacctctttcttgtatcgcttatcagaggcagaaacttcagcattataagttttcctagcattggcaatagtcttctcttcgttcttcttgctacttgtcagaatctttgcatagcctgaagttgttaaatgcgtggtggaactcattagtccacgcataattgcctcttgctttctagctcctttatcagttaaagaaacgatttgccgattaacactattgattaatttggcacgttttgaggcactaagattttcatcagaatctatcttgtttaagccggtgtgtaagtacgccaaccgcttttgaacactgttcttatcggctgcatactcactagcagcagttgcattactgataatatggttcttcttcaagtaatccaaccgcttttgggaagcactaaattcttgtttgccttgattatttgcaagttgagctaacttcccgtaaattgacttaactttattacttgttttgccagcagaatctgcccatgcaatattaccctgttgctcaaggttgaccgcctttttaatgtaagaagcgttagccttgcttaaacttgcatatctccaagaattaactgcactcttgacagatgtcgtttgataagcactaccacgaccagaatccctaacgtttgttttaccatgttttgctctataagcagcacgggcttgccgatcgcctaaagagtttgccgcaacagctgcatcgccaccagacaatgcagccccagcgttaccgggtgtggttctactattatccgttggattaatagaaccaccatgctcgatattttttacgtatttgcttgagccaaaggctttaccaattgcgccaccaatttgagcaccaataccagcaccggcaggccctccgagaaaagcaccaatgccaccgccgacaagttgtccgcccgtttgccaagcagccttagaaccttgcgaactagtgatacctttggtgaagattgttgaagcgttgttgattgcttgcacgccttgaatacccaattgcagatagccatagcttttagcaactccgccaagtttgctattatccatccagttacgtacgccactgcgaataccactatagtgaacagccccacttctagaaccaatctcgggaacatcagtattaaccggaacattcccatttgaattcactggctgtttagtatttggaactgaactatttgaatcactgtttaaccacgagatactcttttttaagattcttgagcctgcatatgcagtgcccagcccactcgcaatagcagttgtataaccggcaacttctttcactggtgcaggcattttgatcagcgtatttaagaatttattaccggtagataaaagcttggtgaagccaggcaagaccgttttagtaaaatccagtcccatgacattaagatgctgtttaaagacgtcaatctggttttgccaagaagacatattcttctgagctaagtcttgaatgtagccgcctttgccgtatttaggagctttctcaacttgtgcattaagcgacttcatctgcttaacattgtttgacaaaattagagcagactcttgaccggttgcaccaaataattgatggaataacgtcgctttttgagttcctgtcatgcccttcatgtgctggttaagaagctcgaattcatcatctaatgactttaaattaccttttgaactccgcaaatcatccggtgttaaaccgatcgatttcaaggcagacacaccttggcccatcatgccacttgaaggggcaagcagtgagttgatcaccttacgaagaccagtaccagcaaccgaaccatcttggccgttgttagaaagtaccccgatatcagaaatagtaccagctaaagattgattaccactcttggcagtcgcaccagcgtactttagggattcgcccatgccactgaaatcggtagcggataaatcggcaccatatgccatctggttaagcaccatcttggtgtaggcagccattttcttctgcgaatctccagccttagtcttgtaaccaaactgttccaaagccggtgcaccataattaacaacggcgctgtaagggtcgccagaagctcgcgcagcttgcaggaagtacttgtgagaagccaactcttgtgcaccagaatacccacgacgaaccagctcttcgccaccttttgccatagaagtcggtgaaacaccatattgcaaagcaaagttattgttttccttttccattgctcgactttgagccttggaagcagaagccgactcaccgccagtgtgcagcaagttttgaatggtcttatagcggttctccagctcggtagcttcgtccgccgatttcttgaaagctgccgcaacgggaatcattgccattgcaatcgtattgcccatattggtgagccgactaccagcgtcttttaaacgaccgaaactagttgtggttttgtcggtttcactgcgcgtgcgtcgttgagattccgagaccttattacccgacttgttggccgaattacctacccgtgacagatgttcattaaccttattaaggttgtcattcgtcttttgagtagcttcgctattagtcgctctattccacataccggaaattttgtctttcgttgaatcagcagcccgacctaaaagcgcggtgtgtttggcagcaatattcaaagagttgctgccctcgttgccggtacgtttggtagcatcaccaagtcggttcactgaatcaatgctttggttaatcgaccgattcatttggctgtagttgcggtcagctaaatcaccggtgcgcttgatctcggtattagcttgagccatcccacggcttaaaccggtagtatctccagttttagcaagctgtttattgacaattgcccatttatcaaccagcttatcagttagttcattagctttaattaaaggtgcaagatcagcttcaaaacgaacgccaattccttcatcacgcattaaatctccagccatttttcttacacccctttatttaccaaaaaggccggtgtttacaccaccggcggttacgttctgcaatcgcttgtagtgcaaatcggccagtttaatgtaatactccagctctgttgcggttgcttctttcaattcattaatatcgacactcagtgcctcgctgatgtaccagtatgtctcgtcttcttgcgccatcttttctgctagaaaagtatttgcttcgccaaaactagttttgaagaaaggaaaccgtttctatatagaagtctcccaaaccggtatgggtatcgaagtaatcccagttcaaagtttgcggtgagatcaagatgttgctggttttgtcaaagaccgcatccaagaagttactttcccgaatcacaccagcggagccgcgtgagtcatcaagaatggcaaccgcctggcgacggccagggaattgttcagttacagaaatttctttttcgttctcttcatccaccgagccgtcaggcttgagtggtgcacttttaaaagtgaatttatgttgtcgtaaacgagcctttacatcgttagttgcagttttctttgtagtttcagtcatgagaaattcctccatttattttttaatatttgtatgtactcaaaagggctactaccggagtagcagccctttttgagtaacttagattaccgaatagccaaggttaacacacgttaatccccaatcacgggcagttaaagtgtttgagaatgaaccatcaggcgctttagttacccaactatgctttgattcaatcatttcattatccgatttggcagtaaatgagaagtacttagatgctgccagcaagtcgtttagatctttcatttttggagaagcttgtgacaaatgcaccgtcacagtaccatgcttgtcattggactcagaacctgtaccggttccttgagcatcaataaccaagttgacgttatcctcagcttgagtccagccaaccatatcacctgattgaaagccaaaaagggaaataccatcgacaataatcgacacattcttggcattataaatactcatcaaaccgctgttatcactgttatccatgttgtatccctccttagttcattaccgagccgttgattgtgacattatgaatagcaccggaacgggtatacgagaatgttccaccgttataagcacgtgccaaaatatcggtttgtgactgttgctcacgagtactgaaatcagtatcataagcgcctttaccatcagcaccggttaagataatgccgttattccaggcatcattaagcacgtcccgaacaatctgttccagtgtatcaatacccactttttcataggaaactttgccgttcttagggtcttgtaagcgggcctgaatccgattacgcatctcaacctttacccagatttcgccatgcaggttatcgatatactcaccggataatgtgaagccttcggaagtctcaccaacggagctgccagtggtggtaaagtacacaatcacatgcgcttttttcattgctgtaaattgtgtattgttatactgctgaggtgtgatgccggccacatttttgaacttccaagtttgagaaccaacagtaagggaggcaaccgcaccaactagaccagcatccaatggttcatttgccggatgctgaaggccaatcgtgtaattttgggaacccaaagtagctaacgtggtgtaatcctcaacttgtagaagtaggaatttaccggcattagtttcgaacatgttagttaactcagttgccgtattagcgtcgaatttatccagaacagcaaaataccagccattccagaaaaaatcagccaaggtatcagatgctttgcctgttgggtatgaaacaatcatgaggtaattgccgtgttcagtttgatcaaaataacccttggccttggcatatggggctgatgattcatcataatcagtcgctacctcgtcaagcgatgtatattctttataattgccacccgtaactgatgcaattgcaccagtgggtgctttatagcccgtagcagcttgctcagtcataattaacagatttccataaccaacattgggtacgggaatgatttcttgaatattgataacaacatcagcaatttgtggcactaacgtagttgccattattaatcacgctccttgttttctttgatatttgtttgagtaatttgcggcttatattgatcggcaaccgtgtagtcgtcgcgaacgatgtaagtcactgtaaatagaaaattgtaatcttgggtttgattcgctagaactgtgttgtctaccaccgaatccagtttgtagggacgcatgttggctttactaaactcaattaatacgtcaggacgataaatcgccttacgaacagcttcaagattgtcttgagcttcataaggcgattgggcgtgcgattcaatttggactccggtaaagaacagttcattttcaaccacgtcaatggtggctaactgatgtgagttaaacgggacaatggcaaagtacggaaacggcggtcgtttatcattgctattgccataggtggtttctaatccagtcgcatctttaatgaccgctataatgcgattcataaaatccagatagctaaatgtttggctcatctttatcacttaccttcaattcataaatcacgatatcggaatatccctgaaaatctgtaattgatttaatgagatatttcattcccgttcggacatccacaaccacagaatctttagggaaaaacttggtaccgactagttccatgtcaaaatccaaatcagtaccagtatttcgttggtaagtcatagcagcaaaagtcccaactggtacgagtgcccatttggcttcaaggtcaggcgttctatcagtaattaactgatgcgttttaaagccgccgctagacgcactcttatcactgtcagcactataaatttgaattggcacacccattttcttgacgatgctacccatttttaaatgcatattaaaacttccttacttcatagataattgattgagctaaccggccagtatcgaccaggggattatcaacaccatgcttgcgagcctttgtggctggcgcattgtgaggcgttttccatcctatgattgcttttcgaatgtctgctacaacgatgttgcccatatgatgcatacaaccctcagccgtttggcgactcatgacaatctcatggatttggttgcgatattctttagtccaagcattaaaccgtttgtcataagtctcagtaaagtaatgtcgaggtggaattatgacttccttgaccaaatagaacattacttgccccgaatcatcgaccagaatacctttaccattgccccttgtcctaagatgtaagttgtcataatccttagcgcttttgccacgtggcacgtgttcactcgggatagtcagatacttactgttaatcggcttgatatgtgcaccaaattccagtacatgggcaatcattgccaaattgccgccttcctctgacagaacacctacgaacaactcccgatgcatcagcttctttagttcaggaatgcctttttccagatggttataactcattgtggtaacaccgccaaactgatacgtggcataccgttgtcaccatatagcgaccataagcgataataatcagctccccaggtcgttagttgcagccactttaaccagtcctgtgaaccagccttaaagtaagtaacctgaattggcccaactttttcagcagaaactaacgttgaagaggtaccaacaatgtacttgtggatggttaaatagcgttctgccatctccagaatgtcagtatcggtagttgagaagccatcatgagtcactttgatatgcgcatcagagatgtattgctgaatggtggcttcggcaacatcctcaaacgtatcaggagccgagtttttaacggcatcaatagtcgtgtaatttgccatccagctcatccccttactttagttttgctttgatagcatctacaacgcctttacgatttgcactggtggtttcggattttaatagtgcttctaaaacactttcatctgaaatcgttctaattgcattagtagcatccgcaacattcatgtttgccacatctggcgtttcaattggtgcgtaggtcgtcgcactggttgctggtgtatccttagcaatttgtgaaacgtcctcaacgattaattgtccgtcagctaccaatggcttaatgagcggatcggcaagggcctttttaaccttgttagcttctttttgaagcaggttattcaagcctcgttttatcatcacgccattaatcacacggttaaattgagttctgttttcaactttgaccaaagtagcacctcctaaacgttatcgacacggtttaccaaataagggcgacgcaagataatgccgcctaatcgttcgtacaaagcaatccggtgagtccagaagttgacaatctcttcctgggtgcgagtcatttcgttagcaattccaatttgaaccgtgtcaggctgattatcaaagataactagtgaatctttgccaccttcgccagcgcctgctaattcgggaatcgaaacaatacttgagaaccaattattagcttgaagaactgccataattgaacgagaatcataatcgctataacgacgattaagttcttcgtatgcgtttggagccaatcctagaactggttgaatattcgaaaagccattaatcaatgttaatgttttacgtgctttgcgcaacacttcaacaatagccgcagaatctgtaattgctgaaaatggaccatcggtatttgtggtaaccgtactatccggtgagttaaacaacccattaatgcccttagtttgatcaccaacaaagcagattgagttctctttctcggcaatggctcttgcagccgttgcaattttagtgacattgggggttaaaccagccaaatgagcctgttgaagttcttcatcggtccaagttgcacctacttcaattcgaaataatgattggtcaactggtaacaaatcagtatcaaccatcggaatatcgtttgaccgctcatcagcaagcttggctttaccaaaactgcgagcaacaaagtaacgataagaagtagcaccctgtggaatatctgtatatgtgctgattaagcttcgagctaaaagtgatcgttgaggcgcttgataaatagttttatcaattgcttttaaatctctagcttccagcgtttcatgagaatttggcattttttaaattcagtcctttctatgatccacttgcaatagtgtaaggcgctccaagattcagttgcactggtgccgtggaaacttgtccaaaatcagtatttgaaactgacgaagtgttaaatttaccatcgtctagaaattgtcctatcaccgtatcaccagctacagcagtcttgaaaacaccatttgctccaactgttgctgggtcgccagcttttacatctgcactaatttgaacagtaactgctccagaacgcattaccggaatctcatcttttgcatcccattgttcaacgtctcgtgagtcccagctttgaatatagttacggtttaaggtaacaccatagacgccagtgcctttggcagccggcgcaattatattattggctttagttactgcaatcccaaatggtgtagctaccgttgcgtgatcggtattaacaacatatggttgattactggcaatcgttccagcacctaatgggccagagacatagccagttccttgaggaataaagttagccattatttgtcacctccaaagtttttttcgtataaatgtaaattatttttggctttggatgcactatctttatggaattcgccagcagcgttatcaaaaccagtattttttgcgacatcttgcatagcatcaaaataagtattgatgtaaatatcatccttatctttctcatcgaagctgtcgttcaacttcttgatcgcatccaccttaatctgtttatcatctttgctctcaaactcgtatgagtcgcctagaaccttcttagctttcttttcgagtgctaaacgattctttacggcttcttgaatactgtcggcagcatcttgcttggctttctcagccttatctttttcagcatccttttcagccttagctttagtagcatcactttcagccttctctttatcgtctttagcagacttaagcttcttttcagtttcttcagcggtttctttgctctgcttggcttgctctttagcatcagtaatctgttgcttataagccttaatttgagcttgaattttgtccgcttcatctgattcaagttcaacagtatcgcctgaatccagcattaacttggtcatttgattccctccattcgatttatgtttatctagaaccatttcggcagaatcaccaaacaaattaacatcatgtccggctctgccatggtcaacaatcgcaatatggttaattttgatgttcttttgtgcggcatcatatcgagttccttggtattcgcctgggttttcatcaacgttggctataaaaccaatggatagctcatgtttaccatctcgaatctgatcaagtgttttctgatcagccaccgtcatcgatactttcaaatgcctgccatcactctgcgcatcattgtgtgtcatccctacggcatacctcttataatttgatggcttaaccgtttcattaggatgatcgttcgtaattggcttagaattagccgattgaactgtctcaggtgagaaaatgtcatcagggagcttagcttccatcaattcagacccatcagaaaagcgatatgggaacacacctggcttggcaattggacaagcggtgatattcaaaaaaccgtcgtcgtcaatcgtcgaatccatgattgccattcggtcatatctggtaacagttttcaaatctgccaccttctattcgccgagtggaaccatgaagtaacggtctggtgaatagatgatttgcccgacttgaaccttgcgatacttgcgaatgccgttgtaccaacgtaactgttcagatccacgcttgaaatgattggcaacatcggcaattgactcgccttcttgaacttggtaagttgcatcttcataataagtgcagtcgttgggatgattaacccagaaattcttctgctgattagtcaatctcaaattgccatagtgagaggctacttgctgcgcacgtaccgttggatcttcggagtatacctcatcaactggagaaacagctgatgaactagccggtgctgaattagtaggcgcatcacttttagctagagtacctgatgcagagctgcttggataagtggaagcagcgtatgaagcactggaactggttggtgctgaactacttgatgcagaactaactgagctagttgttgcatcactgcttgaactactgtcttgtgccataatagaatctccttttcctaattttgctaggcatcaaaaaagacgtccatttctgaacgcctcatccctagtaatgtgactatgtgggcttgcaccacatcatgtctttgcactagccactattaaattaatccttgtgcttgatattcatgaagttggtcagcaaacactggcaacgcaacgcatcggcattggatcggttcacctggcaccatcccattatcaccgccagcaggatcaccatacctttgtaagctttggtcaagtaattgatgcaagtcacgcacacgggcgtcttccattgactgccagatataataatcggcaccagcttcctgctgacgatgcgcattgatttgaccgagaatgctgccagtctgatcacgagcaattagatgagcgtgcgcactggttgcattgtcaattttggcaatttccttagcaatttcgcccgttccttgacctttggtaacgccattaaaaacggttgattcgacttgttgggcatattgatcatgtaaggtcgtaatgcgactaacattctccgcaatcttgctttgggtatactgccttaaaaacctgtctgatgatattgggtcgatgggctgcggtcccatttgaactttcagcccgttataactccacttatcaacatctttaataaactcgctaacccaggcttctaaagtaatgtcattgagtccggactctaattggttctctaagtactgcatggctgccctgagctggtcagccacactgtcgttagcgtcgtcgtcttgataaatggctgattgtttgtaaatcgggacaatcgtgtatcgccacaattggtcggctcgttgaaaccaatgcttcaacaagctgtccatgtacttgtgatagcgtgtctctaatccaaagcagaaccgtgttggcacaatgtgcggtaacaattccttgggtactttgatcaactttgccatgccgtcacctacttaaatagcctcttaaaccagttttgatgcttagcagtttcaccgttgtactttttaaccagctcattcttctcactatcagttagctgttcaaagggcttaatatcatcttcagaatcgcccgtaaacgcattctgggcattattcttatcggtatccaggaacgcgtcatgagcttcctctggactcaaagcaccacattgaactagggccgataatccttgcgcttttgccagggatgtttgtgcattcgtctgtgaatcttgttcccaaagtggattgaagttaagctcccaattgatactatctggatcaacattgccaacgttcttagctctcaacaatagtcgaattaaacgttccagaaatggtcgtagaacattctcttgttgtgacttaatgtaagaatagtagttctgcacatcggtttgcgtaccggataccttgccggactgttgacctaacaaaacggttttaggaatgttagtggctgccgataagttgtcccacatgaagctaattaatgaatcaacaccggttaattgtgtgccaaccttagcaacctcatcattctgaccaattaacgccagtgattcagtcgtaaattgataattcatcatgccggatagtttcgctaattgtttgggatctgcactggcagtatcaatactattagatgaataggttttaaacgaaagatcgttcatgatttgccccaccgaccagttagcaatgtcaactagctttagagcatcaaagattgtttcgtaaattgaatgtccctgatcatcgccctcatcacgcccgtattccgcatgcatatatcgtgaagcgtcaatggtcttcatcagaccattctcggtctgtgtgttgttttcaagatcataggctgaattgcctactgaaacttgaatattggcttctttgccatacgttagactaaacggccataggttagtaatgatgttacccacaatccgtctatcgaacggttgaatgtacagaatatctaataaggcgtcaggatccagtggtttagatgaatcatcatctttttggttctcaatgccaccgatcgcaataaacgaatcgccccacttgaggcgatcacttagaaattgggcaaaaacattctggctatttaaatctttgagtttttggttaatcaaatcgtccaggtcttcattgtcagacgtgaactcccagccatttcgcgtcatatcggttgctggcattgtaatcaccatatgagcgacgtggttatcatggtcaagttgctgtatttggttatcatctaactggcgataattgccgtgtggcacaagattgctgtaactcttagccgaagcactatgatcatcggccatactgtcaacgatttttactttttcatccagcgaatccttaggtgcttgcttccgtttgatgcgtttgtttgtcacactgtgtcacctcacattccatatcgtgcaaataggttattagacttttccatgtaggttagtccttgcgtcgtactatcaacttcatcgtcgtgggctgcggttgggaagctcgttagctcagtaatataatcgtcaatctcaggtcgccaagccggatgagggatgtagatattaccagcctcgaactgtgcagtaacggcatatgctcgcacttccttgccaccttgcggttcaaccggaataatgccaccaatctcatgctgaagcgtgttaatgatggctggcccgttggctttgtcttcaataaacttccgtgaagctttcgggtacatcttggttactcgtcgaatagcattcagcgtttgcgtaaagtccatacgagcatgttcacgatgtagtagataacgatcagcaccccgggcaccccatacttgaccagctacataatcatcattttctttacttttaaacgtggcatcccaagactgaatttgagtatctaaaaagcgtggcaaaatcgccacgctatcgtctaatcctaattggtgtttaatttgttcgttaggcacgtagtaacgaagccaatccggtttgaatacgccaccaccttcagggatgggattttgttgatataatgccgcccatgttcgagcaccaacactcttctttgtttgttcagcccaggctttgtcatagcttaacggcttctgtggtgcgagcgtgtcgccaatttcacgacctaataaatcatccgattcagtacatactgctggcaattttaactcaatccacggtcgtgctttctgcttaagcaaacggccaattagatcatcgtcgctccacctagtcataatgacaatgcaagaagaatctgcatgtagacgagttgaaaaggttgattgccattcttcccatatcttgtcacggattgtcttggacattgcttcttgggcgttcttaatcggatcatcaatgattaacagatcagcaccacgaccagttgcaccagatagaattgaagttgagtacatcccaccggaatgccctttaattccccagtctgaaacggaacttgtctgttgtgaaagctgtaggctaaacatttgcggggcgtaaaccatgaatttatcacgattcttacggccaaacttagtatataaatcttccgaataggccgccatcataacttccttatcaggattcttcatcaagtagtagctcggaaatgtttcagtaatgctggctgacttgccgtgacgtggtggcatctccacacacaggaacagtttttcaccgttaataatccgttgcaaatatgaacagatcaacttaacgtgcggatagagcttatagcggttctcatgtgacaaggtaaagtagtactcgtacttacgacgggcaagtgctaactcaatgccatactcggccgattgtctcggatcatttaggttccaagccatcgttatcgccctctaacttctctaagtgcttaattaattcatccgtgcctaagttatcgaacgaggaatcaacacgacctgaaagctcaatttcacgcttgtcgcgccacttcttaggctgccgattgttgagccacatcttaattgctgcaatgtttggcgactcgtgctgcacaacattcttcaatcgcttaccgctagcactcaccttgtcttcgtaatagtcgaatccggtagcaagctgataaagggcagcttcaaccgtccgatctgccatctccttgtttgccatgactgcctccgataaatcttgattttcgtgcatccacttatagaaggtcgatggtgcgatgcctatttttttcgcaatttcttcactggtcatcccgtcacgagccatagacgaaataatcgaaatgccatcaccagatagccagtattttcgatgtgattttccagtattagccatttgtgatttcacctcttgttttgaacaaaattaggtattatcgtttattttcaaactacaaaaaaggacccacaatgtgagttccaaaactattttataaaattatctgagccatatgggatagggatgtctccccaaacctcttttagcatgataaagatcaggtaatcataattactaccaatcaatggcacatttgagaaattatcatatgctttggtcataatttccgcatgattgcgaattgcttggtcaatatccccatcttttaactcttgctgaatggcggaattagtaaccttatcgctcataatcatcttagatacttcaggctttagttttgatagttcgtcaacaatcttattaaaatctgcattctcccgattagtcattatttctctccttcgtgatacaattaaattacaggtatttagtaccggttgtgcatatagcatgatctagtaaatagataggctttaaggcctgaggctcttagctagaaattagttaagagtctcttttgttttggccttttagttccaaaattcatcctcaatatgagcaacaccgtgcattgacgggatactaaacaaacgaatttccgagccgtcaaacatcttaataacagtgatgtttttttcatgcttcttgattgatttaatatacccacgatcaagattcttaattgtcacgtacttgcgcttaatgtcctggtctgtgataatccgtcctaattccgaaccgttcgtgccagaagcaatatttaagtcttcaactaaatagcgttgatgattattgagatgaatctgcaaagtgtttggttgatagtcgttgttgccatcaatcaaagggtcatagaacgtctcaccatcattatttatgtcctgcaaatataaaccattgttaaactcgtaaactttagaatcgccccaatgagtatcatgagcgtaactgacaatgttttgaaaatgccgtggtagcttaacccgtgcatccccatggttgattacttctaacaatccatttgcttcggtcttcgtaacagaattaacgtatgtcatttaaactttttctccttcagtttaagctcgttcaatttccgtgcctgtaaggcttttcgttttcgatctttgatttttgatttcttatggctctttgtatgtttattgtgtttactcaattttgcctccaaattcctttactagttcttttgctaattttgcttgctcccgttcaagagccttactaatttttacccttatcgtatttccagatgcatcggtacatatgtcaaaagactttttctgtttttgtctgcgtgctttcatgcgcttaaatgcagcaacatttgtcattttaatcacctcagtctgtaaacttaactcttggattgccaaataatttaattggtgctagaggcacattagaaccgaacttaattggaagccgtttaatattgtctacaatcattttgacagtgatagtgtgatcagcatctaaatagattgctttaattttgtgcggatgaaaatcctttaaattatcagatagaatattaaagtttaacaagataccatcctcttgaacctcaaacagttcatcaggaccaaaacctactagctttttatcatctgctaaaattttcaagttcattgcgttccaaacattaaaattatttgccatgactttttttctcctttttgtgcaaattaaaagcgccctctttgcgaagacgcttctttaagtctttgtccagttgcttgtctatcttaatttcttccttggaagtatagccatagctggtttgcttcatgggcgtatatggatgcttacgatcattcatataatcacctctgcaggaaatacagaattatcaaagcgagtagcaacaagcaacccaccaatatatctgttagctttaatttcataatgtcactcctatgtatttaaatgggcgaggccggtgccagtcccattcgtagccacttttttcactgcttatgaggcagaaacgacttatcccgaagttacatcgcctagctaactttaccagctatttcattgcaaaataaaagcctacgttttccgccgcaggcatcatgtaactcactacagttcaagttctagacaacataacatacaagtttttgtttttgcgtgagctgcatgttcgttgactggacgggtactactcattaatttttaggaagaaattactttgatacaagtccaatcaacaacgtggctggcagggaatcgaaccctgcacggttagctatccgccctcttcgtacgtatacgttacagtcacacatctaaggaaagaaagtgaaactcttttaacaaattccacaataccaatataacccctgtttttgcattttttcggcagaacatcggcagattgtcggcagaaagtcggcagattatcggcgaactttttttgctcgcagtgtatcacgaggacaaactatcgcaaaaacccataaggcttgtttctggtaatcgttatatgtacgctcagccagataacctaaatcatacttctccgctaagcgttcacagcactttttgaccgtgtagtgattaatgaaccggtattccaacaagtcggctaagaaggcgttttgatcatcaatggagctcatgagttgaatagtcttcaaacgtagttcacattccatcttagcggtggcttgtttaatcattttatcttcctgccgggtatgtcttggatctgactgtgcctttggcataccgtccatcatcggcgactgcagggagaaactgaatctagccgcttcaagttgccaatcccgatactcatataaaaattttttagcattttttattgtttgttttctatccaataagccaaagacactatccatctccgcaactcctttattgtcatcttagttgatgttatactgaaattgcctatcaattagcatcaccttggcttccggaaacgggagcttttttatttttcctccaaatcctgaaatgccttaacaacgtaatcagtaaactctttgcgattagcagcgatgtttctggccaatcttgtaggtcgactaagctcattaccgtcaccaaaagaatcaatattatctaaaatgtccacggcaatatcatttgcatcgttgtaaccatccatgtaatctggtaataaaacatcatttacataatctttagtttcttgcaataacattgagattcccctttcatttcccatgcacaaatggcttatcaatatgttcaagttcccataaagccgcttttaaccctactgaatactgcccgttaccgttatcatcatcatgtaacataaacaatatgcgtctgcgtaattcctgcatatcatcctcattcgccgccaatttcatcactctacctccaaatttactgaagttattgaaagctttttcaatccatgaatgagattctgatccagaatcaaaagctcactttcatcacgccgcaagaaaagcgcggttatatcatgcttcttaatatggccagtgaaaataaacttcgatttatgccgctttgcaaatccaatgactgttgctagatctgtggtgtatgagattccatcagtttcgttagacgctggcgctcgataaaccgtcaacttatttggtaagctttttagctcttttaactcgtctggtttcatcaaactaatctctttatccggtcgattgcttgaaaataatttgcgccaaaagtttagatcggcattcacatctcctgcccagacccataaagttgatagcaggaaccagtaaccatagttggttaattcatcacaatgcttggtgaaatagtgaatagcttcagggttcagttgatcttcatacatcagtaagtgctctgagattttggcatcccgttcattgaacttaaatgctgttgaaatatttttagccatctagtccaccttccacaatctcgaagtgcgagtcatccttatcaagctctggcaactacttggaatgtgcatcctgaatcttctggtattcatcactcatttgtctgcctccaaatgatagacatggtcattaatgaaccacttatccttttgagcatcgtagtagacactaggatatttcttttttaaaatacgcctggccttacgatacgaatatccattatcatcaaccagttcccagaatttttgatcgtagttcaaaattaattcttcatcactcattcatctgcctccagcaattccggattttcgtgaatgttgccaactacaatatcttgtgcagggcttattccaccataattatgttctttgttttggattatagaattaaatccagccccgtatctgtcagctttatatatgacaactccaaattctctttttactttggcttttttgttagcaccaaaaaatttaataatgtcgccttcgtagatttccttaccatttttatctttcaggccggtatattgctcaacgatatacttatctggtgacatcgcagcaaacgtcaaaataccactagcttttccatgtaccatttcttgcattggccctttaggcccaaacggcatataccacgctctaaatttaatttctctgctcatttgtctgcctccataattagttttgataatctactagatgtttttttagactcaatatggtttaacgggcttcttacccactcgttaactttaaaatactttttgacctgctcactgtgtggcatcacattcaaagaagaaaatcccaaaaaatcgtcattttcattttggcaaaagaatacttgtttaacacctcggctaagcgaatcaccataaactacggttgcattcatccctctgatcaaaatgttgaaaatcaaaaaaggaattgcagaatctcccaattcttccacttggtaaaaatatttagacggcaagtaatcgaaaggagttgttttcatcctatcactgttccatctattgattagaatccctccggttccagcagccggttcaaaataggtggatccgttatcagctagtctaaccatcaactttgaaactgataatggcgtgaaatcctgtttcttctttcccctgtcgctttgaacttcttgaaaataatcccgaaaccagtcatcggaaacattgtgactaatgttaagaaacttcataaacaatttttctcttttggacttgtcccataatattttcattaaagcatccggagcttgatatgattcatcaaccccaattagctcatttaccttatcaatgctaaaactgttcacttgtcttcctccatattcataaacttatcgaatttatatgaacaatcctcacacaacgatagatgctgcctaaccattcccccagaaccctctgatgaactgttttctgtagcgtagcttaggtcgctaataaagaaaccagcatcaggagtgtattgcttgccacacctatcacatacgtatttttgaattgtcaccgttttaacactcatttatctatctcctgaattttccataaatatattgcttgtcgttgcttcaatgcatcccttagcatccattttcgaattggcttgccggttgcctgacgtagaaagttggctgcatagtcaagtttgctgaagcgatgatactgttcgttatgggtcaggataaacatcacttagcaccgactttcttgtgccctaaagcattttgcgctaatttcgccatgatttggttgcgctggtcaatcgttaaacgctgaaacgcttgtcgttgatactcatagcggtagtcattgccgtgattgatcatccaagtaatggttgctgtaaaatcaaaatgatgattttctaaagccccctgcagccatgtcataatcatgtgcctgtctcgagtcttgttaaattgcatttccattgcggacactccttacttaatcgtttcttcaaacagccctgttcgatggtcgtacacggctaataccaccggcacatgcacccgatacataaacatcttcatgcgtagccgtgacgcttcagtgagagttgcgtcgccgcccttaatgtccaccacactaatcaattcaccgtcttcatagatcgagaaatcaggcttgtatgtgcaggcagattctcgcttgtgcggattatccaagtaaaaggctggttgaatctcaaatttttcatggatcttgaagtgtagtttcaagttctttaagtgcaggtagtacgcaccctcggccttgctatcgaacttgtggccatcaataatcattttgtgggcgttgaacttattgccctttcttggcaatttaattgccgacccaggtggctcttggacacctgtgggatagtttgtcatttgctcaccttcagaccaattcagtttgtccttcagaaactccactcagccgcttaagaatttgtaatgtagcagttgaaggcacccagttcgtaataaattcatcagctacgtcaaagtctttcttgcgtaactgggtccgggttttaatgccagtaacttcgttaattccacgattaatgtctttataaagcattgctcgttgcttctggttaagcacgagatgatgaatgccaatatagctattaactgctcgcttaacccgggtactgatgtaactgtattcaccgggtgcgattggctggtcgtcttccagcttggtaacccgagtatcaatctgcttaacttgtcgattaacctggtcgctgttttcaagtaacaggtgaatcttctcatcaggggtttgcggtaaactgaattgctgctggtaagatttctgaacttgaataaagtactgacgtgcttgtttacccttatcagttctttgaatcatggcaatctctttcgccatgtccaacgttaaggcgtggtcagtaatcttacgtacgttaccaaacgcgctctcgtcattcacatttttgttaatcacggcgaaatcaacgttttcagcgaatccatattcgatcatgcgatccatccattgggtgtaaggggtctttaatcccagaaagtcgtgaagatcacgaccactgacagcttgtccatctgcatagttcaaaattttaattaactgatccatttctgccatctcctatttctccaaaagttctgggtgttttaaatttgtgtagcgaatcagggcaacatcttcaggactcatccgatcttgaataatcttgagtgggaagtcataaaggtgtttagatgctcccttagcaggtcggctgtgtgtcttttgtaggctcggatgactagcttgcaagtgacgaaatacatcacttttttgctcaccaaatgcaatcaccttgccggttcctaattcaagtgctttgtacgtcatcttgcttatcctctttcactttctgcatttcaattgcgtggtcatagtccagatagtcctcagcagtgagttctggattccaaatgatgtctttaactaagccctcagcgtactggctgagcatcgccatcatggcaaaccttcgaaaaatcccgtggcaggtgtcatcggttgacctaccgccgttgcgaaccgcctcacgcatctgttcctggtagcgttccagcagccaatccggatggggctgttgtttagccagctccatcatcgctttggcccaatcgacttcgatcatgctttcatcccctctaaccggtggtctggcattccttcaaacaacatcacatggttctgggtgtgggctgacatccggctgataacccgactgccataaatcttcttgagttctttgccagaccgattggtggtcacaatcgtgttcttgttggctctgccctggaagattcgagtggccacgtccatgttgtactggctggactggtaactgcccacgtcatctccggcttcagatcccaagtcatcaatcaccacgacatcagccttttgaatctcatcagcgacaaactgcgagtactgcttaaaagcagcatcatcgtggaatccttgcttcgtcttggttaagagttcgcggaagtccacgaacatcacgtgctgcttgaaccatgagcgctctaagacttcccacaagcaggctatagccagatgactcttaccagttccagttggaccagtgaagattgcgtggacggtttcaccggtcatcatgtcatcaaccacccgcttggctaccgctttggcttctttttgctctttggttcgggtgataaagttactgaattttttgttgtagacatctggatcagtaatcacactggaatgccgcatataacccaaggcatccgctttattagcctttaactgccagctagttgattcagattcattggttggggcgtccttgcgtgcttctttgtgaccacaagccatacaagccggcatactccgatccttacccgtttccggattcacaaatacatacatcggctccccacaaattgggcaatcatcacactgacgcatcttccccaaccgagtgaagatactgccaactgcttcttgcattgtcgatttttcaggcattttgacacctcgattgctatataattaatcccaaaggagggattatagttatggaacttaggaaaacacttgattcattggttcaaagggacgatttcaaacactacgacattacggtccatttagaaaacggtcaggtaattagtgttggtgattttttcgatccaaatatcaaagtaaaacgaagcctcgacttttttaagaaacatcctgagtacaaacttgataagtcaagctatattgtcatcaacagttatgaaacttattacgttttgtcggacgctgttgttgcttatttcacaattcgctacaaccctgatgtattacctttctaggtcaaaggtaagttcttgatgtgacgttcaatttccttttccatttttgtaaagatggtgagagttcgtgtatagctcacaccctctttttttagaatctgataaattttgcccgcaatttctgcgtttttttctgcttcttctttgttcatggttttgcctcctaaaacggaatatcatcatccgaaaaactactgttaggcgccactgaaatcggtggctttctttgacttcctcgtgtctttcgattttcccaattaacttgatcggctttgatgtcatcaagggttttgatattctccttttgccaccgtcgcataacggttcgagctgttggaaactgtcgatgactttcagcagcaatcgttaaagcggcaatcacccattcagggctatggtcttcaagccaatcatcaagttcttgtatgacaacaggggctggctgtcccaaattttgctggtaaaaagctaagactttttcgcgaggagaaggaactggttcttctgtagtcttctttggtttacttttatttactttactttcctttactttactttccttgctatcagaggccattagcaccccattagggtggctattatttttggatggggtggctatagggtggctatcttgttgccatcttttcttggccccccgcttgcctgcttcagctagcttcttagctttggaatctttgagcgccattcttttgttgaatccgtcggagtagaagtacttaccatcatcggtaaagacaaataacccaaaatcttcaacaaccgcttttataattgaagcatctacacgaaggtcaaaggctatcacgttataatctttgatactcatgtagtttgcttcgtcacggagacgttccaggatcataaagtaaacgccatatccctcagcaccgtatttcatccgaactttgatcattttttctgaattccgtgcgttactgtcatgggaaaaatagttgttcaagttcccacctcctagtagaacggaatctggtcaatatcaatcacgtcatttaatactttgtaggaacggcagtagtcacagtgaccacaaggaactggtttctcgcgaccttcttttacagcttggatatggggctggtcacttttgatttgctccatccggtaatccatcaagtagtctggaatgctgaagattcccttatcgggtaccttttgcttggacaccgcaatgatgagtggcgtgcactcaacgccaaaggtctgtttgattaattccttgtaaacggccatctgcatatcatagcctcgggcctccgcaaaggagacaggcgcacgttggttgggtgcccagtgcttcttgtggaagtcatcaaccgtcttgaggtcgtagaacatgtgatgttccaagtccaggcaatcaatcttgccccgccacttaacaccaaagatagtgccagtgacaatcacttctttgtcaccgtggtaaatctgcttgaaagtcggatctgaatccaaagctttaatcatcttgtcagcatcgagaaattgtttcttgataccgcgctccggcttaccgtacttgcagagttcatcagcatgctcttcaatgaacttctgatgagcttctgggctctcaaagtaggagtggaggtaattgccgaccaataatggggtatcgtcctgctgaggctcccagtcgccttttagctcggccaatgcttcagcttcacactgacaaaatttccagaaccatgacttggactgagtcaaccaatcctggtcattggagtagtaattactttgactcagcttcttgggcttgcgtgtcgttgaggttttcgaagaggctttcttggttggcatcttctttggtttcgttgtcgtggtcatctttacctgcatcccccttctgctcatgcttctttaaaaattcatccaccggatcgtcttcttgaacatcaatcacatcatcctttcgagtgggtttatttggttcaactggcttaacaaaatcggtaatggatttcttggctgatccctctggtgtgacgtccttgcgctcatcgtcatattcgtctgaagttgtgtcgttaatcgctttaacaaataaatcattgtcagagcttgagttgatgtagtacttggctgcacggttgatgactgttcgttgagccatttcctgactgaacttgttttgaactgtgtggttcttggactgagcccatgaggcatcaatttccttcttagtcatgacagtccaaactttgtgaccatcttgttcgcgaatgtatgcgaaagcaccaataattggattgtcccgattttcaaactttggttggtacttagtcacaattaagttcatgtcctcatcagacccggtttcaaatccatcaccctcaaacactacttgggatttgatatcagccacatttgataggttcttaagcacggtaatcgatccaaagtacgaacgttgtaggacacattgcttaccataaggaatgaagtagcattggtttttggctggtgataatccttgaatggccatattcagtaatgctttggccactgagttagaatcacatttactcaggattgatggcccgtgagagtcatcggataaaattaaccaagcactgtttagcgcattccccactgagtaattaggtggcagtttcagcccttcattattttgcattttgtttatttgagactgcacattttgtactaattcattagccatgatttattcctcctcatattttgaataaaacccatctagtggccattcccaggactctagtgttgtgtacggttctaattcttgcagctctttaacagcttcgtcataagccacgttattaccggcatcttcaaagctaactgctaagtacctgttgattgactcagtttcatcgggaatgaacaaatcgtgcgagtaaagcatcgggattcgccaatactccagatcatcatccaattgttccccatccgtgtctttgaattgctctttccattcagccaattcatattcataggcgtacttcttagcccccatatccatcatgagaaccacctaccaatcttcttgacagcccgttgcagaaaattcaatttacgagtagaataaatttgaagaaaaaattgatatgtgccaaactttgaagtgcttagcaatccgacttgctgagcgctttttgttttgtcatttttcatcagtctcagctccaatctttaaaagttgagctttggctttatcaaaagtttcgaacgcatgcacgagatagtcatagtgactgtccttagcaaacttacgattatcaatgcggccaacctctttagccatcaaggttccggccacatggttaatgaaatctcgctgaacattaattcgttctgatattggtgccatcgtcttttccataatgcttatctcctttaatcgaaccattctttccagaaagcctttggatctttatgccactgatcgtactgaccttttagccagaaccccaaagcgcctgccaacaaaatttggatccaaaccggaattgtaagaatcaatttctatatttcccctgcaaatacttgatgtttcttgaaatacttgatgcactctgcccgattgtacttggtgcgactaccttgtggcagatgtgggcaatctgagtaatatttgtcaaaagtctcggtattgcatttaaaaacttcgcgtgcaacttgttcctttgtcagcgtttcattctgataccgttcatctaacttctttgcaacctcgtcggtaataactggaactaattgtttgataactgcttcaacgacattttttgaatccacattgtcaagattgaccgtaactttcataggcgacacctccttgtggccgattgatgatccattgttgaatcagattgtgaatcgaaacttgcatgctggtttgactgtccgtttcttcactgagctgctgtaaataaaactgaacatcatggatatcttgctttgtgacttctgaagctggtttgttaaaaattaacatcaccttgtcatcaagtgctttgcgttcagcttcttccttacttgtctcaataaaacgagtttgcggaatgtcaacactgatctgatcaggtgaaagtaatcttaatccgcaaagatattcagctacttgatatctgaataaatcatcatccagataattcatcacgcctaacaaccgattcagcggaatatcacgatcaccagtcaaccagtttgtaatgtttgattttgataaatgcatctcggcggcaacctggctctgtgaataccctgacctcgtgatgacatctctcaggtccttccttatatcaatgctcataaatatcgcccccttaaatttgtgtaattttagtaatgccgttcatcccctaaaaaggtacattaaaagtagcagaggattaataacactagccattaactcaatagcgttagccgttccacttgcggataaacatctttggaagccagagaatcatatatgttgaataattctgtaagcctaaaacttctttgacgacttcaattttttcagtgtgtgtcatttgatcacctctttattgtcacgattcgtgatttcatcatcaaaaaaaagggtccctacatcaacgccataaaactttgcgactttcattttagttttgtcgcttccagatctttccccagattcaagcatagcaagcatagattgagaaattcccatttctttggcagctttgctttgagaaagtcctaattttaagcgttcatttataagtttcatcagatcacttccttatcaccttatgtgattatattacatcacatttcgcgataagtcaatcactttttgtgattaatttcgaaaaagcttttatatcacatattgtgatagtataatcacattgaaaggtgcgtgttaactaatgacattaggtcaaacaatttcctctttgagagaacgtcgcggcctctcacaagttcaactagccaaaaagttgaacatagggacaagcactttaggaatgtgggaaactgacaaaagaaaacccaacccagatgctcttgtttcattagcaaactattttgatgtatcaaccgattacctgcttggaaataccgcttctgaaaagggatcagctccagaatgggcaactgagcaagacagaaaagatcttcggaaattccttgaagataatgctaattctatgacgtatgggggcgaagaattaactgatgatgaaagacaacaattacgagtggctatggaaaccattttctggaaacgtcacaaacatgactaattacgcaaaatcagcaattaaagaaattgtggcccgatatggaaccgcggatccatttataattgccgaaaaattaaatgtcgattattattttatgccattaggcaaacatcccctcggagatacaagctatgacaatcatgaaccgattattatattgaatgaatcaattcatgattcaccgcagaaatattttacattagcccatgaaattggacatgtggtgatgcatgctaaccttgcgggatatcattcagggtatgcaagctacggcgtatgtgaacatcaagccaatgaatttgctactggtctaatgggactactttatgtagaagaaaataggtatgggccggaaagctattatgatctagtgcatcactatggatcaccggtcaatgaattggattaaacaaactgggggaaacattatgaatagcaagtcatttttagtgggtattatcactattgtctcgacttctggaattattgcattaaatcctacgtcggccaatgctcgcacgtataccaccgttccaacgtctctgcgtggacactggtatcatttaaattcaaacaatcgtacgtatacaaaagtgtttgcatctaagtatgtatttaatgccaatggactaaaactctatggaaataaattcccttggtatggctatggacatagtcaattgtttgtatacaaaaactcaaagggatattacaacattggtcagtatgctagtgatgagtggccgtattggaaacgtgttaggcataatggaacttacgctttaaaggaatatatgccattaccgccttacgactatcaagtaaaatatttttatcactactcgcatttcaccgcaacgaagtatcgaaccgtcaaaagcaacggtttctattttaacaaatacattcctgggtttctccaagctggatctactgccaacgtttatacaacaccagaagatgcagcggctaaaacaggcagatcttaccacgtaacaaatattttcaaaaaaatgtcaattaaatggaacgatggcaaccacgatgacatattaaaaataaactatgatggcaatacgttctattacaacgatacggatggtgcatttcagccatataatacttttcgtgatggtactggcatcacatcaccctataatccaaagtcaaaatctaagatctatctcaaacatggaaaccatatttataatggtacacggtgggacaaatcaactacttataaagatggaactttgatctctaattcttacaaattaaaaaatgatcactgggtaaaagtgtattaattgttgggggaagatcatgaaaatacaaaagagcattttattgggaatcatagcattatcacttggtactgtcggcataatcagtcagcccactacaagccaagcaatgagtatttataatcctgataatccattttggctgcactcgcactggataactacgacgaagcggatcgtagttcataaaattaagtatatggagccagaatataagagttaccaagttgcgagctatgttgtaccaagaggataccattacaagatttatgcttcggctacgaactatcactggttctttgattccggaaaatttaaatcaaacgcacactatatgtatgtttcaaacagacacagtcacgactggtttagatttgggatccactaaataactagtccaaatactgatgactataaaagctgaaaattgaagggagaatttttatgaaggattttgtagaaatagcacagatcataacgggttttgcagcaattgtttctattttttttacagtatacgcctttagaagccaaaaaatagataaacagttagatacggcaaaaaacatatctagttggaatgtcacaatggctaaagataagcaagaatctctgtcaaaggaagccaaccctggatttgatggtgaaaccttcaccgatgaatggcataatgcaccaaattgtaccaatattacggttaataaaaatcctttccctgtatataatttgataattgtttttgttcccaatcatttaaaattcaaggggaataattccctatctagccaataccaatgcttttactatgaaatattgactccgggaaagataataacagattttgttaatgaccatacaatgggaaatggacatttaattccagaattgtattttacagatactcagaacaaccaatggcgtcgcagcaagaatggagaattaaaaaagactgcctatttgaagaaggcagtcaagttaggaattattcaaaagcatttgtaaaacagccaaaaaagttaatatgcaaaccagtgacaacgaacttgaaattaacaaaataaatgtttttccaattgctgtttcatctttaccccaatcaaaggaaattttaattatgaaaaaatcaattaagataattgatacttgaaaaataatcagaaaagtgtatgatatttgattcataagcgatcctccttctgatgtaaatcatacatattataacacatttcaccttccccaccggtgccagcgataggtccgactcctaccggggaattagtccaaatgctgatgactataaaaatatgagttggagggaattatgaaattaaagaaaagtattctagttgggatcacggcattaacctttggtatgggattcagtgcaattaacatttcaactcaaacaactgtccaagcaagtgcccatcgagcgcaggtcgttcgcggaattcgtgtgtaccactggatttggggaaattcgtttgctacaagtcgacttggtaaaagcatctatctacacccaggaaagatcattcacattgctcccttctatcacatgggtaaagatggctacatgctacacgttaatggtcatggctcgaagctttactatgctcgcacaaatagtagtagctggtttagatactaagataaatgccctcttgggcttttatttagcacgttaaaagaacatatgtacccctatttatgtatttaagactgatttgtacacaaaggaaggaattgagataaatggcaaaagtagcaaaaagcgaaaaatggaagcccatgaagcgtcatcccaacgtctacgaatatcaaacccaacgtggtaaaaagtacgggattcgcttcacgtactacgatgctgaacataaacggcgtgagtacaaaaaaagtggctttcgtgattggcaagaagccgaagttgctttacacaaatttcaaaacgatattgataatggcttcgttaacgctttgaataaccggcgaacaacagtcgaagcgtactatgaagtaattcgtaaacgatcagttgatatcggtaagtggcgtccggcaacaattgcgcaaaaagatatgtatttcgcaaagcatctcaaacctgtatttggaaatatggcgttaaccgatattagtcggcaacagtatcagcattttattgatagcaaagttaaagatggctacgctaagacgaccatcagtacaataaattctgttatgcaaatcattatgaatgctgctgaacgtaatgatgtgatttctaaaaacaaattaaaagacatctcaattgaaggtgctaaggagcctaagccggccaagctggaaccacaagattatcaattattcatgaagacagcaagggaatatttgagcaaatattggtataccctcatctgcttattagcgctgggagcgcgtcgtgaggaaatttctgggctacggtataagtcccttaagttttttaagcaaggtggccaggaagcctgtgagatcacgtacgatatggcacgcactcgttaccaggaaggtggtggaaaattaaagaatcacgccagctatcgcaaaaattatgttacgggagaacttgttgagctgttgaaattttcgcttcaatactcaaaaaacatatgtactcaatgtggcagacaatacaacaacgactcatttctattcgtaatggaagattatggtgaacccatacatccagaataccctaacaaaatttttaaaaaggtagaacgtgcctgtggtgtccacgtttaccctcatcttctacgtcattattttgccacaatggctagatctaacaatttttcacccactgatattatgcattggctcggccattcatcattaactatgacggattcgtatactcgcccgactaaacagggagctttaaaactaattaatgaaatgaacggcaccctctttaagcctaataacggtaattgattcaaaagtgtggcagaaaactgtggcacttttctaatttgccacaaaagttgccacataatcttcaacttgtttggatttaaatcaatcaaagtaaagcaaaaaatcgccctgtatcagcattgaataccgatacagggcgatttgatttgaactaattataactagcttacttaagggtaacagttccaccaacggcttcaagttgttccttgatcttgttggcttcgtcttctgaagcgccttccttgatgattgatggaaccttatcaacaagtcctttagcgtctttcaaaccaagaccggtgatgtcacggatagccttgatggctttaaccttttggtcacctgattcagttaattcaacatcgtatgaatctttggtagcactgtcgccaccagcagcacctgcagcagcaactggtgcagcagcagaaacgccgaattcgtcttcaattgacttaaccaagtcgttaaggtcagagattgaagcatcttttaattggtcaataatattatctttatcaaaagccattttattttcctccattaattggaatttatttagttctgattaggcagcgtcgccatcgtcagattgtttcttatcagcaattgctttaaccccatatgcaaagttacgtacaggtgcttgaagaatgttagcaagagtagataacaattcttcacggctaggcaatgcagcataagcagtaatttcttcaagactggcaacttcaccatcgataacgccacccttaagcttaagtttgtcgttagtctttgcaaagttgtggacaatcttaggtccggcaacaggatcttctgacgagaagacaacagcagttgggccgttgaaagttggtttcaaatcatcaaaaccggcttcagcagcagcacggtccattaccttgttcttgataacttccatcttaacgccttcatcacgtaattgctgacgtaaatcagttacctcggcaacagttaaaccacggtagttaatgataacgacagatgaagcattcttcaattcttcagtaacagatgcaaccttttttgctttaatcgcaacagtttgttcactcacgaatttcacctcccaaaaatttgttgggacttaataaaaaatccctatgcccacccagacataggaaaaaagtaaacttactttcctcggcaggatattaaggcatagaagccacctgagtcttaggcgaatatatcagcaactaacagtctatcacacaaagtaataacccgtcaattagggattttttatttaaatcgaaactaattaagcttcaacgcttgagaatgagtcaaggtcaactttgacgccagggccaaatgtagttgagattgaaacgttgttaacgtaaacaccacgtacagaagctggacgtgccttcacaataacatcctcaattgtcttcaggttaccaacaagcttgtcggtatcaaatgaagctttaccaactggaacggcaacgttaccgtcacggtcagtccggtaagtaaccttaccagcttttgattctttaaccgctttggcaacatccatggtaacagttccagtcttagggtttggcatcaaacctttaggtccaagaactcgacctaaacgaccaacttgagccatcatatcaggtgttgcaatggcaacatcgaagtcaagccaaccatcttggatcttttgaactaagtcagcgtcaccgacaaaatctgcaccggcatcttgagctaccttagcgttgtcacccttggcgaatacaacaacggtctgttccttaccagttccattaggtaagacaacggcaccacgtaattgttgatcggcctgcttagtatcaacgtttaatttgaacacaatttcgacagttgagtcgaatttagcaaaatcaatatctttaatcaattcaacagcatctttgattgggtatgctttttcagcatcaaccttttcaagggctgccttgtagtttttacctcttttacgagccatgtgtgttttcctccttgcttgtggttataacggattaacctcccacgcgatgtgaaacagtgtgtcatcgttaaagtaacgacgtaaccgggttgactatccttcgacagtaaagcccatgctgcgtgcagtaccttcaaccatgcgcattgctgcttcaacatcagctgcgtttaggtctttcatcttagtttcggcaatttctttaacttggtctttggtaacagttgcaaccttgttagtatttggttcgccggaacccttttgaacaccagcagctttcttgagtaacacagcagcaggtggagtcttggtgatgaagtcgaatgaacgatcttcatacacagtgataactacaggaataatcatccctgcctgatcggcagtacgtgcgttaaattccttagtgaatcccatgatgttgatacctgcttgacctaatgcaggaccaactggaggggcaggtgttgctttgcccgctggaatttgcaacttaacaatattcgctacttttttagccacgagacataacctccttaagtccgtgtgtggtaaatggagatcaaaatttctcctcccacgttggtatgcttaaacataccatactaatataacataaacattttcattcaacaacctaaattattggttccaaagaaacttggcaatttcttggtcgacaatgacattttcatgaagcagccgatgggttgcccgtttgcctcgaatcaccaattcatggtattgcgcggccggatcctgcagtaaatagcgcaatgaaaaagcactgttcaccgagacttctccgtcattttgctgggtgttgctgatccggccggcaatattgagaaccttaatgtcccttggaattgcaaaaacgcgttgtgacagcgcccgataaatcggcattcgtttggttggccccttggcgttcaacggataagcgtcaactttatcggtacttctggcaatctctgaatcattgaatggtccggcgatcgccacaacatgcttcacgctgacaggcgtcattttgctctggtgggtcagaaaccaaaaaatggtaatacagcccatggaatggccaaccagattgatctcttcaacaccatagcgggtattgagcacctccaaaacttcagagagccacactgcctgctgccttgggcgggaagacttgtcggcaaaaagaacttggatcaggacctttgacttcgccagatggcctgaaacatggattttaccgtggcggtcgactttgatgaccatcgatttgttagcaccgtactgtcgagttaatcgattgatgagtctgccaaatgacaatcgattaccaaagtagcccggaataaaaagtgtgggaatggcctcaatcccatttgccggatcggagtcaataccaacctggttgggcgttccaagccgaatcagccggccgacaaccaccatcgcaatcagcaaaacaattatcaaaccagccatccataccatcgtgaccacctacttttggttaaagggttgtatcaatttgattgaagtcaagatctgtactggtctcacggccaaacatttcgatattaaccttaagccgttgcttttcgttatcaacttcggttaccttgccatcaaggccggtgaaggcaccatcaacaattttaaccgtatcgccaatgttgacatccaaatcttcatggcgagaactcatgccaatccgtttgagtaccaaatcaacctcatccggcagcaatggcgttggcttacttccctgtccatgagagccgacgaatccggtcactccgggagtgtttctgacaatgtaccaagcttggtcggtcatgatcatttccaccagcacgtagccggggaaagtcttgtccatcttaactttgtccttaccgttctttacttcatgttcttcttgttcagggacaaccgttctgaagatgtaatcctgcatccccatagattcttttcgactgtccaaattcatcttaactttgttttcgtatccagaataagtatgcaaaacataccattgcttttctgctgactcgaccatgtttttctgctccttcgtaattccagtaaatgagttcaaataaaaaaacctgacacttttcgcaggtttcaacaacttaactatatcaaacattgactcaaaaggctatgccagaaattggagtgcccattgaacgatccagtcaaccaagcctaaaaagatggccatgatgattgaagtcccgataacggtactggtatcagtccgcgtctgagatgcgttgggccaagtgaccactttcatttcctgagcaacttttttgaaaaaattaattaatcgcaaaattttatccccttatatcatgattaacgagtttctttatgcaaagtatacttaccgcaatacttgcaaaacttattgagctccaagcgtttggttcgattggggttggcgggaatcgtataattccgtgaaccgcaaactgaacaagccagagcaacttttctttgtgccatagcggcacctccttacaagcatagtaataatagcattcaaaaacaattccgtcaatttatctcaccgtcaaatttgcgccgacagcgttcaaaagcgttgataattcctctttgcgctttgggatccaaatccgcataaccattttcactgagcatcaggttaaacgcccgcttttccaatggtgaacagctgctgtatagtttgcggagtgcatcatcgacgatcaccgcatcaattggactactagctgagttatcggcgattttggcggcgtaaaaatactcgttggcttcaaatgatgtcaatggttctaccggcacccgtttttgggcattgttggtgcgaatcaggtcaaacaagcgatttcgcagattatgactgaaaaaggttccaaaactgacttttcttgcagattcaaaccggcacgccgagcgaaacagaaccattcgggcttcctggtccaggtcgtctttatcgtagccgttgatataatactggcgtttgtacttgcggacgattggataatattggtgaaataactgcgcaaaggcctcttcatttcgtttagctgtttgacgaatcagttcaagtcgattgttaggtaacatattgttatccccctcaaatgtttttattaatcagattcgattacgaaaaacattaacggaggattcaacttccggcaagacgaaccagcgttcattcagtgaatatcccacctataccaattttaaaatatcagcatactaatatttttattgaccatcatgcatcattttgtcccgcagcttctctaattcaaggagctgtttggcgtcaaatggcgtgtggcgaaacacttggccttgatcagtcatcttgcgcgcttcagtatcaacttcctgtttggcacgctgaacatctctgagcaattctctggctgggatccgcaatgcgccggcagcaaaaatcgtccattgctcggcttgatcgctggtagcaacgatcacctgggtaaatcgattttgcttgcgatgggccaaggcctcaatgtaactatcggcagtctgatccttactggtccagacaatctccatatcaaacttacggaagctttttgaattaccgggaacgtacatcgcgtcaaaaacgacgatcatattgatgtcccggtactttttatattccgacaattcagccagcagttgatcgcgggcatcttctaaacggttggcctgcttgagcttgttgaggtgcggccaattgccgatcatattataggcatcaacaattaacaggtcttctttcattatttctcaccgactttattttgataatgggtggcgggaattaaagccctgataaatcaaaatgctagctgcaacgctggcattcaggctttgaatatctcccaccattggaatggtcaacatttcgtcgacttgtttcttcaacagcggcgaaattcccttaccctcgttgccgataataacggcgattgagcctttggcatcccaacgacggtaatcagttccggaaacatcagtcccaaagacccacattccgcgttgctttaattctttgatggttgccgacaaattggtcacgcgggcaactggaacccgttcaatggctccggctgaagttttggaaaccgtggccgttaatccgactgctcggtgcttaggaatgataatgccagacaccccggcagcatcggcagtccgaataatcgagcctaaattatggggatcttcgatattgtccagaatcacaaagaacggttcaaccgcttgcttcttggcattggtaaatagatcgtcaatcgttgcatacttaaaggctgcaattgataataccaccccttgatgattttggttattggaaagcttgtccagcttttgctttggaacctttgaaatcaccagccgctttttatgcgccaatttcatgatttcagagataatattgtcgtcatctttgattcctgactggataaacagtttgttaaccggattttcactctttaacgccgcaaccacggggtgtctgccaatcacaaactcttcaggctgatcctgactgtcatcgctgcgatgatcttgacttcgattatcattcttcatgtttgaggttcccactttctacttgttcaatacaccaatttgcgatttctttcattcgatccgtctggtcactcagtgataggtagccaaagactgcttcaaacccggttgaaatgcggtaggtaatcacgtcggtattcttggcgtgcgtgtgactgttggcatttcggccgcgtttgaagtagtcccactcagtttcattaagcagaccatctgttttcattaaatcaattaaagctgcctgcgcctttgcggatacatagttggtagcaacatgctgcaggcgcttaggcttggtcaacccctgggcaatcaaatgccgacgaatgaaaacttcatacgcggcatcccccatgtacgccaaggcaatcccgtttaactgggaaaaattatcaatcattaaagttgttattcctttctaaaccgggtcccctgtggggtatcttccagcacaattccccgggctttaagttcttctctgatttcatcactgcgaataaagtctttgtcatggcgagcctgttcccgttcgtggatcagtgaccaaatctcatcatcctttagttcactttgctcaagcttaatgccaaagacaccagataattgacgcagggtgttgataatgaactgcaagctcaatttgaagacagtctcgcgttcactataggtgttggcaaattttgcgagttcataaacggcggcaatcccgttttggacgttaaaatcatcgtccatcgcgtcagtaaagtcagcgacaatctggcggacttcctggtcggttttgggatcatcaccctcgtcagcattatgaagccgatattcgaggttgttgaaggccgtctgcagctttttcaagttgctgctggcttctttgacactggcatcactgtactggattggacggcgataatgggtggtcgacatcaatagccgaatcacttggccatccaaattcttaagcagatcatgaaccgtgatgaagtttcccagtgacttactcattttctcgttatcgtcaccaattgtcacgaaaccgttgtgcatccagtatttaacaaacgtctggcctgtgttggcttcgctttgagcacgttcattctcgtgatgcgggaaaattaaatcttctccgccaccgtgaatatcaatcgtttttcccaagtacttggtggacatgaccgagcattcaatatgccatcccggccttccctttccccaaggagaatcccacgaaatctcatcgcctttggactttttccacaaggcaaaatcaattgggtcttcctttttagccatttcttcaggattaacatgctggctggcaccgatttccaattgatcaacgttgatgtgtggcaaggcaccataacttttgaattttcgagcccggaaataaacgtcaccgtcaacatcgtaggcatagcctttatcgaccaaggttttaacgaagtcgataatttcaggaatgttctcagtggcccgggggtgaatcacgttgcttgaaatgttcagcgcagccgtgtcctgcataaatgcgttgatatacttgtcggcaatggcgccaactgtcgtatggttctgtcgagcagcattaatcatcttgtcgtcgacatcagtaaaattcgaaacgtacttgacttgatacccccgatactccaagtatctgcgaacagtatcaaaggcaatcgcgcttctggcatttccaatatgaatgtagttgtacacggttgggccacagacatacattttaacaacacctggggtgatgggttcaaatttttctttttttcgcgtgagggtattaaatatctgcaacatttcgaattcctctctttatcttttatattcaaataatatcataattcacattgttttattacttcctcaattgtcaaatcaagtgcaacactaagaatctattcttagaagtggtctagttgctaagctagttcaggcattagatcggctgggcagcgatagttcaatgaccgccgtagccggttgtttaaggtatcttgagccagctgaatgtcaatgagtgaggccgaagccaaggatctgcccttcgggaagaactcgcgcaaaaggccgttagtgttctcattggttccacgttcccatggtgaataaggatgggcaaagtagatgtcagttcccttgacttgactcaagcttgagaactcagcaccattatcaaaagtaatggttttaaagtgctcggttccatagtcatataaggtattctggagggctttcaagcaagtgtcggcatgataattgggaagtttaacgatgatctctaagcgactaacacgttcagtcaaagtcattaatgctggctcagattcaacccgtttgcctttgaccaagtcaccttcccagtgtccaagctcttgacgcgcttgaaccatggcgggacgctcttcgattgaatggcccagatttttcttattgattcgatgatgctttgccccggggcatttaatccggcgacgtagtttagctggtaggtctgaattgcggatagctaaacgctggtcatcaatataccggtacaccgtcggtgttgaggggcagacaagccttgggtgatcagtcttgaattggtggacaaaagtatccacactatgcatcctgggacgcgcttttaaagctgtcaccaaagcattacagaaggtttgacaatgatcaaagagtccacgataacagctatttagtcggtgcttacgataaattgcttcaccagtttctgccagatatgactgttcaaagatatgagtactagcgttaatctgtgtcgttgtcccacgttttaattcacgtgaaatcgtgctgggattacgatgaagggcctgggcaatccggcggatagaccaatctaagtcccttagggattcaattcgaccacgttcagctaaattgagttggtgatactgattagatatgatattcttaattcgggtcatgaagatacctctttcttgtttgtggtgaattaagaataggtcttcatggcctttttgactagtctgaataaagaactggtctagtagagcaggtgttgcacttcaattttaaatcgaggttgttttattactttaactataacccataataaaaggtctcgctgtaaatgcaacgagaccaatcgaatcaataatattttttataaattacgctttatcgatttgagccagtgtttctttgatatgcgcgatggctttttgctttccgaccagttcaacggactctggtagttccggaccgtgcatttcgtgggtcacggcaattcggattggcatccataattgacgtcccttgatcttagtgtccttctggatggctttgatgactttaaagatttcaacggagtcaaaaatgtcgagtttttgaattcgctcaagaaattcttttaagaccaccggagccgtttcattggaaatctctgccaatgcatcaccgtcaatttgttccggctcttgaaagaagaccgaggccatgtcgttaatctgagccatataactcatttcacgcttatagagcataatcaactgacgagcccactcgattgttttgttgtcgggattttcaggaatattcccaccggcaatcaactggcgcagcgccaaatccatgatcgtactgttatcggcttccttaacgtactggttgttaatccattccaacttcttggaatcaaatttggcaggtgacttactcaaacgagtctcgtcatacatcttgatgaattctttcttggtaaagatttcatcttcacctaccggcgaccagcccaagagcagaatgaagttaaacattgcatcaggcagataacccaatttgcgatactgttcaataaactggaggactgattcgtcacgcttacttaactttttaccggtatcagcactgatgatcaaactcatatgcccaaatcttggtgcctgccagccaaaagcttcgtaaatcatcaattgctttggcgtattggcaacatgatcatctccacgaaaaacgtggctaatcttcattaaatgatcatcgcagacaacggcaaagttgtatgttggcatgccatcacgtttccggatgacaaaatcgccaccaatggtatctgaattaaaggaaactttaccttttacgatatcatcccaagcatattcatggttcttgggaactcggaatcgaataaccggttttaaaccttttgccttggcgtcagcaatcgcttgggccttctggtcttcggtcattccttcatattcatattcataatgaggcatttcgccgcgtgctttttgggcatcacggtcggcagtaagctgctcctcagtccggtatgattcataagctttaccctcatcgatcaactgttggatcaatggtgtgtaaatatcttttcgttctgattgacgataaggaccataatcgccaccaacatcgggaccttcatcccagtcaagaccgagccactttagattatccagttgactcttctcgccgtcggcaacatttcgtttggtatcagtatcctcgatccgaatgatgaatttacccttgttatgacgggcaaataaatagttaaaaatggctgtacgtgcattgccgatatgcaagtggccggttggacttggagcataacgaactcgaattgcattgtttgccaatgtataacgcctctttcttaaaaataatcaaaattttgtcagtgtttaaagtgtacaatgaacttcgccaaaaataaagggaaggcggctacttcttgttatttgacccattcttgccattccctttattctgatcaggcttatcggtaatgttcttggtcgaatgttccggacgggcgaagaccattttacctgcatctgtttgaatagcactggttacgacaacatcaatgtgatcattcaagaagtatcgaccgtcttcgacaacgaccatcgtcccgtcatccaaataagcgaccccctgttggcgttcggttccgtttttaacaaccatcacgttcaacttctggccgggcagaatcttctgccgcagcgagttggcaagcgcattaatgttaaatacctggacgttttggaattgaatcactttgttcaagttgaaatcattggtgataattacaccatcaacgtctttagcaagctggatcaacttactgtcaacttctggaatgtcctcgtaatccttctcgtaaatttcgatcggaatcagatcttcgttctgcagcttgtttaaaatatccaggccgcggcgaccacgaacgcgtttgacgctgtcactggagtcggcaatgtactgcaattcatacaacacaaacttgggaactaacaaggtgccttcaataaacccggttttgacaacgtcataaattcggccatcaatcaaaatgttggtatccagaattttgtagtgatgatagttcttatcgactggtttatcgataatcttttcgtcgccggccttggcagtttctgacttccgccgggattgaaacatttttcgccagcgatcactctgcgtattgccaattcggaagccaaaatagcccagtaccaacattaagatcgttggaatcatggtattcaagaagaacgtgcgggttctgaagaatacaatcgaaatcaggatggcaaccaccagcccgataatcaggcccaaggtcccaaaaaataacgacaacggactttgctttgtcaatctgacttccacccgatcgaccgctttgagaatataattgccggttaacaacgaaataaaataaaaaataattgcacccacaactgcgtttgtcgcagtgttgttaaacagcgtcccatagcggacttggaatatcagccagatcatcggaaaataactggctccaattgcggcgccggctaatgtaaatacaattctaacaattctctttcttttcaaaaatatcgccttctctcaattttcctttaaccaagtgcaagctttaaagcttgagcaagggttgaaaccccaactaccgaaatgccagtcggtggattccagccctgaagattgttggctggaaccaagacccgtttgaaaccgagtttttgggcctcagcaacccgctgctcaattcgggtaacgcggcgaacttcaccggttagcccaagttcgccgacataacactccgtcgggctggtgccgcggtttttgtaagatgaagcgatgctgaccgcaattgccaaatcaatggccggctcatccagtttaacgcccccggcagcctttaagtaggcatcctgattctgcagcatcaatcccgcccgcttttccaaaacggccataatcaacgacacccgattgcggtccagcccagtggcagttcgttgcgcattaccgaaaaccgaggccgttaccagagcctgaatttcaaccaggattggtctggttccctccatggaaacaacaatggccgatccggtagcgtctttcagccgttcttccaagaagatttctgaaggattcttaacctccctcagaccgtcagtccgcatttcaaaaacgcccagttcattcgtcgagccaaaacggtttttgacagtccgcaaaatccggtaagaatggtgcaggtcaccttcgaaatacaacacggtgtcgaccatgtgctccaaaatcttcggcccggcaatcgcaccgccttttgtcacgtggccaacaacgaatacagtgattccctgacctttggcaatgttcattaaatcagcggtcacttctcgaatctgtgccaccgatccagttgctgactgcagctctggaatctgcatggtttgaacggagtcgatgaccactgcatctggcttcatctcgttaatggtatctttgatgacatccatatcggtttcggggtagacataaagattttccccattgacaccaagccgatcagcccgcattttgatttgggaggcactctcttcacctgaaacgtacaaaatcttaccggatttactgagctgaccggaaacttgcagcatcaaagttgatttaccaatgccggggtctccgccaattaagatcagcgatcctggaaccacgcccccgccgaggacccggttaagttcttccatgtcggttttaaagcggatatccttatgaaactcaactttattaattgattccggcttattgtcatggataccgtttctgcgaaggctttgggttgccattgtgctatttttgggggtgatggtttcttcaaccaaggtgttccattcattacagttcgggcaacgtcccaaatatcttggggaaatgtagccgcagttttgacatacaaattgggttttaacttttgccaactaaattctcctcttatacttacactatcaatattttagcactttatgaatcaaggttgacgaaatgccggcggactttacatcatcttataaattattgacctgacgaaccaaaaccaccgcttcgggtctgttttttgcgttggtcgtcctggtccgccaacagatatggcaggaaaataccttgggcaatccgttcgcccttcttgatcttaatgtcagtgattccaaagttgaggatctgaacaaagatttcgccctcattactttgattattataataatcagaatcgatcacgccaataccgtttggaatcaccaatccacgttttaatgggttgctggatcgattggcaatcacgagcacttcatcaggctgcatataggacttaatccccgttggaattaggaatggcttaagcacttttttggcctcggcaatgctgtcttcccgaaccgttttctcatgtttaagtgcccaaaggactttcaaaaaattcaatttccagatcgatggaatcaccatatcggcagcactttcaaagtcatatcctgctgcgttctccgtcgttcggtaaggcaggcttaagttttcgtctgcatattttgagacaatttcaaatccacgtttcatatgtctggctccttctgtcaatatattctattattgtagtataaactatgtgaagctgtttgcacagattgacaaagatggtaaagtatcgcagtataatggtgtagtcaaacctttaaacaactttgaaatgagggaacaaatatgaaacatcaagacgagttgaagcagtctgtggggaaggccgctgttaagttcatcgaagacggcatgaccgttggtttgggcactggatctaccgtcaaattcatggtcgatgctttgggcgaacgagtgaagtccgaacacctctcaattgtcggtgtcccaacttcagaacggacccgtgaacaggccaacagtctcggtatcaaaaccaagggattagacgagattgaccacattgatctaaccatcgatggtgctgatgagattaaccggaccttccagggaatcaagggtggcggtgccgctcatctttgggaaaagatcgtagcgattaattccgataagaacatgtggattgtcgacagcagcaaaatggttgatgagttgggttctttcccactgccactagaagtcatcccttacggcagccaccaactgcttaaacgccttgatgccaaaggttatcacccaaagtttaggatgaatggcgatcagtacgtcaaaaccgactccaacaattacgtgattgatttgcacttaggccaaattgaacgaccccaccatttggcacttgaattggaccaaatgaccggaatcgtcgaacatggactgttccttgatctggttaacactgtcattgttggccgtgaagatgggccgcagaccattcaagcccgctaattgaataaaaactgacaacagccggaaatgcgatcaaaacgattcgcagccggctgtttgccgtttaaaagcaccctgctcactagccctttttaataaatgagcgtaaaataagattctattaaggagagtgatcatttttgacagcagaaattaatttagatcaaatcagcaagtaccagaagaatcttgataatcgaaaagattcgaaagtgattgaacgggcagttacccaccagggcattttggaaagcagcgaagactttaccgctgaaggcaaaatgagcccggtattttcaatcgatctttcaactggaaaagttgctgatcaaaagcaaagtggtcgatgctggatgtttgccgccctcaatacgatgcgcattcacctcatgaacacttataaggttccggatgatttcgaattatcccaaaactacaccaacttctgggataaatttgaaaaagccaattatttcttggaaaacgtcttaaaaactgccgaccagccccttgattcacgtaaagttgcctggctgatggcaacgccacaacaagatggcggtcaatgggatatgctttgtgccctgattgaaaaatatgggatcgttcccaagtcagcaatgccggaaaccttcaacagtaatcgctcatctcagctcaacaagttcttgaacctgaagcttcgtcatgacgccgttgccttacgtgaattggttgctgacaaggcgtctgaggctaagattgccgaaaccaaggacaatatgatgagtgaagtataccgcatgttgacctacgcactcggtgaaccagccaccaaatttgacttcgaataccgcgacaaggataagaattatcactttgacgctggcatcaccccacaagaattcttcaaaaaatacgttaacttaaacttggaagactacgtttccctgatcaactcacccactgatgacaagccattcaataagacctacacaattgaaatgttgggcaacgttgtcaatggccggccggtcaaacatttgaacctggaaatgtctgaactcaaaaagttggcaattaaacagctgcaaaatggcgaatccgtttggttcggaagtgacgttggccaaagttccaacaccaaaaaaggaatcatggacaccagcctttatgcacccgacgaattattcgattcagatttgtcgatgtcaaaagctgaacgtttggattacggcgaaagcttgatgacccacgccatggtgattaccggagtcgatctggtcgacggccaaccaaccaagtggaaggttgaaaacagctggggcgaaaaagtcggcaccaaaggctacttcgtgatgagtgacgactggatgaacgaattcgtgtaccagttcgtgatcaacaagaagtacctcaccgacgaacagcttgaagctcaaaaacaagagccaattgttttgaagccttgggatccaatgggtgccttagcctaagaatttgttcttaaaagataaatacgacaagtcaggttatctgatttgtcgtattttttatggtctattaaattgcaacgaactactccatgaacgatttactgataatgtttaattgctcatcgaaatcgtatcgaatcggtttgccgttaggaacctccacgttggggatttcttcatctgaaatattttccagaaatttgatcaaggcgcgtaaggtacttccgtgagcgacaatcaattggttcttgttgtctaacaacttcggcgcaatctgatcaacccagtatggaatcaatctctgttgtgccatttccagactttcgcccaacggaatttggacaccataacgatcataacggggatcttcgtcccgcttggccaaaagcggcggcacaacggtaaaacttcgccgccaaattttgagctgctttgcgccaacccgttctttgactttaagtttatttttcccacgaaggccaccgtagtgacgttcgttaaggcgccaggatttatgctccggaataaagttttgaccaatttcatccaagacaatgttggtggtgataatcgcccgtttcagaaatgacgtatgaacgtcatcaaactgaatttgagatttggcaatcactttcccagcactgtgggcctgtcgaacccctttatcggtcaagggtacatcgctccagccggtaaaaatattgtcccggttggcttggctttctccgtggcgcatgatgactagtgttggcacgtttacatcctctttactcaaattaatttgttcacaaataaattcataaaaaagatgaccgaagccaccttctaatcttctcaacctctcaagtcgttgtgtgaacagactcagtgtagcatttctcctaaagcttctcaaccaaaaccattagaaccggaatcatgatcagactcaacaacgtggtttcagccaccatgatggaagcatattcggaatcggcatgatacaacctggaaacaaccggcgcattggtcataatcggcattgcagactgcatgatgaaaacttgtttcatcatcaccggcatcggcgttggaatgaccaatagcgacataatgattggggccagcataaaccgcccaaacaaaatcaagaagttactgcggtcgaaatgaacgttcgttaaatcaacactattgatggaaattccaataaaaatcatggacagcggaatcgttaaattccctatgtaattaaaatcctgcatcaaaaaatcaggcagggtgacgtgcatcaataccaatacgacaccgaccatgaaaccaagcaaaggcggtgaaaaaaccttcttgagagtttgcttccaattaaatgaagcctcacctttgccatctttttggatcaaataaacccccagtgtccaaaagaatgtcgtgttggccatatagtagaccaacacaaacggcaaactggattttccaaacagcgccatgttaaccggcagcccaacgaaaacggtgtttgagttggaaaacatggacatgaacaacccagaatgcattttgggaatcctggcaaatttgaccacgaagattgaaacaatgtaaagtgacagcatcgaaacgattgggaaaaataagtcaggaagtgtggtcagcaacttcttggcagtaaatttttccataatggttgaaatcatgtaggccggtaaggcaacctgagttaccaggcgggcaatcatgctggtcatcttaccgtcaaaccaatcgtttctggctaacacaaaccccaaggcaatcatgatcaggataattaaaaccccagaaacagcattataaaaaacttccataaacattcctcaattctaaaaatcaataacaatgaattattataacacaattagaatccacagccggttataatttttggtataattgaacaagttggtcacaacagatgttacaattattaaataatgtttaaataaccgaagatttctgcaatcaagtccaaatctgccatatacttttgggagaattttttgtaaatgaggagtcaatatgccatcagataaagataacaataatgattttgaaccagtgtattctcgtcgatcggacaagaaaccccactataagaaaaagaaccaccgtcgaagaagaattatcggctggagtatctttttcgtcctgctgatcgccttgggcggtggcctggtctggggatacggcgcatacaagagtgccaagtcgaccttcaagaagacctacgattcaaccaatgttaccaaagctcgaaacgtttcgtcagtgatccagcaaggaaagccactatcaatcctgctattgggaactgatacaggtgccttgggtcgtcacgacactgggcggacggatacgatgattgtcgcatctgtcaacgcaaagaaaaagaccattcatttgaccagtattgcccgagacaccaaggtggtcgtccccggcgatacccagccatatgagaagattaatgccgcttatacaattggtggcgccggaacagccgttaagaccgttcaaaatctgctcgatattccagtcgacttctacgcgatcatcaacatgggcggtttggaaaaaatggtcaatgcggttggtggcgtggacgtgaccccaccactgacgttccagtatggggctgcaaatgtcgtcaaaggcaagaaaatccatctaaatggtcgacaagctctggactactccagaatgcgtgatgacgatccacgtggtgattatggtcgtcaggcgcgtcaacgacagattatcaagaagttagtcatgaagggtcttaacattacctcccttccccgttacaaatcaatcctctcgtcactgtccggcaacatgaagacggatatgactttcgacgatatgatcgccatccgggcaaaatatggcgacgccactcatcacattaagtcacaaacccttcagggagaaaacgcgatgatcgatggtctttcctaccaagtggttcctcaaaacgaactgctgcgggtctccaacgacattcggacatcccttggcttggctaagtcaaccaagcttcaaaccagtcaaacagataccgatgacggtcaaggggcaacccaatcatcatcgacatataatggctattaaataatcatgaaccataaaatagcggctcagataaaagcaaaccaacttttatctgagccgctattttttcacaatcaattttatgtaacttttgctttttaaaccaataccccggcatagtagccaagaactccgataacgaacaaccccagaataatccagattggcgaaattcgcctgcggatcagccagacacaaatcagggtcaaggcaaccggagcaatcacgttaaggccgccattaatcatcgtgtccacaaaccgggaagtcgttgaactgccaaagagtccccgaactgatgcaaaatcaacggtgacccaccgagcaacaatcacgcccatcataaagacgccaaacattgaagtggcactcccaacgtacttaataatcccggtattaaacaagttaataatatcggctccccgacgataaccggccatttgagtcatataacgaaagaccagccgtaaaacgttccatgcaataaaaaatagaattggtcccatcatgccatagccactcaaaaccagactggcagcaaatgccgatagaaccggacggatcgtgcctaaccaaaccggatcaccaaaaccacccattggccccatcatagcagtcttaacggcattaatcgtgtcatcactaatatcggcaccatttgcccgctgttcttccattgacaaaaccactccagtaatcagggactgcataattggtgcggtgttaaaaaagcccaaatggcgcttcaacgcagctttacgttggttcatatccggatacaatcgtttaatcgcaggagccattatataagcaaatccgaggttttgcatccgttcaaagttccacgatccctgctctgtgccagagcgccaaaaggtccggaaaaaatcgatctgacgaagatgaatcggttgatgggaatcgtgaatcatgttttgattatttgccatttatacccaccaactcctataaatcatcaagttctttgtcaaagtcatctaaatcgtctttcccttccccatcgccgccggttgagccatgccgtctactcttaagccaaacaaagctgatggctgcaaccaagcctaatcctgctaaaataaaaagattcatcttcgtaaaaatggcaattaaaaaaccaacgataaaccaaatccataaagagcggctgaccatcatgttaatcaggttggcaaatccaacggccgacaccatgccaattgagatggcaatgccattcgtgatccccgctggaatttgctgcattaactgatgaatgaattgaggagatatcagcatcacgagtcccgtcggaatcaggactctcagcccttgaattcccaaactcagcagatgaatgcgatcaatctgctggatttgaccattttcggcagcttggtcggccgtatggataaatttgacaattgatttacggatggtgacgttcaaaagttggccaacaaccgcaaagggaacggctaaggcaatcccgtgtttaatacttaaggcggccggaccgcacactaaaagagccgagacgactgccggcagcgcgatatccggtgcaacagaagcaccaatattgatccagccaatcgtgatcatctgtaaaattgcgcccagcataatgccaacgccgacgttgccagttgccaaaccgatcagcgtacaagcaatcattggctggtacacctgccattcgtcaagaatgccatccattccgaccacaaatgcaaccaacaaaaccaggctgattgaaactaagctcattgaattcccctcggttccttaaaagccctttttatccaacagggtcaacaaattttcctttttctcagcaggaattttttgagcatagacatctagatgaaagtcatttgccaatgttcgaatttctttggcaatatctccattcatcgaaatggcatcggtaagcatcgtcattccgtcgttataggcaatgctgccgatattgatgccaatcttggaaaaatcgatgccgccctctgctaatttcaacatgtcagccactgtttcggtcaacaacaacgtgttgaaggaatcaaacctggagtcgaaataggctcggatcatcttgttaacggtgacgacattggctttgacaccaggtggtgccacctgggtaatcaatgttttccgcaaaggatctttggcaacagaatcagagaccaccataatccggttcggcgtcaccgcccgtgtccaaaaagttgccacttggccgtgcagcaggcggctgtcgactctcgcaaggcgaatatccattgtcattataaatcatctcccaaattgtcatcattatcagtagaaacttcaaactgacgaatcgaatcgtcagcaatctcattgatcttattaactaattcactcagggttgaatttcgggccatgtaggcctccaacagaatcggaaggttgactccggcaactaatgcaatcgattgcggattcttggctgcaaattgggcggcggcattaaacggcgacccaccccacaagtctgccaaaatcaacgttggcgtaccctcaggaaagtcagccaatgcagaagcgaccttatcactaagtgaatccaccccatcatttgcggccagacttacccaaccaacctgttcctgtttgccggcaatcatttctgcggtcgtcactaagcttttggcaaaatcgccgtggctcacaaccagaattgaaatcatctactcacccatttcttaaatttaacaaagtctgtttacaccaaatatatcacaaaatagcaatttcgtttgccggaattactgaatcgttagtaagtctgcgggcgtctttaaatcgtaatccgtgtccgcaaagtccgcggttttcttggtccgccaaccggccagggcaaactgcacgttggcagcgtgagcagcttggagatcaaatttggtatcgccaatataaatggtggttgccggatcagcgtctaatttctcaatgccctttaaaatcatgtcaggagcgggcttgccttttttaatttcgttggaaaaaacaaaggcatcaaagtattgatccagtccaaattttgtgacatcccggtgaaattcggcttcaaccttggaagtggcaatcgcggttttgatagtcggatcagcatgcagtttcttaaccacatcctcaatcccatcataaacgtgggcatattgggtgtaatctttaattttggcaaaccattggtcccgaatgtcaaccggattcttgacaccaagaattcgaaccgtatccatggaggtaatcccaaagagcttaacgacgtcttcataagagaagtcatagccgttttccagcagcgtcttatgtagtggtaacatatacatcttttcggtatcaatcaaggttccgtctacatcaaaaataaaatatttcattcctgtactccaatcgcttattatttgagcaaaatattacatgctacacaataaaaaagtccgaatcactattgagatgatagtgattcgaactttaaccatgcggccaagaagattcgaacttccaccgggataattcccgacaagatccttaatcttgcgcgtctgccaattccgccatggccgcatcaacaattaaaaattatagcagaaattttggcaattgacaaatggtttttgaaaattattcaccgcgaacggtcgcgccttctgtatcaatttgcagcagccgcaaactaccatttagattttgttgttccaaatcaattcttagctgggttaaagcagctttcttacccagtgtggcaacggtaggaccggcaccactcaagtaagtaccaaagatgtctaacttgtgggcagttgaacggatttgatcaatttctgggaccagctcttttctgtagggctcgtggagatgatcattctcaatcagcttaaccgcctgctcccatttgccctgggcgaccaaggcgatgaaaacattctcctggctgctggcatggacggccacgtcataatcgatttgtttcggcagcttcttgcgactttctacctcgctgacaccatccggtcgaatatacattaaggccgagacgtctggtacaggaagagtcgcagcagtgacggtttcaccgtcatatgtcgaaacaaccaagttgccaagcatcgcagcagcaacgctttccgggtggccttcaatctttgttcccaaattaatttgatcttcaattgaaagccccaaatcccctaacttgttggcaattttaatcccggcaaccactgcggttgtgctggagcccaaaccgtgcgcaatcggaacatccgagataacggtcagttgatgcggatgaatatcagaatcgacctttaagattgtctgaacaatgaggttgtgctcatcagttggaatgtcgtgtcccaaagcatggttgaccttccattcatctgtcttttcctcaacaatcaccgtgtaatacagctgcagtgccaacccaaccgaatcaacacccgacccgaggttagtggtcgttgcaggtactctgataataatttttgccatgtgatggctcctttctacgctccgatttgccgcgtttggctgattaaatgaagcttaccgcgacatctgccgcagacatacttcaccagattgattcttcgtcttctatgatactccaaaccgcagtcttcacagcgataaatataacgcgtttggaccctggtactctggactctgggagcgtatctggagccgccgaccgcttttaacagctgtttaaactgcttggtattgtgtttggcgctgtatcctgccaaatggagatgataatggcacagctcgtgtttgataatcccaattaataccgcatgatcagccccctcgtccatttttggattaatgtcgatgttgtggtcattgaggtggtaacggccgccagtcgtctttaaacgggcattaaaataggcccggtgggtaaacggtttggcaaagtattgcagcgaaatatgttcaacgagttgctgtagttcttgatcagtcatgagttctttgttcacctaaccttcaggatccaccatggttaattgaatccggtgacgatccagatccactgagtcaatccaaaccgtcacgatgtcgccgaccgaagccaccttgctgggatccttgacgaatgtccgactcattttggaaatgtggaccaaaccgtcctgcttaacgccaatatcaacaaagacaccaaagtcaaccacgtttctgacagttccctgcagtttcatccccggcttcaaatcttccattgtcaaaacgtcttttcgaagcaacggtgcaggcatttcgtcacgcaagtcacggccaggcgtttcgaggcccttgataatatctttcaaggttgcaaccccaactccgatgctttcagcttcctgggccaaattgagctgactcaaagcagttgaaacggccggctcgccgagttgattaatggtcaatccgtgctttttcaggaggcttttggccgcagaataactttccggatgaatatcggtgttatccagtggatttttgccgccgatgattctcaagaaccccaccgattgctcaaaagctttcgggccgagccggggaacttgtttgagatcagagcgagcactaaattcgccattttcatttctgaatttgacgatattgccgctggtcgttttggtcaacccggaaatgtggaccaacagatcgggactggcagtgttcaaattaacgccaacccggttaacggcggtttcaaccaccgtgtccaactgttcacccagttgtttctgcggaacatcgtgttgatattgaccgacaccaattgcctggggatcaattttaactaattcggcaaggggatcttggattctgcgggcaatactgacagccgaacgctgttcaacactaaagtccggaaattcgtctctggcgacttgacttgcagaatagaccgacgcccctgcctcattaacaattacgtaataaatgggcgttttgatttctttaattgcatcggcaacaaattgttcagactcccgactagcggttccgttaccgatggcgatcatttcaacgtgattttggttgatgaaatcaatgaacagccctttggcagccttacgtttggcttcactggcaggcttatggggatagattaccgttttgtccagatacttgccattttgatcgaccaccgctaatttacagccggttcgataggccgggtcaaatcccatgacaattttgcccttgagtggcgcctgcatcagcaagttgtacaaattcttgccaaagatatcgatggcgtgatcagcggccacttcggtcaactgcttgcggatttcacgctcgattgccggtccgatgaagcggtgataggcatcttcgattgcatcggtgaccacatcggcagcaaatccttgatgactgccgacggtgttggcctttaaatgccacatgattggtgcctcattgacttcaattttgaccgaaagcactttctctttttcaccccggttaatggccaaggttctaaacgaaggaattgatttgatgggttgattgaaatcgtaatactgctgataggtgccctcttcgtccaactctttaccaccgcgtttaactttgacaaccaactgaccgtatcgttgggtgttttggcggacccattcgcgaaaatcggcccggtcgccagcgtcttcagcgataatttcgtggactccggcgaagactgcgtcaacatcaggcagttctttgtccgggtgaacatactgcgcagccagttgcttcaaatcgggggcaaacgacatggcggctttggctaagggctccaaaccatgttctttggcaattgtcgctttcgtccgccgtttttgtttgtagggcaaataaagatcttcaacttgttgaagaaccgaggccgcctcaatctgctttttcagttcgggggttaaggccttttgttcatcaataattttgatgacttcctgcttgcgcttgtccaaagtttggatgcgatgagcagcgtcttgaatgtctcgaatttgaacttcatccagattggaagtccgttcttttcgataccgggcaataaaaggaacggtgtcaccttcatccaacatcttgagggtttcgacgatctgtttctcccggattttgggtaagtcttgctgaatcttatgtgctaatgtgttgtccatgtattcccacctcatcaatagtgttacgtttaattatagcagaatgaagcaaatgccggggactccaaccaggttttctcagggacataaaagcccaaactgctggcaggaacacttgtctgcagtttgggctgaatgttgaatgttaattttttaattttgggaactcctgttgtggagtgggtttctagatggtttggggaaacgtgcttcgacgcaactgacactacgatctaagcctctttgatttaaatctaaaccccggattttaatcaaagcgaccttagctctccgtgtcaaaacgttgcttgtcgcactctggttgaaacgtgcttcgcgggcctgacgctaacctctaagccagctttgatttaaacccaaacccggggttcaaaccaaagttggcttagaaaccgcgtcacccagcccgcttcgcactctttaaatttctcccataatccgcgtagtcgtactggaaaccttagcgatactattttcctgatccttctcagcttggttgaacttatcaacgtccaccgttgaagcctgcgggtcaatactgtccgtcattgcctggcaggcgttggcatagtcctcataatgacgaaccagcaacttgtgcttgcctaacaatttaaccggcacagccacctgctcaagcttgttcacgttatcttggtacttatcggttccggattgaaaatgggcttgaatgcccgccagctgatcactggtcaaatcagcaaccgtttggttatcaatggcctttctgagtgtttcgtaatcagcgtttaaatcctcaccattttttgacgtctcatcaatcacgtccgagacggtttttgcatatcgctgcatatcttgtggtttcaaaatatcagcctccattcaattttatttatgggaaatgtgtctctgaatgtattttactacttctgaaacaacaacgatcataaagccaccgaagacaacgaccagccattgtgaagcagtcaactcagtcacgtggaacatctcgttgaatcctgggatgacaatcgtcatgatcaacagcacagccgatcccaaaagtgcccagttaaagaatttattcttaaacatgccaattctaaagattgactcatggatggtcttggagttaaaggcatggaacaattgaatgagtcccagagttgcataggccatcgtcaaagcatccgcatgagccaacgcatctgaagcatgaaccgggttggtgatggcaaatgcataaacacaaagggtaataaagccctcaaaaaatccctgatacaagatgttgctcatgatcccaccggacaagaagttggacgttcgtcccctgggtttgcgtttcataataccgggttctgccggctcaacgcctaaggcaattgccgggaaagtatcggttaccaggttgatccacaaaatctgaaccggcgccaagatctgccaacccatcatcgtcatcacaaacaaggtcaagacttcccccaagttggcggaaagcagatactggagtgacttttgaatgttggcaaacaccttgcggccagccttaaccgcagttacgatcgtggcaaagttatcatcggccaacaccatgtcagaggcttctttggaaacctcggttccggtaattcccatgccaacaccgatatcggcggtctttaacgctggcgcgtcattgacaccgtcgccggtcatggcaaccaccttgccctgtttctgccaggctttgacgattcgaaccttatgctccggtgcaacccgggcgtaaacggaaatgtcagcgacttcccggttaaattggtcgtcggacatctcatcgagctgagccccattgatgactttcccgccaggattgtcaccccgacccaagattcccaaccgtttcgcgatcgcttgggcagtatcttgatgatcgccggtaatcataatcgatttgattcctgcagatttggcttccgcaactgcttgagcaacttcgggccgttcaggatcgatcattccgatgagaccaacaaagatcatatcgtgctcctgggcggctgatgtgagctcagttggtatcgtgtctacaagacggtaggcaaacgccaacacccgcagcgcctgagtcgccaaatcatggttggtggcactaattaaccgtttgtcatcgtcagtgatgtctcgaacaccgtccccatcttgaatcttggtgacccgttccaacagctgatccggtgcccctttcatggtcattaggatttggccattgtccatttggttgtaggtagacatcaatttccgctcagaatcaaacggaatttctgccagtcgccgatgggaattgacaaacttttggactggctggtcttgatgtaagtaaaacgacaccagagctgtttcggttggatcgccagccaactcattttcttgatatttggtgtcattgttcaaaaccatgatttgcgctaatcgatcgtttaaagttaaatgggtgtcagcggaatcttgcattttttcattcaagaagactttttccactgtcattttgttttgggttaaagttccagtcttatctgaggcaatgacatcggtacttcccaacgtttcaacagccggcagctttcgaatcaaggcgcggtggcgggccatttgctgggttcctaatgccaacgtcacggtcacaatcgctggcaggccttccggaatggctgcgactgccagggaaattgccgtcagcagcatgttaatcaagctctcttgtccccgccacatcccgacagcgaacacgatgacagcaatcaccagaatcaaaacggttaacatcttacctaatgatttcaggttctcctgcagcggcgtggtcgtttcttcagtggtgtttaacatatgggcaattttgccgacttcagtattcatccctgtgccaatcacgacgccggttgcccgaccagacgtcacgttactgttcatgaagcccaaatcctttcgatctcccaatggcaggtcgtcttccctgattgggtccacctgtttgttaaccggcacagattcgcctgtgagggccgcttcttcgatcttaagggaattagcctcaatcagtcgagcatcggctggaacgacatctcctgcctctaagaggacaatgtctcctgggacaatgtcctcactcttaattgacatcggttgattatttcgcagaacggtcgccatgggggccgacatttcttttaatgaatcaatcgcattttcggccttggattcctggaaaaccccaaacaccgcgtttaggataaccacggccaaaataatcgcagcatccaccgtttcaccggcaaacccggcaataatcgccgcaataatcaagatgatgatcatcaaatctttaaattgggaaatgaacttctcgattaacgtggtccgccgctttgacgttaatctgttggcaccaaattgttcccgacggtctttgacctcctgctcagacagaccagtgggatgggccttcatttgactcatcacatcatcgactgttcgttggtagaacatcttcttctcctgtgtcataaacttcctcctctaaaagaaaagagacccacaaattcctcgctaaaagaattcataagtctcaccatttaagatttatcccggaaatacgagtatttcacgttgacgagataatcgcaatcgaaattgctggttactccctttatttatggtaattatacctaaccactaatgaaaagtcactaaatatctatttccaaaatgtgtcataaacgttaatcggggtgtgacgtttgtgttgcgtcttgtcataccagctctcaatggtctcagcagccttctcagaaacttcgcggccttcaagataagcgtcgatatcctgatacgtcacacccagggcaacttcgtcgggtaatgccggccgattgtcttccagatcggcagttggcgttttttggtaaagatgctcgggggcaccgagtaattttaagagctgcttgccctgctctttgtccaaacgccaaagtggcgtgatatccgctgccccgtcaccaaatttggtataaaatccggtaacagcttcggcagcgtgatcggtcccaaccacggcaccggatttggcaccggcaattgcgtattgggcgatcatccgttgacgggctttgatattacccttattaaaatcagcgacttcgatatcgtttgcctcaactgaagccaccgcggcgtcaacagcaggcttgatgtcaactctggcgacaacatcagcgtccatccacttgatggcttccaaggcatcagactcatcggcttgaacgccatatggcaaacggaccgcaatgaactggtagtcaggatcgccggtttcatcccggagctcggaaatggctaattgagccaatttgccggccagcgttgagtcttggccgccagagatgcccaagaccaatgtttttaggaaagaaaattttttaagatagtctttcaaaaagtcaacagaacgacgaatctcggctttgggatcaatcgttggtttcacttttaacgcgtcaataatttcttgttgtttagctcgcatatgcatccctcgattacaaatttagtagttgatatcttgaatataattgcgaatcttttcgatgatgtcacgcttgttatcccaacacttttgggacagatcgactggatacttctggggatttaactcccgtttgtattcaggccacaatgatgccaattccttttcggcgtagtggacaatctgctttaagtttggctggtcgtacactaatttgccatcttgaaaaattggtttgagcagtggcattgcatcaaaattatcgacagtcttattgatgtaagtatagttgggatggaacatgaagatcgacttttctttgcggggatcttcatcggccagtgtgacgtaatcgccttccgacttaccatccttactgtcagtaatgcgccaaacctgttttttgccgggtgtcgaaaccttctcagcattaccggaaatcttaattgtatccgtcattttgccgtcagcgtcttcaacggaaaccatcttgtaaacagcgcccaaggctggttgatcaaaggcagtgatgactttggtgccgacaccccaaacgtcaatcttggcatgctgcatctttaagctggcaattgtcgtctcgtccaagtcattggaagcatagattttggtattcggataaccggcattgtcgagaacttcacgtactcgtttggaaaggtaagccatgtcgcccgaatccagtctgacgccggcaaaattgatcttgtcacccatttcattggcaacccgaatagcactgggcaccccacttttcaaggtgtcataggtatctaccaggaacacgcagtcgtgatgggtctgagcgtaggcattaaaagcgtcataatcattaccaaacgactccaccaatgaatgagcgtgagtcccgctgattgggataccaaacttcttaccagccaagacgttggaagtggcgttaaaaccgccaatgatggttgcccgggttccccaaagggctgcggaaacttcctgggctcggcgggtgccaaattccatcaacggatcgtcaccgaccaccgtccgaattctggaagccttggtcgcaatcagcgtttgataattgaccatattcaaaatggccgtctcaaccagctgacattcacacaagctcccctcaacttggagaattggttcattggcaaaaacaatatcgccttcataggctgatttgatggtgcctttaaattcaaagtttcttaagtattctaaaaaactgtccggataatctgtcacttcccgcaaataatcgatatcatcatcagtgaattgtaaattttcgatgtatgaaataatgtgttccaagcctgcaaataccgcgtagccgttgccaaacggcagcttgcggaaaaacacttcaaaaaccgccttacgattttccatatgcttttcaaagtaggtggccatcatgttgatctcataaaaatcggtatggagcgttaaattatcgtcttctgacatattgtgtcaatatcctccccggagatttgttatataattagtttatattctatcatttttccgattattaacaaaaaataatcttgcaattcgcatgaaacaaagtctaaaggagctgctatgaataaccaaagtcccacccaaccagttgatatcttgggcatcccttttgaaaataccaccgaaaaggatttccaagcaattttacataacgtcatcaatcaacaccaaaatacgtttgtcgtcaccgccaatccggagatcgtcatgtatgccaaggcgaatcccgattacgaaaaactcattacgaccgctgactacatcgttcctgacggtattggcattatcatgggtgccaagatgctcaaaacgccgctcaaagaacgggtgaccggatatgatctctttgtccatctactggaatggggaaacgccaaccaaaaatcggcgtactttgtcggcgctcagccggcagtgattcgcaagctcaaaaaagtcgtccaggaaaattatccgtttctaacgattgccggcacccacgacggctattttggcgatgatcgcaacattgtccacgatatcaaacggacccagccggatatggtctttgttgcaaccggttatcccaagcaggaagcctttatcaataagaaccgccgggctgccgacgccctttggattggaattggcggttcatttgacgtcttagccggaactgtcaaacgagcacccaaagcatggcagaaaatgcatttggagtggttgtaccgggtcgtcaaggaacccagtcgctttggcaggctgatggtgctgccaaaatatttgtggcagatcgttaaacaaaaatattcacgaaaatccgggagggctcaatgaagaaagtttcaccgaagttttggacctattttctaattatttatgtcggcgttggcatcattgttaatttgctccatcatcaggcggccattcaagacacccagtacggtatgctgggaatctttgcgctggcttatgtcaccagttatctgcggatgcccagatttaacttctatgtgatttactttgtgctgtggatggtgattcttcgtcaaattggcggttatcgtgattggacgtcttggattatcttcgcgtttatgtctgctgtgatggcctgggtcaccgattggattcgatccggctacgctcagcggtatgatcagccaaagaagaaaaatcagaaaaaacaatcataggacgataaaaccaggccaacaaatgtgatggcctggttttttgtgtgaaaagtttttgtgttgctggattgatttcttggaggacggctccgacgacccagatgctcacttctaaggggactgggattcaaatccctcaaaaccgggatttaaatcccagtccccttagaaaacgcatctcccgggtctcgtcgcccactactctttttccaaataaaattcaaaccgatcacccacatattgggtgcggacatactcgaacgggcgaccgtcttggagtgaagtaatctgtctgagtctcaaaatggcgtcgccccgtttgatgttcagatattcagcaatccgctccgatgccagcatcgccgacaccgtctgctgggccttgccgatttgcaggttcttcttttgctccagggttcgataaagcgaactggttacttcggatttttccaagccctcgacaatattttcaggcaccgtggcgacttcaaagcaaatcggaatgtcgtcgccataacggattcgttccatccgtaaaaccgcttgttcctgactgatgtgcaatttttccatctcgctcaaagatggttccatcgtgtgatacgaaattgttttgctggaaggctttttcccctgagccagcatcagatcggtgaagccggtaaccccagacattttctcctgcactttctgattggccacaaacgttcccgaaccgactcgacgctctaaaataccttcgtccaccagggcttgaatggcttgacgcaacgtcatccgactcacaccaaagtcggtcgataactcacgctcagagggaatgcgatcaccaattttccacctatttgcttcaatgtttcgtttaatctcattatgaatttgaatataaattggtaaacccactgataccaactcccttagtttttattcactaatttgccataactatacgttgccataaggtctaggtgattgtcaaacaaatttagatcggcatcatacccattctcaatgaatcctttgcctttcaggtgaaattcctccgcctgattggtcgaggtcattttgacggctgaagcaattgaacaatcggtaaattgaataatatttttaaaagcgtccgcatacttgagaaccgatcctgctaaatgcccattagccagggttgcccttccccgaaaaacattgaccggttggccgccctttggcttccatggaatcagtgatcagttccagccgatccggaccgatcgtttgataagcaatttgtaccgcttcaggcaccacatggaacccatcacaaatcaactccactttggcttgagaaagcatcgcataccccaccacaccgatttctcgctgatggagacctcgctgggcgttaaataaatgggtaacgtgcggtggccgagcttgattaagcaactgataggttgcatcagagtggccaactgccatttgaatcccttgttcttgacaataactgacggctcttgggtcaacgcgcatttccggagcgtaggtcaaaattttgaccagcccacccgagagaatattccacctggcaattttatcaacgtcaagcttttgaatcttttccgtcggctgggcgccgtggtacttgggtgaaataaacggtccttcaagatgaatacctaaaattcgcgggttggtttcagccgccattttaatcgtctgcatgctcttagcaatggcatcggcactttgagtcatggtagtcaagaaaacgccggtaaccccctcgttagccatcaggttgacgattcggctaatcacttgaggatccaaattcatggaatctgcaccataaccaccatgtgtatgcacatcaatgaagccagggacaattgtgcgttgagaagcatcgatgatccgatcacttgactgcggtttaaaactggttgtagggccaacgttgagaattgtttgaccaaatctgaggtagccgtcttggataattcgtttgcctgtatagatctttgcatgaattaatactgttgacatatctgctccacaagtcgactaatggttaccggttgacttggcaatcgtcgcgtcaattcccttgatgacagaaggtaggaatccagcctcttccatcgccagaatgccggcgatagtatcaccacctggcgaactgactttatcaatcatttcagctggcgatttcttggatgccatcaatgagtgcgcagagccaagagttgtttgggccgcaatttgggtggccatttctttggtgaagccatacttgaccccggcccggctgagactatcgataaagaagtcaacatacgctaccgcactaccggaaatggcgctgaataccgaaaattggctttctttaagctctagcacacttccagttgcttgatatagcgagatggcttgagcttttcgatccccggttaagttctcgttggccgcaaccgcggtcatcccctgaccgaattcagagttgatatttggcagactgcgaagaattggcaggttgtaatcggtcaactcttctaatcgatccagcgaaacccctgaaacaattgagatcaacgtcttcttggctgacagttcaccacggatttccgccaccacatcggtgacaacggctggtaccactgccaaaaccaccagatcactgccgtcaacaaccgccgtgttcgattctttcggggtcaggccatattgagccgcatatttttcgtaatgatcttggtgagcactgtgtactaaaatgtcttgagcaggaacaaattctgccttcagcagtccttgaatgatcgcttgagccattgccccaacgccaataaaaccaattttcataagctacctcctgaatttacaatcggactattccaattcttctaacactgacaatagcggaaaatgcaaaattttgcaatatcaaaatggtcgatcgttgaaaatacaaaaaaacgcccgcgacgagttcctttcgtcacagacgtttagtaattgggctagctgggttcgaaccagcgcatcacgggatcaaaacccgttgccttaccacttggctatagcccaaaaataaatggaggggagtggattcgaaccaccgaacccgaaggagcggatttacagtccgccgcgtttagccagacttcgctacccctccaaaagagtgttgctatcaaaccaacgaatataataatacaaaattttagtgattccgtcaagcgcaatcatcaaaaaatttggaacattttcaactgttttgcccattcagctatgaaatcattcgtctgccactcattgtgacgatggttgtggtatcccaccgctgcattatagtatgtcgtcgccttaagcctaataggcaccagtcgttgatgaatatgcccgaaaacgacccgttcaacctgatagtcctcaatcaatttttgaaaatgcagactgcccatcatggcattggccatattccagaagcgaaaatcattcgtataatgaatgaagtgttggttgggaacaaagtgagtcatcaaaatcactttcttgcccgctgattgcgcgttctggagctgttgggtcaattccgaaaggactatctgctcacgttcaggatcgctcataggctgcgaaatcagcccgtctatccagtaggccattttccaacgatgaaattcatcttcagttttatcttcattcacggcaaaagtgtagtcataccagccgttcatgccaataattcggtagtcggtttgagggacgtcaaagaattggttgttcagataccccggccactggccattttccaactcgtcataactgacacctttgatcatgtcgtggttgccggcaatgaaaaaactcggattggagcaacggctgctgacagctgctgaacgtaatccaccgacttctgaaaatcattgaatagatcgccggcaatcaggtaatcgtctaccccttggtcctgcaaaaaagtcgcctgctgtttaattgtatcggccagtgctaccttgttcaaatcaaggtgattatcactggttacggcaatctttaccatcacgttttctccccaaaataaaaatgtgctatccaaattaggataacacattcggtcgttcttgaatctaattgacaccttccattaaccgcttaattggtttaaccaggaatgccaacaaaactccggcgacaattgcaaccagaccaacgatcaagaagtaattaatttcattgtccggtgtatagtatttaacaatttgtgagttgaccgcttgaccagctgaatcggctaagaaccacatactcatcatctgagattcaaaggcttttggtgccagcttggtcgtaacagagagtccaattggtgaaattaacagttcagcaatttccacaatggcccagcttccgagcagccatagtggactcacttttgcttgtgcgccaaataaggcaactggaatcaccataaacagataggataatccggcaatacctaatcccagtgaaaatttggatggtgagctcggctgctttttgccaagtttaatccacatccaagcaaagaatggcgtgtacagcataataaacagtgggttcaacgattgataccaacctggcgaaatattaaaaataccgccaacattattattcgtttggattccggcaaatagtgccaaaacaacggatccctgctcttcaattgcccagaaaatcgcagctgcgataaacagtggaatataggcaacaactcttgagcgttcggtggaagagatttttttgctggaaataatgacgacaaagtaaataattggtgtggccacggcaatgatactcagcaaggtaataaatgagctgagtgataatgcccccatgacctgcatgagcaacaggatcaagccgaagacaaccactcccaaaccaacccggatagtcaatttcttggcatcgttgggttctaatggatcgcttggatacaagctggcactaggcaaatgttttttaccaccgcgaatatattgcagtaatccaaagaacatcccaatagcagccagtgagaagccaaggtggaagttgacgttgaatccgagccaactaaccagcagcggcgcaatgaatgatcccaaattaattccgaatacgaaaattgtgaatccggaatcgcgccgtgtatcatactcggtatataacccaccaaccatttcagaaatgtttggctttaatagtccagtcccaatcgtgatcaggacaattgaggtgaataatgccggcgcacccattggcaacgacagcgcgatgtgcccaaacataatcagaacaccgccatagaacacggtccggcgactacccaggattcggtcactcacaaagccaccgataaccgaggttaagtagactaacgagccataaatcgacataacagacgcagctaatggcttatcaaacccaaggccgcctttagttacactataatacatgtagtaaagaagaatagcacgcattccgtagtaactgaaccgttcccacatttccgtgaagaacagggttgagagtccccgaggctggccaaagaaagaggcatctgcgcgacgttcctggtctgtttgatcttgttgttgcatgtgataccctccaaaaaataaatctaatcttattaacaaaacaagttaatcagattagatttttgattttaaattactcctgaagttcattacaagaataaatcatacagaccattataggccagattgaattttaattcaacagaatcggaggtcacgacaagttatatacacagcaaaattaggcaagacctatttcgtaagtagtatcaaattaataaccggatgccggattgaacttatgaatgatttgtaaatgcagcgatagactttctaatcacaaattcaattgtttccgtattcatgagtgtgtcttgggcatgcgtgaagagcaatgagtatccaactgtctcagcttcggcaatcaccaaattttgttgctgatgtgcctggaccaaccactgatgagcttcgtttaattgggcatcaatatcactatcatgacttgatgagttgagatgatccatcaagtccgataagatgctctttgctttgccagaataagtcagcattttcatggcgatcccgtttaactgctcatcagtcattttaagctgccccaatcggagataattgggctatgatgaacttaacgagcttctccccgtttgcccaaccataaatctcgtcaggaattgttttaatttgcgttgcgcggtcaaacaattcaagttcttttttgtgataactggcttgaggagcaacgagcactaagtcaattggatcacccaaatatgtgtccgcattgttaatgttagttggaatcagttcaatctttgcatcatacagttcaataaagggcctagccgatttagcgagaaagttgctggaaattccactctcgcaaattaataatacttttttcattttgttcactcccaaacaatttgtatttaccagtacagcataacgcaaaacgatgtataccacaagcccgatttttcctgattatccaatcgggtaccgttacgtcaggctatttcaaaatattattatcatataccaatctgtgatatttcttgtataccaattctcgtctgacatcgtccgcagactttatgatggtgtttcatggagatattacaagcaggaatacaaaaatagggaacccaacaaattgtggctctacaatatctgttgttggtaatagatttttatctattactgatgacagattttttgtttttcattagaataaaaaaagcggacatttcctgtccgttcatcaaaaccaacaaccacgaagattttagagaaagaaggaaatgccctatgtcaaatgatactacgaaaatgttgttaggaatagatgatgaacacttaaaaattgagaatggcaaaataggtgatgatggggtaatcagattaaatggatcactgaactattctcccaaggcctgccgcaattgtggggttattaatgatcaccagatcattggctatggttggcggaagaccaccattagattcgctaaaacattgggcagcacggttatcctatgcctcaatcggcgaaactttcactgtaaggcttgtcataccaacttcctggcgcagacgagtgcagtgccgaagcactgcacgatttcaaatacaacccggaaacaatgtttagagaagttaacggaaccagtgagcctcaaacacattgccaatgaattgtccacttcggattcattcgttggtcggcagctcttgcgcgctgaacacgactttcaaaccaactggcactacttacccaaagttctcctcatggacgaagttaaaagtactaagagcgccaccgacgcgatgagctttgaatttatggacgcggaaacccacgaattgattgacctgttgccctttagaaccatctatcagcttcaaaagtacttccaacattatgaccaagccgcgcgagaaaatgtgaaaattatcgtcaccgatatgaactatacctatcccaaattggttgggcagatcttcccgaacgccatcgttgtcatcgatcccttccacctggttaacgctttaaaccgggcttttaataagacgcgagtgcgtctcatgaaaaccctggccacttcctcacgccagtatcacgccttgaaacgctattggaaactattattaacgccggccaatcaccttaactacgaggctttccgtaagtggacaaacttcccttatccggcaactgccacggatgtggttgatgctttactggacattgatcccgagctcaagcaaacttacgacgtgatgaatcggttacgtgaaaccatcaaaaaccgcgactggcccaactataatcaagcctttcaccacctgcaggggtgctcggaagagatgttggcagccctccaaaccttggcggctcatcatgatgaaattggcaacactttcacccaccactacaccaacgggccattagaaggttcaaacaacaagattaaagtcattaagcgcactggatttggttaccgaaacttcttcagattccggctaagagtgctgttcgcttttcgagttcatacaaaaagagccctaatcaccaagtgattagaactccaatattttgttcaccaacaacagttgacgaagaacccaaattgtcattcgttggtttccctatttttgcgaaatgctatgccgactgcaggcacaagtgtcccttacaaacgttgatataaaagcatttataattttaattggccgttatttgaccgttattagctattttgtcctcaaaaatgatagttcaataatcaaaagctaatatatgcataatattatcaaaagcacaaaataatattaattaatatataccaatatatgtattcccccccaaaaaaataattatccaagggggattcatctcacataaatttctcaattaaataaataatcaacggtacaataattcccgttgccactaaagaaattaatgcatagttaatatgtgtaagattatcaattcgatgttcattttcaatagacttagccaaagctttatctgttttagcattcaaatcagcctgatcattcagttgttgtttaatggaagaaatatcttctttaatgccaatgagcattttagtcatattgatttcatcaggaactcccaccattatttatcaccagcctttactgcaaaaataaatttaactttatctttgtttgctgtatagtaaccggttggtgtagaaaggcgataaatttcaccatattttattggggtagcatagaatcgacttcctttaatcagacgagtatgccgtttagacttgaattcagcatcgttaaattggtgaattacgctttgtgttgcttcgtataggcctggagtttgataatattccggtttagcaggtttaataactaccccacttccggacagtgaaccatcaaaatctaagctggcgtcaacctttaatccatcatagttatcggtatattgccaggcattcgcattatcaatgcccggttgactaacaccatacgccgctacccaaatatgcttatcaataagtttcgctcgatcaattcgcttttcagcaaaccatgaaccggatccataagtaataacattggtaaatccgttggcttttaactcctttaaaaaggcatttacttcagctgtggtcttccaaggaaggtcttgtgcttccacatctagggccaagactgtggatttatccaacccaaagctttttacccaagctaagaaatacttagcttctgatgaaccatgaccatgaaagaaatgataaacactcacagtaccaaatactttgaatccgttagccacttgttctctagctttagggttaatgtatccagtgccttccgtcaatttaaccaccgtggtatcaattccgtgacttttcagtgacttcatataagactcggagcttccttgaaatactgataaatcagcaaccttttttgtcattttcgtcacttcctacttttgttcagatgattggggttcgttaaatacttccggatcgtcatcgactggaacgtcgggtgtaacgtcattggtaggcgccggagtaacaggtgctttgtgattatctccctttagagtgtgtttataatactggtaagcttgttctgctaatccttcaattgtttctgctttaaaattaaagccggaattttttaaattggaatcaataaattggttaaccgcctttttgcgatctgagttacttaaagcaggcatacttgccaccacaggaacgaaagcattcgctaatttcaagcctaattccatcccttgcttgatatgagtattcttttcagttttaattttagcttcaatcaacggtttaaccaatttgtaagttgctggaattacagcaattaaaaaagcaaccaatccggttgctttaagagaattaaaaatatcgacaatttgtgtgtacataaaattacctccataaaatttgtgtaaaagaaaacgccccgctttaaagggcgtcctcaattcatatcatattgaagaacatgaaattccttcttggaggaatggaattccacgaacacattgtatcacgattatatagtcgtaacaactaattattaaaaacaaacacgcccatcttatgacgggcgtgtatacatcacatacattgaggggaatgtatgagcaaataagtatggggcattcataaatgctcagatgaatgttcgaatgcgtaggcaccaaaggggtaatgcctacgaaaattattataccactgttccaaaaaagtgaaggactttaatttaattaaacttgcattccaaaaaacgtctacatgtgagtgtactcaactgaccgtcaattaagaagcagttgatgaattttccacccctgtgtcataattcttaccagtaatatcagtaaactgatcttttgttaattcattccaaccaacgaacagtttcaatttatcataagataaccaaccgttatcatattcaattttaagcattccgtgccaatcaatattaaacattgtattacctccttttattaagctggtgaattagttgtatttgctgccggtacagcagttgctttttcagaagcatttaattgagtttgaatattttgtagttctccgaggatttgtccttgaaccactgaaatgttacttaccaaagctcccaattgtgaatcagtttgcgtacctgttgattgcaaagattgtaactgagtttgtaaggttgttacatctgtacttacttggttcaatgaaacactcggtaagttacctggattaagcaatttttgatttgttgcatcatatcggaatttatctggatattgagcgaactgattaatccacgaatctaaaacgaacacctttgtataaccatcagtttcgacttttttataatcagtaacaaaaccatttgaatcaaacgtaacataaataaacattttaatcatcctttctaaactaatttgtcataattaacaaaacaaaaatcatgtttgccagtaaatgaactataaagagaacttgcacaaccaccgccacctgtcaatgcaatatttaacaaatttttgctaacagttgttgtgctattcgaatcattattttgtgcaaaataattattaaatgaaggtaggcttggttcagaaatattgctaactacactgctaaaatcaactgtaaccgtagtttctgctaaaagagcatttatcgtgaacataaaaagcaatcgtttattaagggtatctaacctataaagaacgtaagttccattagcaaaacctccattatttgaatcttttatatatttattatctaattgacgccaagcatttgcttcaacgctttttaagtcagccgccgtggcgacatcgatacctcctgactgcaagcctgctgtaaagtttgctaatttatcagttgtaaccacattacttgttgcagtattaactgccttactaacatcagttttggttgccacgtcaattccagacttttgaagttttctcgtaaaattagtatcttgccccgtgcgtgctaggtcagatggtaaactgcttgctagtaataacggattattgttgaccgttggaacggtatcaaaattgttagcaccagataggtgggctactttactgtcatcagcaaacttaacccaactagtaaaaatattatatctattccaagaacgcattcctaaaatagtattattcgttccatatgcaagttgaaccccatttgtaccacccacagtaattacttgataaattgtaatccaatccgcattaggcatcccattaattccactaattaactgataaaacccagcagttaaaatagtattcatatcagctgaatttaattgagttacagtcgtgtgtaacactttactatcgtcagccggtgtgtaaccaattttatcttgtttggcgtttaaagcattgttcatatcagccacttttacataatcagctaaatcaggcgtaatgcttcccatgttttgccatgaaccatctatccagatatataagtccgttccgactaagtaaccatcaccctggttgttacccgttgtgggtaaattttcctctttatcagctttccccctaacaaccaaaccatttccttgttttccttgtgggccaactggtccaattggcccctgactaccggtgtcacctcggctagaaacaaaattagtttctttagttgttccgtcatcgtaggtaaaaataattttagtccacagataaggaagctgatcggttgtcgccaaaatagtatctgaccagccccctgtgggaactgtaactggtgaatcacttaactgatactgattgttggcagacttaataccattaccagggttaccttggtcacccttatgcacattgtggactgcattctccatttggctacttagatcatcaaattgttgctgaaaatcattcaaagtaattgtcggaattacttcaccagtatcactcatcagattctcttcaattgaaaagcctaatgtaccatcacttggaaagatagcctgtgtaccatcattcatagtaacccaaacttcaatatcataatcatccggaaccaatgtgttcataatatcctgattaattggaaagcttagtgttccaccaagcggactagttacagtggttaaatcaatagtttgttgcatgatgtagccatcatcattagctatttttaccagaactgacttagcattagttaaatcaaaggccaccccgtcggccgtgagtgccagattaaaagcagtggttgtatctaaatatttaaccacatcattatcatccgtgaatgcgagctccttactcattagttttcaccttctttctaagctgattattttcaatttgtaataacgcaatttgttgattttttgctgccatatcttgactgtactcattaactaattggttaattaaatcttgcgcgttaatatcattcatcagatcaccttacatttttaatttcttttcaatcttattaatttcactaagtaaattggttccatgtgaaatgacgtcaccggcatgaagatcaatcgtcgtaccagcttcattgtggaaataaatatcagttcctgaaactgatgaaatataacctccaggaccacatttaattccttctgccaaataggtccatgcattttcactaccaatatgagtattgttgccgccatatgcttgaaaagtttgtccttcaatgattgaggatccaacgttaattgaatcaacatccaagccaccacgaatttgagtgtacccattactatttccagatacaaattgaagatatttaccattactaatggcacaaaaaccgtttgtgtctaatgtgatccttccattattaccatcttcctcaattgatgcccctgtaattgttgaagttgcatcaagcttggcggctttaatgattgatgagtcaacttccacagagttcaaatatccggcttcaatagttcctaaatcagcagataacgctgaaagctgaccaactgacaaggctgtttgggacatcttagtcttaacccaatcagatccatcataagtatacatttcactagttatatgattactgtcttgaacataccaaatatcaccttcatcatgggttttcccatcatcaaatggttcttgagatgaaacagtgattttcccatccaacgatgttttaatcttacccgcttcatcagctgcagaattagcggcacttttggcatcgtcagaagcttgctgggcaagcttagcattttcatcaatatttaaagttcccgttgcaataatcaatcgttatcaccatcctcaacttctgtcccttcgccagttgactcatcaccatcttcatcactatctgaacttgcatccgaatcatccgcattatcatttccagcaattactggttgttcagcctcatcattctcgccttcatcttgttcaggatattcaacaactaagtctttagaatcatcacgaattttaagtggagccgtatataatgcactatgagcaatagacacagtatgtgcagcatccctatattcagaaacgttaaagccaacaattaacctagaattattaacatcttcatatatgccctccggctccaaatgaccgccattttccaacggtactgttaacttaatatcctgcattggttccaccacataatcaaataccattgactgtgtaattaagttaatacacataacatgtttgtcatcagcattgttagcatcacccgccgtaaaaaaagcaaatggataactaatcccatttgcctgaagagtgttataagcgccattattagtggttccagctggtaatggcttccacttaaaatcttgcaatttaaattcaatgattggtttgaagtttcctgtctgtaaatcgcttatctgacaaacatacactttcccactcgtcgtacttcctagccacagattgttcttcaaatcaacgttaactcgaaaatattgttttacttggcaccacttggttatattactagcacttgtattggcttgatatgccattgttaccaaataatatttcccatcaattggatcttttatttctgtataaattgtgttggaaccttcatcatagccaaacgatccgcaatggccacctccagttacaaacatcatgctttgtaatgttccatcagcgttccatttaataaattcacaatctgaatggtttttgtctttagaatagtgataactagacaacaccgaaccatcactcaataaatatgaaaattgtaaggccccaatatgctgatcgccattaaaatctttgttggcggcatccttagtttcccaaagcttctgccaagagccgtcagctgaactactggtatcaatccacatttcagcttgatttttaacgtaagtatcatcaattgttacaagtaaagtacctacaaatggtggttcaatagtaacctgataaccatcttttgcatggtcagcttcccacccaatatcacgggtaccgtccatattaattttttgccaattaaacgcttgtggtgatagataagaggttacattctcaccttcaataaatagtcttgcaatcacccgtttggaagtatccgtgttataccaagttgaacctaacggcgtaatcaaactgactgtggctgcattggcattctctcgggcttcttcaaatagtttcttaacgtgatcattccaacgctgttccatattgcgaataaacgccggcgtaattactttaactgtactgaactctcccaagacgactttattttgacttgggtcactctctgaagtggtttgctgaatgactcttgcctccgttgtcaaaatcgggttcatagataaatcaatcaccttaatagtatcgcccaagttagcttgaaaatcttgagttacctccacggcatagttaattcgtggatgattgtacaatcttaattcacgtaatccccaatcaagtaatgctttaggttcagtaatggtatcactcgtgatggtcccttctagccaggtattgctatcattgttataaagagaatttgctgaaacgtcagtaatataattcttgccgttattaacctctgcaattgaagcattatttgctccaacgatatagagtttagtaaccaaattagtatcaactgtttctcgttgaacagataacatgttttgcccataggtaattgacttaccttcatcttctcctaattgatcagctaattctaaaattagatcagtcacgataccgttggagtcaatatgacaataggcatcggcttctgcatcgtaagttgataagactgtctgcaaggctgcttgactagaagccgtaccatcaaagctaatatcggcaaataatcctgaagagcaattattttgtaaatcccaaccggtatctgccatgatccattgcatagcttgatctaatttacaatctttaatttctttttggggtggaatggtcttatttaatttatagattgctaggttaatagcatcaaccgttaccagatgagctccactagttgcatcaatgttttcgtcaacctgatagattcgataaatacgccaatgattatgcacatcatcatacactgcgacactattaccaaccgttaagtattgagccgcaggggcactttgcaacatggttagtcctgttaatgtatcattccaacttttggagttagcatttggatccgtactattaaaagtgctaacgccagtaataccatcatccgagttactgttatcatcggcaatttggcgttcaactacttcaccccaaaacgggttggcgtctgaattagtcgataacgtggcaactcgctttaaatttttatccaggataatatacaaatctctaacctccttatttatgtataaaaaaagtagtcgctttcgtgactacttaattgctggtcgatattcaattgttacatcagcatttttgggatccgggaaaaagtgtagagtttgtggaaccccaccggttaatttagggaaggtcgataaccatgaaacgtatttatcggccggctttccatcaatagtaactttattgttggccgtatcaataataatttcttgaccagccttggcaataatatgtggtgtatcatccggatcagtagagccatcactgcgccattcttcataattggttaaagcttcataatctgacttatacgccaccactggattaactaagtcctctttaatatcatgcttaccaaagaaaacgcctaagttggctaaagcaaaaccaaacttaccggatttatccaacttttccttatgcatgtgagttttacttgtattgttaacactatatggctcaccggttttaggatcccactggttaatttctgctacccagttatcgtagatattccccgaactatccgattttttctgtcgttcaagaataaattcaccataaaaattcgagtaggcatccttattcatatacgaggtttcagttacatattctttttcctttttctttttcgttgtagctttgggagctgatgtttttttaccccctttactactactcttcttgccaccctttttagatttcacaactcgtttctttttagtcttagtctttttacgagtttttcgtttcttccgcgcaaagaattgtagattcatttatatcacttcttcttctttttggctgtcttcttcttaacggtgaccgttttggtgtaggcaactttaacatgcttggtagcctcattttgtttctgctgaccattaccttcatcaaacagcaatgtcaagtagctatcagagttactactatcaaaattattgcctaattgaataaacgcccgtggataacggcccattgagtaatcttcaatccccatccggccacaaacattaccattattatccaataaataagcttcaatctttcccattgcccgctcatttttcattcgtttaacatgatgcaaacgcaccgaaactttccaataaggagttatcttaggtaagccattatgcataactgcggggccgtaaaagttcttgtgtttaccacgagtaccccattcataatggtcatctttatctttagccaccataattgaagtaccagtggctgccgattttccatctaactcacccttataaattggaaaagcttgtgtattttcactacattgaatccacgttgctaatgagttacatgggtcgtcaacctgttgagtttgggattgtcccatgactgtgacgttgccatcactatccgtagtcgtatcaccgtcatcaacattatatccaaccgctacataatcatcatttgtttcataacccacataataaagatcggttttcggaataatatgaataattggatcaacttccgtatttccttcgggaataatttgctgatcattgtctgtaatttttatttccttctgtggtagaaatccacgtggatctgccagcatgaagactaacgtagtttgaaagtcctgaacaccttcattaataaatgtcggtgttggaatactcgtaaagtgtccataataagttacatctggatcgtcattaaacctcaacggatattcagtatcagcatcactgctggtattaactaaaacgttagttaatgttttaattcgttcgttatattcatcgcgggtggtacagaaacaggtaattggaatgtcaaattctttttcaccgtaatctgttcccaagtacacaccaccataacgtttagggacgtcttgaaatgactcagtaatattgggggctaacggtttcgatacatgatttagaaatatgcctaaatcgtcttccgaattaaaaccaccatttccatcttcatcaaacgcaaaatcaaatgtgtttacatcataattatcgttattagccaaaggttacacctcttccccaattattcttagccgttgttcgtttgttatgcttattgactgcctgaacaacttgtttgtcagttacgactgccggaatcggattgttttggccgtcgaccaattgactcataagtttaatcattgtatcaaacttagcttcaagtcttttgacagcctgaccatccgaattgcttgattggttggtgtgctgatctgtttgcttaaaatgagccatagtatcagctagcaattcataggctcgtcctcgtttattaatatcccatggaatgatggtttccggtttattacgttcggctactttaattaactgttctttatcaactaagccgccattcgcatatcctaaataattagcaactttcttcgcaccgttaacgtgttgccccgtataaccgccacgttcccaatcttcagaaaactgactggctaacgaagcgatcgaaccgtggccttccaggattcgtttaaatacagaagaatcggaactgtcatcgcttaacgcaaactttaattgggtagctgcattgcgccagttttcaccatgacgatgagcatatgatttcaaatgattcagtctaccacctaaccactgcccaagcccagaagctccaccagatgaatttcttgcgttaggatttaatcctgactcaaattcccaattaccaagaattgcagcaattcctgctttagttgcgcgtgaatccagctttttcaacgcttttgctaaggttttggctctagccgccacatcgccacttaatccaaaactacttaaactaccgaacaatttttgccataatggttttaagttttttgatacccaaccccaaactccagaattctttaattgtgactttactagtgcttgtaatccggagctttgtttatgagatttagttgactttttaactttgtcaatcaatccaggcactcttcggatcccaacaaaatcaccgaatcccttgatggtagaatatttaatcccgtcctttggattttcagcactgaacatatgtccagaaccactgttatcgaccacaataccaacgtgttggcttcctccacgaccgaagaacgctaaatcgccagtcttcgcattattccaagatacaggcttagaaaagttgtattcagggacagtagtcgagccaccaggaactgtaattcccatgtgtttcaaagtctcataaactaagccagaacaatcataataattcggtcctaagcggacattagagccttcagaatatcggtgatgggcacgatttgccaatttcttagcttcattcaaaaatgctgaatcagtctgaccgccgccttcggaaaccatgccatgtagcatattccaggcagtatcccaccaaaccgaaccctgttgcttgtcccgtttgccaaacatattggcaaagttctctccaaccgttccctttatatcgccaaagtcaggttgaaaaacttgtttgaaagttgtatctgaatgcttagcaatatgtgatagtgccgacaacttctgttttaaagaaccccaaatacctttaaaaaatttgccgataccaccaaacaaaccagttcctgacgcaaagtgctgcatgccatttaaagccattaacatcttagactctgtagcatttaaaacgccggaaccagcttctaggaaccggtgagtatctttaccttcaactggttctaattgcccatctgcgtggacaatgatttctttattatgtgtttctggtgaatcgtgaccatcattaagcttagccaaaactggtttggttaataagccatttttcaacaatccggtacctgttgcccaagctaccgctgggatctgatccaaagtttgtgaaccaccgtattgtttaaagactttgttctgggctgaaatggcattcttattcatcccatttaccagtttgccaatccaattaccaactgacttccaaattccatgccaggaaagactgtaattatctttagttttggaattgtttttcttgatgttctcatattgagaaacagcttgatccgttactttatgattttgattatgtgcgtaatcgtacactttgtcagactgctgtttggctttagtgattgaatcgtttttttgtttatcggcatgattaatcacaccaattctttgtttacgagcctcctcaataattttttggcgttgtgccttggcagccgaactatttcccttgtactcttcatctgctgctttaactgtatttttatatttcttccaagctgaattatagacactatgatattcatcgttagcttttttgctgacagacttttgttcttcatcagcgtttgccaccaatttaatcattttttctttggaatattttttactcttttcagtgagcgttttataatctttagcaatcttattagtagacagtttaatctgaccagctaaggttgtatgcagtttggcttctttagcagtcacttgagtagcaaacttaagatgttgtttctcaagtgcttctttcttttccttctgcattttttcaacttgaacggaccctttaccgtatttattctcagcttttagaatctttttattccacgattcggttaatcgttgccgtgattgcgcataatatttggcaattgcctgctgatccttttgactcatcagagttaatcggttggctttagatccttcacctttaataatttgcaggcgtttttcgtactcttttttagtaatgtccccgtttttataaagtaattgtaagttcttcttgtcctgagcttcacggtttttataatagcttgtcgcttcatcagaaagtttcttgaaagaagacttagtagataatttaggtgtatggattttttgtgctgaaagtcctttttgaatagctttaccaaacttacgaccaacaccttcaccaaccaagccacccaaaccagcgccaacagctgtgccaattccaggaagaatagctgtcccgattgctgcacctactgcagtaccacctaatgaaccggtagcagcaccaatgtgggaaccggcagtcttctttttcataccaattaaatcagttgcagaatttaagacgtctaagacacctacggaacctgcagcaacctttccgaatttactaacacccttaaacttttcagctaatttagcaaatcggcctaccctcccggtatcttcggcaactttacttgtatcatctatatcgtggatggccgttttaccatctttttcggcaccttcggcaaccttaccttcgccaccagagttatcagcaatatcatcaattgcactggtaccatttccggcatccacattagcttctttagccttagtgttacgttcaatagctaaagtttgatcatcatatgctgatgtcaatcggttcacctttagcttttgaccgccaaagacagaggtaatatcactaaatattttaaaatatttataaactttaccaactgcccaaattgcagctaatgcttcaccaaaatgtttgacgccttcataatgcttaacagcaaaaataccaatattggcaattccttctgccacatgtgcagttaaagtagccgttttaccaatatctttctgaaatcctttttcaccaaaaagcttggtcatttgattagctgcttttgtcatatacggcaataacttagacccaaacataattgataattgatcccaggcttgcttaaatcgtttctgagacatttgggcagtttgagcatttttgttagctaatctttgaacgtacgtcccagctttgcttgctttagaaacattgttggttaaatcagccaattggccattatatttagctaagatttgagctgcttgcatgccggttggaccaaaaatatttttaaagatgcgtgctgtatcagctccaccaagttttttagtatgttcctcaataattttaaaaattgcaggcaacgttttgaaattaccattggcactttggaatattttagttgatttaattccaatttcatttaaagcgcccatagctgaatttgttggagctgctaaactagtaataatttttcgcagacctgtcccagctttatcagcttccagaccgtggttacttaattcgcctaaagcagcagaagtttgctcgatactaaagcccgcattattagctgaatcacctacatactccatacctttgcctaaactttggaagtcagtagcagtcatgtcagcagaataagctaatgcattaactacacgtttagtgttgtgcatcatttttgccgtattattggttttcatgccaaatgcttcaatcgcctggcttgatactttaaccacatctttaaagtcgtcacctgaagccacactggcctgtagctcagttttcataaccgctaacgactcagctcctgtatgaccacgcttgattaaatcctggtattgatcagcaatttctttttgactaaccccatatttgagagcgtacttagccccatctttttgcatttctgtcacggttttaatagcagttttagccttgtcgccacccgtaaccagtaagttttggtttactttataaacattttgaagttcagttgcttttttagcgccagaaaaagctgctgctcccaatgtccccatcgctacgctggcacctagtaaactacctttaattgatccaaatgaatttttaaatttattcttagcaatgttagctttatcgcccaatcgcaccattgcatcactcatgtgaccgacttgtaaatcgtacttgaccacatcagaacgcacattggccagtgaagtggctgttttgttgactcgtacttgttgggtgttaaaagcttcgttagcaatgtccaagctaccttttaattgattaagtttttccttttcttgaacatattcatccgcattcttgtgggtatcattggcgaggcggttaacaacattttgttgtttttcataggccaactgggcttgtttataagcctgtgagtttttactgagttcactattttgtaatctgtactgatcagataagctattcaatccttccttaaggcctttaagctttacttgaccagcctggttaatctttccttgagcctttagcgcatccacataagaattagttacctgattaaggttatgatagttacgctgcaatccagatagtcctgaattaaggtattcaaattgcttttccgccttagactgttgatcatttaatccagcaatcttctcttgtgctttagcaatctgattagcatatttagcatatttttctgatccttggttggttgtttgatcaaggcctgactgtcgacgtttcagctcatcaatttttaagttataacctttaatttcttctgatattccttgatacctagtttttaaagcatctagtttatctccagaagactttaaagccacctcctgagaacgccatgcattggtattagctttaatgtaattggttaaagtctttaatgaccgtgcgggttgtactgcatccaagcgaattgaagtactcattacatcattaatagtagccatcagtcagtcccctttcgtttatttaataattcgacaaccggatctgttacttgtttcttcttatctttagcatttaagactgccataaattcaaagtaatcttgtcgatttaattcatctggtaagattccctgcttcatcatttgttgtttaaaaaaaagcatatcttgttgggatatgcttaggtcattaattaatttggctaatcttaattgctttcttttgggtctgctgattcctcagtttgttgtttagtaacagtttcccaatcttcatcgctcattccttgaaatctaaatagtacataggccatgaaattttgaaaatccgtaaaatccaaagttgatttaatcttttcaacttctttgtcggatagcttaaaaatatcaatcataaattgcaataatccttgaaccattttcttttgcgtttccaaaactgctagtgggtcatcattagtaaaatcaactgcatctgatttcaacaattgaatttgtaaattttgggctttctcaacaacacccacagtggttttaacttcagctgactttttacgtaaacctaattttgtaatattaattttcatgatcaaagctcctttattttatttgattatgtatgcggggaatatcccccgccttgatctattttcctggtgttgtaccgccagtcgttgagccagttgtgctacccgtagtcgatccagtggttgaaccagtcgtgctaccaccggtagtagctgaataaccaccaaagacttcagccagcattttggctttatcaaagccagcatcttgagacatccaaatcttgtacggttctccgttgaagattgtattgtcagctggtgttaatgcttggtaagttaacgccgtattggcatcagtttcagcattattatccgttgcatgagaactaccagtttcaattagttgaccattagcaaagccttcgtacatatcaatgttcgtgtatgaacgaaaatgtaacaacattgctacatggggctttggcaattgacgtgtccaaccaccattagccgcatcctgaatatatcctttgagtttttgcaactcgtcaaaatcaatatccaagaattccaatgcgacctgtggttgtgcctgaccatttgaaactcgttttgcttcatcattagcataggcgacagtaccctcggcttccaagccagaaactgtggccgtcgtagcaccttcttcgtcaccatcgactaaatagataccattagttcctactcctgcatcgctagtcagtaatttaccattagcatcaactaaaccaaaggtgacatctttaataccatgtgttgacatttaaaatccttctttcttcattgtaattgtcttagaaactgaaaaagttgccgtaatttgatcggtatctggatccacagtgttaggctcatgtgagctaaccagccaatcctgattttccaaattattcattaaagtaacttcttcattaaaaatattttcttgtgtttcttttttccaaaatatttgaatttgaatattagcttgcatattgctaaatcgatcgttccgatatccacccaacggttcagtaactgaagtaactaatacaatggtctgctttccagaagtatcagctccgggaggaatgttcatggaataaagctggtcaatccaaccatagtgcaaagattgaattaactgataaacagtcataactggtaattccattagtgacccagctccttccacttaatatattcagattttaatatatcagaacgagtttcctcacgggtcttttccacaaagtggtcaccgacaatgtaaacagtgccatcatttagccagcgagcaatcactgcttttttcttgacccagccaactgtcgctgtcccatccacatcaccatcaacatttttcgaactaactaatacactatcagccaagtgaggatcatttccggtagcaattcgattactataatgtagccgtttagtttcatcagctaatttcttttgcaaaacatcggcaccggctttagtgattatagttctttccgcccggttgggtaccaatcgttttattttcgctaaataatcgtctaattgttcggccatactaaccatgttttttaccaaccctctcattaatctgtagagtcaaaatgtcataagtcacaattttattgctatcatctaaactcaaattaacgatttgatatagttggtcctgatattgaactagcagacctttgtcaattaacggattgtgtcgaataacaatttgaatagtatcttcaaaatctgttcccaaaagcgaaacgttctgtgtgttagttcgcgtataaggcatgcaccataacacgaactgtggtttaaattgcgttcctgatgcaccagtattaggattaattgttggtaaagccgttccaaactgggcttgccgattaaactgctccggactaaatttattaagtgccatccggatcacttcctgaaaccattccttggagttgatctagcatcatcaacaaaccagctgacatccctttagataattcccgatcataatataattgagttgccagtgtttttattgctaggtcgtaaattgatgaggcttgatattgggtttcagttgaactgactgaatgattgacaatctcagttgcctcattaatcaaattggtaacagtcgttaattcagtcggactttggtcaatatgcaactcatccattaattctgtcggattaaccgtcacatgacacccctcctaacagccgcccatcactgtattgtttatttcattggcgacttatttaaattacttgccagttgaactagtagtcccactagtctttgcagcaggagttaaatctgctaatccagtaaatggcgcataaatgaccgattcagtatcccacaactcaacatcaaagcgatcaatggcacgaatcttagtcaagtcactttcaaaagaaccagcaccaatattagtagccaacaaagacatctgttggagatcgaaaagtctaactgcttctttcaaagcaccgatgtacagtgggaaactgttaccatcgtttggcaaaaaggcatcagcaataactgtaattgtcttaccagccagcatcttttgtgatgggttaagcgggttaggctgaatgacgtattgtccgttattatccttgaccttgtccaagacagcaaagcctgattggttagtaataaaagcagattcattccaaattaatgggtccagttccttgttgtaaatatccttaatggcgtcaaaactatcaactgtggttttttgtgtggttggcaatttagccaatgcttttaaaatttcactgttccgggtaataacatccttcttagcaatccaattttccaaatatgccaagaggtttgcatcactgtcattcatcaaagtgttggtaatactggaaattcctgcatatcgatggattttgtaagttaaaggcttaaaggctgccggctcatcgttattcccaatttgagctgtttcatcgtccaaattagcaaatggagttaccgactgacgtggttcaataactcgtgaaccagatggtgcgctaactccttccacagttactaatggctccagcgacgtaaaggtttgcttcaaagtattgatggccgtttggacatcttctggaattgtcaagccaacaccgtttccattggcatcaagtccactagacatcaaattcaaaaactttggatcaccctttaaggctcctttaacaatattaataaatttaggtttgtcttttggtgtaacatttttctggccaccagtagctggtttacctggcttagccagtttagccgttgctaaagcatcatcatatgcacctttagcaaaatctcgggtcttctttgctttatcaattgaatcagcaattttagttagatcctcatctgaatatttttcaggagaatcgttcagttcaactgccatttgattgcgcttttcttgaaggtccgttactttttgaccagcttcaagccaagcatcgtgcagcttatttaaatccataatttaatttccttctttcttaaataaaatagccaacttatgtgatcgtaattggtcactagtttggctattagtttctttaggcttttcttttactttggttaacaatgatttaattttactaattgcctgattactcaacatcaagggcgacatcatgttagtaactttggctggttgatctgcaaacatcatttcgtctgcaaatccttgttcaacggcatcttttgcattgatataagtttccttggccatcatttgcatgactgtttgcggatccaaacccgttcgttgcacataaacatttgcaattgattgatcagtcgagttcaacccctgcaaatcgctggataaatcatctgcattcccttgagatacagtggaagcccgatgaatcattaattgagccgttggcgaaattttaatcgtatcaccagccattgcaatgacactggccgcactcgctgctaatccaacaatgtcaacttccacattaccggtataattcttaagtgcggtatatatttcagaacccgcaaacacatcgccaccaggtgaattaatttcggcaacaatattttgaccatttgcagtgcttaacgcatctttaactgcggaaggagtaactgttgaatagccaaagaattcatatacttcagcatcatcatcactagatacaacacctttaattggtactgttgtcattatcatcacctccttccactgctgaaactttcaaatcaggaaaaactcccgcttgtttcagaattgtttgcgcttgttgcgacgttaatgctggtgactgaccagtacttaatttagtaatattactaattaattgctgatgatcaacatcaatagccgaattaatatccattttaatgtcgattcccaactttaaagacaattctgattcaattggccgaatatataggctcaaactattttgatacaaagaacgaatcatctcaattgatgattgttcgtcaccttgaccatttaaataactatctggaacacaaaaagccttggcaatctgggtctgactaaacgtggcattatttaataatttagctatatccggattaatctgtaaggaatcaagctgagcagattgatccaaaacaattggtcgaccagcattcgaaccagaattctgattctcaaacgattttctaatattttctttagcttccggttccaatttggccgccggaaccgtaatcgtataactaggcgcaattgcattctttaaactgctcagtgacaattgattactatagttctggatgttaatttctttagctaaactgtttagcggactgctacccactagttcagtggcaacttgcccagaaacaaacaagcgaaaatgtaaaatatcggcagctaaatatgtcacctgccctcggtcatcaccgtaattaactgtgtaataaagaacattttgttgattatctaaagtaatgctgacctggtaaaacgggattaaggtcaaccctgctggacttccattgccatttcgctgaattagaacaaaggcgttgccagttaacatcatttgagcactaactgcttgccaaaaattataagcactcaataatgtgctgggctgatttagcatgttgctatattggtctgttttaaattcacagctggccacatcacctgcaattcgattaatcaccgcataaatatcactgttttgcagtgctccgtctgcatccacagtgttagtggataacaatgtaccatttaacataaatggtgaatacccggtggtactaattgtttgtgtttgttttgacataaaatttttaaaggggttcagcattcaacgcctcctttcacgaaatgacataggctaaaacgattaaagcaatcccggccactacccaacctacaataaaattaataaggcttgcggcaaccacaaatgcaattaacccaaataaaaataatataaaagacaggttagtgaataaacctatccatagttgtttcagattcaactaatctgcctccctaataatttattcactacatatatcacccaacaagtgttgaaaatattaaaaactaaaatgatcactggtaaagaattcgttgacctcctcattactcattccattaaatggattctttttatcttctttaaggccatgattaggattttcaaaataaaaaagggcttgagacatggcatcgatagtggcatcggcacaatcaattttcgaagtcaacgccgttcgatcaattttaataccatatggattagccactgttacagcgttagccaaacaggtctgcaaaatcggatcagccaacatctcaatatttcccgcaataaactgatttctcaaaaatactgtgggcgagctcaaactaaccgtcccttgctttaaagtaataaaaggcacttctggcatattattatccaaccaatcagtaattgcgctagcttgataaggatcataaataaacgctttgactctcaaatgatgatcgttaacaaaatccaggaaccagcgcccaacaaaatcttcatcaattaagccataagaattttgcgaaatatcacaaaagcctagcttttctgcgtttgagtaattaattccatcttgttttcctttcacaataatggaattatctgctcgggctaacggaacaaatgaatgctgcaagatgaaatatttcttttgttcgccattcaaatgtgggaaaacaaaactataagccgtatcatctgaagcatgtgataaatcaaaacccacatagcaatcttgattatcaatttcgaaatcagaaacaactgacttttgtatatcctctaatttcaaatatttatctttagcagtctgcaaccacatattgaggttacggttaatgaaatcatttagcgtaccgtcttccagcttagaatcacgttcactaattaaccctttcagtagggtatcatgcttagccggtaaatctagtaatggattgcttttcacccatgtttctggattctcaacttcatcttgatcatcctgctgccaaattaatgccaacgttgaatcttccgttcggttagaatctttttccatcaccttagtaagtcgtctaacatcactatacatcgggactttagggttactgtatgccgtactgataaaaaatgtttgccggttactagtttgaacttgtccagacgtgactttagaaatcacatccgaattaaaattttcatccccgtattcatccacagtggcaaagagaaaatgaaaggcatctaattgtgcactaccagctgtcattcttaatatctggttttgagtcttcgtggactttaaaacatcatcattaatagcaatattttgatccttgatcaatttacgaaagccaggcattgactgtaaactattaaaagtctgtttaatgtaacgccaagacttcttagactgcttatcaaccggcgccaagtaacacaaatcagcgttaaactggtcactagcctcgaccaagtaagcgtaaagtatcaagatattcaataaatatgacttgccattagtccgagccactgaaaccatacatcgctcaaatcgcttttgcttgtcttcctttgttcgccatccctgagaaaggcacaagattgcttgttgccaaatcatcaatggtatcggcttgttttgagaaacatcagggcacatgcgtgcgaagttacagatatttcggcatttatccaaatcatagtaatacggaaaattaccttccgtggatcgctttaaatcatttaaatgtctaaacgctgctagtttaattgttttgcaggctaactgttgaccagttaatacccggtaacaataaacagtggccggatcacggtatttccttttaatttcatcaaaataaccttcaccatcaagtcgctgaaagattttatccaagtcaatatttctttgagtaaaatcaaattcctgtaccactaaaactcacttcccccatttaacatctctttaatattgggttcctcatcgttgtcatctgagagttgcagtaatgaggctcgtgcagatggtgttaagcctaattcgtgtgctaagctgtttaattttgccgtagcagaatcaataatttgtgatgccggattacgtttccagcctgcgttgtcttcatatgtttctccagttcgttgattgaccacagttttagaaactttggtgacaacaccatctgttttaattgagtcatagcctttccgcaataattgatagttaatacaaaacgcttcaattgttcccttgtcggcctgtttaacatatcctgatgcttgcaaaattggtacaagtttcgtccacattgctcgcgcataacttgacagatattttggacaactcttttgaatcaaatccattccagaagtttccgttattagtttttgagttctaactcgctgatccttgcgagcatgcttgtctgtagttagtttcatttgttttggcattttttagttcacctccaagcaataaaaaagagcccccaatagggactctttcaatctgattcatttagactaatgaatcacaaaaaaatcattaaacacactgttcgaacgtatacaccctacaatcgtgaaaaaacgtctaattatattaacttttaggaggtaaatatacatagtcattatagtagggttattcatataagcaatttgtgaaattgcgtgcacccagttatagtaagcccataaaaaagttttgaatttacaacttttaacgtgcgctactgctgggcgtgcgctcccctaggctttcaccaccccgggggtgtttaaacattcacctaaattgtatatttttttgtaaggttcaaacagtaagctttaaacaattttttctttatatctatatcacccagaggaggttgaaaaaattgtttttaataagtaaacctcatcagaaatatttattccgattacctacatgataccacctgaaaaacactttgtcgtttcacaaagacatcttttttaattttgttgatgaagatccccaccatccaagctggcaggagtttcctacatcagggatgtttatttcgtgcgttcagataatactttaatccaccaacgtttgctgcagtgtttgagttggttttgattgagtgattgttcaatcttggttttggtattatgcgtagttggtgacaagcaccataagttatccatgtctaaccatttatcaacagatagtacacgtctaggcacaatgtggtcaacaataatcttatcgtttgagactggcaagccagtgactgcatctaaataataatctcgtgcagcaacaaattgccgaatctttttccattcctttgagtgataaaacttattcgctgtttgatcacgatagtacatattgtactctcggtttcgtgcagaactgactgcatggttgggcttctggtgctgtgtaacgtgctcactgcaatacctttgccccattggtatcaatgcttgacagccaacctcatgacagatatgtagcttcatataagctcacctgtccttctttcggtacgaactgtttacttaattcctgctgtaaatcaatgattgaatcaattaatttgtattcatccagtttcaattgatgatcattaattaaaccaaacgatttccaaacaatgccttggtatttcattccatatactttagttgcgtaatcgaatatatcattgaacaagtcgctattgctgataaataaggtgtgaacttcgctgtttaatgtcattggatcagcgtatttattaaggcaatattcaaaatcgcctaatacctttagcttatctaacgtatcctgatgatcgaaaccacttaactgctccgtaaacatttggacatttgatttaacgtaagctatacgatcatacaatgcatgttcaaactttttatcagtcattgaaaaaatatccattgtagctatttttccatatttaagcaggctttttacaaacagtttggttttatccgtcgggaataatgaaataaccttattcactaatgaattctcaactgacactgaatttttacaatttataggcgccaattgtccaagttcatcagatttatcaaaattctctaccaataacgtcttgtgaccataataatcttcaaccacatctttagcagcataggtaattgcccattgcttattcttaaaatctggattgctatgatcgctgaatgccttaatcaaggtattagcattgttataattccaaaaatgaattcgtcttaatacttgctcaattaatagactaaaagcgtcgctttttgaacaatgaattgaataatgaatccggttaatgccgttttcaaaattccggctctcagtaattgcttttactaagttttcatttcccattttttcaccgcctttaaacttggtttacttacagctagacattgacgataaggagaaactaattattaacggatttctttgcgtttatttcagaaattgtccatccacagatggtttgatgatgctgaacagatttttcaaccatccaggttttgattggcaaaccggtttctgctttcaaaactgcttgaatgctgcgaaactctttcagtttatgaactttcccttgctttgttatcacatacgtcatataaatttcctcttctaatcacataattttacatatacttattgtgcacatttaacagctaattggcaagctttcataagtcttctgtaaagtgttaaattggccgtcactggcaccgcgtaaataatcctcgttgttgctttaataccatcttgatcggaaccggctaaatagcttccgtctttaaactgaaatacctgatagctgatttcagctactttaattttcatttgtttacctcccgagattcaagaaggcgtagaattccagtaatggcactcaagccattcttggtaaaccgcatttgaataaccttatctttcttgcgaggatacttttgattcataataaaggtaaaggtaccatctgaatttggctgaattccaaaagtgctttcaataatccctttttctgacattgcttcatattcaaactggctcatttatctacctccattttgactttaactgcgtccttccaatttttaacggtctcgtcgaggccttttttggttaggttaaactcgccattttcagcaaccaacgtaaaataatcttcttggatgtaaactgggtattcctcgcctaccttaaaaacacgatgctcagctacaaaagtatacttcggaacgaaataacaatagatcttcatttgtctgcctccaataattccggattatcgtgaacattgccaatgacttcaatgatattagcatctttacggcaagcacaatccagccattctggtgaactataggacttatcgctctcttgtaccgcaaatccagctccgcgatacagaactactcctacccaatcatgctttctataaacgtttgaatgccaagctagaatatccccttcgtagatttccttgccattggcatctttcaggccggtatattgctcaagaacatcatcagggttatccagctgaaagatatcagacatagagtagttcataaggctatcccatgattccatccagaatgttttgctatactcatcgggtgctctccaaatacggaatttaatttctctgctcattaccgtcactcctccacactttgaatgcttgaattatttaacaaatccttcagaaattcagcttcatcacgtgtaaattgctgcgtaattgcgcctcgatcaacgcgcgggttacgaactccacagatgaaatagccaccacgatcatctactcgtcgagatacatactgttgcccatcactaccaaccatgccattcattttcaagcgatacattggtgcagacaatttcactgtttcatgatttaaaattgcatctataacactagctaaatcatcacggttagaaatagtttcatcatcggcatatttatcaatgaatttggcgaatttagctattcgcttccaatcagaaatactttctcccattacgcattggtacattttgaacaattccctatcaacaatttttactgtcattttatttacctccaataatttttaatgcgtcatctactgatcgagctaccccatataacactggatattgcttaataaactgtgcaaaccgcttctgatcatcacgtaacttgcctcgttcgtttttaacttcaatcaaaatcatttttccgctatgatgttcaaaaccggtaatatccggccaacctctcggaaataacataattcgtctgccatcatcagttttaatttttccagcgttactacggcaaacagtacaatcatgtcgcgataatgccaaaagaatttctgtttgaatttcatgttccgatttaatctttacacgcctccaaataattatgacggatatgacggataacatgacggatgattaagctgctgtattccttgtcactctaagaacaaactacattttttgctaatatgacggatcttttcaacaaacctttatttatatatcttttttactcttttatcttatatacttttattaatttatccgtcatatagataataaagagtaataatactaatggtaccaagggattgagcgatttttttatccgtcatttatccgtcatttatccgtcattttatttaacccaattcaatctaggatccgtttttatctttattccttcgtaaaagcgtcccgtcatagttttcttaaattcaaatttctgcttcatctcacggctaaacttctgtttactcatagaatattccgaattatcttttgcccaggattgatatttcttaaaaagttcacctgcaggcgctcggtaactatcacttacctcacagcaatcatccacgaatagactaataacatccatttcttcacgatattgccgactagcacgagtaacacttattggtggattcaagccttcacgttgccataataagcaaccctcaacgatccaattaaggattcccacggattcgcgttttaatttatcctttaggtttttatcaacttggccatcgggaatttttaccttaaaaggaattaacatcaatcgtcgccaaattccgtcatcagtaccacgaatgattggtttatggttagtggctaaccacagcttaaactgtggtttgaattcaaattccttaccatataagtaccgtgcggttactttatcgccaccggttaattgtttaaccaatccctcgtccaatctcacaccctcattaggttcgcttgacgtaactaatcgggcactttccaaacgagcaatatctgagttggctcccgatttattttgccgtaccataattgaatcggcttgcattgacttggcataggttcccagaatatcagaaatcgtatcgatgaaaattgatttaccattgcgaccatttccatacagaataaacatcacttgttccttgatacttcccgtggcagagtatccaaccgctttttgaatgtaatggattaattcctgatcaccagcaaaaatttgatttaaaaattcatcccattctggacaatcgattttgtcggtgtattccacacttgtctgatgactgaacattttcttaatgtcgtggtcttttaagatacccgaagttaaatcaatatagccattaaccgtattcaataaagttttatcttgatcaaactgcccatgtaataccggaacccgatgttgtacttcgcttatcatggcttgtttagcagcatgactacgagacttcttcaaaaacttttcccaagctactttagccttttcaggatccacgccggcagcaacatgcaacttctcattcttcatattatccacagtcatatcaacgaattgagctgcttttccctgatcgtccatttcccaataactgccattatagaaataccaggacttatcaacataggaatatttaactaaatttccaaaaacatcaataaatcgatcagcattcccagtgtcatcccaacttctaggtggtaatttctttttaggcttagattgtaggaatttaagattatatttatgcaagggatgctgctgtggattaaaggtttcccgtgtttcgttgatagatttgttaagaagtgaaactccataagtggttttcccatgtttttcatcatatttcggtcgcataaggctagactttcgaaatatttcatccattttattaaaatcacggcccgtccaaaaggccaagtcattggaaaaggctagatcagcttctgaatgggaagtatagaagccctcccaaccaccgtgcataaacatcttgaaacgtttaccagtccgtgaaagttccgcgcgtttaataatttcatcaacacttaaatcatttggcctgattggtgcctgattgggaagctttaccacattactttcaccaaaataatgtttataaataagtttcatcacttcggaattaggtgtatttatccgatcactgtatggaccaatagtttttccagttaacgcgaagaatcgtccggactcatacatctcaacgttgcctttgcgacgtcgatcaccaggaattttgcccttaaaaatggcatgaattcctttaccggataaactaatctccacataggatttagtcatcgtcaacacatcttgaacttcattttgttgataatcctgtgcagcgtatttctccaactcatccccaatgtgatcaatatccaacccaacataaccattagcaaagtaaaacgcgagaccgtccattttatacgtttggagtgcttttaaggctgtttgataatcagtccaggtacttgggtcattcgtgcgtccagccccaccatcgagcgcattgtggggtattttggtgtacttatttcgctcaggttgccagattttctgaaacagtccccattgttttaaggcccgtaattcatttggaatgttttcatatgccactgtttaccctcctagaacggtaaatcatcgtctgaaatatcaattgaatctccagaattgtcaaatggattatctgttggggctgatgctggttgattaccagtaaatgggtttttaccgtccttttggtctttccatacatgctgcacttgtggataatcgctcttgctaaaattccaaggggcaatctgattgatgtctttcttttcaccgccataatcatcaaccgtttttttgacatacactttggctggcttgttagcaactgctttagtaaaatcattaattgtattcaatagtgttccttctggaatttgaacagcttcaagaatgtattggaaactatcaaaatcgtactgattagtagttttgcgtttccaattgtccataaagacatgacggttatggtacttggcattggtattttttaatccagtaaccccatctaagtcatttcgaaccactaaatccaattgcagtgattctgccccgttcttagttgccttctcctgagctgacttaataatcatctcgtaatttccacttggtaaagctgaaaaatctttgtgttcattgttcttgtaatttgcttgcataaatgccatttttaaaattcctccattagttaaccatttttagtcgtttagcttgtacataggcccaaccagctttatatccacgggctttagcgatttctagtaactctttgtaactttgtgcatcttccggcttttttcttgccgtctggatttttgaataatcagtagtcagtttaaattccccaattttttcaatactggccgtttcatcaatttccattccgtcagcgtcatatttaatctcattaccacactgtgggcaaacacggcattgtgtcggtaccacagcaaaacaatttggacaagttttgaccggaattgattttgtgttattctgccgttttttcttaggtcgtccttcaaggctccattgtcgtggagtatcaggcagaccaaaacgggtatagttagctgcatgatcaatgatagtggccattttatttggcaaatatcgcatacaacgcattgttgcttgaatatcaaataccaagctttcagttggccgtgcgattacacaacacgtacactctttgacgtcatatccttcatcaaccaatccaaagttacataaaacagtgatctttccctttctaaaatcactcataatacgttttctttcgtcactaggagttttagaatcacaatgttttgcactgatacccgcttttctaaattcagccgcaatttgtttgctatgttgagtatcatgagcataaacaatggttcgctgtccaaatgctttatccatccaagttttaacaatatcgccatacagagtgggctttgctgaatcactaacagattgattggtataatcgccagtgctcgatttctttagcttttcgtcattaaacaatgtcacactgtagtatttatatgggcttagctttttgtgttcaattaaccacttaaccgtggggcctttgaccatagcagaataaatatcgtcaaaccctgctccgttcattcgccacggactgcctgagaatccaagcctaggaacatccgaatagtatttaaaaatttttaaatatgtttttgcccgactatgttgcgattcatcgcaaataattaagtttggtttaggcaagtgatctaatcgattagcaactttgcccactgtcatgattgtgcaattcatcaaatcaacatcttgcttttgaaatgattttacgatctggttaactaattcttgacggtgaacgaagaacaaaattctaccaccctttgaaactgttaatctcgcaatttcagctataataactgatttcccactacctggtggggaaacaattagtaccccattattgccttggccaattttttggcgagtttcatccacaattcgttgttgataatcaaataatttaaatggcatttttttgacaccggatttctgcaaggtgacgttcttttactgcttcctcatagcttgtaaatgacctatccaatatgattcggtttcgatacatcattttagcgacccatttatttttgcttttatcaaaagaaacaccacgtacaccgctgatattgtctgcccgcaatctattagtcactggagagtttcgtttacgcctattgttggcctgggttttccaatcagtccaacggcaattagatgggcaataattaccatctacatcaattcgatcaatggattttccactttcatatccattttgaatagaccatctttcaaaagcataaaaactatttttccattgattacagatagatacacctcgaccaccataatcggaaaagcttttattattcgggttgaaacatctttgcttcatagactcccaaacaaaataaagtttcgtatttgaatgaccgtgttttctaaaccttttactagcgagttcatcgtgtagacaaccacaagattgtattttcccctttcgaacatcgattcctgaagcataagtgacatttccgcagtcacatttaaatctccaataagcacgggtagatcctttaggacgttgagaattatcaatgcaaactgctgtcagccttccgaatttcttacccgtaatatcaattagttttgtcatcgttgccactcccaaacttaaacagatccttagcagcacacatggttcgattgtccaaacgatttttggcataaatcgagtcatttccttgcagcataacgccacgaccgttagtcttcggattaataatcaaccgaccaaccacatcacataatcccagcattccatccatcacgctttgacgaatttcgggtgcatattgattaaattgctgaccattttcagtagtaatttggcgttgtgtctcccaagctgtggttagcacattaactggcaacgcatagatagcagtcatcactctagaaaaataattagtccactgtgaataatcctgcaattcatttgagatgccgttatggctacccttacccttttccacaaaccaatctttttcaaagcttgacacattatcaataactaaattgtcgtaaccaacaatcaattctgatgcctgttcaagatactgcttcatgtcttcttcggggtgagttcgatccatttcatcgactgtaacgttgctaatgccagctaatactttagcggagttatccaaatcaaaaattctagttttaccaggtaaatatttaacacaagttgttttcccagttccgggtttagcatatagaatgactcgccaattcaaggttcgctgtaaatctttagcttcaatcgtcttcatgattaagcacccactctttgataacgaatttggttactatccatgaaagccctcaacagtttcatttgtggaattgttgccgttatttttaaagacactgaatgggaaacaacttcgccagtattagtatcaatcgttttatctttctgctgaatttgatgtgtttgtgcttccgctgcttgtgcttccagagtctgctgtttttgtttatttagtttgacctgattatcaattgcttgaagcaaataattaacatcttggccttgcttcaactggtcgatccaaccagctggatcaatgtgataagcttgagcatatttggtaatagtactgataccggtttttaaatcatcatgttgctttttaatgtaacccatcacatcagcaattccttcggttactttcttcttggtggtggttttatttaaccaagtaggatcaatttcaacctcacctggttccacatggtaattaggtgccatttcagcaatcagagattgaacatgttttaagcgaagctggcgttgctgatcttccaattcctttagcccagcatcgattggattaattgatgaatctaaagtggcttctaagtctttaatttgagctgcaaaccgctgatatggttcagcatatttttttctaatttccttacgtttatcatcaagagcttgcttcaatttccgaagctctgcccggctagactttgattctttttctgtggaagttgttactgccattccttgatatttattggcatatgcttctacagctgtttttaattgatcaaaattattaattgtaataacggttggccgatagtcaatcgtgtattctggtagggataattcatttgccatttatatttacctccatcttttaatgtaaatagtgtcgttgatcaattgaattcttcatttctgcaatctctttgcttttagattttgtgattctgccacagattaatctaattggttcgggataaattgggactcgttctttccgcttcttcataaaatccttgtcggtcccagttacgacgtaagtcggatactttatgctgagctttcgcataacgtcggcacgagagacaccagtttctaatatttgggaatccattacaccaactgctttccaaaatttagtcattattccacctcgtgatgtaaaatatattcagatagtcgttgcttttctttatctaggacaaagaaatatgccaacaagctatgatcgttttccacgggtgtgcgcccaataatcatattcaaacgtttgatacggttctgtattgttaatgttttcattctgatgaccctccaggtgttataatattagtagttatagttgttagctggtccacccatttgcggtagtgggctatttagtgcatataattaaggtggtgaattcttatggatttttacaattggttaatgcgctttaaagacgttagcttaccagttggtgatgtagcaagagaaataagatctgatagatcgtttcctaagggaaatttagattggaaacatttaaaagaatatcttaagtcaattggtttttcagattccaaattagaaattgttaaaaacgtcttcaactattatttagcggagaaaagtcgctaattaataaaatccagtaatcatttggaagcttcatattttcttggccatatttgcctcgtatttcagtattggcataaaggccaccatggaacagttgggcttcctttctttttcttaattcacctattaattcagatgtcgaatacttttgcaatttattcatcgatatgattcctttctattttttagtgacgcccagttggtataaagtattcaatgaccagggctgctaagaacaataaaactagtacttccaatgattccattaatcaaatcactcctttttaatatttgtagaattttgaattcaacccattaaggaggctaagtcgtatgattcatcaaattgttgctattcgattacgaacttattccaagggaaagcaagcatcaccagaaaatattgatttaataaaacaggccagtgggaaaattgaacttattcaagccacagcagccaatattattcgtggtgatcactacttttacattctcggtaatggtacctatgaaatcacttatgattacaatcatgacaatgctttatatattaaaaccaagaattcctcaaatcgtcacgatcgattattagatttgccaagaatttaatgtttttaccaattgaattcactccaatgatcctccaggaactgctgcattttggtagctttaaacaaccagggactacctttactgccacgatggactaaatatctatcatccattaaggcttgcatttcccgtgaatattttggattttccaagaaattttcttttaaccattgtggtgatttgttcccacaccatttacgaagatcgtttaaattccaagtccgtccaaaggttgattcccgttttaatttttggtaatcttccttatttatcaattcaaaattatcaggaatttgaattgatactttagcactaatgacttgagacattttgtcacttcctttagttgtataatttatttatcccaattaatcgagatgataaatatgaatttaaaacaagcagccctatttgaatatagctttgaatatttcttgagtaagattcacaatgcagaagccaaaaaatgtatatgggaatttaatgggcagttattgaccgctacttttcacgacagtactctatttagtggagatgaatttagcaagcaacttttcaacgaccgattgaaagaagatgctctaaagctcaatacttctcatggagattcacttggtaaatttcaaagaaattttccgttattaattaacgcgttatcaacgttcgttgtcgatcttgataattctcaatatactttgactgatttttttctggctaaaaacgtttcatttcttgggaaaaacatagataacttagatttttatcttttccctaaagatgcagattttaagattgtatcaatcacttcatccgaaactcgggattaaagtgcttgatatgattcagcacatctcctagctcagcacttagctgctgagctttttttatttctgaaagaagaatacttccattctccaagatgagagaaatatttgtgctttttgcctgatctaataaatcaatttgttttaattcaaaactggtgttcttatcgatcatctttctcacttccttttgataagatctgacgtggattaattaatcgtcgtttttgttgtcttcaatttctacattcttcactccataagcgataaacttattaactaccgctgtgacagttaatccagtttcgtgcttaatgtccattaactggttatacaaatcagtgttaatgctaatcaatcgtgatactcgtggttctggtgctttcttttctaaaactaaacgtggttttgccattttttattacttccttctattatttactgacgtataatttaattaattcaagtaatcgaggtgaaaattgtgacttataaacgtgctgaaaaagttttgaagaaactactatcattctcaaaagaaccgaatttagcgtttgaattcaatcaaataattaaagactctttaaaacgtatttctggcgataaattggagaccgacttagattttttaaccaaagaaggtttaattggatccattagtattaactcctatcaggcaatttatgttacaagccacggttacacttactttgatgaaaagcacagtctggataaaggagttcacctgacagaattaagagttcatgtgctttatccatctatagttgcgttcataacattttggcttggcttctttctaggacatatgaccaagtaagtaaccaattgtcataaatagaactcctatcgccatatttaaaataggctgaatattactatcaaagtactgatgcagttttcctttttccatttaactcacctcatttctatgctggctgtgtggacgaatccggagtaaataaaaggttgatcgtcactctgaaaagctaattcaagatcagtcacgttcagtgtcttttaggacactagttcagcaaaaaaaatatccattacgtcttcggaatttaaatctaatactttagaaagagccattatctcatctgctttaaatgggcgaatatctcttaagcctttatagaaagtggaattagacattgaaactcccatattgtttacagatttaataacatccgaaactctctttcctttgagcttaatggcagccaatagtttatctttattcatgtaatcatctccttcgtttcctttaggacacttttaattaaaacacctgtcattttctttgtcaatagaaaaatgtctttatttgcatttaatatgcgtaaaaaaatattatgtgtattttaagacacttttgtgatactattattgtataggagtgatgaactttgtctattaatttaagaaatagaagaaaagaattaaatttaacattggaagaagttggaaaaatggttggtgttggtaaatcaactattagaaaatgggaaactggatatatcgagaacatgaaaagagataaaattattgcactctcaaaagcacttaaagtaagtccaatggatataattgatcccaataaagaaatttcgaatcccatgattgataaaattgaagaaatatcaattcagctccacccttctcgtcaagaaaaagtttacaattatgccagtgaccaattagacgaacagaataacgaaaaagtaacttcaatgtttaaccacaaaccgctggttgatattccttacggtcgttcaactgctgccgggtctcctatcaatggtgaggatcaagatacccaattaatccacaaacttattgctggtgaaaaagttcctgccggtgcagatgaattaattactgtggatggtgattcaatggaaccgctcttaaaaaagggtagtcaagtttttatccactaccagccagaggttgagaatggtgaaattgcgatcgtccacattcgtgatgttggtgttacttgtaaaaagttttatgtaaatgaggataataccgttaccttaaaatcaatcaatgaagcgtatgatgatatggtgtttgattgtgatgaagttaatgtaatcggtaaagtgatcttatgagctcccaaatgtgggggcttcatttaaagttttaaaagaacatatgtttcgactaaccaggtggtttgcttaggttcgagtcctaaatagtcaatatttgaccgaaaaaaataaccaacgttctctggataaacgttggccacaggaaagaatcgatcgtgaagcagctaatatgtattacaaatttttggtaaatatccacgataggatcatcagtaattttaagggacttgctaagcatgatcctaataagtggcgacactttatttcagttaacgaaatgctaatacacaagctttgcagcaaacaataattatacacagtaaactttttcagattccggctcagagtactgtttgcttttcgagttcatacaaaaagagctctaatcaccaagtgattagaactccaatattttgttcaccaacaacagttgacgaagagccaaattaatttccgaagcttttttgcgtgagttgggacttttgtcccagccacttgagtatgttcacgtgtctactgcttaccttataaaacacgcttgtaactatacaacttaaccattagttaaaatggtgtatatgaaccactgttggcaattgttgggaaaccaatttcagtaggattggtttggttataattatagtatacacttgccggggtatcttggccaaaatgacctgctaaagcagtttgagcggtgtaagtgaactgattccaatgatcaatagtaccattcatattaaacactggataagctggtgatttcaatgttgaaagttgattatgtttttgaacataagtcataacatcatttgcactaaatgcagaattcttaggtccgttaaacaaatcacttgcagataagtttgcaggggcaacatataatgtttctgctttagctttaacggcagcatttacagcgtctaacttagtctgatcaccatttacagcattcttaacaacgttttgaagaccagtatcagcagttgtaccggctgcaccagttgttgcatcaacatcgtttgtaatcaaaggattagtcaaagtaacacccttgatatcgctattcgtaaacgtagcatttaatacaccatttgaagtcttgttgttagatacattaggagcgatttcttgtgcatcagcgggactctgtgtactagtgtataactgtggtgctaatctctgatatacagtttcacccttagcaagaggaatattcactgttgaaccagtagtagtttgggcaactaatgcttgattagaagtattagttgtgatgtcaaagctataaccagtaccgcctaagagagcatcaatcttactctgcaaatcagtgatggtgtttttatcaagtgtccaactataaccacttgcagtttgagttaattgaccaaacacatcaccttttttagcatttgacttagtataatcaagtgacttgatagtctttccacttgcatcaacaaagttcaaacgaattgcattgtcagcaaccggagtagtcacgggtgtaggtgtttggttttgagcagttaatgctgaatacttaatccagccgttaatcttttgaccattagtagcgttagtgtcagcaatctttacccaaaggtcgccttcacgggtacgggtcgtttggtccgtaactttgaaggtatcgttagcgtaaggagtagcatcagtaacggtacggcccttacggtactcagtccaagctgggtaagtgtaagtggtggcagtgccatcatttgcagtaccggctttggtgatcttgtaggtagcattcttttgagcgtcagtcaatgcagtggtttggccctgagtattgattgaagctgaagatgctgaagatgaagtgtttgcagctgctgcaggtgctgtagtagtgctgaatgaagcaataccaccagcaaatgcagtaactgacttgccgccgtagatccagccacggtaagtcttatcgaatgaaacaaccttgtagtaaactgagccacggttagtagtagctacacgataagcacggaagttcttttgaccttgcttagagttcttaagaccagctaatgtagtcttagttgcaacggtcttagcacccttcaaagtaccagcctttgtataaagagcgttagtaccgttaacagcaacgttacgagtagtagcatcagttgtcaaagctttgtttgatgtaactttggcatatgattttgcactagcatttgagctagatacaccggcaacagctacaaatgataatgcagctacaccagcaaaaagagtctttttcaatgactttttcatgtgtaatttcctcccaaaaaaattgttttttcaagctacctaggcatgcaaaaacatgcctcaactaacttgctgtaaatagtataacataatcaaggttgaatgcaaaagaaaaaaggagttgtaaaggctttaacatttttctgtaatctatatgccatgatcattgataaatgatcgatctattaaggggattccctccactatgtgttagtatattatccaaaggagggtaataatgccatcaatacgtaaacatggtcatggataccaggtaagatactactattatgatgccaatggtcaggaacacgagaaaacaaagagcggctttagaactaaatcagctgcaaaactatttgcgagtcaattggaaatcgatatccacaatggtttggatctcgttcctaaagatcctaagtttgctgactattttgactatttttatcacacgtacaaagagcctaagattgaaaatcagactaagaatcgctataaaataactagtcgagtattacataattatttcggtgatgttactttaaaaagtattgaccgaccacaatatcaagcatttattaatttctatggtcattctcatgcaaaagatactgtttataaagttaattcactgattagagcaactgttcaaaatgccattcttgacgatctgattcataaagatttcacccagcgagtcagtcttatttatgataagtcacgtgataagcatgtggaatacctcaacgtggctgagattaagcgtctcatcgcttatttggagaatcacttaaactatcactttacctccacctttatgatcctgacggccgttttaactggtgctcgcttgggagaaattcaagcattaacttggaatgacgttaattttaattttaaaacgattagcattactaaatcttggaattcatccgaaggcggtggattcaaagatactaagacggctggttcaaatcgaatcattgcagttaatgacgaattgctgaaatcattaaagatcttgaaggatcacaataatggagaactaatttttgttaatcaatataaatccattccatcatcctctgccgtgaataaaaagttgcgttctatactaaaagacttagggattcaaaaacagggcttccactttcattctttacgacactcacatgtagcttacctactatctcgaggaattgacatttacatcatttctaagcgtttaggccatgctgacgtatccacaacaacaaagatttattcctatttaatggatgaatataaggccaaaaacgatcagcagattcgtgaagagttagataatctttcctctcatgatgaaactataccaattgagcggaacctttaatgaggttccgtttttattttgttattttactctgtatcaggttaaacttcttctgcccgtttggccgttatttgcccgttattatttatattttaatactttctagtacgtttttataaattaaaaaaattaggaatgcctatttaacagcattcctaattttaatatttcttctaatttgtataattatgccgactgcaggagtcgaacctgtgaccctcggtttacgataccgatgctctaccaactgagctaagtcggcaaatccattgtacaaaaaatgctaacaattaagttagcatttcgacaaagctccggcaggcgggctcgaaccgtcgacaacctgattaacagtcaggtgctctaccaactgagctatgccggaataatcgcgtggcaacgtcctaccctcgcagggggcgatcccccaactactcttggcgtgcagaagcttaacttctgtgttcggcatgggaacaggtgtatccttctggctatcgccaccacactattttccttgaaagaacttcgttctctcaaaactagctaatattaattttctgcccttgaacaccatttctacttggttaagtcctcgaccgattagtattggtccgctccgtacatcactgcacttccacttccaacctatctacctgatcatctctcaggggtcttacttccatataggaatgggaaatctcatcttgaggtaagtttcacacttagatgctttcagcgtttatctcatccatacgtagctacccagcggtgcgcctggcggcgcaactggtacaccagcggtatgtccatcccggtcctctcgtactaaggacagctcctctcaaatttcctacgcccgcgacggatagggaccgaactgtctcacgacgttctgaacccagctcgcgtaccgctttaatgggcgaacagcccaacccttgggaccgactacagccccaggatgcgatgagccgacatcgaggtgccaaacctccccgtcgatgtggactcttgggggagataagcctgttatccccagggtagcttttatccgttgagcgatggcccttccatacggtaccaccggatcactaagcccgactttcgtccctgctcgacctgtctgtctcgcagtcaagctcccttctgcctttacactcgttgaatgatttccaaccattctgagggaacctttgggcgcctccgttactgtttgggaggcgaccgccccagtcaaactgcctacctgacactgtctcccgccacgctaagtggcgcgggttagagtgttcacacagcgagggtagtatcccaccaacgcctctgccgaaactagcgttccggcttcaatggctcctacctatcctgtacaagctgtgtcaacacccaatatcaagctacagtaaagctccatggggtctttccgtcctgtcgcgggtaacctgcttcttcacaggtatcttaatttcaccgagtctctcgttgagacagtgcccagatcgttacgcctttcgtgcgggtcggaacttacccgacaaggaatttcgctaccttaggaccgttatagttacggccgccgtttactggggcttcatttctgggcttcgccgaagctaactcatccacttaaccttccagcaccgggcaggcgtcagcccctatacgtcatcttacgattttgcagaaacctgtgtttttgataaacagtcgcctgggccttttcactgcggctgtgcttgcgcacagcaccccttctcccgaagttacggggtcattttgccgagttccttaacgagagttcactcgctcacctgaggattctctcctcgactacctgtgtcggtttgcggtacgggtagttgatgactcactagaagcttttctcggcagtgtgacgttggttgcttccctacttaaatttcggtcctcatcaccacttgtcaacccgccaaaaagcatttgactctttgactgacttgtggcttgaacatccctttccaactggatgcacaacttagcctcctgcgtccctccatcgctcaaacatcatcaactagtacaggaatctcaacctgttatccatcgcctacgcctttcggcctcggcttaggtcccgactaaccctgggaggacgagccttccccaggaaaccttagtcattcggtggatcagattctcactgatctttcgctactcataccggcattctcacttctaagcgctccaccagtccttacggtctagcttcattgcccttagaacgctctcctatcacttgaccaaaggtcaagtccacagtctcggtaatatgcttagccccggtaaattttcggcgcggaatcactcgactagtgagctattacgcactctttaaatgatggctgcttctgagccaacatcctagttgtctatgcaactccacatccttttccacttagcatatatttagggaccttaactggtggtctgggctgttccccttttgacgatggatcttatcactcaccgtctgactcccggataaaaatcaatggtattcggagtttatctgaacttagtaacccatgacgggcccctcatccaaacagtggctctacctccatgattctacgtccgaggctagccctaaagctatttcggagagaaccagctatctccaagttcgtttggaatttcaccgctacccacacctcatcccagcacttttcaacgtacacgggttcgggcctccagtgcgttttaccgcaccttcaccctggacatgggtagatcacctggtttcgggtctacagcaacatactaaaacgcccatttcagactcgctttcgctgcggctccggcttttaaaccttaacctggcatgttaccgtaactcgccggttcattctacaagaggcacgctatcacccattaacgggctctaactgcttgtaggcacatggtttcaggaactatttcactccccttccggggtgcttttcacctttccctcacggtactggttcactatcggtcactagagagtatttagccttgggagatggtcctcccggattccgacgacgtttcacgtgtgtcgccgtactcaggatcctgaactgagggtcattgatttcacctacggggctatcaccctgtttcgccaaccttcccagattgttcgattatcaacaactttggtaactcaaatgttcagtcctacaaccccaatgagcaagctcattggtttgggctgttccccgttcgctcgccgctactgagggaatcgaaaatttctttctgctcctgtgggtactgagatgtttcagttccccacgtctacctctatacagctatgaattcactatatagtaacagtcgattaaaactgctgggtttccccattcggaaatctccggatcaaagcttacgtacagctccccgaagcatatcggtgttagtcccgtccttcatcggcttctagtgccaaggcatccaccatgcgccctttttaacttaacctgtacatcactacgtgatgcaaagttaattgagtatttgcgattttttctagttaacaaactcaaaataacgcggtgttctcggttgaaattatataaatacaatttcaaaaaattattacagaaaattaatattatctagttttcaaagaacgaattgagagtaggcctctcaaaactaaacaaaactttcgacaatgtgcaggattccgtttttccttagaaaggaggtgatccagccgcaggttctcctacggctaccttgttacgacttcaccctaatcatctgtcccaccttagacggctggtccccgaaggttacctcaccggctttgggtgttacaaactctcatggtgtgacgggcggtgtgtacaaggcccgggaacgtattcaccgtggcatgctgatccacgattactagcgattccaacttcatgtaggcgagttgcagcctacaatccgaactgagaacggctttaagagattagcttgacctcgcggtttcgcgactcgttgtaccgtccattgtagcacgtgtgtagcccaggtcataaggggcatgatgatttgacgtcatccccaccttcctccggtttgtcaccggcagtcttgctagagtgcccaactgaatgctggcaactaacaataagggttgcgctcgttgcgggacttaacccaacatctcacgacacgagctgacgacaaccatgcaccacctgtcattctgtccccgaagggaacgcctaatctcttaggttggcagaagatgtcaagacctggtaaggttcttcgcgtagcatcgaattaaaccacatgctccaccgcttgtgcgggcccccgtcaattcctttgagtttcaaccttgcggtcgtactccccaggcggagtgcttaatgcgttagctgcagcactgaagggcggaaaccctccaacacttagcactcatcgtttacggcatggactaccagggtatctaatcctgttcgctacccatgctttcgagcctcagcgtcagttacagaccagacagccgccttcgccactggtgttcttccatatatctacgcatttcaccgctacacatggagttccactgtcctcttctgcactcaagtctcccggtttccgatgcacttctccggttaagccgaaggctttcacatcagacctaaaaaaccgcctgcgctcgctttacgcccaataaatccggacaacgcttgccacctacgtattaccgcggctgctggcacgtagttagccgtggctttctggttggataccgtcaagatgtcaacagttactctgacacctgttcttctccaacaacagagttttacgagccgaaacccttcatcactcacgcggcgttgctccatcagactttcgtccattgtggaagattccctactgctgcctcccgtaggagtttgggccgtgtctcagtcccaatgtggccgattaccctctcaggtcggctacgtatcatcgccttggtaagccgttaccttaccaacaagctaatacgccgcgggtccatcctaaagtgacagccgaagccgtcttttaaaccaaaacaggtggttttggttgttatacggtattagcacctgtttccaagtgttatcccctacttcaagggcaggttacccacgtgttactcaccagttcgccactcgtctcaatgttaaatctttcaggtgcaagcacctgaaatcatcaacggagacgcgttcgacttgcatgtattaggcacgccgccagcgttcgtcctgagccaggatcaaactctcatcttaaattgtttaaaatgataagcctgtgatagctcatgatttaaatttattatttgtttttacgaattgacttcgcaaatgtttggttccaattccgaagaattggaacgccctgcacatttgtttgtcgaaaattttgttcagttttcaaaggtctacttggttgcgggtgagatgaatcatctctcgcgacaactatttaaatataccacgctgattgctcagagtcaacaaaaacttttttgattaacacgctttgttgtgtattccgttcaaatcagcatatataaatatatctgattctcaccgattcgtcaagtaaaaatcgaaagttaatttgcaatcacaattcaaagtggtctacgtgaaggttacgactaaaaagtttgaagcttcttcaaaaaaatcaccaaaacaaaaagcaatccaagttggattgctttaaaaaaattaatcgttattcgtattatcctcgggacgcattgttgggaacagaatcacgtcacgaatagatggtgcatcggtcaataacataaccagtcgatcaatgccgattccaagtccacccgttggcggcatgccatactcaagggcttcaatgtagtcttcatcaattccttcagcctcttcgttaccagctttacgttcagcaacttgagcctcaaatcgttgacgctgatcaattgggtcattcaattcagaaaatgcattggcgaactcgttagtcaaaatgtataactcaaaacgatcggtaaatcttggatcatcatggttcttcttggccagtggtgaaatctcaaccggatgcccataaataaatgttggctgctccagcttaggttgaacgagctcctcaaaaaatgcattaataatatggccggtcttccaccatggttcgtaatgaatatggtgttcatcagccaattttttagcgtcatcatcagacattggttgccaaaaatcaattccggtatattccttaattgcatcaaccatatgctgtcgtttaaacggtttgttcaagtcaacggtgtggccttgataagtcacaacattatcatccgtaacagcagctgctgctgccttaaagatgccctcagtttcatccatcacatcatggaagtcataataggcaacataggattcaagcatcgtgaactccggattatgacgggtatccattccttcatttctgaagacccggccaatttcatagacccgttccagtccacccacaatcaatcgcttcaaatgcagttcaagcgcaattcttaaatacaagtcgatattcaaagcattgtgatgggtaataaagggacgggcattcgcaccacccgcagaattatgcagaactggggtttctacttcttgataatcgtttgaatccaaatacttacggacagcagaaacaatcttcgtgcgcttaacaaaacgatcgaagctgtcctggttggaaatgagatcaaggtagcgctgacgataacgctgttccttgtcctttaagccatgaaatttatctggtagcggccgcagcgcctttgacaggaaagtaactgactctgcacgaacagtcagttcacccatgtctgttttgataatttggccggaaattccgaggtgatcaccaatgtcggatcgtttaaaaatatggtaaatgtcatcaccgacaatatccttacgaacatatatctggatttttccagttcgatcctttaaatcggcaaaaccgaccttacctttaccccgcttagcaatcattctgccggcaatggtaactttcttgtccttttccattaattcatctttatcttcatcatcaaaatcatgatgcagttgttcagcaagatatgtacgcacgaatcgatgtccaaatggatcgattccttccttgcgtaattcgtccatcttctggcgacggacgatcatttggtcattcatttctttgtctttggccactgtgaaacctcctaaatgaaaatttactattaataatcataacacaaaaagcgccgaatttattgtgctatccggtgctgacgtgcttttcgctgttcttttttctccaaaaattcatcaaaaatatcatccatcgctgattcgccggatgcgttcgtcaaggcaaccttggttcgagctgaatgaggaattccctttaagtaatagccggcttgaccgcgaaattcgtgggaaccgatataatcacctttcaattctaccaaacgatgcaaatgttccttggcagtaaccaccttttcctcaggtgtcggctcagctaacagctcgccggtttccaaataatgctgcgtctgctttaagatccacggattaccttcgaccgcacggcccatcataacagcatcggtgccaacttcagttaacatctttttggcatcttgcggtgttctgacatcgccatttcccataaatgggatgtgaatctcctgcgcaacctgcttcaaaatgccccagtccgcatgcccctcatacatttgtttccgggttcgcccatgcatcgccaaagctgaagcaccggctctttcagccgctaaagcgttctcaaccgcataaatatgatcttcatcccaaccggttctcatcttaacggtcaccggctttttaacggcatcagttacataagaaaccatctcgtagactttctttgggtccagcagccaacgagcaccggcatcagttttgacaaccttattcacagggcatcccatgttgatatcaatgatatcggcagcagtattttgatcgacaaatttagcggcctgaaccaacgtttccttggttccgccaaaaatttggatactcatcgggtgttcccggggatcaacaaacatcatatccaacgtttttttgtttttgtacataatcccgcggtcagaaatcatttcacaaacaactaggcctaccccatattctttacagataattctaaaggcagaatttgtaacccctgccattggtgcaacaaccacctgattagggattgtgacattaccaatattccatttcatactttcacctcaaaattcgtttgcaattgtgaaattccgcttgctatattatcacatatttgtgaaaaacgacagccaactttaatggtgtccctcagctttagcgactttgatgattttccccagctcttcttcattaaaatggtacttgctttcgcagaagttgcaagtcacgtcaattcctttatcctctttgagcatcgtttccaattgggggacggggaggccctcaagatctcggccaaaccgattcttcgagcagttgcagaagaattccaccggaacagtttccaaaaaatgcaactgacctttgccaaaaatgagttccaaaatatcttcaggactttgattgtccaataaaagctcagaaatcatcggcatctgtttaattcggtcgatgacttgattaatcgtgtcatcagttgcatccggcaatacctgcacgaggtagccgccggctgcgccgattgaattatcatcgttgacaaacacagagacccccaccgctgatggaatctgttcagattgggcgaggtagtacgtgaaatcgtcgccaatctcacctgaagccagcggcacgcttccagtatagggatcctcaccttcggcagcacgactcacctcaattaagccgttgacaccaaccgccttgccaacatcaattttatgatgggcattaagtggtaaatgcacatgagggttttgaatatagcctttgacatggccgttcgaatcactatcagcgacgatttggccaactggtccttgaccattgattttaaccgtcacagcttcaccatttttttcaaccgattcagcaagcataactgtgccgactaatgtccgtcccaaagctgcagatgatgcactccaggtatcgtggtcttgctgggcagtcgttacaagttgcttggcattcacagcgtatgcccgaaacatgccatcggtcgttgttgctttaactaaataatcatccatatcttgcacctcttctaaaaaataaaaacgagtttagagataattctaccctaaactcatttttgaaatattcaactaattgttatcgtcattgtcatgattgttatcttttggttgaccattgttagagacgtcatctggtttttcagagtcatccgtgctttgatcatccgaattgttttggtcagtgtcttgagtttgatccccagttgtatgacccttttccaattcagcttgacgttcagcttccttacgttccaattcacgtttggcttcttcaaaggttgccgcacgctcacttggaaattcacttgtatcggaactttcaggcattttacctgtgtgccaaagtgaaagaatctgcttctcatcaagggtttcatacttcaacaaggcttccgcaatcagcttgtgcttatcacgatgctcctcgataatcttcttagcagtgtcgtgagcttcgttggttaaacgacgaacctcttcatcaacagcagcaccggtttcttgagaatatcttggaccataagtgtcttgggcaggattttcaagctgtaccggaccaagtcgtttgctcattccatactgagtaaccatggctcgagcgatgttggttgcctgttcaaagtcattggaagcaccagaggattgtgagtcaaagacaatttcttcggcagcacgaccacccatcaaaccggcaatctgttccatcgcgtccttcttagacatcaactgctggtcttcacgcggcagcataatcgcataaccaccggcacggccacggggtacaatggtaaccttgtggacaactcgggcatcattcaagaccaacccaaccacagtatggccggcttcgtgataagcaacggtttcccgttcctcttttgaaataacccgattccgtttggcaggaccggcgatcacacgatcttcggcctcgtccaagtcactcgcgtcgatttgcgtcttgttgcgacgagcagccagcaaggccgcttcattcagcaggttggccaaatcggcaccaacgaatcctggcgtttgcttggcaatctcgtgcagatcaacgtcgtttgccaatggcttgtttttagaatggactttcagaattgcttcacgaccgttaatatctggacgtccaaccaagatcttccggtcaaaacgacctggacgagtcaaggcgggatccaaaacatcggcacggttggttgcggcaatgacaatcacgccttcattgccactgaatccatccatttcaaccagtaattggttaagggtctgctcacgttcatcatggcccccacccatgccggcgccacgacgacgaccgacggcatcaatttcatcgatgaagatgatggcgggagcagccttcttggcttgatcaaacaagtcacgaacacggctggcaccaacacctacgaacatttcaacgaaatcagaaccggaaattgagtagaacggcactccggcttcaccggccaccgctttggcaagcaaagttttaccagtaccaggaggtccctcaagtaacaccccatgtgggatggtagcccccaaagttgtaaatttccttggatctttcaggaattcaacaacttcgaccagctcttgtttttcttcctcttcaccagcaacatctgagaaacgaaccttattttgcttactgtcggctggtttggccttggatttgccaaagctcatcactttgccgtttccgccgccttgaccgccagcacggcccatcatcatgtagaagaaccaaacaaacaataacagcggcaagacgtaaaccaatagatttacccaaaaaccgcttgactcttcaggcttggcattcatcttaacattgttagattgagctgccttggtgatttcagcaattgaggagttattctcgaggacagttgcggtaaatttggtaacattcttagactgagtctggtttccaccaatgagtccggattgcacctgtaccttctgaccctgtctataagttccagttaccttatagacaccgccacttggctgtactgaaaagctttttactttgtcatccttcaagttcttaacaaactggcttgattggatttcctgcgatgtggtctggttggtatttccgttaaagaaatagataacccccattatcagcagaaatatgacaatgtaaaacagactatttttaaaaagcccatttctattcgagttcatcaacgtcctcctcaaaactaaatattttcatgttgatagtcaaaatactaacacacttgaccttttttgactattaattgtttgtataaatttcaggcttcaagacaccaatgtacggcaggttacgatacttttcgtcgtaatccaaaccgtagccgacgacaaattcgttgggaaccttaaaaccaatgaaatccgactcggcatcaacggctcttccagcgggtttgtccaacagggtacaaaccttaattgaactggcaccacgatcggcgaacgtgtccagcaggaacttcaacgtccggccagtatcgacgatgtcttcaacaattaagacatcacgcccatcaatgtcggtgttgatatcctgcagcaattccaccgtcccggaagattcagtcgcaccatgataactggaaacgtcgataaagtcgatttgcatgtatgaatcaactgctcgggcaatgtcggtcatgaagaaaatagcgccctttaagacacccactaccaccggcgtcttgcctgcataagtctgagctatttcttttcccagcctttcaacggctgcttgaatttcttccttgctgtaaagtacctttaagatgtcgttattcattacaaattccttttctttccaatcattatttttgtcggacttcaattaaaaaataaggcctagtgtcctcggaatcccgagaaacaacggcatttttcagacccaacactgataatacggtacctctggcatcgaccagcaacaaggtccgctcacgttggtcgttgggaactttggcattgatcagcacccggctgaccttttggtgttgtccgtgaccgattgataatcgatcccctgcttttggagagcgaacctgcaacggtaaatctgtatcctgcaggtaaaaagttgtcagtttactgttagcaaccgttttgtgtgcagtgaacacaccaaatttggtggacggactcagagaataccatctgtctaatattaccataaaagttcgatctttttcaggtttaccaacgattttttgtggttccttacaaattattagtgattgatacacccgcctgacctgccatccagcctctaaatccattttggcttgtggtctggcggtctgctggatcaggcccaaaacttcgtcaagttgatcaactgaaacgttggggattcgaagataatgttcgaacacttcctcaagcaaacacttgacgacactgtcgggaaaatctttgagtgaatcgagatcaatttctgcccgttgcttttctggaaaaccaactgcggaatgaatcagcggctgaatcaagaattcaatggcggccaagttgtcggccaactggttggtataactgagcacatgaggcagcagctgcggattctctgctttgagtaatggcatcacgccatggcgaattcgattacgttcaacagccagctgctgattggtttcgtcttcaaaccacctgattccagttgtttgagcaaatgattccaactgctgcttactaaacgacaaaagtggtctaatcatgttggcatctgcaaacgatcgggtttcgcgaatgccggtcagagaagctaattgaccgccgcggaccagcttcataatgacggtttcaaccagatcatcgccatgatgagccgtcaacaggcaggtactaccggtttccttcaaaacacgctcaaaaaagcgataccgaaaggtccgggctgccgcctcaatcccgacctttgggtggtcgtctttcggccagacagcttgtttgagtaaaagcccgtgttcactgcaataattcgatatatagcgggtctcttcaacgctttgatctcggagctgatgatccacataggcgacaataattttgggccgaacagctcgcggcaggtgctgcagcatatatagtaacgtcatcgaatccactccggtggaaacggcaaccaccactgcatctccagcctgccaccacgctttttgcttaacaatgaaattaaattgtttctgtaaatccactgtggcctccgcttatgacttgcaggtataaaacaaatatggccggcagcaaatgattgccccagccacaaacttattaattgtcaaattctaatcgattaactacgccggccgccgcgaccaccacgtttgccttcggtgttcttacgcagtgtggacaagcgatcttcactttctttcaaaaagccggacatcatgtcatcaaaactctcttcatgattattcgagtgattgttgtgagcagaactgccgccacgggaatgataaccgtgactttgatgattcccgtggttctcatgaatttcgtggttattctcgtggaaatttctgtgagaatgattttcattcttagaatcttcatgttcatgattgtcagaagctttgcggatcgaaagactaatcttgttgttgccctcaatcttgaggacctttaccgtgacatcatcgccgaccttcaaaacatcatgaatatctttaacaaatccgtcagaaacttcgctgatatgaaccaaaccggttcgatgatcacctaaatcaataaatgcaccaaaattcgtaattccggaaactttaccgttaactttttctccaacttcaattgccatctaaaaaaatgttcctcccatgtaatagtgttaccagtatatcatattttattttatctcgactagcgattgtcaaaataaaaggcgaagacaaaagtacaaatacttttggcctcggcctccttgactcatcttatttgacatcgtaatcattaacatcttttggtgccttattagggaaactatagactgtttcgccaggttttgtatagtaataacgatcacgaataatttgttccacgtaattcttgtcattcaactgggcgacttgcgttttgagttgtttctggtccgccttttgctgttttaaggtcttttgctcacgggcaattcgaacatgcacgtcagcgtaattcactttggcacgaacaatttggataagaaaaattgacgcaaagaataggaaaatggcactaataactaaggcccgcttttttcgtcgattagacaaaacagcagtcacccttgagttattcaattcaatctctcggcgacgagtaaaatcgttgtcgagcttccgtactttcccactttgctgcgtcatgctaaatcccccgatcattcgcacgttctagataaattataccaatctatgggcatttgtctaggtgattccacatgttttcgggatttttatggatatttatttattcgttgcgaaagtcgcgttcatagtcctcggaggtaatctcatacatccgttctgcatcatcctttttggttgtatccaacagttccttgaccaagatagtcagagtcttgttaccaaatttgatgacaacctcatcgttgggtttaacttcggttgaagatttggcggcccgcccgttgataaagatccggcccttgtcggcaatctctttggcaacagaacggcgcttaataattctggaaacttttaaaaacttatcgattctcatgagttgtgactcctttaatttttaagaacttaccaacaaacggaatggccaaccattcacggacagtaaatacgtccaacagtcgacaccccgcaaaaaatatgatcacgccaatcggaatggcgatgcagacaaccagcaaagcagcgattcttggattatcagccaagtcagccaggttaatcccaaataccgttgcccgaaccgcaatgaacatggtcaccagcacaatcacaagcttgccaagctgcttaaaagaaatcaatttggccaactcttttcgactgagcaggttcattaataacaccattaccattaagcttaacagggttgcaagactagcgccaatgattccaaagtgtgccacgaacaattgattaaccaacaccttgatcaaaaagccagcaagaatggcgatcattgtcctcaaataattatccttgctctgtaaaatcacgttataggtcatcaacacgctggttaaaacgatgctgatgcagtacaagctaatcgtcaaatttaactcggacgaagcaaataacaaccggttaatttggggcattagagcggccaacccgacactcatggcaagggaaacagccaaattagttctcaggttcgtggccgcaacgtgttgaaacgtgacatcttgacggtgtttatttgccaacaccaaaccaggcaaaacggcggttgcagacgcaatgctcaaaacttgtcccagttgaacaagggtctgagaacgatcgtaaattcccttgatattctgggcagcaaccagcgaatagccaaacgatcgcaatccagacacaacggaaaatgaatcagccaactgaagcaatagcatcactgccgataccaagcacagtgtgccgccctccagcaaaatgcgcttaattaacagccgtgtttcaatagtcggacgtcgatttcgccagtttgttggcaatgatcttgatttcatccaaatcaggatgaacaacagggcaatcaggccggcaattggtgcagacagcatggccaactgacccattcgatacggactgaccgtcgatttgaaggcccagtaaccaaccaaaagaatactcgatactcgaacaacctgttcaatcacttgcgaatacgccgtcggccgcatttccattttgccttgaaagtatccccgccaggttgacagaaatgggacaaacaggaacatccagctgactgattgaaccaccggtgccaattggggatcatccattttcccggcaatgaatccggcagcaaattgcaatatacaaaaaaccaccaggcaaaccacgattaggatgttttgaattcgaatggccaacccgacctgatctcttggatctttggtgtcgaccactaatttggaaataaaaaccggtagccccgtcaaagcaaaggtcatcccaataccataaattggataaatctgttgataaacataaaagccgatgttaccaaccatgttttggaagggaattcgatacacggcacttaacaatttggcaacaaatgacgcgaccgtcagcagtaaggttcctttaagaacgagttgtcttcttgacctatttttcatcagactttaccttaccggcagcaccatgatgattccgggtttttgatagttgtttgactaatgcaatcagcccgtccaaccactttgtcatgttgggctgaacagttaattgaatttgatacctgtcattttcggtgttaatggttgcccggaacttggtttgggcaatcgcttccaacaattccttgctggagaactctgtccctgcccgaggtgaaaacgtgatggtaattttgggctgattttgatggattttatcaaccaacgcataatcggagaacatcttcagctgagagatctttaacaggttggcgacgggttcaccatagtccccaaatcgatcgattagatcatcttcaacttcgtggagctgatcttcattttcaatttggcggatccgtttatacaattcaatcttttgttgattgtcctgaatataatcactcggcagataggcttccaggtcaagctcaatagttgcatcagttcgatactcaaagttcttgccgcgttttttggcaacggcatccgacaacatctgggtatacaggtcgtacccaaccgaatcaacaaacccgtgctgctgcttaccgagcaggttacctgctccacggattgataggtcccgcatcgcaatcttgaatccggatcccaattcggtaaagtcacgaattgcctccaaccgtttctcaccaatttctgtgaggaccttatttggtttgtacataaaataagcataggccactcggctgctgcggccaatccgcccccgcagttgataaagctgagagaggcccattcgatcagcattctcaacaaatagcgtattaacgtttggaatatccaccccggtttcaataatcgtggtagttaccaaaacatcatattcaccatttatgaaatcatacaaaatgtcttccatctggttttcggacatttgtccgtgaatgtaaccgactctggctgaagggaccaaggcactgatttgttcaaccgtcttttcaatatcagaaacccgattgtggaggtaaaagacctggccgccacgcgacatttcccgttcaatcgcctcccgaatcgtgccggcattttgttcgatcacataagtctgaatgggataacggttggatggcggcgtctcaatcacagacaaatcacgaacccccatcatcgacatgttcagcgtccgtggaattggtgttgccgtcagtgtcaagacatcaacgtcagaacgcatttccttgatgcgttccttgtgtttaacgccaaaccgctgctcttcatcaatgattaacaggcccaaatcattaaacttaacgtcttttgaaagcagtcgatgagtgccgacaaccacatcgaccttaccgtcttttaagccttggagggtctccttgacttgtttggcggtctgaaatctggaaagcactctgactgtaatcgggtactctcgaaaacggtccagcatggtttcataatgctgctgggctaaaattgtggttggcaccaaaaaagcgacctgtttaccaacttcaattgctttgaaagcagctctcaaagcaacctcggtcttaccgtaaccaacatctccaaccagtaaacgatccattggatgctgggtttccatatcccgcttaatttcagtcgcactccgcagttgatcgggtgtttcactgtaaggaaaggcagcttcgaattctgcctgcaacgaatcgtcttgaggataggcgtaacccttttctgcgcttcttttggcgtataaatcgattagttcatcagcgatgtcttcaatcttggaagcaactttggccttggtctttgcccactcgctgccgcctagtttattgatccgcgggtgcttatcttcggaggaaacatatttttgaattaaatttaactgggtgaccgggatgaacaatttggcgttatctttataggaaatcgtcaaataatcctggtgcttaccgtcgacttccatggtcttcatgccttcataacggccgattccatggttgacgtggacgacataatcgccgggcttcaaatcggtataactcttgattctttcagcgttgttaaaggtggtttggcgggggcgttttttagtcaccgtgccaaacatttctttttcagtgatcaccacacaactggccaacggcagctcaaatccgttgtccaagttgctggaaatgagctggacttcttgttttaaaagatgatccttatcagtctgagtcgccgtaatttcaaaatcgttcagcgttgaagcgacctttgccagtcgtttctcatcttgaaccataatgatgactgtctgcttcattttctgccagcgcaaaatctcggttcgaagcattggaatttgggagaagaactgctgcatcggccgtacggtaatgtcttcaatggcatccagtcgcatccggcccatccctttttggaacagtgacagaattaaggtggcgtgatgattagcgctgaaggctttcttgaaatcattggtgtatgtggtcgacttcaaaacctcatagtgcttaatcttgtcgttcaaccactcatcgtcatcgctctcaagctgtctggcagtttcagtaattctggcataatcgtcgaaaataacaacgccatcggcagccaggtaatccagcagggaagactgttttttataaatcatatccgcaaataacaaccagcgtggatcactcaacccattttgcagatccatgatttgcggttccaagttgccctgaagctttttggccgccttgtcatccagttgactttgttcagcaattaaccgtttggacagctgcttgctgacggcttttcgctggtcatcggtcattaataagtccgtggctggtagtaccgtgattgacttgatgtttttgatgcttcgctgattggaaacatcgaatgtccgcattgagtcgacatccgtgtcaaaaaagtcaattcgaaccgggtcttgatggtttaatgggaaaatatcgagaatcgacccccgaattgaaaaatctcccggagccgcaaccattttttgaaaaacgtaccccatttgatgaagctgaagctttaattgctccaggtcataggtgccgtccatttcaagcgttaacttagcggcttgaaactgctttttctccggcaccagtcttctaataccggaaacagaggtcacaatgaccgccggatcgccgctggcaagcttgtccaacgctaatacccgttgggctttgtattccggtgaactggtggccagctcagctgctcccatttcttccaccgggaactcaaacaactgatcgtcatcaatcaagttagataagtcattcaccaactggtcagcatgaaataacgagtcaactaccacaacagttggtttgtcagtcgaatgaattaaattatcgattaaaagtgtccgggcggaaccgccgactccggtcaccaattgacgcgtgcccggtttcaaggttgcgaccaactcctgatactgaggaattgttgttagtaattgatctaacttcaaaataatgtcctttcgttaattatactgattttccaaatccggaatcgacatcccgtcaatccaatcatccaaggcattcacggcgtgatcagcagcctgcttaaacattggggcttgatctttgctgaatcggcccagcacgtaattaacgaccgtattgccatgatccgggtgatcaattccaacccgaatccgatcgaaattttgggtgccgacactggcaataatgcttttaatcccattatgaccgccagctgaacctttatccttaatgcgaatcttgccaaccggcagatccatgtcatcatgcacaatgatgagatcttcgattgaaacgtcaaagtagtccattaaggggcggacagccaagccggagtcattcatgaatgttgtcggctcgaccaccatcactttggtgttgttgacaaacccagagccatacttggcgttcattttacgcgtcttaattgaaatgtcatggcttttggcaaattgttccactaccataaagccggtattatgtctggtcccatcatattgcgggccaatatttcctagtccaacgatcattttcattgtttaaattcttcctcacgtttcttccaacacaaaatgctgaacaaagactgttcagctgtcgaaaaattaattaacataaagattatatcatatcagacaagcttttaagtcctggaaaaaccggaaaattaaaagatgtttatcagtgaagacgccttcaaaatcatgctataattagcgtgttctaggaattatatattaatgatttggagatgatttttttgactttacaacgccaaaaagtagctttaattggtgacggtgccgtaggttcatcatatgcctatgcaatgatgcaacaaggcctcgctgaagagtttgtgatcgtagatgtgattaaggaacgaactgaaggagacgcactcgaccttgaagatgcccaagccttcacctccccaaaacacgtttactcaggtgattatgcagattgtaaggatgccgacttggcagtcatcactgccggcgctccacaaaagcctggcgaaactcgcttggatctggttaataagaacctcaagatcatgaaatctatcattgatccacttgttggctctggattcaacggcgtcattgttgttgctgccaacccggttgacattttaacttatgcagctcaaaaattctccggcttcccaaagaaccgtgtctttggaagcggaacttctctggatacttccagattgcaggtcgctttgggcaaaaagttgcaagttagcccacaatcaatcagtgcttacattttaggtgaacacggtgattccgaatttgctgcctattctgcagctcaaatcggcggccgtccattcttagacgttgccaaagaagccggtttatcaatggatgacttaaaagagattgaagaccaggttcgtcataaggcatacgagatcatcaaccgaaaaggtgccacattctatggagttgccacctgtttgatgagaatttcacgagctattttgcgtgatgaaaatgcagttctgcccgttggtgcgccaatggatggcgaatacggacttcatgatgtctacatcggttcacctgccgtggtcaatgcatccggcattcaaaaagttgttgaagttccacttaacgccgatgaagctgccgcaatgaaggcttctgctgagacccttcaaaagacgactgctgatggcatggcagaactttaattccgctgtttgtactaacgataaagggatgatgaatcagcatcctcagcctcaataatgaatcaaaacgggcaattattcctatgggatagaaataattgcccgtttttttaggaagtcctagcaagtcaacatatggaacatttccttgtgtccagcttgtcagctgattcaagccggattttcaatagctattctaatttatttagagattaatgagaataattcaagtttaaatgttcttttctaaatttctctatgttatcatggttgtatacaggttaatttggaggaattaaacatgctattaaaaacattagtaaagcctaaggaacgactggtgaccgtcaaagaagacgccaccttggaagaggctttacagactctcgaagattccggttatcgttgtgtgccaatcttagatgaaaccggcaagattttccgtggcaatatctacaaaatgcacatttatcgtcataaatcacggggtggtgacatgtcacttcccgttaccacacttttaaagaacgcaaccaagttcatcaacgtgaattctgcgttctttcaagtattcttttcaattaaggatctcccctacatcgcggttttggacgaacgaaataacttttatgggatcttaacccatacccgtctctttgacatgctgtcacagtcttggaacgtgaatattggcagttacgtgttaaccgtcgttgcaagcggcgagcgtggtgatcttgaagaaattgccaaaattatcaccaagtacaccaacattgccagcgtcatttccttggacgctcaagaaggtgaattggttcatcgcattatgttcaccctgcctgccgaagtggatcaggatcgtttaaacagaattattgctgctttggaacgcaaggaattcagagtgcctgaagttgaaaatctgcaagaagaaaaaaattaggcacattgtacgtgcatatcaaaagaagaggctgggacacaactaattggaggttgtgtcttggcctcgcttgcgttccaatgttatctagttcaaacatggaactatcggctgatcccggccgtttaagccaagaagcgagtcattccatgacaggaataactcgcttcttggcttaaattctgggatcaagacgcctcgcgtcgcactcccttttgattataattgtattcaattgatctaagcgttgtgtgatgttttatgtattgcggtccgtcactagcctttagctaatcccaagcttatctttatcgctttatcgaccttactcataataggcggatcgagatgggttactttatccttcaatcgctgcttatcaatggttctgatctgctcgagtaaaataactgaatctctttctatcccatttccagccaagatccccacgtgtgtgggcattttgggtttggaaattctggcggtaattgcggcaacaatgacggtgggactgtaatgattgccaatatcattttggacaatcaagaccggtcgcatcccgccctgctcggaaccgataactggtgatagatcagcataaaaaatgtctccacgtttaaaaataacgtcagtcaccctcatacctcccatcatcgtaacttacattactgtaaattccgtaatctttgacgatactgagttaaatggatatcagcgtcttcttcacagcaggaaaagtccttactgatctcacggttcaaactacccatttcgcgatatcccctcattaagccatcaatgactttcgggtcatcaaaaaagtagttgattgcaatctcaaccgctgcactttcggatattccaaccgttgcgataaactgttccaaacggtctgcaatttgatcattgatcataactgaaaaatgctttgaattagttgctttttccattggtattttcccctatatgttccagattactgtactgtctaatataccatgaaattacagaaaaatcatacatattttcgacgcaatcgcggactcaagccacaaataacctcataactgatggtatgcagataatccgcaacatcatcggcagtaatctgagcatcacccgattgaccgatgatggtgactgtcgtgccgtaaggataatcatgaggcaatcgaatcataaactgatccatgcaaactcgaccaacgatcggacacttgtggccatcaaccaagactgaaaagccctgcattgcccggggaattccgtcggcatagccaaccggaacggtcccaatccattggtcgctatcagtggtgtaggttgcaccatacccgattgagcggccctttttaactaattttgaaaaatcaatttcggaggttactgataaacctggtttcaactgatatggaagctgggtaatatctcttccggacgggttcaagccataagccgcaatcccaaagcgaatcatgttgccgccgcaaactttgtgccacaagctggtagcggaattggccacgtgaacatacttcgggcgtttatcaagaactgccataaagtcctgaaaattctggtactggaatttgaaataggtatcgtcaggactgtcagcagtggcaaaatgggtaaagattccttcaaaactcatccgatcggaatgggcgttgagaaccccaacggcagctttaagctcatccgcagtttgaaagccaattcgacccatgccggtatccagtgccaaatgaatgtttagccggcctttaaatgcgctggtgtcgagtaatttggcagcttgattaagccagtcgatcgaaccgacagtcagggaaatgttttcggaagccgctaattgggcacattcaggatcagtaatccctaataccagtaccggcagcctaattcctgcctggcgaagttggagagcttcatctaaaatagcgacacaaaaaccagtggcgcccgctttttcagcaatctcggccacttgaactgccccatgcccataaccgtcagctttaaccacttggaacaagtcgtctccgtcatccaaacgctgcttggcatggtgaatatttgaataaattgccgccaggtcaacagttacctgggcatttcgtaaatttccaactgtcattacctaaccccgattctctaaaataacttgagtaacgacaatgtcatcggtgtgagaaatcgacacaaaggcgttcccatcaaatggttgtttcgaaaagaagggtttgccctcctcgttattaacaatacaaagatcctgaaatctcactttcgatccaaggccggaaccaaaggccttcgaataggcttctttggccgaaaaacgaccggagatatattcataacggcgcttatcagacaattcagccaattgtttcatttcatctgctgttaaaatacgctctgtgaaatgctgattccgttccacggcagcgacaattcttctaatatcggtaacatcaatcccaattcctgcaatcattttctaaatccctcgcaaaccaaaaagataggataagtttaacataaaaacggcctcgtcggggcagatttgaaagacttgtcacgaagtcaatgacgattaacgacatgcttgcattacaagttggtgcatacaagaaccctcatcaactcaatcaaaaaagtgaccattcatcatcgaatgatcacttcgttaaaaatcttaattaactatttttaatggtaaaacggcgtttcttattgcttgatgaccgtctgtcagaatgcttacggtcgttactgccttcataatggccccgatttcggctgccattattccggtcgccattacgatgactctttgagcccttgtaatgaccaccatgaccgccaccacgacgatcgttgcgatgaccaccgtgtccatgaccatgatgtggtaatgggcgttcaggggtaatcttaaccttaacgttgtcgcgagtaacgtcgttgagcagagcagcaaccaaatcagttgcttcatactcgtcgagcagcttgtcagccatcttctcatacttgtcagtattcgtcttcttaattaagtcggcaatatctgattcagcagaattcaattgaccaacaaaggcttcttgaattgttggtggcttcaaaggcagcatacgcaccttggtcaacttttcgatttctcgaagataatccatttcattaggcgttgcaaaggtaattgaaaccccatgcttaccggcacggccggtacgaccaacacgatggacgtagccatcaggatcttgaggaatatcgtagttataaacgtgggtcacacctgaaatatcaattccacgggcagcaacatcagtggcaactaagatatcaatcttggcagctttgaattcctgcatgatctgagtccgacgagcctgagtcagatctccgtgaagaccggcagccttgtagccacgggcctggagtcctttggagacttcatcaacccgacgcttagtccgacagaagacaatggtgacttctggatcctgaacgtcaaagaaacgggtcatggtgtcaaatttttcgtattcttttacccgaacatagtactgatcaattaaatcagtggttaattctttagccttaatcgttacttgatgagggtcacgcataaactgaaccccaacccgtttgatttgggcaggcatcgttgctgagaaaagcaaagtttgacgttcctttggggtttgtttgatgatatcttcaatatcgtctaaaaatcccatgttcaacatctcatcagcttcatccaacactaatgtcttaacgtgctctaactttaaagtatggcgtctaatatgatcaagaattcggcccggagttccaaccacaatctgtggatgaccctttaaggcgttgatttgacggcgaatatctgcaccaccataaacaacttgaaccttagctttttcatcttttcctaatcgatagatttcttcttgtgtctggattgccagctcccgagttggtgaaatgatcagagcttggacatttggattgtcaaaatcaatcttctgtaagattggtaaaccaaatgcggcagtttttccagttccagtttgagcttgaccgataacatcctcacctttaagaaccattgggatggtttcgccctggattggcgtagcttcttcaaacccactgttattaatcgcagttaataagtggtctgataatcctaattcactaaacttcaaatatgtttcctcctaatattgaaacaatcaaggttccgcggccgactggggaaaaatccgtttcccggaatgcgttgaccacttgacctacaatcatttattacaaaataacctttttagtttacaccgtcacataacattaagcaagcaatacaggccaactcctctgttgaccgtgcttatttaaccagtttggcaacaacattttccaaatgcagaccgtgactggccttcaacaagacctcatcgtcagcgctcaattcggcttgaagatcagaggtcaattcatcaagctgatcagcttggtaatagtggagattctctggggcatagaccggcttgagtttctcatatagggcgtccatatcggcgccaatcaggtacaccaccggaatggaggccggatccagggcatccgctagcgaagcgtgcatcgcttttgattgagtcccaagctccaacatgtcgcctaaaacagcaatccgtcgccccttggttgtcgtgttcttaaaagcggtcaacacttctttagcggcggtggggttagaattatagacgtcacttaaaattcgctcgccctttgaaccactcaaccactgggtccgattcttagtcagatcaaatttagccaacttgtcagccatcatctgcggatggattcggaaaattcggccaaccgaaatggccgccagggcattgttgacgttataatcaccgatcatcggaatcgtaaaatcaatctccggccacaaattgacgtgaaattgcgtctgatactgaccatctttggagtcgatggcaaaaacatcattgctgtcttttctgccaaaagtcgctttgatcacactctcatccacttgttgggcacgctctgtgagcagcggctcgtcaccgtcatagacgaagaagccgtcagctttcagaccatgagtgatctccattttggcgtcggcaatcttatcacgggtgccaaagaactcaatatgggcttcaccaatcatggtaataacggctacatcgggccgagccagtttggatagaaaatctagttgcccgggtcgatccatccccatttccgccactaaaaactcggtattggattccatctgcagaatcgtataaggcaggccaatctcattattaaaattgtcctgggttttggtgacattaaacgtactggataaaattgcggcgatcatatctttggtggtcgtcttgccgttgcttccggtgacggcaatgacgcgtggattaatcttatcaagataatatttgctgagctgttgaaatgctgtcagtagatcgtcaacaaccagtgccggaattgttagtggtaagcgatccgcgtggtcactggcccaaagggtagctgaggcgccgcccgcaattgcattgtcgatgtaatcgtggccgtcatgttctgcaaccagcggaacaaacagttgaccagcttgaatcttccggctgtcaaagcacaccccggtcaaagattcgtccagcattgctttgtcaaaattttcagtgttggcattaattgcttgagcaacttcgccaatcgtcattttcattattgaacgctccaattgttaaatagttatgttcaattataacaaaaaatcaaacggctaaacacccaccgtttgatcctgccattctaaatgccattttgatgtttgtaaattataggtcaagtccccggcatagacggtattttcatcgactttaccggttcgcaaaataattgaaacctgatccgggtccttcaaaatccgtaatggaatatgataagtccgggaacgttcccgcaaggaatcaaaggaaataaacaggccgtcgttagctttggtaatcaaatccaagagaatcgagcggtcaatgtctttgatcgccaatggacgcaggaagactctcaaagtgttatgggtctctcgcaaattgcgcttaatggcgatttccaagacgtggttaaagtctgagaaacgccggtaatatgaacgaatcgttccgttgtcttgactcaaataaatgtaatgattgttcaatttggaagaaaaaggccgacccattggcgttcccatgtgggccagatacaacagttccgcaatttcaaatggtgacaagttgttaacactgtcttccacgtcaaaatcaataaacttcttcttttggtcgggattacggaggagataggtccgaatttcacctgtgccattgatcagattgaacttggaatgagagttgtacccgttagcagcctgatcatcattatttaacaaaatgatattttgaggcaattcatccagtccattaataaaatcggccgcagtgatccctgatgataaaatcatgttggagattggattcgtatttataaaaatcaaattgcccttcatcgtttcattaccccgtatttatatctaaactaattgtactaccctcacgtttagttgtcttataattaagacagaaatgtcgtaatttgcccttttcttaattcattggtaacatggtggttaacgcaatattagtgtgaggttattaatatgactaacgtattatttgtttgtctgggaaatatctgccgttcgcccatggctgagatcatgttccgtcaaatggtgaaggatgcccatttggaaaatcaaattaccgttgcttctgcagcgattagtaccgaagagcatggcaatccgcctcatccaggtgcgattgccgaattagccaaacacggcttgtccgtcggcaataaaacgtcgacgcccatcaccaaagaagactttgatcaggctgattacattattgccatggataatcaaaatatcttttatctcaatcaaatggccccaattgccgatcggaaaaagattttcctttgctacaacattattcccgacaagcagggaaaagatatcccggacccctggtttgaccacaaatttggccgaacttaccgtcagttatcagaaaccctgccgaaatggttggataaaatgaaaagccaattggcttaattattgacgggtcccaataaggctcgttttaattttggtgtcgcatgactgattcgataacttttttggagtttaccgcgaatcatcaagcgtcccgcgccggtcgcgtcacaggtgatcaacgtgacaatcggccgcttggtttggcggacaacgtcaacccgggtcgctgcgataaacttgcgctggtaaaccttgtattgatagactttggtcatattactgagatagatccgatcaccaacttgggttttgaagtacagcgggccaaataaaacgtggcggttaaccatgtggtgccctgccaacggatagttgcccttgcccatctgctggtcaggccgcatggtcccggcagctagcgccaaggtattattagccactcccaacccaattggcaaatgaatatgtgatttgggcaggagaatttcgccgataacttcaatggcgttggtgttcatccgcgcccgagcagcagtttgaaaatcaagggatttgacttttttaaaatcataactgacattttgcttgtgacgcttagtttgtgctttttgccgccgttcagttttggcaacggtctggcgggtgatttttggctgataagatttgatcaattcatttttgattggccgattaaaaatcatccccaaagcgacaattatcaacaacacaaaaaccacgttaatcaatattttcttgagaagtccttttctcataactacctccactcaacaacgaattataatatgtacaaaataataaaggaggaacctcattgttaacaaaacaagttggtccaaactcctggcggcgcaatttagccgttctctggtttggaaccttcatggccggaatcggcttcagcgaagtgatgccatttctgtctctatacgttgattcgctggggcatttcacccataacgaattgagcctctacagtggattggcctttgcggccagttacctagtgaccgcgattgcttcgccactgtggggaaaattggctgatcgaaccggccgaaaattgatgttggtccgagcatccgccggaatggccattgtcttcattttgatgggattggtcaccaacgtctggcaattaattggccttcggctcctgcagggtgtcttttccggatacatcagcaatgccaacgccctgattgccacccaggtgccgaaacgcaaaagcggccaggccctcggcactttggtaaccggtaacgtgtccggtgccctgctcggcccgctgttaggcggaactttggcctcattcttcagctatcgggtcacattctttattaccggcgccctgtttgtcggtgtcttcctggtaacgacgttgatggtccacgaagatttcaaaccagtcgccaagtcgaaaatgctcaacacgcgtggcgtaattggtgaactggccaattcaaagctggtacttgggatgtttgttaccaccatgattattcaagcggctaacaactccatcgttccaattttagcattatatgtccgccaaatcatgaataatagcccggcgaccaccttctatagcggaattgtcgctgcggtccccggcattgccaccttggcagctgctccgatgttgggacggctgggcgatcggattggtgctgatcgcgtcttgctggtcggttttctgctggcaatcgttgtctacgttccaatggcatttgtcactaacgtctggcaattgattggtcttcggttcctgatcggcgtcgccaacgcgtcaatgttacccgctgtccagtcgattctggctaagaacaccccacctcacgttaccggccgtgtgtttagctggaaccagtctttccaagcgatgggcaacgtggctggtccaatgattggatcagtcgtctcgacctcatttgattacgcaggtgttttcatttcaactgccgtcctggtagtcattaacctcaccttagtattcaacaatacgcggggaatgcgccgagcacgcaaacaacggattgaataaacccgtttaccaattagtatgagaacgaaaaataggagttggacagtcagtatcgcttgtccaacccctatttgtttgcataaaaaacggggaaccgttaagctcctcgtcttcgtcatgcttatttgttgtctgtaagaccgtatttcttgttgaaacgatctacggcaccatctacttgattgaacttctgcttaccagtgtagaatgggtgtgaatctgatgaaatttcaacacggatcaatgggtaagtcttgccatcttccatcttgatcgtttcgtcagaggttttagttgatcctgagatgaacttgaaacctgtagatgaatcttgaaatacaacttgttgatatgctggatgaattccttttttcattatatatcgctcctttgccctgaatcaatccgatgacccagagattatcgattagtcaactttgttagtgtaccataaataaaatcgtcaatcaatcatcaattgactctttcttcaacttctaatttaacgtcggcacccacaccccgcagcttatcaacgatgtttccatagccgcggaggatgttgtcggcatggcagatttccgtggtgccatccgccatcagcccggcaatcactaacgacgcgccggcacggatttcacctgcctgaactttggcacccattagcttgggggagttatcaactacaatgatgccttcatcggtatcctctgatttgactttaccgcccaatttattcagttctgtaatgtgcttaatccgtttgggataaatggtgtcaatgatcacactgcgcccctttgccttaaataatagcggcgtcaatggctgctgaagatcagtggcaaacccaggataaggcatcaccttaattcggattggcttcaagtcatgtgatggtccgacataaatgctgtcctcataaaccgttaagtcgcagcccatctcttctaatttggcgacaaaagcttccaaatgttcggggatgatgttggtgattaaaatcccatcccccacagctgcagcgagtgacaaataagtgccggcttcgattcgatcaggaataattgtatgagtattacgagcctgaagggttggcacgccttcaattcgaatgacatcggtcccggcaccacgaatattggcacccatgttgttcaagaatgtcgcaatgtcaataatttcaggttccttagccgcgttgccaataacggtggttccaggcgccttgaccgacgccaagattgtattgatagtcgcacccacagaaacgatgtctaagaaaatctgggcaccatgcaggccatccgggccggtcttaatggtcactgtcccatcgtgttcactgacttcagctcctaaagccttaaatgccttgatatgctggtcaattggccgcggcccgatattatcgccaccgggaaaactaacggtagcacgctgaaaacgacctaacagagcgcccataaagtagtaggaggcccgcaagcttttaatcgccttgcttggcagtggtgcctcgacaatattggtcggatcaattgttaggacatcgcctttgaactcagacgaaacgttcatcgattttaaaattaacattaagttgtgaacatctaaaatgtctgggaccgagtcgaacctaacgggggtatccgctaatatggcagcagggataagcgcaaccgtgctgtttttagcaccgccgatcgatatctctccggacagccgtttccctccatttatgattagtttactcatcaaaaattcctcactttttgtattcgcacatttttcatgtcaagaaatatattatccaatatccacacaaaaaacaatacctatacttgaattatacaatctgtaacaattaaaacaattgttccgtacaaacgttttcatttaatgagtgctagtcgggctaatttgacgccgttttcagcgaattattacaagacaaaatgagcacctgtttgcagtaatcgataaccagcgaacccgaaagcgcttttaaaatccaacaattcagtcggtttgtttcatcactcaacaaatggtcagatctacttctttaactatccctgaaagtccttagactattcaggcatacagaaaaaaggagcggttagaaatgaaacgactatttacgacaattggcgaaaatattcatcggcaccacaaactttggatcacggtcatcttgatcatgaccatcggttttgcatttggattgccaaagattcaaatgaaaatgggcaacgacgtcttcgttagttccagttcaaaaacctatcaggattcccaaacctatcagaaaaagtttggtggtgactccctttatctgttgctcgacggtaaccagtcgacattgttatcccacaagacaatgcagcaggtggccaaatttgacagtaaagtcagccaagttgataacgtcagaaatacgaccgacatcgtcagtagtttaaatgatcagctatcccatgccggaactggaaactccagtgcccagttcaacttcaatagcaaaaagcttcaacaagatctgatggctgaactgagttccaaacaaaaacaaaacattcagtcgaaaatgcaacactcgttaacaagtacgcaacaaaatcaggttcaaacatatttgctgaaacaactcacgcccgcccaaaagaagctgatggcagcagctggtgcccaggcgcagggttccaagcaacagcagcaagcaatgcttcaaaagcaattgaccaccaaacagcaagctgcagtccagtcctacaccatgtcgctgcttaaccatcagcagcaatcacaattggctgacacggtcatcccgatgctgccgaaagttcaagacatgtcaaccaaactgctgcgggatatttttctcagcgataacggtcatgttccaagtgcgatgaagcaattattacctaaggacggcaagcatctattaatcattatcaacaccaataagaaatcgtcggatatgaacaccgcggttcagattaatcacgacgctaatcaggcaattaagcaaaccaacttttcctcaagcattaagacccgattgggcggccaacctgcagttcttggtcaggtccgcagtaaagtcattaccagtatggcaaccatgttggcattcgcagtagtcttaatggtgatcatcctcctattgatattcccggtacgaaagcgtttgttgccactcatatttgtcctggcctgcctcgtatggacatttggtttgatgggttggcttcacattccgttgaccttggcaaccatggcaacgttgccgattatcattggtttggggactgactttggtgttcaatttcaaaaccgatatgaagaagaagtcaggaaacgacaaaattcccaggaggccatttcagttgccatttcgagcatgggaccggcagttggcgtgtctttaatcgtcatggtcttcagctttttgacgatgtatctctcaaaggcgccattgatgcagcaatttggcctcacgttggccattggtgttgcctgcagctacgtcgttgagtttggactgatgttttcaagcctctcactcttggataaacacgcttcaacagctaagttggcacccaagaagctatctcagccgtcgcgtttatcactgttcctaagtcactatgctgaatgggtaacccatcatgcaggtattctgctgacaattggcgtggtgttggctggactaggcttttcatttgaaaaatccatcaatattgaaactgacttcaccaaaatgattccccaaaatatgacggccctgaagaataccaaatatcttcagagcaaaattgggtcgacaacctaccttacctatttggtagagggcaatggtcgagatatcagggatcaggacaatttgaagacaatcgatcaagttggtcaaaaagtggaccataagtaccatgacgtcaccgatgtcaccagcttatcgaccgcctatcaacagacgaacggctcattgaacacttctcaaaagcagttaactgtgggtgttgacaatttgccaacgtctttaaaacaaactttgattagcagcaaccatcacgatgcaacaatccaattcaaaattagaaacggtctgtcctcaaaagaacaacttaagttgatgaatcggattaatcatgacattaaaggaacccatcatggcttaaaaatttctcctgcaggagcccaagtcatgatgctattggggattaataatatgtccgctaatcatgatctgattattattgccggtctttcgatcattttcattgtcctattccttatttatcgggactggcgactcgcactgtacccagtcattccaattttacttgtattaggactttctccattaaccttaaaactgttgggaatttcctataacccggtcacaattgccctcagttcgctggttcttggaattggaaccgaatttaccatcttaattctggaacgctaccgcgaggaattacaacggggaattagtacccgggacgcgattgtttcagcaaccgcgtctgtcggtcaggcaattacagtttccggcttcacggtcatgggcggattttcggccatcatgttctccagcttcccagttctgaagtcatttgggctgattactgtgctggacacaggttattcactcatctgtgcattgacgattttgccggcagtcatttatctgctgcgaaaaagaaagccggcagccactcaatcctcatccgaacaggcaactgaaagtaaggattaattgaccgattgaaatacccttttctaactaaaaaatggcttccataaatgaaattgattcatttgtggaagccatttttgtgttttgcgctgtttcttggcatctttgcgccatcaatcagccgccttaattactgggcatttagtttattgatgatcgaaatgagaaacgactccaactgcggccaatcaatattcgccttgagaagctgctcttctaaaaagcccattattgtattcgctaaaaaactgatcatcagcggttgtgaagacgattgcttaattaacgttacgacaggatcattttgataggctggattgttggcccgctcgttaaacaagttctccaaaatgttccgaaattcatcatagaacttactttggctttcgggaatcaggtgacgaattaaatcaatgttgtcggaaataaaatgggtaacttgggttaaaacaacggtttccctgaagtcggtccccagcaattcttcagacaggttatagataattgtatttgccagatcaaccttatcttggaaatatcggtagaacgtgctgcggtggatcatcgcttcatcacagatttctccgatcgtaatatcatcaaatttcttttttctaagaagcgtcatcattgcctacaaaatatctcgcttggtgcgctgttgagattgggtgtcggccataatcaaagtcctttcaaaatttagattataaaattaagcatacatcataaccaactattcttaaagaaaccaatgacaactttcacaaatttgctgccaacaaaaaagccccgacccaccatgggatcagagcttcacttgaattgttaaccgtcaatcagattcaccctaaaagtgcatcgtcagttacagacggtttagttatttttttcaagatacagatcatttgccgcagcaacgaagtccttgaagagcccttctggacggttgggacgggaaataaactctggatggtactgtgaaccaacaaagaaccggttctttggaatttccaccacttcaaccaagtgattgtcaggtgaagtcccagaaatgaccatgccatttttctccattgcgtcccggtaggcgttattaaattcgtaacggtgacggtgacgttctgagatgacgtcggcattatcgtaagccttggcagcaaccgttcccggctttaatttacatggataagcgcctaaacgttgagtgccgcccatatcgtgaacatcttcctggtcagccatcagatcaatcacattgtgtttggtccgcggattcatttcagtcgagttggcatctgggtaggacagaacgtcacgggcgaattcaacacaggccatctgcatccccaggcaaacacccagatatggaatgtcttgttcacgcacatatttgatggccgtaatcatgccttcaattccgcgatcgccaaacccgccgggaacaatcaccccatcggcatctgacagcaagtcggcaacgttatccggcgtaatcttttcagaatcaagcatctccaaatcaatgtcggcgtcgacaacgtagccggcatgtttcagtgcttcggcaacagaaatgtaagcatcttggaggccaacatacttcccaaccagggtgatatgaatcgtccgtttgagatgttgaacgtgatgctcaagctgcttccattcagtcatgtcagcagctggcttatcaatgccaaagtgatcgaggatctgttgatccatcccctgcttttgcaggttcaacggaatcgtgtacaaggttggcacatcaagtgattcaaccaccgcctgcggcttaacatcacagaacagtgaaatctttttgcgcattgagtcggtaattggcttttcggaacgaacaaccaacagattaggttgaatgcccaaaccacgaagttccttgacactgtgttgtgtcggcttggtcttcatttcaccagccgctctcagataaggaatcaaagttgtatgaacgtagaacacgttttcgtcgccaacttcagtcttcatttggcgaattgcttccaggaatggcagtgattcaatatcaccaaccgtcccaccaatttcggtgatgacaatttcagcatccgaaaccttggcagcccgcataatcttttctttaatcatcccggtaatgtgaggaataacctgaacggttgctccaagataatcaccatgacgctcttttcttaggacttcatcataaatcttaccagtcgtcacgttggagtatttattgaggttgttgtcaataaaccgttcataatggccaagatccaggtcggtttccgtgccatcgttggttacgaaaacctctccgtgttggtagggattcatcgtgcctgggtcaacgttgatatagggatcaaacttttggatggtcacattcaacccgcgatttttcaacaatcggcctagtgatgccgcaacaattccttttcctaaggaagaaacaacgccaccagtaacaaaaatatatttggtcattatataatcctctcctcttgatagttagccggggaattcaaaaataaaaaaatccctatccaaaaaagtgaatagggaacaattcaatcatcgttcagatgtccttgaaactcaaggagcccaaaaaacataatacatactttttaaatattagtcaagaattaatggtcgtcttttgaattgaaatcatcatcgtcatcatccaatgaatcgtcatcatcattcaattcgttaagttgaccttcgataccatctggcaagtcctcatcgtctgagtcatcgtcaatatcctgcaagtccttgttgtacttgccaagatcttctgattcatcatctgaatcgtcgtcatcgtcggtatcgtcatcaaagtcatcgtcgtcctgatcttcaggatcatcgtcatcgtaatcgatcacgtcgtcatcatctgaagcgtcggcaagaaaggcattcaccttacgacgcttctttcgcttgggacgatcctcgtcttcttctgtatggacagttgcttcatcaattgattcataagggtaccatgttcgtaagccccaaagattgtcaccaagtgagataaagctgccatcaatgttcaaatcggtataaaattgtgataaacgatcacgaatttctttgttactatcacctaaataagcctgcaccgcattggctaaatcggcaaatggcattgtgtctccacgttgtgccaagattgcgtgtgcgacctcaatcatcgatagttcatttttgttttggcctttaaagacttctaactccaaactggtacacgtcctttcaacagtctaacaacagtctaaaaattactatactcgattaaattgtaaattgcaatcgaatattgtatttccctaataatgcatcgccggcatacagcaaataatcaattccgatgttgccccgaagcggtgcatctaaaatttccatgtccaaagcagaagtaacggtttgaatatccatcaagccatatggggttcgatagcgggcagcaatccgtttgccgtcgctaaacaataattgcagtcgattctcacctgagcgggtcagtttgacattaccgttatctgaaattttaatggtgaccggaaccccgccatcctcagtttcctcttcataccgaatatacaggctgctgcctacacgaactaattggccggtgacatcaaaaacaaagtttgatttctggccttcctgtaaaatgttggtttccaaatgaatttgaactggaacgccagttgttaaattgtccataatacaccttcttttaaatctcgttctaactaatttattatatatcccacggcaacattttgcactcatgttaccctgacgatttccggcaactttacctatttatttggtagtgtctgttataattaagaagattgtttattttatgaaacggagagttggcatatgtcttttacaaacgttccgattaccgtcatcaatcaaatttattctaaaagcaccaagctggatgcctttgcagacaccaatgccttattggaaatctgtgaccaaacgttgaagccgttcatccatttttggacgacttccgaagcaactttgatcttggggatcaatgaccgccacctgccgaagctggccgacgggctcaaaagtctgctggccaaccactatgattattttctgcgcaattccggtggcctagctgtcgtcagtgatccgggaatcctcaatatttccctgttcattccccaaccggataccgtctacacaatcgatcaggcatatgaactcattaaagggttgatcagtatgtcgtttccacaactggacatcaagagttttgaagtcacaaactcctattgtcccgggaaatacgatttgtcggtcaacgggcaaaagattgccggcatcgcgcaacgacggacaaccaatgcgctggttttgatgctttatctgagtgttaatggcgatcaagatgccagaagccaaacggttgctgaattttatgaaactgccgatgcttattcgcagtctcgttggacctttccaaaagtcgacaaggccacgatgaccacggttcaagatctcggcttcccaaatatcacgctcgaggacgtcgaacataaatttttagcgagcgttaaccagcaaaatatcgaagttgacgtaaccagcggtcctgattttatgctttcaccggctttcactcaagagcgggccaaacagttacgcaaaattcagctgagaaatgaccaattaccaattgtctaaggaggcaattttttggattacgcacatcaacagttaaaaagagaaaaggtctttcgagatccggttcataattacgtttacgtcaaatatcaagtcatcttagacttgattaacaccaccgaattccagcgcttacgtcgggtacatcaattgggaaccacgtcactgattttccatggtgcggagcattcccgtttttcgcattcggtgggagtttatgaaattgctcgaagaatcattgaatcttttcaaaagaactttatgtcacaacaacctggcgatggtctctgggatgattcagaaaaattagtcgccctctgtgctgccctgttgcacgacgttggccatggtgcctattcacacacctttgagcacatctttggcaccaatcatgaacagattacccaagccatcataacatcgcccacaacggaaattaaccaggttttacgaagggtctctcctgacttccccgaaaaagtcgccagtgtgattaacaagacctatcccaacaaacaagtcgtcgaaatgatctccagccaattggatgccgatcggatggattacctgcttagagacgcttataacaccggcgttaaatatggcacgtttgacctttccagaattctggaagtgatgcggccgtacaaagatggaatttgctttgaaatgagcgggatgcacgccgttgaagattacattgtcagtcgctttcaaatgtaccaacaggtgtatttccatccggtttcccgggcaatggaagtggttttgaaccggttgttgcaacgggcaaaagttatctttagcggggaggttcatcacgatccacagaccccctacctattactgccgtttttcaagggtgattttaacctggacgactatctccaattggatgacggggtgttaaacacctacttcatccattggaaacggtacccggatgatattttaagcaacctggccagccgttttatcgaccgaaagccactcaagtcagtcaaatttgacaagtcgaccgccgacttgttgccaagactcagagagattatcgaacaatctggatttaacccggactactacacggcgaccgacaacagttttgacttgccttatgatgcctatcaggcggacaaaaaacaaattcatttaatgcaggatgacggtaccttggtatccttgtcatccgttagcccattggttcgggcaatttctgatcgacagaccggcgataaccgcttcttcttccccagagagattttgaagccggatgaaaacgtcgatttgttccagccagaatacgatgaatttaatcgccatattcgaaacgacaaattaattaaatagctaaaggagattctcccatggatatcaaactcattgccatcgatattgacggcacccttttgaacgaaaaaaacgaactggcgcaaccaacgattgacgcgatcactgaagcccgcaataacggcgttaaaatcgtcttgtgtaccggccgaccgctcagcggagtacagccctatttagataagctagccatcaagggtgccagtgaatttgcgattacctttaacggcgcaatggcacaatcgcttgacggtcaagtcatggtcaatcacacgatcagctatgataacttcttggagaccgagatgctcagccgcaaattgaacgtcaattatcaaattgagacaaccgacagcatctataccaccaaccgcgacaccaacccctatggaatcgccgaaagcttcctggttcgcctgcccatcaaattcagatcaccagaagaaattccgcgtgacctggtgatgtcaaaggcaatgtttgtggactacccggaaaatatcactaaagccaatgacctcattcccgccaagctgcgtgatgagatgtacgtggttcaaacggaaccgttcttcattgaaatgatgaataagcaggctagcaaaggaaaaaccttaggtgaattagctgatcagctacatttaaccaaagataacctgatggcgattggcgatcaggggaatgatttaaccatggtaaaagctgccggcttgggagttgcaatgggaaacgcaattgatgaagtcaaagatgcagcccaatttattaccaaaccaaatacagaagatggcgttgcatttgccatcaacaaatacatcaaccattaatggctgagtatacgaatagaggctatgaacaaaacgttggttttgtccatagcctctttatttgtatcaatatctgttattatccttgccaagtacaatcaacaactcagcatcaaattgttcaccgcttattggggcaaactggtgaggatgacccctaacacaatcaaaaagccacccacgcccaggcaatagcgggcgtatttattaactttgattggctgatttttaattgaaccgacatcctttgccttgggatgcttgggatcattttcagcttccaagtcgcttttcttgcgaatatggaatcgccaaccggtaaataggtgccccgagccgacgataaagaccgatcccaaaacaatcaggaacaatccaaccaaaaaatcaaggttaccaagcaccatttccggcattcggaaaagaatcagcagaaaattgatgatcacaacaacaataatcgaagaccaaaccggcgattttttaaccaaatcgaccattaattctcttcaccacgaaatcgattgttgaacagcggactaaccggtttgttttcattgatgcgtttaattgcatccccaattaacggtccaactgagacctgttcaatcttatcgatttgtttttctttgggtaactgaatcgtatcagtcacaaccagttgtttgattgcagaatcttgaatccgctgaatggctgggcctgaaagcaccgggtgggtacagcaggcgtaaacctcgctggcaccggcatccattaatgcctgagcacctaaggtaattgtgccggcagtatcgatcatgtcatcaatcatcaaacaacgcttgcctttgacatccccgataatattcatgatctcggcaacgttggcccgtggacggcgtttgtcaataatggcaattggtgccttcaagaattccgccagagctctggctcttgatacaccaccatggtcaggcgatactacgacatcatcactgccaaagccttgcttaataaagtgatcagctagtaatggagcacccattaaatgatcaacgggaatatcgaagaaaccttgaatctgagcagcatgcaaatcaagggcaactacccgatccacaccatcggtctgtaacatgtttgccactaatttagcggtaattggttctcgtgaacgggctttgcgatcttgacgagcgtaaccatagtatggaatgacaacgttaatcgtgccggcacttgctcgccgcaaggcatccaccatgatgagcaattccatcagattgtcattcaccggtgcggacgttgactggataatgaaaatattgtcgccacggatactttcgtcaatattgatgcggatttcaccatcactaaatcggtcaaccgaggtcttgcctaatggaacaccaaccgtttccgcgattttctcagccaaaggccgattggaattcaaagcaaagatctttagtttcgaatcaaaatattgctgagccatatgatcctccaatatgttttttgttaactcacatctcaataacttaattatacaatgttttaattaaaattcagagttaatctttctgataaggcaattttttgaaatagccggctttatttgtctggcgggcacgggcaatcgccatgtcgtattgattaactgtcttattaatggtggatccggcagcgataaatgaatggtcagcgacttccagcggcgcaatcaaattcgagttgctgccgatgaaggagtcgtcaccaacggttgtttcatgtttgtgagcaccatcgtagttggcgaagatgaccccgcagccgacattgatattcttgccaagtttggcattaccaacgtaggttaagtggccgactttggttccctcgccaatcgatgacttcttgatttcaacaaagttacccaaatgaacgtgcttgccgattttggcttctggacgtaaatgactgtttggcccgatgtctgagtgatccatcatttcagattcttcaattagtgaagatgtcaccgtgacgtgatcatgcaggattgagtcgcgaatttcggagttggcgccaatgtagcagtcattgccaatgacggtgtggccctttaattggacgccgggttcgatgattgtatccgaaccgattttgacatcggcatcaatatacgtgtgttccggatcaatcattgaaatgccgtccatcatatgttgacggttaatccgtgtccgcatgatctcggtagctctggctaaggcaatccggtcattaacgcccattgactcgtcaaaatcatccatcttgtaggcagcgatggtttcgccctcagacttcaaaatttcaatgacatcggtgaggtaatattcaccctgagcattgtcattggtgagcttatgtagtgcctcgaataatgcctgattgtcaaaaacatacacaccggtattaatctcatcaattgcttgttcttctctagtagcgtctttttgctcgacaattttttcaacaatccccaaatcattgcggacaatccggccatacccggttggatcaggggcttgagacgtcaaaattgtcgctttggcttttttgttttggtggtaggtaaataaatcttcaaaagtcttggttgtcaataacggggtgtcaccactgacgaccatcgtcatcccatccaagttgcctaatagtttttccgcctgcaaaacggcgtgcccggtcccgagttgtttttcctgaacgacatattgcgttcgcttaccaaggttttcccggacggcgtcggcaccaaagccaactaccgttacaacgttatccatatcagctttttcgacggcggttaaaacgtgatcaaccatcgttttgccgcagaggcggtgaaggaccttgtaaagtttggatttcatccgggtccccttaccggctgccaatatgattgtgttttttgttgccattatctatttctccccaatgcttaattaaatattttttcgatatagtttccaggttgtgaaacaaccgtgttattctcagcgtcaactcgcatcaatgacgtgtagtcgccgatcgtccggccgtttggtgccgtactttctgccacaacgccgacaccgatcagattggcgtcaaactcttcgaccatcgaaatcatgccaccgaccgttccgccgccacgcatgtaatcatcaacgattaaaacgtttgaatcgggtttcagacttcgcttggatagcgacatcttttcaattcgggtggatgatccggacacatagttgacgttgacggttgagccttcggtgatttcagtatcgtgtctgacaatgacaaacggcacgtttagaaaatccgcaacactctgggcgattggcacccctttagtggcgatggtcataacggcatcaacattttggttcaggtactgagtcgcaaaaattcgaccgatttctcttagagtcgctggacttcccagcaggtcggacatgtagacatacccacccggaagataacgggtgtcagaagacatctccgcaattaatttgttgacgacctcttgggcctcttctttaagaatatacggcaaaaacctggtcccaccagcggcaccaggaatcgtttcaagcagaccggtcccccggttctgaaatgttcgttttaaaattgttaagtcttcactaatcgaggacttggctgaatcgtaacgatccgcaaaaaaggtcaacggcacaagtgtgtgtggccgctccaataaataacgggtcatatcgatcagtcgatcacttcttcttactttcaaaaattccacctcgagtttatgtaatatctatttgattttatcataaatgttcgtctttcggggaagatatagcaaaatataatcacagtttaaacttagcggcttttgttggcaattgaattataaatcaacgccgatccatagatggccgcttcgatgctggcaataaagaacgtgaccggccaattcgtgacgtaacccagataaaggccaaaccaaacgccaaagattgcaaagccaattgccaaaagcatcatctggattacggtgtgggcaaagtacttcgaactggcagccggtaatgtcaacagaacgaagatcaaaagcgaaccgacaatctgtgcggcaacactcacgctgaatgccaataagaccagaaaaataattgaaatcaaagagctgtgaatgtggttggttttggcaccaaccgcatcaaaagagtcatccttaagatttctaaaaataaaaaagagcacaaccagtactaaaacagacagggccgccatttgaacaacctcttggtgactgatgccgatcacactcccaaataaaatgttggtcgcgtaactggaatttttgttggataacgataaaaacaagatccccagcccaatgaaaagtcccgaaatggcactgatcaccgactctcgacgggattccaccgcgccgctgagttcgccaaccaaaatcgaactgactgtggtaaacgctagcatgccgtttaatggtgtccagccaatgaagattccaaaggctgccccggcaaatccaatctccgacagcgtatgggtcataaagggcatgttgcgggcaacaacgaagacacccataatcccgctgacaatcgcgattaaagtgccggccaggtacgcgttacgcataaattcaaaactaaacatattcgccctccttagaatcattatgcagctcactgattggcccagcagtgtatccgttcttagtcagccacaggaaatgatccggatattcatgaatgacctgcatgtcatgagagacgaagataatcgtcagtcccaaagtttgattgagccgcttaaccacatcaagtaactcccgcttagtgttgggatcaaggctggccgtagattcatccaaaatcaacaggtcgggatcattaatcagtgcctgtgccagataagctttctgcttttctcccccggacgccaatcctaatggccgtttggaaatgtgctcaagattaacctgcttgataacgatttgaattttttgcttttcttttcgcgacagccagggcaatttaataccggtgaaattaagcgagataaagtcttcaatggacaatggatactcgacatcaacgttacgaaattgtggcacgtagccaatttttaaaccggcttttagcttgatccggcctgctgaaggcttcaactgattcaagataaccctgaccaaggtggtcttgcccaccccattttcaccaatcacgccaagaaactcaccccgatgaaccgcaaaggttaagtcagaaagcacttggtgattggggaaacttaatgataaatcttcaaccgaaattaatgtttcactcaaatggaaatccctccacaactttgtaaaaagtaattattactattttagtttagattaaattgaatttttgtcaatcgctgttggcaaattaaaaggactgcttgaacaaaacttaagctttgtcggcagcccgttctgatttctttaaatgaccggatgtgaatcgcattccggttgggaaatgtaggcttcattacagaagccggaaatactattgtaaacgcggcgagcgcgggattcagttcggcagatgccaaaaacggtcggtccgctgccgctcatttgggagccgtcggcaccatattcaatcaaccgcgatttgagcgttttaatttggggatgaccagcagttgtaatctcttccaatgagttgccaatgtttgccacaatgcggtcataatcctgattttcaatgcctgctaataattcgtcaattggcggatgactgacagacgttgtcgcaagctgtttgagaattttgggtgttgacacactcacgtggggtttggccaggacaaaccacattttaggcagtttgggaagcggggtcacaatttctccccggccgctgaccaaggctgtgcgactgtagacacaataaggcacgtcagaatcaacctgaacgccgatttgggctaattcttcaaatgacagcccggtctcaaacatttcgttgagtgcacgtaaaacggcggcagcatcggatgatcccccgcccagtccggcagcgaccggaatattcttctcaatggaaatctccaggccaaccttaaagccaaccttgtcaaagaataaccgggccgcctggtaggccaaatttcgccggtcattgggcagaaaactgctatccgaaaaaatccgaatcgccgagtgactgctcttggtttcaatttggatatgatcacttaacccaattgaggtcatgaccatccgccattcaattgagccatccggatggacaaagggggcatccaagcccaggttcaattttgctggtgcgctgactattcgcttcacttggatcgacccccttcatttattaataacaaaattatactaaattattaataaaatgtcagttattggctgataaaaggcagtcggagcaaaaaatggccaaaataaaaaggcctcaatggccccacgctgactttgactccctgcagttaaactgcttgggatgcatcaaaatcgacctcaatatttttggtcaaaatatccgtatagctgtacgaaacccgttcaaaattcgcgttgcccggatccaattcgacaacaaaaacagccggaaacgtttccctcaaaattccccggcgcttggttgtctttcttcgcccaatttgagaagttactaggacgtgctggccgatatgatcgtccatcttatgcttgataacagataaagtcactggcattctactcacctcacgatatttaattataccataaaagtaatagaaatgcaatttttaccacaaatcacactatctggcaataataaaacactaagatttagattaaatttttcaaagtgtgaaaggcattcgccaaggtcacaaactgatcaacagtcaaattttcgggccgaacgcccgcgtcgatattgacactggctaaaacttctttaatgttgcccttcacttccggtgttttgccaaatatcccctgtaaattattccacagggtttttcgctgatgcataaaacagccacggacgaaactgataaaagccttttgatcaaagggttcaacggcccttttaacccgcggtgtcaatttaacaatggccgaatcaactttgggctgtggaataaaagcggttttgggaacaacgaatgaaatctcgacctgatttaattcctgaacaatgacagacaacgacccatagggctttgttgacggttcagcgttaagccgctcagcaacctctttttgcatcatgacaacaatcgcatcaaactgggtttcgccggtaatcaagtccatgacaattggcgtcgtgatgtaataaggcaaatttgccactaccttgagtggcttttcagtgtcaaagacgtcatcaatgattttgggcaaattggccttgagaatatcctgattaataatctcgatattatcgtatggcgccaaagtttcatccaaaaccggcagtaggttggcgtcaatttcaaaggccacgactttattggcggccttggccaactgttccgtcaacccaccgattccgggaccaatttcaatcacgttgtcggctttggtaatctttgcggcagcaacaatattgtccaacacaccgagatcgactaaaaaattctgccccaagcttttcttggcggataagtggtaacgattcaggattgcctgagttcgtgtgggactggcaatctgtggatattcagtcatgagcttcctcctgattaatctgttcaacagcggctaaaaattcatcgtgtttgatgccaaacattctaaggcgatgctgcagctgtttaccgttaacatagccgattcgcaaaatttcgccgaggcgctcccgccgttttttagcactgggattccccatgaggccgtacttcattaattcagcctttgaaatgagttcaccagctgattcatcctcagtataaacctgactcaaggcttcgcggatcgattcaacgctggcgtgctcgacacctaacgacccatcggatcgattcggaactccctgcttcttggtgataaaggcatgcttagcgttaggaacttccgcagaaatggttttccgaattttttcaccagaaaaatcaggatccgtgaacacaataatcccccgagtttgggccacctttttgatcaggtccaaggtctcttccgggatcgccgagccgcgggtttcaatggtgtcggcatcgactgctctttgaacgcgtttggtatcgtctttgccttcgacaacaatgacttctttaatttttttcatgattcctcgattccaaataaacgcagcgtattttcataggtatgcgccgcaatgacatccgggttgacatcacaaattcttgccagtgcctctaccgtgtaaagcgaataagccggctcgttttgcttgccccgcaatggttcgggtgataggtacggcgcatcggtctcaaccagcatactgtcaaacggtgtttgacggacggcgtcatggacttcatgggttttcttaaaactggcaacgccactgtatgagaccagcatccccaagtcaagaaacttcttgagccattccggatcgccattaaagctgtgcatcaccccgcggatatcggagacatccatttccttcaaaatggcataggtatcctcaaaggcatcccgattatgaaccgaaatcggtagatgcagttgtttggcaatatcaatttggcgtttaaagacccgcttttgcacgtctctgggagaagttgtttgatggtagtccaagccaatttcaccaactgcaaccacctttttgctctggagctgttcaatcaacagctgttcttgttgttcatgataatggatagaatcttccgggtgccaaccgatgattgaatacatgtcagggtattgggctgccaattccaatgatcgatcgttcagctgttgattagaaccaacgttggccaacttaacgacccccaagttctgtgcgtgcttgaaatatttagccgcttcaggataaaggtgttcgtcattcaaatgggtatgtgaatcaaaaattttcattatttgctcccaaactatttagatagaaatagggattgtgacaaaactcgcgtcttgttgccaatccctagtctttcacgatgttaactttgccacaaatcggcaatttattccagtgtgacaccattttccaagtgagatccgacggttaccaactcaacgttgccatctttatgttccacggacagtaacattccttggctgacttgaccgcgcatctttcttggtttcaggttcgacacgataatcacttttttaccaattaactgcttataatccggataccattcagcaattcccgacaaaatttgtcgatcgccgtcatcaccggcatccaagcggaattgaagcagcttgtcggcgccttcaaccttgttaacgtctttgatttcggctactttgagttcaatcttttcaaaggcttcaaaacgaacttcttttttggttaaattcaaattggtttcttcaggattaaaatcagcttcggcagcttctttcatggctgcacgccccttagccttatctgtcttggtcatttgctgtttgatgtaatccacctcatcgtcaacttcgactcttgggaagattggggtccccttggcaacggctttcacaccggcaggaacgtcttcaaacttcaaatcttcgaggtcaatgtcttctgtaatccctaattgagcaaagatttctttaggggcgtgagtcataaccggactgattaattcagcgatgacccgaagaccggctgcgagatgagccatgacagcgtcaagcttatctttgtcatcaggatttttagccagattccatggttcggtctggtcgatgtacttgttggtttgggaaacgagtttccaagtttccgccaaggcatcggagaagtgcaaatcattcattaattgcttgtaattggcaatcacggtggcggcagtctcttccaattctttgtcagcttcgttaacgccggccttgtatgcaggtaagatgccgccgtcatacttgttgatcatagaaactgttcggttcaacaagttgccgagatcattcgccaaatcaaagttcaaccggtcaatgaagtcctctggcgtaaacagaccatcattggcgtaaggcattgcgcggagcaagtaataccgcaatgcatccaaaccataacggtcaactaaagtttccgggtaaatgacatttcccttagacttggacattttaccgtccttcatcagcagccagccatgcccataaaccgttttaggaagcggcagtcccaaggcgtgtaaaatgatgggccaataaatcgtatggaaccggacaatttccttaccgaccatttgcacattggctggccaatatttcttaaagttgctgtcatctttgccgtcatagccaagagcagtaatatagttggtcaaagcatcgatccaaacgtaaaccacgtgctttggatccgacttgaccgggacaccccaagtaaaggtcgtccgcgaaaccgctaagtcttccaaaccgggttcgatgaagtttttgatcatttcattcatccgggttgccggctggatgaagttaggattgtctttgtaatatcgcagcagccaatcagcatacttactcattttgaagaagtatgactgctcgtgaaccaattgaacttcgtggccgctgggtgctttaccaccggttaccttgccgtttttatcgcggtaaacctcggcgagttgactctcagtaaagtactcttcgtccgataccgaataccagccggtatattcacccaaataaatgtcgccattgtccagtagtttctggaagatatcggcgaccgctttttcatggtaatcatcggttgttcgaatgaatttggtgttggaaatttccagctttttccaaagttgtttgattgatgcagccatctgatcaacatagtccttaggcgacatccccaactgttctgctttttgttcaatctttaatccgtgttcatccgtccctgtcaggaagaagacgtcatagcccattgcccgcttgaaacgtgcttcggcatcacaggcaattgttgtgtaggaattgccgatatgtaacttcccggatggataataaattggtgttgtgatataaaatgttggcttactttctgccatgaaagtacctcttttcatgcttaattattctttaggatattacaatccagtatagcaaatattttttggaatggcgatgagaattggatttgggtgagatggtcgtagtcgaagttcaatatcgctttgaatcggtggtgatttgcttttacctagtgataacgtgctcaacggagcagcaacctgcacctaagtatggtcggacaaaaatcaaaatgattttcatccaaccacacttaggtgcaggttgctatgcgctccggatcgcagtcatttaaaacaaatccatctgcaccggcgacaagccgccaaattcaatccccaacatcttctttaactgcagggcgttgtctgctgcgtccccgccgctattattattgaagatgacacaaacttctttggcctgcttgtccagatccaggaccacttttcgaaaagctgccagttcttcttccgaataccggtacaacgtccttttcccgcgccaatctgctgactgctccgtccagcctttgacgtttcgaccgtgaagccgcaacaacgccagattctccgttgtcaccagcggttcgaaaggcacgccggcattggtggtatgcggttcgtcaaccgccaccaacgtcattcccagttcgctgagatagccggcgacgtcatcggtaatctcgtcaccataccaagttgagttgcgaaactccactgcaacaggatatccggccatcaactggctaattcgacgcaggtactgaatcgtcgcaatctttctggcaaagtatggcggaaactgaaacaggatcgccttgagctgaccggtgtccattaatggggcaaccgcccgcttgtattcgttgaaagccacaaaccgctgctcattatcaaccgggtcggcgctgccctgatcgtgcatggtcatcacccggttggccttcaaaataaattgaaagttatccggtacctgtttttgccagttggtgatcacttcaactttgggaatcgcataaaacggcgtgtccagttcgacgaccggaaaatacccactgtattcagttaagcggactttacgtttagcaccgtcgatcagtgaaggatgctcggaaaacgtcgttaacccaatggtaatcaatcagcccacctcccggctgtttagacatttaccgtcaaatctttgaagaagtcaacggcattttctttgaccatcgtaaacggaaaaccaaattgaagcggctcttcattaaccgccagaactttggcattttgagaacgataatcaatcaagccggcaaacgggtagacccgcattgatgtgccgacaatcacgatcagatcagcttgggacactgcctcaacactcttggaaatggcaactggatcaagcccttcaccatataacacaatgtctggtcgtaaaatgccgccacagttttcgtgatacatactctttaaataatccttgtaattgactgtcttgtggcacttctgacaatacactttgtacagattgccgtgaaactcgactaaattctgcgtgttggccttgcggtataggctgtcaatattttgggtcaccacaacggcattgcgtttctgggtaaactcagcctggcgctcatgaatcacgtttggcttggcatccgggtaatacatatttgatttttcgtactcccagaaaactttgggttcatcacgaagacaatcggtacttaaataatactcagcgggtttatcagatttgtcattggtgtacagcccgttctttgatcgatagtcaggaatccctgatgccgtggagacaccggcaccagtcaaaaagacaattctttttgcgttatcaaattcagcttgcagcttagaatcaatcatcgtattcctccttcaaaagttcattacttgcgaacgatataaggcattttaagatcgtcgaacaactgcttgacgcttttatcatagacccctttgaaaaattccggatcgtcctggttgcccttggggttggccagcacaaatgagttctgatcatctacccggttaaagccgacgtaacccttggtgttgctggtaacctcggtcaagtcggaatgataaatttcaaatagctgtttaactttcaatcccagttgccgttcagacaaaacactggtaagggtggtgaactccgtgttgtgcagagccggcagttcccagtcctttaactgttcatcaaaggctttaaagagcttgacgacgttgcgccgcaatccaaatggtgaatcggtcggcttatcggtgatcacttgatacaacttttgggcagcctcaaaggaaaccgggaaatcctgtttgaatttgtcagccaccttgtcaattccctcgccgtaaaagaccagcgcatccaataacgtggttaaccgtaacatcatctgatcgtccagtggatccggttcaggtttgatggtcgcatatacgcctttgagatacatctcttcgatgtcgtcattgatcaaattgtgctttcgctgctcggacacaaccacaaaatgagagacaatgtcgtagagttccgttcccatcatttttaattgttcatccagggtatcatcgccagtggtcagtgaataaaagacctgcggaaagccgcggaggaccatcaataggtgcagcagttcatgtgaagccgtgtagtcgggagcacttaagtctgcgatttggacgatgatattttttccgtcctgaaccgtttgggcctgatcgtgacgtacatatcctgattgcagcttgccgataaaagtcaccgttaccgtcccgggaaagaagttattaacggcgtcaattaagccgtgaacgtctttgtttaactcgatatcaatattgttatccatcatgttctcctatctgcgaagtgtttttaaaatttctttaactgtttgtgaactgggatgatccatcccctgaagctttcgaacaacaactggcaactcctgcattgtggttccatttgaaagcgctaaggaccttaattgaagattcatatggcccttttgaataccatcggtcaccaaagcttttagggcagccaagttttgagccaaccccagtgcggcgaccacctgcatttcctcacgggaattgccgatctgagcgatctgcttgttaatgccggccaacggcaaaaccttgctggcaccgccgacaaatccgattgggactggcagcgacatgcgtcccaccagttgatcttcgtcaatctcccatgtactcaagccttgatacgacccacttcgagccgcaaacgcatgagctgcgctttcaactgcccgccaatcattaccaaaggccatcacggcggcgtcaacaccattcataattcctttgttatgcgtcgtcgcccgccgaatatccaactgggcgacctgactggcatcggcaattttttgggccacctgagggccagataacgacttggttcctagtttggccatcgccaccttaccggaaacttcaacgatcgcttgatcaacgaaattcgttaagattgccatcgtggtttcaaccgtcaactgctcagaaagccaattcgacacagcttccaacatcgtattgatgatgttggcgcccattgcctcaccggtatcaaccagtaggtcgaccgacaggaactgcttagagagaatccggacatctaggcctttggcacctccaccatactttaaaacgcttggatgactctggtctgcaatttgaatcagctgctgctgataatcatgaacaaactttgtcacctgatgaggatctgcgtctttgacgatgatctggccgctcaccaggttatcaggaacactgcaatgaatgcctgctcctgccgataacagtttggcaccattgctggcagccgcaatcactgacggttcttcagtcaccattggtaccaaatgttcgtggccgttgacaaccaggccaactgcgattccctcagggagtggataatccgtcagattgttttcaattaattctccggaccttgggttcaaggaccgtccaagcaaatcgagttgagcctttgataaattggcagcttcagcgatcagcgaaagacgctgctcgtaagactttttatagaaatgatcccgtttattttccatgatatcaccatcatctgttagaggcacaaaaagctggtacaattgccagctttactcgatgccgtattctttttgaatgtactcggtaatgatgccttctctgacaccactttctgaaaataagacttttttggcatcaattttgtccattaaaacaatcaacggcaacaggccgccgacaataatgtcggcccggtcgtgctcaagcccctgaattttccggcgccgattgacgttgcccttcaataaattcagataggttcgattaacttgttcagcagttaaatgataaccgtgaattgcatcaattcgaaccatattttggcgacggcgattgattctcgccaaggtccgattggcaccgcccaagagaactaacggctgatgggccgcacgattcaaccaatcaattcttgaataaatcttcctgatattaaattgggcgttaaataaattcgcaccggtaatattatcatttaaatgatatctttcagtgatattcactgcaccaattggaatgctggtgagatttgagcttttgccctcattgacccgaatgagttcacaactggcgccgccaatgtctaggatcagacaattcctgattcctaatcgattaatcacgcccagataatcgtaataggcctcttgattgcccgaaaggacctgaagcgaaataccaatgcgctcagaaacggcctttaaaaacttcgcctggtttttggcttggcgaacggcggccgtggcaattccaatgacccgtttggcttcatattgagaatagatttgtttaaaatctaacagtgacttaatcgtccgttccatggctgccggctggaggatcttgcccctgcccatgccttcggaaaggcgactgtcacttttgatgcgtttgatttcacgataactgccatcatcagaaatttgattgattgccattctgaccgaatttgagccaatatccaaaattacaaggttttccatccctgccaccctttctggacatattagtcaaaatagttaatgccaatggcatcgcgaacttctttaagggtttgattggcaacctcgttagcgtgttcactgccctttttgagaatttgatagacaccctgctcatcttcagcgtaacgctgacggcgctcacgaattggtttgagttcggcttgcaagacatcgtttaagtaacgtttaattttaacatccccaaggccaccatggctgtattgatcttttagttcctgaacttttcgtttgtcaggatcgaaaatatccaagtaggtgaagaccgtgttgccctcgacttggccgggatcttcaacgtgaatgtgatttggatcggtgtacatggacatgacctttttttggatggtgtcttcatcgtcggccaaataaatcgcgttgcccaaagatttgctcattttggcattcccgtccaagccgggaattcggcccattccctttggtgggaaataaccctctggctcgactaaaatgtcatcattataaacggagttgaaagttctgacgatttcacgggtttgctccaacattggttcttgatcgtcaccgaccggaacagttgtggccttaaaagcggtaatatcagcggcttggctgattggatacatggcaaagccaaccggcacactttggccgaacttcttttgtttaatttcattcttaacggttgggttccgattcaggcgggaaacggtcaccaaattagaataatgctgcgtcaattccggtaaagccggaatctgggattgaaccaggatagttgatttttgggggtcaattccaacggccaaataatccaatgccacttgaatcaaactgtggcggatcttttcaggatcacgggcattgtctgttaatgcctgcatatcggcgatcataataaatgtttcgtagtccccagagttttggagctcaactcggttctttaatgagcccacataatgaccaatatgtagtttgcctgtgggtctgtcacctgtcaaaataattttcttcgtcattgtaaccatcctttcaaaaaacgccctattgctttaacaataggacgcttatacgtggtaccacctaaattgtaacttatatcaagttaccgctcgagacgatatgggcgtcaccctttacatactccaattcgtttcgtcgtggccgttttcagcaagtcgacctctctgttgctgacgattctactcagtttttaataacaatctaattttactgataaaccgctaaaaagtaaaccccgtttgcgggtaaaatacgggaagttttggcttagtatcctgcagataaatcaaccttgttcacagcaactttgccggtttggatgaagctggtcaggttttgatacaaaatgccaaatgcctcatcaccatattcttgaaagccaccggaaatatgtggcgttaaaatgacgttatccatcccccagagtggtgaatcactcggtaacggctctgattcaaaaacgtccagcccggcaccagccagttggtgttggttcagtgctgcaatcaacgcctcggtgtccaccgatggaccccgaccgacgttaataaagattggctggttgcgcatttgatcaaagaacgcctggtcgaagaaatgatgagttgccggggttaatggcatgatattgatcacaaaatctgccttggcagcttgcactactccttgatcgtctccaaccacttggtcaaaatgagccgtgggtttgccatgccggctgacgccaaccgttttggtaccgaaagcttggagcttttcggcgattgcccgaccaatatggcccgttccaaaaatcaccgcggttcgatttttgattgtgtagttctgcattcgaacttggtcaccgagccacttttgatcacggcgggccgcttgagtggtgacgatgcccctggcaaatgccaaaacgtaggcgatcaccatttcactgatgggttcggcgtggatgccgctgacgttggccaaggtaatttctttatccgcgaagtcgttcaatggcatgtagtcgaccccggcagaatttgactgcacaaatttcagcttcggcgattcacccagcacggtgcgggcttgctgattccaaccatagattgcatcgacacttttgacattgctggtattcaaatcagccggttcgatgacctgcacatcgccaagcgctgtgagtttggcctgctgttcggccgttaaattgaataaatccagaatcttcatggtcccatccctttcattcgtcttgatctcaataaaaagtatacgcttgaaattggttcaaacaaagcaaaatccccaccccacattgaagggcaacacaattgacaacggggttaataccaactaaaattgtcgaagcattcttaattcacagtcgagtcgaatccgaatggaggaacccttttggaaaataatgaaaagcaaatcgaacagtcacgtgtggacaaagtggtgaccaaaattgaccagaaaatcatcagcacggatgacgaacttaaccgtgcccacgcagaaaccaaaaaggttcagcagacttattccgacaatacctcggttaactattttgaggtggatgatcgaattgaaaccagtgccgaactccagcagcagcggggtttggtttctcgtttaaccgaaaatgaaagcatcttaaaaaatcagctttcaactttgaaagatctcaaaaaatccccgtactttggccggatcgatatccaagacgatgacgaggacgaaaccgaaaaattgtatatcggcattgcttcatttgaaaatgaagacggtgagtttctggtgtacgactggcgggcacctatctccagtgtttactacaacggcaccctgggtgaagtcgcttatgataccccaatgggccgacagcaaaccaatttaaaaaagaagcgtcagttccaaattgtcgacggtcaaatccgcaacatgtttgacaccaacgaaacggttggcgatgaaatgcttcaaagtgctttgggtgaacaaaacgacgaatacatgcaaaatatcgtcgccaccattcagcacgaacaaaacgatattattagagataccaccagtaatctgctggtggttcaaggggttgccggatcggggaaaacctccgccattttacagcgaattgcctttttgctgtatcatagccgcgatacgcttgaagccgaccaaattattttgttctctccaaataaattattcagccactatatttccgaagtgctccccagcttgggtgaacgcaatatgcgccaagtcacctttgatgaatttattgataaccgactaaagggcctcaacgttcaaagtttatttgaacgatacgaaactgatggtaacttgaccgaacagcagcgattggttcgcggcttcaaagaatctgccaaatttatggacgaactccaggaatactgtgataatctccagccagcccaaatcttcttcagtgacatcatttttaacgaatcaaccttctttagcaaacaggaaattcaagacattttcgacagttttcccaaagcagccaaagtttatgatcgcttcttacacaccaagaatgaattgatcaagcgactcaaacgccggatcgacgacgaaaccaaggctgattgggtcaacgacgaaatcgatcaaatgagtaatgagaagtaccacgatctcttggccggcaaagagctgggtgagttccaaaatgaagatgccgagcgcttcttcattgcccgaaaaattgtcagtgcccgcctgcgggtggtctacgatgcgatctttaacgacaacttcttcgatgcctacctgcagtacgccgacttcttgaaaaaagtcgatctgccgcaaaacattgaaacgccgcagtggctgcagtccgttgacgagtttaatcattcaattgaatttcatgccatcaaattggacgattgtgcgccgttgctttacatgcgcgactatatgtctaacagcggacagaacaacactatgaaatacctgtttgtcgatgaaatgcaggattattcagtggctcaactcaaatacctgcgctacgcctttccaaagacaaagtggacactattgggcgacagtgagcaggccctgttcaaagacgttgaacagccaaaagaaattcttgataaattaaacgccgctttccatgtgcgccggtcccgactaatcagtttgatgcggtcgtatcgctcaacgctgccgattaccaactttgccaaatccattttgcctaacggagatgacattgaggccttcacccgccccggcgacattccggaattggttttgacatccgacttcaatgacggcatcaagcagcttgaaaaagtaatcgctgaccaacgcaagcaatacgccaccgttgctgttttaaccaaaaacatgaccgaggcccagcaggtctatgaacgactgcatgccttaggagatgttacgttattgcaggatgcggacagaacacttccaaagggcattttggtgctgccaatctatttggcaaagggcttggaatttgattccgtgatcgcttgggatacctctgagaagaactattccgatgaaagtttgcttggaaccctctacacgattatcacccgggctatgcaccacttaaccttgatcagtctgggcgacgtaaccccgctgatttccgatgagagtttaactgatcgcaagattaaaatcgaaaaaaagattcggaagtaattggtgtgaaaacatctgattataagcaaacccggagctgtggtcattgatcacgctccgggttttttagtttcacttagattgtatggggatagacactgttcacttttatctcgcaaaaacgtgccccttgagccagctttctcttgattacactaatgctcagaagctaaacggctcaatcgcactctagatcaaatactgcacatcactcgccagagttggataagcgagaatttcccggttgaagtcgccgattttcatgtgctgatcaatcatcatcgtcaaaatattgatcaaataatcagcgtgattactcaacacggtggccccaacgacagtttccgtatcgcgattgatgaccactttggccttggcgagtggctcattgagtcgatgataactgtaccacttggtcatgtcattggtaatcagcatatagcgactatcatccgtcgcgatattcgatggcagtcccacttgaccgagtgagggttggccaaagacaattgtgggaatagatttgaattgaatcggatccgttgacccgttaaagtagccggccaagtagccagcttcaaaaccggcaaccggtgttagcttgggacgtttggtgctgacgacatctcccatggcaaaaatctttggatttgacgtctgcaggtggtcgtccacgatcacaccgtgttggtcggttttgacaccaacattttggattccaatcgtatcaacgttgggaatccgccccgccgtgcagaagaccatgtcagtcggcagcttaaaattgtctccggataaaacaaactgctcgcccacttgggtaatttcttgaacacccgtattcaaatgaaaatcaacgcccaacttggccagtctatcaacttcttcgtggactaattgttggtcaaactgtttgagtggccgatcgttatgatgaatcaggtgaaccgtcgctccggccgcgcgggcaatcccggccagttcaaagccgatatagccaccaccgacaaaagtgacgtcgtttggcagatcatcgaggttcaaaaagtcggtactggttttgaaaaattgactgccgggaatatctaaaattcttggccgctgaccagtcgcaataacatattgatcaccggaaaggctttgatttccagccgtcagcagcccatctgaattgaattgggcatgctcatgatacgtgtcgaccccatctgaaatcaacccgttgttggtggcatcagaaattggattggtatactgccgcttgtggcacatgagatccggccaattaaccgataccgagccactgatcccgttaccctgcatatcattgacaacttgagtgatctctaaaccggacaataaaattttcttcggatcgcacccgcgattggggcaggttccaccaaacaaattgtcttcgacgaccgccacggttttgtgctgtcttctgagtgagtgggccaaagacccgccggcaaccccgccgccaagaatgacgacatcatattgttttgtcatttagtattcctccataagcacctaattcatcgttgattgacgatttcacacgactaatttcataatcttaaatccattgtagaacacttcggaattatttccacgttgccttgattgacaactccccacggaatttgtatcttagataatgtaattaaaattttattaaattgaggtatatcatggtccatgcactttggcgtcaatttccgcgcattaatttaaaactaattgctttggaaccctatttgttaaacgccgtcaatcttcccaaccagcccattcatcataagatcagccagttgctcaaatccggcggaaaattcctgcgtccgggcttcttttacatttattcagaatttggtcaagaggtggatccagctaaaattaaggctggtgccgccgcagtcgaattactgcatgtggcaactctgattcacgatgacgtgattgatgagtcgccgatccgaagaggcatcgagacaatccatactgaatatggccaaaaaaacgccatttatgcgggggattacctatttacctgttactttacccaggtgctcaaatcgactcaggatccggctaatatgaagcgacacgttgatgccatgcaaaccattttagccggcgaattggatcaaatgaaatacaacttcaatcaacaaatgactgaggcagattatttccacgaaattaccggcaaaaccgccgaattattccgcctttgtttccagcaaagtgccttggtaagccaagcttcggatcaaattttcaaacttggcggcgaaattggtctaacgatcggccaagcctaccaaattttagatgacatcttggattacagcggtgatccccaccagaccaagaaacccgtccttgaagacctcaagtccggcgtttacaccctcccattaatttttgccctgcagacggctcagaagcaattaaagccactgctggataaacgtgaacaactgacccacgaagacattgcccaaatccaagccatcgtcgttcagtcgggaggattgcagcaagcaatccaatctgccaatcagttaaccgctaaagccgagaagctcattgcccaattgcctgagcgaagggccaagcgcgacctccagaccctgacacagctattattaaccagaaagcaataatttattttgaaatatcaattgccacagccagaggacagatatctcctggctgtggcaatttttgcgtttgatgcggttgattgagatgtgtgccgatgaccctgccccctactgtgtaaaaccaaccgcccaacgatgaaccaaacccgttcatcctttggcggtttgctttacactccggggccacccgggtctcgttacactcttcctaaatgtgtgccgtcgaccctgtcccctactgtgtaaaaccaaccgtccaacgatgaaccaaacccgttcatcctttgacggtttgctttacactccggggccacccgggtctcgttacactcttcctctgtccaagtcatacagctgtctgaatcttggctgagtcttatacagttcctgcggggtgccctgcatatcgaactggccgttttccatgaaacgaacctggtcgacgtgggtaatccctgccaaatgatgagtgacccaaataatggtcttgtcatgaagtaattcaaagactttatccaacaacttcttttctgtgatcggatccaaacttaccgttggctcatccagaataataatcggtgcatcctggagtaaaatccgcgccaatgacaatcgctggcgctccccacctgagaagcgtttaccagcctcttgaacttgggtgtcgtattggtcgggcagcgactcaatcaactctttcagtccaacggcggcaatcgcatcttttacctgctggtcactggcattcacgttccccaagcggacattgttcatgaccgtcgtgtcaaaaagatacggttgttggtcaagaatgccaaacagtgaagagcggacgtcctggaggcttaaaatattttgctggttaatcagcacttggccatcggatggtgtcaaatctccaacgaccagcttcaagaaggtactcttcccagttccgctgggtccaagcaatgcgaccttttcgcctggatgaatggtcatcgagatatgttgaaccacgtctcgatcaccatcggcatacttgaacgtcaaatcgttaattgaaagttccttgaacggttcagccaacgccgtctgcttaacgggtttgaccgtgcctgaatctagggcgttaacccgctcaatcgaccgtttataaaccggccactcactggcaccttgactcatgttgacaaatggtgacaccgctgggaaaatggccagcgcaaaggcagccacccagttggccaaggatttggaggcggtgaactgattagccgaccagaccagcagaaccaaagtcgttagtaaaataacaaattgaaccagaaatgatcgccaccactggaagtaatgatctcgtttccgcagggctgcaatggccttaattggtttcttctgcaggttaatgaagtcgttgtaacgaccggaaatcagccagtcgcccaatcccaaaacttcatcggttaaattcgtatagaattcgtgttgaatttgatgctgtttaaattcccgaaccccgttggtggcgactgacgccaaaggcatcacaatcgtgataatccctaataacagtaacatcagtaaaccgaccacccagttcagtgaaccgacaccgatcaccacgaaaatgtacaacagccaaccgattaccataggaaaaacggttcgcagatacaagttttcgatgtgatcaatatcgtcggctaaaatactcaagatatcaccggtttggtgagagcgttgaatggccgatgccttttgctcaacggtttgatacagcttttttctgaagtcagacacgattcgcagcacccaattatggctggttaaccgttcaacatatcgaaagactggccgggcaattccaaaggctcgggccaaaacaaccggtacataaatataaataatacttgaaggctgtctggcagcctcactgatcagatatccggagttaaacatcaaagcgccgccagagaagaaggtcatgaatcccaggaataagaccaggaccagtaagcccttgtatttacgcaggtaaggcatgacccaggtgtcgttttcgaatgtttttctaaaatttttcataggtctgccgcctccatttctgaacgaagtttgacgtaatcaccatttcgctgagcgagttggtcaggtgtcccctgttcaaccaagcgaccatgatccatgactaacacatagtccatctcaccaatccagtgaagccgatgggttgcgaagaacaccaggtgatcattgaagacgggcagaatatcctgcttcaaactggcttcagtttcaatatccaaatgagcagtcggctcatcaaataagagcacttttcgattgggatcaagaaaagctcgggccaaagcaatccgctgtgcctgaccaccactgaccgtccgggcaccctccccaatcatggtattaagcccgtccggcaaggtattaatccagtcggtcaggcccgccttgtcagctgcatttgaaatcgcagcttcagtggcatccgcgacgtaaaacgaaatgttatcggctaacgtggcgtgaaagagatagggattttgaggaatatacagaaagtttttctgccaattagcttggttcaggtgtggcagcggctggccgttaatcgagatttgattttgaccatccggggacaaaaagccaccaatcagattaatcaaagtcgatttgccggatcccgatgcaccgatgatgccgatcttctgcatccccttgatatcaatcgaaatatctttaagcgtcggttccttgcttcccggataggtcaaggaagcttgattcaatttcaaggttgaatcgttgttccatttcaaatcaggcaaaacttcgcgttggctcatctcaggctcatgaaggacgtccaagacggcgctcatcgcgttcttaccgttcaaagttgcgtgatagtcgttggcaaaattccggattggcagaaaatactccggcgccaataccaaaatggtcaacgcgggtaagagcatgactttaccatccatcaaatcaaatcctagaaagactgcgacgactgcgatcgacaaagtggtaaagaaatccagggcaaatgtcgatgttaaggcgattctcaacgtggacatcgtttctgtccgataagattcgctgacttcatagacattgtcagcatagcgcttagaaaggcccagctgctttaaagtcggcaggccccgtaaggtatccacaaagtgattagacaggcgctgatagccttcatattgccgatctgccttactctgagctgccagtccaagaataatcatgaataaaatgataattggaaaaatagcaaataagaaaatcgcttgttcccaacgcaggaacaggacgtataacaaaatcagccacggcgtaatcgacatatccaagatcttgataacaaccaacatcaaataagtctgaacctggtcaattccttcaagggccatcgtgacgatgtttccagttccccgtttatcaatttcagcgggaccgagtcggaaaatcttggccatcaaatcttcccgcatatcgccacttgtcttttcaacgaacggaaataatacgtggttttcggcgacagtcaacaaatgccgccctaaaaatgcaacggtaaacacaacggtgggccaaataattgtgttgatcgactgcagattccacaggttcacgattgcaattgacagtgcgcgagcctgagcaattattgcgattgcctgaatgaagaccagaatccctaaaataacggcatactttttcatccccggcagatcaaacaatcttttatcaatcaaacttttcactcccccagaacaaaattaattacaattcctagtataaagaattattgcgcacaatgaaatatgtgagcggtttatttcttgatttatttggtttttaacacgagttaccgccaaaaattccgggcaaaacaaaaagaccagcgataagccgaaacgtttatcattggcctttcagttgatacgcatatcattaactgaaaatcatttacccggatcgttggattcagttaaatactattcagcaacttgctttggtgacttgattcgcttgtagaatacccagtagctccaaatgaagtagatgagcacaattggtaaaatcgtgaatgtcaaaatcgtcatcaagtgcagcgtatatggtgaacttgaagcatttttaattaagattgaatttgcgttgttcgtcgcaatcataacccgtgggaataaaccgttgaaaatcaggacaacgacactgattaaagaaagcccactggcaatgaatgatgtccaatcatggctggactgagcgccccaccatgcagccaaggtaaagatgaccaaggcgatcaagattccccaagttgacattggtttacgagtaaagaagtcagttgttaagtaaagtaagataacaaagacaacttcaccggcaagcagaaccggatagagaactttactccacttttctgctcgttctcttaattcaccgctggtcttcaaacgcaggaagtttaatccatgaatgaagcaaagcagtgaaacggcgacaccgccgacaatcgagaaccagttgacataagtggtgaaacttccaaagatatccccatttttatcaatcggaacaccttgaatcatactggtgaacatcatcccgaataagaatgcggcacagaaactaccaattgatgatgcccattcccagaaattacgccaagtatccgtctgcatatttgcacggaactcaaatgaaacgccacggaaaatcaaggcaaccaagattaagaacaagacaaggtagtatcctgaaaatagtgaagcataccacattggaaatgatgcaaacatcgcaccaccggcagtgatcagccaaacttcatttccatcccaatgcgggccaattgtttggatgacggtatcacgttcagcccggttcttagcaaagaatcgaacggacatcccgataccaaagtcaaacccttcaaggaagaagaagccactaaacaacacaccaatcaatagaaaccaaataaattgataactagtcattatgagccgcccccatttcgtatggatctaccttttgatcagctgcttgtggttcgctggagtatccgtcagtctgaactgaatccggtccttgtttgagaacccggtgactcaggataatcatgacagctccaagcgatgcaaagatcaagaagtaaacgatgttggtgaacatcaggcttgccacggtagacgttggcgataccgcatcggcaatggtcaaaagtccgtaaacaacccatggataacggccaaattcagtaacgaaccagccacaggtgttaacgataaacggcagccaaaccatcaagcccatgaggtataggaaccagcgttgcctcataatgctttgtgacttcttacggttgaaccataacccaatgatggcaactaagccgaataagccggcagaaatagccatgattcggaagctatagaacaaagtacgagttggaacataataattccgtgtttcaccatttttattgtactttgcctttaattctttgttgatctgttgttgacctttgaaagttccgttcaaactatggtgaccaagaatattcaaaacataaggaacctcaattgaccaggttgtcttgtgattcttagtaccctggatcactgaccaattgcccttttgagttgagttcttccagaggccttccatagcagcaaacttcatcggttggttattaatcaggtaacgtgtttgcgtatcacctgaccatacagaacctaagcaggcacaaagcccaatgatgagtgaaaccttcattgacttgcggtagaagtgctcatgatccttcttaagtaaacgccaagcagaacagccggcaacaacaaatgcagccgttaagaatgccccgaaaataacgtgtggaaattcgttccacaactgacggttcataataacagcagagaaactggtcatttcaactttgtgttgagcagcattcattgcgtaaccaactgggttttgcataaagctgttggccgccaaaatccaaagtgcagatagtgtcgaaccaaaagcagtcagccaaatgaacaaacagtgaaccactttgttgaaacggtcccacgtgaacatccaaaggccaatgaatgtcgattccaagaagaaggctgccaaggcttcaattgccagtggcgcaccaaaaatatcccccataaatcttgaataatccgaccagttcattccaaactggaactcttgaataataccagttacaacaccaacggcaaaactatacaggaaaatcttcccccagaattttgtcatgtttttgtatgtttcatccttggtcacaacgtaacacgtttccataattgcaacaataaaagctaaaccaatggaaaacggtacgaagaagaagtgaaacacagtggtcatcgcaaattgaaaccgcgacaacccaagcatcgtgacgccaatatttaacattgtcgtatccccccttactaaatattaatgagttatcctcatatacccttattgtatatagaaatggttcaacattcaatcaaaatactaattaattatcagcaattactcataatcctgcactgttattgacacaatcccgcccgaaacatgtaaacgtcgtcaatcaatcaatgtgaaggacttagattagggaagaaatgcttgtgaaattattgcaatggctttcattagacaattgtcaaagccacatttataataagggtgataagattagtttatgctattattgtaattttctaaagcaatcttattttaattattccaaagggggaaaatttcatgacaaagaacatcgtcgtcattggtgccggtttcgcaggcgtttacgcaaccaagcaattggctaagcgattcaagagcaactctgacgtccaaattacattgatcgatcgtcactcgtacttcacttatctgacccgattacacgaagttgcgaccgagcgggttgacccaagcagcatccagtatgacctgcaacggatttttcacaagcagaaaaacgtgcagctcgttacggataatgtcacgtcagtcgataaggacaagaaaattgtcaacggtgaacatggcacgtatccatttgacagcctgctgatcagtatgggtggcgagcctaatgacttcgggacacccggcgttaaagaaaatggtttcacgctctggtcaatggaagacgcactccgacttcgagcgcatattcgtgaaatcattggccgaggagctgttgaacgtgatcccgacaaacgtcgtgcaatgctcacaattgtggtctgtggttccggatttaccggtgccgaaaccattggtgaattaattgattacaagaaagtcctggcaagagattacaagctggatcctgacgagattcacattctcttggttgaagctgccccaacaattatcaacatgcttgatcgaaccaatgctgctcacgcagagaagtacatcaaggatcacgacgttgaagttcgaccatcatccatgattacctcagttaatccagacagcgtcgacattaaggatcaggattcaattccaaccaacaccttgatttggactgccggggttaaaaccaaccacgttgccgacagtttcggaattgacgccggccgtggcggtcgattgattaccaatcaatatctccaggcaaagggctttgaagataaaagtatttacgttgccggtgatgactccaacgccactgagcaaggtgctgaacgtgccgttccacaaactgctcaagaggctgaaaatgaagccgttgtttcctctgccaacattgctgctgacattgaaggcaaccacaactacaccgaattccatgacaagaacatgggcttcaccgtttcatttggtgctcgttatgggattgcccaagtattcggcggcaaacgagtccgtggctggctggcaacgattatgaagcacgggaccaacctcttgtacttcatgcgaattcattccggttacttcatgatgcagtatatcttgcaagaattcttccgggttgataacaaccgaactgtgctgcctggtattactgcccgtcaggggaacgctttgtggagtgttccgctaagaatgttcttgggaatcgtcctaatggttgatgcattctcttacaacgccattattccagtgggctttggcctgactgcgattgaaggcattattggctgcctgttgttcttcggtctattcacttggattgccagtttggcattaatcgtgatcttcttcatggggattgccagctggccgcatgcttggatcgtctttgcggcgattgccttaatgaatggatccggtcgttccattggtttggactactggttcgttccatggctgcaaaagacttggggccgttcacgttatggcattccaaagtcactttacaaaaataaataaccgttaaatgaaataagaggctggaacaaaagattttgttccagcctctatttgtgtctgaatgttatctagcacttatgattcagcttgagtttccggtatctcaacaatgtacttgccataatgaggaacatcgacaatttgaatattagtctcaaaaatgttggctagtaattcacgatcgtagcattcttccggtttgccgacttttaccagttcaccccgtttgaccagccacaaaacatcactgatcttaaatgcctgattgatatcatgaatcaccatgataatcgtgatgtgcttctgctcattaagctgcttcaaaatccccatcagttcggcttggtagtgaatgtccaagtaagtcgttggttcatccagcaatagatatgtcggatcttgggccaaagcggaagctaaccagactctttggcgttggccgccagataacgacgacagcggccgctgtgccaatgatgtcaaatgagtgacctgaatatacttggccacctcggcgtcagaaattgtcgccagcaggccgtggtgtgccaacctgcctgttttaacaacatcaatcactttcatatcatcaaaaatatcgttttgctgactaacaactgcaaccttggtcgccaactgtttccgaggaatcgaactaattggctgcccgtcaagatcaacttcaccaccggacggttggaaaatgcccgccatcaattttaacagggtcgacttgccggcgccatttggaccgataatcgatagaatgtgccccaccggaattgtcgcactgatctcatttaaaagggtcggttgttgtggataatgataactaacttgatttaagtccattaaaattcttcctttgcaacatcaagattaagaatgggccgccaatgacggtcataatgaccgcggcggacaattcactgggcaacacgacaattcggccgatggtgtcaacaactaataacagccaagcgcccatgagcatcgacagcggaatgatggtttgataatctctccccactaaataacgaacaacgttggggacaacgattcccatgaacggaaccgtgccgacaactgaagaaacgccggaggataaatagacaaccaccaacagcaatgccagacgcatcatcgaagccgaaacccctttggtctgcagctgctcggttgataatttgagatagttggcccacggtgaaataacgactgccgcgaacatcccactgacacccaaaaataacagtacttcggtctgcgaccaggtaatcccgttaaaagagcccgtcgtctggccgccaaatccattggcaaacagctgctcgaacccggtaaaggtcagcatcatcgccacaccaatgataatcagccggtatgggctcttgagtgccggcccccgggttaacagtaagagtgcaaataagccgccaaggatggaaaaaataaacttgctggcaggaaatgccggtagaagcattgtcccaatgagaatgaagaagtctgaagcgctggtcactcccagaatactggggtctgccaacacatttcgaaaggcagcctggctggcagctcctgctaccgcaagcatacccccacacagcatggttgaaagaatccgcggaaagcgaatgttaatcaacacgtccagttgattgggattgcccccttgaaaggcggtcatcatttgttggggggtaatgaagctggcccccaacatcatcgcaaacaaaatggtgatgacaagcatcaccaaaattgtcgaataccatattttttcagatttagtcaattcgtttggctcccttcttgaggatacagccaattcgaaacgatctgcaaggctttggcagcccgcatattggcagttgcatcaaagttgggttcttccagatcataaacgcgatgattcttaacggcaggcagcgtcttccacatcggatcggatttaaattccgagttaaattgtgggatcacgatattgggtaaggcgtgtgccaatcgcaaaataacctgtggctgcgcttttttgatggcttcatcgttgggagagacaaactcttgtgtctttgaagagaaaacattgtgaccaccggcaattgcgactaaatcaccaacgtaggattgattagtggcaatcatataggaagccccaggtaaccccatcaagacaagcacccgaggtttggtggcatggcgcttggcaaccagtttaacatgctgctctgcctggtcaatttgatcaactgcgtgtttggcctgggcttttcgctgatattgtttccccattgcggtcaccgtttgtttcaatttggtgacgctggttaaatccagaaaatggggcgtaatatggcgttccttaaatgcccttccaaattggtcctgcagggtcgtcacggaatagacgacggtcggttttaaactggcaattttttcaacactaggattcatcggattgccaacccgggcagcgtgcgcataacgcgccggaattttattttgagttgtcggcacaccgaccagcgggagatcgagcttatctgcaatttgaacgaccgcaaaagtcgttgccacaatccgagcttttttctgatgattggcagcaccgattcggctcataaagataccgcccaacacgccaactaccaaaacaagtgagagcacaattaaagcgatcttacgagatcctttcattatccttattgccccctctaatgtttaaagtaaatccacaatcctgctgaaagtccggcaatcacagtcacgccgccgacaatccaaggaaccccgctcttttttgcttggggtttgtctgaagtctttttagctggtttggtcaggttactgctggccttacttggctgtgatgaggctttcttggcggaagactgttttgctttgggttgctttgtcttggttgagctagcagtcttagcagcttttttggtcttctttggtgcattggctttgggtcgactgttggtttgctttgccttcgtacttggactagtagccgccttaggctttgtcgttgacgtagctgtcttaggtgtcgccactgcggcgtgcgtccttcccaagcttggcagaccagccgtactaaatttgaacgaaatcaagtgatgggccttataaaccttgggcacgtcaatagcgagcttggcattgatccgtttcttcaggttattagcataaaatgaatagtacagcagcgaatctccggcccggtctttcacgcgacggacatttaatggcgctttaccgttgacccaattcactttgactggaaatgatgacaaactcttggcagttttaatttccatcgtgacgtaatagagatgatttttcaccaccacattggccggcttaacaaaatagccgtctgccattgacgtttgattggttccatagcgcaatgggtgataggcaatggtttgagcactagcttgaataattgaaacgatgaacagtccaatggcgacaaagaggcccaatagccactttgatctatttgacaattccatgattactcccccaaacaaaagataatcctgatacgagtgctaatccaagcattgacaagctgttttggctggcatcaccagtttgtggtaatttagtctggctggaagtgctcagcttagctgaagtagctgtcggtacaacagcaacatgcttgctggccttggcaggcgctttttggctaaacttgaaacgaattggccaagttgtattgatttgggcttgagggacaaccacatggattgaacccttgataactttcttcaaagttttgaatgatgaaacgttaaatgaataagtcatggtgtagtaattagtcgtttgaccataactaacaactgaggatttcactttgcggccattgatggtcactgggcgaacagcttttgaccccaactttaagttcttcttgtaagcaaccttcagttggacgttgtagtgcttagcaatttttttaatcacggccgttcgagtgtaatattggttagccattgactttgaatttgagtcaccctttaaaaccacatactttcgagttgtggttggcacctttgctttagcggtggtcttctttttggtggtaacagttgacgtggtcgttgtcgtcggagttgtagccgaactgctggtagctgcaggcgttgtggcactgctgctggtggctgcaggttcggtcgtggtacttgaatcagttgtcgtggttgtggcggcatctgatccaggaacctttacagcatctgcccagttaaacgaaaagtcggcagattcttgcatttgtccaagaattggaatgttatgaagcgtaaagctaaccggcatagtgctgcttggattggtcaaattgaacgttaaggttccattgttcccagaggtcacaattggcaatgccgtttgatcccccatcgtcatgctggcaatatagttggcaccgtttgtcgtaatgacagtcgtataggttcctttagacactgtcacctgggcagtttggtcaaaaaaatgattggcaatcgattgagaactgctgccgctcttcaataaagtaattggtacagtgtacgaagcgtcacttaggttgacagaatcagccttagcattggatgaaaatgcacccccccacaaatgcgaaaataattgctacaaaaacaaactgaataaaatgtacaaaacgttttttcatgcgaaaatccccctttaggtataaaaataattgtacacagtaagtttaccattagtttggaggtaaataacgtcaaatttgtgaattgataggcaaaaagcattactttttctcaagcgctttcttgccacattgtttatggattttgctcttaaacaactgacgaagttaattaatcaaaatatttatctggttaatgaacaacggctgatttgttaggaacgcactgaacaaagaaaacccagccagtacttcacgtttttttgccggaacaagcggtcttggcgatcgtgtgggtgccaacctcaccgccggtatcacagcaagcaaagtccatataagagcatcatacatcgtctgttgtttgagatacttcgataccactgagtccttacaaaaaatgcctccagccctcatcataagaggctggaagcactgggcggttcatcaatctaaatgtatctgacagccattgccaggatttgaacctgggaccttttccttaccatggaaatgctctaccttctgagctacaacggcatggttgaatcaaagaacataaatcgatattatcaaaaaaagcactgatagtaaatactatcgatgctttaggattgcgtggcaacgtcctaccctcgcagggggcgatcccccaactactcttggcgtgcagaagcttaacttctgtgttcggcatgggaacaggtgtatccttctggctatcgccaccacactatttttccttgaaagaacttcgttctctcaaaactagctaatattaattttctgcccttgaacaccatttctacttggttaagtcctcgaccgattagtattggtccgctccgtacatcactgcacttccacttccaacctatctacctgatcatctctcaggggtcttacttccatataggaatgggaaatctcatcttgaggtaagtttcacacttagatgctttcagcgtttatctcatccatacgtagctacccagcggtgcgcctggcggcgcaactggtacaccagcggtatgtccatcccggtcctctcgtactaaggacagctcctctcaaatttcctacgcccgcgacggatagggaccgaactgtctcacgacgttctgaacccagctcgcgtaccgctttaatgggcgaacagcccaacccttgggaccgactacagccccaggatgcgatgagccgacatcgaggtgccaaacctccccgtcgatgtggactcttgggggagataagcctgttatccccagggtagcttttatccgttgagcgatggcccttccatacggtaccaccggatcactaagcccgactttcgtccctgctcgacctgtctgtctcgcagtcaagctcccttctgcctttacactcgttgaatgatttccaaccattctgagggaacctttgggcgcctccgttactgtttgggaggcgaccgccccagtcaaactgcctacctgacactgtctcccgccacgctaagtggcgcgggttagagtgttcacacagcgagggtagtatcccaccaacgcctctgccgaaactagcgttccggcttcaatggctcctacctatcctgtacaagctgtgtcaacacccaatatcaagctacagtaaagctccatggggtctttccgtcctgtcgcgggtaacctgcttcttcacaggtatcttaatttcaccgagtctctcgttgagacagtgcccagatcgttacgcctttcgtgcgggtcggaacttacccgacaaggaatttcgctaccttaggaccgttatagttacggccgccgtttactggggcttcatttctgggcttcgccgaagctaactcatccacttaaccttccagcaccgggcaggcgtcagcccctatacgtcatcttacgattttgcagaaacctgtgtttttgataaacagtcgcctgggccttttcactgcggctgtgcttgcgcacagcaccccttctcccgaagttacggggtcattttgccgagttccttaacgagagttcactcgctcacctgaggattctctcctcgactacctgtgtcggtttgcggtacgggtagttgatgactcactagaagcttttctcggcagtgtgacgttggttgcttccctacttaaatttcggtcctcatcaccacttgtcaacccgccaaaaagcatttgactctttgactgacttgtggcttgaacatccctttccaactggatgcacaacttagcctcctgcgtccctccatcgctcaaacatcatcaactagtacaggaatctcaacctgttatccatcgcctacgcctttcggcctcggcttaggtcccgactaaccctgggaggacgagccttccccaggaaaccttagtcattcggtggatcagattctcactgatctttcgctactcataccggcattctcacttctaagcgctccaccagtccttacggtctagcttcattgcccttagaacgctctcctatcacttgaccaaaggtcaagtccacagtctcggtaatatgcttagccccggtaaattttcggcgcggaatcactcgactagtgagctattacgcactctttaaatgatggctgcttctgagccaacatcctagttgtctatgcaactccacatccttttccacttagcatatatttagggaccttaactggtggtctgggctgttccccttttgacgatggatcttatcactcaccgtctgactcccggataaaaatcaatggtattcggagtttatctgaacttagtaacccatgacgggcccctcatccaaacagtggctctacctccatgattctacgtccgaggctagccctaaagctatttcggagagaaccagctatctccaagttcgtttggaatttcaccgctacccacacctcatcccagcacttttcaacgtacacgggttcgggcctccagtgcgttttaccgcaccttcaccctggacatgggtagatcacctggtttcgggtctacagcaacatactaaaacgcccatttcagactcgctttcgctgcggctccggcttttaaaccttaacctggcatgtcaccgtaactcgccggttcattctacaagaggcacgctatcacccattaacgggctctaactgcttgtaggcacatggtttcaggaactatttcactccccttccggggtgcttttcacctttccctcacggtactggttcactatcggtcactagagagtatttagccttgggagatggtcctcccggattccgacgacgtttcacgtgtgtcgccgtactcaggatcctgaactgagggtcattgatttcacctacggggctatcaccctgtttcgccaaccttcccagattgttcgattatcaacaactttggtaactcaaatgttcagtcctacaaccccaatgagcaagctcattggtttgggctgttccccgttcgctcgccgctactgagggaatcgaaaatttctttctgctcctgtgggtactgagatgtttcagttccccacgtctacctctatacagctatgaattcactatatagtaacagtcgattaaaactgctgggtttccccattcggaaatctccggatcaaagcttacgtacagctccccgaagcatatcggtgttagtcccgtccttcatcggcttctagtgccaaggcatccaccatgcgccctttttaacttaacctgtacatcacgacgtgatgcaaagttaattgagtatttgcgattttttctagttaacaaactcaaaataacgcggtgttctcggttgaaattatataaatacaatttcaaaaaattattacagaaaattaatattatctagttttcaaagaacgaattgagagtaggcctctcaaaactaaacaaaactttcgacaatgtgcaggattccgtttttccttagaaaggaggtgatccagccgcaggttctcctacggctaccttgttacgacttcaccctaatcatctgtcccaccttagacggctggtccccgaaggttacctcaccggctttgggtgttacaaactctcatggtgtgacgggcggtgtgtacaaggcccgggaacgtattcaccgtggcatgctgatccacgattactagcgattccaacttcatgtaggcgagttgcagcctacaatccgaactgagaacggctttaagagattagcttgacctcgcggtttcgcgactcgttgtaccgtccattgtagcacgtgtgtagcccaggtcataaggggcatgatgatttgacgtcatccccaccttcctccggtttgtcaccggcagtcttgctagagtgcccaactgaatgctggcaactaacaataagggttgcgctcgttgcgggacttaacccaacatctcacgacacgagctgacgacaaccatgcaccacctgtcattctgtccccgaagggaacgcctaatctcttaggttggcagaagatgtcaagacctggtaaggttcttcgcgtagcatcgaattaaaccacatgctccaccgcttgtgcgggcccccgtcaattcctttgagtttcaaccttgcggtcgtactccccaggcggagtgcttaatgcgttagctgcagcactgaagggcggaaaccctccaacacttagcactcatcgtttacggcatggactaccagggtatctaatcctgttcgctacccatgctttcgagcctcagcgtcagttacagaccagacagccgccttcgccactggtgttcttccatatatctacgcatttcaccgctacacatggagttccactgtcctcttctgcactcaagtctcccggtttccgatgcacttctccggttaagccgaaggctttcacatcagacctaaaaaaccgcctgcgctcgctttacgcccaataaatccggacaacgcttgccacctacgtattaccgcggctgctggcacgtagttagccgtggctttctggttggataccgtcaagatgtcaacagttactctgacacctgttcttctccaacaacagagttttacgagccgaaacccttcatcactcacgcggcgttgctccatcagactttcgtccattgtggaagattccctactgctgcctcccgtaggagtttgggccgtgtctcagtcccaatgtggccgattaccctctcaggtcggctacgtatcatcgccttggtaagccgttaccttaccaacaagctaatacgccgcgggtccatcctaaagtgacagccgaagccgtcttttaaaccaaaaccaggtggttttggttgttatacggtattagcacctgtttccaagtgttatcccctacttcaagggcaggttacccacgtgttactcaccagttcgccactcgtctcaatgttaaatctttcaggtgcaagcacctgaaatcatcaacggagacgcgttcgacttgcatgtattaggcacgccgccagcgttcgtcctgagccaggatcaaactctcatcttaaattgtttaaaatgataagcctgtgatagctcatgatttaaatttattatttgtttttacgaattgacttcgcaaatgtttggttccaattccgaagaattggaacgccctgcacatttgtttgtcgaaaattttgttcagttttcaaaggtctacttggttgcgggtgagatgaatcatctctcgcgacaactatttaaatataccacgctggttgtttcatgtcaacaactttctcaattgattgaattgatattggttggtcacgaacaaaaacagcatctataaatatatcgaagtttgatcaattcgtcaagccccaatttcaaatcaattgaactttaacgatcgggactgtttatcacaaacgatgacttgttttaatccaaattaaaagtggaacatctctgttccacttttaattcgcaaacctatttcaattcaggtgcatcggtcttgtacaaattcatagtcgatttaccattgttctttgcttcaatgctggttggttctttcttttgggcctgctttaaattatcaagagccttggtatattggtaagtgaaatctttgcgattaacttttttgaatcccttaggtgtgtagaacctgagtaaatctccccagatgacccgatcggataatgataattccgttgtcacatggttttggatgctagccaactgccgtttttgagcggcatttggcgtaatcagtttgcccgtcttagtcaaataaacgtcgctgccaaccttggtatatttcggtgtgacaaaatcgccatcccggaatgcaacccgctgatcatgctgcttggataacagatcggttccaaactgaatcgtattattattcttgtcgcctaacagatgcaaaatagttggcaagacatcaatctcaccaccatatgtgtgattgaccccacccttaaggccaggtgcatgaatcatgaacggaaccttctggaactgtgccaaatcataattgttaatcgatttcttatggagcagctgggcgatggccgggcggtgattattggaaataccgtaatgatcaccgtatacgacaatcatactgttcttcatcaaaccggttcgcttaagataattcataaattccgcgaaggcctggtccagataatgggcagtttgaacgtatgggtcaaccgttttatccccggtcttagtggcaggaaaatcagtattttgtttatccagcaaatatggataatgattggtcaaagtaatgagtttggcataaaacggctgaggcagctgttgaatataattggcagcatctctaaagaaaatcttatccttgagaccatacccgacactgtaagacggcttcgtcttgtaatattgagagctgaagaaataatcatatccccaggacttgtacgtactgtcccgattccaaaagctgggaacatccccatggaatgcagctgttgtgtagcctcgttgatccaagatagcgggcgccgcctgatacgtgttctgggcaccatatgtcaccatggcagatccttgaggtaacccgtacagagaattttccaacatcatttcggcatcagaagtcttcccttgagcaacctggtgaaagaagttatcaaaaccaatggtatttttattgtggaaaaaggcattcaggtggggcgtcacttccctgccgtcgactttataattaattaagaactgctggaaactttcaagatgaataatgaagacgttctcgcccttggccttgccaaaataagccggattggccttggcccgactatgatctaagtatttcaaaatactatccatatcgctggccttggcttttgatcgggtagcggattctttttgggtttggtatgcattaaaagcggcatactcgtttaaccctaagtatttaacaatataattattgtcgaaggttctggtcaacaaaccagaccgatcagtgcttgccagaccgtattcgccacccatcaagagaaaagaaacgaccgtaatcaaaaatgcataacgcttcttaaatggagcggcgtcaattcgaatcacatgaaaagccaacaaggcaatcaaaataatcacatctagaaaaacaaaaaagtcactgaagtgaagaatttcaaccaggctcttccccaagttattttgaacattgccggatcctttgatgacacctaacgaaagaaagtcggaaaactcacggtagtacagaatattggcaaaaatccagatactctccaaagtatcgatgatcatcatcaaccaataagacagccggccactaaaataaagggcaatgcccaatgtcaatagtgccgccgggatggggttgactgccagcaagaattcctgcatgccgcctttaacgcccagcgtaaatttagtttgatacgcaatatacgtcttgatacaaaacaaaatgacaaccagcaaaaagaagccaattctggtgtttaaaagatttgaaaaacgatatttcttatccgttaacattcctgttcctccaaatgtttccctgcccgctatttaatgcggttatcgggatcatcaactttatctggtttgactaataaagcacaggccccagcagccattccaaagtaatacgttaaaattctccaaataatcattgccaataccaatttgctgttactcgaaataaagctatggaaaagtgattcaaaactgaattcggcaccaccagaaccaccaggaattgggaacaacgaaataatcatcacaatcatgatgtgtaaactggtaaccataatcacgttgatacccgtatagccgagcgatagcataatgaaatatgggatgaggtaataaaaaagaagttgaaaaaatgtgagaacaacgatttttaataatagcttgggttgacgcccaattctgacgctttcctcaaacaaattatcaattttggaatacatcgtttcacgcattgaataaaatttctcgtccttgatgaaccatttgacaggatgaaaaagtaattttgaaagtttcttggtaaacgacggccaatacattatcaacagtaagccaacgatgacaaataaatgaattaaaaagccaaataaaacaaacagcgccaaaaagtgcaatttggttgcaacaaaatggaatccaatgaccaagctgataaaaaagttgatcacaatcattccttgatacaccacaaacttcatcaacagagcggagcttgcccgaccgccatcaatcccagtctgcagcatgacaaacaactgtccgggttggcccccagatgaaaacggggtaatcccattaaatagctgttcaaccagcggaacccgcagagcatccttaaacgtgaagtgttcaacgcgattggacaccaagacttttgtaattacgccctcaattaataaataggcacagatgcaaagaaaggcgactaaaatccaccaaggattcagggtgaacaggtcatggatcagcacactcaatttaacgtccctcaaagagtatgcaataattgcaatcccaattatcaccatcgtaaagagggtaattttattatttcgtgacattattaaccttccttagattgttgattataaaaatcataccaaactttggcgagatgatcttcagaatagcgttcactggcaatcgtcgtttcatgctgtaaagccgccaatttgttaggattcaataacagttggtgcagctgttcattcatctgtttttcatcagcagcaggaagataataaccgctgatgatcgacttgtataagtcaagatctcgaagcatcaccggggtattagttgaaaacgcttcaagaaccgacatcggaaacaattcattataggacggaaggagaaataaatccgccatattataatattgaaccatcttggcgcggtcaataattcctggaaacgataaattacttgggggatccttgacgattttttccaaatcagcataaccctcggtaattttgccaaacgaaaaaccacccgtccaaataaattggatcgtcgggttttgcttggccagcttcacgaaatccaacacccctttacgagtttgaatttggccgctgcctaaaatggtgaatcgttttggatcgtatccatgcttgactcttagggcttgtttttgttggtcatcaacatcatagaattcggctttgctgacgaaattaggaatataagtaatccgttccttgttaattccgtagcgttccagcttgggaataaacgatggattaaccacgacaatgtggtccatccgcttataaaaggcaattacatacttataaaaaatcgccttaaacggctgggggattttaatgctgccttccaaggtttccggcaggaaatggacatagccgatttttcgccctcttcgcctcgaaaatgtcgagaggtagaaactgggattaattgtatggtaatgagtaatatccgcaggtgcatagctattaatggtgattttaaaatcattaggaaagtggtccttgagcattctcaccagttccacataggcactgccgacgccttgacccttgaccttatccgcggttgaaaacatattaatccttaacatacaaactcctcacaaaatatttagtcgatattagtagtggcattatcttgtaattcttgggccaccgctactgaatgataaaagttaatcacccgtttgccaaaggtttctgcagaaatcgcagtcagtttctttttcaagatttgtttggctttgggtgtctgggtattaacctcgtgctttaaataatgagtcacaatcccaacaaattcatcgtcgtgctcaaatgtctgccccaaagtttcggagctcaacaacccattggtataatcactggccgaaacgactactggaagtccggcagccattgcttcaatgtaggtcagtccttgagattctgatttagaggtggaaacaaagacgtcgcatgcccgatagaaagcattgacgtgatcgttggcaacttcaccggtaaagataacatgatcatccagctgcagcgcatgcacctgactcatcaaatcatccttggcaggaccgtcacccacaatcattaagatggcgtttggaacctccgtcaaaatttttggcagatagtcaatcacctctgagatgtttttttcgtatgccaaacggctaatcgaaagcatcagaggcgtatccggagaaatatgatactctttgcgaatgtcggtcttgatttcttcagcgtacatatcaacgtcgattccggttggaataatccgaatctcgcttttaacgccataatctgtcaatttgtccaatacacgatcactgggggcaatcacacctgacaggtggtagcaaaaagccaacgtcccttctttaacgtggacgggtttgagcaacttgccattagccacatagtgcaaataatcttcatacattgtgtgataagtatgcacacaaggaatattcaggtttttggcgacaaatttgccgatcattcccatcgaaaactcggtttgcgtatgaacaatatccaagttgagttctttggcaatttcgtaagcttgaaataatccgcggaccgcaatccgccgatccgtaaatgagataaaggggatacttgagaaacggaaaatattctgctcgtaggtgtccttatcgacgtgcggatctgttgtggtgaaaatatagacctggttaccctgtctctccaattcatttttgagagtcttaatcgaggtcgcaacaccgctcacctgcggaaaatatgtatccgtaaaaatcccaacattcacggctgacacccctttctaataaaaatcgattaattatgctcgtgaaatgtgccgtcaggccgttacccggtgtgacgcatagtctcacaatcattgtaattatattggtttagttctgctattgcaaaccacccgaataaaaagaggctctacaatatctgttgttggtaatagatttttatctattactgatgacagattttttgtttttcattagaataaaaaaagcggacatttcctgtccgttcatcaaaaccaacaaccacgaagattttagagaaagaaggaaatgccctatgtcaaatgatactacgaaaatgttgttaggaatagatgatgaacacttaaaaattgagaatggcaaaataggtgatgatggggtaatcagattaaatggatcactgaactattctcccaaggcctgccgcaattgtggggttattaatgatcaccagatcattggctatggttggcggaagaccaccattagattcgctaaaacattgggcagcacggttatcctatgcctcaatcggcgaaactttcactgtaaggcttgtcataccaacttcctggcgcagacgagtgcagtgccgaagcactgcacgatttcaaatacaacccggaaacaatgtttagagaagttaacggaaccagtgagcctcaaacacattgccaatgaattgtccacttcggattcattcgttggtcggcagctcttgcgcgctgaacacgactttcaaaccaactggcactacttacccaaagttctcctcatggacgaagttaaaagtactaagagcgccaccgacgcgatgagctttgaatttatggacgcggaaacccacgaattgattgacctgttgccctttagaaccatctatcagcttcaaaagtacttccaacattatgaccaagccgcgcgagaaaatgtgaaaattatcgtcaccgatatgaactatacctatcccaaattggttgggcagatcttcccgaacgccatcgttgtcatcgatcccttccacctggttaacgctttaaaccgggcttttaataagacgcgagtgcgtctcatgaaaaccctggccacttcctcacgccagtatcacgccttgaaacgctattggaaactattattaacgccggccaatcaccttaactacgaggctttccgtaagtggacaaacttcccttatccggcaactgccacggatgtggttgatgctttactggacattgatcccgagctcaagcaaacttacgacgtgatgaatcggttacgtgaaaccatcaaaaaccgcgactggcccaactataatcaagcctttcaccacctgcaggggtgctcggaagagatgttggcagccctccaaaccttggcggctcatcatgatgaaattggcaacactttcacccaccactacaccaacgggccattagaaggttcaaacaacaagattaaagtcattaagcgcactggatttggttaccgaaacttcttcagattccggctaagagtgctgttcgcttttcgagttcatacaaaaagagccctaatcaccaagtgattagaactccaatattttgttcaccaacaacagttgacgaagaacctaaaaagaacaagccgaaaacggacggtttaacgccattaacagcttgttctttaagttatttataaatctattggacgttattagtggcctggtgaacaaaggcagtgacttcttcactggtgctggccatggtaaccgccttgttggcaagggtgaccatctctcttgaatcgagccgtttgattaacgcccgggacttgagaattgaagaagcgctcattgaaaattcgttgagccccattccaaccaaaataggaatagcggtctgatcgccagccatctcaccgcacatataggcaggaagattattatcatgacaagcatcgataatatgcttgatcattcgtaaaacggccggattataaggctggtaaagatatgaaaccatccggttgccacgatcggcggccatgatgtattggattaaatcattcgtcccaatactcatgaaatcaacctcagtggcaaattggtcagccagaatggccgcggccggaacttcaaccataatcccaatcttaaccggttttacccgaaccttttcccgaatcaatttgatccgttcctgattgaaaatattcttagcttttttcagttcattaatggtcgtaatcattggaaacatcactgacagatttccaaacgaagaagcccgcagcagtgcgcggacctgggtgcggaaaatatccggcttatccaggctcatccgaattgcccggtagcccaaaaatggattggcctcctttggaacatccaaatacggtaaatccttgtcaccaccgatatcagcagtccgaatgatcaccggctttttgcccatcttttgaagcaccgtcttgtaaacattgaactgctcatcttcagtaggcaggtgattagagtccatatataaaaattcagttcgaaacaagccgattccctcggcaccattttcaatagcgccgtccaagtcgtccaaagtgccaatattagcagcaatgattggatgcttaccgtcagaagaactggtcatttgatgtttgaaatcagccaacttgctcttgcgttgacgatagtcagcctgcttttgagtatattcgtctgtttgggcttcagtcggattaacgatgacgttcccagttgatccgtcaacaatgaccgtatcgccgttcttgatatctgccagccggcccttgaaccccacgactgcaggaatctccaatgaacgcgacattatggccgaatgagaagttcgtccacccatatcggacacgattcccaacacataactcggcacgaattgagctgtatcgctgggagttaagtcgtgggcaatgataatgaccttgtggtgaatcaaggccggatcaaccagcggtactcgcagcaggtgacttaaaacccgcttggtaacatcacgaatatcgcttgaacgttggcgaatatattcgttatccgtcattgaattaaagattttgatgtagccgtccgtgactttggttaaagcatattcggcattcaccttctctttttcaatcgttgacttgatccgattgagtaattcaggatcagacaaaattgcaccatgagctttaaagacctcagcttcactgctgccgaggtcttcaagtgttcgttgttgaattgttaaaagctcgtcttttgagacatcaatcgcagcataaagccgcttaatttcatcagaggcatcagtaatgctccgctttttaaagcttaaatcaggttcagttaaccgaaatgcagatgcaatggcaattccatcacttgcggcaatccccttaaactctttcatgaaattattcagtcagtccttctgctttcatcgtttcgctaattgcatcaatggcttctttttcgtcatcgccgtcagcagtaatcgtaacagctgcactttgaccaactccgagtgacatcacacccataattgacttcaagttaactgacttttcttggtattcaagggtgatatctgagttgaacttgctggcagtttgaaccaacaaagtagctggacgagcatgaattcctgtttctgcgatgatattaaattgacgtttttccattattaatcaatctcctctgataagattataaattttgaagatgatgctcaaaatttaaatttgttctttacttaattaagaatagcaatatataagggaaaatacaagtttaaacttaaccgcttacagggtttttaagaacttttttgcttgtcgtctctctcataaacataggtaatcacaccgccttcggtcgcggacccaaccacgcgctttcgatggtcaaagttcatgtatgcggtctgaaaggccatgaatgattccggcttgacttcgattttttcaatctcacctgattccaacttttctaacaactgattgtagtcttgattctcttctgccacaacgtctcatctcctttcaatttaagtgaagttcaattacttgattacatataatcatgttgtataataatttcaaaggtcaaagttggtcagtgattaacagatcctccttgtccttttatttctatattaaaggaggaaagcaattaatgctatgtcaaaattgccataagaacccagcaacgattcacttgtacactaatgtgaatgggcaaaagcaaactattaacctttgccaaaattgctatcaactcctatccaatcaacaacgtaatacaggaggtgctcaaaatatggctcaagatccatttggttttggtggattagatgacattttccgtgcaatgcaaggcggaaacgttgatccaaccaatggtcaacaagtgccaccaacccaaccaatgggacccaacaatggcggccccaaccgaccaagaaccggcggagcgggcggaaattccctgcttggtcaatacggaattaatttgacccagcttgccaaagacggcaaagttgacccggttatcggccgtgacaatgaaattcaacgggtaattgaaatcctgaaccgccggacaaagaataaccccgtccttattggggaagccggtgttggtaaaactgccgtcgttgaaggacttgctcaagaaattgtttccggcaacgttccttcaaagcttcagaataagcaaattattcgtcttgacgtggtttctttggttcaaggaaccggaatccgtggtcaatttgaacaaagaatgcagcagctaattaaagaagttcaagataatcccgacatcatcctgttcattgatgaaattcatgaaattgttggtgccggtaacgctgaaggcggtatggatgccggaaacgttttgaagccagcattggctcgaggcgagttccagttgatcggtgccactactttaaaggaataccgtgatatcgaaaaggactctgctttggctcgtcgtttgcagccgataacggttgatgaaccaaaccctgaggaatccattaagattttgaaaggtatccagaagcgttatgaagattaccaccacgttaagtacacagatgacgcgattgaagcagccgttaagctgtcagaccgttacattcaggatcgattcttacctgataaagccatcgacttacttgatgaagccggatcacgaaagaatttgaccatcaatgccgttgatccgcacacggtcgatgaaaaaattcaaagtgccgaaaagcaaaagcaagctgctttaaagagtgaagattacgaaaaagctgcttactaccgtgatcaagttaccaagcttgaaaatgccaagaagaacggcagtgtcgactcggcagcaacgccaaaggtcactgctcaagacatggaaaagattgtcgaagagaagactgaaattccggttggtgaacttcaaaccaaggaacaacaacaacttcgtaatttggcccctaaccttgaaaaacacgttatcggacaaaatgaagcggttgaaaaagttgctcgggcaattcgtcgtaatcgagttggcttcaacggtaccggccgaccaattggttcgttcctgtttgtcggacctaccggtgttggtaaaactgaaatggctaagcaattggcctatgaactgtttggttcaaaggattcgatgatccggtttgacatgtctgagtacatggagccgcattcagtggctaaattgatcggttcacctcctggctacgttgggtacgaagaggccggtcagttgactgaacaggttcgtcgtcacccatattcattgattttactcgatgaagttgaaaaggctcacccagatgttcttcatatgttcctgcagattcttgacgatggtcgtttgactgatagtcagggacgaacagtttcatttaaggataccatcattatcatgaccagtaacgccggccagggtaatgcggaagccaacgttggtttcggtgctgcagccagtgggaagacgcattcaattattgataagttgaccgactacttcaagccggaattgttgaaccgtttcgatgacattgttgaattccactcattatcaaaggacaacctgatgaagattgtttccttgatgattgacgatgtcaacggtatgcttaagcaacaaggattgaagatcaatgtgactgacaaggccaaggccaaattagttgacttgggctacaatccagctatgggagctcgtccacttcgaagagttatccaagagcagattgaagacaaggttgccgacttctacttggatcacgaaaatgctgctacattaacagctgacgtagattcaaagggcaacattgttatcaagagcgacagtgcggctgaagtaaaagcttcaaccaaagcaaagcctgatagcaaggattcagataaataagtattaaaacattaaggggtaacggtcagagtttgaaattttgatcgttaccctttttgtattctcaccatgattgcccaagtatggcgctaactgtcgccttttctgggttaaatcgttaaaataatccttaaattcggtggtgccaatgctgattatgctataatttttattagaagattgtagatcggagcgcttattaaatgaagttcatggattgggtcaaacaacagttaaatatctttgtgtcgccacgatcccatcggcaatcaaatcgtcggggccgtcgccgggactatcaccaacgaaagcggtggcagtctgcacaagtcgacccggataataatgaccaaatggcagaagtgggtaccgcttccaatcaagatgcggttgaagaccaagcggatgggctggccaacgacccttcccctgcaccttttaaagccgaggagaccattcaaatcaagtctcaagtgaccttcttttatctcgatgaaaatgataatccaatcaaaaagcctgacattttaattggtaacgatggcgaacgcttttctctgcagctacctcattttaaacaatattacctggtatcgattgataacttttcgacttattttgccgataccgatcaagaagtgacattccgatatgccctcaaacaagggttgccggtcctaacctattatttggacattgataccggtgaaaccttgcatcacgtcacaatccactccggaaaactgggggaatcttatgacgtttcagctgcggatatccccggttaccgcgtcatcaatgatgtcggtcccactcacggccactttgatgaccgcacccatggaatgatcttttattatcgacgaaccccttggcaaactgtccaaccagttgagtattatgtccgtctgaaaaagcgacacgctgtcttggaccaaccaaatggccatgcgttacaaaccggattgccggccaatgttatcaccaagatttttgcccgcatcgaaacgacggacaatcaaagctggctaaatattggcggttttgaatggattaaaaatgccgaccttgaacccagtgatccgcctaccaatcatcttgtcccaccgattaccaagacttccaggaatccggtcatgctgtttgggacagttgatttcgtagctggcaggccaattgaggtctttgataaaccgtatggcaccaatactggaacattggcagacggacaacgggtttcaattaaagcccgaattatcgatgatcagggcctgatttggtacgagctggctgatcagtcagtcatctttagtgaatatgttagaattgattcttaatataatcagattgggatcaaaggcgatttgatctcagactttaagtaaaaatcgagttattcctgtcttgggaatgactcgactttttgtttaaatggctgagatcagccgttagccatgtaggcttggcaagcacgctggccggcgccgcaagttttgttagtataaacgtgatgatcaaagctgccggctacttaaaaatggcaaataggaaaaccgatactaaagcaatcatgcaaacgaccgccgcaaacccaccaacaatcattaatttttccaaccgattctttgccgggttccgcttttgccgttgctcctcaacatcttggccatccgtgaaggccaagatttcagcataagttctcaggtttttgcgtttctttattcgctcgacttgagatgcgctaatgaacatgaccgcaaaacagatgatcggcaccaagataatcaacgtcgattgctcaaagtaaacaactaaaccgattgacattgcgcccaaaacagctgcgataagcatcacccacgtataaactgacattgccgtattgactttcttatcagataatttagctttcatcgcttccaaatcccccttaatgagttcatctacagaaacgccaaataaaacacttagtagtaaaacattttgaatatccggatactgtttgccggtttcccaatttgaaattgtctgcctggaaacgtatattttagacgctaattcttcttgagaaaaaccacggacttctcgataatcccgaattttattgccaatgtccatttcctcaactcctcatccaaaagtatacctgaatgttgggacgatttctgtcacgttgccgtatattgtcaccaaaatgctcaatgaaaggtcaatgtgacacctcgtgcggcaggttggcgaacgcaaaccgcaatctcaaagtttgccttttttatataaacacgttgtatctagcgcttcgctttatcaaccacgacctaacacattggacaaaaatgccggtgaacaaatatgttcaccagccagttcttcttcatgagaccacaagagtgaatttgttccctcgttggtcgaaaaatgttccgaagctaatcagcttggtcttgtctctaaagatttttatccatattaaacgtcaacttggacagcgtcagtcccttttcaatcagttggtgattgaaatgttcagtggcaattcgcatcattttgacaacttcatgattttgctcagtcaagtagctggtcaattcttcacccttcagtgcctgactttcatcaatcgcgctttggacgtggcgacgcagttgttccttcatgtcagttaagaagtcgacatcatcttgaataaattcagaataatgggattccactaacatcgataacttgcggtacatccaataagcactgacatcatcgaaatggaccggcgtgttggcataagtatcatcggtatccgttgcattggcaaagaatggcacatatggtgaaaatgccggtaccccaaagcacagccacataattgcattactgttatttttgagatcattacgaatctgcaaaacatgtgaattttgggtccgattcattgaaattggccgaaacagcgtcttagtatcctcatgacccttactgaacggatcataaggcgtttcgttgtaatgagagctcaaaatgtactcaacatcttcgacactaattttatggtcggtatgacagatgaatggcaaatttgaggaagttggtgactgctcaatttccggattcaggtatttctgaccgaaccaaacgcgaggcgtgttgtaatgacggtccttttcgttatccgttccaaagatgtggcggaagttaaatccctgcttgtcagtattcaaatgatacttctcgacaaattcttggatgccgtctgaatacatgaagttgtctggatcatcaaatttcacctgttggatagcaacttgattggcggcaatcgcataggcgtcatcaggaattcgttgagcaacccagtgatgaccggtaacaatttccatgtaccagacttcattgttatcgctaaacaaaaccccattaccctcgggtgatccatactgcttgattaatttaccaagatattgaacaccgtctctggcagaatcaatgtaaggcaaaaccattgactgcaacgagtcctcggctaagccgtctttgaccaatggatcaaaagccagcgcccgttcattcccgtagacactttcagtggcactcatggcaacattcttttcgttaaagccactttcagcatagacgccttccttatcgacttcaacgttgggtgtcaatgaataacgataggcctgctcgggcagtggtgccttaaaaccattttggttggaagcccactcaccggtttggtgatcattggcgggttcaacatagaaacgttggggtgttagcggcaaaaatgtatcatcatttctggcaatcatcgttgagccatcgatggaagcttttttaccaacaagaactgtggtgcatgcggacaaatgtttggaaaccatcatatctcttctttcaaagttaaattatagtttggcagtcaatgtaacatcagggtacttatctttgaaccagcgaagggcaaattcattctcaaataagaataagggattgccggcgcgatcctttaccaataagtttctggaggacgacatcttttcgtcaagttgatcagggtcaatccagcgggcaatcttatggcccattggatccatattaacctcagaattgtattcgttcttcattctgaattggaaaacttcaaactgcagctgaccgactgccccgagaatatagtcattggtggtataggattggtaaagctgtaccgccccttcttggaccagttggtcgattcctttatggaatgatttttgtttcatgacatttttggcagaaactcggacaaatagttccggagtaaattggggcagcttttcaaactcgacttttttcttaccagtataaatcgtgtcaccaatctggaaattaccggtatcgtataatccgataatatctccggcaaccgccgtctggacattctctctggtattagccatgaactcggtcacattggataatcgcagtttcttctgtgtccgataaaggttaacgtccatccccttctcaaactcaccggagcaaacccggacaaacgcaatccggtcccgatgattcgggttcatgttcgcttgaattttgaagacaaagccagagaaagtatcgtcatccggcttgattaagtcgccttcttccgtcttgtgggcacttggcgccggtgcatatttcaaataagcgtcaaagaacgtcttgacaccaaagttgaccagggctgacccaaagaataccggggtcatatcaccagtcgcgattttaccctcgtcgaattgattaccagccatatccaagagttcaatcgcgtctttggcgtcttcaaactgttcgtcttgggcaagttgatcgttgttcaccggatcattgttatcgtccaaatcaacaatttctgaagactggttgtttttttcgtgattataaagttcaacgtgatggttatagcgatcaaaaattccagtcaaggtcttgcccatgccaattggccaattcatcgggtaggcttcaatgcctaacacattctctaattcgtcaaccagatccattggttcccgaccatcacgatcgagtttattcataaaggtgaaaattggaatgccccgcatcttacagatttgaaataacttcttagtctgcggttcaatccctttggcggaatcaatcaccatcacggcagagtccaccgccatcagtgtccgataagtatcttcggaaaaatcctcatggcccggggtatccaaaatattaattcgtttgccaccgtaatcaaactgcatcacggaactggtaacggaaatcccccgcttctgttcaatttccatccagtcggatttggcaaaattaccggtctttcgggcttttaccgttccagctgagcgaacgacgccaccaaagagcagcagctgctccgtgatggttgtcttcccggcatcggggtgggaaatgatcgcaaatgtccgccgggtactgtcttccttttctaattgttgggtattcatgtttacttcctttcaggcgagtcaataactaattaattttaacacgttttcgtcgactctcctagaacccgccttaatttcattggctgcaatccaaaacaaagaggatggaaacaaaacatcagctttgttccatcccctctgtgatgtgaaattacataccactttcaatttgatgcatgacgtagttaaccactttcaatgaactcaagccatcgttaatcgcacagaagcggttatagaagttcataaacttctcattggctgacatatcaggatgcgccaaagcatggttgatttcggctaacagctgcttggagttttcagcaattttgccaggcagatccttctcatagttgagatagaacccacgtagttcctccttgtacaaatggtaatcgtaagggtagaacaaaattggccgcttcaggtaggcatagtcaaagaagactgacgagtaatcggtgatcaataggtcggataccaaatacaagtcactgatgtttggataattcgaataatcgtaaacgaagtctgaataatcggaaatatccaaagcgttggaaatcaaataatgcatccgcagaattaagaccgtgtcatcgccaaacgacttccggaagtcatccaaatcaaacggcaactcgaaggtatacttacctttctcggcaaattgattgtcccgatacgtgggggcgtacataaccacctttttatccagcggaattcctaactgctctttgatagcatcgatatcttccggttgagtattgattaattcatcgtttcgcggatacccaatctttaagatttggttattgaagccaaatgccgaacggaaaatctgcgttgagtagtcgtttggtgaaaccaaggcatcccaacgattggcttctctgacaaagttcttgtgatatttaacggtggtagtcccaggcattgaaacgttttcgatatccaggcccagctttttaagcggtgtcccatgccaggtctgaatataggtcacatagttaggcttcttaacccaagttgggaagcgggcattactgatccaaaattgggatttttccaagacccgaacccacttgttggttcgcctaatcacgtaggcaatctgattttccttacaaaacttcttctgagaacgatcaatggaccaaatcatattaataccaggatacaacgttttgaagaccttataaatggcgtacggactgtcactaacctgacggccgccaaagctttcaaaaataatcgtggtgttatcgtatggtgaatggcccgacttgaacaggaaccgcattctaaccaggttcagtttgtcttgaatcatcttaatgacatcaataatggtgccggccttgccgccagctgcacccaccttctggagcagagaggcaccagcaaattccttgaccaggatgccattatcatatcgtttttccaaagtgatctcacgattaccagccagttgaatatcggttgattggccggctaatgacttggagataattaatcgctgcttgatagatttgccgttcaactcgtattcgatgaaaagttcaccaactgaattttggggaatgtcggttaacggaatggcaaccgtaaacatcccttcaaacagctttttggtcactgggtattccagtgtgccctcggtcgtgtggtttttcaggatgatgcgttgatttttgattaacgtcccgttgatcttgttataaccggtaatttccaagttttcatcggttaagttgaccgaattgatcatgaattcttcatcggattggtgagtccgaatgttaaacaacgccattccctgggcatcgctgttgaattggtaataactggttaattcaagttgatgacgatcacttaaatattcactttcaacttgaatcacatttttgttggtcaagttgttattgatgagaaaaatctgccattcaaattcagtttgatcctctgattggaaatggaagtcttgggcatcgatgttgacccggataatattgtgggacagcactttgctgatcggcttcatgatcgaggccaagctatttttttcgacaaataaaacgtaagcagtatctaatgacaccgcaacgtctaataattcaaattcaaggacttgtttgcccttcttttgatggacacctgataatatcgctcgcaatttaatttccccttaataattaaagattcgtttgcctggcaggtacttggatgcatcgacaatgttgtcgatatcgatgtatgtccgggcgtcttcaatattcatgtttaacaagacttgatgataaaaggcattaatatcgtcgtagcgatggtaatcgctgtatgataatgctttggtgaaggtcgacttgccttggccttcgtaggctgtcagcatttcgtcctttgaattagacttgtcatcttgaatctcgcttaattcctgaggggcagcaatcgttgaacttggggtgacgttataactcaccttttggtccttcacgtagttggtaaatcggtaaaccagttcacctttagcattcagcagcaagctttcagtcagtgcatcatcaacatatttttcaatcccaaataatcgatcagcatcatcgtaactgttgatttggctgatccggctgcttttgtcaaagtaaagggtatgtatccgggtgttgtcttcggtaaataaagtttcagcgacgatgtttccgtcagcgtcaatgtatctggtcaccggcaatttgccctggtgcgccttaaaggtctgtaatccagacagatccggatccatgaaatcggcggcctttagactcacaccgtcatgttctgcgtaaatatctgccagtgaaattaagcgcacgctaggagttcccttcggtaggtcaatcttggaaaattcacgctttgcctgccagatttcatcaaaatcggtcattgccaacaagacaaccacctgatactgattattaattaacgctaacagctgtcgtcgaaatgtcgctttgcgaattccttgaatcgttgttgccaaaaaaattgctcgtcccatgattctcctcctgaataaaaacgaggctggaacaaaacatgtagtcttgtcctcagcctcatttgaatcttgtgtgctacacatttgattgtgggtattggtttggaatgtccgtggcgggaaagcccgtccagattggccaagtgccgggataaccagaatctcagatgttaagctttccaatcctcggtatccgttaagcctaaatcttctttgatcttggtggttgaaataccttccgttcttgggaggtatacgacttcgcaataatcctttaagaagtcaaacttccctttccagtcatcacccatcacgaagacatcaatgtctcggtcctggacgtcgtgaattttttgatcccagttggtttctggaatcacttcatcaacgtatttgatggcttcaagaatgtatttgcggtcttcgtatgacgtgtatgctttcttgcccttctcagcgttaaactcatctgatgacaagcacactgtcaggtggtcacccaacgcctttgcccgcttgagcagacgaacgtggcctttatgcagcaaatcaaacgttccatacgtaattacttttttcatagaatctcctacttaatcattactctgaatgtgaactaaaataaacacatcttaaatagtagcataatcaccgacaacgtcaatatttattaaagattattaacgtttttgtgttattccagttgataaatattatacatgtgcacaaccactactttgaccactgcgtaaagtggaacagccagaatcatccccatcagaccggcaatgtttccagcagccagcaagatgatgatgatcgtcagtggatggatttccagggattttccaatcacgtttggatagaccaggttaccgtcgatttgttgcacaatgaggaccacgatgatgttataaaccacggaccacaagccaccgtgtgaaaacgaaacgatcagtgccggggcaattccgatataagggcccaagtaaggaatgatgttgcagatcccggcaatcacacctaacaataaggcgtacggcgtgccaatgatgacatagccaatggccgtgaaagtaccgacaaacaaacattcaatcatctgaccggaaatgtatttggaaatggtgtggctcattttgcccagtaaatccatggtctgttcacggtgacgttcaggcaggaatttcttaatcgttggggctaatcgatagccgtccttaagcatgtaaaacaggaccaccggcacagttacggcgataataaccgcattggcggcagcagaaataatgccccccaagccgttggttacgccattaaaaatcgtttcagcatatttattgacatttgccgacaacttattcgtcaaggtcgtaaaatcaatcttcttgagcatctgctgagagttcatgtccttaaacagtttatcgaccaacttctgaccctggctggcagcgtcaggaatctgattggccaacgtaatcaactggtttaaaattttgggaataaagacggttgcggctaacgcaaccaatcccaacaagagtaagaacaccaacgtggttgcccaggttctggtgatttggtgcttcccgaatttgattttggtaatcaaattgacaattggattgagcatgtaaaataaaatccccgccaacaagatgggaataaagaccgtggaaaagaagatggcaattggcgaaaagacaaagttaatcttcgtagagatccagatgatggcgaccacaatcaatatttctagtgaccaaaacatcagtggggaattttttaatcgttcgaacatcgaatgactccttaccttgattatttgaatagtcataacagatcatgataattgcttataacggtaattgtaccatacatcgtaaaaggaaatgatggggctttggagatttttattcaccaggaaatcatccttggccagcgaaaaacggccacaataaaaggctgtcggcaaaatcctcattttgcggcagcccatccctgaagagttgattatttattttgacgagccagttccaaatagcgttcgtaccaaatggcgataaattctttggaaaagggtcccttctcattttcaatccaatcaacgagaatgcggacattgcgttttaagatgtgatcaatctctgggccataattccaacgcttactgaaggccaaatattcatcggcatccagtaatttgcgccggccgtctggaaagactttgacgtccaaatcataatcaatatattttaaagcttctttatccaaaacataaggtgatgccagattgcaatagtaagcaatcccatcatctcgaatcattgccaccacgttgaaccagtaatgcttatgaaaatagaccagcgccggttctcgagtgacccaatggcgaccatcgtcctcagtcaccagggtatggttgttacatccaatcaacgaattctcactcgtctttagtaccatcgtatcccgccaaacgcgatgcaggctaccatcatgcttgtagctttgaatcgcaataaactgaccttctccaggtaatttttgaagtcgtggcatgtatggtacccactttctgactaacctaaaagcatcgattgttcccaatccatttttcattatatcagagtgggcattattttcgaaattattttattcagtcagcttcgccagggcaattgtgatgtcatccatcaaaaagcctttccggaaaagtgcctgttttactttttgattgcgttcatagggctgaagtttgcgatactggcgccaatacttttctgcgacttgatcaataaccgcttgatcctttgttgccatgtcggaagtatcgacttgattcataatctcctcaatatcaccataagggaacccccgacgcatcaaaagctccttggtcttgttgatggccattttggcagaatcgcggcgatagcgtttcaactgtttttcggcaacttcaccgccaatttcaatgacctcttgagccggataatattggttcagcgaattttctgcctggtcggaagcaacgtgtttgtctttcaaatgacgccgaatccaatccgggccatttttgcgttcacggaccaccgtccgaacaaagctgtctgcgtatcgttgatcgtcaattaaggtttgatcagccaggatatcaatgacttgatcgatggcgtcctcgtcttcagtcagctcagcgagcttttgtctgacttcgtactcggttcgcaggttgtgagcgagataattcagcgcccggctgtgaagtttggaaatgttatcggcatttttcagggtttcgattaattgatcgtccagttccattcccttgaaaacccgatatttgatgaagacttcttcactgattggaaaggcgtattgaccgtccacatagacgttgaagcggcctttacgtttctgggcttcaattttagtaattgtttttgccataagcgtcctttcttttctgcgtgattgaaattcactttgtcattttgatttggtatactgagaacaatttaagatagaggatgaaaaatatgattactgctcatgtagtttacgcaacaattaccggcaacaatgaagatattgccgacatcgtgactgaagcattggaagatgcggatgttcaagtcgaagaaaccgaaatttctcaaactgacccgtccgtttttgaaaacgtcgatatttgtgttgtctgcccttacacctatgatgagggggctttgcccgaagaaggaatggacttttacgatgatctctccgacctcgatctaaagggtaagatctttggggtcgcaggttcaggggacgttttttatgaggaattttacaacacatcggttgataaattcgaagaggcgtttgaaaagactggggctaccaaaggcgcagagagtgtcaagattaatttggaacccgaccaaaaagatatcgaaaagttggatcagtttaccgccgaactggttgccaaagtcaatcaataaccagtcggttgaatcatcaatgggggaggctgagacaaaagtatacgcttttgcctcggcctctatttcttgtgatcccatattatttatcaacaacgtgcgacgacggccagcatgcttgcctagcctacatggcaatcggctgatcccggccatttaagagcacagatcaatcattccaaaaccaggaataaccgatctgtgcgcttaaattctgggatcaaaacgcctttagtcccactctctcctttttggttgtcaagattacctgcccaccttcatttatgtttcctgatcttgcgggcccgtttccaaacattttcaatggcgtcttcctgctcctgaattttgccctggcgaatttcttgaatcgtggcattgaccaccccgccaaacagcatgatgaccccggagaagtccagccagaacattaagacaatgaaagttccgattgtcttataagcatcgattctctgagagaagaatttcagataaacggtgaaggcttgggccaacagcatcaaccccaaggtggcgatcaaagcaccgacccagacatagcggaatttaactttggcagtcgggacaaaataaaacagcagacttaacagcagccaggaaacggcaattgttcctggccatttaacggtactgatcaggttcaatatccatcccgggacgttcaaaatcggcgttaaccattgaaaaaacatctgaccaaacgcaaaaaccatcatcaagacaaccagtgcgagaaccaacaccagcatccaaacgaaggaaatcagccgatttgagatcgctgtttggtcggcagcaacgccgtacgttttattgatactgcgctgaaaagccgcaatcgcccggctggctgaccaaatggtcacaattaaaccaactgataattggctggcacccccactttgcaaggtcgaattgatgatcggttccagcatggaatagattcgatcaggaaacagcggtcgcagatagacttcaacttcggtgatatgaatatgaaataagttcaaaatactgccgacaatgaagaaaattggaaaaatcgacagcaacgtatagaacgctaacacagcggcagaatcggaaacgtctccggatgaatagcgtttaataatgatttcgataaagtttttaacggcttcgtataatcgtttcatcaggcatcgacttcccgcaattattagttgaactggtctcggatcgcttttaggattcgttcggcggcatgaccatccccgtatgggttcttggcttcagccattttctggtattctttgggatcgtcaagcaggcgctccatctctgacttaacaactttgggatcggttccaaccaaccgcaaggtcccagcctgaataccttcgggtcgttccgtggtgtctcgaaggaccaacaccggtttcttaagcgacggggcttcttcctgcacaccaccggaatcggtcataataaagtaactccgagcggacatgttatggaagtccaaaacatccaacggttcaatcaaatgaactgccttgacgccgtcaaagacttcatgagccactttttgtaccgctgggcttaggtgaaccggataaaccacttcgacgtctggatggttcgccaagacttctttaatggcttcaaacgttcggcgcatcggttcaccctggttttccctgcgatgcatggttaagagaatcatcttcgagttttccttcagttcatcaaacacagaatgttggtagttttcggtcaccgtctgcttgagggcatcgatggcagtattgccggtgacaaaaatattttgatccggatgattttctttaagtaaattatcccgacttaatgacgtgggtgcaaaatataagtctgccaacacatcggtcaattgccggttcatttcttcaggatacggtgagagcttgttccaagtacgcagcccggcctccacgtggccaattttaatttggtgataaaaggcactgatactggcagagaaggtcgtggtggtatcgccatggaccaagataatatcaggctgggccttttcaataatcggatccagttcggtaatgacccgggtggtaatgtcgctcaaggactggccctgtttcataatgtttaaatcatagtccggcgtgatatgaaatacatccagcacctgatcgagcatctctcggtgttgtgcggacacaaccgtaatgggttggaattcgtctaaatgctgctgcatcagtaggataatcggggccatcttgattgcctctggccgggtgccaaagatggtcattacttttattggtttcatcaattaattctccttttatgtggttaattatatcaaaaatggcaagaaacttaacagctacttaattttgtaaaaaatatgatatggtataatctgttagatgttcatttttacatagcgaggtgggattcccacttcggccactgatttggtctgctgctccaaacggattccagcttaccaataaaaattggcaaaagcaaagtcattaacaaacgtactggaggaaatattttgaaaacgatcagtctaattgttccttgttataatgaggagccaacggttgaacttttctacaacacgacagaaaaagtattcgataaattaaacgcgtcccatgaagagcactaccaccctgactatctgttcatcaacgacggttcggcagataaaacgctggacgtgatgcggcggcttcattcacagcacccagacgaagtccattacatttcattttcaagaaacttcggtaaagagtcggcatttgctgccggcttagccaacgcccatggcgattatgtcgctgtgatggatgtcgacctgcaggatccaccggaattattgctgcaaatggtcgatattttggaagatcctaaacaagattatgacgtcgtcggctgtgtccaaaccagccggaaacagaatcccatcagagcgtttctttcagcaagtttctacaagatcatcaacagaatgtcaaaggtccagatgaaacaaaacgtccgtgactaccgcttaatgagccgcaagtacgttgacgccatcttaaagctgcccgaatacaatcgctttagcaaggggcttttctcttgggttggtttcaaaaccaaataccttgagtacgaaggggttcctcgggctgccggggagacttcctggtcgattttccagttatttgaatactcgatggaagcgatcgtcgacttttcggatgtgccgttaaaattagcgacttttgtcggcatcctgaccttcttcttgtccattatcggcctgttcttcgttgtcattcgggccctgttctttggcggatccgtcaatggttgggcatcaatggtctcgattatcctgttcctaagtggtgttcaactgtttagtttaggaattttgggaacttatgtcggtaaaatttatctggaaaccaaacatcgtcctaaatttgtaattgcggagaaacgttaatatgattgatcgattgaagaagctatatgataaatacgaagaactcattgcatacgctttttggggtgttgcaacaaccgtggttaatgtcgctgtctttgctgcgctccacctattcaccagttggaattacattatcaacgcatcaattgcgtggtttctcagcgttttattttcatacctcaccaataaagcttatgttttccattctccttcaaaatccttgaaaagcgattttttcgaaatggtttccttttttggtggcagaatcgcgacattgttattagaatttgtaatgctttggattggtatcacgctcatgcatcaaaatcaaatattagttaaaattactgaaaacattgtcgtaattgcgattaattatttctggtcaaaattattggtctttaatcacaaagatcagcccaagcaaggacggtgaatcagttgccaaaaattaacagacaaacgctcagacagcagcgacaagaatttcccgaaggctattacaccaaagcggacggcttcaagctgttggcaatcgccgcagtgatggttgtaattttggttgtggttgccaactatctcatgtaaaaacgatatgaaaaaggtcgaaacacaattaatctgtgtttcgacctttttttgaaccaattttttgtatcacagttatcgagccaactcccgttccaactgggtttgaccaatcgtcatcagccagcagaagaaccaataaaccactgcaatcgtgatgtaaatggtcatgtaatcctgattggcaccggcaacaatctgagcgtccataaacatttcactgactgtaatcatcgccgccagcgaagtccctttgaacagatccagcaaaatatttcccaacgccggaatcgcaattcgaaaagcttgtgggaaaacaatcttggaaatgacttttcggtatggtaagcccagcgagtaagctgcctcccactgaccgtgatcaaccgcactaaacgatgaacgatacacctcggacacaaaggcactacagttgatcgtaaaagcaatcaccgcggccggcaatgcatcggctcgaaagccaaagtaaataatgaacagcaagaccagcatcggcactccgcgcataaaggaaataaatgcccgcgcgggatagtgcaacaatttgtggtgacttaattgggccagcgttaagaacaatcccagtattaatgacaaaataaaactgatcgcggttaatccaatcgacatcggaaagcccgctaaaattctgggaattgaacgaaacgctaatggtgcgttaaaaaaatccggaattgataaatacttaataatatccaacagcaccgccccttacttaatcgtaaaggtctttgaaatgtggacatggggctgtttagtaacgtcagcgtgataatacttctctgacagcttcttcaaagtaccgtctttcttgagctctttgagggctttgttgacctgcttttggagcttggtattgcccttcttcatcaagataccaacacctttgccatcttcattggttctaaagtacatgtttggcatgatcttcaaagtattgttgggaacggcagccaatgctaatttctgcagatagtagtcattcataatcagatcagtcttgccgctttcaacgtctcgcagatacacatcgtttgaaacgttgttgtagttgacggtcttggcgcctaactgcttggcaagtcgttgataatcggttccggcttcaccggcagcttttttgcctttaatgtcggcccaggaatgaatgcctgaatcccccttctttcgaacaataatactgttaaatgagtgcttgtaaggcgttgataaagcgaattccttctgtctttgtggtgaaacagagaagtcattagctgccatatcagccttacccgtctttacagccgtttcctgaccatcaacgttcatttctttgaaatcaacttttctccccaactttttggcaactgcacgaacaacttcgacatcaaagccggttagcttgttagtcttttgatcatgaaatgatgttggataaagcgtccccgatgtggcaactgtcaatggacccttatctgctgattttttctgaccgcagccagtaatcaccaagcccagaaccgcaaatacgcctaacaacatcaaccaacggaacttaattctgcgcataaattgtcaacctcctaaagtttttggatcattatcattataggcatgtgaaaccgatttcacaatagctgataaattaattgttaaatattataaatcccctcaatttttgataaataattgttggtcgccaaagtgatcgtcaatttagtgttggctccaaatgctttaacgtcgcatattttagccaatcagtatttagtcatattagaattgcccttgaacgacactgagattggcatataataaaaacatttgaagtgacaagcatcacttgttaatcaattcgaatggaggcttttgatggatatcagaaaagaggctgctcaggcaaattcaaaattatcaacgcttgagaaagtcagttattctttcaccgatatggctggaaacttgctctacgtcagcatgtccagttatattctttatttttatacggatgtttttgacattccggtttcagcagcgggcatgattattttgattgcctgtatcgttgatgcggtcagtgcgattttttggggatcaatcgttgaccacacgcatactaaatgggggcagagcaggccatactttttgtggcttgccgtcccttttgcgttaagcacctttttggcatttaccgcaccaaatatttcaggcgtccccaagctcttatatgccgggattacttatgtattggcggctggagtgatttacaccggcatccaaacgacgatttccgcaatcctgccaaatttaaccctcgatcccaacaaacggattggcgccaactcttaccggatggtcggcagtctgattgggtcattcgtgaacagtacctttaccctgccgctggtagcattctttggcaacggtaatgacaagcacggcttcatgatgacaattgccatctttggcgtcgcagcaattgtcctgctgatcacggcattcaagaacatgcgtgaacgggtcccggttagccaaaaatcactgccgttcaagcaaagtttaaaggcaactgtcggcaacgtcccttggtacctcctagtgatttcttttgccaccttttggatcgcccaagctgatcggaatagtttctcgacctactatgccaaatacaatctgggtaatgccgaacttgccgcggtattcagtggtttacaagttctggggatcatctcaagcatttcaattccgtttattgttaagattgccaacaaaacagcaaccatgttaatcggcttgggaattcgtgctgttggccagacaatgatggcgctggttggcggcaacttcatcttggtgatcgtttcttggtcgatcggcgttttgggatcggctctggcaatgtcaatgccatttgccatgttggcagacacggtcgactttggcgagtggaagaccggtgtgcgggcacccggcttcttaaccgctgtgggaagcgcattctgtatccagctaggatcaggctttggcagctttattccatccaaaatcttggatatgactggctttgtcgccaacaagacccagacaccagcagcttcaggtgcgattaacttttattttatctggctgccggttatcatctacgcgattgtcgccggcattatggtcttttatctcaagtatgagaagatagagccaaaaatcaaagccgatcttgtcgcgcgtgctgaacaacgtgacgcctaatcaaattgaattgatccgataaaacaagaacgtcaacgatgaacgaaatccattcatcattgacgttcttatttttagttcgtatttcgtaaaagcgatcgaatacgccatgaccccacccggactcgaaccgggatcaaccgcttaggaggcgggtgccctatccagttgtgctatggggccaaaacaactgcactacaattttctcatttatctcagaggctgtaaagagaaattatccctccgtgcgcttatggtgcatccccttgcgtttggagtgtttgtgcttctttttgccgtgcggtttggcggggattggctttcggccagtttttttagcctcactgctccgcttgacatcttgagacgatacagtctttgaagttttgggttcatcatccaaattaaccggctgcttaggtcgagtatcagacaactgattaccatcgaagtaaatgttgctcaattcatatccgtaaggcttaaccaacttctttaaatctctcaaatcgtgatcgtcacccatattgatcaccatgccgtcttgatgcatgcggccagtccggccaacccggtgaacataagttttcggatcggacggcaagtcaaaattgaccacgacgggcagcttttcaatatccatcccccgagcagcaacgtcggtggtcaataataagcgaattttgccgtcgcgaaaatcccggagcgccttttgtctggcagtttggcgctgttcactggtcaactgagcagcctctttaatgtgtcgatgagacaggaaaccagcgactttttgcagggtgtccagttggtcaaagaacactaatgccttgaagtccttcatgtgaaggaaccgcagtaacatctgtgcctttttccgattggaaacttccagcaaggtatgtttgacttccccgcgggtatcgtcaatgtcagagacatcaaaggtctgaatatcttgcacaaaccagcgattcacatgcgccaataagtcgttttgggttgcggagaaaaagcccagtgtcactgagtcgtcagccaaatccaccaaggagcggatggaagcaagcgtatcttcacttaataagttgtcggcttcgtctatcacgatcgccttcagtgaatccaatttaagtttgcctaaatcgattaagttcacgattcgaccggtcgttccgacaatcacgtttgggtgctgttttaatttatcaacttgacgattgatattggcaccaccgataatcccttgaactgataagccgatcagcttaccccattccaataaaactttttgggtctgcatagccagttcggcagatggttcgatgactaataacgacagcccgtcttcgggttgaatattttccaacagcggtaaagcaaaggcaacggtcttcccggatccggttggtgccaaccccagaacactttggccatctttaagtggttgataaaccgcttgttgaatcgcagtcggttggttgtaccctagttgcttagcatgctctttaaattcttctatcaatatggttctccattttctaatcgattactttttctcgcccacaaatgagatgtgagcatcctgtctaagattataaattaatttattgacgtacacactgagttgacgccagtaatcataatcatgtttgttttgcgggttctttggatcgttaatcactctggcaaaatcttcaacctctggcagcattggattctcatcaatggtgttgccaatgacctgcttgttgcgatcgtcatcaatgtaaatcactgcatttatttctccggcatcatcgatttcgattaagtctttgaggccgtaaatctccgatgtcatatgtgagttggtgatctttgagaagtttaaagtcacattatactccggatactgcaaaattgctgttccttttccgtcaaccccggtccgaatcagctgtgagtaataagcagcctcttccggcatcccgaacaaggcaacggcatcataaacggtataaacgcccaaatcctggagagcaccgccggcatatttgagtgagaagacgttgggttcttcaccctccaacaccagatcatacctggaagagtattttgaatacgtgaattcagcgccttgaaccgttttaagttgaccgagctttttttcgatcgcatgaaaattttcggtgtgaatattgcgggcggcttcaaaatagagcacttgtggattctcgtccaacaaagcttgaatcttcgccatttgtttttgagtactaaaggccggcttttcaacaatgacatttttgccgtgttgaatggccatttgggcctgttcaaaatggaggctattgggtgaggcaatgtagaccgtctcaaactgccccttggtaaagaacgcattcagatccgtaaaggtttcttgggcgccgtttttggccgcaaaagttttggccgtttggtcgtgtcgtgaatagacactggttaagtcgaatttgcgtgatagtttaattgcgtcaataaattgctgggtaatccagttggttccaataattcctaatttaatcaatttgataaccgcccttctttaattaaattgtaacaaggttttaacccaatgaaaacgaaatcagacactctctgttatatttatcgactatactgggtttctactatgactagggggatgattttttgcgcaaaagaagtttttttatctttatggtgtcgtttttaattagtctgttccataccaaacggacaccgaaacaccggccagatcctgcagacccaatgtttttcgttgggacctggcagtttaaggaccaccgagagcgagtccatcgacttgaaatcggcccggatctaaaattactcattgacggaaaagatatgtctgccaaggtttcattattaaccagatatgaattgtcgtacgttgacaaatttggttataaattggaaattcgggggaatgaagcccggccaatcaaattctacgatgaatctgaaaactatacctatgatttacaatcggccaatgaaattgaacagtcaaattgagtgaggacttactgtggtaaggcctttttgttttggcctgctccatacgctttaattgatgtattcccgccactgtctgcgattaccgttaaagaccgacatcggcaaaaagatcagttgcgagtcaagcttaaagccggccttatcgtctgcctgaataaacgttgcatcggcattgggccggccaatcttaccgtcagtcaaccagaattgggtcttagcattcgcctttaactgcaggctcttgatgatttgttgggtcgccgaaatgaccaccggccgtttatagtactgtcttaacaggtgcgaaagctgccggacttcttttctggctgcctgccaatgaattgttgactgatcaaacgttccgtaatactgaatttgaatacagatcggtaaactaccggtattgtacttgacttgccggacaaagtttttgaattgggcagttggtgaactggtaaaactaaaataatggtagaccccaatcggtaactgtgaaccttggctgcgttcgaaattactctgaaaactgtcatcggtgaaggcagctccctgagtggcctttagatagacgaaactgatgcctttacttttcaaactttcaaagtcgatatagccattactttgatcgatggtcaccccatgaattgggtattttttcagctgctgattttcgtgccagcgcaacagcaaaaaggtcgaaaagccaatcaagattaacaaaaaaatgccgaaaactaccctgcgtgtgcgtttcctgcgctggtaagtttcagcatatattggttgaatgtctcttcgcttcatataaaggtcatctcagttacccgaaaaatccagttaaattaagtccgggtactttcaataatattttgaacgttgcgaatcgcatcttctgtcgccggacccatccgaaccgttgccatcataaacaacgtatcgacaattgcgagttgggcaagcagtgaatacatcccttcagaacggtaattggattcatcactagacgaaataaatgtaatatcactatgcagtgcgagcggtgagtccggatagctggtaatcccgataaccggcacctttcgcttctttaaggtttcggcaacttttaaagtttggcgatttttgcccgagtgggaaaccacgattgcgcaatcttcttcacccaattttacagcttccatcaactgtacgtcaaagtctggataatagaagcagtcaatcgacgtccgcaagaacttatgataaccgtccagggccgcaactgacgagccgccaaggccaaataagcccagacgacgacaatgaataattctgaggactgcccgagcaaattcatcttcatcaattcctgcccgggtatcttgaattgcccgctgactgctgttaaaaatcttgtcagcgatcgttcctaaagaatcgttggcatcgatatctttaaaaatcggcaggttctgcggccgtaactgcgtgtaggccagcgccaaagtaaactcacggaaattgccataacccagtgtcttcactaaccgagaaaccgaagcggttgaggtttcagtcacttctgccaaatcttcaatattggcttctgaggccgcttgaggattctccatcacatattttgcaatttttttattagttctgcttaattcatcaaacgattgttttaataattgaactggcgagctcataatgatcacctttcatggattgtaagtgtcttattttcatcaatgtaaatattttacaacaaaattcttgcattgtgaaattgtttttcatataattgtgtttgcgtttccattaccaggaaattcaatggtcgaaatatttgaagtctcccggtgataatgatatttttagtgagaagcggtaccgagccaattcttcagcactcgacattggtttaacgatgcagctatattttttgccattatttgaaagcgcttcggccgttgactcaactaatacagaagggaagttatttacatggattatacgctaggtgttgatattggaacaaccagtgttaaaaccgtgctctacgatgttaagggtaaggtgcatggatattccaacaatggatatcccctataccaggacacccctgatatggccgaggaagaccctgaagaaatcttttcagcgatgtctgacggcattaccgaattggttcgaaaggccaatatgaaaccaggagagctgaagggtgttgcattttcctgtgcaatgcatagtttaattcttctggatgagaatcacaaaccactcacccgggcaattacctggggtgacaaccgggcggtcaattatgctgataagttgaaggccagccctgagggaatggaaatctataagcataccggaacgcccattcacccgatgaccccactcaccaagctgatttggctgcgcaatgatcatgccgatctattcaagcaagcccgctggttcgttggcattaaggaatacattctttacaaattattcggtgtcttaaaagaagattactccatcgccaatgccaccggaatgtttaacatctacaatatggactgggatgaacaagccctgaaacttgccggcgttacacgggatcaattgcctgatttagttgataccacttatcaattaaaagggatgcgtgaagagtacgctaaagtgctgggaattgacatcaataccccatttatcatcggtgcttcagatggtccactggccaacttgggggttaatgcgattcaacccggggttgtcgctgtcaccattggaacttccggtgccgttcgggttgtcactgataaaccgcataccgatccaaaggcccgggtattttgctactacctagccaagaacatgtgggtcgttggcggccctgtcaataatggtggcgttgtcttccgctgggttcgtgatcaactctgtgccccggaaaaagtcactgctgaacaaatgcacatcgatccatacgacctcttgacagaaattgctgccaaagtgccggctggatccgatggcttgctgttcttcccattcctgggcggtgaacgtgccccaatctgggacgctaatgcccgtggctcattctttggccttaaccggacccacacgcgtgcccacatgattcgggccgttttggaaggtatcgtctacaacctttacacggttgctttggcccttgaagaagtcgttggtcaaccaaccagcatccaagccagcggtggttttgcccgttctgcgctttggcgtcaaatgctgaccgatattttcgaacaggacgttgcgattcctgaaagtttcgaaagtaccgctttgggggcagccactttggggatgtacagtttgggcctgattgacagcctttccgacgtttccaattttgtcggcaccacggttgttcatcacccggatccaaagaacttccaggcgtaccgggaattgattccaatctatattcgcctaagtcgttcacttcaacccgaatacaagaatatcgccgagtatcagcgtcgtcacgaacacgaagatgaagacgccgagaagtctgaatagcacctgtccgttttttatttgaaaggggaaaactatgatattaaagctgctagccttgctgatcggaattattttcctgttggttctgattatcaagttcaaaattaataccttcgtttcgttggtattaaccgctgttgttactgcgatcatgctgcagatgccactaggtacgatcgctgattccgtctcaaatggtattggaagtcaactgggcgaattgtccatggtcttcggctttggtgccatgttagggcgattggtttctgattccggtggtgcttatatgatcgccgaaacgctgatcaaacgatttggtaaaaagcgtctccagatcgccgttatgttggcttcatttattttaggaattgcgttgttcttcgaagttggaatggttttactggttccaattgtcttcgcaattgccgttgaagcaggtgtgccaattctttatttaggaattccaatggccgctgccttgtcagttacccacggatttttgccaccccatccagcaccagttgccattgcgcaggtcttgggtgccaacgatggtaaggttctcctgtttggatttgtcattgcaattattgccgcttatatcgccgggccattgttctcaaagatggctcgtaaattttcacccgctgcattcgagcgaaaaggaaacctttcttcaatcggtgaagtgaaacaatttacccctgaagaatcaccatcgtttggactgtcagtattaactgccctgttcccagttctgctgttggcgattgccacaatttataaaatgaccatcaatggtggagttgatccaaagaacccttctgtgattgattcaatcattgaattcattggatctccaagtatcgcaatgttgatttcattattcttcgcaatgtataccatgggctggggtcgtaaacgaaccactgctcaaatcatggaatcacttgaaaatgcggttaaatcaatcgccatgctgctattagttattggtggtggtggtgccttcaaacaagttctgatcgacggtggtgttggtaaagccgttgctcaactgttcattggttcaccaatttcaccattaatccttggctggttggttgccgttgttctccgaatcgctttgggttccgcaaccgttgcttcattgacagctgcaggaatcgtcgccccattgatggcccaagctggggttgacccagcattgatggttctggccattggtgccggctcattggccgcatcacatgttaacgatgccggcttctggatgttcagagaatatttcgatttaacaattaagcaaactcttcagacttggaccgtgttggaatcaatcatttcagtcgttggtatcatcatggttatgggactgaacttgattttccattaatgagagagtgtgaactcaggcgctcagcttttgagcattagtttaatacaggccgttaacgctgattttgcgtttacggcctgtattggactaagcggaaaaagctgcctgagagaacacattttaaccagagtgtgcccccaggcgcccagcttttgagcgccatttcaatcacacaaactccaaaaagactcgagcaaaccaatcatatttgctcgagtcttttgtatccagtcaattaaacccgtccagctgctccactcatcactttcattcggacggctaccaagtatgcgacaactgccttcagcgtgtcgccagggataaacaacaggcctgaagtcaatgcaccgatcagtgagatcggcgtcacccaccacagccagagggcgcccatcacgttaacaatcaaaacactgctgatccaaatgacaattagttgaccccatgaatggctcataaacggccgtgagcggcaacaacccatcatgagaggcgttatgagccaaccgaacaaatagcccgctgtggggccgataaagactgctgggccggcttgaccaccggagaggaccgggaaccccaaaaatgccagcagtaagaataccccaactgcgatcgtgccgttctttgaccccaaaaagaggcctgctaacataatccctaagttctgcatcacaatcggcacgggaatgatccctaaaggaattggtggaatcatccccaacacgataatggctgcaatcatcaaggctgtttgtgtcaattgtctaattttcatatcattttcctttcaaaaaacggttaaccgacttctatgcgccgcttaaccgtcattggatattaaattagcctgagtaaccatttccaggcagataaactttcgttacttcaccgcttgaaacggtaatcggttctccagagtcctgcttgaccaccaaggccccatcaccagtaaagtgatcagccagcccagtgatggttcggttccccatcacaatttggacccgcttaccaagggtttctgataacttggcgtattcctgcagaaaattaccgctggtgtaagtttgatacatataaaaaaagttgtcgatgagactggcagcaatccgatttttgtcaattgctgtgttggtcacaatcgccccggctttatgggcaatttgatcgggaaaatcagtggaatcaatattcaacccaatcccgaccaccacattttcatgaagaccgtcttcgagactggaaaccgtttcggtcaaaataccaccacattttttgtcatgaaccaaaatgtcgttgacccatttgacccgaaagtcctcatcgggaaaaaactgttgcagggttctgaccacgcaaaccgcggttccggtggttatcaacccagaatgaatggttcggcgattctgtaaaggaatcaaaatgctcaaatagattccacccttcgccggggaatagaaatgtcgccccagtcggccatgcccctgagtttgcgtatcagccacaaacacctgtggaatggtaaagtcctgactgctgccaaactgcttggcgtaatcgttcgttgaggaaatgctggcaaacgcatggatcgccaccggaaaagtagttgtccgataatgatcgatcacagcgtcatcaaaaaattgggatttttgataacaataacccagccctttgcgtgtggtaatcacatgaccgcggtgcgataatttttgaatattgttgtagacggccggccgactaatttgcagtttcttagccagttcattgccggaaacatagcggccagccgccgttagcaatgcatctaaaatttgtctttgatgattgaccattggccatcccccacttacaatcgtcgttaaattaaatggacacctttatcaacgtagaccacgtcaccggtcatcccagttgacaggtcactcatcaaaaaggcggcgacgttaccaatttcactggtggtgacgctcttttgatcaactgtccgtgactcggattccttcaacaattcaccatgatgtttaatcccagtaactgctaaggttttaaccgcgccggcagaaattgcgttgacacgaatgccattttcgccgagatcagatgccaggtaacgcacgttggcttccaaagcggccttggcaacacccatcatgttgtaatttggaattgcccgggttgagccaaagtaggtcaaagttaaaatgctggctggattattcaagaccggttgggcataacgtgccacggcaatcagtgaataagcactgatgttttgtgccaaatcataaccgtccttggtcgtgttgaccagtccggaagtcaaagtatccttgtcagcataagcaatggcatgaatgaccccatcaattttgccatactgattgccgatagtttcaaaagcctgcttaacgtttgcgtcatcggcaacatcacactcgatcaaatccaagtcgtccggcacaaagcgttccaaactttttttaatgcggtcattttgataggtcaaaataaccttggcgccttgatccaaaatcgcttgggtacagccccaggcgatactgcgtttatttgcaacccccatgatgacgattgtctttccatctaaaaagccactcatatttgagcctccaaatcttatcttcaattaaaaattccggtaacgttgatttcgacggtccaccaaatcatcaattggtaacttggccaattgagaaaattcctgatccaagaagtcacgtaacgcactcaaatcttccccgggttgatactcatgaataattttatcaataatgccatctgctaataatgcttctggagttaatttgagttcttctgcggcttccttgaccttggatgaatctttccacatgatgctggcgtatccttccggtgagagcaccgaataaatgctgtcttcaaacatgaagacccgatcgccacaggacagtgccaaagcaccaccagagccgccttcaccaacgatgatggtgatatatggcaccctgagctgcatcccctgaataatattttgtgccaccgcggacccttgaccatgatactcggattcaacatctggccaagcaccgggggtattcaccagcgctaaaattggccgatgaaatttctctgcctgcttcatcaaccgcaacgccttgcgataaccttgaggcgttggactgccaaaatgtctggcaatattctcatcggtatctgatcccttttgaatcccgactactgtgattggtttatcattcaacaagccaataccgccaatgattgccggatcatcggcttccagtcgatcgccatgctgttcaaaaaagtcactggttaaatgattgatcaactcggcagtcgtgattttatcaggacggcgagctgctttcacccgctgatatgctgttttatctgccatagacgttctcctttgtgtgcagagaaattaagcgactcaaagttgctttcatttgtttacgcggcacaatcgcatcgataaagccatgagccatcaccgtttcagcactctgaaagtctttggggggcttttgcataatcgtctgttcgatcactcgccggccggcaaatccgaccaacgcgtgaggctctgctaaaatgacatcaccatccatggcaaaactggcggtgaccccgccagtcgtgggatcgcataagacaacgacatacaatagtccggcccggctgtgttccgcaaccgcccccgatactttggccatctgcatcagcgaatgaattccctcttgcatccgggcaccgccggaagcggtaaacatgatcaccggcaattttttccgggtcgcttcttcgaacaatcgcgtaatcttctcaccggttgaacttcccagactgcccatgacaaagaatggatccatgatgcccacaccgacctgctgcttatcaagggtgccaatacccgtgaggacactttcgttgattccggtgacttttttagcctttttcaccttggccaaatacttttcatcagtgtactggtccggaaccgtcattgatttgtcaatttcatcaaatgaatcaaaggtaattttggcccgtcgtttggccgtgattcgaaaaccataaccacaattgggacaggttttcgtgctgccagcccttaatgaaaaaaaggttgcgtgacaaattgggcattcccgcagcacatgatcgggaatggcatccatccgctttaccagttcttcatggcttggcatattaaaccgactgcgtagcatggaatccctccttatcactcaacacttcattttgaatgtaactggtcgaataaattccctgatgaaatttgtcggtgccaatcaaataatccaaaaagctttggttggtccgaatgccgtcaatttccagttcccctaaaattcggtgcatctttgagataacggtatcgcgatcgttcaaatgaacaatcactttggcaatcattgaatcatagaacggcgaaataaagctgccgttggtgacacctgaatcgattctgacgccgagtgaaccggcggggaaaaataaatgattaatctgaccgggttgcggggcaaaattattagtcggatcttccgcattcaaccggcattccaaggcgtgccccttcacggcagcatcggcttgggtaaacggcagttcttctccggcagccaccgccaattgccctttgaccaattcaattccggtcacttcttcggtaattgtgtgctcaacttgaagtcgggtattcatttccatgaaatagaagtgatgctcatcgtccattagaaactcataggttccggtattggtatatcccagcttaagcgtggcgttggcgacaatctcacccaaatgccgccgctcttcagctgaaatcaaaacacagggactttcttcgatcactttttgatgattccgctgtagtgaacagtcacgctcaggcagatagacgacgtggccaaaattatcggcaatgacttgcatttccacgtgtttggcctgacgaatcaacttttcaacatagatatcttcgtcgtcgtatgaaattcgggcttcctgctgggtctgctcaaaagcatttttgagttcttcaggtcgatcaacttcacgaatccctttaccgccgccaccggctgctgacttcaacaacaccggaaaaccgatttggtccgcgacttgttcggcttgggcaaccgtattgactaccccgtcacttccgggaatcacagggaccccggcttttttcatcgcttctctagcgttggccttgtcgcccatcagagcaatcaactcatggcttgggccgatgaatttaatgtggcaggtttcgcataattctgcgaactcggcattttcggataagaatccgtaaccagggtgaattgcttcacatccggtcaaattggcggcactaataatctgggccatgttcaaataagattcactgggctgcggcccgccgatacagatggcttcgtctgccaaatggacaaacaaggcgtctttgtcggcactggaatacacggcaacagcggtaatccccatatcgtgcaaagcgcgaataatttgaacggcgatctccccacgattagccactaatacttttttaaacatgcgctcacctctattactcaactgcaaaaattaaatctgcttcacaaatctgctgtccttctcgatgaatggtgccgtggccaaggccaatattgtgctttaacttctttaattccacggtaaaggtcaatttgtcaccagggcggaaatcatcttggaagactgcattcttgatgccgccaaaaaaggcgtttttgccttgatattccggcattgacagaattgcggctaccccggtctgggccatcgattcgatcataatcggccgtggcaccactaggttattggcttgtttgttggcaaaaaaccattcattaattgaaatcagtttaacagcaacggcactctcccctggcttgacatcaataaacttgtcaatcatttggaaggggtagcgctgtggaatcacatcttgaacatctggtttcatctcattaccccttcgttacttgaaaaattggttgatcgtattcgaccatgctgccatcttcaaccaaaatgttggagatcgtcccggtcacatcacttttgacctcgttgatcattttcatcgcttcaatgacacaaaccacatcgcctttttcaacgtggtcaccctgcttcttgaaagccggcttgtcaggacttggggcaaagtacacaacgccaaccagcggtgccttgatttcggcaacgttttgggcgaccggtgtttctggctgctctaccgtggttggttgactattttgtccatggcctaaaccatttgtgctggcagatgccgcttgcgcagaatcttccacgatggcgtggtcatcgccctcccgtttgctgaacttaagcttgaagtcatcttgagccaattcaaaattcttcagtgacgaacggtcaaatttgtctaataaacgttcaatttctttctcatccattacctaatcacaccctttaaatgcaattacggcgttgtggccgccaaaaccaaacgagttgctgatggcgtagttgacttcggcatttttattgctgtcgtcaaccagctccacgtcacattcttcatcctgattaaccacaccgacgttgacaggcatttggttatgcaaaatggcaccaattgttgcaacggcttcaatggcaccggcagcccctaatgcatggccagtcattcctttagtgctgctgaccttgacatgatcattattggcaaagacttcgttaatcgccttggcctccgcgctatcattggcgtgagtactggttccatgggcattgatgtaatcaacctgggtttcatcaatcccggcttctttaacagcctgttgcatggcacgtttagcacccttaccttctgggtccggcgcagtcatatgataagcatcactggttgtcccatagccgacaacttcggccaagatcttggcaccgcgagcttttgcatgatcgtaatcttcgagaattaaggttgctgacccctcacccatgacaaacccattacggtctttatcaaatggaattgaggcctttttcggatcggtttccttggaaagagcggtcaaagcggcaaacccggcaatcccgatttcgttgacggaggcttctgtcccgccggcaatcataacttgggctttgccctgcttgatgtattcaaaggcgtttccaatcgcattggtacctgaggaacaggcagttacgattgcttgactggtattcttggcattaaaggcaattgaaatgttaccagcagccatgttaatgatggagtcaggcacgaataatggtgacacccgtttgggactcttatcatgcatcttgatgacctgttgttcaattgttgtcaagccaccgatcccggaaccataaatgacacccagttcttcggggtcaacgccaccgtcaatcagtccagcattttccatggcttcagtggcactgtacaacgcatatgtacagaagaggtcatttcgtttggcaaacttcttatcaacccgttttaaaggatcaaaatctttgacttcaccggcaactgtaatgccagtgggctctgaatcaaatttggtaattggggcaataccaaccttggatgcaaacagattttcaagaaaactgtcaacatcgttgccgattggcgtcacagcgcccaaacctgtaacaacgactctactcatttaattactcctttaacaatctaaattgtcaacccgccatcaaccgtgatgacttggccagtaatgtattggttacccaccaaaaaggcaacggcatcggcaatttctgtcggttcagcgaagcgcttcagtggaatttgatcagtgaattcgctttgtctgcgttcactcattttgtcagtcatatccgtcttgaccattcctggcgcaacggcattggcacgaatattgcgcaatgcgccttcgcgggcggccgtcttggttaacccaaccaagcctgctttacttgcggaatagttggcctggccaaggttgccgtggaggccggaaatactggaaatgttgacaatcgagccttttctggccttttgcattaatttcatcgcaaacttggtcatgttaaaagcgccgaccaagttagtctccaagaccgcctgaaaatcggctaatttcatccgactgagcaatttgtccttggtgatcccggcattattgaccaaaacatcaatttggccatatttttcgaccaccgaattgatcatttgctcagcatctgcttcactggcaacgtcgccaactaagacatcgaatgaatacccggcagcggctaactgctgactgtcttcgtcgcttaattcatgatgggcattgataaccaccgtcatgccatcgtcagccaaccgtttggcaattgccaaaccaattcctttggcagccccggtcactaacgcaacttgttttgtttccgtcattatttcaccagctttttgtttgatcgaacttgatttaaggtttccacactatcgacatggaatttgtcagcgttacaaatgagcggcttggcaaatttcatcaaggtatcaccagggccaatttcaattaaaacattggcatccaggttcaataattccttgaggcattcgttaaaatgcgttgggttgacgagttgattaaccagcgtttgcttgacgttcagccgcgtaaacggcttgataatcgtattgctgaacaccggaaaatcgggatcttgaaaattgaccgtctgcagtcgctttgacagctcgtcgctggcttcctgcataaatggtgtatgggaagccacggtcattttcaaaggaaccacccgcttgatgccgtgctcatggagatactcggtcgcagcgtttaaaccggctgccgatccaccgatcacaatttgggtatccgtgttgtaattggccggatagaccggtccgacttttgagccgacccggcaggcctcatccacaaggttggcattagcttttaaaacagctgccattttacccggataatgctgtccagcctgatccatatagtgattgcggtcgccgaccagcggcagaccatcttcaaagctcagactgtcagcggcgatcaggccgctatattcgcccaagctcaatccggtggcgccgactggctgccctaaatcatgcgccagaattcgataaattcctgtactcaggatgacaattgaaacttgtgtattggcgggatcatcaaaaatctttgaatcactcatgtcttttccaagtatctgagaagcttcttcaattgtttgacggtaaatcggctcctgctggtagagatcctgtcccatcccggcaaattgtttaccctgaccgctaaataaatatcctagtttcaaattatctacctgcctactttctgactacttggtttgttgttttaaaacgtaatcaaccaactcgccaacggtttccataccttcatcggtgtcaatttcaatatcgtaagtatcttcaatcttgtcgacaacttcaaagatgtccaagctgtccaaatcaaggtcgttcttgaagttggtatcttccttaaccttgtctgcgtcaacgtccaattggtccacgataatatcttttaccttgttaaatacttcttctttagtcattttaatttcctccaaattttatgttattccaatttttatttttagtacttgataatcattgtgccaacagttaatccgccgccaaatccggatagggcgatgacatccccccttttaatgcgttgtttggcgaccagctcagcaagcaaaatcggttcgctggccgctgatgtgttgccatattcattgatattgacaggaaattgattcatcgaagcgcccaaagtatcggcaatcttttcgatgatccgttcgtttgcctgatgtaagacgaagcagtcgatgtcatcaatggtcaggtttgccttctcaagggcacggttaattgattctggaacattcttaaccgcgaaaccataaacgcgatggccattcattttgaaaaatggcgagtagctggtttccggtgcggcaaatggtgacttaacgccaacttggccagctgttaaatgcttacccagcttacccaacgtcttcaagtcctcagagataaacgaaccggactcactagattggttggtcatcaataccccagccgcgccatcgccaaacaagacggccgtcgaacgatcatgccaatccaaaagcttacttaatgtctcggccccaatcaaaatggcgtgcatcggccgatcagctttcaacatctgacgaacgaccttcaagccgtagacaaaccctgagcaggccgcgtcgatatcaaaggcaatcgcctgatcagcacccaggttgccttgaaccatggcactgactgacggtgtcaaataatccggtgacatggtagcgacaacgattagatcaatctcagtgggtttgaggccgctttttgccaacagctttgtcgcaaccgcggtcgccagtgaactggtcgtctcttcaacggcaacgtgacgccgcttgattccggttcgttgagtaatccacgcatcagaagtatccatcatcgatgaaagctcatcgttatcaaccacgcgctgtggaactgaactggcagtctcaatgattttgaaatcttcaaaggtcattttgcagatacctcatcaataaagtcttccaggttaaccatcgcctgcttgatcaaccgaatgtcgtcatcgtcaaagcccctcaagaaccgtttgaccaacaatttatgaaacgcgtcatgggcccgatacaacaatcgccccttactggtcaatcccagattgataatccggtgatcttcctggttggcgattcgcatcacataccctttgcgttccaaattattcaaattggcggtcaaagttcctttgctcaatttcaaaatgtgggccacttccgaggttgtctttcgatcatgcaggccaatggtatgaaccaagtgaacttccttcgcagtaatgtctttgaaccgactttttcgaatttcgctctcctcaatccgcatgatgctgtcgtagacgttgatgagcgactcattgataaagtcggtatcttttttaatttcatcactttgcgaattcatttcttagctcccctagactgataattaaattttcttctttggatcagggacaataaaggttaattctgcagagcaggcgactttgtcatcaaccttggcttcacacttaactttgcccatgttctcacgctgcttttccatggtaacgtgaagttttaagacatcccctgggcgaacaacttttctaaacttggcattgtcaattgcgccaagataagctgttttgcctttgtacttttcagttttcaaaatcaagattgaagccgcttgagccaatgattcaataatcaagacaccaggcatcacgggatttccggggaaatggccctggaaaaattcctcgttaatcgtgacgttcttggtaaccacaattgactcaccggggtttaattcatcaactttatccataaacaaaattggataccggttgggaattaaatccataatttcagatgcatctaatacactcattgatttcttcctttcacttacagggtggtcaatgccatttaaaatttagttcgactatcaaactattagctaaaactaaacgctcaaaattgacatttaccgaggttcttttcggaacacacaacataataacctaatttagtttgaatatcaaactaaatttcaataccacgtgttgcgtttctgaagtttaccacaaaaggccttctgtgactagtcgtccggaaatggcagacgtctttcttttgaacttgcgggttggcctaacaaaaaggccgagacataactcattatcggttatatctcggcctcgcttatgtgcgacttttgtgaattccactgttatctagttaaaacgtgggaaagaggacagcaactaaatttaaggcgctccagccgaaaatctgactcggtttcctggtgtctttcttttatttggattaaacctgtgaaagaggacagcaatcgaaatttaagccgctccagccgaaaacctgactcggtttcctggtgtcttacttttatttggattaaacctgtgaaagaggacagcaactgaattttaaggcgctccacccgaaaacctaactcggtttcctggtgtcttacttttatttagattaaacctgtgaaagaggacagcaatcgaaatttaagccgctccagccgaaaacctaactcggtttcctggtgttttactgttatttggattaaacgtgtgaaagaggacagcaattgaaatttaagccactccagccgaaaacctgactcggtttccgtctggagtggcttaaatttcgattgctaaacgtcctctttcacactctgtttttattcaactgtttcataaaccaacgttggtttgttggcggactcagagatttcaatattgtcatacaaccgcttcttaatgtcatcgacatcgtcacgattgctatatattgtcagcagtgactccccggctttgacctggtcgccaatcttcttatgcagcataatgccaaccgcgtagtccagctggtcatcggccttctgccggccaccgcccaagagcatgctggcaatccctatctcatcagccacaattttggaaacgacgccgctgcttggtgcgggcaggtcaatcttgaattgagcttgcggtaagacatgttctggatcgtcaatgactgccggatcgccgccctgatccgcgatcattgcgcggagtcgctccaacgcctgaccgttatggatcactgcggtacatttttgctggccttcttcagtcgtttccgcttggccacccataactgccatgtagccgccaatcacgacgatcaatttttccaaatctgccggcccattgccctttagcaaatcaattgattcttggatttccagcgcgttaccaactgcatcacccagcggctgattcatgtcggtaatcagcgccatacactgcatgccgacacctttgccaatctcaaccaaggctttagccagcgctcttgaatcgtccagggtcttcatgaaagctcccgcaccggttttcacatcaatgaccagcgcgtctgcccccgaagcaatcttcttactcataattgaactggcaatcaatggaatagagtcgaccgtatcggtgacatcccgcaaggcataaatctttttgtctgccggggcaatattcccagttgcgccaataattgccagttggtcttttttaagttgggcaataaagtcatcctcgctaatttcaacctgataccctgggattgcttccagcttgtccaatgttccgccggtatgtccaagcccccggccggaaatcatcggtaccggaattccaagagcggctaccacggctgccaatggaatactcgtcttgtcgccaacccctcccgtggaatgcttatcgactttcacgccgggaatttggctcaagtccaaatggtcaccggatttcatcatcgtcatagtcaatttggcttgttcctcgctggtcatcccttggaagaagattgccatcaataaggcactaatttgataatccggaatgtcgcccgaaaccaccccatcgacaaaaaattgaatctgctcatctgtcagctgtttaccagctcgtttggtgtgaattacgtctaccattctcattgtggattctcctttgatttttcatttaaaataaagcgttttcatttgagtgttgaacaaacgcccaaccctgattggttcgaatatggattgggcgttgccgttaataatctagtaagagttgtgccaaactttgatccagaattgcgcaattggtgtagtgcgcattgattgccgcatggactgctgccgcctttcgattgccgctggcgaccaagattgcgtgcggcttatcttttaaatcatccagctgaatgccgatggtccgatcgttgatttcttttgagacaatttggccattttcatcaacaaagcgtgaaaaaatatcgccgacagccagtcgctgaatttcagctttttcctgatcattgaaatacccaagttggaaaatcaatgcctctgatcgaacagtcccgacagtaaacaaggcaacgttggctcggcgcccaagatcaagaatgtgtttgatatgccggtcggtttcaaccatttccttggtgacttggttatcaaatatcaccggcagcggcagatactcgggatgggtatgataggcttttgccaattcattgacagactcataggcccaggttttttcctgggaatgactgatactacctttgagttgaaccacctgaacgccggcaatatcctgctcttcgagttgcttggtaaccgaatgaatggtttccccccagccaatcccgatgatgtcaccagcttgaacgttggcagacaaaaagtcggcggtatagcggccaacaccgtcttgaatactgacggtcccgccgtaattgtttggcaccacatggaattcaattccgtacttatcactcaactgtttggacaacacctgcgaatcaaccaagggattgacaatctggatcttcaccaaaccgttatccttggcatattgcagcaatcgtgacaccgtcgggcgggagacccccaatcgagcggcaatttcgatttgactcaaattatcctgaaagtataattcggccacgcgcaagctttgtttgagtttggtgatgtccttaatttcatccatgtgatcgctccaatttctctttatgacatatttttaatggcggtttccagtgataatctggccatttcatcaaatgacgtttcccgttccttggcggggagggcttcgccggtcagcaaatgatcactgaccgtcagaatggtcagtgcgcgaatgtgatgtttggcagccagcaaatatagcccggaggtttccatttcagttgccaaaacgccataatcaattaatttgtggatatccaactcatcgttgtagaaacgatcagcggcaaaaatgttgcccaccttggtgttaattcccatttgttgcgcggtatggtaagcggaatccagcaggccaaaatcagcaattggcgagtagtacattcctgggccaaaggtgttttgaatgatcgatgaatcggtggtcccggattggaccaaaatgacgtcacggatcttcacgtctggactcatcccaccacatgacccaacccgataaatggtcttaaccccatattctttaatgagttcagtcgtataaatagccaaggatggaatccccatcccagatccctgaaccgaaattcggtgacccttataagttccagtatacccgaacatgtttcggacttcactgtagcggacaggattgtccagataagtttcagcaatgaactttgcccgcagtggatctccaggcattaaaactgtgtcggcgatttcgccgggctttgcgccaatatgtgtactcatatgattgcctccgtttatttcaaatcagccagaaaactatcgccaaccccattgccggcaacgttaaagttatccagcacggttgcgccaaaatcggcaaaggttttacggatgcctaagctatcggcatgttgcattgaaggtgaataggccagcaatggcaccagttcgcgggtatgatcggtgcctttaaaacctggatcgttgccgtgatcggccgtgatcagcagcaggtcgtcgtccttcaaattcttcagcaccgttcccaaacgtttgtcaaaatccattaaggcttggccaaagccaatgggattacggcggtggccgtacattgcgtcaaagtcgaccaagttggtgaagcaaaagccggtaaagtcttctgccatcacgtggtcaacgtgatccatgccgtccatattactttcattatggtagccttcatcaattccgtggcctgagaaaatatcgttgattttaccgatcccaacggtgtggacccccgccttctgcaggtcgtccaaatcagtcgtgccagtcggctccaacgtgaagtcgtgccggttggcagtccgagtgaaatgatccttatccggaccaacgtatgggcgtgcaatgatccggccaaccgtgtattcgggaccgttgaccaacgttctggcatactcgcaaattttatagagttcttcaagcgggatgacgtcttcgtgggcggcaatttggagaactgagtcaccggacgtgtaaacaatcagatccccagtcttcatctgttgctccccgagttccgcaataatcttggtgccggattcgggccggttaccaataattttacggcctgaaaaatctgccaagtttttgagaatctcttccgggaacccatttggaaaggtgctcaagggcttttcaaccggcaaccccatcatttcccagtggccgtccatactgtctttgccggcggaaatttcttgcatcttaccatagtagccgattggtgaagtcactttgtcgacgccttcaattgccgtttggcgcaaattggaaatgccaagtttttgtaaattgggaatctgcagctttccctcataagcctcgccaacgtgtcccaaagtgtctgaaccgacatcgccgaatttagcagcatctggtgcttcgcctgttccaactgagtccattacgatgccaaaaatgcgtttatatttcttaactgtcatctaaattcctcccctacaaccagctgcttaagataaaatcttgacggttgcgctgacacctaaccggctggcaccagcttcgatcattgccaaagcttcttctcgagaatgaattccaccggaagccttaacgcccaacttgttgccgacagtctttctcattaaggcaacgttatgaagggttgccccttccgagctaaagccggtcgatgtcttcacgtaatcagcaccggcagcttcagaagcgtggcaggcgttgacaatttgctcgtcgttcaataatgatgtttcaaaaatgactttgagcattttgtgcttggcgtgaaccgcttcagcaacggcttgaatatcggcagtgacgtaatcgagattgccgccgatcagttcaccgacatttaaaaccatgtcaatttcttcggcaccgtcatcaatcgccgtaatggcttcgtaaactttggtttcagtgttggttgccccgagtgggaagccgacaaccgtaattgggttaacagttgtgtcctttaaaagctcggcggcaagtggaatccagtgtgaattgatacaaacagaagccgtattatacttgattgcttcttcacaagtttggcgaatgctggcctcagttgcctctggttttaagtttgtgtggtccaaatactttgcgagttgagcagtcgtaatttcttttgtcatggtcatgtaacccctttcatttctttacaaggatagtttacaggaatttagaacatatgtaaagatgtttgttgaaattttgttctgttatgtgaacttgtgagcttttagtgggttgataaaagccatcgtccttgaggggcggtggcttttgggaggtgggaatattgattagttttactttctgttgttgaaaacatccatggttgcttgtgcatgttaaacgagctggttggtggagatatcgataatccgagccttggttgtccctacttacatagtgaaaatgtgctccgacgaccctgatccctactgcataaagcgaacccttcaataaggcacagaaccacgccttattgaagggttcactttatgctccgggatcacccgggtctcgtcgcactctgttctgaaatgtgctcctcagcccagcccctaacgcataaggccgaagcgcaaatcgataagcacaccccgcttatcaattcgcccttcggccttatacaccggggctaaccgggctgactcgcactctacttcaagtctccaatcgtattcacattcttcatatacgttgggacagccaagccgaccttggcgccatgcaagttgacacccaaatcgtcaaacttgcccttgtagtccttataatacagtccctgagttgtcggcagccaggcacttaccatcccatccgctgcatttgtagcaattgatgcccacagtggttggacttccattgcttggatttccaccttgtaacctaatgaccgcaatacgttggccaccacattggttgaggcaatttcagaatcccaggcgacatacgtcagcttgatcgattgaccatgcacgtgggcaatgcccttcgtccaggtatcaacctgcttttgattagccttgatccaatcattggcagctttatgcggatcttcgccattgttgactttcagcatcacatctgccatttgttttggccgccaattaaagcggttcagcatttcgtacgcctgtggtttgtccttcttcaatccttttcgaacgatggtgtgaatgtcttcggctttgccgtatacgttcttaggatctttcaaaaattttaaattgtatttggtaaacatccagtgcggagtccagccggttacgacaatcggctgatgatttttgatggctttacccaatgtactggtcattgccgcggtggaactggtctgcagctgccatttacctttgtccaaaccatatgccttcatagccttctgcgtactggacatgatcccggcaccggcctcaatcccggtaattgtgtagttgatctgcttgccaaggctttcgttagcatgataccgagcaggcttactaccacatgccgaaaggagaatcatcgagaagaacaaggcaatggttaatagaaatcgattgttcttttttcgcatagtaacccccttctatgacttagggacttttgtgcggttaatcgcctgggtaatccggtcaaggatgattgccagaataacgattgccaaaccggcagcaaaaccgccaccagcatcgtttcgaccaacggcaaagtagaccttgtttccaagtcccatcgccccaatcatcgaagcaatcacaaccattgacaacgacagcatcatactttgattaacgccggccattaaggttgatttcgctaacggtaattgaaccttaaacaacttttgccaacccgtagatccataggaatccgctgcttcaatcaagtcattgggcacttgacggattcccaggttggtcattcgaaccgtcggtggcattgcaaaaataacggaggcaatgacccctggaaccataccgatcccaaagaaggcaactgccggaatcaaataaacaaaggctggcattgtttgcatgaagtccaaaattggcttattgatcaccgcaaaaacttttgatttagccatccaaattccaagcgggactccaatcaccaacgcaatcaaactggatgtcagaaccagtgtgagggtctgggtcatatcccgccagaaaccttgattccaaatgtaaaggagaccaatggcttcaaaaatcagtaatgtccaatgcttagtgttgcggttcagccagtaggtggcccccagaacaatcagcatgaacagccaaatcggcaggatgtcaaagacccattggaaaccgttaatgatgccgccgataaaattggtgacaccgttaaagaagccttcaaagccggcaagccagtcgacaaatttatcaatccagctggagactggtaattgtggaatgttattcatcctctgtcacctcatttcctgaaatggcgcctagaacggcacctcgaatgatgattcctagtaaatgtttttgatcgtcaagcaccgcaaatggaatcggtgtctgcgagattttttccataatctccgtaatcggtgtgtctggatgcgtcgttgggacatcggtttggacaactgacatcagatcagggtttttctgtttaattaatcccatcacgtgatcagcatccgcaacgccaacgaattcccgcttactattgacaacgtaaacagacgaaatttcattctcacgcatccgacgcattgcgatccgtggaccatccttatcgatattgacaaaagttgggcgaatcatcacattggaagcagttaagaccttcgtccggtcaacatcttcgataaatttctcaacgtattcgtcagcaggctgagtcagaatctcttctggagtcccggtctggacaatcacgccgtccttcatgatcataattcggtcaccaattctcagggcttcgttcagatcatgagagataaaaacaattgtcttgtgtaagttctcctgcagatccagcaattcatcctgcatatcttttcgattcaagggatcaagggctgaaaaggcctcgtccatcaacagaatttcagaatcagttgccaatgctctggctaacccaactcgctgctgcatcccaccagagagttgggttggatattggtcgtcgtagccgtgaagaccaactaattccaaggcatcgtgggccttttttaagcgttcatccttgtcgacgcctttaacttccaatccgtaggcagtattttcaatgattgtccgatttgggaataacgcaaaattttgaaagaccatgctcattttgttgcgacgaacatccaacagctcttttttatttaggtctgtcaaattctcgccatcgatcattaccttgccggatgtcggctcaattaagcggttaatcattcgaatcatggtcgacttaccactccctgataatcccatgatcacgaagatttcaccatcattgacctcaaagttggcatcgctaacaccaaccgttgccccggcattttgtaaaatttcagcttttgacttaccttgttttaatagttcttcagctttttgaatcctgcggccaaagattttggtaagatgttgcacttgtagttttgctgtcatgtgctcctccttacatcattcaggataaataaaaatcaattaccggcctaaagcacaaacgtatgtggaagccagtaattgaacgacttataaaaccttaacaaaaatatgcattcagttcaaccatttagcaaatccgtcagattccctcactgggggattgtaaccggttttatggttgaccttatctacataatagcaattttatacatttgcactgtatcttgttgccggggttgctacatttacttttagaataggatttcaacgggattggaaaatatttttggctttttttaaatttgctgataaaaaaagagggaatcaggacaaaagtgattgcttttgtcctgattccctcacacattctctgttaactgcaacattgaatgacctctggcaataatgaaaatcgatggaatcatcaattcgtttttgtaaattgaacaaatatccgttggatgggctcattcaacgcttaatgaccacgttccaagacggtaattgattcaacatgcacggtttgtgggaattggtcaacgggttgaatcggttgattaacctgataaccttgctcagtaaataatttaacatctcgtgccaaagttgccggattacatgacacatagaccactcgcttgggctgcattttcaccacgctgtcaatcaaactggcatcaaggcctttacgcggcggatcaacagaaatgacatccggctttaagccgtcttcctgccatttggccatttgcgtctcggctttgctggcaacgaagtgcacattggttaaattgttgagcttggcgttcttcttagcatcttcaacagcttcagggacaatttcaaccccataaacctgcttggccacgcgggccatcgaaagcgaaattgtcccgattccacaataggcatcgatcacaacatcgtcagccgacaagtcagctttcttggtcgccaaatcatataatttttccgtctgcaccgggttgacttgataaaatgagctggctgaaatatcaaacttcagtccaagcagggtatcctcaatggtactcttaccagccaaaactttatttttcttgcccatcaaggcattcgttttttcaggattgacattttggacgatacttttcacttcgggcagtgactgctcaacttcagccacaatctcgctactgcttggcagtttctctgttctggtaatcaagacgatcatcatttcatgagagtagtagccgcggcggaccatgatgttgcggacaacgcccttgttggtttgttcatcatagggttgaactctgaacttgcgcaaaatgtcacgaacaaccaccactgcctcatcaatcttgggatcttgaatatagaagtcttcaatcggcaccaagtcatgagagtgtttccgataaaaaccggtttgaagctgcccattaatggagcggacaggaatttgagccttattacgatagtgggttggatcgtccatgccgatcgtgggattaacagtcacatcaagcttcattttatcaaagtcaacttgaatttgatgttgcttgaattttaattgcgcatcatattttagatgttgaagcggtgcaattccggtttgggtgtaagctttatccaccaattcaacccggtctttactcttttgattgatcttaactacccgtccgaaggcaaagttctttttaaccttaataaccttcatggtcacgttttcggttggcagagcattttcaataaaaattgggaaatcatcaatcttggcgactcccagaccttgatacgttaaatcagtaatgtcaacgtcgtagttctggttcttttcaactggtaccatctttttcatttattcacctttttaattcctagaaacaaaaattgcgaaacgaaagcttcgtaacgcaattataacatcttattaaactattctttatcagggagtttgtcaacgcctgtgacgaagttcttttcaactcggcgcatctcattggtttcatcagagtacgcatcatcgggaatttcgtcggtattggcaaaaaattcaatgtgttgtttgagatcaacgaaagtcatcggtgcatctccaccatattcaccgtccagattgatctgcattcgatcatgaaccggcttggcagtgactttacgcacctttttatagataatccgtggatcatcgacatgccggccaccgttgaggacttttgatgctaaatggagaatttcaaccaagttgctggttttaacgataattaaagtgaattttccatcatctaacgaagcgtctggaacaatttgctcaaacccgccaaccgagtttgttagggccaggaaaaacatcgaggccttacctttaaactcttcatcgtcatacttcagatccatctcaatcggcttaatgcgtggcaacagttcagctccacgaaccaaataggccaagtaaccaaagaaggttttcaagtctgagggaacatcgtaagtcagttcggttagcaatccaccagcagcaatattgataaagtaattttcacctgctttaccgatatctatccgcagggtttggtccttcaagactaacttggcagcctcgacgggatcttctctgggaatgtgcagcgctcttgcgtaatcgttagtcgttccagcaggaataatcgccatcttgggacgcttcttcagtggcgcgatgccgttaaccacctcgttaatggtaccatccccacctgcagctaccacgagttcaaagccgtccttggcagcacggcgagcctcgtttttagcagaatccttggcgggggttgtcgcataagcgctggtttcataaccagcttgctcaaaaatattcaaaatgtcgactaacttttgcttgagaagttcccttcccgaagtaggattataaataatccgggcccgttttcgcatatccatcctgactttctatttactcattgaatcctttagcattttgttgattacttgcgggttagctttcccgtgggtttgtttcataatttgaccaaccaagaaaccgatggcccgatccttaccattatggaaatcttcaacagattgtgggttagccgctacgacttcatcaacaattggctgaagcttggctgggtctgacaactgaaccatgcccttgtcttcaacgaatttcttgggctcttcaccattggtgatggctttaaagactttcttagccatctttgatgaaatcgtgccgtcagaaattagtttgatcatggtggccaaatgctcaggggtaatcttggtatcttgtagttcaacctgattatcattcatataagcattaacgtcaccttgcaggtagttggcagccaatttggcgtcggcaccggcagcaatcatcttatcaaagaaatcagacatttccttggtctgggtaatgaccattgcatcgtaatctgtaatcccaagttcattgacgtaacgctcacgacgttttgcaggcggctcaggcagttctgattgaatctcgtcaatccagtcctgggaaatattcaaaactggtagatcaggttctgggaagtaacggtaatcatcggagccttccttagtccgcattaagatggtttggccggttgactcgtcaaaacgacgggtttcctgggcaattttgccgcccgacatcaaaacacgttgatgacgagcttcctcaaatgccaaaccttttttaacatacgtgaaggagttcaaattcttcaattcagtcttggtcccatattcctgctggccaacggggcgaacagaaatgttaacatcgacacgcatggaaccttcttccatcttaacgtcggatacacccgtgaactggataacctgacgtaattgttccaagtaggcatatgcttcatctggggaagaaatgtcgggtttggaaacaatttcaatcagtggcgttccctgacggttcaaatcaacgtaagaatattcggaagcatgcgagttcttaccagcatcctcttcgatatgcatttcagcaattccgatcttctttttcttaccgtcaacatcaatttcaacccagccatcatgggcaattggggtttctgattgagtgatctggtaagctttaggattatcgggatagaagtagttcttccggtcaaagtgtgggtggcgttcaatttgggcgtgaagtgccaaaccagccatgatgccgtcatggacaactcctttattggtggttggtaaaacaccaggatatccccagtcaatgacgttggtattggagttgggttcatcaccaaattctacaggagatggactaaaaattttggaattggtttttaattcaacgtggacttccagtccgattgtcgtttcaaaattcattagttgttacctcccatctttggtgtttgttttgcaaaatcagtttcttgttcaaatgcactacctgcttggtaaacggtcaattcgtcatatgggcgaccaatcaattgcacacccactggtaagcccttggagaacccggcaggaattgacattcctggcaagccagccaagttaaccggcagggtcaacacatcgttcatatacatggtcatcggatctgagacatcctcgccgattccgtatgcaggcgtcggtgcagtaggtgccaaaatcaagtcatagtctttgaagacattggtaaagtcattaatcatcaacgtccgaacttgagcggcttttttgaagtaggcgtcataaaaaccagctgaaagtgagaatgttcccagcatgattcgacgcttaacttcgtcgccaaaaccttctgaacgggatttaacgtacaagtcttccaagtctttgacatcttttgcccggcggccataacgaatgccgtcaaaacgctgcaggttggaagaagcttcggatgaggaaatgatgtaataagccgccacaccgtacttggtatgtggaagtgaaacttcttcaacggttgcccccaactttttgaaggtttccgcagtatctaagacggtttgcttgatgtcgtcatccagtccctgggccataaattcagtaggaattccaattttcatgcccttaacacctttgttcaatgtgctggtgaagtcgggaacttctttagtcgaagaagtcaagtcatgctcgtcgtggccggcaatggcgttcataatcgttgcattgtcactgacgttacgagtgattggcccaatttgatccaaactggaaccaaaagcaatcagtccccatcgtgaaactcggccataagtcggcttcatgccgaccacaccattaaatgatgctggctgacgaatagaacccccagtatctgaccccaaagcggcaatgacttcaccggcagcaacagcagcagctgaaccacctgacgaaccaccaggaactttggttgtgtcccaagggttatgagtaatcttaaatgcagagttttcagttgacccgcccatggcgaattcatccatgttggtcttaccaactgtaatggtgccaagtttgttcaacttgtcaacagcggtagcatcataaatcggcttgaagttttccagaattttcgacgctgcggttgtggtcaagcctttggtcaccatattgtccttaatggcaattggcattccggacaaaaggttatcagcgtcaatgcccttagcatcaacgtcggcagctttcttcaaagccccttcatcgttgacagtaataaaagcgttgatgtcattatcaaaggatttaatgttatccaaagttttctgggtcaaatccttcgcagagatttctttgttgaccagttgtttgtgaatgctggaaagtgattgatcgaaataattcattattcgttatccccgctttcatcaataatggttggcactctgatgtagccatcggccgtgtctggtgcgttatcaagcaatgcttgacgttggtgccaatcttcggcaatatcgtctcgcatcacgttaatttgatcagtcacactactggtaggttcaacgccgtcagtgtcaacttcgctcagtgtttcaaacaacccaatgatttggtctaattgagtggtgaaatatggcagttgatcgtcggcaatttttagctttgctaattcagcaacgtgttttacttgatcttcggagatcttttcagtcattgaaatccttctctcttctgaatatatccaaaatttaataacaacaataattctaccatataaagaatcgcattttttagaaattaataactattgaaaatatgggcagaaaatttcttctcattttgcttacggctcaagaaactctgaatgccttcagtcgaagataccgtaatgtcaattggtgcattggccggcaaatatcgctgggcggcattttgaatgtattgggtaaaactgatgatctcagtctgactataaaattgagtcgtgatgctgatattcatcccactgagtgaaccatcggtgtattgtgcttgagcagtcaccccactcaaattcgggaagaagccttgaatttctgatttgaagttatcaaacgaatcagcatcattttggctgggacccttcttgtcagattgtaatgggaagacgtagttcttttgattgattttgtcccacttggcaactttggtttcaccatcgtcattcatggaatatgcaaagaagttcccgccgaccaggctatcatccgaagcttgcttgtataaagcaatgatgattggaatgttcttcagcgatcgccgttgtcgcagccgcttaatcacttggttggcgatagctttaccctgctttttaacttgggcatcagaaatgtcggtttcataagttggcccataggccgtcttcttataataatcaaccgagttaatccccagtccgatggtcatccctgacaagcgaagcgatttgccgctttgagtcataaaatcctgctcatcaatttgggaaagataaattggatttctagtgttagggttggtcgatttggacttaaccggatttaagccggttgggtttgatttggattgacggcccaaccaattttcaaccgtgctggtagaaagatattgaccttcttggaagatgtattttttagttgaaaattcttttttggaaatatccaacaggccgttttcaaaccctttaatattgaactgattcgattcttgagaaacactcacaccacgagatttactggtctgataacggccattcttaatcacaccttgataatagtcggtgttcgtttggccggttaactgcgtcttggcttttgagccactggaattgctggtatccttcgacagattatcaacgcttccacacgctgccaacataaatcccgacagaatgattgaaatccccaggataatttttttcacgattcgttcctccattgtcacttttcatcggccatttcttggtggaaacgggcttcgtcccatgtctgaatgccgaggcttttcgccttatcatacttgctgccggggtcttcacccacaacaacgatgtctgtatttttggaaactgaactgctgactttggcaccatggtcctcaagccattgagttgcatccggccgggtgatattttgtaatttccctgtcaaaacaaacttcttgccggtgaagaatgaatcactttcagcaagttgttcatcagtcacacccagataatccatgttaacgcccacttgtttgagttggtcgatcaactgcttggattcaggcattgagaagtaagtaaccacgctgtcagcaatgatcattcccattgtagcaatttcggcgatatcttgcgcgcttgcctgcataaccttatcaatatttttaaaacgttgggcaattaatcgagctgccttgatcccaacatggcggattcccaaaccataaagcagtcgttcacaagaattcgatcggctgttatcaatggcagccagcagcttagtggctgatttttcaccaaatttgtccaaagttaatagttggtcaaaggacaaatcataaagtccggcaacatcggagaccatgtgtttttcaaacaactgggcgatgatttttggccccaaaccgtcgatattcatggcatccctggaagcaaagtgggttaagccttctttgagttgcgccggacactgaggattaatgcagcgaagcgccacctcttggtccaagtgaaccagcgtggaaccgcatgatggacactgggttgggatttcataggcctgactgttggcaggccgtttatctggtaagtactgcgagatttcagggatgatgtcgccagctttatgcagcttaacggtatcgccgacccggatatctttttctgccaaataatccggattatgaagtgatgcccggctgacagtactgccggctaatgtcaccggatccataaccgcagtgggtgtcaccaccccggtccgtccaacggtccattcaatgtccctaacaatcgtttgaacctcttctggcggaaacttgtatgcaatcgcccagcggggaactttaacggttgccccgagtgagcgctgcagcggtagtgaattgaccttaatcacaatgccgtcaatcccatagggcaaaccatcccgtaaatctttgtatttatcaacgtaattgtcaatatcagccatattgtgggcaactttgaaatctggattgatcgtaaagcccaattctttgagttcggcaagcatcccgctttgagtgtcagattgcagatcatcgatatcggcaacgttatacataaaagtacttaatttgcgactgcgggtcacacgtggatccagctgacgcaaacttccggccgcagcattccttggattggcgaatggttcttcaccatccaactggcgctgttcattcaatttggcaaacgattctttgggcatgtaacattcgccacgaacctcaatattgatcggtcgagtcaacttttgcggaattgacttaatcgtctttaagttacgggtaatatcttcaccaatttgaccgtttccgcgagtggatccttgaacaaagaccccgttctcatatcgaaggttgattgccaaaccatcgatttttaattcgcaattataatcaaatgcgactgaatcattttcacttagacggtcgacgaattccgccaactcttccttagagaaaacatctcccagtgaaagcatcggaatttcatggttaaccttggtaaagccggggagcgtgtggtcgccgactttttgagtaggtgaatcaggagtcacaatctgtggaaattggttttccaatgcgaccagctgctgataagtttggtcatacacggcatcttcgacacttggtgcgtcataggtgtaatactcgtcagcccactggttcaattgtttcctcagatcgccagccttagcagcggcctgttgctcggacatattttcaaatgccacaataacaccttctgttgattaattttcctgcttcttaattggggcaaatgcagccaacagccgcttgatgccctcttgcttgaatgcaatatcgagctccatatcctcgccggttccggtaaccttgacaaccgtgccggttccccaagccttgtgtgatactttatcaccaacggcccaagcgagtttgtctgcaccggatcctttagggctttcgacgacttttccaggtcgccgataagtagttgccgttgcccgcctggttcggcgatcaaacggcgtgcttaggggggactcagtttgctgttgattatccgaatggataagctctgggctaatttcgttgacgaagcgcgactctggattgttttggcgacggccatacaacattcgcgagtaggcattggtaatatagagtttttctttggcacgcgtaatgccaacgtacgctaatcggcgctcttcttgaagttctgattcgtctgctgcggctcgtgaaagcgggaataatccttcttccattcccatcaaaaagaccactggaaattccagtcccttggctgcatgcaaagtcatcaaagtcacttgggaattgtcttcttcgagactatcctgatcagaaaccaaggccaaatcacttaagaaattcactaagttctgttgaccggtttcgccctcgttttcttcatcatacttttgagtcacagaaataaattcttccaagttttcaagcctggtttgagcttccaaagacttcgaagctttcaaggtacttagatagccactcttatcgagaatttcttcagtaatttcagtgattgataattgtgccatcttctctgaaatcgttcgcatcgtctgttcaaattcagcgatcgaattttttgcacgggtagaaatctcattggctaaatcaacgtttttagcagcctcaaggagactccactgatgatcgttggcgaatagtcgtaatcgttcaatactggcttggccgatcccccgtttaggttcgttgatgacccgttcaaagctcatggagtcgtttggattagctaacagagtcaggtaagacaaggcgtctcgaatttcttttcgatcatagaacttgtgtccgccaaccatggtgtagggaatatttgatttgagcaaggtttcttcaattacccgtgactgcgcattggttcggtaaaggattgcaaaactgccgtaattgcgttttggcttggccatttcttcttgaattttggcaacaacgtatcttgcctcgtcgttttcggtctgaccacgataatatgaaatctgatcgcccttgggattttcagtccacaaatttttgtcggcacgattgtcattatgggcaatcaccgaattagcggcatcaagtaccgttttagttgaacgatagttttgttccaataaggtcacatgggcatccggatagtcttttttgaaatcaaggatgttctgcatgttggcaccacgccagccgtagatactttggtcggcatccccgacgacacagatgttacgatttttcttggcaagggtattcaccagtcggtattgagcctcattggtatcctgatactcatcaacatggatgtattgaaatttgtcctgataggattccaaaacatccggatgttcatcaaataattggatggtgatcataatcaaatcatcaaagtccaatgattgattctgcttcagctctgcttggtagcgatcatagacgtcagccacgatttgatcgaaagcactattggcctgagctttgaatgctttgggtgtgagcagatcatttttggcgttggagatagccgataaaacggctctgggatcgaactttttgggatcaatattcaaatctcgcagtactcgtttgacaagcgtccgctgctcactggtatcggcaatcgtaaaagccttattgtagcccagcaaatcaatatggcggcgtaaaatccgcacacatagtgcatggaatgttgaaacccaaacatcgttaccaccttcacccaacaattttgaaacccgttcacgcatttcccgggcagccttattggtaaaagtgatcgctaaaatccgccacggcataatatggttatgttcaattatgtaggcaattcggtgggttaatacccgggtcttgccactgccggcaccggccataatgaggacgggtccttcagtatggataacggcgtctttttgatctttatttaatcctgctaataaactttcttctgccactaaatattccatcctctcgcatttatcttttcaattataacaaaaaagtcggcttcccgactctctacatgttgctatattttgttttgtaatctatgtcatgccaaatcccagtggcctccagtttaaccagggtgtctgaaatagatttggtcggaatcaggacatgcccaaccagctgatggtcgtcagttggctcgttgccataaaacgtgaagtgccaattatctttgatgacccattgggtttggacacgttgatattcctgttgtcgaatggcctgataaaccgttgcaattccgggaataatttgtgtcaaaggcaaaccggcaattgcccgcaaatgttgttcaaattcatcggcattagcagcgtaatcaaatacaaacccagccgcactcaatttgggagcaactctgctgacataaatcgaaccgctcttggccaagaagagtgtgacttcgaaagtaccgacatagtcaaggttgttggcaatttcattggtaattcgggtcatttccttcttcacactgggatcgagttttgccggcgtataggcggtcattaactgatcgccttcatacatcacttcgactggtggaaacatcacaattgaccctgactcggtccgggtaacgaccacggagtagtcagtatcatgttccacataggattccaaaatgtaagttccggaatctaaaaaaccggatgccaggacaatatcagcctggttcttaatcagcaattctttgccgccatttagtccccgctgaatgggctttaaaatagccgggtacccaatggaattaatggcttggtaaatgtcttccaacgtgacaatcgtcgagtaaggaaccatgttaatattcagggtttcaaaaaacgttcgttcaatcagtcgatcttggacaatatccaataatccgtcccgttgcggcacagccgtgtattgggaaatgtatcgaatgacatctgaatcgataaattgattgtcatagatcaccgcttcacagcgttcggcaaacattttcaaggtttccttgtcagtgtaggggccaatgtatttatagtctgccagttccatcgccttactgttttcgttggaactgtacatgccaacattaaagcccatttgttttgcgcgagccaataacgttggggtgctgatactatctccaagaatcccaattgtttgaccgggatagataacatttgcgtttgccaattaattcactactttcatatcgtcattttattaattgtaagtcatcattaaacttatcgtaccattattttcacagctctaatcaacaaatgtgactttttggttatccagagaggcaattcgagccaaagactccaaacggacacctgatttttcaatcatggtgtgccctttttggaagctcttttcgatcacaatcccaacaccttcaactttaacatttgccaacttggcaatttccaacagtccttgaacggcttgaccatttgccaaaaaatcatcaataatcaaaattcgatcatttggcttcaaaaatcgtttatcaatactgatatcgttgctaacttgcttggtataagaataaacgctggcggtgtacaggttatcggttaaagttaaactcttatgctttctggcaaagatcaacggaacccccatatggatcgccgttgtcaatgccggggcgattccggaagattcaacggtcacaaccttggttaccccttcatctttaaataagcgggcaaattcggcaccaatttggtccatcaattttgcatcaacctggtgatttaaaaagttgtcgacctttaatacgtttcctggtaatacagtaccatcctccaaaatgcgtttcttaagtaagtccatctcaaaattcctttctagtcatcgtattgataaagtttgtattgtctgatgatggcgatcaatttcttggtataagcagggtcggtcgcatagccatcctgctgaagaccatcagcggcctgcaggtagttgtttgcggccaccacgtccttgtactgctgtgggttccatttcgtgccataggcaagcaatttggcgtgatcagccaaggattcattccagtcctgatatacttggaaccgagctttgatcgtcacataacggccattcacgaattcctgcgtattcaggtagaccgagttggtggtattatcctgagctttgacgccaaacagattataatacttgctcgcaagcttgctggtgccccagttggactccaaaatggcctgagctaaagtaatactcggtaagatattatattgcccctgcagccgctgggcttgtggcgctaatttgttgataaatttacggtgctcaatggccacttcgtcgttcgagctttgaatattgctcgaatgataaccgttttcgtacaaagcgtggaaaccaaaaatgatcaccaacccacagatcaccagaatcaacatcaaaacggcatttgctttttttgcgcggcgtttccgccccttcttatattttgccaatccaacctcaaactttctaactttaaaattaattctaacgataaatccgaataaagacaaacgaaatttgtgctttgttcaatttttataaatgcgtaaaaattgacaaatctgttaatttcggttatgttatcctctgacacttaaatctggagatgaaaaccaatggctaaaaacaccgaagtatcagaagctcaatcaaaatttcatgttggtgatgaggtttcattcaagatcgaaaaacagacgtttaccggtttcgttgataagagttacaccaactcatttttaatcacttttgaatcggatgatcctgagattatcgacaagtaccacaaaaaggttgtcatcaataatcgacatctcaaaatgatcaaggcagctccccaacctgaagttgaggatgaggacgaggacgataatgaaactaaatcccccaaagccaaaaaatcgagcaagaaataatgattaaaagtagaccctgcatatatttgtgcaaggtctattttttatctgctggtccggtcaaaaatctttttaaccggcaccgcaatcaacggtgtgacaattccgctaaagattgcttccggaacaccattcgtaccaaccacccctagtaaatatgggaggagttctttgatattaatctgatacagttgaggggctttcgccttataaaacagataaatgagtcccagcaccaggaccgtgttggttaatgaacccaagacagccgatacagaaatactggctgcctggcttttcaagtgtttcttgagatacgtgtacgtcataccagcaactacgccaatcataatccgggggatgaccgaaataatcgggttaacaaagacgattgccgctaaagggctggtcggccatacaaaagctcggacaaaagtcgtcagcccccaaacaccaccaatgatcgctccgtcaacagttccaagcaaaaccgttgcaacgacgacagtcatcgggataatcgtaatttcaagtggaccaattgggatgtacccgatcaaaggaatcgaagtttgcaacagaatgatcgcaataaacattgccagcatgttcagtcgtaaagtatttttcttaacaggcatgtgttcttacccctttaaagttgttggaaccattatacaataacggattgtattctaatacaattttgctggtgaatgtcagtttaccaacaagcttaaaatattctcaacaaaaaaacactcctcaaaagagaagtgttttgaaaaagcaaagtaaattttaacgctttgaaaattgtgaagctttacgggcctttttaagacctggcttcttacgttctttcattcgtgcgtcacgagttaataaaccggcacgcttcaatggtccacggaagtcgggatcaactgcaagcaatgcacgggcaattccgtgacgagttgcgccggcttggccggagaatccaccaccgttaacgttaaccaaggtatcatagttacctaaagtctcagttacgttgaatggttgcacaacaacttcacgcaagttagcaaatggaatatagtcttcgattgctttgtcattcatgataatttttccagttccgggtaccaaacgtactcgagcaactgaatctttacgacggccagtgccgcgatattgtacttgagccaaagtgaattcctccttaaattaggttattaatgtctaatacttctggtttttgagcttgatgatcgtgttcaggacctgcatagacatgtaacttcaaaccaattttatgacctaatgttccatgaggaagcattcctttaacggaagtttcaattaacttttcgggattcttagcacgcaaatcaccggcagttcgttgcttcaagccaccaataaagcgactgtgatggtaatagatcttccgagtgtctttgtgaccagtcagaccgactttacttgcattaattacaatcacattatccccagtatccacgttgggtgtgaatgttggtttattcttacctcttaagattgatgctactgctgatgataaacgtccaagagatacgtctgttgcgtcaacaacgtaccatttacgttctacttcaccaggttttgccatataagttgtacgcactgtatattcctccattgttcctgtgtttgttcgacaccaaataagattccggggcttatcgtggggcaaacaataccaattaacataatacaaattattctgatgaaagtcaattagtttcctaaattatcgttgtcgttttggcaatttcgtgggatgcttcggatcttcaccctcataatagactttctttaagtacaaaccggatgccggcatggttcgtcgggcctggtcacgatctttcacctcgtataagcgcaatatatcgtgctcagggcgcatttgagacccaatctcaacaactaccccaaccatgattcgaaccatgttatagaggaaaccattgccatagaactcaagccgaatttcgttggctgatttgtccaaaatcgcattagcttcataaatcgttcgaacattggatcgtgcagtcgaccccgaagcgacaaaactggaaaagtcatgttcaccaacgaaatcattcattgccgtttgaacccgttcaatatcaatgggaaaacgccaatttccggtataattccgtttgaacggatccttaaattcgcctaaatccagccgataaacataccgtttaccggacacatcgtagcgggcatggaaagtattggataccttttccgcttttttaatctccatgtcaagcggcaggagactgtttagtccccgataaattgccttggttggcaaatcgaacgggaaatcaaaatggacaacttgtccaagggcatggacaccggcatctgtcctgccagatccgtagacgacaattggtgggtcgggattttttgccatgatattcactttttgggtcaaaacaccctcaatcgttctgcgcttgggctggcgctcaaagccgctgaacaacgtgccatcataggctaacgtcactttgtatcgaatattgaacacctcaactctttcttatgaataaaacgagcaccccgactaacaaaaagactgcccaactaatggtatcttttcgctgccaccgataaatccggtatttgctgcggtgctcactgtcggtaaagccacgggcttccatggcagttgacaggttttctgcatgattgattgctccggtaaataatgggacgagcaggggaacggctgcttgaatccgatggcgtaagcttccggacccaaagtccacccctcttgaccgttgagcatttaaaatagtttccatttcatccattaaggtcggtacaaaacgtaaagcaattgaaagcatcaacgccaatgtgtccacaggaaagtgaacttttttgagaggccgaagaacggtctgcaccccgtctgcaatcgccaagggcgttgttgtcaaggtcaaaaccgtcgagatcatgataatcaacagaaatcggatgaaaataaaaccaccgttaattaagctggtatcactgactgaaaatggaccaaaatgccaatagacatgtcccccactgctgaatagaatctgcagtaagacagtaaaaataatcaaccaaataagtggcctaatcccttttagaaaataaccaatcgacacgcctgacatgaggaccactatgagaatcaacacactcaatgccacataagtccaaatgttattggcaaagaaaatcacaaccacaaaataaaagcttagcatcaatttggattggggactcatttgatgaacccaagaattgcctggaaggtaccgaccaaatagaaaattactcatggacgtgacccccttgaacagcttctacgattgcatccgccaatttgtcaattgtcagtggaacactttttaacggaacccctgcagtgatcaatcgggaagcaaactcagcactactcggcaaatccagatgcatctgatatacccactggggatccgaaaaaatctcttgcggtcttccatgtttaacaatcttcccttgatccatcacaataacgtcagaagcgtaatcaacaacatcatccatttgatgcgtgacgagaataatcgtcatgccctgatgttcgtgcaggtcttcagccaagtccataatttctttgtggccgcgaggatccaaaccagcagtgggttcatccagaatgagaatttccggcttcattgccaaaaccccagcaatcgcaactcttctcatttggccgccggaaagatcaaatggcgacttgtcttgtaaatcttcatcgatgccaactaatgccatcgcctgttgggcatcgcttctggcttcttcgtcagaagccccataatttttggggccaaacataatatctttgataaccgtttcttcgaataattgtttttccggaaattgaaataccatgccgacgtgcttacgaagttgctttaaattcttattggtggtcgcaggtgtaatcgttcgccctgacacctcaatttctcccgtagtcggcttgagaagcgcattaatgtgctgtaccaaagtggacttgccgctaccggtgtgaccgataattgctgtaaatgacccgctggcaatggttaaggatacctgattcaaagcattttgagcaaatggtgtatcagcttgataagtatgagttacttctttgaaattaattgtttgatccatgtaattaacctctcatcattgagatattgactatgtgagtcgattccacgctttttgagggctgacagtaattcggacgtaaaaggtgcggataagccaatcgatgtcaatttttcaatatcaccaaaaatatgatccggctgatcagcttcaacaacttgaccttggttgacaacaatgacttggtcagcaccggcggcctcatctatgtcatgcgtaatggaaatgacggtcagattattttcgcgtttaatctgattaaccagttttaaaatgttttgtcggccgcgaggatccagcatgctggtagcttcgtccaaaatgatgattttcggactaagggcaataattccggcaatcgcaacgcgctgcttttgtccgccagataaattagcaggaatccgatcacgaaagtcccacatgccaacctgtcgaaggctctgttcaacaatttgatgcatttgctcacgaggaactcggcgattctctaagccaaatgcaacgtcatcctctacggttgctccaacaaactggtcttcgggattttgaaaaaccatgccaatcttatttcgaatatcaaagatatttgcatcgttgaccgtcagtccatcaacaacgatttgaccagacttcaaaacgatcaagccgtcaattaagcgggccagtgtactcttcccacttccattttggccaatgatggccgtccatttaccttcctgaatattcatcgaaaaatcattaaaaagtttttcttgttcggggtaattgaaagaaatgtttttaatttgaataatatccttcatgatgttcctcacgctgtgcaaagtgttttatctatgtacaaaaaaatcacttacaggtaatcggtgcatgagataagtcccacattcaaactagactaggaactgggttccaccatcataacgttctataccaaaaacctgagtgattctcgtgataaatatgtgatttggtttaatactagttagtcaactaactctaaaatgaccattggagcaccgtcgccacgacgaggcatagtcttcaaaattcgtgtatatccaccattacgatcagcatactttgtagctaattcgccaaatactttttgcaaagcagtcgtaacgttaatatcgtcaccatcttctttaacatcagcaacaacatcacgaacaaatgatgcagcttgacgacgggcgtgtaaatcgccgcgcttgccaagtgaaatcatcttgtcagcagttgagcgaacttccttagcttttgcttcagtagtaatgatttgaccatgaataattaactcagtagtcaaattacgaagcaatgagcgacgatgtgcactactacgttgtaatttccgataacccataattggatgtcctccttctttatctttattagtcttctttacgaagtgaaaggcccaatgcagcaagcttttctttaacttcttcaagtgacttgcgaccaagattacgaaccttcatcatatcagcttcggtcttttccgtaagttcttgaacagtattaatgccggcacgtttaagacagttgtatgaacgaactgataggtccaattcttcaattgtcatttccaacattttttctttgtgggtttcttccttctcgaccatgatttcggtattcttagcttcatcagtcaaatcaacaaacatctctagatgttcggttaaaattttggccgccaaactaactgcttcactcggagtaattgaaccatcagtccaaatatccagtgtaagcttatcaaaatcatcgcgttgaccaacccgtgtactttcaacctgatagttgacacgttcgattggggtataaatagaatcgacgggaagcacaccaataggcatttcagaactgcgctttttgttttccacagcagaaacgtatccacgacctttgttggcggttaaccgcatatggaatgtggcaccttcagcaacggtagcgatgtgcaaatcagggttcagaacagtcacatcactgtcagcttgaatatcaccggcagtaacatcagcaggaccaattacatcgatttccaaattttcttcttcatcttctggcccatctaatttcaaagaaattttcttaacattcaatataatctgagtcacatcttcgacaacacctttgatcgtcgaaaattcgtgcagtacatcatcaatctggatgctggtaacagcagcgccaggaagagatgacagtaatgtacgtctcaaagaatttccgagagttgtaccatatccacgctcgagcggttcaacgacaacttcaccaaaattatttgtttcttcaattttatgaatgttaggcttttcaaattcaatcattcttatcattaacccctttcaaaacgcgtgagtcttcatgcaaaatatcaatatgcttaaaccaagtaaaattcactatattgaatgtcttaattaaactcgacgacgctttggaggacgagaaccattgtgaggtaccggagtaacatcacgaatagcagtaacttccaatccagtagcttgaagtgcacgaatggcagcttcacggcctgaacctggtcctttgacagcaacttcaacggatttcataccatgttccattgatgccttagcagcagcttcggcagccatttgagcagcaaatggtgttgacttacgacttccacggaaacctaatgcaccggctgatgaccaagaaaccgcattcccagtggtgtcggtaatcataactaaagtattgttgaatgttgaatggatatgtgcaacaccagcagcaatattctttttagcacggcgtttacgacttgtctttttgtttaccataaaaactgatgacctccttctttaattattttcttctaccagcagcaactttgctacctttacgtgtgcgggcattgttcttggtatgttgaccacgaactggcaatccgcgacgatgacgcatcccacgatatgatccaatttcttgaagtcgtttgatgttcatacttacttcacgacgtaagtcaccttcgattttaagatcgccgacaacttcacgaatcttgtcttcttggtctggtgtcaaatcacgtacacgaacatcttcagaaactccagcttttgctaagactttttgagctgttgtgttaccaataccaaaaatgtaagttaatccgataacaattcgcttgtcacggggtaaatcaattccggcaatacgagccattgagcatacacctcctgtttatgtttatttaccttggcgttgtttgtgctttgggtttgctgagcaaataaccattactcggccttttcgtttaataatcttgcaatgttcacacatttttcgtactgatggtcgtactttcatttttaaccctcctcgaaaaaaaatgacgaaaaaggactacttaaatcgataagtaatacgtcccttggttaagtcgtaaggagacatttcaacggtaaccttatctccaggaagaatccgaatgtaatgcattcggatctttccagaaacatgagctagaatttcgtgtccattctccagttcaactctaaacattgcattcggcaatgtttctacgacttttccttcaacttcaataacattatctttagccactcaatacacctccaatgttaaattagattgaataaattaaattaatcttgacaaacctttgacagtttaacacattcattatatttcatcaatctaaccgactcaacacttaattagtgaggtttagagtgtgctcaagattttgtcaacattttgccaaacttcatcaatgtctttgctgccatcgacattgaataaaagatttcgatccttatagtatgcgatcaatggtgtattcatcttaacgttaaccttaagacgatttttaacagcctctggtttgtcatcctcacgctgataaaattcatgcccaccacagacatcgcaggtaccgggaactttaggcatatggtacaacttatgataagtggcaccacagtttttacagatgaagcgacctgacaaacgctcagtcaacaacttaggatcaacatcaatgttgataacggctgtcaaaggtttatccaagtctttggtcatttgcgacaacgcatctgcttgttccaaagttctgggataaccatctaataagaagcctggtttagtatcatcttgggctaatctttcctttacaatcccattagtcacttcatcaggaactaaatcccctttatcagtaaaggatttggccttaaccccaagtggtgtactattcgagattgcatctcggaacatgtctcctgttgaaatgtgaggtacgtgatacttgtccacaataaattgggcttgagtacctttccccgcaccaggtaatcccattaatatcaagttcaatgacattttattgtcctcctaattaatagcggaattgctcaaatttagtcatcagttggtcgagtatcatgaatgaagccaacgtactctcgcttcatcattaaaccacgaatctgacgaattgtttcaatagcaacaccaacaacaattaacaggctagttccacctaacccaattgattcatctaagttccacaggttttgcgcaatcaaaggaatcaaagcaaccactccaaggaataacgcaccgacagtacttagcttcatcaacagatcagacacataagattgggtctcatgccctggccaaacaccaggaatgtaactgccttgcttttgcaaattctccgaaagcttttccgggttaacttgaacaaaggcatagaagaaagtgaacatgataatgagaattgtatagaaagctgcaccggtcggcgtttgcatattgaatagattattcaatacctggaaccaagttgcagttgagtaattgttagtgaatgccatcaagatagtttgcggcgttgcaataaatgaacttgcaaagataactggaataacaccagcaacgttaaccttcaatggaaggtaactgctgtctggggatccagaaactcgccttgtatattgaattggtactcttcgttcagcttgttgaacccaagtaacaaaggttacgatcactaacacgattatcagcaatgcaatcgcaaaaaggattggttgccatagatcagcgccagaaacgccaacaaaatactgggtccacaatgactgaagtccgactggaattcgggcaatgataccagcaaagataatcattgaaatcccatttcctaagccacgctcagtaatcatgtcccccatccaagttgttaacattgttccaccggttaaaatcaagccgatgatcacaaatgttttgatacttggattttgaacaagattcagactacttaattgattaaatcctgcggtaattccaacggattggaaaaaggctaggatgacggttaagtatctcgtatgttgatttaatttacgacgaccaacttcaccttgcttaccccattcaacatattttggaacaatgtccatctggagcaactggatgataatttgtgcagtgatataaggtgagacccccatcgcaaagatggaataattagtcaacccaccaccactaaaggtgttcaggatactaaccaaaccagaagatgcaacggatgttaatgctttggcattgatcccgggaacagttatgtatgctcccagacggaatataactagcacaaacaaagtaaaaagcattttattgcgaatatccttcactttgaatgcttttgctaaagtcgaaagcattaaaccacctcgattttaccgcccgcattttcaattacggattgtgcagcctttgaaaacttgttagccttgacggtcaactttttagtaagttcaccttcaccaagaatcttgatgcctgatttggcattcttaacgagtcctgattgttgaagtaattcaggcgtaacttccgtaccgttgtcaaagctttcaagcttaacaacatttacaacagcatattccttgcggttgatgttgttgaatccgcgtttaggaattcgacgatacaatggcatttggccaccttcgaaacctacacgagtcttgctacgagctttttgacctttttggccacgaccagcagtcttacctttaccggcagaacggccacgacctttacgagtacgtaatgaacgagaaccttcagcagccttcaattcatttaatttcatgaaattggcacctccttactaatttttagtctttaacttgttcaacttcgattaagtgagcaatttggaaaagggctccacgaatagattcgttgtctggtttaacaacggtactattaactcgacccaagccaagtgccttcacaattttacgttgctttggaaggcgatgagttacgctacgttttaaagtaatttttaattgagccatctaaaacaccctccttattcagctaaatgttgggttgaaaccccacgtaaagctgaaatttcttcagcactcttcaactcaaccaagcccttgaatgttgcccggataacgttgataggagtattggaacctagtcgtttactagtaacatcgtcaataccagctaattccatcacggaacgaacggcaccaccagctgctactccagaaccttcttcagcaggcttcaataaaattcggccgccaccaaatgttccgagaacttcatgaggaatcgttgtaccaacaatcggaacctcaattaagtttttacgagcagcttcaacggctttacggattgcttctggaacttcttgagctttaccagttccaaaaccaacatgaccgtgcttgtctccaacaacaactaaagcagcaaaacgaagacgacgtccaccttttacaactttagtgatccggttaatcgaaactacgttgtcttcaagctctaacttatctggatcaataaatttcttcatgtgcggttattcctcctttttagaattctagtccattttcacgagcagcatctgcaagagcttgaacacgaccatgatacaagtatccaccacgatcgaaaacaacatctttaatgttcttttcgctagcgcgttgagctactaatttaccaacactagctgcttgttcagtcttgttaccactactgattgcagaatcaagtgttgaggcactaacaagcgttacaccctctacgtcatcaattacttgagcgtagatgtttttattagaacgataaacattcaagcgtgggcgctcggcagtaccagaaattttattacggacacgattatgacggcgtttccgattcttattcttatctggtttagaaatcaaaatagtcacctcaaaattttattaggctggcatcttactacttaccagtcttaccttccttacgaataatatgttcattctcataacgaatacctttacccttatatggttctggtgaacgtactgaacgaactgatgcagcaaagtcaccaactgcttgtttgctgataccattgatgtgaatcgttgtgttatcaggaacttcaacagttagatcatctggaacagtcatttcaactgggtttgaataaccaacgtttaatgtcaggttcttgcccttaagttgtgcacgataaccaacaccaaccaacttcaaagtctttttgaagccagtagttacgccatcaaccatgttgctgacgttggcacgagttgtaccatgcaatgcacgtactttgtcgttgtaatcaccaatgggctcaaagttaacttcgttatctttgatagtcatcttgatttgtgatgaaatctcgcgggttaaagatcctttggcacctttgacagttacagtattcccatctgcttttacctcgacaccttttggtaattcgatggttttataaccaattcgactcattaattacacctccgatttgatgaattttaccagacgtaagctaacacttcgccgccaattttttgggcgcgtgcttgcttatctgtgatcacaccatttgatgtggaaatgatagcaattccaagaccatttaaaaccttgggaacagcatctgctttaacatacgaacgtaaacctggcttagaaattctcttaagaccagtgatgacacgttgcttatccttgccatactttaagaaaacacggataatgccttgtttgtcatcttcgatatattcaacatcgcgtacaaaaccctcacgtttaaggatttcagcgatgtcacgtttgatttttgatgcaggaacttcaactgtttcatggtaaaccatgtttgcattacgaatgcgagttaaaaagtctgcaattggatcagtcatagacatcagcgcacaacctcctttttaattattaccaactagctttcttcatgccaggaatttgacctttgtgggcaagttcacggacgcataaacggcataaatggaatttcttgtatacagaacgaggtcgtccgcaacgttcacaacgtgtgtaattctgagttgagaacttagcagagcgttcactttttacaattaatgattttttagccaatgtgaaacctcctctttatctggcaaacggcataccgaattgagctaacaattcatgtgactcttcgtcggtatttgcagtagttacaattacaatatccaaacctctaacacggttaacattatcgtaattgatttcagggaaaatcaactgttcacggacacccaaagtgtagttaccgcgaccatcaaaggcacgagtgctgacaccatggaaatcacgaacacgtggtaacgaaacgtttactaacttatctaagaagtcatacattctatctccacggagtgtaactttagcaccgattgacattccttcacgtaatctaaatccggcaattgatttcttagcttttgtaaccagtggcttttggcctgaaatcaatgctaattcagaaacggcttcatcgaggttcttggagttagtaacagcgtctccaacacccatgttaagaacgattttatcgatcttaggagcttgcataactgatttgtagctaaatttatccatcatatgtggtgtaatttcgctattgaatttttctcgtaaacgacttgacatttaaaaggtatcctcctttcgctagtgattaatcgatcgctttttgcgatttctttgagtaacgtacttttttaccatcttcaactttaataccaatacgagttggctcgttggttgatgggtcaattagcataacatttgatacgtgaattggggcttcagcatcaacaattccaccttgtggattcgtctgagaagcttttgtatgcttcttaactttgttgattccttcaacaatcacacgatcttttgaagcgatagttttagtaactgtcccttccttacctttgtccttaccactaataacacggactttgtcaccagttttaatgaacatctacggcacctccttatatcctggttgtgattacagtacttctggggctaatgaaacaatcttcatgaagttgctgtcacgtaattcgcgagcaactgggccaaagatacgagtgccttggggactcttgtcatcacggataagaaccgcagcattttcatcaaaacgaatgtatgaaccatcattacgacgagtaacagccttagtacggactacaacagctttaacaacgtcaccctttttgacaacgccacctggtgttgcttgtttaaccgtagcaacaatagtatcgccgattccggcataccttctggttgagccacctaaaaccttaatagttaacaattctcttgcacctgagttgtcggcaacttttaaacgactttcttgttgaatcacaggtatatcctcccttcatcattggatcgaatacgataataatgataattaagtaaagttaaataataactgctttttcaacaatcttgattaaacggaaacgttttgtctttgacaatggacgtgtttccataatttgaacaagatcaccggttttagcttcgttattttcatcatgagccgtaaatttctttgagtatctaacacgcttaccatatgttgcatgtttcttgtaagttgaaacttcaacagtaattgtcttatcactcttgtcagaaacaacgcgtccttgataaaccttacgctggttacgttcttcagccattaattatacctcccttatcgtattctatttgttgagttcttgttgacgaagtgcagtcttaatgcgcgcaatgttcttacgaacctgcttcaagcgtgcagtattctccaactggccagtggctaattggaaacgaagattgaacagttcatctttgtaatctttttctttatcaatcatttgagcagtggttaacttgctgatatctttagccttcatttgattcgccacctacttcctcacgttctatgatcttagtgcgaacaggaagtttgtttgatgcaagtcgtaatgcttcatgggcagttgctttgtcaactccaccaatttcgaacaatactttgccacgcttaactggtgaaacccagccagctggtgtacctttaccattacccattcgaactccgacacctttttcagtatatgatttatgagggaaaatcttgatccaaacttttcctccacgcttcatgtgacgagtcatcgccacacggcatgcttcgatttgacggttagtgatccaatgagaatcaagtgcttgtaaaccgtattcaccgaaagcaaccgtcttgccacccttggcagttccacggagcttgccacgatgttcacgacgatgctttacacgtttaggtactaacatgtttatttccctcctttagcagcgttgctgtcctttggcttttcagggagaacttcaccacgatagatccaagtttttacaccaattgatccataggtagtaaaagcttcaacccatgagtagtcaatatctgctcttaaagtatgcaaaggaacagttccatctgagtatgattcaacacgagccatatcagcaccgttcagacgaccagcaacctgggtcttaattcctttggcaccggaacgcattgtccgttgcattgcttgacgcatagcacgacggaaagcaacacggccttcaagttgacgtgcgatgttttcaccaaccaacttggcatccaaatcaggcttcttgatttcgatgatgttgatgtgaactctcttaccagtgaggtcattaagttctttacgaagattttcaacctcagatccacccttaccaatgaccattcctggtttggcggtatgaattgaaacattaacgcggtttgctgcacgttcaatttcaacagtagaaacagacgcattagcaagacgcttctctatatatttacgaatttgtaaatcttcttttaagtaagctgcatagtctttacctgcataccacttagcttcccagtcgcgaatgattccaactcgtaaaccattaggatttatcttattacccacgcgttatccctcctctttttctgatacaacaattgtaatgtgacttgtccgcttgttgattggtgaagctgaaccttttgcacgaggacggaatcgcttaagcgttgggccttcgttaacaaatgcttcacttacaaacaagttttcactatctaaatcaaaattattttctgcattagcaactgcagatttaagaacttttgaaactaccggagaagcaccgcggggtgtgaaatccaagattgcggctgcttcagcaacactcttacctttgataagatcaactacaagacggaccttacgtgcggcaatgcgaacagttttggcagttgcttttgctgatgtaacttgttcagccatttgttatcctccttgttattaaacagtcttcttatcgtcagttccatgaccatggaatgtacgagtgggtacgaattctccgagcttatgaccaaccatgtcttcttgaacatatactgggacgtgtttacgaccatcataaacagcaaatgtatatccaatgaagctagggaaaatcgttgatcggcgtgaccaagttttgataacggcctttttatcttggtctttttgggcatctaccttcttgagtaagtactcatcggcgaatggtccctttttcaaactacgactcattttgcaacctcctctgcacagatattaattgttattaataaatgcgttctattacatctttgaacctttacgacgacgaacaataaacttgtccgaacgtgctttcttagaacgagtcttcttaccaactgtcttcttaccccatggtgataatggtgatggaagaccaactggtgctttaccttcaccaccaccatgagggtgatcgttagggttcattacagatccacgaacatgaggacgttgacccttgtaacgtgtacgaccagctttaccaacattgataagttcatgttcttcattacttaccgaaccaatagttgctcggttagtgctaaggattaaacgaacttcgccagatgcaagtctaacaagtgaatacttgccatctcgaccaagcaattgagcagatgcaccagctgaacgaacaagctgaccacccttaccaggcttaagttcaatgttgtgaataattgtaccaacaggaatgttggataatggcaatgtgttaccaggcttgatatcagcatcaacgccagattcaaccttgtcgcccacctttaatcccttaggtgcaataatgtatgatttgattccgtcagtataaacaatcaaagcaatattagcagtccggttaggatcgtattcaattgctttaactgtggctgtgacatcatctttaattcgcttgaagtcaataatacgatattgattcttgttaccaccaccacggtgacgaacagtcatatgaccgtaattattacggccggctgttttactttttgattcaagtaaagacttttcaggcttacgcttagtaattgcgctgtagtccaagcttgtcatattacgtctaccattgctggttggcttatatgttttaatggccaaaacgtgttcctcctatattagagatttgtttgattattcttcgttgaataattcgatttcttttgaatcttcagtcaatgtaacgattgccttacgacgcttcttagtgtaaccagcgtaacggccttggcgcttgagcttgccacgaacgttcatgatgtttacacggacaactttaacatcgaaaatgtcttcgatggcctttttaacttgggtcttagttgctcgtaaatcaacatcgaatgtgtatgtcttgtcgtccatcttactggttgtttcctcagtaataactgggcgtaaaataatatcgcgtgattccattatgcgagcacctcctctacttgagaaagagcagctttcgtaataacaactttgtcgtgatcggcaacatccaaagtgttaatgccttgagcagaaacaactttaacgttttccaaattacgagcagacagaactgccttttcgttgtcgtcttccaaaactactaatgtcttagttgaaacgtctaatttacctaacaattcagcgaattctttagtcttaggtgcatcaaattgtaaagtatcaacaacaaccaatttgttgtcggaaaccttttctgataacactgacttcaatgctaaacgtgaaaccttcttaggcaaacggtatgagtatgaacgtggagtaggtccgaaaacaattccaccgccacgccattgtggtgaacgaatagaaccttgtcgagctctaccagtacccttttgacgccaaggcttctttccaccgccgcgaactgcggaacggttcttaacggaatgagttccttgacgtaaagaagcacgttgcataacaattgcgtcaaacacaacattgttgttaggttcgatgccgaagataccatcgtttaatgcaacggtaccattcttgcttccgtcttgtttatataatgctacgtcagtcatctatggttgcctcccttctacttgtttgagccgtgaacggcacttctaattgtgatatatgatttatttgcaccaggtacattacccttaattaagagaacattgttgtcagtatcggcatttacgatctccaaattttgaatggtaacagtcttgttacccattcgtccaggcaatttcatgccaggaacaacacggttaataatgacaccgagtgaacctggacgacggtgataacgggaaccatgagtttctggtccacgtgattggccgtctttatggatgttaccttggtatccatgaccttttgtggttccagttacatcaacgatgtctcctggtttaaagatatctgctttaacttcatcagatactttatagtctcccagctcaacatctttgatttctttaatgaagcgcttaggagtcgtatttgctttctttgcatgaccttgttctggcttattagtaagcacagtacgtttgtctgcataacctaattgaactgaatcgtaaccgtcattttcaacggtcttgatttgcataatgacattaggtgtcacttcaacgacagttactggaactaattcgccgttttcagtgaagacttgcgtcattccaactttctttcctaagattccttttctggccatgagtacacctccgatatattgtatttattatagtttgatttcaatatccacaccgctaggcaagtcgagcttcattaatgagtcaactgtctttggcgttggatttaaaatatcgattaatcgcttgtgagtcaaaatttcgaattgctcacgagaatccttaaacttatgtggtgaagctaaaacagtgtagattgtacgatcagtaggcaatggaattggacctgagatagtagctccagttctttgcgcagttgcaacaatcttgtctgcggattgatcaaggatacgatgctcgtatgccttcaatcgaatacgaattttttgttttgccattgtgttccctccttcgtctattttgaaaataggactaactccgtgaaaattaccgccaaacccatggcaaagcatccgggtgtgtcgcaacctttcacatcaaagctaatacatattgctttagggcaaacttatccctaaaaacaagtactcaaatagtgtactaaaaaaagccgcataaaacaagtgttaacagcaattaattcgttttgtatcattactgttacttgaaaaatgattttaacttcttttgatattcaaatgaacgtaaataacttcaaccaatttattatacattgccgcgggatgatttgacagacctttagtcaaaaaaagagaccggaattaaattccgatctctacgtttgaaattaatcttcagcaggttggttcccaccgtttttcttaataatttcagcttggatgctctttggaactggctcgtaatgatcaaatgtcatggtgaaagtaccacggccttgtgatgcagaacgaagtgtcgttgcataaccgaacatttcagcaagtggaacgaatgaatgaataacttcggcaccgcttcggctttccattccatcaacccgtccacgacgtgcagtaacttggcccataacatcacccatgtactcttcagggacgttgatatcaaccttcatgattggttccaagattactggagcagcggtcttagcagcattacgaagagcgattgaagcagctaccttaaatgcagcttcactagaatcgacttcatgataactaccatcatataacttggctttcaaatcaattaatgggtaaccggcaagaacaccgttggccaatgattctttcaaaccttgttctacggctgggatgtattcacgaggaacaacaccaccaacgatggcatcttcgaattcgaagccttttccttcttcgtttggtgtaaattcgatccaaacatcaccatattgacctttaccaccagactgacggataaacttaccttgagccttggttggcttggtaaatgcttcacggtatgaaacttgtggggcaccaacagtggcttccacatggaactcacgtttcatacgatcaatgatgatatccaaatgcaactcacccattccggcaattaaagtttcaccggtttcagggttggttgttgctttgaatgttggatcttcttcagaaagcttttgaagagcaacgttcatcttatcttggtcagccttagtcttaggttcaacggcaacctgaataactgggtcagggaattccattgattccaaatgaagtggatggtcaacatcagtcagtgaatcaccagtagtggtgttcttcaaaccaatggcggcagcaatatcacctgagaatacttctggaatttcttgacggtgatttgaatgcatttggagcaaacgaccaacacgctcacgtttgtctttagttgcattcaaaatatatgaacctgactcaagggtacctgagtaaacacggatataagtcaaacgaccaacgaatgggtcagtagcaactttgaaggccaaagcagcaaaactggcgtcatcattagctttcagttcaatcttgtcacccgttgcaggatcagttgcattgtatggcttaacatcaagtggtgatggtaagtagtcaataacagcatccatcaacatttgaacacccttgttcttgaaggctgatccagctaatactgggaacagttccaagttcaaggtagctttacgaatagcagccttgatttcaggaattggaatttcttcaccctcaaggtacttgttcataatgtcgtcatcaacatcagccaaagtttcaactaattggtcacgacgctttttagcttcatccttatattcatcaggaacatcaactgtatcccaatttgaaccaagcttatcttcatcgtagatgtcggccttcatttcgatcaggtcaataaccccttcgaaatcatcttcagcaccgattggcatctggattggaagtggcttagcattcaaacggtcttcaattgagccaactgagaaatcaaagttagcaccaactttatccatcttgttaacaaagacgatccggggaacgtcataatcagatgcttgacgccaaacagtttcagtttgaggctcaacacccgcttgggcatccaaaacagcgatagcaccatctaagacacgcaatgaacgctcaacttcaacagtaaagtccacgtgtcctggggtatcaataatgttgatacggtggtctttccattgagcagttgtggcagctgacgtgatggtaatcccacgttcctgttcctgtggcatccagtccatttgtgaagcaccatcatgggtttcaccaattttatgaatcttaccagtatagtacaagatccgttcggtcgtggtcgttttaccagcatcgatatgggccataattccgatattacgagttttttcgagcggaaactctcgtttgttagccattgtgtaactccttccgattcgtacaaaaagtggctaaatcagccacttattagtttgagctgtttagaaaaatcctgagattaccaacgataatgtgcaaaggcacggttggcttcagccattctatgtgtatcttcacgcttcttaactgatgcaccggtattattagcggcatccatgatctcacgcgcaaggcgttcagtcatcgtatgctcaccacgtgaacgggcatagttaacgatccaacgcaatcccaaagttgttcgacgatctggtcggacttcgattggaacttggtagttagaaccaccaacacgacgagccttaacttcaaggaccggcataacgttcttcatagcttcttcaaagacgtcaactggttcgttgttagtttctttcttaattaaatcaaatgcaccatataaaatttgtgatgcagttccacgtttaccgtctaacatcaaacggttaattaaacgggttaccaattttgagttataaattgggtcaggaagtacttcccgcttttgaacatttccttttctaggcatttcgttatcctcctcatgattctataaaactaaatatttagattgcattagtaagattattctttaggcttctttgtaccgtattttgaacgaccttgacgacggtcttgaacaccagcggtatcaagtgcaccacgaataacgtgataacgaacaccaggtaaatccttaacacggccaccacggatcaaaacaacactatgctcttgtaagttatgaccaatacctggaatgtaagccgtaacttcaattaagttagacaaacgaacacgggcatacttacgtaaagctgagttaggtttctttggtgtcatagtaccaacacgagttgcaacacctcgtttttgaggggctggaacagtaacttgcttcttcttgaaactattgtaagcatagtttaaagctggtgactttgattttgaagttctagaatgacgtcctttacggaccaattggttaattgtaggcatctaaaaagttctcctttcaaattttcaatgtaagtccacacatccaggcggttcttttttatgtaaaaagaaatgtgtaccgcccaacactttttgtcatatacagtcagcatgtctgaatattcaggaatctgtcacaaaaagcaccttgtctaatttatcatgactggccgtttgtgtcaatgaatcatgttgaataatttaaaacgtaacaacgtacataaagtacagaggtaaaaactatgatgatgattattcaatttttgctgggtgcaagcctggcgtcgttttttaatttggttgctgtcagacgacaacgcggggaatcgattgtcgctccccgctcccattgtgattgttgtggtggtcagctgaagaattttgatttaattcctgtcttcagttacatcattttaatgggaaaatgtcgttactgcaaacaaaagttttcagcaaatttgttcactgttgagttggcggccggatctgttgctgcgggtttgaatctttttgagataaattgtctgtacgttggcatgttgattattttaatcgcactcagttcctttgacattgtcgaccaaacaattccaacagacggaattatcatgctgttgcttgtctgcggattatcaaacacccatccagtccaagaaattttgattgccattctgatctatctgctcatccaatttttaaaccaccacttttcctggatgggcagtggcgacatcgacatttatttttgcctgtggctggcactggatattccaagcttactttggcaaacgtttattgcttgcgtcgctgcactgctttatttaattgttgcgccgtggccgaaaaattccaaaattccatttgtgccattcatcaccattggattctatttaacccaccaattccaatcaatcttattaccgttaatttcatagaaaataaaaaaggattccaacccattgcaggttgaaatcctttttcaaattgattcattcaatttaatgattatttggtcgtcttgctcttgttagcatcttcagctttcattttttcttcaagctggctaattgagtaaacaccatcagttgatgaactaccaatttcttcaggcttaattcctcggtaatctggcattccagtacctgcagggattaatttaccaatgataacattttccttcaaaccaaccagtggatcattcttaccacgaattgcggcatcagtaagaacacgcgtggtttcctggaatgatgcggctgacaagaaactatttgtttcaagagcagccttggtaataccaagtaagacaggacgggcagttgccggaattccaccattaacaaccgtgtcaccgttacttatcttgaagtcattgatatccatcaaggtaccaggcaatacatcagtgtcaccaggatccatgatacgaaccttacgaagcatctgacgaatcatgatttccacatgcttatcagccacttccacaccttgcatccggtaaactttttgaacttcatgaagcaggtagttttcagttgagagaacatctctaaccttcaacaattccttaggatcaacagaaccttcattgagagctgaaccacggtgaatgtagtcaccttcagcgactctcattcgagctgtgatcggaacggtgtaagttcgagtatcagattcacctttaatggtaatttcttttgttctttcagcaggattttcttcaattgactcaactgtaccagtaacttcactgatctcagctttaccttttggattacgtgcttcaaagatttcttgaacacgaggaagtccttgggtaatatcggcgttaccagcaacaccaccagtatggaagttacgcattgtcaactgggtaccaggttcaccgattgattgagcagcaacagtaccaaccgcttcaccaacttcaacctcatcaccagtagccatgttacgaccataacatttctcacaaacaccgtggatggtgttgcaagtaaatgctgaacgaatcgtaacttccttgattccaaggtcatcaatcttagtagcctgatcctcagtgatcatggtgtttgcaggaacaatcacatcgccagtcttagggttcttaacggttttgtgagcataacggccaacaattcgatcatacaatggttcgatcatttcgttaccttcagtaattgcactgatagtcaggccacgatcggtcccacagtccttttcacgaacgatgacatcttgagccacatcaaccaaacgacgggtcaagtaaccagagttggcagtcttaagagcagtatcggtcattcctttacgagccccatgggttgaaatgaacatttccaaaacagtcagaccctcacggaagttggaagtaattggcaattccatgatttcaccgttaggagcagccatcaagccacgcataccagccaactgagtaaagtttgaaatgttaccacgggcaccagagtcactcatcataaagatagggttctgtggatcttggttttccaacagacgcttttgaatatcatccttggcgtcattccaaataccaatgactcgttcataacgttcgtggtcggtaatcagaccacgacggaactgcttggtaaccatatccacctttttatgggcggcgtcgataatttcttgcttatcaggcaactgagtgatatcggtaattccaacggtcaaaccagacttggttgactcgttgtaacccagatccttcattctatccaacaagaatgaagtttcagtcactttgtagatcttgtaaacttcggcaatgatatcacttaagaagcctttcttgaatggcaggattaatttggcattcttcagatgctcatgaatgtcctcacctggttcaaggaagaatttgtcatcaacataaccattcaaattggtttctgaaggttcgttaatgaatgggaaatcttctggcaaaatctcattgaagacaatcttaccaacggaggttaccaaaatttttccaagttgatcctttgtaaaggtcttctttggatatgcggaagccttgattccaacacgtgtgtgccagtgaacgattccgttcttaaatgccaattgtgcttcgtcaggtgagttaaagatcattccctcaccttcgcggccggcttcctccatggtcaggtaatagttaccgataaccatatcttgagatggggtaacaactggcttcccatccttaggtgccagaatatggccggcagctagcatcagcaaacgtgattcagcttgggcttcatcagacaacggaacatggatggccatttggtcaccatcaaaatcggcattgtaggcttcacaaaccaatggatgaagccgcatcgacttaccacttaccagtacgggttcaaaagcttgaattcccaaacggtgaagtgtaggcgcccggttcaacagaactgggtgttccttgataacatcttccaagacactgaaaacatcgtcatcttggcgttcaattttgcgtttggcgttcttaatgttggatgccaaattgcgaccaaccaattccttcataataaatggcttgaataattccattgccattggaactggtaatcccatttggttcatcttcaaatgagggccaacatcgataacggaacggccagaataatcaacacgcttaccaagcaagttctgacggaatcgtccctgcttacctttaagcatgtgagaaagtgacttcaatgggcggttacctggtccggcaactggacggccacgacgaccgttatcaatcaaagcatcaacggcttcttgaagcatccgtttttcgttttgaacgataattccaggtgcattcaggtcaagcaatcgtttcaaacgattattacggttaattacccgacggtacaaatcattcaaatcagaagtggcgaaacggccaccttcaagttgaaccattggtcgtaagtcaggtgggataactgggattgcatccattaccatccatgaaagttcatttccggattggacgaaagcttccaaaatatcgagtcgacgaacggcacgggtccgcttttgaccggttgcattcttcaattcatcttttaattcggtaacttctttttcaacatcgacatcttcaagcagtgtcttgatggcttcggcaccaatttgagctgagaaccgaggaccatattcctgcttctttttgcggtattcacgttctgaaagcaactgcttcttttccattggcgtgttacctggttcggtaacaacgtatgaagcgaagtaaatgatttcttcaagtgcacgagggctcatgtccaagacaagacccattcgacttgggattcctttgaagtaccagatgtgagtaactggagctgccagttcaatatggcccatccgttcacgacgaacctttgaacgggtgacttcaactccacaacggtcacaaacgattcccttataacggatccgcttgtacttaccgcaggcacattcccagtccttggtaggaccgaaaatccgttcatcaaacaaaccatctttttctggttttaaagttcggtagttaatggtttcaggctttttaacttcaccatatgaccaactacgaatcttatcaggagaggctagtccaatctgcatactttcgaatttattaacatcgaccactagtttgacctcccatttctagtcattactgttgttaacgttggttgatttacttggtgtttcaacttgatcagcaggttgtttagctgcatgatcttcctgctctttcttcttgtcagccaatttgctcaatgcgtcaacgtttacaacgtcgtcatcgtcatcaagatcacgaagttcaatctctttatgactcgcatcgagaaccttcatatcaaggcctaatgactgcaattccttaacaagaacccggaatgattccggtacacccggctttggaattggctcacccttcacaatggcttcgtaggtcttgacacggccaacaacgtcatctgatttgtaagtcaagatttcttggagagtatatgcggcaccataagcttcaagtgcccaaacttccatttcaccaaaacgctggccaccaaattgtgctttaccaccaagtggttgttgggtaaccaatgagtaaggtccaattgaacgtgcatggatcttatcgtcaaccatgtgggccaacttaagataatgcatgacaccaacggcaatcttcttatcgaatggttcaccagttcggccatcatacaagatgtacttaccatctgaaggcatgccggcttctttaactgcatcccagatatctttatcacgagcaccatcaaaaacaggtgttgcaacgtgaattccgagtctgcgggcagccattcccaaatggagttccaaaacttgtccaatgttcatccgtgatggcacacccatgggactcaacatgatgtcaactggtgtcccatcaggcaagaatggcatatcttcttctggaataacaacagaaacagtacccttgttaccgtgacggccggacatcttatcaccaacttgaatcttacgtttttgagcgatgtagacacgaaccatcttattaacaccaggtgaaagctcatccccgttttcacgagtgaagatcttaacatcctggatgattccgccgccaccatgaggaactctcaatgaggtatcacgaacttctcgtgatttctcaccaaagattgcgtgaagcaaacgctcctcagctgataattcagtcacacctttaggggtaactttaccaaccaagatgtcaccatcatgaacttcggcaccaattcgaacagtaccatcttcatcaaggttcttcaaagcatcttcaccaacgttaggaatttctcgagtcatttcctcaggtcctaatttggtgtcgcgagtttctgattcgtactcttcaatatgaattgaagtgtaaacgtcatctttaaccagacgttcgctgatcgcgatggcatcttcgaagttgtatccttgccaagtcataaatgcaacgacagggttttggccaagtgccaattctccgccttccattgatgggccatctgctaagatttcgtcagcatcaactcggtcgccaaccttcacgattggacgctggttgtagttcttaccgccatttgaacgacggaatttcattaatttatatttatcaagggacttgtcgtcacgacgtactcgaatttcacgagcatcaacgtattcaacagttccttcattcttacagatcagtgcaacaccagaatcatgagcggccttgtattcgataccagtaccaacaagtggtgcatgaggatcgatcaaaggaacggcctgacgctgcatgttggcacccatcaaagcacggttggagtcatcgttttccaagaaaggaatacatgcagtggccacggcaactacttgcttaggcgaaacatccatgtaatcgaccttgtcgataccaatttcaatgttgtttgacttgtgacgggccataacgatgttattgacaaacgaaccatcatcattcaatggtgagttggcctgggcaataacaaagttatcttcttcgtcagcagtcaaataatcaattcgatcagtaaccttatgagtggtccaatcaacacgccggtatggtgtttcaatgaaaccatatttgttaacccgagcgtaactggacaaactgttaatcaatccaatgttagggccttcaggggtttcaatcggacacatccggccatagtgggtatagtgaacatcccggacttcatatccggcacggtcacgagtcaaaccaccaggtccaagggcagacaaacgacgcttatgagttaattcaccaagcgggttggtctggtccatgaattgagaaagctgtgatgaaccaaagaattctttgattgaggcaacaactggacgaatattgatcaattgttgtggtgtcacagttgaagtatcctgaattgacattctttcacgaacaactcgttccatccgtgacaggccaattcggaactggttctgcagcaattcaccgactgagcgaattcgacggttacccaagtgatcaatatcatcaattgaaccaatgccttcttgaaggttaaagaagtagttcattgctgaaatgatgtcagctggagtaatgtgcttgaagctcaatggaatgttgtcattaccaattaaaggaaccactcggtcaggatcgttaactgattgaactttaatgatttgaacagtcattggttcagtcacaacggcttcatctgaaggggtaaaggtgtaagctttaaattcatcgttatcaaggaatggtgccaagtccttcataacatctttcgtgacaacggtgcccttttgagcaatcacttcaccggtatcaggatcggcaagggtttcagccagtgtcaaacctaacaggcggttctttaagctcagtttcttgttggtcttgtaacggccaacgggcgccatgtcataacgttttggatcaaagaaacgagcagtcagcaagcttcttgatgaatcagcagtcttaggctcacctggacgtagacgttcgtaaatatccttcagtgactcttcaacacgtgaatcgtcagtgtctttatgaacatctttttccaaggtcaaacctaaactgtcgttgtcgcccaagatgtcaatgatttctgaatcactgccaaagccgagggctctaattaattctgttaaaggaatttttcgtgttcgatcaattcgaacgtacgcgatattttttgcatcggtttcaaattcaagccaagcacctctgttaggaataacagtagtaccaaatgaatcacggccattcttatctttatcagcatggtaataaacgccgggtgaacgaaccaattgtgaaacaattactcgttcagcaccattaataataaatgttccttgatcagtcattaatggaaaatcgccaaaaaacacatcttgcgtcttaatttcgccagtctcatgattggttaattttaaggtaatgtgaagtggagcagaatagtttgcttcgtgttcacgcgcctcatcaacggtgtactttggtgttaataattgataatcgacaaactctaaagaaagcttgccctgaaagtcatcgattggcataatgccgtcgaaggtttccttaagtccctcatgtaaaaaccagttgtaagaattagtctggatttcaatcaggttcggtaaatcaagcacttctttaattcgtgcataacttcgtcgggtacggtgttttccatatttaactaaatgtcctgccaagtttttcacctctccaaaaaattccggaatcgaaatgttacagtttgattacaaatgcactttttagcacatctgaccgggttttgggcaaaaaaaatccaaaaacaagactttcttgcttttggctttttatgcaggccaacccggacaatagatcgcgtcgaccatttcgattcacaacaaatacagttaaaagaataacaatttatagaagtaaagtcaaccttttagaccatggttcattttgaatcgcaatttattttttatcattcactaaagttttgcgttccggcttcttcaccgaaatggtaatctggttgtttctaccgccaacagtgactgagtcgccagggacaatttccttggcaagcaacttggcacttaaattatcctcgagttcagtttgaattgctcttctgattggacgagcaccgtactcagggtcaaaaccacgcttggaaataatcccgattgcagtcttggtaatcttaatgtcaatgccttgatcgtgaatccgcttgataaccggtttggccatcaggtaaacaatttgatcaagttcgtccttggtcaatgagtggaagacaaccacttcatcaattcggttcaggaattcaggacggaagcgttgtttgagggtagcttgaatcgtgtccttcattgctgcatagccttccttggcatcctcttgaccaaatccaacagtcttcttatcccgcaatgtggttgcacccaggttggaagtcatgatgataacggtgtttctgaaatcaatctttcgacccttggcatccgtcaagtaaccatcatcaagaacttgaagcaagaggttgaagacatcaggatgagccttttcaacttcatcaaaaagcacaactgagtatggcttttgacgaaccttttcggttaactggccaccttcatcgtagccaacgtagccgggagcagaaccaatcagacgactggttgaatatttctccataaattcactcatgtcaactcgaatcatgtcctcttcagaaccaaagactgcttcggccaccgcctttgccaactcggttttaccaacaccggtcggtcctaggaacatgaaggaaccaattggacggttcggatctttcaaaccgcttcgagcccgacgaatcgaacgagaaaccgctgaaattgcttcttcctgaccaacgacccgcttgtgaagaatcttttccaagttgactaagcggtcagcttcggtactgctcaaacgagtaaccggaatcccagtccactcgcccacgatttcagcaacgtcttgtggcgtttccttaacggggtaatgcgcatcctctgagccttcctcggaatcattatcttgagcaagttcatcctgtaactgattcgtttgtttgcgaatcttagcagctttttcgtaatcttgggctaccaaggcttcatttaattctgataacaaatctgacagtttcttatgatcatcaacggcatcagatttttgaaggtgatcaattcgaactttggcagctgcctcatccattaaatcgatcgccttatcaggtaagaatcggtcgctgatgtagcggttggaaaggttaaccgcagtttcaatggcgtcatcagtaatttcaacgtggtgatgttgttcatactttggccgtagacctttgagaatttccaccgtttcatcagtcgttggctcatcaaccataactttggcaaatcgacgctccaatgcagcatcagattcaatgtacttttggtactcgtccaaggttgtggcaccaattaattggagctcaccccgggccaatgccggcttcaaaatgttggaagcgtcaatcgcaccttctgcaccaccggcaccgatcaaagtgtgtaattcatcgatgaacagaataatgttgccatcttggtaaatttcatcaatcactttcttgagtcggtcctcaaattcaccacggtatttggtaccggcaaccagtgagcccatgtcaagcatcatcaaacgcttcttggacatgtcaccaggaacgtcgccgctgacaatccgttctgccaagccttcagcgatggcagttttcccaacaccgggttcaccaattaaaacagggttgttctttgtccgacgagctaaaatttgaatcacgcgtttaacttcgagatccctgccgacggttgggtcaagacggtcttgacgggccatttcagtgaggtcacgagccaatgaatcaattgttggtgtctttgagtcagctggcttttgttgacggccacgttgtttggaagccaggtttgaggccattgagccaccactgatgcccatttttcgaagggttacttttctaatttgtgatagatcgagtcccaagttaatcagaatacgggaagataaaatggtctcatcagtcagaagtgaaagcaaaatgtgctcggttccaacctttggaacaccgttcttcttggcgaattctcctgcttgagccaaaacttcctttgcctttggagagtatggtagataatcgttactgctaaggtccttaaggttgccatagccggcgaaacgctctacttcttcagtgacatcttcggcagttactgaaaactgctgaagcgccttgtaggcaattccattcgtttcgatcagtaagcctaatagaagatgttcagttccaattgcttggtgcttgaatttcttggcttgttcttgtgcaatggtcaaaacgttcttagcactcggagtaaataaattattcatagataccctctctttctatcgttcgtatcgcagccggttcaatatcgacaccatgatattggcacgtaaaatgtcggttaaatcgctgttattcaggtcaattgcatctttgtcaatcgcagctaatatgatgctcacctcgcgacgattaattaattcattattatataacgtttgaacgatcgtttcactatcccgcttcgataatttgttaccaattgcggcaattaatgaattcaaaacgtcaatgtcatctaataaatgaactttttctattctaatgtagccgccaccaccacgtttactttccacaatataaccattctggatcgtgaaacgcgtgttgattacatagttaatctgagacggtacaacgtcaaacagcccagcaatttcagaacgacgaattttaacctgctcgttctcggcaaggatttctttgagataatgttcaattaaatcagaaatgttttcgtccgccatgtaatcacccaattctttgactaatattgactattattatacgaatgtgacgccaaagtgcaaggaaagtgtttgagagtgcgacatgccctgggtgaccccggagcacaaagcggaaacatcaatggtgaacgaaccttgttcatcgttgatgtttccgctttgtgtggtaggggtcaagggcatcggagcacgtttagagtcgggatctcttcacttatgcagtaggactctggggtgtcggagcgtattttcgaagtgggataaagcagaaagaagcaaaacgatcgtgcatttaaactgacccattctaaaatcaaaacataccagaaagtcacatcaacaccagcaaccacgattgccgttcgccgagatgtcaaaaaaggccagaaccaaagtacagttctgacctcaaacacgattcaattaatatgtaatttcccacaaaaaaatcgggaaaacaagatttgaacttgcgacccctacgtcccgaacgtagtgctctaccaagctgagctacttcccgatgatttaagtactattgagttaacaatataaatataccatatgatctatgttaaacaaagtcgggaagacaggattcgaacctgcgaccccctggtcccaaaccaggtgctctaccaagctgagctacttcccgaaaaggaattcattgcaataaaaaatgcacccagtaggagtcgaacctacaaccttctgattcgtagtcagacactctatccaattgcgctatgggtgcataataagtattaaattaaggaacctcaatcatagtacttgattgaagcggaagacgggattcgaacccgcgacccccaccatggcaaggtgatgttctaccactgaactacttccgcaaaatgccgactagacgattcgaacgcccgacctcttcattactagtgaagcgctctaaccaactgagctaagtcggcaaaatgtataaattgttaggtaactagcacctatgcgggcgaagggattcgaacccccacgtcataagacactagaacctaaatctagcgcgtctgccagttccgccacgcccgcattgttaaaaactggcaatgagccgtggcagtctcgaactgccgaccctctgattaaaagtcagatgctctaccaactgagctaacggctcaatggaggatacagggatcgaacctgtgacctcctgcttgtaaggcagatgctctcccagctgagctaatcctccatgaaactaaatgaatcaaatgttggtagcaacatcatcaacacaactattaaattttacaataccaatcaactcaagtcaagatgaattttaaaaaatcctgattggttagccgttagttaataacgtctttttccgacaaaaaatattatatcctatctcggaaaacattgctagtccaattttgaattaattggatttttattcgtgataaataaaaaggcgaaggacagtcagccgtccttcgccttgctcctggtacgataatcacgcccacattcaaaattcatcatgcggtaggattgatttcatccaaaaactagttttgcttttcaattttagtcatgccgtgcatatatggccgcaatacttccgggatcgtgacgctgccatcttcattctgataattttccagaatggcggccaccgttctgccgactgccagtccagaaccatttaaagtatgaacaaagtgaagcttcccttcatcatcccgatactggatgtgtgctcggcgagcctggaagtctgtacagtttgaacagctggaaatttcccggtacttatcctgggctgggaaccaaacttccagatcgtgggtcatagcggctgtgaagctcatatcactcgtcgtcaatgtaataacgtggtaagccaacccgagtttttgcaggttaacttctgcttggtgggtaatctcttccagtgccttccacgagtcttcgggcttggtaaatttcaccatttcaaccttgttaaattggtgtaatcgaatcagccccttggtatcacggcccgcacttcctgcttccgatcggaatgccggtgacaaggccgtaaccgataccggcagcttttctgtcggaataacttcattgcgataatagttaaccaatggaacttcggcagttggaatcagggttaaatcactgtcctgaatctcatagccggatttgttctccaaaaattttggaaattgcccggtgccatacattgaatcattattaaccatgtaaggtggaatcacttcggtataaccggcagcggtattttggtcgaggtagaagttgtaaacggcccgttccagtaaagccccgtcgccaatatagtaaacaaaccggctgccggacacttttgcggcccgctcaaagtcaaggatgccaagattttcaccgatttcccaatggtgttttggttcaaaatcaaatgacgggatctgaccaatcttacgaagctcaacggatccttcttctgtgagtgacaccgggacatcatcatgaggtatgtttggcagatgagcagccaaattgtgttcatcttcctcaacttgacgcaattgctcgtcaagttccttaatccgttggcccacctgtttcatttggttgatggcctcagttgcatcctctttattgcgcttcttttgtgaaatctggtcagaaacggcattccgctttgctttgagggactcggattcaacgatcaaatcacgacgtttggcatcgtagcccactaattcatcaatggtttcgggcttggttccccgcgtagcgagcttttctttggtaaaatctggatcttttctgattttcttaatatctaacatttcaaatcctcccaatctgtatacaaaaaggacccctcgtctatgggacgaaggatccttttcgcggtaccacccaagttctcgacaatcttgccgagctctcaaagtatggtaacggcatacaccgtgcagcattacctgcccgttcacttgtgctggaatattcgatgacagttcacaccaaccactgtctctctgaaatctacttaataggcacaaaacgttttatctgaaatcgattataacgaatcaatccctaaaccacaagagcggtctgaaattaaattgccaacttatccactttggcgtcgattagatcgatcaccttgtgtttatcggcatcattttcaacaaaatcatacttgtcaccgtcaatttgaatcttaggtgatttgtcatattcttggtaccacgtctggtagcgggcattcaaatctttatagtattggtacaaatcgggatcattatcaatctgctcataagaacggccgcgcttttgaatccttcttaacatcgtttcaaacgagatgttaatgtggatcaataaatcggggttcttgctgtgatcggtttgtggcatctcctgcatcatgttctccagcaatgagtcgtaaattgtcacctcagtttcggtggcccggcccaagtcggcattcaaatggaagaggagtgaatcttcaaaaattgaccgatccaacacactctcgtcattttgccaagcttttttaatgtcatccatccgacggtttaaaaaatcaatttggagcaagaaggcatacttcttgggatccttataaaacaacggcaggatccggttgtgttcaactgattcataataggcaggcgtgcccaaatgttgcgacagcatcttggtcagtgatgtctttccggcaccaatcgttccagcaagtacaagcataattattcccctaacgtttttgcgtgcaatcatcgcacaatattttatcaacgctacatattgtactagttagaagagataggtgcaacatattgtggaaatttagttaatgtttgagacgtcaaccacttggatgttgcccaaaccaccgtacgcttcaaaccacggtgtggcattctcagacaagatctgggttaattcagtgacgtttctggttcccttgcgtttgagccagtcaaccaggccgtctttaccgtcacgaatgtaaatgtcgacaccttccaaccaagttgcccgaccgcttaagacaccgttaaacttggcaccggcatctccagccagcttcaattcccgttggaaaacaggggtcggcacaccggcactcaagaaaataaatgggcgggtcgcctcgtcgctcaactctttgagacagcccttggcttggtcttcggtgtaggcgtaatcgccaccatcagcccattctttgacgtaggtcgggttaaatggaatttccatcttcaaaacgtcaatgtgatatttctccttagtgaattccatcattgactgcagcaccagatcaggcttgatcttggcaaaatccaacgacttgctgtcgtaacggtcgtcgtaagtgacaatttcaaagaaggttggcgtctgggctgccaaaccttccgtcccgtatcgttcagcgaacgcttttttaacgtcgttgatttcatcaggatcattgggattgtagtagaccaataccttaagggcatctgctcccttctcaaccataatttgagctgattgatcagaaatcaagcttggtaatcgtcccggggtgtcggcattgtatccagtcttttcataagacataatcagaccagtgtctttagccttggcctggatccccttgaaacccatttgttcgtccaaaagcacggcagaactcagtggactcaagatttcagagacaatctccttgaaatcatagaccatcttcatactgaaaagcttcccgtatttttcggaggccgttttcattcccttaacaagtgatccacgttggtctaacgccaatgcatcgataatgttctgatcattggacaatttgttcattctttcaaatttaccttttgacataaactttttcatatatctttcacctcatatttttaatataccaattggtaaaattgtaccaaacattatgccccaatatcaagttttaggccgataaaataataaaaatcggcccatccaagacggatagaccaattcattattaatatattacttgttgttcaattttgaaagatcctcgtctctatgggccggggaaacgtcaacctgatccagcggaatgattttcgtatggtgcttgagcttataccaaatgtacaaaatcaataccaacggcacgctaatgtaagtgaccagaatctgcttccagtcaaagcttgcaaaggcctgcggattttgaccgacaattaccagaatacacaaaatcaggcacaatacaggaccgaacgggaagagcttggcatgatacttgagttcgctgaggtcatggccctggcgaatgaacgcccgtctgaatcggtaatgtgaaatggcgattccaaaccatgcaataaagccggttaacccggaagctgccaccagccacatatagatttggggcccggcaatactggaaataaaggtcaatagcgaaacaaaagtcgttgccaataatgaataatatggaatcccattggcagccgttttacccagggattttggcgcatatccgctgttagacagtgaatacagcatccgggtagaggcgtacataccggagttcgccgatgaaataacggaggtcaaaataacggcgttcatgacactggcagcagcggccaaaccagcccgctggaaaaccaatgtaaatggactgatcgcaatgtcagtggcacttgatcccagcagtgaatggctggtgtaaggaataatggcggcgatgacgaaaattgtcaaaatgtagaacaaaataatccgccagaacacttcattaattgcctttggcacactgtgttggggatcttgggactcgccggcagtgatgccaaccagctcagttccttgaaatgagaacccggcgaccacgaagacactcaggattgccggaaaaccgccgacaaatggtgcctgcttaatagaaaagttacgcatgccgacaaaatggccgcccatgattccaaagatcgtcaaggcacccactaccaggaaaataataatcgtgaccactttaatggcggacatccagaactcggtttcaccgaaggtactgactgacatggcattaatcaggaaaataatcactaaggcaattgcactccaaatccaggcaggcacatttggcagccagaatttcataaccaaagcggcggtactaatatcaacagccaccgtaatcgcccagttaaaccagtaattccagcccatggcaaatcccaaggctgggtcaacgtatttggatgagtatgcggcaaacgagccggaaatcggcatattagtggccatttctcccagactggtcatcaggaaatagaccatcatccccatcaggacgtatgccgttaaagcaccaccagggccggcttggctgatagctgaaccactggccacgaacagcccggttccaatacagccacccaaagcaatcattgacacgtgacgggcttttaggccccgcttgacttgtccgttggcttcttggctctcattatcgttcatcttttcgtctcctatatccaataatttcaaaatctcactaaatctacaaaaaaatccctttcaaaatattgaaagagacagtttgcgtttctcaacatctttgatagctctccgcgatttccgcgacagtccccagcttcttaaactgggccccaacaaccaactggaaggcagctgatcgtttcggcactcatccctttttacttcagtcataacttccttcaagttcctgaaatatactcttgatgaatgcgcctctactcgattagattgattaatttagttgttaataacttcgacaatcaaaattgtaactcacttgggttgaattgacaaaccagaaagacttttctcaatgcaacgccagctgataaatggtcttttctttgccgacaagcggatcaatcagtgtggtcttcacttgaaacccgaccttctttaagacacccatagaggcttgattatcgctgaacacctctgcattcaacgtctcaatcgttgggttaacagcgagttcctgaattaatttagtaagggcttcagacatgatcccttgacgccacagttccgggtgaagaaaataactcagttccaaattggcaggatcgggttggtgatcaaaaccaacttgttcatataaaagaattgccccgaccagccgatcgtggatccggatgccaaaggagttaggcgttgtaatctgtcttttggccactgcccccagcatttgttgattactgaccagattaaaaccggcgccggcggcaatttctgggatgctgattaatttttcgtaagccgttaagtcagccagcgttaattcagtcagttgaagtcggttggtctcaatcggtaaatccatggcgatctcctttcaaaaaaatgcccaggaaaaatcctcggcattttcaatcagattttagtgtgaaccacaaaccggtagcgggcaacctggggcgcgtaactggcataaagcatttcagctaccaacagccaggaatagccaaccaggcaggctcccaccgtatccgttgggtaatgggcgttcaagtagacccgggaaagcatcaccaacgccaagacgatgacgagcagtactttcatcaccactcgaatggacgcccgctcaatcaacggcaggacgatgatccataacaccccggcaaccaggaaaaatcccaggacgtgaccacttggaaaactgtagccattatcgacacccagatgcagcggcggtcgatgccgtctaaccagttgtttgacgactgcgccaatcacgtcgccgccgactatcgtccctaatgcccaaagtgcgggaactttgtacttaaatccccaaaggaaaaaggcgatgatgaacacccagaaaatgtccattttcgggctggccagaaatgtgattactgagtagaaatgttccagtcccggtgtcggcgcggatccttgaatggccgttgtaaaaattgaatctaaaaattgcaaataatcaaaattaaacgctaccgaaattgacagcaaggtcgtaaaacacaaactcacaatcagcttgaccaaccggtttggatcgcgttccatcagcatgtaatcttcgtttccgtacattagttcaacaaccctctcgtatgtattactcaaaagtgagtatatcacaaatcgaaaacccggtttctggtttctgaaaattcttagctatcttttaattatttacagaaagtgtataatcttgtgagttagagatcacatttaaaaggagtgaaagacttgataaactatgctttattgatgattgccattggcgtgttcgccgggtttgccggtgccatcctcggcctgggtggtggaatcatcttaacgccgattttgacattgttgatgggtgtcgacattaaatacgcaatcggagccagtatcattgccgtgattgccaccagttccggagcaacgattgcctatctccgtgacaaagtgctcaatttgcgggtcgcgatgtttttggaaattgccaccactttaggggcattgagcggcgccttgttgaccggtgtgattgatccgaaatatttgtacatactatttggattattgctattattctcaggctacaatatgattcgcaaattaatcagtcaccaggaagtccttcatcgggctcatcccgatcaattatcgtccaaattcaagctggacagcagctacttcgataatgttgaaggcaaaacgatcaactaccaagttgaacacattcccggcggcttggcagtcatgtacggtgccggcattgccagtgggctgcttggaatcggctcgggtgctttcaaagtgatggcaatggacaccgtcatgaagatgccgctcaagccatcgacttccactagtaatttaatgatgggtgttaccgcggctgccagtgccactgtctatttcttcaacggctcgatcaaaccaatgattgccgttcctttggcactgggaatcttggtcggcgcccgcggtggttcacgaatcatgcgggatatgtcagcgcggacgattcgaatgattttcgttccgatcttgttttatatcggtatcgaaatgtttatgaaggggatcagataagatggacaaaaataccagagaacaaatgactgaagaaatggccgacgtccaattgattatcggcaagattcttcggttgggggtcatgatttctgcaaccgtgatgatcattggcttggtgcttttaattgtcaaaggcaacggcggctatcctcacaatgcctttcccaccgactttacccaaatttgggcgggaattgccgaactcaagccgtacgccatcatgatgctgggaattttcctattgattttgacaccggtattgcgggtggtcgtttcaatttattccttctatcgcgaaggtgacagcttgtacgtttggatcaccacaattgtgctggtgattttaggaattagttttgtgtttggaattttaagataatcaattaacaatcaagaggcgccggtaagggaacattccctttgccggcgcctcttttgagttgattaacatttttaactctggtgaatcgtgacatcgccaacgtcgctggtaaatctgtaagtcaccggatttttggcattgctgtcaatcttcttgttgtgtgagctgccaaacaatgatgcatcgccaacatcggcactcactgaaatctgcgttcgcttgttcttaaccacatgtcctgaaatatcgccaacgtcgctgtgggcggtaaaagacttgccgactttttgggaattgaaattaatatccccggcaccggtttcaacggccattgagtcgaatttattggacgtcagatcgacatcgccggcaccaacatcaagatgtgcgctgggaaaagtgctggttgttaaattcacatcaccggtattctccaagtccaagttttcagtggtcgtcacgtgattcaaattaacatcgccgaccccagacgaagtgatcgtcttgatggtcatattcttgatagtaattgagttggcaacatcactgttgatcgtaccgaccttcatgcttcttggaacggtgatgatggtcttgccaaaggcctggcgcgctcggcgaaaatcaccaaagaagatgataccatggtgcttacgtggactttttaaattgaaatgaagggtattgcctgattgcgtgatcttggtagcacttggataagtaacctcgattttagaaacgttacccttcttaatttgcaccggactggccgttaacaaagaaaagtttttcacgccggaaaatttggcactggtttggtgtgacttaaccggcgtggactgatcagttgtgaacccgtgatcccaatagaccgtgcgggcaccaccattgcctaggccgagcgccaacagaacggttccaaccaaggtcacagttaatcccacgatgacagtttttttcatttttggtcaccctttccttttcgttcagcccggttcttcgggacaaccttgttataaatccatttcgaaaataacgtgataccacgaatcagaccgttgatgacggctttgaagaccggcaccagcataatcatgaccccaatgaccatcagacccattcccaaatagaaaatgcccgtccaaaacgaactaaacagggtgcccaatccgacgacaaacccggtaataccaaccacgaccaccgcaaagaagatcgccaaaacggcaataatcagtgaacccgaaactgcgattccggcaaaaatcacccctgcaagcgcaagtgccagcggaattgtcactggagtcgaaagcaatgctaaaataatcagccaaatggttttaacatcatttttcggttgttgctgtcgagactgctgagacatcggtgcgtccagtgtccgaatggaataatctgccaacaccttccgagccaattgatgaggcgttcccaactccctgatgcaatcgtcgtaactcgcatagccgccgtcttgaagatattcacggtagaaatcgactgcttcatcccgctcttcaggactcaattgtcccagcagtgcctgaaactcttcaatgtaatcattcattctgatcatctcctaacatgttatcaatcccttgcttaaattcctgccactcctgctgaataatgccaaactgtcgttttccttccggcgtaattttataataccgtcggttgcgaccctgatatggctcatcataagttgtcaacagatcgttcttcttcaaccgtcttaaaaccgggtacatcgtcgactccgaaacagaaatcgactcttggaccttctgggttaacgcgtagccgtaataatcctgaccattcagaattcccagcacacatccatccaacaattccgaacttatttggatcgccatattgccacctccatagtattatacgcggtataatattatccaagacaaataatacgcctctaaccaggaatgtcaaacaatttatggcagaaaaaaaggatgggttatttatcccatcctttagacacatatttaatcttaattcgaattttgttaatcaactcggccacgataaaccccaaggcaatcgatccggcaatccagacgacctctgaaagataattaaaggccacctgataatcacctaatgcaaagtttttaatcgtgttatacgcctgacccccaggcaccaatggaaccaagccagggacgtcaaataagatactcggcatttttttgaggtgggcaatcaccacggacaccaaaccaatcgtcaagccgccaaaaaaattagcagctcccaatccaccccaggtattcatgacgccatagtacaccagccaactcaaagtggcggtgatcccggcgacattcaaagcccggtgtggcaggttgacgattaggccaaagccaatgcctgaaaagtaaacacaaatacatttaataataaacagactcataagcatccctcaaaagaagtgcagcgcgattgccacaccaaacccaagcgcacaggcactaatcagggcttcaatcccccgtgccggaccactaattaagttgccggacaacgcatctcgaaccgcgttggtcaagggaattcccggcaccagtggcatcatcccgccaatgataatatcatcggctttgacgccgatcccatttttcacagcgatcagagctagtgcacccacgacaactgcggccaggaactcacttaagaaccgtatttgaatataaatattcaaaaaatagtaaactgcccagccgaacatgccgacaataaacgtgatccaaaaatccggcagattgttttgaaacaccacgaccaaggtgccgctcactagcccagcgcccaaggtctgcaaccagagcgggaaagttgctaccaagtcatcaatgtggactaaatcgtcacgaaactcatagatatcaatctttttggcagcgtaggccctggacaattcattgaccttggctactttttccatgtcaaaagcccgtttgtcaatcgaaccgacttcggcgccaacttccttaacgccgcctgacatgataatcccggtcaaagtcgcgtagacttgggcatcctttaacccggcattcttggcgattcgcataattgtgtcgttgacccgggacatttctgagccggattcaatcatgatccgtccagccagcacacaggtgttcaagactaaatgatcataattctcctgccgagttgcagtatcggccatttcaatcacctcacgaaaacataatgagccgttttaaagccaatcaccaattttttcttatccgtcacattcttgacggttaccgacccttcgaagggatcgtgagaaataattttcaacttatcgccaatatcgagcttaatatcgcccagcaacgttaataagtcatgattgtcaataaatcggttaacgatgacttcttcaccgtcttttgcatcagtgagcagtttatcatgatcggggtgataattaccattccgatctggaatgacgccgccatggggacaacgcttgggattgcccaaaaagtcatccaggtggtcaatcatcttgtcggacgtgacgtgctccaacagttcagcttcatcatgaacgtcggaaatgtcatagtgcagcgtgttcaccaggagagtttcccaaatgcgatgcttgcgcacgagttcttcggcataacgcttacccttttgagtcaattgaacaccggaatacggttggtgggtgaccaatttttcagccatcatcttattcaccatttcggtcactgacccggcagcgatgtttaaactgagagcgatctgcttgttgctgaccaaatcatcagttccgccaagttcaaatattatttttaaatagtcctctttcattggggtcatttaactcaaaatctcctatactttatggaatatcattaccacggtcataaatgatgtcttcgtgctcaccacgggtcgtttctgcttgaatcgtcacgtgacacatgtggtacttgtccttcaataccttgctgatttctgaataaatcggctcagcctcactcaacttcatatcatgcatattaacgtgggcggaaaagatcacgttgttttcatcaattgaccatgcatgaacgtgatggacactgaagacaccgtcgatttgcaacagatcttttttaatctgatcgtaatccaggctcggtgccccctgcatcaaaattcggcaggtttggcgaataatcgggatcgactcatagaaaatatacacggcaaccaacacggtgacaattgggtcaaccaatgtccaattataaagatcgattaaaattccaccaataataatcgccacagacgacagtgcatcactcaagatgtgcaggtaggttgctttcatgttaagactgcttttggaacccgagttcagcagaaaggccgacagcaagttagctgccaaaccaataaccgcaatggtcagcattaaattaccgttgatcggttcgggtttgctgatccgtttgagtgcttcaataatcagaattacacaaatcaaagccaaggcaattgaatttaagaatgcggcaataatctcagctcgtttatagccaaaagtattgcgcccgttttgccgccgtttgctgattcgactagccgcgtaactgaaaacaattgaaaccgaatccccagcgttatgaaaagcatcagaaatcagtgacaaacttcctgacagcgccccgccgatgaactcggcaatggtaataacaacatttagcacggtcacccagaaaaacttggcaccggctaattcttcgtgattatgatttttttcagccatccattaatcactccaatctactatcattattgcattagttcatgaaaatttccataacacgtgaacaatccttttagggataccagaaaatcgctctactaagccgttgaaaatggcccgacagcaatcgaaagctaagccattcctgcagaaaacctgtctcggtttccgtcccgagttttcctgttattttgattaaacctgcgaaagaggacagcaatcaaaagctaagccattcctgccgaaaacctgactcggtttccgtccggaatggcttagcttttgattgctaaacgtcctctttcgcactctattaaaatttatccgccaacctcctggactcaatttccgcatccgcgacgatttgttctgcttgatccgggaaatgatccattccttcaacacttaatttagtcactgactgaacgccgacaaaattcaaaattcccttaacatactgagtcccaaaatcctggttattgtacttgccgccggccgcctggatatggaaggcttttttgccgctggtcaacgggactgcagttcccgtatcagtatatttaaacgtcttcccggcgacattgatcgtgtcgatccacgcctttaatttagttgggaccattaaattaatcaagggatttgcgataaccactttatcagctgccaaaaactggtcagttgaggtattaaattcagcgagcttcacttgttggatcgacgttaagtcgctaaactgtctgccagcttcaagttcatcccacgcagaaaaaatatcgccgtcaatttcttgaaaatcaactttgtacaaatccaatttttcgataacatcatttggatggaccttcacatactcatccataaacgcgttcaacactttcaatgtccgcgactttgggctttcgggacgggcaatcaccactagtacttttgccattattcaagacctcttttacgattcaatcgggttgtcaactccgataatatagcatgatttcgtgggaatgacaacgctttcattttctagtaaaacatggtcgctgttttggtggggactgctttgcttctctctagccaaaatgtgctccttggggcaatgatggggacctaagccaccttctggcaaagcctgactcggcttcacccgagggtgcttataatcttattgctaaacgccccttgtcgcactcttaaaaaagggcccagtgcactctgcactggaccctcctgcggggaatcggccactctaatggttttaatcaaatatcacttcgttcatattcgaatactgatccggtttataaccgaatactcaaagtgcttttattcgcacgatggaactcttttgtcacattacttgtgcaatctaacagttatacaaacgatcatctaattaatgacttaaagagtgccgataccccacgtgtttagaatatcattcaattcttggtttaacaataactttgtctagatcttacaacgtttaatcagttgtttgacgtcttctaccgacgagccattttcaataaaacagttgaccatttccatccagtacatatcggtgtcgtcaaattctgcaccgactgccacttgaggcttgcttggaaccaggccgtttttgatataatcatcaatcacgtcaggactgacgttaaatttggctgccgtttcattcaatgtcaatttcataaccgttactcccaaatttcgttaaaattcaaatcaaatgatagtctaacagcttaccgacaaaatgcaacagcgaattattcgaccatccgccaattgccctcatcggctttcgaaatttgatctaagaagtgcagaatcgacgctgccaagtccttgtcatgctgaaccagcatattgagcgcctcaccggtaataatcggattactcaacgaaaattgctcgccttttttctcaccggtagagaatgccaacaccgtgttgccatcatcaatttcagtaataatgaagaacatactgaaatcatcgtcatctttcatataggcaggcatcgcccaaatcccatcactaatttcaaccaattcttcattgttgaatcggtaatcccggtgattctgttcattgactggcttatccagcacaaacatcattttgtcaaaaaccgggttgccaagcttaatattatcttccatcgaattcccctttgcattcatcataattcaatcacgcaaaaatcattctactgataattaccggttcatgcaagttcaatgaaaaagccagtcgatgaattattctttatagaccttggtggtgagaatttcataaatcgccatcgtcgctccaaaaaatagcccgcttctgacgtttggccaaatcactcccatgttttcgacactattgagtggactggtgccgtcaaagtaccaatccattaaaatatctgccatcaacataattaccatgaagtatattccaaaaccaattcctttcagaaccgcttttttgatgatctcctgccgactggtcgcttgaatctcacgcgtcacaatgtgtgcccgggtagtcgcaattaagatataaatgtttaccacgaagccaaccatcacaatgttaatcatgaccagacccatcagtgcttcttctgggtgcttttgacccacaaaaatggcgacaatgctcgaaaccaataggtagactgccaaaatcatataagcgttggtgccaatcctgccgatttgttggtgcttgtactcgtcgaatggtcgtttgaccccaaaccaatgcatcaataatcttgatccaaaactttctttagctttcattattttctcctcttgacatcagattccaccacaacgatatggttgattgcttctcgggcctcccagacacaagcgaccaccaagaataagaaggcaaagactcctgggaagggccgatcagccggactgacgttcatccagacagcaaataggaccaccccgccgagaaaaccaacccagacgctgcccatgaccgcatcttcaaccgcgtcatcatactggttggcaatcaccttgcggatatccaaacccaggtcagctgcccgccgtcgaatataaaggccggagccgcccacgccaatcaatagacttaaatagacaaacagcatccaagattcgctattgggggtattctttacgaacagtaaaacaccaccgttgaaaaccaatatgtataaccacatgaataaaaacgccttggagatgacggcattcatttgttgccgggcgtctttgtctaacaccccgcgaatgtgaaaaaagtatcggaataattttgtggaaatcgtatcgtcttgtcgcatgattttcctcctattcaactttgacaatgtgggcaatctctcgatgagtatcagatgtccaagaaatcaaaacaatgaatatcgcaaagccaatgctaacgatcgagaaaaaaccgttaaattgagcaaacatcaaatacgtaaccaatccataactgatgccaaaccatgcgccatggatcacggctttatgaactgcctttagatactctttagttgagacttcttgataattcagttttaattctgaaactttatgcgtgacgtaaagtcctacgccaccccatacaataaacatattgaacagaataaagccattgatcattgacccggtcttaatggcctgtgggagaagcagaaaaacggcattagcaatccctgtatacatccacaaaaacataaaggcgtttgtggcgaccttgccgatttctcgagcattatgctcatccaatacgccgcgaatactgaaaaagtatcgcatgattttaatcaagaaaccctctttcatgaattttcatctaccttccaaaatagtgtgtttaaatccgtccccaattcttccgccaagctgatacacaattttaacgacggattgtacttatcattttcaatcaaattgatggtttgcctggccaccccgactttttcagccaaggcaaattgggaaatgcctacctgctttcgatattcccggactctgttcaaattaacccgcctcccctggctgctttgtcacatatatgtgtcatcaataatataatgctactggcagataatgtcaactatatatgacaaaaaagagtgggacgcgaggcgttttgatcccagccatttaagcaaagaaacgagttattcctgtcttggaatgactcgtttctttgcttaaatggctgggatcagccgatagttccacgtttaaactagataacagtggaacgcaagagaggccaagacacaacttccaattagttgtgccccagcctctccttgagtattcttacttttatttagctgaatcgtggaaaaatgagcagcttccgggcatataaggggggcaaacaaatatccaagccctggatatttgtttgccccccttatattctggaagctagacgctcatttttccacactatttatacatacaacaaactccgctgcttggcggtcttttgcatatgatcgtacaagtggtcaccaatcatctgagtacccaccgtcttaaatccttttcgttcatacaatttctttgcttggggattttcaaaatccacattcaagccaatcaccgacttaccatcatttaaagccattcgtggcactgcagccaataatttactaccaattccatggccctgccaattaggatcaacggcgatggaatccaagtaccattcgtcagaattggtctcggaatcagggatatacggctctttaaaatcagcactctttttcgataaattgatcagaaccttattaatagcgtcctcattttcgctggggtagccaaagacgaccccaacaacttggccattggcctcggccaccacggtggatgccttactggacagatacgtgtctgtctggtaagccctcgtgatgaccttggctaatccaggttcgggaacgtcttctaattcatcaagttccatctcatcaaaaataatatcaattaacggggctatctggccggcgtcatcttgctgtgcttctctaacggttatcaaaaaaatcctcctaagtaaatgaacattcagtatgtgttacatcatatattactgaagttttcatttattgtcaaaattgaggatgaaactactgatcattttcagaatggttttcatgaccctgctgatcattttcattcagattactcttggggttgccaaactggtttcgttgaatcatgtccaattcagtgcggatttggccaagaatttcaatttccaatttctggatttccaaagaatgtggtaattgattttgggttaaattatccaattttgcatgtaagattctcagttcatgttcagatttctggttaacgtgataatcattttcagagctcatccgatcacggtcggcagcccggttctggctcatcatgataattggtgcctgaatggcggcaatacagcttaacgccaagtttaagagaataaatggataaggatcaaagtgcatgccaaacaactgcaggccattgatacacatccaagcaattaacacaaacgtaaaaacgccaatgaaaccccaactaccaccgaagcgggcaacggcatcggagactttctgaccaaacgttaaactcttggccaaattatcattgacgtcaataatatcgtaatcatcactctgcatcgccttggtcagtcgacgattaatctttttagtctgcttgacgtcggcattcaccatcccatcgacgcgcattaattggtacttcagtaagtcatggtcacaaataaaatcggtaaccttggctttcggataatcccccttgatcaaatttctggttgccggctccaaatcccttaggtatcgaccatcgatcaacatatgctcccggtggtcgataaagcaaatcgctgttttagcttctggcatgttctcaatccctccctaatgtatgtatgcaaaaaaaagaatgtctcaccgattattatatcagtaagccattcttttcaaatcatttaatagtcgtctaaaactagcgcctaaccaaagcgtgaaacattatgccttaattaaatctgattttgctttcaacaaagcggccttcaaagcacggatgtgctcgcgggtttgcttgtcttcctctgccgccttcatccatgataatacagacaagttagtttccatctcagcaataattttttgaaccgtctgatccgattcaccattggtagacatatctagtctcctccttaagttgatacccatactataccagaagtatgtgaaaatacaacggaaatgaacccgctttcatcgaattctaatttgaaattaacgcaagccgatcaaccattggtcttgcaatgttcatttgtgcacaatatgagtagacctctaatgaagaagtgctgaaatgtcttgtgggagttgagatttaaagcttaacgccctgttggaaaatggatcttcaaaattgagctgggtggcatggagtgcctgacgaccaattcccaattccattgggccgtgatacagggcatccccaagtaacggatgatcaatcgaagcgaagtggactcgaatttggtgggttcggccggtatgcaggaccacatcaaccaatgtccgatcctcgtacgcctggtcaacccagtattccgtttgtgccggcttgccatcagcggtaatccgttgaccgtatccggtggggtctttagcaatcggccggtcgatgaaaccgtgtttctgcaatccaacccctgccaccacagcctgatactgcttgtggagcgttttggccgccaacatctcattggctaagctgttggccagccgatgcttggcaattaacaccaggccgctggtaaatcgatccagccgcgtaataatatgggggaccaagtcttcggcgccattctcaaccaggtggcccttgactcgattcaccagggtatcatcgcggttcgccggtcccggcaccaccgttaggccagccggtttatcgacaatcagccagttgtcgtcttcatagataactgaaattggttgcctgctgacggcaacgtttggatcgcttgcctcagcaggaaaatcaaccgttacctgatcaccggctcgcagaacaactgttgcatcaacttttcgcccacctactcgaaattgaccaccatcagttttagcgctcttgtacatccggtggctgatgcccttggtattcaaaaattttttcaacgattgtgggtcattgtctgtcactgtccaagaaaatttcaaaatggcctccaaaaaaacatttttatattgtgtacaactattttgtttacgttataaatcccgccctaacagcaatcccagcatgtgaaccacattgcataacagaaaaaggcttttgtcaaggtcttgacatcgcttgcgcaacttgtaatatgtaagtacaagcaaacgcttgtgaatcttttataaaacgaaggagaagttaatatgaaagttgcagttattggttgtactcacgcaggaacctttgccatcaaaacaattttagcagaacacccagacgcagaggtcaccgtttacgaaaagaatgataacatttcgtttctttcatgcggaatcgctttatatctcgggggacatgtaaaggatccgcaaggcttgttctattctagcccagacgaacttaaaaaactaggcgccagcgttaagatgaatcacgaagttaccaacgttgaccccgcctccaaaaccattgaagtaaccgaccttaaaaatgatcaatcatttgaagacacttacgacaaattagttgtcactaccggttcatggccagttattccaccaatcaaaggcgttgacaacaaaaatgtttacctttgcaagaactggaatcacgccaaagaactctttgaaactgcacccgaaaagaaacgcatcaccatcgttggtgccggctacatcggtgccgaattagccgaagcttacaacaccaaaggacatgaagtaaccttactggatggtgccgaccgcatcatgagcaagtattttgacaaagaattcaccgacgttgttgaaaaagacttcaccgaccacggcgtcacccttggcttggatcagcaagtcacagaaatttccggtgacgacaccgttaccatcaaaactaccaaaggaacttacgaaaccgatttagttgttctctgcgtcggcttccgtcccaacactggtctattcaaaggcaagttggcaatgaccgacaacggtacgttgattaccaacgaatacatgcagacttcagatcctgatatttacggtgccggcgatagtgttgccgttcactacaacccaactcacggcttggcctatattccactggcaaccaatgccgttcgtcaaggaatcttagtcggcaagaacattgaaaagccaacagttaagtacatgggaacccaatcttcatcaggtctgaagttatacgacaagaccatcgtttccaccggcttgaccatggctgcggcaaaggcacaaaatatcaacgccagcgaggtgatcatcaccgataactaccggccagagttcatgccaaccactgaacctgttttgatgtcattggtttatgatccagaaacccgtcgaattcttggtggttcattactaagtacctacgatgtttcccaatcagctaataccctgtcggtatgtatccaaaatgaaaacacgatcgacgatttggcaatggttgatatgctgttccaaccacaatttgaccgcccattcaattacttgaacattttggcacaagccgcccaagagcaagctgccaagcttaccaaggccacttcaaaataacggttacattttagctttgtaaataagtctgaaccacgttataatatttactgcatggtgatgacgatctttctaaaccacatttagcgtctcacaaatgcatcccgtctgacttcggtcgggcgggttttcttatatcatgcttgtgctatcaataattcaggctatacttatggcagattcagacaggaaattggaggtatgaataatggcagaagaccattttatcatttcaacaactgaaaacatccccggaaaagaatacgaagtgatcggtgaagtctttggcttaaccacccagtccaaaaacgtcgttcgaaacatcggtgccggattgaaaaacattgtcggcggcgaaatcaaagattacaccaagatgttagatgaagcccgcaacatttccgttgaccggctaaaacaaaacgccattaaaatgggcgccgacgcggtcgtgatgatgcgctttgattccggatcgattggtgcggatatgcagtcagtcgctgcttatgggactgcggttaagtataagtaatccgccggttttatttggaggcctgaaggtagtgatacctttgggccttttttctgtggatcttttgatggttaaaagcagaaccttttgccctccctcctccagccaaaagcctgactcggctttcgtcgctcttctgttacttagctgaaacgtgcttcgggggacagcaaaaggattttaagcccctccagccaaaagcctgactcggctttcgtcgcttttctgttacttagctgaaacgtgcttcgggggacagcagggagaacctaagtcgcaccacccgaaagcctgactcggctttcgtcgctcttctgctacttagctgaaacgtgcttcgggggacagcgattggattctaagcccctccagccaaaagcctgactcggctttcgtccggaggggcttagaatccaatcgctaaacgtcccccttcgcactctttgtaaaattcacgtaaccaacacgtaaaagtttaaccaacttcaattcaaatcccctctttcacgatactatgaaattgcagaaacaaaatcttaagaattcatggagatgaaattgatgattgttaagttgaaaagttctatctttatctcagccgttgcgctggggattctcggcgtcagttgcgttgctcccagcgcccacgccagcgcccccaaagcacttacggctgaacatccgttaaccggaagtcctgccaaccataacgtaacctttaccgggacgtctgcgctttactccaaaccacccgttggcaaaggtgcccacgttgttgccggcaaggcgactttaaagcaattagcctcgtctaaatcttctgctgacaattttgcggctgatcgtcaggccactgccaaaaatggtgccgtctactacaaagtgacttcctttgacggccaataccatggctggatttacggtggcaaaaaagctggtcagtttagtggcggtctggaacctttctggacgttcaaccaaacgaccccaccggccagtctgagtaaatacaccttcaaaattgccgctcccgggttccaaaacgatggcaaaaccgttacatacaaagcacccatcaacacgacctaccaagctggcaaacagattggcgactccgttagatatgccaataccacgtttaagattgacggcatgggcacccgggctcgcgaaggcgatgtttgggttcacatcagtgcgctgaattctgccgacgccaaagcaaatggctggattctttacaaaggcctgcgtcaagcagaatcccccattccaaataatgccttgcgaatcgacctggttgacagcaatggtagtttgatccgctacatcaattacaccagcgccaacgcccaatacgaccaaccactgggtatcccatacgaaacttcctggacgctcggcaacgacgatctcgccaacattcaagttgccgttcgccaagcactccaagggaccggctacaacctggacacgatttctgccaaccaggccggctttcttgcccaggctaaattttgtcaccgggcctcactgaccgttaagaatgccgatcccattcccggaaacgccatccgcatcaatctggtcaacgatgccaacgcagtgatcgatactgtcgactacaccccaacaggcgcccaacccggccaattactggggaccagttcaaacggaacgacctcattaaatgatactgatcgaaaggcaatccagtccgccatttccacagccttaaaggattctgggtaccaattgaccgacttgtcagcagatcaaatctcagacttggccaaaaccaagtttggcggggccgtttacctgaaagccaacagctccgatacatcaatcgccgataacgcagttcgcatcaattttgttgacccaagtaacgggaaagtcatcaaatcgattgactatgtcaacaccgatgcggatgatccggccaagaaaggcaccactttaggcactcaaaaatccggcaagtggctgcttggcgatagtgacgttgtcgaaatcaatgccctggccgcctcgtcgttgtccggaaccggttatctgttgaaccaggaacacctttccgatgaccagcagagcactttggccaaagccaagtttggcagttccgtttcgatcaatgtcggcaaggccaacaactcaactcactttaatttatacgctgccagttcttcaggagacagcgccaacgctcaacagctgaccccaaccggattgacgtacgtgaacaacagctgggaatttccagatgtcggcggcagcagtcagccaacttacagccagttaagtgcggctgacattgccggtttgtcagccaccaatctggctaacttcaaacaggcactggcaaaatacagttctgattcgctggcagcgatcaataacagttttaaatcagctgccgagatgcagtacgtcgataatggccaaactgccagtttgaaccaggcagacctggattctgccaaaagcaatttgaagaacagcagttggtcaacgcttcaatcgccaaaatatccggtctttagaaaagacgacaacgggtcgattaacattgcttggcaaaccattacctaccacgccaaatcggtcaaacaaaatgcggatgaccaatccctcagcctgacctacacattcgacgcgcaataatcatttatttagaaaaggacgagataagatgaataaacctttaagaacgatcttcacgtttgccttggcatttaccgccgcgggtgttctcgcagcctcgaccaacgcccaagccgacatcatcgacgttcccggtgcggtcaaatcaattccccaagtcaacgccggcaatgtcctcaccaactatgattcaagtgatctgaaaaatattgataacacttcgccgatcgggaacatggatcgcaaatataaccagggcaccatcgatccaactcaggacaacgccggcgacacctttgcgaccactgacgcgacgacaacgaccgctaattcgtttaaaactcagtggttcctccccgacggtttcaatgtaaccgactaccaacacggtaacttccaaagcgtcgcactggacgactctgggaacgtgtactttgtcgaatctaacggcagtgataccaacttgggcgtgatcatcaaatttgataccaataagctcaaacaactggggctggaaaatgacccaatggccctatggaacgcctttaactacttcaatccgtatactgaagacggcgtcacccacaacaaccagtacgatgatctgtatgagtcgatgaaagatacctttaaaactgtcaagtcacttaccagcaaggaagccaccgttaaggcagcaatgaatgacctggcaaacgccaagcggacgacccaggcgaaatatcgaaaggccagcagcacgactaagaagcatttagccgcgagtctaaaagcaaatgccaaaaagatggccgctgacaggaccaaattaaccgcgttgcaaaaacaaattgcgcacggccagtcacagctcgccaaaatcaaggcgaaaaatcctgaattattcaagaacattgaaattgccgaaaccgctcagctcagtccacaagtcgatattggccacggccaaacattgaccttcaacccacaaaacaagcatttgtacctggttgaagataatacgttgaccgatctgcgcaaccgggatgaaaacaacaccgtcctggaaatggatcccaataccatggagccgatcagacaatacaatttcaaaatgttccagggaaccaaaggcaacctccagctgcacacgttagtctttgataagaacggtaacgcttattggggtcgaaagaacggcatgggctacatgttcttctatggtcgactcgacgaaaacagtgtcaaattcgccgctgcccctgaaaaattaaagacccgcggtggctcgcctaatcaaggggtcgctttcaacaatgtcaataatcgcatttatgtggtttctgacgatgtcttgacctccgttccggttgataaactgactgcaggcaccgcaaccccggatgacgtcaactactcggttttccaatccaaacgtgaatgggaatgcctggcatttgactcccaaggctacggccaccttctcgctctgtggccggcggaattgatgaagagtaccgcaccactaaactaaatttgaatggcacctaaaaagcctgcaactcagtatgatgctgaagttacaggcttttcctgtgccttgaacgtttaatgagtgcataaatcaaccacaaaggtccgaaaagcacaatgagaagattcaaacacaaatttttaaaaatgttaaagccaaaatcagccgcgcccttgtatgattgggtctgagtgtagcggaactcccaagggttgacggtgacgccattggccgaccaggcacggttcttatgattggcttgaacgtcagcatgatgcaggcggagggctttgtctttataggtttcaaattcaaccgattcttggctgaatgcctgccgcatcaggattcgaaccaccggcagaatcaggagcatatctaacaaaaagtaccaatcccaagcagacaggttaaatgccaaccgcagactgcctttggtggaccactcaggaagctgcagcgcaccatcataaaaataaatcagtaacagcgcaaccaagccacccaacagagaccacccataattcaagaaatgtctcacgattttcaagttgatccacctctcaacggcaacagaatatcttaaagataaccgttgcgacttgggatgtaaaggcattattaaaattattcacatttatttcacattttagacggattgtgattcagtgaccgcagctacctttgccaaaacggcggcaatttgatcaatcccggctaacagatcagcctcgctcattaccaatggtggcagtaaccgtaacgtattgtgcttagccgacaacgtcagcagcccgttttcttgaagttggccaataacatcctcgactttaacggcagcactcaaatgaatcccgatcatcagacctaatccactcacgctgtccacaacggttaatggcgaaatttgtttgtgaatggccgcaaagaccgcttgagatttttcttgaacctcagccaaaaatgtcggggttaactgttctaagactgcttttgcggaagccaaagcaatcttgttgccgccaaaagtcgtgccgtgagaacccggaccaaacgccttcgccagttcctttttacccagcatcgcaccaattggcaggccattgcccaaggctttggcacacgtaataatgtcaggatcaagatcgtagtgttggaaggcaaacttcattccggttcggccaatgcctgtctgcacctcgtcgatgattaacagaacgccctggtcgtggcatttagcggcaactttttgcagccactcgccattgccgttaacgacgacgccttctccttgaatcacttccaaaatgacagccgccaaatcctcattaatcgcgtcaagtgcctggggatcgttgtaatcagcgaaactgacctctggaaccagtggcttaaatcccgtctggatgtcgggattgccggtcaaggacatcgacccgtaagttcggccgtgaaagccattgttaaacgcgagaactttgcctttaccagttgccttgcgggccaatttaaatgcggcctcattggcttcagtacccgagttacagaaaaaggccagcatgccagctggacacagcgaagcggctacttcatcctgcagactgctggggtacagattggaggtatgccaaactttcccaagctgattaatcacactctgctcgatccaatcattgctgtaaccgaagctgcagaccccgattccgctggtaaaatccaaatacgatttgtgatgactatccactaaatgccaatcatgccccgaaacaatttccatcgggtattgggcatacgttggaaaaacatgttccatattctacactccttaaattgccagctgcttgaccgataaactggtccctgaatgctgcagctgattagtaattttaacttctttcacgccatgctttaatgcgtcaaatgcggctttgatttttggctgcatccctgatttgatgatctcagcctcgaacagttgattggccttctgcaggctcaattgatcaataacgtggctgttgaccatcacaccgggcacatcggttaccagatacagcttttctgcccccagcagtctggcaactgctgcagcagccacgtcaccattgacatttaaattcttacccgacttggtcacggccaacggggcgcacacgccaattccatcggccaaggcgtggtcgatgtaatcccgattgatgccggtaacctcgccaacctcaccataaactgcctgatccaggtagtcaccaaccagtacaggctgaccgccggcatttaatccgacgaccggaagtccatgagcagacaactggcgacagagtgccggctgaaccagtcccaataatacagcttgggtgactttgagggtttgggagctggtaacccggacgccgttaatcttggcgaccggcaaattgagttgggcgctccactcagagatttgtggcccaccgccatggacaatcagaatctgtttgaccatttggcgccagctccgtagctgttcaaaaaattcttctgtcagctgatcagtggcgtgaccgccaactttgacaacaattatctgactcatttccttcacctcctagcttcgatatgatgcgttgatttgaacatattgataagtgagatcacagccccaagcagttccggtagcttttccggcatgtaggtcgacgtcaatcacgactttgttctgtttaagggttgctgcgactttatcatcatcgatcccggtgcccaagctgttgtgaaccagctgcaggtcattaatggcaacgctgacgccgtttaaatcaacgtgggcggttgtctggccgattgcctgcataattctgccccaattgccgtcttcgccaaagatcatcgctttgaccaggttggagccgacaattgccttggcaacccgttggccctccaaatggttataagcgccagagacattgacttcgactaacttggaagccccttcgccatcaccggcgatctcctgtgccaaatgggtgaggacctgcttaaaagctgccgcaaaggttgggtaatccggatcggctttggttaagggctgattctcagcagcgccgttggccatcacaaccaccatgtcgttggtggacgtgtcgccgtcgacagtaatctgattgaaggtttcatcgactgtcgtgctgagcagctgctggagatctcctccggcaattgctgcatcagttgtcacaaagcccagcatcgtggccatgttgggatgaattatcccagaccctttacaaaatccggtggtggtcacctcctggccatcaatcaaacatttgacggtcatcgttttgggatgggtgtcggtggtcaagattgctttagtgacgccaacgttttgggtcagcttcaattgggaaatcccggccttaatcttgtccattggcagcggttcgccaatcacgccagtggaggcaatccccaccagttgcggatcgatttgaagtcgatcggcggtcattttctgcatcatcaaggcatcggtttctccttgcgccccgttgcatgaattggcattaccactattcatgaccaccgcttgtaattgatgtgccaagttgatcgtctgtttggtcagcttggttggtgcggcctgaaactggttcgtggtataaaccccggctgcgtttgcgggggtactggaataaagccatcccatatcgtcctggtcgggcttgaacccggcgtgggtcgagtcggcggaaaagcctttcggccaagtgaactgactcacttcaatgagtgtcttacttgtcatctgcattcaaatctctcctcggtttacggcaaaaacgtttgtaggttcaagccgctggtttcttcataatcaaacatctggttaaagttttgaacggcttggccggccgctcctttcagtaaattatcaatcacgctgtcgacgaccaccgtctgagtgaccggattgtagacaaccccaatatcgcagttgttagtcccgactacctgtttgatatcgggtaaatgctcaccggtataatgaacaaatggcttattgccgtaggtggtgtcatatgcctgatcaatttgggcatcgccaacgccgggcttaaccttggcataaatcgtactcatgatgccgcgggtgattggcagcagcgtcgtcataaattggatagcggccacatcatcgttccagcgctgcaattccaacatgatttccggaatgtgctggtgttgattgggtttatatatctgcaggttgtcattagcctgtgtgaaatgagtggcctgggcgggatttttgccggcgccagaggttcccgatttggcatcaacgacaatagactccgggtcaatcaagtcattttgaaccaatggtgccaaacctaataacgttgccgtggcataacagcccggattggcaacgtaggtctgatgagcggccgattcgaaatctgccaggccataatgagcttgccgcattgccggttgtggcgccgctggcttgtgataacagcgttgatactcgctggcatcctccagccttaagtctccagataggtcgatcactggaaagcctgcctgaatgtagggttggctgagctgggcggttaccccggccgacgtcgcgaaaaagaccatttgattgtctgccataattgtttcaggatcgtatggctgcacttgggtgtcatccgtgtaaaaagccgaaaccatttgcgacaatttctcattttcagttaatttatggtcatacaggttaataccggctacttctggatgccgacgaaggagttgatacaataccattcctgcatatcctgtaatcccgactaaagccacttgcaaaccaatcgcctctcatttttctaaatattcctctaattgaatattaatgaattgaaaacatcttacaacaacatacagattaatgcaatgttttttgggtattattcatatttttatttaaagattgatatttattcattattttgagtatacaggtgtatattgggcttgtgaaggaaatttattcacatcagtattcatgaataatattgtcgttttattcatatcgaggttctttttgcttagactgccgtggtgctcagttcgtcggctctgcctaccatagtggcctggatttcgagcctgtagtctcgaaatgccagggtgttgtaatcgccgctttcagcgactcaacaacacctttcactatggtagtcaatgccaacgaactgagcgccacttctttggaacgctgatggaacccccgttacgagttaacatccacatggtttgaaatatccctcacctggcagcttgtaaccctcatttggcagatggtagaaaaattagattcgaatagtcgaaacccttggaaggtcttggagacttgcaaaccaatatagcttgagaactgcatgaaccaaacatcagtcattttgccttctcggttgcctgattttgccggctgggcattgccagccatagtgaaagtgctgttgagtcgctgaaagcggcgattacagcacctttgtatttcaagactacaggcttgaaatcaaagccactatggcaggcggagcccagctggcaaaatcacaaacgttaagttaaattcccccacagtttgaccaactgagtcgacaatcatccacaaaacaaaaggactaaccacatagtgcagttaatccttcgtcaaactaattcaattcaaggtttcggtgccccaactgtttcctgaacgtcttccggaattttatccaaagcctgactgagatcggcaatcaggtcatcagcattttcgacacccaccgacactctgattaggtcgggcgtaatcccagcctcacgcaattcttcttcattcaactgcgcatgcgtcgtcggagctggatggataattaatgatttggcatcggcgacattggccagtaatgagaataacttgaggttttgaataagctgcttgccagctttttcaccgcccttcaaaccaagggtgaagattgagccgaccccctttggaaaatacttttcagccaaatcatggtacttactgtcttcaagtcccggataattgatccaggccaccttgggatggcgatccaagaagttgacaattttcttggtgttttcaacgtgacgttcaactcgtaatgaaagtgactccagcccctgaagtaataggaacgaattgaacggactaatcgtggcccccagatcccgcaaagattctgctctgactttggttgtgaacgcactaccaccgagatcggcaaataccaggccattatattgagcattcggttcggtgaagccgggataacggccgctttctttccagtcaaatttgccaccttccacaatcacgccacccattgtggtcccgtggccgccaatgaatttggtggccaaatggacaaccacatcagcgccgtgatccaatggtcgaaccaggtatggggtgccaaacgtgttatcaacaatcaagataatgccatgtttgtgagcaatctttgcaacggcttcgaaatcaatcaaattaattcccggattcccaatactttcgatatagagtgcttttgtgtgctcattaatcggtgcttcaaaattggccggatcgtccgggtccacgaaatgggtcttaatgcctaatttcggtaaagtgacgttgaagaggttaaaggttccgccatacaacgtgctggccgagacaatttcgtcacccttgccggcaacattcaaaatggcggcggtgatggctgccgaaccggttgccagggtgacgccgccggtaccgttttctagagcagcgacccgcttgtcgacaacatcggtggttgggttggtcagacgcgtatagatgttgccggggtccgtcaagccaaatcggccggcggcctgctctggattgtcgaatacgtacgaggtggtttgataaattgggactgctcgagaaccggtttcatcaaccgtttgacccgcatgtacctgaagtgtttcaaagtgtaagtgactgttttcttctgtcatattgataaacccactttcttatttgcgatgattttcgtccagttatcataaatctgaatactgctgtttttccaagaatagtccaccgttccggaatcctgatcaatgaagtagttttgcggcaatctgatcggcatctgctcatataaatcgcggtaatattccaataccagcgttccttcggaatactcgggatgaccggtgatgtaagtgctgtgaagactgtcagctgacaagatgatcgggccggtaacagctgatgaaacatccaccatcaaaccttccggaagatgatcctcgtccaaaacaatgccggtatgtctggattggggcatcttcagcaatcccccagcgccaaatccacgggcaatcggtgattccgcgttgatggtttctgccggataaacaccaaacaatttgctcagcagcaagtgtttccgaacaccaaagtcgtggaacaaacaggtttgagcagcccaacattcatacaaacattcagtgacatgatcctttgaccagtcaatgatttcctcaagttcatcccaataatcaacttggttgaacgggagcgtttcgattggcgctccagtgacaattaagccatcataatgggcatccctaatttgatccaaacagacataatcccgttgaatcaggtctgttgacgtcccacgaaaatgatgggatgacggatacataaacgttaattccgcgtcggaaccaatttcactgaaccgcgttaaaaactgacgctcagtattctgccgtgttggcattaggttcaacaccaagattgatagcggattagtaacttcgtggttaacccacttttgtgctgccaataagaacccattaattgcatttgccgtcatccaaatcatctccttaagtcataaaaaaagcttccttccacatagttatttcaactacgggacgaaagcttcgcgatgccaccctgatttactgtcacctcacaatgacagccttaataagtactccttggaatacccggtccaatatcgcggactcgcggatatcctagccttttgaccggatacctgactcagagctcatcttcacgtcgctgcaaaccacttctctcaccaaacgaagctctctttaggaatgcgttaacgttactcttctcttcaatgtctaatgtatttttaataattgctagtaactttatcatcacaacatgcccttgtcaacacccatttgaaaaatctttttgtcatgattaaaaacatatgagtttataatggaatgcaaagagatttttcaaggggtgaaagtatggatcaatcaatatctgaagatgagctgatcgccgtctgcggcaaggtcggtaaaattctgctcaccagcggtgcggaaacatcgcgtgtcgaaggcaccgttgaatatatcggccgcgctgcccattatgatatcagctgccacgcgacgattaccgccctgtttgtcggggtcaaaaatcagaccaaaacccacttggttaaagtccgcctgggggatttcaacttggaaaaggttgacgaaatcaacaccatgtcacggaaatttgtgaccggacagattgattttgccgagctcaaacgaaccatcgaccaaatcgacaagaaagtgattgactttacttggccggaaaaagtgtttggtgccgccatggtgtctgtcgcaccaatgctgctgttcaaggcaacttgggccgatctttcactagcgtttttcgtcggcatctttggctacttggcagcggccctttccagcccccggatcaagaccccttatgtggcagctggattaggcggttttacagtcggctttttggcagccgtcctgcagtccctgggaatcgccactaacgccgggaacatcattgtcagtgctttaatgccactggttccaggagtggccattaccaactcgtttcgagaaatcatcgatcggaatactatttccggagttgtccgggcggttgacgccttgattatcgctggatccatcggtgccggagttgttttgggcgttgggctgtccggaatcattttccatctgattggaggcggcctatgaaagtcctgattgaactcatcgtcagtttcgcctcaacggtcggcttcggattggttaccaacgtcccccggagatcactgttacccgccggcatcaccggatcactggcctgggtggcctattatttagtcttgcaagtcgataacgggttaattctccccaacttcaccgcggcaattgttatcggcattctgggtaatatttctgcggtgatgtttagagtccccgtcaatattatttatgtccccagcttggtttcattagtcccgggcggcattttatacctggggatgcgcagcttcactttggggaatgaaatccgcaccgggcaatacatgttcaatgcgctgacaattgccattgccttggcagtcgggttcgtcgtggcagaagttattttttatcgaattaaaccgcttttgctgcgacttttggcaaagcagcgtgaacgataaggtgaccgccctcattaatcataaggaatccaaatcaagcagacgtccagttgaatcttgggcgcctttttgagtgttgttgtttcgaaaatcagttcaaaatgatagcgtttccgtcataatggttctaaataaaatgttatcatgataacttttgaatgatggtcggcggtgggcattatctacctgtgtattcaccttttaaacaataatccgcattttatggcaaaagaatcaatatgtagtttataattattctaatttattcgacaaatcacctcataaatatgttacgctgtatttagcaagtcaaatacttgtaaatatcgaatctagaaaggcggaatcgttgatgaaagttattgttgttggttcatctcacggtgggtttgaaactgtcagggggattttggcagaaaagccggataccgaaattcaatggtatgaaaagggcgacttcatttcatttctctcctgtgggatgcagctttatcttgaaggggtcgtcaaggatgtcaacgctgttcgttatgcaacgccggaacaaatgcgggcccaaggtgtcaatgtgtttgtccaccaagaagttacctcaattaatccagacgagcatacggtagttgtccataatttggacgatgattcaactcgtgaagaaaaatatgacaagttggtactatctgccggtgccgtaccggcaagaattcctgttcctggcggcgatctcaaaaatgtctatgcaatgcgtggacgtgactgggccatcaaattaaaggagaagacggttgaccccgatgttcaaaatgtcaccgtcgtcggtgccggctatatcggtattgaagccgctgaagtcttttccaaagccggcaagcatgtgacgttgattgatattctccctcgtccattggccctgtacctggatcaggagtttaccgatgtcctttccaagacgctaaaggatcacaacatttacttggcaaccggccaaacagtcaagtcattcaatggtgaggacggccaggtgacggcagttaagactgatcaagctgaatatccaagtgacctggtcatcgagactgccggcatcaagccaaataccgactggttaaagggcacccttgatttaaccgataagggtctggtcaaagtcaatgatcatcaagaaaccagccagcctgatatttacgccgtcggtgacagcaccaaagttccatttgccccaactggtaaggaactccagattgctttggctaccaatgctcgacgccaaggcaggattgctgcgaaaaacgtcctgggagacgacatgaagatgccggctgtttccggttcatctgccctgtctgtctttgattaccactttgcttcaacgggaatcaaggaagggacttccgcagccaacggcgtgttgagtcaatccgtcttcgtaactgataccacccagccaccattcgtaccaaatgaggccggcaatcaaaaggtctacttcaagttgacctttgatcccggaaatcaccggattttgggtgctcagattatgtcgaagcgtgacgtcaccgccaacatgaatgccattagtttggccgtccaagcaaaaatgacgttggatgatctagcctatgccgacttcttcttccaaccaggatttgaccggccgtggaatatcatgaatgtagctgctcaaaaagcactccaaactttagccaaataatcagttaaacaaaattcctccctaaaacgattgctcaccgttacgcaaacgcaaatctgcgttatagtaaaggcgtagctaaaatcattttagggaggaatttttttgaaaactgtcttaattcttggtgctgccggacaaattcccagtttcttaatcccccagctcttaaaacaaactgattttaatttaaaactttacgctcggaatgccaccagtcggcttcacgtaacggatcccaagcgcgaaacagtcattgatggtgactttaacgatcacgatactttgaacaaggccatggatggtgtcgacgctgtctatctcaatgagatgcgggacatcacgtccgttaagaacatcattgaggcaatggatgccaaccacgttcgccagttcattggggcgaccgttctcgggatcgaagacgaagtcaaaggtgcctttggtcagtggaataccagcatgattgaaagctcgatcaccaagcgcaaaaccactgccaaagcgatcgaagattctgatctgacatataccctcttgcgattggcatggctgtacaacaaggatggcaataccaattacgaattgactgaaagcggtgaaccgtttggtggtacggaagtcactcgtcaggcggtggcccagttaatcatcgacatcttaaacgacaactcacggaaatttactcgcaagagtatcggtgtcaatgaaccgaacaccaagttcgataagccgtcattttattgattcaatttcggtgactttgattaccactgttatattgataaaacgtgcagagtttaaacaaaggagcgagtcattccaagacaggaatgactcgctcctttgcttaaatgatgggtcaaaacgcattacgttccacactcataaatttccatcatcaattaatgaaaaattttcttcgcaatgtcaaacgcagaccaagcctttggccagccggcataaaatgctaaatgagtgatgatctcgacgatttcgtcttttgtaaccccgtttgccttggccattttcatatgggcttccagttgtgggaacaacccctgtgacatcaagctggcacaggtgatcatgctgcggtccctggcagacagctttgattctcttgaccagacttcgccaaataaaacgtcgtcatttagttcggcaaatttgggtgcaaaatcacccagtgcatctcttccagcagtttgttttttagccatgattattgaacctccaattgatcgtattcttcatctgagaccggttcgagccactccggtgtcccagcggtaatcgcaatgtgtgagaaccaactgtcttttgtggccccatgccagtgcttgacgccatcgtgagtcacgaccacatctcccggaactaagtgttgagcgggcttgccggcctcttgataccagccttcgccaccggtgaccaacaaaatttgataaccatcgtggtgaatatgccaattattgcgacaaccgggttcaaaagtgacgttgccaacccccacattaaccgctggatcattgactaatccctgaagataactctgacccacaaaatacttggcataagcatcgtttttcgggccagctgggaaaatcacaccatttttaacattttcatttttaatcattttatttcctcctcatccaaaacatttactttacaaataggagcatacaacttaaagttaactttaagtcaaacacttcttaaaaaataatggaggaaatatcatgccagctattcaatcagaaaccagttatgaaatcggcgaatttgccgaaattgtcggcctctccgctccaaccatccgctactatgaaaatcaggggctactcaaagcccgtcggacagacaacggtcgccgatattttaccgaacaggacatcaagtgggtcaaattcctcttgcatcttaaaggcaccggaatgagcatcaacgacctgaaaaaatacgtcacttggcgggctgagggcgaccagaccatccctgaccgcctggatttactcaagaaaaccaaggccgatttcatggaagaataccgccaagtccagcatcatctgcagattctaaatgataaaattgactggtatgaagccaaagaatccggcaaagataccggtaaggaaccctttgccacctacttgcagcgactggggcaccatgaataagtttctgagaatttcacagaaacttgtcagggactaccactttcaaatgagctgccagtcactctacaatgttcatgattattcaattgaaccagaattgaggggaaattatgacgaataccatcctgctggttgaagacgaggaagcactcagctcgtatttaatcccagaattaaaatttgaagattatcaggtattgttggcaaaagacggtcttgaagccctccaagtctatgacaataaccgaggcaacttagatctgatcattctggattggatgctgccaaagcttgacggactggaagttctacggcgaatccgcaaaaatgatgacatcccagtcatcatgatgaccgccagagattacgtcggcgataaagtcgctggactcgacagcggtgccgatgattacattaccaaaccatttgaaatcgaagaactgctggcccgaattcgagtcgttctccgccacgagagtcatcaccaccagcaaagcgaactgtataccgtagaggacctgaccttaaacaccaagtcccgccaggtttcgcggggaaatcaactgattcaactcacccaacgggagtacgaattgttattaaccctcattcgccacggcggcgaaaccctcacccgtgatgagctgcttgacgcagtttggggggtcgacttcgaaggccagccaaatgtcgttgacgtttatatccgctacttgcgcaacaaagttgatcggggatattccaaacagctgatccacacggtccgtggagtcggctatgtgatgtccggaaattatcaggaataaggagtcttagtttggcaaagaaacagcatcgcaccacctatcaggcaatccgtcaccactttattatcctgctaaccttttttgccctatttaccggtatcgccgttgtcttggtggtgggcgtgaatttggtccgccaaagcgaaagccaatcggtagaattactcagaagccttaatcgctcattcattgacgacaaaccggattggaaacagtggcggaaaaacagcagcatcaatactgaaaatacttatgtcagggtaacggatcaggttcatacggctaaacagccggaactattttattcccaaggagcacctcaatttttggcggcagcaccaaccccgatttcaaaaatgatccacatacctgttttcccggctctcatttatgccaagggctatggcctcttctattatcgcagcggtgttcggcatggtagtcaaaagaatatccgctcagaaatttggctgagcctcaatccaatcgttcaactgttaacatcggtcattttaatcgttctgttggtttcacttgccagtctgtcactgggctggttcgtcatttccctgattgcccgccagttaacggagccgctgcaacccctccaggaagccgccaaggctcatagccaatcgattaatcgggttgaaacccttctaccggttccggagtccccaatcgaggccaaacagcttgcgattagctttaacgatttgttatcagccatcatcaaaaataaccaaaaagaaaaagcatttatttccaatgcatctcatgaattgcgaacaccgattgcagctatccggggtcatattgcccttgttaaacgccgcggcaaagcgcatcctgaaattatcgacagctcacttcattttattgacgacgagtcagcaaaaatgcaggcgctggtgaacagtctgctggccctgtcgcgagccgacaaggaagtcgtcaccaaaagtcattttgatttagcagccatcgtcaacgaaaccgtcgaagaacagcgggtgcttttagagcaaccaattcaagttgtgggcgagcaatcagcaatcgttcatgccaaccagaccaatattacccagattttatctgcccttttagataatgccggcaaatattccccgccggatgcccaaatcacggtcaaaatcagcaaacgtgaccatcaaacaattttggctgtcgaaaacaatggcccaagcatccccgaggctgaccaggcccatatctttgatcgtttttaccgcggggatcctgcccacaacagtcacattaccggcaacggattaggcttagcaattgccagtcagcttgcccagctaaatgatgtcggcttgcgggtcacaaatatcttgccccacggcgtctcgtttgaagtcagctttcccgacctcgatttaacaaaatagcaccatcaattgccttgcgttcttcttaactgacacttacatccccactttgagaccttctgagaatttatcagaaggctctttttttagccctgtatttcttcgccaaaaatcacagtattcttggcttgtaagttcgataaccaagtgattggaggaatattcatgcagacatcaacaatcaaaaatcatccgctgctgttcttcggctggctgatctttattggcatcacaggattggtcctcctgcaaaatgttcagttgtatttttgggaccgcgattttcttaactatctccagcgatttattaccccagacagaacaagttttttcaaaggagttgccctgttcggcagcccaatgataacagttgggttggcgattatcgccagtgtgtttctttggcagcgaaaaatgctggaggaggctctgacaaccctggtggtagtcgttaccggcaatgcgggtggcttaatcattaagcatctaactgaacgtccacgaccaaccaccatgctagcccatgactcaggctacagcttcccaagcggccatgtcgtcagtgccgttattctgctgttaattgtttttcaattcatcctcccgctcatctcatcggtgaggttgagaatgtttttcagcatgatgttagtcttctgggtagccctgatttgcctctcgcgactctacctacaggttcactatccaactgatgtgattggtgcggcgctgtatggactgctgtggtgggaatcagcaatggcagtccttcaccgccagcaattaaatacccaaaaagttatccaacacaatcgggggcagtcatcatgaaccttaaatatacaaccagaaatatcctgttaatcgtcgctttatcggcagccctgaccggcgtggtgttggtgatgatcttcacagttaaccaaatcaccccatttgggactcacaatctattagttggtgatatgagtgcccaatacgtcccatttctgaccggctttcgaaacgccctcttaaccggacacttctcattattttctttttcgcttggcgtcggtgaaaacatctttccgctcatcacgtactatctattgagtccatttaacttactggtcctcctatttccaacgagccagctgccggtggccatttcctggatttttatcctcaaagacatgacgattgccgcgacgacctgctggtttctcgctcggcatttcaatcgaattcatcttttactgccatttttcgctctagctttcagcctttgcggttttgcttcggcaaacttcgtcaatatcatgtggctggacggcctcatttatttgccgttaatctgtgacggaatcgatcagatcaaagcgggaaaacaatcgatcagtttatttgtctggctgacggcagcgatcgtgtccaactactatatcggctatatgctcggactgtttaccctcatctacgcagtcgaaacgattatccgaaccaacgatcttcacttctctttgatcaccgccatcagccacaatcgacagtttattaccagattcattttcaccgaagccgccagtgtcatgtccagtatggtggtgctattgccgaccatgttgggcatgcttcagaccgccaagaccagcccgtcaaccaccaatagtctggctgcggcagccaagccacaatttggtttggagatcttttcccaattgggtttgggcgggcaaacgtacgataatcggctgctacatgctccggcgattttttcgtccttagcgatcgcccttttagtgatcggctactttttccatccccaaatccctcgaaaccacaaactagcggtctcggtaacggctggaattctctcactcagtatgctgattggaccgatcaatctggtttggcacatgctcaatgaaccgtccggctctccatttcgctattcattcttgctgagttttgtcttgatctccgcggcttacgaaatgctgttggccaccccccaacgcttgtcattcaaggctaaattgagcactccaacaattctagcgggattgttaattgtcggttatctcgacatccgcctgggacgccatgtgctcacaaacgactatttggccgttcagcccaactcactcaacgtcctcatagtcaatctccttttaacggtcatcttctcatacctcctgttcacagccgtccatccgatgcagcaattattaattggaacaattgtctgcctggaaatgggtaccaacttcggctacaccctcaagagcgaaccgctgcctttgcaaacaagctacgagactgcctatcctcgagttgataccatcgtttcaaagactaaaaccaccgacaatcagctataccgcattgaccagtctcacagtcagttggctcccatattcaaagaaacttacttaggctataacgatcccatattgttcaattacaacggcattcaagaatacagctcgacgttaaccgaatccacccgtcaatcactgaaaatgatcggtctgttcagtaagaatcagcgccgaatcagtactgccggctcgactgccatttccgacatgctgttgggggttaaatatcagctgaacccagctggaaaaattgagaaaaacacatcctttgcagggatcggcttcccggttaccaaccaattcgctcatctacaactcaccgccggcacactatttaccaatctggaaaggattctccaacgactgacaccttccgaccaaccgtatttagtaagcgaatctggaaccaacccacaacggcaaacaatcagggctcgcgaaaaatacaccctgacgatcattcccaagctcagcggtccgctgtacttcgatacttcagataaactactggattacagcgccatttatgtcaatcacacccgattgaaaaccatccccaatcaacttgataaacagtacctggttaaattgggaactgccaaacgtggcgtcccggttaccctacagctcacatccaaaagtcaaaacacccttcacgatagtcatttcaacagcctgaatgaatcgcaattcagcaaagttgatcaacacctgaaacaaagcgcttttacccccacctataccaacgatcgtttggtggggacggcagttcgcccaaattcacaatcagaatggctgtatacagcaattccatatgatcccggatggacggcaaccgttaatggccaacccgttgaaccaattaaggtgttgggtaactttaccgcattaccactcactgatcagtcaaaccacatcgtgatgtcttatcacgtccccgggttattgcttgggatcattctttctcttttaggcttattggcgtttagttggcgccaatttcgcaatcttgcccttcgaaaagacgtgagtcaacaggcgccaggagatggaacaccctcaaacggggaaacttactagtaatactggcaagaaacgttcgatcaacgtaactgctgcgatcctgcctgcctttgaatttcaaatcatgtagaggtatactcatttaacaacataaaaatcaaaggaggcaactacatgatctattcaccattaaatgaatgtgatgttccaactatccgttaatagcgggttattccgctaatcatttcatacgaaatctaaaaagcggaggaacatcatattgaattcaaaaaaaatgctcggtgcattgctgctaagtttagctgccagtatctgggggggcatgtttgtcgtggttaaagtggtggttgagactatcccgccaattgaactggtctggttgcgatacctgattgcgttggtttgtttaatgttatttgcagtcatttttcacattaaatggcgtttcaatcaacgtgatttgggaatcatcattttaatcggtattattggcaatgccatttccatcgtgacccaagaaaccggaacttggctgtcaaacgctcagactggggcggtgattacttcagctacgccgaccttcatgatcatatttgcctggtggttgcttggtgagaaattggatgctgttaagatcatttctgttaccatggccactttaggcgttatctggattgttggcgttcacttctcaggaacccatgtgttactcggaattttttcgttaatcattgccgcattgacttgggcgttgatgtcggtcctggtcaaaaaagtttcaggtacctataactcacttcaaatcacaattatgtcgacttttgtcgcattcgtttgcctcacgccatttgtcttgagccacatggatgtgattacccaagctcattacctggaacccaaaattggtctcagtctcctttatctgggaatcgtctcgacagccttgggctttgttatgtggaataaaggccttcagttaatgaacgctgccagttctggacttttctttctgtttcaaccgattgtaggaacgctacttggatggttggttttaggtgaaaccatttcgtggggatttgtctttggcaccatgatgattatcggcagtgtttgggtatcaattcgattcgctaaataatgacacttaaaaagggaaacgcaaaattgcgtttccctttaatcgtttctaaaaattttattcgcccttagcctggtaaacgtactgacgcgtcattggcagaccggttccacttggggaattggtcaacaagtactgcataacatcaatattaccggcttcaaatgaagcggcactggcttgtaagtacatgccccacattctggagaacggcacaccgtacttttctttgaccttatcgatgaccttcatgtagttggcgtaccagatttccaaggttttttgatagtgacggcgcaacggctccaaatcactcatctgcattccggcatccatgatgtgagtcatgttttcagcgacgtttggaatatagccgccatggaaaatatacttgttcaagaacggatcaacgccggctccctggtgctgaccagtaatcccgtggattaaggctcgtccttcaggtttcaagaaatcatgaactttctggaagtataagccaaggttttccttgccaacgtgttcaaacattccgactgaagtgacgtagttaaattggcctttgacttcccgatagtcttcaagcaaaacgtcaactttaccttcaaggtggcgttctttgatttgttgcttggtgtagtcatattgttcctggctcaaagtaattccggtagcctttaaatcaaagtcttcagcggccatgaacaacaaagtgccccaaccactgccgatgtccaataaagtattaccggcaaccggattgagtttgtgtaaaatatgccggtctttgttcaactgagcttcttccaaagtatcgtcatcgtgttcaaaataggcacatgaataagtcatgctcttatcaagccacattctataaaaatcattaccaatatcataatgcttttgaatgtctgactcactggctttctccgagtgggaaacctttggtaagtgcttcaagaatgggttgttggttaagaagctatggtcggcacgaaaggctgaggcaactagctcttgaatgctgccgtcaatctcaatgtcgccgttcatataggcttctgccaataccagtgttggctgtgaagtcattttctttaatggaatttctttcttaatcgtaatcttaacttgcggctcaccatctccgtagttatcggtcttaccatcccagtaagttacagatactggaatatcaaacgcatggctaagcagctctttataagtgatcttctctaacatgaaatttcctccattgtttttctatcagtaacagtgtaacgcttttaggggtataaaaagcaagcataaattcttttgaatttactttcctgttggaacgactttaaatttagtgccgtcttttttaaccactgcatagaggatcgaatcttgattatcgtccagatagcccaggtcaactgcaggatggccgtcgatttcggtcatcccttcaaatcgatcgaataggacctgtctcgctaatttgagttcgtggcttttggattcggccttttgggcagcgactgccaaagtgtagccctgatccaataaaactttcatctgatagaccttgatcagcatactataggaaaatttgcgattctggccttttccctgggtgctttcgatatagccctttcgttcccagtaccgcaatttggtctgggaaacgccggtggcattcgcaacgtctccgatgcccaagtgccagtcgttctctttcatgatttgagccagcttctgctggaactctttatccaaaatgatccctcgtttctcattttcaaaagttgtaattgcttccattgccttaaaaccggcattccaattattaaatcgtctgataccagtgagacattaattaacattaagtatatatttttaaatatgtttgtcaacttgcttgacaattatgttgaaacattttatattagtccatgttcgattttgagagaaatcaaaattttaaataaagaaggtcctaaatcgtgggtaacgcagtagataaaaacgggaagtcatacaaccgtggtttgatgattatcgttattctggtcggaacattttgtaccgttctgaatcagacgattctttcaaccgcctttcctaccattatgaaagcattcgacgtcaacacatcgactgttcagtggttgaccactgggttcatgatggttaacggaattatgattcctgttagtgcttggttaagcacaagattcaattctaagtggctttatattagtgccatgaccactttctttgccggaacgatcgtttgttacatcgctcccaactttgcgaccttattaatcggtcgtttgattcaagccctcggtgttggggttaccatgccattacttcagacaattatgctttccatcttcccacctgccaaacgtgggactgccatgggacttgccggaatcgttattggcctggcacctgcaattgggccaaccctttccggatgggtcattgataactggacttggcgtgatctgttcggaatgatcattccattgatgttcttagttattcttgccagtttctggctcgtcagaagtgtattggataccaagaagacgggcatcgacctgctttcaatcgtcatgtctaccatcggatttggaagtttgctttacggcttctcatcagttggtgaagatggttggggcagcacaatcgtgatttcaacgttgatcgtcggcgttgtcttcatcgccttgttcatttggcgtcaattgactatgaagaccccattcctggaatttcgggtctaccgttcagtaccatttaccgtctcagcgattttgagttccgttaccatgatggccatggtcggagtcgaaatggtcattccactttacctgcagattgttaaaggcatgtccgcctttcattccggattaacgttgctggccggcgctttaatgatgggaattatgagcccaattaccggccgggccgttgaccgttttggtgctaaacgcctgtcaatcttaggaatgagcttgttaacattagggtcaattccgtttatcttcattaccaagagcacgtcaactttatacattgttgtcttctacgctattcggatgtttggaatttcaatgacaatgatgcctgctacgactgttggaatgaactcactaccaattaatttgttaagtcacggaactgccgtcaacaacactcagcgacaggttgccgcttcagttggaacggctgtgttgatcagtatcttgaccaacgtgacgaagagcaacaaaccggctcactcaatgctgacaagtaacccgcttggctaccgtgatcacatgatcaacgccacgttaaccggttatcacgccgcatttgccatttcactgctcttctgtatcttagctttgatcactgccttcttcttgaagaaccgtggtcactcaactgattacactaaaaatggaggtgaagactaatgatcgttatcacacttgtaattggggttgttctcgcgtttgtcttcttcatctacatttcaagtaaaccggtcagttatacccttactgcgctctcactattgttggcagtcgtatcaatggtcttcatcattaagaacgaccacgatcattacggcatgaaacaagtgacaacagaaacatcacagcaaatttacccaatcggcagcaagcaaatgcagatgattctctatcagccgattggaacagctaataagcatcaagtttatatttatcaaaaatcagccaatgctaaaaagaagtcccatacgcaaacgactgataccaccaacaaagtggtcatgaccagcggtacgactcacatggtcactcaaactacgcgttgggagtacaagagtgatgctgccaaattgtggttcggcatttctggtgaaggccacaaattcgtcaaacgtcacaacatcttgtatgtcaacaaatcagttcaggttctctccgctcaacaagccaaagcccttaagaaaatgatggcaagcaaatcttaccaagctaaattaaaggcccaaggtaaagcgtttgtcaccaagcaggtgatggccgcaatgaagaagaacccaaccatgtcagctgctgaccgggccaaattggtcaagcaggccaccgctgaattccaagcacaagccattaagaatgtgctggcacagattaaaaaataggttccatttctcttccaatattaaagcgcaccaattcaacaataaccgttgagttggtgcgcttttttagtcaattaatttgttaggacttcggtcaactttgacaggaagaattctaattctgcatgagttcccacggtgactctaatgtgatgcggatacccccagggcgtgcagtcacggacaatcaccccatttttcatgagggcgttgacaacgcttattgcatcgggtgcgccatcgggaagttgggcaaacacaaaattagcttgggacggggcaactttgaagcccagaagtcccaacgactcaaccagtccttcacgatcaccgagaatttttttgcgcgccttattagattcggtttgatcaaattgaagcgcagcacttgcgccggcgatcgccgttcggttggtgttgaacggttctgtcacagtatcataagcctgaattgcctcaggatcacccagcacataacccagtcgggcacctgccaggccatagaatttggaaaaagtccggatgaccatgacccgtttattgccaatatagcgaagaaagttcgccaagctcaagtgatcggcaaattgggcataagcttcatcaacaatcacccagacattatcaggtaactgatccataaaagcctcaagtttggctgcatcggtcaacgtcccggttggattgttgggattacagatccaaatcagcttcgttttgtcggtgatcttttgctggaattcgtccagatcgaactggtaatcatcggtcaatgggatttcaatgaccttggcgcccattaatcgagacacttcccggtacaaccggtacgactgtttggcaatcagcacctcgtcaccggcattaataaacatcttggctaccgtttcgataatgttgccggcaccactacccaaagccacattctctggttttaagccattttcatccgccaatagctgaatcaaattgacaaagtcatcttccggataccgattcagcgtactaatacttctaatcattgcattcttggagtggtagtacggcgcatagggattctcattagagcccaacttgaccactttatccaaatgatactttcgagcgacctcatcctctgtttcaccttgaatgtatggttgagtcacattgacttcatttcgaaatgttgcatcaaattttgccatcatttcaccgccttaatcacaaattaaatatctttataagtccatcctaccgcgaattggttctggattgtgaattcttgccctttaatttgcattaaaaaagaggccgggacataaatggtaaagatggctgtcattgcaactttgattaccacttgtatatggataaaacttgtaacaatcggctgatcccggccatttaacgcataaagccagtcattccaaaatccggaataactggctttatacgttaaattctgggatcaaatcgcctttcgtcccaatctcttgaaaatcattgatcaattgtgactgattccatcacaacgtcttcattaggcttgtcttgagcatttttctcaacctggctaatctctttaaccacgtccatgccagagataacctgaccaaaaacagtgtgtctgaagtccagccaaggcgttccgccattcttgtaggcttcaataatttgttcaggataaccggccgtcttcatttgagaaatcatcccgtcatcaacatgttcgttggaaacaatgaagaactggctgccattggtatcagggccggcgttggccatcgacaatgcgccgttaatgttgaataactcaggtgaaaattcgtcggcaaaattgccaccaaagctgctctcaccacccatgccggttccagttgggtcgccgccttggatcatgaattcaggaatgacccggtgaaaaataacgccgttgtaataacctttttctgctaaggcaacgaagttttcaacggtctttggggcttgttcagggaacaattgaaccacaatatcaccgtgattggttttaatggtggctttgggtcccttggcattctttaaatctaattgaggtaacgtcatgatatatctcctttagttaacaaaatctatcttaaatgagcttatcacacccagttcataaagtcaggaacttcgacggtatttcccccgttttaaccccaattacggtaaaatatggataaagtttactttataaaataacggggtatttgtgatgagggttaatcaagcgcactggcggcgaaatatttatttgttcttgacgagtcaatttttgactgggattaccagcatgatcgttcagtatgccatcatttggtatctaaccaaagaaaccggctcggccaccatcctcagcatcgcgacaattttgggcatgctgccgatggcactgctcagtccatttgtcggaccactggtcgatcgctggaacaagaaggccttactcatcgttccagacgtggtggccgcaatctttgcaattatcctgtcggtttccggcggggtctttcacgtctttccaatctggctgatttttgtgtcgctattaatgcggtccattgctcagacttttcaaatgccgacgattcaatcggtgatgccaacgatggttcccgataaggaattgacaaagctcaacggtcaactcggcatggtccaatcagccaatatgattattgcgccggctctcggtgccttcctatttgcgattatccccctgcaatatctgattttgctggacgtgcttggcgccatcctgggtatcagtatcttgatttgggtccagattcccaacaacgaaaagatcgacgctgctctgcatatgctgcacaacaccaagcttggcgttcaacaactcatgcacaataaggggctctggtacattaccatcaccggagcagtcttcaccctgctgtacatgccggcggccagcatgtatccgctaatgacaatgaaatatttccagggaaccgttggccaagctggctttatcgaagctttgtactccggtgggatgctggttggcggggccatcatcggtatctggggcaactggtccgacagaatgaaaccagtgatcattgcattcttccttgtcggcatccctaccggtttaagtggcctgcttcccggtaaccagaccgggtttatgtggtttgccattttaaatgtcgtcgaaggaattgccacaccgtttttcaacacgctcttgatggcgatgattcagcagagttacccgcctcagcaactgggacgagtcctgggggtactaaattccctaatgagtttaaccgggccaatcggactgattttcgccggcccccttgccgatgcattgggagttgagatgctctttgtcatcgccgggattggcacggtcatttgtgggatttttgccttgatgatcccaatcatgcgagaatatgatttaaaacttcaagcccgactcgccaaagaagattaattttaaattggtagttgccttaaagtggacttcaaggtctacaatgactttgtaaataaatgtaaggggagattatttgatgaaatcaacattatttgtaaaaccaggaaaagttgaaattgaagagattgacaagccaaccatccaagctgatgacgacgttattttacacattgtccgtgcctgcgtctgtggatctgatttgtgggcttaccgtggcttggaagataaggaacccaattccgaaaacagcggccacgaagcaattgcgatcgttgatcaagtcggtaaagacattactaccgttcagcccggcgactttgtgattgccccatttacccatggatgtggacactgtgctgcctgccgtgccggttatgaaggcagctgccaaactcatagcgataacttcagttccggctaccaagccgaatatgtgcgttaccagcacgctgaatggtcactggtcaagatccctgggaaaccagccgattacagcgatggcatgttgaactcgctgttgtcgttggctgacgttatggcaaccggctatcatgctgcccgggttgccaacgtcaaagctggtgacacagttgtcgttgtcggtgacggtgccgttggcctgtgtggcgtgattgcttctcaaatgcggggtgccagccggatcatcgcaatgagccgccatgaagatcgtcaaaaattggctactgaatttggtgcaactgatattgtccctgaacgaggcgacgaagcagttgccaaagtcatggcattaaccaacggtgccggcgcggatgccgtactggaatgtgttggctctgagctttcaaccgaaactgccatgaaggttgctcgtccaggcgcaatcgttggccgagttggtctgccgcataccaagaagactgacctcagcagttcgttctatggcaaccttggcattgccggaggtccagcttcagtaaccacctacgataaatcagtcctgttgaaggctgtcttagacggtgacattcacccaggcaaggtcttcaccaagcgcttcaatctggatgaaattgacgatgcttatcaagcaatggctaaacgtgaagctattaagtcgctggttgttgttcaagattaataagagtgtgaaagaggacgtttagcaattgaaatttaagcccctccagacggaaaccgagtcaggttttcgggtggaggggcttaaaatttggttgctgtcctcttgaacacatttaatccaaataacagtaagacaccaagaaaccgagtcaggttttcggctggtggcgcttaaatttcaattgctgccctctttcacacatttcaactagatatcaatagaacccaagagaggccaggacacaactaacaatcagttgtgtcccggcctctagtcttttggctgattattctcttttccgcttcttaccaaatccaagccaaccaaacattgccaataagatcatgccaatgattgaaaccgcttggccagtttcggtatcaccagtttgtggtaaggctgcttgtcggccttcgttagttcctttctctgtagctgcttggccaacagcttgggttgttgcttgcttagcttggccagcttgagcatcgttagcaaccactttgccaggatcattgaccttcaattgttctttgctattttgagggtcttttgcggtttgcttcttcggtgcttcaggtgccttttcgccagtcttgatcattcccggttcctgagactcggtcgtgtcttcatgaacaacattctcctgcggtgtcggatttgtctcatttggcgtaccaggtgtattcggtgttggcgtcggagttcccggagttggcgtgcttggtgttggagtgatcggcttgttaggatccacgttgccaccaggcgttaccggattctcagccttcttcggtgccactggggcaaccggttcttgtcgctggtcaaggtttggctggtagtctgccacgactgtcgttccagcttcaggtgcggttggaccggtcacatcaaccactttggttccgttattttcgactggtgccaccggcgcaactggctgttccgcgtcgttggttgggcgggtttcatccaaaattggttgggctggttccttggccttttcatcaacgttgacgactttaattgcggccaacaatggttccgtatagcccatttgattaaccccgacaacgtatgagttgtaagccacttcatctttgagtttgtcgtttaactcgccaaccccaacctgtttgccggcttcaacatatttcgagataaaggtcgatttgtctggaactgccaagttaaaggtaatcccttctgccggacggccattgatggtttgccctgaagtgccgggaagcatgattctaaaggcggtgatcttcgaccagtcggtcactgaattttccagctgccaagtcactgcactcagatccttcaacagatttgcctggtcctcagtggtgtagtaaacgttgactttccctgtccaatcggccggcagaacaaccggaccagtcaaaccggccgtataggttgaagttctcacatcagatgttgagacaccttcaattgaaccggcttgcggtaagaaatcaagtaagtcaagctgtgacaaactctcgtccgtattgtcggtaaaggtaatcttgacggtcgcctgcttaccggtttcaactgcaacggcgtggtgataatcacctttgtcgctttggctgaccaattgattgctctgcagtttggaatctttatccaaaatgtagtagttacctgatgtaatcaaaggtgtcttggtatcaatcaaaccggttgtcgagccgtccgcaattttttgggtcgttgacagcgtggcattattaatcgctgggactgagacaatataattctcagtatcgggaccaacattaatgaagttctggaaaaccatatcttttggcgcactcttatcaatgttgacaatcacccgagtcgcgccgttctttcctggtgttaagttggagatgtctgtccagacaatcttaagcacctgttgaccagaacctttaaagttatcaataactgagtattggttaccaaacggaatgacgccggactgttttgaggcggctgcatcgaacgtgacaccctttggcagaactgtgtaagtctcaaatggcgtgtctctggcaaccaggttaccgagcgaactcttgtccaacacaaacccaagggtcaattgatgagcaccagtctcaagaactgagcccgtggccttgccgtccaggaaaatcgcagaagtcacgtaacgactggcatttttatttggcgccgcaatttcgattgttgacgggttgaggaattgccagacaacccccggccaacctgatccttcatcgatggaggcttgctgttcggcctcgtcctttgccagccaacgccataagccttcaggggcattggcatccgacacccaatcctgcaaactcacataggttctggcattcgaccaactgaccttaggggtcatctgatgcacgatcgttccaggcgttgcgcctgatttgacgacagttttgaagtagacgccgccataggtgccatgcggtgcccaggatccggcaggtaagccaccatcttcaggagatttcaacagatcccgtttcaaaatcgttctttgagcaccgttcttatcggtaatggtgattgtatcattcttataagccttgtacgggtaatccggatattggtagatactttcccgactaatggtatccggattctttggaatgtcacccatgcccttcttatgcatatagagatacaattcgaccacattctttgtcggatcaagtccggctgccaataattgttggcgattgatatagatgtacccgacagaaccatcgttgccgccagtcgcaaagattgggttaccatctttatccttttcgacatctgaggtgatggttggcagattatcaaataaagtgtggtactggttctgtccctcaccctcatatttcacagccagtgacaagtatggattttccttgaagtacgtccattcgccgaccaccccagatggtgtcttggaatccttgatactatttgaaggcaggtagacaaagttgtggatgataaccgtctctaaatcctcacgcggatcaatcgactggtggagtgcataatagttaaagtcacgcagccgttcgttttggggaacttccggatctacatcattaaatagaaatagcggcagcaaagcatcatagaattccaagacagcgttcgcgtcggaataaacttgtgggtccggattgagcaaatccctatccgccaatgcgccaaaaccgtcttttgagccgtagtgaaccatcggtttccaactcccaccagtcacgttccaagtggttggatcatgcggcagtaccatggtagccgcgatcttgtccattagctgattgattggctgggcaccttggaaagtgaaaccgaccccgacatcagtcttaagccactggaagttggcggcatctttgttgaccttggcgatcacttggaacttcagggtttggtccttggcaatttgatccgccacgtcaccggccttaattgtccatttaagaacggttgccggagacccatctttcagttggccggtcgaaatttccggagctgagtcaatcaaaccgttttcagcggttcctttagtcatcccaacataggtctgctcgcccgccagatagtaataaacgttcacatcactacctggttccagcagtgcattctttggttgggcggttgggatcgtcacactgaagtcccaaacggcctgatcttcttgagccggattcttatattcgttaccataggaatctgtgtagacgttagccggggtgttggtcaccattgccgaatacgccatggccatcgtctgtgaggcactcagggtgacaggcgctgagatttcgtcagccttaaatgagatgcccatcgtgaccgtttggccattgatcacactgcccttttcggtgccataaacatagtgaaggtcttgagcgacaccactttctaatgtatcccaatggtaggtcaatgtcttagtggtggcatcataaaccggtgtcacgccggcaattgcgtactgggcgagatcgctggcatcaaaggagaggcctttgtcggttggtaagttaaccaccatttccgcgtttgtgtaaattgtccggatcccattggcatcaaaatgcagatcaaatacgccgttatcgccgacatcaactattttagcagtcggtgtaacctggatgccgggtaggatcggattagcagtcttttccggcgcactttccgctaccgctttctcgaatgccattgccttggcgtaagtttcatcccagactttcatttcttcttggtaactcttcaattcaatcagatactggtcatttaactcagccaaacgggtggttaaggtatcataagccccctgggcaacactatacctctcggccagtctgtcgtgaacggctttaacggcatcaaaatcagctttcaattgattgtaagcatcggtcttggcgataaagtcaattccggcatcggtaaattgtttttccaggtttgcaaaggtggtgtgagcttgttgatactgctgattgattttttgatattcagcgtcgattgctttgaattgatcggcagttgccttttgtttttgatcagcatccttgaactgcggctgcaggtcgtcgatttgcttttgagcggcgtcatattgggtcttaactgtctggtattccgcttcggtcttttcataatctgccttggtctgcagataatggtcctggatcgccttaaactgagcatcggtggaggttccctgtcctttctcatactgagctcgggcagcttcatacgcacttctggctgtttcatatttggcgagggcactgtcgtactcggtcttttgagccgtatgggtggtgaccgcagcttccaccttatccttggcagctcggtagtcagcggctgctttgtcattcaatgccttggtctgatcgtaatcctgtttcttttgatcgtaagcggttttggcagcttcatattcggccttagctttctcataggccgccttttcgctggaatactgggtttgattaacctgatatttttcaagcgcctggttatattcggccagtttgtccttatagacggttaattgttgatcataagcattcttggcctgatccagctggttggtaatgatgccgtagagtttcttgctggcgttatacacgttgaccgcttgatcatatgacaaatcttcggcaacggttggctccgtagttgcccgagctggcgtcggtgtggcttcagctgtcttagattccggtgcctgagtttctcctgccttggtgtcagctgccttggtttctgtttccttggttccggtttccttagtttctgctgctttatcagcggtggtatcgttggatgttgatggcttggcagctggctggttagtgtcagtctcagctgcttttgtcggctgggctgcttgaggcgtcgctgttgcctgagcaggctgttgggctgcctgtgatgtacctgggttggcagcttccgtctgaccggaattgaccggttgtgactgtggctcagttgttgactcggattgggcctttggagtctgcgcagtcgttgactgttgggtctcagctgctggcgccggttgagcagtttgtggtgctggcgtcgctgtttggtctgcagtcgtcgtagttgccgtagccggttgggctgctggtttctgtgtggcagctggagtggttgctgctgtcggtgcactcgtagttgtcttaaccagttcaggagttgcagtcgcactattacccgcatttccttgggcggtcggcgttgtgtctgcagatgcgtcggtgaccgtacttaactggctgccaacgccaaaggcagcgaccgttaagccggcaatcatccatcgcttgcccgctttatacatcttataatgtttagcagtaacatcctcctgattaataattcccctgtttgatgatttcattgttttttcctccaaaaatgacagtaaagttgtctgcttccccttagcaatattgacatcatttcttttacaatataattatatcaggcgtataaagataagtcataagtaatgacctaatcccggtatgacaagttttcatcatatttttccattactcatcaattatcgtaacgtgcaaaaaaagaacggttatgataaccataaccgttctgatattgaagtgcgttaattaattcctaattttttcagcggtcaatcccattgcattcaaggccacgatgatggttgacattgccattacagcagccccaacggcgggatccaaaatgatgccggcaaatgctaagataccagctgccagtgggatggcaataatgttgtaaccggctccccaccagaggttctgaaccatttttcggttggtaatcttggctaaatcaaggaagtgaagaatgtcactgggttctgatttaaccaggataacgtcggccgaatcaatcgccacgtcggtcccggcaccaattgccacgccaatgttggcttctgccagacttggcgcatcgttaacaccatcaccgaccataatgacgtgattgccctttgcctggtactcagagacaattttttgcttgtcattcggcagcaatccagcatgaaattcgtccaagccaagcagtccggcaacgtgttcggctgctttttgattatcaccggttaacatcactggcgtaatgccacgttgtttcaatccggcaatcagctctttggccccgttcttaatcgtatctccttcggcaaccatccctaaaacctgttggccttgaagcaggaaactaaccgagttgcctttggctgcccattgatcggcagtcgcgttatcaaatgaaatcccgttttttgtcagatagttaccgttgacgatcgtataattctggccgtcaatctcgcctgaaatgccgacaccagggatgttttgcgaattgttagcagcctgaaccttgatgcccttttcttcggcagcagcaataatagcctgtgccagcggatgggtagaattgctttcaagggctgccaatttacttaacagtgattgttcatcagtatttgctgctggtaccagggcgttgacagtgaatttaccttccgtcagcgttcccgtcttatccaacagcacatgactgacgtgttgactggcttcaatagcttgacgattccgtaccagcaaaccattttgcgcaccaatcgacgttgaacgagcgacaaccaatggaatagccactcccaaggcatgtggacaagcgatcacaaagactgtaaccattcgggttaaaccggtcgatagtccctggggtaaccaggcaaagaacgcgatgattcccactgataaggcggcatagaagagatacttggcaaccaaatcagcccgatcctcagcctttgatttcgactgttgggcctcctgaaccattttcatcacttgtgacaaatagccggattcaccggtcccggtgatttcaactgtcaacgttccgttattgttggtagcaccaccaatgactttgtcgccaacattcttgttaacagcggcagattcaccagtcaccaaggcttcattaacggttgattgaccattggtaatggtgccgtcagcaggaatactttcacctgagcgaacttgaaatgattgaccaacttgcagatctgatacttgaacatctttggtttccccattttcagttaccaaatgagcggtcttcggcaatagagcagccatcttttcaacggcatcgccggcacccatgaccgcgttcatttccaaccaatgacccaacagcataattagaatcaaggttgccagctcaaacgagaagtccatcacatgagtggcagtgtgcatcaagttattggcaatgaatgcataaatactgtaaaaatatgaaactgaaatacctaacgtaatcagggtcatcattgccggtgccttactcttaacttcagcccaggcgccctttagaaatggtgagccgccgtaaaaatatagtgccgtatcaaataaaagaatcgcaattccttcaatgagtggggcgtggaagttcaacacagcgacgtccaaccccatgatgggtgctaagagtaatacgggaatcgccaagaccactgagacccaaaacttttgtttcaggttacccatgtgcatcatttgaccgccatgcatcatcatgtcgccacccatatccatgccggacatgtccatatcgccatgatccatctgcatttttgaatgatccatttgactcatgtcatggtccatattcatcttagaatgatccatgctgctcatatcatggtccatattcatcttagaatgatccatgttgtccatatcatgatccatattcatctcatctttattatttgccattttaacgatcctcctcacatgtcattttccccggcagacagttgcattgaaccatttccggagcatccttggctttcccagccaatatctgctgcaattctgcaatgtcactttttgacaattcgcgtgtcttgatcacttgggcaattgtagagccggctcgcatcgcgcacatatgatcaaataaatcgtccgccgcagcggacattgattccttttcgccgacgaccggtttaaaggtaaatggtcgactatcgccgatttgttcaacagcgccctttttaatcaatcggtgcaagagtgtcttagttgttgagtcagaccagccctgtagttcgttcatcgcgtcgatcagctcacgactggttgtcgaccccattgtccaaattgcccgcataacttcccattcagaatcggtgatggtaacatttttagcatctatcattttgataacctcattttatttttcttttaaagtttacatttgtagctctcagcaactacagtttacatctgtagcctataagatgcaaccatttctgtttgaaaattctgtttcatccacaaaaaaggcgactgggacgtgtcccaatcaccgttcactcacattaaaaatgtttccccaaaatatccaaactgcgccgttgcccatccatttcggcaacatctggcaaatgtccccaaaccgtaaatccattgtggataaagagcttttggctcggcaggttatggctgaaaatgaaggcaaccagggcatccagcccgaggcgttccaattctccactgacaaagtcgattgcctgctgtcccaagccttggtgacgataatttgcgtcaatgtaaatactaatctcagcagtcttgtggtatgctggtcggccataaaatgattccaagccaacccacccggctatttgatcgtcaaccttcatgacccacaacggtcgggtttcatgattgaactcagcaaaccagttctcacgagaggcaaccgaaaccggctctaaatcggcggtagcaaggcgactgggaataatctcattatagatttcaacaattcgtggcagttcatcgtgcgttgcatattcaaatctgactgacattccatgacctcattttttgtattatccatctattttacgtcaggcaatcccgaggcgcaatatcacgccaacgtgtcacaaatgaacaaaagaggacgggatattactcgttatggaggctttcattgcaactaggattactactttgaaaacttgcggcggccattcaacgaagaaacgcagtcattccaaagtccggaataactgcgtttcttcgttaaatgctgggatcaaatcgcctgtaacttcaatttctttttgacttatttcatactggcagccatccgaattgcgacggcgggatcggttgcctgcagtcgatagacaacactgccagcctgccaagtaatcacttgagctgaactgccaacgttgaatttgacgactccttgggtattcggtgccggtaatgagtagctttcaaacatattgacacttgaaagtgctaatttcttcggcgtcgtgttattcacgggactgccatgaacactaatcgaccagttgccctcgttccaagaaatgtattgctgaccggctcctgattgagtatgaccaacaatcccgtgaccaaggtcaactttcgggagccctttaatttctgaagcagccgtataatcgacatgactttgagcttccgaagctgaagagtagctgcgtttggctaagaccgcatacggcttctcagctttcaaactactgtcgttgagcgcgagtgcatcattaccaacgctgtagtatatggtactgttggtagaattcccattatatctgatatgaacgttcttggatgaatcgttcagtcccgaattttgtggcaataacgtatctgacaacttacttgacagatccttagtcagcgatgagaaatcgtacgattgaccgtctgattgagcgttgctgtcagaagaagctgttgaggcactttgtccgctggtggtatcagagctggtggtcgaactgcttgagttctgcatatcggtctttgattcattattagaactttgtttaccggaattgccattactgcagccgacaagaaccagactcagtaataacactccacctaatttatagagcttcatcgtttccctccaaattgtttgcgtgaattattgtacgaaattcttattggcagttaagtagcggccgtcggcagtttcaaaatagtatgaaccactgtctcgtttgtgaattaccgtcacgttaactttggttcccggctgaactttaacaacccggttggctttcttaaagctggttgaatcatacaggtacagtttctgagtggtcgtgacgctgctgacaacgtcggtgaaataagttggttgcgcagtatcagctgactgagctccgccgatccaccaagtaattggcttgctggaattcagaattgtgctggcgtcaactgattctttcaatgcgggaacgtacttcttattagtgtactgccacaaatcggtttgaatggttggccgtgaagaataattggcgatccattgggcatcaaaattctttctggcggtgttggcatgagccgttgcaaaggactggtaggaataaaagattaatttcttaccggttaatgaacgcatttggtcgtaccaggccttaacagcagcattgcttgaacctgaagtcacgtcattttcttcgtagtccaaaacgtagaatttggcgttcttgttggaattttgatagaagacattggcttcattacgggcactggccgcactggtgaaggtggcgtaatcatattcaccaaatggaatgccatattggacgtataaattggtgttattggtcgcgtacttgtcttgatagttagcgccatattgccggcggttaataatgaaggaaacctgactcttcaagtttgaaactttcgaagccgttaatttcccctgccactctgaaatatctggaatgacagttgtggcagccgatgccttaactgccccaaaaatcgaaaccgataagataacggtcaaaatcgataggatgatcgcccgtccctttttcctcaatgaactcatttaaaaccactccgcatttatttatttgcttacgccaaattcaattagctaaacagttgtcgtcaatttctctaccaacatatgacagaatgggtttgagcacaagaaccccagcagtaagcaaaaagaatattacagagctgagtcgcgtcataaagcctcagcgattacttcttttcaagaatgttataaatgtgtaacataactgaaaaaatatcactccgacaaccgtcaatgaataaatcggaatgcgtagccaaatcggcatcagccgataacaaaagggttccatcagctcgatggaaccctcaagataattgaaaaattatttaacagctcgtgaaactgcctcattaacgtcagctttttcagcttgaactaactgaacccgactatcaatgacactaatatccatcttgatttcgcgagtcaaaccaggcgttgggatctttggttcaaagaattctttgaattcagccaaccgttgcggtgtgtggaagatacctgaaataacggtaatgtaggtggcaaattccatatccccaccaaccgtatcttcgagccattgccagtcttttcgaatccagtcccaagcagcttgttgaccgtcatcattggcgaggaccccacggaaccaggcccgcaagtcttgcggtttgatggtgtcggcattctcaaattgaccaaccaacttggcaatcaaatcggggtcagtggtactcgtcaaagtagcgcaaatgtcttgcttgtaactggcatcggcagtttgccggtaagcagccaataatttgtcaaataaggcttgactgccaaagttcttaacctcatttcgaaggacaaacacccgaatatcagcagataagccggccagactgccctcgttttgtttaaacaacgtatgagctgcagccatggcatcagcgttttcagcatacaatgaagcacttaaaatgtacggccgagtcaattggtcatcatttgactcaccagccttaggggcaaagcccagtcgatcaagttgggcagcactcagtcgatcgaagaattgcttgagtgctttttcttcattagatttaggagtcacaaatttcttcaaattgttggcaacccgatacattgccgcattgacaatgttggaatggctgtccgcaaattttggcagcaacggcacaatattagcataggaattttgacgaccatcagctaacaaacggaggtcttggagaatctggagctgagaaatcgcgtccagatccgccacatgatcaagaatatctgccattgaggtttcatcatattgaataatgaaatgtgaattgttaccaacattcaagaagaatggtttgccgttttcttgacgcaactgttgataatcaccgactgtgagtgttttatcagccatgatttcaggcacggcgtcgtaattgctgttaagcggaatctgccacttgcggtcgacatccttgccgtcaccaatgaagaattgttgttgtgacaaggtcaactggccgttttggactttggccgtcacaactggatatccaggctgctccagccacgagttcatgatggcacccacgttcatgccagaggcgtcgcccaaagccgaccataaatcggcaccggtagcgttatggaacttgtgggcggcaaaataattcttcaagccttcccgcaaggccttgtcgccaaccaaagctcgggccattactaacattctggcacccttggcatacacgatggccgagtcaaaaattgaatcgatctcggccgggttttcaacttggacgtgaaccgactgaacaccatcggtagcgtctcgttggagagcagccggggcttcagaggtctggaagacttcccaaatgtgccaatcaggctcgatcgcatcgattgcaacgtattccatcatgttggcaaaactttcgttcaaccacaggtcgtcccaccacttcatcgtcaccagatcaccaaaccactgatgagccaattcgtgggcgatcacggtggcaaccagctgtttcatttcaaatgaggtgttcttgggatccaagagcaggtaagcttcacggtacgttaccaagccccagttctccatggcaccggcagagaagtctggaagagccagctgccatgagtgtggcaatgggtacggtgtttggtagaagtcttcataaaattcaatcgaccgtttggcgatatccaaggcaaaatcaagctcatcggccttgtgcgccttggtagcaaacacaccaactttaacaccgctcttggtggtcgttttcttactctgcatctcaccaaatccaaaggcgatcagataagtcgacatcctcatggtcgtatcaaaatagtgaacaccattttctgtgcggacttccggcatgttgctgatgatcgtctcgccggcatgctcgtcaaacttaatggccaaatcaaaggtggctttggcttcgggttcatcgacacatggaaaggcctgacgggcagcggtggtctcaaactgggttccgatcagctgcttcttaacgccatcaacttcgtaataagatggataaatgcccatcatcgtgtcagtcaatttggcactaaattgaatggccaaggtcacaaccccagttgtcggcaaatcaatattgattgcttcctgatcgtcgtccttactaaatgaaacggctttgccgtcagcttggaccgattcaatattgagaaacttttggtgaatcgaaatcgcggtcgtcatcgcgtcacctgtaatcgtagaagtcccggaaaattccttggtatcccggttgatgtccagatagatattgtaatgacttggttgaaatttttcgtagaaatgggttaattgttctgccatgagttgcctccttgaaaatttgttaattatattatacgactctggcaacgcttatgcggctcgaatggcaaaacattgatttttagctgaacatccgcgtgaccagtcgatcttgaatccgatcgggaatcaatttcaacaatttggccgtcacttgttcttgaaatcttatctgatagcgtaactttggtttgcgcgtcatggccgctttgacaatcactggtgccacatcgttggtagttgcccgactgtcctttaatgtcttcgctaaacgctcggccacccgccggtagggagaatggattggagtagccgccaacagtttatccacggcaattttctgccatccggttgctgtattgcctggttcaaccacaaccacatcaactccaaaaggtttaacttccaaccgcaaaatatcagacatggtttccaatgcgtgtttggaaatatgataccagccgcccagttgggtatacatcaaacccgccagagaagaaatattaatgatgcggccggacttttgggttctcatcgtcggtaagaccaactgaattaatcgaaccaacccgaataaattgacgtccatttggtgtttggcttcctcgattgtcacttcttccagcgcgccaaatgaaccgtagcctgcagaattaaccaacacgtcaactctgccatatgaatccaagacaaaggctacaaaggctttcaggcttgactctttgttgacatccaattcatgaacctttccgccgagttcagtcagcaccttcatttgttcaacatgtcgcgcaccgccaaccacgtaatagccctgcttcaaaagcagtttggcagcagccaggccaatcccggacgacgcgcccgtcacaatcgcaacttttttcatcaaaaagacctccgtttcataagcgataactctatcgttaatgcttactgtgtataatagcgatagtcttatcgtttgtcaaggttgcaatgccggcactttccaatataatgaagatatgaaaattaaaacgacagaacaatataatcggattattcagggtgcgaccgccattttactgaccgaggggttggccgctttttcgaccactaaagtcgccaaacacattcaaatggcacagtcgaatatctatgtgtacttcaaaaataaagatgatttgctggtgtcggtctttcggtaccaccagaaaaagtacattcaatttttagtcgatcgcattgatctctccctgccacccacggatgcgcttaaaaatttggtttcaacactcgatgaattccatagcagcgacaaagaatcactcgatgttatttggtcaattcggcagagcaccactttacggcaactgattccaaaagtcagcgacgatcaaatttttattgccatttttcagtggctgaaggatttgcagcatcaaggaactgtccgccaactaccgctcatgtatctcaccaatttggtcttttccgccattatcgattactttcagttaattgatagtaaggaaatgtcaccaaacgagctggctatcgaggaaattgtcccacccttatcagcattactctttgtctgagagaggcttgtcggccggcctgattactcgtatacttaaattctgacgtgctggtgattgaacaatcagcaccaattgatgcgaaattcattattctagggggaatcgtcatccaaaacacaaaatctcagcgttgggtcggcctgatctcgggactgattttaaacgcctttggcaatgcgctaaccatttcagcgaacattggaagtgccgtttggactgcttctgctgttaactacagtcactggttcaatttgaatgttggcattatcctgttttttatcggttttttgaacacggtcaccaaccaagtcctgctgcgacatccggattggccacggttcgttggcgaaatcctctatgtctgcttttttagttatttcgtgaatatctttgcccaactttttgaccaaattgggatcggccagttaccaattgtgattcggggcatcctatcatgtttggggattatcttcttctgtacggccatctcactgtatcagcgggcaaatattctcatgcatccaaatgatgataccaccaatattttgcggtttatgtatttgaaaaaaagtgccgtggctgcccagctggtcgattttgttccgccaattatcgcgatggtgatttcctttgcggtgacccacaatttgtatgccgtcaacgtcggaacgatcttttcgattcttttcaatggcttgattattcaaaccgctgatcgatgggtttggccgactttgaagcataattttaaaactttggggaatgattagtatcgtcaccaatgttctaccccttcaattgaatggtcgctacagccaaatgaaatcataaattgtcggtaaatccagttgcatcttcccgttaatatggtaaattaaaactaaataagtcagacttaatcgctatttagaaaggagcttggacaatgatctttatgttactcatgctatttttagtggggtatttggttctaaatgtcagttggctgttcattaaggcctcggcttggctgataatactcgcaattgggtttctgatcctgtccaaactgctggtagttgggctgatagtcgccgccgtttatggcgtttatctgctttttcaacgctcacaaattcagccatacaagaatcgccactaatccaattatcttgaaaatgttttacataaagagaaataaaatcattcaattgatcttatttctctttatttttagataattttacgattttttaaactttgtaaccgttttgatagaaaatttctttcataaggtatagtattacattattacttaaaattgaggagagttttgattatgaatttacttattgcgttacttcccgcccttggttgggggttaatgccactaataaccggaaaagtcggcggatcgccagccaaccaaatctttggaattggtgccgggacgaccatcatcggattgattgtcttcttggtgacccgaccggccgtcaacatgactgcgtttctttttgcaatcgtttgtggtgctttgtggacgattggtcaaatcggccaattcatttccttcaaacgaatcggcgtgtccaacacctacccattatccacggtgtttcagttagttggtaactcgattcttggcgtattgatctttggtgactggcagggaactcaatccaaaatcattggcttcatcgccttgattattgtgattgccggagcgttgttaacgtctgtcagtgacgaaaaaggcggcaaaattacctttaaggacgccacgttcttactttgcaccaccgttggttactggatctattcgtcattccctaacattccaatcattaaggcacaaagcggcacttccgttttcctgccagaaatgatgggcattttaattggtgccgttattttcggcttgttcaccgaccgtcaatcatttaaacaaaaagaacaatacctcaacatcatcgccggattactttggggagtcgctgcgctttcctacatttactcggctcaggcaaacggaaacacctccgcattcatctggacgcaattaagtgtcatcattgccacttttggcggaattacaattctgcacgaacacaagagtcgccgggaaatgatctttaccattgccggcatcctgttgattgttgttggtagtgttgccacctcgtttgcataattaatagatcagttgaagttgaaaagagagtgggacttaaggcgttttgatcccagaatttaagcgcacagatcgattattcctggttttggaatgattgatctgtgcgcttaaatggccgggatcagccgattgccatgtaggctaggcaagcatgctggccgtcgtcgcacgtttttgataaataatatgggatcacaagaaatagaggccgaggcaaaagcgtatacttttgtctcagcctcttttctatttggatttaaggttgtccaatcccactcttggtaaaatcattgagcagacgggcggtgacccgcttaaagaagtccttcatgaataggccgacgatcaagcccccaatcagcatgcagatcagaacaaagaagtccaagaccacggtaccaacattgggtccaccaacggcctcgcggaagccactgacactgtatgaaaatgggaaaatcggctgaatgattctcatgaacaacggattcaactgaatcgggtagattgccccacttccggctaattggaaagcgaccatcatcactgccaacgcctttcctaagttaccaaacaccgacgccattgtataaacgattaccgagaacgtcagtgatgacaccacgccgatcatcaccattaggaacaaactttccacgtgaaccctgagaataaagacagttgaaaggacaatcaccatcgtttgaatcatcgacaaggtgttaaacagcagcatcttgccgatatattcttcacgcggccgcaaatttttgaaacgatgatatttgggcgccgaggtgtgcagaactgcgaccagcatcgcacaccctacccaaatcgatagggccatgtaagttggtgcaaacgcctcaccaaatgaactgacccgataaatgttctcatttttgacgttaaatggttgggccagtgcgttgcccatcaacttgggattgttctggaggatgctgataatgttggcaatattatcgtctgaagtcaatttcaactgattacttgcctgcaaaatcacgcccttatactggagcagttggttctccaagttgccggtggtgtcactgaccagttgattgcctgaaataatcgtatccaacgacttttcgttcaagctgcgaatgtcattaacattgttcaagacatccgaagcgtgattgctggctgacagcaggttgcgttgaatcccgttcaattctgatttaacgttgcgattataactcgccagtgaatgattcaggccgctggcaactgaataggaatgactggcaattcgctgctgcaggccggtattggccgtactgcctgaactaagcgcccgctgtagttgggtgacttgctgagactgggcatccaggagattcttgacgtcattgagttggctgattaatcgactcaccccactcaaccgctgcgattgattaatcgtctgcagataagcaattaatggcgtaatctgccctctcagtaacttaatctgcgacaaaatttgactggccaaaccagtggcctgattacggccggccgcagaagtctgcttgttcaactgattggtgagggaccgcagtcgtgcggcgtcagtttgaatcccattcaagctggtttgaacgttgccaaacgattggttaacgccctgattcacactccgaatcaactgctggttcgacgagccaatcgcttggttaatattgatatcctgagatgctgaaatcaccggcttcagttcagaaaagaccatagccagcccgctggaggcttcactgatatctcctaaggtattggttgccagttccatactgtctccaagattgataatcaggtcctttaaattgagaatctcggattcgttgtcaccagcctttttaccagccacattcaaataggtaaaaatggtgctgttaacttggtatacgaattgttttttgatcgtgttcaacagcgtctttgaggcggcttcggtaattttgtaactcattggactggccttggtgtcagcgatatagtcgatgtgggccttcttcggattagcagtcacaatactgcccaaatcagccgaaaaggtcttgggaattttgatttcggcgtaatactttccagcgcgaactttcttttgggcagtctttgaatcaacaaaccgccagccgatctgattattgtgttttaactgggctatgatttgcttgcccaaattcatctgtttgccttgaactgttgtgccttgatcgttattaacgacggcaaccggaatcttttgaacctcgtgggaagtatacggattccaaattgctttgacattcaccaaagtatagagacaaggcaaaatacaaagcgcgctaatcgtcagcaacgctgctttgtacttaaaaattgccttgaggtcccgttggtaaatcagtttgatatttttaaacattgttccatccctcaaatttccttgctacttgtttctgtcgaaaaatgcattatactgataataacgcgtatgcgaatgattaacaatggtaactatagttaacaacattaacctacttttatgagggagctataatattatgaaacattcagttattaaatggatactatcactgaccatcttaggggcgctatttgctattcaaccaaccaccgcgtcagcgaaaaccacagcggccaaggttaccagcacccagactttaaccaaggcaccctaccgtgcagtcagtggttatctgtacagttcggccaaattaaccaagaaggtccataacgccgacaattatcctttaaccaccttttacgcttctaaatcggcgaatatccaacgggctaacggcaacaaggcagtctattactatgtcaagaatggtaacggtaaggtcgccggttggatctggcgcggtcatctggtaagaatgatcaatgtgactcgtcagcgacaacaactgaatcagattatcggcttgattgatacgttgtccaccaataataaggaccagctgatttcaattctcaacctgatgaatcatcaaagcaccctgcccgacttgctaacccagttaaataactggatcgaatcaattcaaaatgatccagatattgccaagctcaatcaaatctttgaaatgatcaaatccgatggtcaaacactcaattacttgttcagtgagggaatcaacaagctatatcccaagatcgttgtcattcataacctgaacaaccgcgtgtttgcgctcgcccaaggactgcttgatcgaatcaattaaaaggacccatttatgcgaacaatattaaccttactcaaacgtgacttacacaatatatttcatagccggccggtgtggataaccctgctggctttttgtctgattccggccatttatgcggtccccaacatcatggtctcctgggacccgtattccaaggccaataccagtcgactgccgatcgctgtggtgaatgacgatgagggcagcacggtcaatggcaagcagctgaatgtcggcaaacaaatcgtcggcgaactcaaacaaaaccacgccatcaactggatcatgaccaatgactggcagggaaacaatggcttggatgaaggaaagtattactcgctcattgaaattcccaatgacttttccagcaagttggccacactagtttccaccaatcctgagaagcccaatattatttataagtccaatgaaaagttaaacccggccgcaaccaaaattaccggccaggctgtcgacacgttaaccgagcaggtgcgggacagtttcatcaaaatcagtactaaagccgccttaaaagaaatgaatgccgccggagccaagattaacacccacaaaccggagattctccaaattcgttcctcactattggatgccatcaacacggtgaagaaaaccaacggctatttggataaagctaacaaagactcagacaatgtcgagcaatacctgaagacggtccagggagacatcccgaaaatctccagtcagataaccgatctgcaaaatgttgtcaatcatggccgcaacttaaccaaggccaccaagcaatctctcagttctgcgcaaaatgatttatcaaacggattaaatgaccttcagtcagataataaccgcatcaactcattggtcgatgacatgcagactggcggacacgcttcaagtaagtcgctgttaaacagtgaaattaatcaactggaaacgctgaatgagtcgacacttaccggcatcaataatgccctgcgaatcgccgatgtgttgaacaacttactgccaaacaatcagacgacttcgctgatcagaagcctcagcaatgccaaacaacacgtccatgagcagcagcgcaatttaaccagcctgaaaaacgctaaccaagacaatcgatcgcaaaaatcaattaatcaactgattaagcagctcgcaaaaacgaccgatgctttgggtaatagtctgactgacgcgggatccacgttcaccaacacggttagccaggtgattgacgacctcaatgataccttggacacccagttgaacggcaatgatgaagtgctgtcatccttaagaaccctgttaccacagctaaatgcgttaacttcggctggaaaagcaatcagtaaaatctccgtttcccaggtcaatcgaattaaacatcgcttaaacggcattgaagataaactgaacgacttaaatgaccaaaccaaattcatcaacgaaaagaatttgaataaaatcattaacttattgggtgaaaatcccaagatttcaaatttgctggcatccccaattaccttgaaacaaaagcagctgtataacatgggcctcttcggctacggcatggcgcccttttacacagtcttatccatgtgggtgggcgtcttgctcctcaccacgattgtctcatggaaatacctgattccagaagacaaacggtttccaaaagccaaccggattcaacaatacgttggtaaaggccttctgtatctaattctgtcatttacccaaaccaccttcatcatgcttggtgaactggtcatcattggactgcggccacgaagcttgttggcaatgttggcaactgcctatctggcaacgaccgttttcaccatcatcatgttcacgttggtctatatgttcggtaatatcggcaaagtctttagtgtcttgatgatgattgctcaactatttggaaccggtggtgtgtatccacttgaactgattccttcccatttggcaagcttggcaccgttcctgccatttacctacgtcatccaagccttcagagaggccattgctgggccgattccaagcgtctattggcacgcaatgctgattttggcggcgtttggcggattcttcctcctaatggcgccattgtggcgggtgttcgtcaaaccactttcgaagatggaaaatgggttccataagtcccagttgtaaaattaaataagtgtttcaaaaagggcccacaaaatcagcaaatggttttgtgggccctttttgtaccaatttacacgcctaaaggattctgcgcatatccaacccccgggcactgcggatgttttcaatcacaattaacgcattcttatcttcactttcgatgatcggtaccaatttggtgacccgccgaggaccagcaatcatgtacaacatgtgctgatcagcatcactataatagccagtgccattaaaaatcgtcatttcctgatttaattctttggaaatggtcaccgcaatttgccggtactttggtgaaaccaccagaacggcctttttagcaccaatattcgccaaaaactgattagtgaacacggagtaaacgtagaggtagatcaccgttaaaacggtattggtgaacccaataatcatgataaacggaaccacaatgaacaggtcgaatatcaaactcccggtacccagtgagatgccaaaaaaataattgagaatcttaccaataatcgtatctccagcaattgtgccgttgaagcggaaaatcaaaccaattgagatcccggttaaggcgccggctaacagcgtcggcacaatcaattcatgggtatgatatgtataaaacaccggaattttgaggaacaccgtcatccaggcaattgcccaaattgtcagataagtggttttcttttcaaacaacctgtagccaatcacaattaaaacagcattgataaggaggtttgacagatatgacggcaccccaaaagcatagtacaacagtgctgtgattcccatcgctccaccttcaccaaggtgagaaggcaacaacagatagttataggtcatcgaatagatgaacgcccctactgctaccccaattaattcggtcgatttaatatttagttttcgccaataattccaaattgaattcatttcgcacctcaatcttgatatgtgattttcattctaccattaatggggtgcggttggcagtccccctttcattgtttaggctgaaatcatgaaaatcacagaaaatataaaaagtccaaaatcaaaatctgattttggactttcataatatcaattaatttgttattcccattcaatcgttgccggtggcttgctcgtaatgtcatacactacgcggttaatgccatcaacttcgtttacgatccgagtggagacattttgcagaacatcccatggaatccgtgcaaagtcagcggtcattccgtcaacagagttcactgctcggatggcaacggtgtaatcgtaagttcgaccatcacccatgacaccaacactcttaaagcctggtaaaacggtgaagtattgccagatatcgcggtctaaaccagctttagcaatctcatcccgcaggacccaatcgctatcacgaacgatcttcagcttttctggagtcacttcaccaagcactcgaatgccgagacctggtcctgggaacggctggcgccaaacaagcgtttctggcattcccaatttttcaccaattgcccgggcttcatccttgaacaacgtgttcaaaggttcgatcagcttaaacttcatgtcttctggcaggccgccaacgttatggtgagacttgattgtctgagcagtatcagttccactctcaaccacgtcagtgtacaacgtgccttgggccaagaaatcaatgccgtgaagcttgctggcctcatcgttaaacacttggatgaactcattaccaataatcttgcgtttcttttcaggatctgtgacacccttcaacttggaaaggaagcggtcctgagcgtccactttgataatgttcaagccgaatttgccgaccaaactatccatgacctggtcagcttcgttcttgcgcaacaagccgtggtcaacaaaaatacttgtcagttgcttaccaattgctttgtgcaagagaacaccaacaacacttgaatcaactccaccagagagacccagcagcactttcttgtcgccaacttcttctctgatatgttgaatctgcagatcaatgaagtcatccattgaccagttggcctctgcatggcagacgttgaaagcaaagttcttcaagatgtcgttaccatacttggtatttctaacttcagcatggaactgaatcccatacaaattacgctcaacatcctgcatagcagaaattgggcagtcacgactggtggcaactgtctcaaagccttcaggaacttcattaaccaagtccccgtgactcatccagactggctgctcacgtggggttcccttgaagagaactgcatcatcagaagtaatctgaatatcagcatgaccgtactcggaattggaagccttctcgacttcaccattaagggtatatgccataatctgcatgccataacaaattcccaagattggaattcccagcttgaagatgtctggatcaaccttcaaagcgccatcttcgtacacactatttggacccccggagaaaataattcccttggggttcatgtctttgatctgttttgcggacaatgcgtgggacttaagctcagaatatacgcctaagtcacggatccgtcttgtaatcagttggttatactgactaccgaaatccagcactaaaatcttatcgaagcttgataagtcaacgtttgccaaatcatacaccctttcaaagttcttacataaataataaacgattcacctaggtttggtcaacattattctgaaaatccaaacattaatattttctcaggtacaaccgatcgatcaaatgattgtccgtcttgtgcattatcatatcagctcgcgagcgagttggcaggatatttgctcggaggttgggcaggtcgatggtgtcccacactctgcgggccatatcaaaggcctcctcacgatccccttgcgcgtaatcatagtaatagttgtcgggatcttggaaggccgtgtccatcaagcggccgaatcgttccaagtaccacttctcaatcaaatggacgtcagcatccatataaatcgaaaagtcggtgaagtcgctgatataaatctgctcgttgctgggtaactgcaacgtattgattccttcaatgatcagcacgtccgggcgatcgaccaactcaaagcggttgggaatgatgtcataactttgatgggaatacaccggtgatttggtgaccggaactcccgacttgacctcgttcaaaaatgcgattaacttgcgcatatcatagctctcaggaaaccccttcttgtcataaatcccgcgttgtttcagctcggcattcgaatagagaaacccatcggtcgtaatcaacttaatcgtctcgccggtgaagtaattggaaagcagttcctcaagcacccgggccgtggttgattttccaaccgcgacacttccggagattccaataataaacggcacggttcgcacctttttgcgcaggaaccgggccttggtggtctgccattgatcaaagttgtttttctgcaggcgaatcatgtgcaccaacggtttgtaaatgtcagcaacgtcctgcaacgagatttggtcgttgaaggccttaatgtgccgcagttcgttagacgtcaacggcaaatcgacttcattgtcattattaaaatgtttccactcatctttggtgaatgaataatagtttattaaatcatccatgcattttctccgcttattctttactcaaccaaataagtataacattttcagactgccccgagaaccggagatatgttttcacttgaagtccgccagccgacataaattaggtaataaaaaatcggaccatttcgatccgactcatgcttaatttaactcatattcatcttggggcaccgtctcaaaaattggtgacaacgatttgactgccacaaccgtcaatcggtgcattgcccgggtacaaatcgtatagaccagttggcgatcgctttcgtccgggtagcaggccttcgaagcatcccacataatcacactgtcgaattccaaccctttggcaaggtatgaaggcacgacaatgatgcccttcaccaaacgctgattttcagttcgaatcaatgttgacttgacacccagttcagcgagtttgccactcagctcttgacattctttcagtgtcttgccaatgatggccgtcgtttcatggtcggccaagttcaactcggactgctgtttaacctgctcaactgcagcatcaaccccgtccttgacgtaaatgtgcggcaggtcgccttgacggttgaatggaataatattctcaccattggtcaacaggtgcttggtaaagttggtaatctgttctgttgatcggtacgacttggtcaattgaaccacgcgggtcttatcctcagggaacatgctgccaagttcgcccaacaatttacggctgttttcatgggtgaaaatcgcctggttcaaatcacccagcagcgtgaatcgcgcccttgggaaactgaattttaagaaggccaattgaaaggctaaataatcctgcacctcatcaataaagagataacgaatatctttatcgccacgtttaccagtcatcaagtcgtacaagtaaatgtacgatgacgcatcagctaatgacaatctgcccttcttcaaacggccgacggtggctttgatctcttcggcccacaactcgttagaaatgccaaaatcagccagattgaggatctttggcatctctttaagcatatgaacaaactggttattgatactcaaccagtggttgcgagaaatttgccgctggacttttctaaatgacttgataacaatccgtcgggccaggaacttgaattccttatcggcattgagaatttcttcttcaccttcggcatggaactgttgaatttcttctttagataggttttgaacggcatcttcaacccactttttccgcatttcgacgtgaatcttgcggttaagaatcttcatcaattcttccttggttgactccagtcggttgcggagattgtagttctcattgaaaccataatagatttcagcgatctttttttttggaatcagaatgtcaccgttaaacatcaggtttctaaagcgcatgtcttccttattcaaatggttagcgtaagcactgactgctcggaaataatccaagctgcctttgacgtcggtcagcttctgggcagtcttgtccagctgctcagtaaagcgctcagacaaggtttcaacttggacactcggcaaacgatgtgaactatattgatagaacgtcatctgaaccatattctgctcgcccagttcagggagcacctggttaatataatcattaaacagttggttcggtgaaaataaaataatttggccggaatggaggttgccgcggtattggtagagaagaaaagcaactcgctgcaacacagcggccgtctttccggaacccgctgagccttggacaaacagtaaatcagaatcggtatcccgaataatctggttctgttctttttgaatggtggtcacgatgctcttcatcttggtgtccgaacggttgctcaaggcatccaggagcatctggtcacccacgacttcttcggtatcgaaaactgttttgatctttgaattttcaatttggaattggcgctttaatttgacatcaacggtctgttcaccgtcgggggtcatgtaactgacatcgccgatcccaccgttgtaatagatactggagatcggtgcccgccagtcatagatcaggtagtggtcgggccggtcggtaaacgatgccatgccaatatagatggtctcgtctcgtttttcgtccccttcacgaaagtcaatccgtgcgaaataggggttctgctcaagcttgttgagcgtcccaagttctcgggcggcatgttcctggcgattttcacgttcagaaagcatttgctgttgctgccgaatggacatggcagtttccatcatcccgctgtacgtttcagttttgagccgaacatcattgttgaaattgcgattgatatctttaacatcccgcttggtcgccttaatcttttgctcaaggtccttttgggaaatgtggatttcatcaatgacgtggtccaaatggtgttgttcttgtgttttgatattatctgccattatttaccccctataacttgacttaatagtttagcataaaaacggtaccaattcaaaagacattatcgtttctggcttaacggtaacttaaatggcctgacattgttaattggtatacttgccattcgaccgatacactatggtataattgagatgttttaaataattgtatacttaggaggacacatatgacgatctcactatattttgttagacatggtcaaacatacttaaacaaataccaccgtatccaaggagtgatcgactcacccttaaccgacaagggaattgccgacgcagtggcagctggcaagcggctttcacaaatcaaattcgatgcggcgtacagcagtgatacttcccgggcaatcaagaccggccaattgatcttgaaagaaaacccggcagcaatcaaggatccagtgccaaccggtgcctttcgtgaactgaactttggctactacgaaggtgaagatgacgtcaaaacctggcatacaattggcggccccatcgggatcaactcgtttcatggcttaattgccgaatttggtattgaaaaggccgaggacatgattgcggcggctgatccatacaaagatgccgaaagcggcggaacgttctggaaacggcttaaacttgccattgatcaggtagtggccgatgcccaagacggtgacaagattttgttggccacccatggcaccctcatccgaaatgtggttgccaaattcagtgacattccagtcgatgtgtcaaccaaaaacggtagtgtcactaaggtcaactgggacggcaagagctattcggttgagtactttaataatgtgagtgaagatttatagaagaaacccaaacagccgcgagcaaaattctgctcacggctgttttatattatttaactggattgaatcagtctcctcagctgtcaaaccagcccctattgttcgttgaaccgcttcttcaatttggcctcgctaaacgccatcaaactatccgggtcaacttgatatttgtcgcaaagaatcaagacttgatccatcacatcggccaattcttcatgcagattttcattgcgtttctccctggtctcatgttcacctggatgatcgcggccgatttcaattgctcggatcgcccgggacaattcaccgacttcttcagttaaaaagttcaggcgaatgaacgaggagtatttgtaccaatctcgtcgcttgtaaaaatcgaccagccaatcttgatgctgctttaacgtcattaatcatcactccattgtcttatgtctacttaaaatcatacacctcaatgcttggttttccaggtcaacaaactaatggccgtacaaacaacactcggaatcacgaagttcggtaccatcaagtcggcaatcgtctcagaactagccaacgcccagccaaaaagtgaaatggcaaaaatcaattcaagcaccaaccaagttgctatgtacgggtgttcagtgaataatttatcaatcatctcctaatcttagtaaaccacataaatttgaagaaaatatgaccattctacccacctgtggtctgttataataagggcaacagggggttcacatcatgaaaaaaattttgccagccgcaatcatcggactcgccggtattttgcttctcacaggctgtgggaacaaaaaagccgacatgcaggataaaacgacggccaatcccaatgcaaccaaattaaatcacttgttgtcaccggcaaccgccaaggtcccggaagattcgcagacaacgaccgataaccagctttattcccaattttataagagcaagggtcagtggtactggaaactatcttccaaacaagccgggaccattgataacagtaaaatcaaatcacttagcgccactgaccaaaaagatgtttataatttctccatggtcagcaaccagcgcaagtcttacacccttaaattcaattggattaacggcggccaccaagcttatactgtcaatgccagctaccatcatgtcaacagcaatttcatcttggcagacgccaatactgacactgattggcagacaggtgccccacaggccgtccagggaacttgggcaaccgacttcgtcaacaactcaggtagcgacgcgcaaaagctgccttataccaaacaatttttgaacattaccagctccgctatcagcagcttcaccaatgaatatgacaccaaccaccggctttacaactcagacacgattgctaaagccagcaatgtttcctacaagcaaaccggcgatgacacttacgtcttaaaagcctacggcaatgaccaaacgccaatcgtttataacatcagtgtccaaagtaacaatcaaattgaagtgaatgggctgacctcgggcagtttgaccatgagcaaatcagccactactgaaccaaccactggttcacagacggccagttcgcagtccccatcaacgaccagcggctcgactgccaatcaagcagcgacaaccaccaaccacctcaccgatcaacaggtggtcaactggatttggccttacgtaaaagccaagtatccaaatatggccgtcgattcaaccgactttacctacatgccacagatgagaaacggtcaactgtacgtcaacgttttggagaatcacaactctcaagcatttaagaagagtggcgttgataccggcactaatccacaagtcgccagctttagggtcaccgccagcggtgctttggaacagatggacgcaacgacaggtgactgggcagttgtttccaatagctatggcggatagcaatgaccatctaatttagttttaaaaattcaaaaagtacccactcctcaatcgggaatgggtacttttttgtcggaccagacgcactgttaatgcgtgctggctattttaccttgataatccttatcaatatgttcgtaatgatcaactttgtatttcagcttatcgtaggatgcctgcattttagccaggcgttcactgacggatgccagctgttcgttcaagagatctttgcgtgcctgaacagtctgcttgccctgcttaaacagagaaatatagtcaatcaaatattcaacactgacaccggcgtctcgcatacacatcgcaaaagagacccagttcagatcttcttgatcatagtttcgataaccggcttgatccctggaaacagcgggaatcgcaccaacccgctcccagtatcggagcgtgtcggcggcaacactaaattttttagaaacttcgttaattttcatcagctcacctcattactaactgatgataaaccttgaagtgcactttaagacaagcatttcctacagtttgataacgagcgagtcgttaaccagttaatcctcgttaatcggcggcagctttttaatcaattttgccggaacgccgccaaccattgcgttgtctggaacatctttggtgaccactgcgccgccggcaatcacaacgttgctgccaatggtgacgccgggcataatcgatgccttaccaccaatccaaacatcgttgccaatcttgaccgggaacccctgagccatatactttcgtcgctgaagggcatcaaccgggtgattgaccgtataaataccgacgttggggccgatcatgacattatgccccattgtgactggtgcgatatccaagatggtgagattatagttactcaaaaaatcttctccgaccgagatatttttgccgttatcacaattaaaggttgcctgaacggacacccgctcaccggttttcccaaaaatctgcttaattttagctgtttgcttatcggattcagttgccggaattgaattaaattcctggcataacttggccgccctggcctttctggcagcaacctcatcatctaggaaataataaggttcaccagcatctaatttttctaattcagtcacttcaaatccactccttatagcctaactgatcagtatgtctggcagttgcgacgagattcacattttcttgttgtgccaagtaagcggccaatgagtgaccaaatccagttgaagtgccagttacaaaccatgttttatttgtcattagattttctctccttgtttgattagattacacattcatgctacaactttaaccaaggtttaagtcaagtcaaaatattggaaagaggtatccatatgtattctattggagatgtggcaaaaatcatgggaatcagcacgtcggcaattcgcttttacgaccgcaaggggctgttgcccttcgtagagagggatgacgccggcagacgaaaattcaaaccaaatgatttgaatttcctggaagtcatcgactgtttaaaacaaagtggcgttccgatcaaagatatcggccatttcatcagtctgtgcatgcagggggacggcaccttgaagcaacgctatgactatttggatcaagaagaagctgccctgcagtcaagcatcgatcggatgaagtcgcagctcgctttcctgcgctataaaaaatggtgctacaaaacatccgtggaagccggtaccgaatcaattcacttcgccccgggttccaacgttgttgatccaaagaccaaaagtcaatatcaagaagcattgcagcactgtaccgacttacgtgacttgattgatcttaagcaatctaaagctgataactaaagcaatcaaaaacggtttctcagatgatttgaagacacgtcatctgagaaaccgttatttgttatcggtaaattactgttttaacctggaatcttcctgagcacgcttttgatacattggaatttcgtcctcactggcacgaacccagtgatgcggcacaatttcaactaatgaacgttccttgccgtcaaattcctggctggcatcgtaaggaatttgaactcgggcccgttcatactctggatcgggtaccggcacagcggacaagaggctggctgtatagtcatgtagtggatgcgcataaatctcatcagaactggcaatttccagcattctgccatagtgcatgacaccaattcgatcggaaatgtacttaaccattgaaaggtcatgggcgataaacaggtaagtcaggttccgttcacgctgcaatttcttcagcaaattaaccacttgagcctgaatggaaacatccaaagcagaaatcggttcgtcggcaatgataaattgcggttgaacggcgagggctctggcaatcccgattcgttgtcgctgaccacctgaaaattcatgaggataacggctggagtggtctttgttcaaaccgacggtctccagcaaatcttcaacctgcttggaacggtcagcatcatctttggctaaatgattaatatcaattccttcagcgacaatatccttaactttcatccgggggttaagtgaggcatagggatcttgaaagatcatctgcatgtcccgacggactgtttgcttttgcttcttggaattgagcttagaaacgtcctggccgtcaaagacaatcttcccggatgtcggttcatataaatggatgattgcccgcccggttgtcgttttaccagaaccggactcaccaaccagaccaaaggtttctccgcgatagacatcaaaagtaatgtcatcaacggcacgaacttcatttggcttaccaatgttgaagtattgttttaggtgttcaacctgtaatattttgttttcttctgaataatcaatcacagttgctcctcctgttcttcaacatgattccccttgctcttattaatttcttgatgaacaagttcggcgtagtgcttctggcgttcgatgattggttcaggtggcgtcactttgggtgcccgtttgtcgagtaaccaagttgccgcataatgggtatcagataccttgaaaaatggcggctgcttttcggtgtcaattttgagggcgtatttattccgcgcagcaaacgcatccccaactggtggatccaataaatcgggtggcgttcctggaattgatggtaactcagtcccgctggtgtccatggtcggcatcgagttcagcaagccccaagtgtacggatgctttggattatagaagatctcgtcaaccgttccgtattcgacaattttgccggcatacataacggccactcgatcagccatcccggcaaccactcccaaatcatgggtaatgaaaataattgaggtattggttttggcctgcaattctttcatcaaatccaagatctgagcttgaatcgttacatccaaggcagtcgttggctcatcagcaatcagaatttcaggatagttcaccaaggcaatggcaataacgattcgttgtctcatcccacctgaaaattggtgaggatagttgttaatccgctgttcggcattttcaatgccaaccagcttcatcatttccaaagcttgggcataagctttttcacgtttcatgcccttatgaataatcaaaggttcggcaatctgcttaccgattttcattgttgggtccaatgatgtcattggatcctggaaaatttcggcaatgtctcgaccacgaatctggtccatttgtttgcgggacttctttaacaaatcttggcccttaaacataattgttccgctgtcaatcacagcattgggcgagttcaatcccataatacttcttgtggtaaccgttttgcctgagccggattccccaacaatcgccagggtttcaccctttctcaaatcaaaactcacatctcgaatcgcttgaacagtaccggcataagtattgaagttgattttgagatttcttacctcaagaacatctttttcgttttccatctcaaaacacctactctctactctttggatcaagggcatcacgaagcccatcacccaagatattaaatgcaatcattaagactgaaagaacgatcgctggataccacatctgataaggcaggaactggaagttcttctgaccatcgttaatcaacgtaccaagtgatgcctgaggggcactgataccaattccgatgtatgacaggaaggcttcgaagaagattgcagttggaatggtaaacatcaagttaatgatgatcacactactcaagttaggcaataaatgcttaaaggcaatcttccaagaactttcacccaacgttcgggccgccaggataaattcctggttcttcagttccagcgtctgcgcccggaccagccgggccatgttaatccaactggtaatcgcaattgacaggataattgcggtcattcctggcttcaagaccaggattaacagaaccatcacaaccaggttaggaattgacagcatgatttcgatgattcgttgcatcaaggtatcaacccggccgccgatccaacctgaagtaatgccgtaaaccaccccaaatgccaaatcgaagaaactggcaatcaaagcaatttcaagggaaattcgcgttccatataagattcttgagaacaggtcacgaccaaggtaatccgttcctaaaatgtagaaatggttgccggcatgagcctgcgcataagcgttaacccgttggccggattgatcaatggttccgttaaacccgttaatatcaataccgggaatcttcggcggcaagttcgcgaagttcgggttggtcgcatttggattatgtgtttcaaataaaaatgagaagaaagctaaaataaagagaatgattaaaatcaccaaagcaatcattgctgctttattcttccgcaatcgacgccacgagtcttgtaagaaagttaaagatggcgttgcgattttttcgtcgtccagcttagcacgatcggcaccggcaatcggtgtaaaatcgtcagctgaagtttgttttgcattgtctgccattattattctccctcctacttattaattctgattcgtggatcaattaatccataaacaatatcagtaatcaacagcacaacacaaagcatcgcactatacacaattgtcagtcccatgatggttggataatcgttggtcaaaatcgacttaacgaattgttcaccgattccgggaatcgagaagatattttcaacaaccattgaaccggtcataatgttaacggccagcggtccaataatcgtgacaactggaattaaactgtttcgcagtgcgtggtggtaaataattccaactttgttgagtcccttagcctttgccagttcaatataatctgaactcaacacgtccaccatttctgtccgcatgaatcgggcggtttcggctaatggcgacgcggccagcgccaaggtcggcaggacggtatacataaacccgccccagtcggcgattgggaataatctcaatttcaaccccaggtagtactgcaagaggaccgccaaaacgaatgaaggaattgaaataaacagaatcgagatgatggtagctgaagtatcaacccaagtattggctttgatggcaccaacggcaccaacaaccaatcctgcaagaactcccagtaccattccttgaccaccaatgatcagagatggtccaagtcgactggaaattaagtatgaaaccggttggttactgaattggaaggaagtcccgaagttaccgtggatgatgccacccaggtaggccaggtattgctgccagacaggtttgtccaacccatactgtttataaatttgatgaatctgtgtcggtgtcaatttggcttggttagtcaatggagtaccaggcattaatttcatcaagaaaaaggtaatcgtactgacgataaacaaggtcagaataatgtagaatattcgttttcccaagtattttgccataagtgttcctctcatttctaattatgttgtaactattttttcataaaccccataataatgtaaaagaggccggatttcaataaccagcctcaaatacatcgaactgttcatttaataattacttaacgtaagccttggaccagtcgtattgtggtgaggtggtgaaggcttgaacacccttaacagatcccttaagcaaagcggcttgaccttgttgataaagtggaactaatccttgttggttcatcaagatcttttcagcttgaaccatatcgttccaacgagcggtttcgttgttggcatcggttgattctgacttcttgatcaaagcgtcgtattgcttgttagaccatttaccatcgttgtatgagttgttagatgtcatcaagtccaagaagttgcttggatctgggtaatcggcaatccatgcagaaagaccaatatcaaattgttgattttccatcttggttaattttgacttaaatggaatgtttgagttggtaatcttcaaaccaggtaatttggttaattgactttgaacaaattcagttgcccgtttggtatcatcatcatcggcacccattaaggtcaggctcaatgacttcttaccaacttgtttcaaaccttttgcgaataaggctttggcttctttcaagttgtaatcagtaccggctttgacatatgcctgatcggcaaagtccttgccgttgtgtttagccatacttgctggaacaaagcccttaggagcaatgtcgccaccttgcataactttgttaaccatttgcttcttgtcaattgctaatcccatcgctttacggatattgacgtttcgaagggctgggatcttcttagtgttgaattccatgtaagtagttgaagcttgtgggaagacaacgtaatctttgttgttcttgttgttggctgccaaagttccactcaaagtggtgaagtcaagcttgccgctgttgaaactgttcaatgaagttgaaggtgtcttaacagcttggaagttaacttggtcaagtttgaccttcttagcatcccagtacttagagttcttaacgagcttccaagtatcgttggttcctgaccagcccttcaagataaatggaccgttgtagctgttcttggttgaattggtaccataatcgctaccatatttggcaaccgtctttgaattctgtgggaagaattctggttgggtaaccatgaacttgaagtagctttgtggttgatcaagggtaacgacgaacttatagtcaccgtcagccttaacacccaacttggaaggtgacatttttcctgcgttgatcttagcagcgttcttgatgttggcaaatatgtaagcatattgtgaagccgtctttggcttaacggttctttgccaagcatagacgaaatcctttgcagtaaccggagtgccatcgttccacttggagtgacgcagattgaatgtccatgtcttcccatctttagaaacgttgtaactcttggcaacccctgggtctactttgttgtccttggccatgcgaagaagtccttcgttggtaccattggcaacttgtgctgaatacaggtcaatcatctttgaagtatccatggttgaaatggcggatggtgtcatccaactaacttcttgcttcttggttccttgtgaagatttacttccacacccagcaaggatcaggccagtaaccagcgctaccccaccgagtttcgctaatgaattaattttcatgttgcgatacttcccttctcatatatgaaatacttaatttgtaatgaccttattttaaattaaaatttgattaaaagcaaacactatctggtcattcaatcgatttgtccggtgccgaattggtatgggtggttaattgtgaacgtttaattgcttaaccaccagtgtttgaagattctctttcactttcaaaatttttaaaaatttattggtaaaaatgattctgtactagagatacgcaccaattaagtcagatatgcgctccaggcgcaaaccgattcacagcaggaatcaatcgcttactcactatattaagagaagtgtcaggtgtcgatatacatatttatatgcataaaaaagctcaccgcgaattgggtgagcttttctatgatattaaagtttatttaacagtaatcttggaccaatcccactgcggtgcagttgggaagaattgaacgccgtgaatctttggcttcatcaaagttgaaattgcgggttgataaagtggcacaatcccttgatcgttcatcaagactttttcagcttgaaccatgtcattccaacgagcactttcgttagcggcgtcagtgctttcggatttcttaacgagagcatcatacttggcgttgctccatttaccattgttgtaactgttcttggaagtcaatatatccaagaagttgcttgggtcaggataatcagcgttccaggcagtaatgaccagatcaaattggccactggcagaacgtgacagacgcgtcttataaggaacgttttggttggtgatcttaacacctggcaatttggtcaactgactttgaacaaattcggttgatcgtttggcaacgtcggtatcgtctgaaagtaacgtcaggttaaccgacttcttgccagtttccttcaaacctttagcccagtatttcttggcttcgttcaagttgtaggccaccgcactcttcacgtatgactgatcggcaaagtccttaccgttacgttgtgacatgtcgtcggcaacgaatccctttggtgcctgtgaaccatcggcgagcactttgttggctaattgtttcttgtcgatggcaagtgagaaggctttacggatatttctattcttaaacattgggaacttcttctcgttcatttccaagtagtagattgaggcttgcttgtacaagtgatagttcttatcgttcttgtattgtttaacttgagttccgctcaaagtggtgaaatcaagcttgccgctttgataaccgttcaaggcggtgttaggatctttgattgcctgcatgtttaaggtatcaagcttaattgccttggcattccagtactttggattcttaacgagtttccaagtatcgttggttccgttccagcccttcaaaacgaaaggtccattgtagccgttcttttgagcatcagttccatatgaagacccatattttttaaccttcgaaatttcttcagggaaatagtaactctgagaaaccatgaatttgaagtaactttgtggcttgatcaaatgaacaaccagtttgtaatcaccctcggctttagcccccagcttggatggtgataatttatcggcgttaattttgtcggcattttcgatgttggtaaagatataagcatactgtgaagccgtcttgggattaacggtccgctgccatgagtacacgaagtccttggcagttaccggtgtcccatcattccatttcggaggttaaacgtccaggtcttgccatccttggacacggtataattcttggcaacgccaggcacaactgcattgcccgttgtcatcttcaacagcccctcattagtcgcgttaacattttgactggaaatcaaatcagtcatcttcgagacatccatggtgttaatgttggcggctaccatccaattggcagattgtttcttggccccggaatcggaggatttgctgccacacccagctaacacaaccgcaatgagcagagaaacaccagcgatctttaaaagtgatttagtcctcataaatatgaaacttcccttctgtcttatgtattatctgtgaactcattcattttaaattaaaatttaattaaaatcaatatcatttgaatattattataagactgatttgccggtattgttgtggaagtcaatgagatcaatgctatgggagatgaatttcagataataaaagttgcatatatttttaatctttgacaccggtcaatgatcagatccgaaaacgaagtgcactttgtccactatttatttacatttgtgtgttatacttacttgaacacataatttattaggaggcaccacatggatttacaagttactttaactcctgttgtcacgattggattgaaccgcaacaccagcagcttcgagtattcaatgactgaattgaataacttggcagaagctaacaatatgaaggttgttgaaaccttggttcaaaaattagaccggcccgatcctgccacttacttcggtaaaggcaagattgaagagttgacccaagtcgtcatcgatgagggtgttgataccattgtggtcaacgatgaactgtcgcccagccaaatccggaatattgagaaaaatacccattcccggatcattgaccgaaccggtttgatcctcgaaatctttgctaaccgggctcagtcccgcgaagccaaacttcaagttgaattagccaaattaaaatatcaactaccgcggctgcataccagtgccagccaacggttggatcaacagaccggtaccagtagtggtgctggtggcgcaaccaaccgtggtgccggtgaatcacaatacgaattgaaccggcggacactggaaaagcgaattacccacgtcaatcaagaactcaaagaaaccgccaaggctgatcagaccaagcgcaagcagcgtgaccgcagtgaaatgccaacagttgccctggtcggttacaccaacgctggtaagtcaacggtcatgaatggcatgatcaacttgtttggcgagaatgaagacaaacaggtcatggttaagaacatgttgtttgccaccttggacacttcagttcgaaaattaaccttaccagaccagaaacgtttcctattaactgacaccgttgggttcgttagtcaactgccccaccaattagttcaagcattcaagtcaaccttgtcggaagctgccaatgcggacctgctgattcaagttgtcgactactctgatcaccatcgtgaattgatgatgaagaccaccgaagataccctcagtgaaattggtgttaacggggtgccgatgatcgttgctctcaataaagccgacaagatggaggttgccttcccatcccgcgaaggcgacaacctgatcatgtctgccatggatgaaaagtcactgcaagaattagcgacgatgattaaagaaaagattttcaaaaactatcatcgattaacgttattaattccatttagtgacggtgacgttgtttcgtatttgaatgagaacacgaatattgaagccaccgattaccgcgatgatggaacggtcattacagcggaattaaatgacgtagatgccaagcgatttgaaaagtacctattaactacggaataagttggttgttaacaacagcagattctgatactatttgttgcatatttttttgagaagaagagaggaaaaaccatgaaagaacagaaagaagtaacgctggaccgtgaccttggtctctggtcagcgttagcccttgtgattggaacgattattggtgccggtgtctttgttcgtcagtctgccgtcctagacgatgccggctcaacgtcaatggccctatttgcctggctggcaggggggattttaaccattaccgccggattgacaattgctgaaattgcatctcaaatgcctgaaaccggtggtctctacgtttatatggaacggatctatggcaagttatggggctttctctccggctggatgcagattattatctacggcccggcaatgatcgcctcgcttggtgcatatctggccattttattatcagatttctttggcttcccaagcaagtacaatgccattctggcaattggcaccatcgtcttagttggtattttaaatttattctcgaaccgttacggtgcgacgtttgctattattacgacgatttgtaaattggttcctgttgccgcattaatcatctttggccttttctttggtaatgaaagtgcctttggtcaaagtttggttcacgtacatcaatctgccggcaactttggtgttgcgatcttggcaactctattcgccttcgatggctggattttggttgccaacctgggtggtgaaattaagaacccgcgtaagcttttgccacaggcgattacctttggtattttggctgtcttagcgatttacctgctggtctcttacggtgtttatcgttctgttcctgctgaacagattcatcgtttgggcaccagtgccattccatacatcgccaaccaggcctttggtgaagttggtggcaagatcttaagtattgggatcatcatctcaattgtcggctgtatgaatggtaagatcatgactttcccacggattatgtatgcgatggctaaacgtggtcaactgccattctcaaagacgctgtcctacttacacccaaagtcacacaccccaattttctcaacggttgccgagttattgatcgtcacagtgatgatcatcttctccaacgctgaccgcttgtcagaattatgtatcttcactgtatactgcttctatgtgatggcctttgtcggcgttttcctcttgcgaaaacgcaatccggatcaacatcgggtattctcaacaccattgttcccaatcaccccaatcctagcaatcggcggttccttgttcgtcatcgtcagtgaaatcatgtctgacctaccgggtgtcttaacatcatttatctttgtcgccgttggtattccggtattttattatgaaactaagaaataccgtgagagccaagcagctgcagcaaaagaagaatcattagataacgaaaactaataactcatacaaaaaacgagctggaaatcaaatttgatttccagctcgttttttgtagttgaggcaattttatggtaagacaacgaccttgccgaaactatcatgactatccaggtaggcttgagcgtcggcggtatgtttcagatcaaacaccttggttggtgctacgtccacgtgattgttgttaatgatatcaaacaaatcatcaaacacccgttggtttagggcaccggattcaaaactggttaaataaccaccattgagttgggaaatgggctcgaagtgagttaagtcccaaatgccgccaagttcaccggtgacacaggtaatcccattttctttaatgaattgcatggagttgggcagcgtcaatgccccaaccagttctaagattcgatcaaattgtctcccggttgcctgcaattggttatcttgatccaagacaacttcatcaaagccgaccgatttcaattcatcggtcttttccagatgccgggtggagccgaccagcttgatcgatggcaccattgcccgcgctaatttaccggcagcaacccctacaccactggttgcaccacgaatgagcagtgaatctgcttcgtcgaggtgcagtttgagcagtgatccgtaggctgtcccataagtctctggaacggctgccaaatcttgaatcgcaaggtgagtgttaaccgcataaatatggtcatttggcagcaacgtatattccgcataactgccgtcaaaagcacggcccatgccacccattacagaaaccacaatttgccccttcttcaagcgctttggatcggtggtttcaaccacttcgccgacacactcaatgcccaggattcttggtaacttgacagatggtgaccaaccatttctggtaaaaatttctgaacggttgatcccaaaacctttaactttcaatagcgtccaaccgtctttgactttgggcgtcggcacatcttcataggataaggcggaaggtccacccgggtgacgtaatacaattgctttcattctaattgccccctaaacactctgtcgttcgacaattttaattggcgtatacattgaataaaattctttaaatgagtcactcaccagcatatccattccgttagcccccatctcgaaaaaggattgggtaacactggataatttaggccgaacgatgtcacacaattgggtgccgtcaatcgtcaagattgccagccggtccggcaccttcatcccatagttggtggcttgattcaaaattccaatgcctgccagatcacttgaagaaatcacggcagtcaactcggtttgcggaccataatgttccatggcgttcacaccatcttcataggtaaaatgccccccgcaaatccaatcctcatcaaatgacaaatggttgtcacgcatggcatcccggtagccttcatagcgcaaatgaccgacaaatgaatccaagtcggttgcggcaagcccgattttttgatgacctttgccaatgagatacttggtggcctgataaccaatatcaaagtcattcgaagaaatgaatggaaaggcactattcttcaacgtcatcgaaataaaaataaatgggatattggcattttccagcaactcatcatttgaagggtccaaatcaatcgccactagtaaaatccccatcactgatcgttcaatgacggttcggatcgcttttgcctggacctcggtatcgccttcaccggcgaaaataatcatgacgctcaggttatgaacccgcgcctgttcttggatcccctttaagatctgatcagagaaattggtttgagtagaactgaccagaaccgcaatcaccttgctgcgttgcgtgaccagttccactgcactggtgttgcgccgataacccagttgcttaactgccgcccgtactttttgagctgttttttctgaataaaaggctttttgattggacaaaactcgggagaccgtcgccggagaaaccccggcagcccgggcaacatctttaattgtcgcagccatgtgttcacctcttcatcaatatagtcggataaatcttcgaaactaattataccacagggccgattaaccatttctgcctcaaacgtttgtgttaggataggtttacgtatttgaataagcacctaggctcaaaggcaaccatttccggttgtcttttttggtgtccaataagcttggcgttataattaaggaaattgttctgtaaaggagggctgcccatgaccgcttatgttttgtaccaactcgaatggattttaaggctatttgtggccgcaatttgtggtggcctcgtcggttatgagcggaaggtgcggttaaagaccgctgggattcgaacccatatgttagtggcggttggatctgcgctgttcatgatcatttcgaaatatggtttctttgatgtcatcaaccatgcggatgtcagcttggacccttctcgaattgcctcgcaggttgttactggaattggttttattggcgccggggcaatcattacccgaaatcacaagattgacgggttaaccaccgcggccggtctgtgggcgaccgctgcaattggcctggcaattggggctgacatgtatgttatcggcattgctgggacgttgtgcatcctagttacccagaccatcgtccgtcagattcgggcattcaaacgataccctaaccgttccttacttcgcctgcaagtgacttttaacggcgaactggcctcgatggatgagctgccgggccgcctgcgagcgatcggcagtgctgatatccgaatgagaatcgtcgcttacaaaccggattcgttctcactggaagtccgggtaaaattgcagcataaaatggatccggacgagtttatccgccaaatgagcgatttggtcgatgtacggaagattgaagtgctggattaaattccgaatataaatacaacactcagcgtaaagccgccagtaaggcttcttttttggacgggagaatggctttatgttatctttacaggaaagcattagtgaccaagtattggagcccttggttcatcagagggtacgaaagttcagggtctgattgaaatatacgaaaggagtaactcaaattcaaacttgagttactcctttttgaactacatttattttgattaatatgttcactgttatttggtgggtttattttgtggtgaacattagttggagcctcacctttacatagatcaaacgtgttccgacgacccagatgagtgatttgatcgatgcacggaggatgaagtactggattaagagtgacaccttcatacgaaaagagccatcaacgatttttgttgatgactcgtatttactgttacaatcctagtgaaaatcccactaagaatgcaaagattagaagtaatatgattggccccataaaacgggcaaatttgattatttccattgagtggccttcttttggtggggttctttgagtagtgttgcttctacttggataaaacgtgttccttggagcagcaacctgcgtacaagtaaacgtctgtcaaaatcaaactcgattttaacagacgttaacttatactccggttgctaagcgctccaatccacactctaccgttctgctccctggacaacttcctccacttcacccgacttcttggctgttcccagtctgtggtcgaggtactgtgacagaagtgacagtgagtaacatacgatgaagtacatgacggctaacgccaagaacattggaattgtataattggtgttttggccgtaaatgatttgtgcatggttcatcaaatccggcagcacaatgatagttgccaatgacgtatccttcaccaaggaaatgaattgactcacaatcgctggaatcatgttcttgatggcttgcggcaagataatgtacctcaatgcctgccaataagacatccccgtcgatctggccccttccatttgtccgactggaattgagacaattccggcacggacaatttcggccaccatcgccgattcaaagaccgccatggcgatgactgacgcccaaattggatccggcttgaagccgatatttggtaagccaaaataggtaaagaagataatcaggattagcggtaagttacggataatatcaatcacaaaaccgacaatcgctgataaatatttaatttcaacatatctgataattcccaagattaccccaaatatgtaactcaggataatcgaacaaactgaaaccaggatcgtgacccaagctccttcaagaaggaacctgatgttaatccatgaataagcacctaagactgttaacatatctcgattcctcctttatgccaatttcttttcaaggtaacgcatatagtaactcaaaggcaaagtcaaaatcagatatagaacaccaacacacagatatgtgctcatactttgcagggagtcagacgcaataacgttaccttgatacatcaaatcgaatccggcaacaaaggctaagactgaagagttcttaaccaagttgatgaattggttgcccagtggtggaatgacatatcgaaaggcttgcggcaaaacgatataacgcattgcctgccagaatgataatccattggcacgagcgccttccatttgaccaggatcaacagactggattcctgatcgaacggtttcagcgataaacgctgacgagtaaaggatcaggccaatcgtaccagaggcaaaaccactgatttcaacaatgtacattggaataaccacgtagaagaacatcgtgataaccagtaatggaatgttccggaaaacttcgatataaactctggcaatcactctaaagaatttgttgggtacaacttccaggatggcaaaacccgagccgatgattaatgcaaagatcaacgcaataatcgagcacaaaagggtttgtcccagtccataaaggagctcaccaccataattttgaaaaatacttatcatcgttctgcccccttaaagtcaaatccgtgaaccttgtggaaccacttataaaggagcttgttgtattgaccggaattttcaaccttggtcagggcgttgttcatcgcgtctctcatctggccttggcctttgtcaacggcaattccataaggttccttggtaaaggtgccaccaacaaccgaataacctgggttttcgatggacatcccataaagaattccgttatcagtggttaatgcatccccctgaccggatttcaaggctgtcaacgcctgagaataatcagacagttgaagcactctggctttaggcgcaaacttcttaatattttgaacggagttggaaccaaccaccccaaggacaatggcgcccttatggttcaaatctttcacattcttgattggactaccattcttaacgaggatggcttgcccggcatcaaagtatgagcgtgaaaagtcaacttgcttggcccgctcaggggtgatggtcatggttgccataatagcatcaatgttgccgtttctcagtaatggcatccgggtttgactggttacttgaatgaatcgtgccttgccgtctttgccaagaatctgcttggtcatcgctttggccaaatcaatttcaaatcccttgatctgattgtcccgtacatccattaaaccaaacagcttggtgtcggctttaacgccccatgtgatcgtctttgtctgcttgtcatccttcagcacatttttctgtgatgctgcgctcgaacaggcactcaaagaaacgaccattaagagcagggttaataataacccaattcttgatatgatcttcttcatgatgcgacctcccaataatgaaatttttaatgcgtaataattttcccaagaaattgtcgtgcacgttcattggagggttcaccatcaaagaatttgtcacttgtgtcatcttccaaaatctgaccgtcatccataaagataacccggttggcaacttcacgggcaaatcccatttcgtgagtcacaaccaacatggtcatatctgaatcttgcgcaatatctttcataacgttcaaaacatcatcaatcatttctggatccaacgcactggttggttcatcaaacaacagacactttggcttcattgccagagaacgggcgatcgcgatacgttgctgttgaccacctgataattgggctggcaatttgttggcttggctttgaagaccaacttggtcgagcaattgcattgccaactctttgttttctttttcaggacgcttcaacacaattcgtggtgctaacatgatattttcaagaaccgtcttgttggcatacaaattaaaatgctggaacaccatcccaacgttctttcggatccggttaacatcggtcttcttgttggccaagtcctgcccattgacgatcaacttaccttcttgaatcggttcaaggccattaaccgttcggatcagtgtcgacttaccagaacctgaaggaccaattaaaacaacggtttcgcctgcttcaatcttcaaattgatgtcctttaaagcatggaaatcgccgtaatacttttgtacgtcttgaaattcgatcattgccatgtcattttcctccaatgctttcaggctatttattaaaattgcctaagaatgatactacatccataatatgttaaaaattttgataggtcaaaaaaatgttacaaaaattttatctccatgtcacattttctatcaacggagttaatccgatgataaagccattcaaactcgaccattattttggatgtataaatttgggtaattatctaattataattcaccatcagcgaaaatggaaaccccatttgaataaaatttaattggaagctcattttgtggctaaaaaatgagagctcaaaaataacgtgcaatccaaacccagcccgggttgaattgcacgttattaagatgagaaaatattaattttcagaaatgtaatcgagaatttgaaacatgacgtttttattttctgctggaacctgacgagccaaaatttcatcagctgactgattcaacaccgaaccttggatgtatgcagcgtcattgacgaccatctcgcgaacattatcttctttgggctcaaagtgaaactgcaacccgacaacccggtgattcaacacaaatccctggttggccaagtggtcgcttgagaacaataaatctgcatcatcgggaagttcaaacatatcctcgtgccaatgcagcgccgtcaattgctcaggtagtccaggaatcacgtcggactttcgatacaccggggcccaaccaacttcttttgccggacccttggaaacagcgtagcccaaggctttggcaatctgctgagccccaaaacaggcaccaaagattggtgtttgagcatccaacagttgttgaatcaattcccgttcttgttgaatccacggcaaatcgtcattaggactcattggtccgccgagaatgatcaacatatcagtctgagctgcagttggcagtaggccaaattgatccggatgataaatgtacatctgatgccccttggcatgcgcccagtcctgaatggatccgggtccctcatcggcggcgtgttgtaaaacattaattctcataatgaggccctttcgtttataacttcttgtaagcaaccattgcccgcagcttatagtcttgtggcgcttcaatcaccccagcccggccgatctgcttgtatggtccaccaactaaggtcactgatgccaagtataacttgacctgactcaaatcaagcgatcgaatcgactgcaggccaatccgcttaatttcgccgaccggatagatctctgcttggttcaaaccgcaatagaccatcaatgacgaaccttgtttttgcatttcaaaataaggaagcaatacgcctttgccaatggcataaatcggcttactattaaccttcagcagttcatagatcttccggtcactcatgccgttatagtcggccttaaacagctgttggcgttccatttgggaaaccagtcgatcaatattagcctgctgcattgggctgacctcaattttagccggtaacaggtgttggtcgtcgaacaagccgttagccggcacgtttcgttcatcagcgatgacggtggtgcccattttggattgcacctgagtttctcgtgggtgctcttgaatgtgcagcagcttggcaattttcggtgaaatatcgaaccacggctgcttcttagtaaagtaataaaagaagttgcaaattgtaaagtacagcaaaatgattgcgactaataaaatcgggacacccttgctaaacatctgattctgtaagaaacgaaaactgatgtaaaacaggtagacgtcaccaaagaagcctaacactgtgtaaatccggctcttaagggtcacattaatattgaagtaccccaggtagtggttaaccatgtccaaaaagctaaacattagttagttccctcccctgtattgccagtcgtcacatcagcgttggcattcgtattattgttattttgagtgttggttccgcccgttgtcccggttgtttgactactactttcactaccggtctgggtattttgatcggaattattgttattagtggtagtaccgccggtcgttgtccctttattagtggttgtacccttattggtagtcgttcctttattggtcgttgtcccggttgtcgtattcttgttgttattggtcgtatcatcgttggtttgatcatctgaagagctggcgttcttttcgctctcggctttttcagacgaagccttggccgcagacgattcttcagcggccttcttcttttcggaggcttccttagccttctcagctttttctttcgcatccgaatcgttggtctttttcttattcccatagatggaatccgaaatctttttttgattggtcgtttgagtggtcctaggggttccttcattggtggacgtcacattattgaccacaacgttagtggcgccgagtgccaaagaaattgagagaatggcaaatggcgtaattaatggtggaattctattatccattcaaaaaacttccttactaaatttttgtagcctccattatcgcataagaatatgaacgaaacctaaacaattcgttaattattcattaagttgacgcactgagggcacaagccataaatctgaaacaaatgaccagtcacttcacagccagccagctgggaagtgatttcaggactcaatggacaatccttgagttcgatcactttgccgcagttactacagataaagtggtggtgatgctcatgttgaaaatcacactggaatttaactgatgcccgatcaccctgcacctgccgctcaacaatccccaaattggcaaactcggaaatgttgcggtaaatcgtgttatgactcatgttgggaaaggttttgcgcatgaaatcatcaatgctggtgacttcaacaaacttatgcgtcgctgtgccgactaaaaattcaatcatcgcgcggcgttgcttggtaatcttgaagttattctcttttaaaactttggtcgcttgttcaattgctgcaggcatactgttcacctctaataagtaattattactgtttattgcatcctaccataatctactttcagcaacaactatcccgccgtttcttgacgataattctcaacgattttatcaatttgttgacgcgtctgctgccaatcctggttaaccacttgataagccttgccctgcagttcataaggcatttcgagatcacgatgatactccttactgctgacccgtttggcaaccatctcagcattgtcaccacgcccctgcattcggcgtttgagttcttcagtatcgccgacctgcagaaaaatgatgactgccttttcgcccagtttctgcttatatgtaatggctccggcagtgtccaggacaatcgtcgcaaatggtgatttctcccaggcattctctaagccttcgtaggatgaaccataatagtggccggcatagtggacggactccaaaaagtgattgtcaaagaacgattggtcgtcctcaaaataatagtccaccccgtcacgttcattttcccgcggcggccgggtggtgtgggtgatcacccgggccatttgatattggtcatgtaaataatcacgaacggttgtcttgccgctgccagcggctccggtaatcacaaatactcgattcttcatcaggcttcctcgatgttttctttattgcggatataggtgtcggcgtgcttaagcagttgtcggagattatcataggttaacttttcgtaagcatcttcatagtcaaaccatccaaatgagttgatctcttcatcctgctttcgaaccttgacttctggcgccacccggctgacaaagaaagtcacgtccttgtggtggccgttgttcatatcgtactcaaccttttctttaaagttggcgtcgatttgcgtctttaagctggtttcctcgtgaatttcacggactgctgtttggatgagattttcattcttctcgacgtgtcctttgggtaatccccaaaaatcagaggtggcactctgcaataacaggtaccagatcttgccgtctctaatttcataaaccactgcaccactcgcatattcagtaaccatcattaatctccttttaaactttcattgttttcttcaataacattggtgccacaatcgtcgacaatacaatgacaataataatttcagagtacaggttcttggccatcaaattggcggacaacccgatttgggcgataatcagcgccatttcaccccgtgataccatcccggaaccaacaataaacgcgctgctccaattcattttggtgatccaagcacccagggcgccgccaaacaacttggtagcgatcgctaaaatcgtcatgatgacaatgaagcccaggttcttgatgacattgttgaactccatatccaagccaatgctgacaaagaagatcggaatgaaaaaggtgtatccgactgagctgacactactggagatttcatcttgaaatttcgtctgtgaaacggccaccccagcaaagaaggcgccaaccaccgaactcaagcctaaagcgtcagcggaccaggccattgtcaaacagatcaccagcgaggtaatcgctaccgagccgtggaccggcaatcgttctgccactcgcagtaccaccgggaccacccatttaaccaggatgatcacacctaaaaagtacatcaattgatacagtgtggcaaccagtaaattcgacgatccactgccgctaactccaaaggagctgacgaagatactcagcaaaatcacggcaatgatgtcatcaaccactgctgctcccagaattgtcgcgccttccttggtgttcaatttcttgaactcgcgaagcacttcgacactaattgagaccgaagttgccgcgaagataacgccccaaaaaattgagcgctcaaagccctgccccatgatttggccgtagccgtaaaagacaatcatggggaacaagacgccgattgccgccacactaattgccggtttgaaatacttcttgagtaaatccagatcgctttcgatcccggcaatgaacatcaaaataatcacgccgatttctgccccggcgtgcatgagttccgtattgtgcaggacccctaagatacccgggcctaaaataaccccggcgatcaactggccgatcacagccggcatccctaatcgttgactaatcgctgccgccaataatgttgcaattaaaatgagtgcaatttgacccacaaacgccatctaataaccctttcttttcttaaccattagttacgtactattgatattagtttaccataccaattgcccgcgttcatgggctgagaccggtaattttaagaacttaatttcacaatcaagatactttcaatttctggtaatattccgatataatgaaagcgattacaaggaaggaatatttacacttgggggtgaataatcatggagcgttccaagagactactcaactttttgttaatgatcacgacgaccgccatcctgatgtttgtggggatggtcttaaataaccaaacgccgatggtcacggccgccaatgcagccactactcaagacgaacagaccatcgacaaaataatgccgaatgagaaactgcgagaattagttttaatcaatatcaaagatcaaaagatcattcaagatcccaactttaccttgagtgacttcacgccgaccacatttaaggaagatttggcaaaactaactcagctgggctgggagattggaaccaacgaacaagtggaccgccaagaaccggtcaatggcggcaacggttcggtcggccctgcaaataagggtaattattcactggaaggcttggaatattgtacgaacctcaccaagcttgaattgaacgcagacttaaatagaggaagtaaatttcatcatgatgacattattgatgtctcaccacttgaaggtctggaaaaacttgaatatatcaacttgtcaggtaatcgaattcaagacatttcaccaattgcgggtctgaagaatgtcaagactttatatctcaataacaactgcatcaataatctaaacacattggacgctgaacaatataccgagggatttaactacctggagcaaatcgtcattaaaccactacaagtgctccactccaacacctacacttggaaagcaccgtttgtggacgccttaccaaaaaacgttaaaaccgaggataacaaaccattccagccttaccagcaaaaatttctccgtccgggaacccttgcttatggcaacccaaccgataccaagtactctcaaattgacgtcttccgcaacggcactcgtgggactggtgtggcccagggaaccacaaccattaacggtgatgatttcacctacacaaatttggcaccgcaaattatcccgacagatcccactaacccatgggccagctaatatccaaacgcaaccgttgttaacaatacctacacttactacatgattgcgcaatataacgtctacccaggagaaccgctctacgcagcactgagctactttatgccatacgtcattcaaccagaagaagcccagccggtcacagttgagtatgtcgacaccaacggcaactcaattcatgcgtcagctacgatcaagggtgaaattgatcaagccttcgatctttcaacagccgattacaaattaaatatcccaggttacaccttctccaaatacgatccggcacaaaccggcaaaattaccggagaaaagcaaaccttcaagctcatttacaccaagaattcaacaccggtcaacccgacgccaccgaccacaccaaatccaccaaccaatccggaaaccccaaccttcccagttcacccaaccccaccaagcggaacgcagttaccaaattatgcgaaaactactggtgaagtcgtctactcactgaagaagatttacctatacaagaatccaaccttcaaaaaagctgagcgactggttggttatactcaaaagccacgggtcttccgaccaatgtttgtggtcaccggatacagctattccaacgcaggccgcttacgtttcaaagtcgtcgatgtcaaccatgacagtccaactgcgggaatgaccggctacatcaccactaagtccagcttcgtttctccggtttactaccaggcagtcccaaagttcatcaccgtcatcagcccaaatggagtcatcgaatacaacgaaaaggacctcaccaagccagtccagacgttcaagcagggaagaatcctaaaggtcgagtcaatcaccacccacaacttgaccacccgttacatgctgggcaatggtaatttcatcactgccaaccgtaagctggttatgaacggtaaacaaaagcagccaaccagagtggtcgccaaaaaagcaatcaaccgctataccactgccaatttcaccaagaaaaacggtcactacaagaaaggcgccaagattaaagtcaacttctacacctatagccatgatgcgtcgaacaccaagtccggtgccaagcgattctctgtcaagggtggctatattaccgccaatccgaagtttgtgaaagtctattataaataattacccaaaagaggcgaaacatcattctttgtcagttatgtcatcgcctcttttgagttccactgtcatatagattaaacctgggacaatcggctgatcccggccatttaagtaaataatccagttattccaaaaccaggaataactggattatttacttaaattctgggatcaaagcgcctcgcgccccactcttcatttaatctaaataccccttggtagccgcaataatttcctgcagccccttcttggcatccgagaacatcatactggtctgatcttcactaaacagtgggttttgaacaccggcgtaaccggtactcatggaacgcttaatgacaacgacggactttgatttatcaacatccaaaattggcatccccgaaatggcgttacccttttcacgagccaatggattggtaacatcgttagcgccaataaccagcgaaacgtcagtattttcaaacatcgagttggcttcatccaactgtttcatttgatcgtaaggaacgttgacatcggcgagcaaaacgttcatatggccaggcatccggccggcaactgggtgaatcgcatagttgacgttaattccggcatccgtcagcaatttcgccaactcagcgacttcatgctgagcctgagcggcagccaaaccataaccgggaacgatcatgacattgtgcgcataggccagctgcatgccgacatcatcgggtgtggtcttcttaatgttggttggcacctcagcacccgcaccaatactgccgttggaatcgccactaccgaagccgccagcaataatgttggcaactgatcggttcattgcttcggccatttgcagggtcaaaattgttccggccgcaccaaccagcgcaccagcgataatcaagacctgattatcaatgacaaatccggcaaaggcaaccgccaaaccggtaaaggcgttcaaaagtgaaacaaccaccggcatgtcggcaccaccaattggcaaggtcatcaataggccaaaaatcaaactggctaacaatgccagtaccataggccagtaagcggaaggaaaaccaatcatccaaacaccggcaacgataattgctaacactgccagaccgttaatcaatttgtcgccgggaaacgaaattggtttgccgggcacatgtccggacaatttaccggttgcaattagcgagcctgagaaggtaatcccaccaataataatgtcaagcagcactggaatggaaaaggccaggctcaaagaggtaccgacagcttcgtgggtgtaatcgaaaatcccgattgtggcagcggcaccgccaccaacggcgttaaacagcgaaaccaattgaggaacatcggtcattggcactttgcgtgcgcggataactccatacaaaattccgattaacagacccgcaaacaataccgtccagccaattaaggtaatctgacccttggagataatttcaactaaaatcatgacaactgccatggccatcccaagtccggaaagtaaattaccattccgagccgtctttggggagcgcatcatgtgaacaccaatcacatagcagaccgctgacagcaggtaaattagggaagcaatcgttttaaggagtgacattatttgtcgcctcccttgtcagctgaattcggctgttttttcggccggttaaacattcccagcatccggtcagtcacggtgtaaccaccggcgacgttgacagctgcaaagaatgcggctagaaatgccaacaggtagaaataccagctgctggcttctgcagcaatcacaaaggcaccgacaacgacgacgccatgaatcgcattggcaccagacatcattggcgtctgcagggttgagggaattttactcataacttcaaacccaactagcaggctcaaaacaaaaatggctaaattcgtatataattcttgactcataatgactaatcccccttctcagctgatttgtcgtcagaatcggcaggggcagcatcgtcttcagccggttttgaaattggcaggttcagcgcttttctgactcgttcagaaataatttcgccatggtcggtcgcaaccaattggctcattacgtcatcttttaaatcgatggtaatttgagcatccttatcagcaacatcattaatcactgcctgaacgttcttagagaacatttcagaagccgacgttgccatttcactggctaaattcccggccccaatcagttgaacaccggaatcagtgatcactgtttggtcgggctttgatccagcgacattaccacccaaatcactggcagccaaatcaacgaagacgctacctggtttagcgttatcaacggcggcttgaggaaccagcagtggcggctttcttccaggaacctgcgcggtggtgatgacaatatcattttgtttgataaacccaattaattcgtcttgctgctgcttttgctcatcagcagacaattgacgggcataaccgccttcaccgacagcactgactgaactagtgagaaattcggcaccgagtgattcaacttcgcctcgagacgctggacgaacatcataaccggaaacaattgcccccagccgtttggcagttccaatggcttgcaggccggcaactccggtccctaagaccaacactttggcaggcttggcagtccccgcagcagtgatcatcattgggaaataacgggcgaatttgtcagcagccaccaaagcagctttgtaaccggcaattgaggcttgtgaacttaagacattcatgctttgggcacgggaaatggtccgcggcagcagttcaaacgacagcgccgtgaccttctgtttagcaagtttttgcaccgagtccaaatcggtcaaggccttcaacaagccaattaaaatctgtccctcatgcaacttgcccaaagtctctgaatcaggtaaatcaaccgtcgcaatcacattggcctgactaactgcatcgtctcggctaacgacttttgcgccagcatcttggtaggcctggtcagaaaaataagcattctgaccagcgccctgttcgatcataacttcaaacttgctgtgaactaatttcgcagccacatccggtgtgattgccacacggttttcatcgccagattccttcaaagcagcaataatcgtagacattaaagcgacccccttcacaatcattttgcaaacgctttatacggttcaaggctagtcctcttcatcgagaattgcaatggtttgtgattaactttataagcatagaaaaacgaaccaaaaagttattttcggttcgtccttttttccaagtattcattgtgatcgttagttagtgattaaccatgccggtattaggaacttcagaattcaaagtatcgtcaatcggattgtcatcaatgacatccagatgttcattctgcttgagatcagtttcacgtcgttccaactctttgacaatttcggcatgcttctcgtcagtcaagtcgtaaccaaagtaaaagacaatgcaggaaatcgcactggcaatcgctggaactaagaaatacacggcactaataccggagattgtgctggcagattgaggttgattggcaacgtatccagtcattgtcaaagcaagaccaggaataaagccggcgaccccttgggcaattttccgcacaaaactgtagccggaataaataattccttctgagcgaatcccggtttgcaactgaccgtattcaatcacgtcattcacaaacgcaaaggcgacggtcccactaaagcccaggaacatgtatgaaatcgtgttgacgatcagataaggaacgacatgtgagccggtgataaaaaagttgaccagttctgctgcaatgaatcccagtgttgcgtatattgcaacgttcttcttaccaattttcttaaccaacggcgtggcaaagatcaccgctggaataatcgataaagcactcaataggctcacaatactaacgattccgacctgtcccaaaacgtactggaagtagtatagttgaatacccattttaaggaacatcgagccaacactaagaatcgtgaaaatggatagaataatgaacggacggttggttaacagtcccttgatcgacttgagatcatcccccttttggcggggcttatggtcaatgatgcgttccttggttccggagtaacagagaatctgtgaaacaacgccggcggcagcaaaaatcgcgaccgtggcaatgtaaccaattttgggcgtcgcaaagatcgctaccagtggaattactactgctccggtaagcaaggcggccatttgtccagttaagttgcgagcggcagccaaagaagtccgatcaccggaatccatagtcatagctgctgccagcgaaccataaggaatatttacaacggagtaacaaaatcccatgatgttatatgaaacgaaggcatagatgatccgcccggtctcaccaaaattaggcgtgacaaaacaggcaactgttgcaattcccaggaataatgagccatagagaatgtatgggcgaaactttccgcgtttggaaatatgctgacgagaatccacgaaggcaccaacactggtatctacaaaggcatcgaagaatttggcgatcaggaaaatcaaccctccccaataggctgggatctgtaaaacatcggtatagaattttagtaagaacagctgagcaaattgaaacatcaagccgttgcccaaatcccccaatccataggctactttttcacgcattttgagtttttctgttttcaaggtaaacccctccttaatcatgtgctggttcttagtttgttaagcgctttcatttgaagcaataaaaaaccggcgcacgcggaatcacgtgttccggttcgaaaattaacgatattattttttataaccaaagttaggaatcttagtccagcggtctttcaggtaacggacaaccatcttcggttcccgtgatctggtgaaaattcctttcttattaccctgaacccgttgaatgccaaatttggtctggaagtcggcgaagttccacaattgctcaccgacaaagtgtgggaattcatcgaagaccttgctggccattcgatagtagtcttcctggaattcttcagagaatggctcgtcgtaattgctgtggagcccaggaatggtgtcggcgccgtattcggtatacataatgggtttgtccgggaatttgtcagaatattcctgcagctcatcgcgggttgcttgttcagccgtcttcaaatcgccattaccaacataccagccatagtagcggttcaaggcaatcacatcaaccaatgaaatacagttatccgtcttcggagtggccatcatgatgctggtgtaggtgcaaggtcgcttttgggggtccagttgacgggcttcatcaaataacggcttgaagtattcatatgccccttttgaaaaggttgccgcttcgttggcaatcgaccacatcgcgacacaggcatggttcttgtcacggtcgatgatttctttgatcacctgtttgtgggcgtcggcggtctttaatttggtccaagtatcgtcttggtagtcgtcgctctcaagcattgacacatcaaacccaaaggtcaccatcaacccaacagctggcgtttcatcaatcaccacaattccttcgcgatcacataaccgcatcatttcctcggagtatggatagtgggaggttctaaatgaattagcgcccatatccttcatcaaattaatatccaagacattgaccggttggttgatgccccgaccatgaacgtatgaatcttcatgcttgccaaagcctttaaaataaaatggttcgccgttaattaagaactgggcattcttaacctcaatcttgcgaacaccaaagtcttctgaataggtatcgatcacttcaccatttcggctgactgtcacttttgcggtatagagataggcgttcaacggctgccaaagatgaacgtggtcaatatgcaaagtagtatcggcagaagtgccgctgaccaccgcctggccgtcttggtccaaaatggtcactttaactccatcaatctccccgtgggtagtgactttgacctcgacgtcagcactggattcagccagatggacgtctggaacgaccgtgatatcgctgatatagtcagctggcgttgagtagattttaactggtcgttgaagaccggcatagttaaagaaatcaaagttttcgtcaacgtggcggagcttgtggccatcttggtcagtgctttccgaatagttgccaaccggcagagtcgtgtaatcaagaatattgctgagtttaacggttaagcggttgtcgctatcttttagataatcgttaatttccacctcaaacggtgtaaagccacccttatgatgggtaatttcctggccgttgaggtaaacccaagcttcatgagtggcggagccaaatcgcaaaactaaccgctggctgcgcaatggtttggcaatatcaaaattagtttcgtaccacacaaagccgttgtgctcacgaatcttctttgacgcggtttgatcattgaaggaagccggaaccgaaatgacgtcttcagttggcaacggctgtttgggatcgattggtgtgatctcctcatcgatcataaatttccagagtcctgataagtccagaaccgttctgctgggtgttgtgagtgggtataacatagttaaaatcctccgttcgttagtcagtatttggatcactgcttttcaatgtctttaatataggctaaactgggatcgaatacttatctaatttttacttaaatcgcattttattgacttttatgtaaccgctaccagaaaggatcttgacgatgaccgcgtatgataaccaatcaactgctgaactgattcattccctgacccaaattgatattgccatcattcaaaaagacggcacccccgtggtgcaaattcaagaaaacgtgttaccagccttccaccggctcaacgagtttgatccgatctttcaacaaattgagcaattccatgctaatgggtacctgacttacacggattccgcccagctgagctacgtggcggcccgccttgaccaacctgacgaccaagttgtcgtcttgggaccgttcctaaccaccaccctgaccatcgatgaaatcaatgacatcgtggcgatgaattcctataccatcagcgaacatcggcaactcacccagttgtaccaaagcttcccggtgctggcagaagataaaatcaacgacttggccactttgatgaccaacttattttcccgacagctagccaccgcccacgaaaaagccaaaatcaccaatgcgattgcctcaggcgatcaagtcgccgtccaccgtctcaatacaaccatgaccaagatatttgattccttctcgaatcgaattccaggcaagccattacgctcctcaaaaaatatctgctttgttttcaatactatttgtcgaattgccgcgcacaaaggcggcgtccacccggtctacctcaacgacatttccgaaaagtacgccttgttaatcgagcgccaaaacacgcttcaaggtttacacatcttagtccactcgatgacgcgggaatattgccaactggttcttaccctctcaacttccggctattccccaatgattcaacgagcggctgactatattctgctgaacctggggcacccgatcacgctcaatcaaattgcccaatctatcggcaccaatccgtcatacctttcaagaaaatttaagcaggaggtcggcatgaccatcaccgattacgtcaaccaccgccgcatcgttttggcaaaacaatatttgagcagaccaacgccctcgattaccgacatcgccttgatgaccggattcaacgatttaaattatttcatcagagtttttaagaagctgactggccagaccccactgcaatttcggcaaaagccgaccggttcagggattcaaaagtaaggtataatggcgttaacaatcatttccaggaggtacttcatgaaaattaatcagtttgcatatgttcccactgatcatcacactattgtcaaagagttggcggatgtccatttcttaaccgcccaaaccaaaaagatggcagatccggtcatgctttatcgccaattcctgctgaaattcttcattgaaaagcagagcttggccacccggattcaaaaggttgctaatttgatggcaacccccactctaaatgcttatgagttcacgacaactcaagctgccgtcagcaagttagccttttataacgttggcttgcagctgttgggatttgaagtcggcctggacttcgagttgaacgacccgttttccgccatgaaaaaatatcgactgccaatggcggttgtcgacgatacgctcgaccgcaatcaggtcattgatgcctggtacaaactgctcaatacgcgaaccaagtttgggcaaaccttgattgattatttggcgggtcaaggctactatcaccaattcttcggaaccgatgaactgaaacggccgctcatctttaacggtaagtcccaggcggtctttgataccactcaactcatccgcgacgtggtttacgttgaagcgcccttggacaatgaccatgatggcaaacgagacctcttgaaagctgaaatcattcgtccgggagaaactgaaaacggcttgagggtaccggttattttcactgccagcccttacgaccaagggactaacgaccaccaagccgatcaaatgacccacgacgttaatcaggaaaaattaacccgcaagcaacccaaccatctgagttatgacgacgttaagttcgattacgacaaccatgacttgccggagccacggaccatcaaggataccaacaaagtcgctgaagaatcatttgttaaaacctggacttattcattgaatgattacttcttggcgcgcggttttgcggtggtctattcatccggtgtcggcactaaagattctgacggcgtccggacaaccgggacgcctgacgaaaccatcagtgccacttcggtcatcgagtggctgcatggcgatcggaccgcatttaccaaccggtccgatcaaattgccattccggcttggtggtccaatggtaacgttgggatgaccgggcgctcttatcttggcaccctctcaacggcggccgcaatgacgggtgttgacggactcaagaccgctgtggttgaagccggcatctctaactattacgattattatcgagagaacggcttggtcgtcgctcccggcggcttccaaggtgaagatactgacgtcttgggtgaactcacctttagtcgtgagcagtcggctgccgattatctcaaaatcaaggacacttggttggcccagttgaagaaactcaccgccggccaagaccgggtgacaggaagttacaacagtttttgggataatcgtaatctcttgaagaatgtcaatatcaaagctgacatgctgctagtccacggtttgaatgattggaatgttaagttgtcccacgtttacaatctcagaaacacgttaaagaatgaaaagattacccaaaaattagtccttcatcaaggacaacatgaatacctcaacaactttcgctcagtcgatttcacggatatcgtcaatctctggctaactaacaaattgttggcggtcgataatcaagctaaccagattgtgccggatgttttggtacaggataacgctgaaccggaaacgtggaacacctacaaagactggggcggcaacgttaaagaaattccccttgacgataagcgctggacagatctgaacgagaaccattcatttagcgatcaattgccagacgatttatttaaggactacatcgaaaataccaagaagtggcagaaggccctatttaccaagaatcattccaagcttgataaacacagtattaaactcgtgtccgagccactggaccaagatatcaccgtggatggaagagcgacgattaccttgcgggctgccagcagtgcggacttaggcttgttgagtgcggctctggttgattatggggtcgaaaaacgtttgaccgctgtcccccaaattttgtctgcccagcagattattaccggttaccaatggcggaaagacgatttgaaagaatttttgcctgagaaaaaagcatcggcttacaagaagttcaccgatgcccatatgaatatgcaaaatcgcaccaacaattatcaatcggacgacctgaagcccggccaatactccaacttcaccatagcgtttcagccaacattttggcgcttgttgaaagggcatcaacttggactgattatttacgccactgatatggactacaccatccgcagcaatcaggatatttcctacacagttgatctgagcgcttcaaagattgaattaccattgttgactgccgatgataaacagggataaatgtgatatgatttttataaataacaataaggataggtgattttatgaagacaggaacaaaaatcattactttggataacggctatcacttatggaccaatacccaaggcactggcgacattcatttgttagcattgcatggcggccccggcggcgaacatgaatattgggaagacgcagccaaacaactcaagaagcaaggcttggacgtgcaagttaccatgtacgaccaattggggtcatggtattctgacagtcctgatttcagcgatcccaagaaccgcaaagatattttaaactacgattatttcttaaatgaagttgacgaagttcgtgaaaagctcgggttggacaacttttatctcatcggccaatcatggggcggcctgttagttcaagagtacgctgccaagtttggtcaacatttaaagggtgccattatttcttccatggttgatcgaattgacgattacaccaagcacctggaagaagtccgtgagaaggcattaaccccagaacaagttgcctacatgaaggattgtgaagctaagggtgactacgataacgacaagtatcaatcatacgttgatattttgaataagggatacattgaccggaagcagccttccaagctgtcgcatctgatcgatgttactaacaccgatatctatggcgctttccaaggcgataacgaattcgttgtcactggtaaattggctgagtggaacttcaccgatcaattaaagaacatcaaggtgccaacgctggttacatttggtgaacatgaaaccatgccaatcgaaactggtaagcgcatggccaagatgattccaaacgccaaattcgtctcaacaccagaaggcggccaccatcacatgatcgataatccggatgtctactatgaccatctggcaaccttcatccgcgaggtggagaatgatacgttcaacaagtagagtgtgacgagcaacgggtgatgcggtgtgtaaggccggaaagattgaaatcccgggcttggatttaaagctttttggacttacacgttagcatcagttgcctcggaacacatttcaaccagagtgtgacgagacccggttagagcccggaacaatctcaaaaaccaaacaagcgccgggagaattgcatgtcatttgcaactctaccggcgcttgttttattttcgcaatgaatctctctgaagtaatttaattggcaaaacatacttatccagcagttgatcgtcatttttctgaaggcggctgaacaacaagcgaaccaacaaatccgcgatgtcttctaccggctggacgattgtacttaattctggatgatactcctggacgtaatccgagccatcgtagccgattacttgaacgtcttcgggggctcgcatccccgcccggcgcgcttcttgaatacatagcaatgcggtttgatcatccgtacagaaaatgccgtccggctgatcagccagcagtttttcacgtaacgtagcccgacgaatggtgggcgtcgaattaaacggaaaggccaccatttgaacagaacagccatgttccttggcaatttgttcaaagccggttaatcggcggttattgggagcccgcttctctaaactaccggacacgaccatgaactttttggagcccttttcgatcatcgtccgagccgccagttcaccacctgcctgattatcactgctgacagtcggaattttcgtttgaaaataacgatcataggaaacaatcggcagccccgacattttatattccttaattccctcgttatgcgaaccagtgatgataccatcaacctggttagccatcagcattttcaaatactgctgttccttttcgggattgtccatactgttacagataatcgctttatagccacgggcaaacagccgattttcaatttcctcaaccacttgggcaatcaatggattctccaggctggcaaagatcaagccaactaatttaaattgttttccttgaaggacccgggcggccaaactaggttggtaattcagctgctgcatggcagaaaagaccttttctttggtggcggctgacaaatagccccgctcattgatcacccgagagacagtggtcacagaaacaccggccaactttgccacgtctgctaattttggttgcatgaaatcaccttctcaacgcgttttgatagtaccagtatagcatattggaaaatctttttatgttaatttatgtcaaacgattgacacatcgttatgtaagcgtgtttcatgtgttttgtgaaaggggtttcaaaatcatgagaggtgagcacattgattaataatcaacaaaatccgacttggtggcggaatgcagttggctaccaaatctatcccaaaagcttttatgacagcaacaacgatggtatcggtgacctaccgggaatcattgaaaagattccctacatcaaatctttgggagtgaacttcgtctggctgtcgccattcttcgcatcaccaaacatcgacaatggctatgacgtgtcagattatgaagatattgacccgcaatatggcacattggatgacacatttaatatgatccggcagttccatcaaaatgacattcgggtcgtcttcgacctcgtcatcaatcatacgtccgatcaacaccactggttccaagaagcgaaaaaatcgattgataacccctaccatgatttttacatttggcgaaaaccgattgccgaaaaagaacccaacaactgggtctccttatttgggggttcggcctggacttataacccggcgacagacgaatattattatcatctgtttgccaagcaacagcccgaccttaactgggaaaatcccaaggttcacgaagcggtcaaacaaattattgactggtgggccaaacacggcgttgacggtttccgattggacgccatttctcacttaaagaaaaatcaatcgtttgccaacgtccaggatcaagaagcagccatgaataacgttccaggcatcgacaagtttctcagtgaactcagtgctgattttaaacgggaccacctcatgaccgtgggtgaagctggtggcgttccagtcacccgcgcccaggaatgggtaaacagcaaaaccggctacttcgacatgatcttccagtttgaccacgtcagtttctgggaaaagttcaccgtcggccaaatcgacgtggcaatgctgcgaaaggcgttaaccaactggcagaacggcctcgagggaatcggctggaacgcccttttcctggagaatcacgatttacccagagcagtttcttatttcggcaatgatggcaacctgcgtcagcaaagtgccacggccttggcaatgatgtacttcttgatgaaaggcaccccgttcatttatcaaggccaagaacttggaatgagcaacgtggactttgacaacatcgatcaataccgcgatctggattccaaacgcttttatcaagaggaactggccaagggcgcaaccaaagatgaaacgttgtttaaactccaaaaaaagagtcgcgataacgcccgtacgccaatgcagtgggcgtcaaccggcggcttcagtaatcatcaaccttggatcgaaatgaaccccaaccatcgaaccgtcaatgttgccaacgaacaagccgatccacaatcagtcctcagtttttacaagcggttgattgctcttagactaagcgatccaattttactgactggtaagtatcacttaaccgacacgcacgatcatcaactttatgtttacatccgcgaatctggtcaccaaggctacctggttatcaccaatttgagtgatacgccggcaagttaccagattacctcggattatcggaacctcgagttaattctcactaacagttcggctgaacagaatcccgccgccatgaagctccagccctggtcagcctacctttacaaatacgaaaggaaataacccatgaaattaaacaatcaagcaatgctcattacctatcccgatagtttgggaaataatatcaaagatttgcaaaaagtcttgtcaacatacctggacggtgtcgttggtggtgttcacctgctgccattcttcccgtcatctggtgatcgcggtttcgcaccgatggattataccaaagtggacgaaaaatttggcaattgggacgacgtgaaaaagctgtccgagtcatactatttaatgtttgacttcatggtcaaccatatttcgaaacaatccaaatactttaaagatttccaagctaaccacaatcagtctgcttatcgggatctgttcatccactggaatgaattttggcccaagggtcgtccaactcaagaagatgttgatttaatttataagcgcaagccaaaggcccctgttcaaacggtcaaatttgccgatggtcagaccgaagatgtctggaacacctttggtgaggatcagatcgatctgaatgtgacttccaaggtaaccaaacagttcatcaaagataccttgaacttcttgatggaccatggtgcttctatcattcgcctggatgccttcgcttacgccattaagaaactcggcaccaacgatttcttcgtagaaccggaaatttgggatctactgaaagaaatcagtgacatcactagtccacgtgagaccaccttattgcccgagatccatgaaaactaccatattgtccgaaagattaccgaccatgattacttcagctatgactttgccttaccaattgtcactttgtatagtctttactcaggcaaagcaagtcgcttggccggctggcttaagaacagtccgatgaaacagttcacgactttggatacccacgatggcattggtgttgtggatgccaaagatattctatcggacgaggaactggattacaccaaagctgaaatgtataaagtcggcgccaacgtcaaaaaggtttattccagtactgcttaccataaccttgacgtttaccagatcaataccacatactactcagctctaggggataacgatcacgcttacctgcttgcccgcgccattcaagtctttgcaccagggattcctcaggtttactatgtcggcctgcttgccggtaagaacgatctgggcttgctggaaaagaccaaggaaggccgcaatatcaaccgtcactattactcattggatgaagtggctgaagaaaccaaacggccagtcgtcaaagcattgtttgatctcctccgtttccgtaatcagagctcggcgtttgatttggaaggtggaattgacgtccaacagaatggtgacaatgaaattgtggttacccgccgatccgaagatggtcagacttccgcaactttgtccgctaacttgcagacccaagcctttaccattacggaaaccaattctgaaggcgagactaaagaaatattaaccagtaatttgtcagcagttaaataagcacacacactgaaaagaggattaaaaatgaaaatgacacaaacattgcctgcgggttcccaatcactcacaaatgatgaacacattaccaacaaagaacgtttaagctatggagcatcggactttgcctgcaatatcgccaacggtatggtcggcacctacttgatgtactactacacggatgttttcggcttagctgccggggcaatcggaaccctgttttttatcgctagaatcgtcgatgcaatttccggtccaacctggggcattatgattgatcgcacccatacacgttggggtaaaagtcgccccttcttcttatggttctccattccatacgccatcttcttcattctggcattctcgtccgttccactaggaccactgggcaagttggtttgggcatacgtcacctatattgcaattgatattttatatttgggaatcaacattcaaattacttcaatgctgcccagtctgaccgccaatccacaggaacgggttcgattcagtactgttcggcaagtgttagctaccactggggctacgttaatctcaatcatggtcctgccggcagtctcgctgcttggtcaaggtaatgacaaaaaaggtttcttgattaccgcgattttggtcgcaattctgactgcgttcttattgttgttaacgttcaaaaacacacgtgagcgtgtccatccccgtcaccaagaaaagctctccctcaaggagtctgctcgggcgcttaagggcaactggccttggatgattatttccttaatgtatttcttcttctggatcgggatgcaaaccaagcttcaagtaacggtttatttctttaaatacaatatgcacaatgcggacttagcttcgttcatgctcggtctgcaggcactctcgctggttgtgattgtctttacgccatttttaactcgccactttggcaaaaaaggcacgatggtaattggtcttggcctttgcgtcatcagtcaattagttcttggcgtcggtgctaagatgatgaacgtccccattctggcgggcgcgacgattctcgggtactttggtaacggcttcttcgctggactgctgccagttatgcttgccgataccgttgattacggcgaatggaaaaacggtgttcgagctgagggtctggttacgtcattctccggaattgcctccaaccttggcatgggaatgggtggtgtcgtcactgggttcttgctcagcatgaacggctacgttgccaaccacgcccagactgcacaagccttaaatgccattgagatgaacttcgtttgggtaccattcattggatttggtattggattaatcttgatgtacttctacaaattcgataaaatgcaaccgcaaatcgaagcagacctcaaggcacgacatgaagctgcttaaaccacaacttaccatttgaattaataaaggacccctgaagttagtgtacagatgctagcttcgggggttctttgactgttacaaatatgcttgataacccaagataattgccaagacaaccgcaaatatccccactgcggttttgataactttagatggaatataccgcacgatgatcggtccaatgtagccaccggtaaataaccccagcaacaaggggataatcactgcccagtcgattggaatcgtgaagataaacatggttgctgccacgatattattcataaacgaagcaaaattgcgcattgaattataaatggcatagttttcatgaacaatttttgaaagcaccgcaatcattaacaatccggatgccgcaccaaaataaccggtatagattcctaccaggaaagtacttacccagcttacaacggtaataattcggctatcaaatgccgatttgccatggcgtttaggcgtcaagatcagaattccggcaaacatgatgaaaactggaactaattttttgaaaccgctattggtgctatgaattaaaatgagcgcacctaaaacgccgcctaaagtatttaaaatcgcaatttgaaacgcctgtttccagtgaccatgcagctccctcaacgaggaggtcacggttcccagtccgccgccgacttgggcaacggtaatcgttgcgttggcagtaatcggtgccacgccaaccgacagtaataccggatacaaggtcaacgatgccatccccacaattcccgttaagactcccgctaagagactcatgagcaccaaataaataattgaaagcatacttttcctttcgcatcacaggcaccgtggtttttggctacgcctgcacataccaatatttgacttaagaataacattctggggttggaattcaaacgttaacgcggcttctggctgtcgatacttatgtaccagggaagcagctcgccggctacttctctgacaattcattaataactcacatgaacatactttggactagccgtcacgtagccaccctttacttggaaacgttgacttccagtgaccctcagagaataaggatgggcataaacaactttgttgactttgagaatggtgcccgttttgagctgtttaacatgtttatcgaagttggtgttgctataaagataagtggctttaacaatcttcactttctttggttgctgatatttttcagccgtgaccattttacgattaccggtgacatagtggccatttgaaagcaggtatcgggttgtcagatggtatttgatgaatcccttaactttcaatttagtcccttgcttcaaatttttaaccttcccggtcaagttcttgtgcgtgtattcgttgactccagttgggttaatgaccgtcagctgttggtgattgctttggtaataaactggacgaacgaatgcccaatcgctagtaatgtagccagtcttgccagctgttgtgctgtgatggttgacgtctcggacagcgtacacaatctggccgttacttgccttcacctgtttggttaccacaaacatcggccgattaattcgtggcttcttggtataggtggcgattcggtcacgtgactgcatgtctttgtccttgtacaagttgatcgttttcactgcgtatacagcttgattcttttgtgctaggggatgatctggggttggaattgcaccgggttgcgaaactgcggtggttggactctctgcggcccctatcgattcacttgagcgatttggtgttggggtagtttggggatttgttggccgtggttgactgggtttcaccggtggaacgactggaatctcaggctgtttaacaactttgacaaacgcacctaagtcgtacccacccagtcgatgaattggctctggattggtggcgttctctcccaagccatcattctgctgagcttcatagtgcataatgaccgtaaattgatttggggtgtcggcaggctttggcaaatctgtcatctgtcgtttgttctgatcgttcttaaccttggcaacagtgacatccgtgtcgtttgccaacacatccacatcaacatggtcggggttaatttgttcaactccggcaatcttgaatgaggcattaattgtctttgttaaagctgcccatgtcagtggatccttggtcaccacatctaccgggagcaaatctttagaaacaagaactaaatggttctcgtcaggaccggttggaatctggaattgatcaccaaaggctcttgcactcatttcaatgtccgcctggccaagtgagatgctcgtcaatcggttttccgaaaatgccccagtcgcaagttgggttgccttgggcaaatcaactcgtgtcagtttattgttggtaaatgcccacttgccaacagtttgaacattaggcagtgacacgctggtcagttcgttacccgtaaatgattcgtcgccaattgtggtcactccaggcaagtcaatgctggtcaactgattgccatagaaggcattataatcaattgtcttaatctggtttggcgcttcaaacgtgaccgctttgatcccgcgatattctggaatcccaactcctgcttcgtcaatatctccaactgtcgataaattgtcggtagagaatgcgtctgggccaatgccagttactgtttcaccttgcagtgttgctggaactaccaaatgaccaccttgaagcaattgacgggccaaatcctcattttcgacatctgtaatgatcccgtcctctatggaaacatcatcgtcagttaaagtaattgtctgattttgttgcatcggtaccttttcaatcttaggtcctgcagagtcaatcgtatctgctttgaccgcaataccgctgattccgaataggagtgttgttaaaaagctgatataaataagtctgctcgtcttcatattggggacctcctcatcaatcctgtcatctctttacacctgtattttaacacgtatgattataattactataaatattgtcttatagttaatgccattataatcattaaatcagctaaattcattcatttttggcaataaaaatgggccatttgtctagtcccggcaaatggtcccagtatgctaactattgaattgtttctgtgattgcttccttcatggcttgtgtactcaactcctgcccaattcccggtcgatcaggaattgtgaaccagccattcttaggctcgacgtgatatttaccggaatcgatattgggctgcttcaaggaaatctcatggtactcatgaatcagagtgttgggcaatactgcctccagctgtaatgcggcagccgttgcaatcggactaccacacacgtgaaattgaatactgacatcgtcaattgccgccagatcgctgatctttttagcttcggtaatcccaccacagatgccaacgtcgggctgaatcacactcagtgatcgttcatcaagaaatggcttgaacccatatcgagttactaatcgctcaccacttgctaagggaatagaaacattatttcggatttctttggttagctggggattcatcggtgagttgggctcttccatatagtaaatgctcaggggctcaaccttagcggcaaacttaatggctgaatcgacgttcaatcgagcgtggcattccaaaattatatcaacattctctcccacggcttggcgaacagccgcaatccgatcataatacatttgaatttgtgcctgggttagcagttgctggtcatgcacaccaaatgttccatctgcctgcatcataaatggatcaactttgagggccgtataaccttcttgaacagctttttctgctgcttgagcataatcctttggtgtcgccaggaattcaacatgcttgccccagccgaactgaatttgactggcgtaagctcgaattcggttttgggtttgaccacccagcagctgatacacaggggcatgaaagtatttgcctttaatatcccaaagagcggtatcaatggcactcacagctgaataaaagacaaccccaccgccttttccccaaaacgtatcttgatagagttcattccagatggcttcattccgcaatggatcttggccgatcactcgatgggccaaatctttcagactgccgacagctcccaaaccgccactgccatatgccagtccagcttcaccaaatcctgagatgccggcatccgtattaattcgaatcacaactggatgccaatctggcatgagtccaaaccactgcaattgaaagatatcaacgctgataattttcataaagcaccccttttcagcctttaaaactgatcatcatgtgagcgatccaacatgatctcggccaatcgtttcggtggaagcggcccgatgctggtcgtcaaatcagcccttgcaaaggcatccgtgagggctgataaattgaattcagtcccatccaaccgctcggtaatggcatgaagatttgaatttggttgtaagaaatccccataaatttgcgaatcaaccacgtggttgtcttgaatcgagaacccgattccgaccgttccaataccgttaaaataaccatctctgtaatattgatgttgattgccagcgccaaaaatccaggtcttgctgccatatttagtatgagccaacgaaacaattgcctgccaatctttctcagtcaatcgataggttggaacttgcgccagattagttgtttgaaacacttgggtcaaaattgtttgttgaacttgatcgattgaaactgttcgatgggcagcatcaaagtgctcgcggagatttgtcacccgactgtgaaccgattgaacgcctttagccctcaactttgcccgtgatggtttcaacactgagctggcagcctcgatatcgacatcaatcatcagcgtgccgccataggacacccgatgaccaattttggaagctgacatcccggaaaacttgcggccatcaactgttaaatcatttcgactgtcactctccgcattgacgcccagggactgcaacgctttaacgactggttgggcgtattttctgaaatggggatgttggacagttggctcagtatcaataaaaacgtacgtcagatttccgggatcaacgtagacggctccaccaccagaacctcggcgaaccaaatcaatcccgtgggcctggagataagccatgttcacctcggcaaaaacgttctgatgaacgccacaaatgacaattggcgtttgcgggtggtagaaatacaccagtgcatctgaaaacttcgccgttgtctgcaggtattccggaaaggcctgttcaaccgttgggtccttcaaatatttcaatccattggatgtatctagataatgaataatgatcccttctttgagactacttcttaatatacatatatttataattccattgtgaccccgttgtattgtgggtaatgccgtgcaaataaggtcgtttcagatataagttgtaattctggaataaaggtgtggccccttgatcctgcatgataatcttctcagctgccaacatcttgttccaacgaatcgatgggttggcgttgttggtataaattgactggctgatcagctgatcaaattttgcattatgccatgagccatagttcattgaattcttgctcatcatcggctgcagaaaggcggttggatcagcaatgtcagctccgcgaccggtaatgtacgcttcaaaatcgccggaaactccgcgggcatactgaacttcttgaggaaccgtctgaagattaatcgttaatccaggaagttgtttctcagcggatgatttgataaattcactcactttcttcacgttatctgaattggcaaccatgaggttaaaggccagcttcttttgaccaatttgttttaatcctttgttccaataatccttggccaacttaggattataggcaaccccttcaccgccatattgttgagaagcaaagtccttattgttggccggatcataagccaaatatttggtaacaaatccagttggcttcagtgattcgcctttcaagaggttgttggcaatctggctgcgatcaatcgttaatgaaacggctttgcggatatccacattattaaaagctttccgcaaggttggattcttgatcttttggttataaaccaaatagttcatgtatgagtacggaccgtggtataggtcggcactattcttataatgcgtgacctgatcgccaattaaaattgtaaaatcaagtttgtgtgcctgatataacgacaaactggtctgtggatcagtcacataattcatatgaattgtgttcatcttgacatgctttttgtcccagtagtttggattctttttaaatgtccaagtattggattgtggggcccattttttgatgacatatggcccggaaaaaacggccttattggcagcttggccatagctggcgccgtatttgtcaacgatctttttgtcttgtggtgaaaaggcctgataggtcatcaatttagtgaagtaggcaatcggccgatccaaatgaacaacaaacgttcgcttattcggtgccgcaacgcccagcgcgcttagcggcagtttcccaaagttgaccttttcggcattcttcacgccatcaaacagataggcatgggtggacttggtcttgggattcaacgtccgttgccacgaatagacaaagctgtcagctgtaattggatccccattactaaacttggcgttctttcgaattgtgaaagtataagtcttaccggcattggacacacgatactgacttgccaacgccggaaccggcttatgattcctattcatgtacaacaaactatcatagagattaccggcgttatcgaagccctgggcttttgaaatatccagggtcacgattgaatagttcgccgacaagttggccgttcgaaccaacttgctgttgtcttttgacttagtctggctcgaacaagccgctagtgtccccacactcaaaacacctgctgctaaaaggagcaaatttctcaaataatggatcatattcttaacaccattcccttcaaataatcctgttaccgcttacaagaggtccccaaaataagttcaaaggacaggtgaccaaggggagaaggtcgctggctttgaacttttaacacgtgaatatcttacaacaggtttaccacataaatcaaggacaaattttggtacaaaaataccacacaaagaattatttgtgtggtatcatatttttatctcattttacgattcttctcgaatcactggtttttcctttaagctcaattgctccacgttcaagactttatcaaccaatccatcatagaagctggactcatggctgacaataattaagttaccggggaaccggtccaaagctcgcttcaaggcctctttagtctcttcatccaaatgattggtgggctcatccataatcaggaagttggtcggggtgaactccatcatggccaatttgaccttggtttgttcacctccggaaagttccccaattggtttaatggcattggcagcatccagaccgcatttggcaagcttggtccggattgcccgttggtttaatttaggaaatttatccgaaataatctgcatcggcgtcatccggttgttatcccattccagttcctggctgaaataactgatgtgagatgatggcgagaatttggccgttccacctttggcaggcagttgaccgaggattgatttgatcaaagttgacttaccaaccccgttaaaccctgcaaagccaaacttctctcccattgaaatggtgaaggtaaccggcttaagtaatggcttattgtaaccaaccgacaaatgatcgacggtcaaggcttcatgagaaccggtttcttcatagggaaaattgaagctggccttgatattagtcgaaggcggatcaattttatccatatgggccagtttcttctcccgcgatttggccatcgtggacttggaacccgccttgttcttacggataaagcgctcagctttctcgatttcgacctgctgcttatcgtactcacgctgttggaattcttctctctcagcccgttgacgcatcgcttgtttgaaactaccacgatatttggtaatcttcccaaaagcaacgttgatgatacagttagtgattttttccaagaaatcataatcatgtgagacgaccagtgcagaaccggtaaacccattcaaatagtcgatcaaccagtcgatttgagcggtgtccagatagttggttggctcatcgagtaaaatgacgtcgggatctgccaacaacattttggcaaggatgatcttggaacgctgaccacctgacatctggccaaccaggtgatcgcgaccaatgttatctaatcccaagccggtaatcgtctgttcaattctggtgtcaatgttatagaaatcgctggaatccaagatgtcctgaagtttcccagcccgctccaacaatttatcatcggccgtcttagcataggtattataaagttcattcaattggtcactagttttgtataaatcagcaaatgccgtgcgcaaaaagtcgatcagggttaaatcttcctcaacatcggcatactggtccaaataaccaattttaatgtttttctgccactttatgtccccagaaagaggcagttcacttccggtaatgatcttgatgagcgttgatttaccaaccccattttgacccaccacgcccatgtgctcgcctttttcaagcgtaaattcagcatctttgtacagatccttctcagcaaagctcattgaaagatttgatacggatagtaatggcaaaaaagttcactccttaattaattcgaaatactacatacaatttgttacgttactcttgtttcctatagtagtcaaactaatcgtgcgaagatttcgctttggtatataatggaaacattacttttaaaggatgatcataaatgaatatcagagaaattgaatacattacaatccccgtctccaacctggaagtcagcctcagattttaccacgaggtctttgacctgcaaattgttgatttacccaacggtgataagggagcggacatgcacaaaatgttccttgacttccacgaggaagacaaggtcgacaacccaatctcatttggcttgattgctaaagacaaaatggccgatatcaaagcccatttgattaactactttgtggatatcgtgagtgaaccgaccgaaaaaactgaagtaaggagaaacgttaattcgatcacgattttagatcctgacaagaatcggatcgaagttaacgagttcagataaatgaatccaaccaggtatctcatcactaaatcaacgcaaattttaaaattcgtggggtttctggcaacttatattgtagcggaatcagtttttgaaattgccggtcaatacatcaaagaccctctgagtgctcgtcaccttctgggactggcactggttttgattgccggggccctggctttgatcggttggcgttatggtaagcagctcgctgctaacaatccacggcattttggccgacggcatccgactgccaagcggatcgcccaactgttatggatttttattttgatgacggctatccagatactttggcagtggctcattgccaaccacgtcttgactacacccagcaatcaacaggctgtcgaagccgccgaagtcaagatgcccatgtggaacatcttttttggcgggattctcgcaccgatttttgaggagcttatttttcgtggcatcttcatgaattatttcttcaataaagataaccggctgaacaatcttttggcagtcatcgtcagcggctcgctgtttgggtttgcccatgagatgagctttgacctgacttggatcatgtattccgccctcggctgctgcttatcgtttgcctacatgcatttccgtgatattcgttatagtatcgcacttcatatgatgaacaatttgattccataggatgagaatatgaaccgcactatttagtcataaaaccaaatcacaattaaaacagagatcgggacacagctcacaatgagctatgcctcgacctccgttgagatccactgttatctagtttaaacgtggaacgatcggccgctcccggccatttaagcaaaaaatcgagttattccaagaacaggaataactcgattttttgcttaaattctgggatcaaaacgccttgcgttccactctatttaattagaatgattcaacttttccttagctgctttaggcacctgtgaataaggaattccctcatagtcaacgacattcttcgatcttgagtaaccaatcttgatatagtgacctttgacgaaatacttaccgtcaaccgagcccacttcaagggtcttaccctgacctttgtcattgtaagccttaatcaaatagtaatgaacatccgggttattgccgggcgaattctcagttcgttccaatttgccaacttggccatagtaaaagattctcgcataattgtgatgataccagataccgccaattgcaccaagcacaacaagaaccgccaaaatgataattgttcttttcttcatggtcgatctccctcatattctgtctatggacaaactatatctaatcccaaccagcctgtcaatcaatttgccaggtcactatttaggcatcatttcttccaaataacgttccagacgtggatcgtgggcgtgcagatacatccctttaatcccccgcctcagcaaaacgttcaatgaatttcttaacagttcaactttactttcttcataatcttttttcgacatgtcggaacgatgcttgaagatctccacgtcagtgactttgctgggatcgacgcccagacggttatcggcagttaaataaaacggcggcccaatgataatcccaatgtagttcagatcaaacccctgaaccgtgtaaatgctgccgacctcgtcaatcgtttgtggctgctcagcccatggggtactggtgaaattatattgatcccaaggtagatgaaagttgccttcgttgaccaaatgtttcccaccatccaaggttgagggatagccactggttgacgtcattcgcgataagccatactggtcgtttttcttgatgatcgtttgaaacatcttttcagcatcggcaaaaatacgaaagtcatagtcgccaacgtcactgggaatcgcgggtataacatccccgtcaataaagtgatccagccaattcatcagcttcgggccggcctgcattctaaactgctgcttaagatgcactaaatcgtgaggatatggggcgatcaatttttccaatctggctttattccaaaagctcttggttcgcaacacttgatgcggatcaaaaacaacaatcgtcacccggcttaaattgatgatgtcctggagctgattgtcaccatagtagttattgtagtgatccggcttgctcagcaacaaatgggcctcatcgacaaccgtcaaattgacctgtttgccctgcttatgcatctgattgataaagctcgtcggccgctgatagtactttttcagcatgtgtggggtttgcccagccaactcgcgatacacttttaggagttcgggatgattgaccagaaaataggcatcgtcaacgacttgggccaactcggtaaacagttgattcaagatcaaacttttgccggtcccggcatcccccatcaaaacaaacaccgcgtgcccgtcttcttttaaatgttggcgagaaaaggcgtcaatttgctttaaaacagctttctggtggtcagtcagttcaatatttttcgaaaatgcatttaaggtgtgcgattccaaagattccattgggttactccttctctcaaagctcataatatcatgataacttttcgccgttttaatttccagaaagatcaagcttgcaatcgctaccaattatcatgaataatagagacaaacaaatcagcgaggagaatcagcatgccaactttcattaatggaaaaatattcactggaattgaccagacgacttttgtttcagcgatgacaattgaagatggtcacgtcacttggattggtgaatccgacgagatcaatgattccgagacaattgacctgcacggcaaaacggtcttaccaggattgatcgacgtccacacccatcccaaatatattgccgacgctctgcatggggttgcctgcacaccgcccaacgtcaatagcatcaaagacatgcaagctgccctacgtcaatcaccggcctttggaaaaggcccagacacttggatcgagggctggggctttgatgaaaccaaattagccgagcaccggacgccaactgtcgatgatctggatgaaatttccaccacacagccgatttttgtttatcggtcagattgccactcatcaatcggtaattccaaagcgctggaactggcggggatcactgcaacgaccccggatccggttggcggcttcattggccattttgatgacggccggccgaatggttacatgaaggaagtcgccgctacccagttgttaatcaaggcgaaatcagcccaaagttatcagggcgatgtcgataatatggcgaacagctccagacattatctccaaaacggcattgtcgccatcggtgaaatgatggggcgcattcgcccgtatgattcgctcaaactttaccaagatgctgtcaaggccggtttcaaaccaaagtcatccatttactacgtctacgatgaagtagccggcaatacccacctgcaaccgacgaatgatgatcagttgcgggttgcaggcatcaaggtcttcatggacggcagtatttccggtgaaaccgcctataatcaacaaccttatccgagcggccaaaatggagtctgcctgacggacgcaaccaaactcaagcaagctgtcacctatgccaaacagcagcatctccaagttgccatccatgcgatgggcgacgcagcgatccaattgattttggatgtgactgataaactgcaaccgtggctatccgaccggccgtcaatcagaatcgagcatgcttccattctgagcaatcaaatgcttaaacaaatcaacatggcaaccatgaactacgccctggtgacccaaccgattttcttctttgccgaggatgaatcgtaccgtcactatctttccccgcagcagttcaatgaagcctaccgtgtgaaatcaatgatgaacaccaaagccgagtttgccctgagctccgatgccccctgcacaccatgggctgaaccggatagcccatttgtgaacatttacgccgcagtcactcgaaccgcggtcaatggtgacgttgttaatcctgaagaagccattacggttcccgatgcagtgcttgcctacaccagttggccggctaggattggcggttttagtgataacggccagctgactcctggatatgccggggattttgttgtgcttgaccgggatattttctccgtaccgcatgaggagttgaaagatattcgggttgctgagacttggatgggtggagaacaggtgtattaggacacaaaaaaggcactcagctgagtgtctttttttatggggttttaacagggtgctcacagatttagaaaatcttgcttattctttaggtttaccgctttcgtcacattcaccagcttgaacaggattttctttcttcaaagcaaatgctgcaaagacagtaacaacagctacaatggcaccaagaatcaggtatgtttgatggaaaccaattgcatcgtataagttaccggcaacacttgagaagatgaagactgatatttgcttggcaaagttcgacgctaaggcatacacagttgcgtatacaccaatatcgaaggcaccagcaatatacttcataattgatacaagaaccaatggcatttcaagtccggctaagagtcgaagaacaatgacccaaatcaaacttggcgacaatgcactaccaatgatccgaatagctaagatacagccataagcgatcaaaccatttcgtgaaccaatccggttgataatccatggcattgggaacatgagcaggaattccagaccaatttgagcagtggtcatgtaactatatgcttgagttccttgagctgcagtattaaagaatgtcttgaagaagatgatgaactgttgatcaaagacatcgtaaatggctgaagccccaatgtagaagattgataggtaccagaagttcttaattttaaagatcttaccgatttgaccccagtcaatcttgtctgaagtgttaccagctgcagatgcattttccaagtgaactttatcactgaagatcagtagtccagttaggataattgctgaaacggtacatgcccagaagattgagtatggtttccagatgaacaattgtccgcccaggaatgaagcacacatcccggctaaggagccacccattcgtgagtgaccatattcaaatccgtttgccaaacttgcacgttgaacatactgctcaattactgaaacaccaccgttgaagatgaaactaaggaagataccagtaataacggctgcaaacatattgcttatgtgagcaaatggtataaacagccactggaagtatggtccaataaagattgcggcgatcgcaattgtgataattaagttctttttaaataatagcttatctgaaataacaccaaatgctggttggaacagtaatgacattccggccatcattgagaatacaactccggcttctgccccatttaaatgggcaacttgttccagccaaagggttaaataaccattaataatttgccagttaaagaagtaggtaaaatgagtaaatggaaagccccaaaaatccttcttctctttcttttcaggcatttttgcactgttatccataacatgtgcctcctattaaaatttattaatcataattataaggaacaggcttgccaaagttaggcgtcccgtcttcgttccaagtaaatggctgaaccttggtgtgacggttcggatcatacagtggatcacccttaatttcagtgtaatcacggcaatggtaaaccaaaatatctgtcttgccatcttccccaaccgtaaaggagttgtggccaggtccgtattgatgggttgccatatcactttggaaaaccggcttcttggacttggtccagttgcttgcgtccaacaaatcttgatcatccgggatacttaacatccccattgcgtagtgttcatcggtggcactggcagaatacgtcaggaagaagcggccattgcgatggataacagctggtccttcattaacccaaaaaccaatcgtttcccagtcaaattcaggttttgacagcatgactggcttcgttttgaacgtccatgggttttccatttcagcaatgtacaagttggaattacccttgatgtcaggatctttttgagcccacacatagtacaacatgtcattcgcctcaaaacaggttgcgtcaagcgagaaactatccatgcctgtcttcacttgaccgtgttcgaaccaatcgtcttcgctgcgcattggatcagcattgtcacattcaatacagaacattctgtgttggaacatgccgttcttatccaaggctgtggtttctgcagcagcaaagtagatgaaccacttgccatcaatgtaatgaatctccggtgcccaaatcaattgactcatgggaccgctttcatgtttccgccaaattgtccgcggagctgcatgggcaagtccttccaatgttttggcacgacgaatttcaattaggttatatgccggtacagaggcagtaaagtaatagtatccgtctgtgtgtttgtagatgtatggatcagcccgctgaacaatgagcggattcgtataaactgtcaaagtaaactcctcttttcttgattgactacgtagtattgatatcccttgtgcacatctttatgatatttcttcagtaaagcggttacaagccataacataaatgttcaattaacttttgacttaaaaccgtggttttgctaatataaagacgattagtaaccggttacaaaaataagattaacatttatattgatttaaacgtttttactgctaatcaatcaataaatgttaattggttgatttagtcagattgagagtgaggtcacaaagatggatttagatatttctcaagattcgcttgaggtatataaagccttggcaagtccagttcgaattcaaattatccaaacactttcatcaaagcggatgagtgttcaagaattgtcaaaaaaattaaaattaagcagcaccattatcctgatgcatctgagtaagctggaagatgccggaatcatcggatttgaacgtgaaggtcacagtaaaatttcctacttaaaagttgataatatcaacgtccactttccgacgaccatttatcccgcgtttgcagaatatgagacacaagtccctgtcggtcaattcactgattactcagtaaccccttcgtgcggtctggctggtaaaaatgactatattggcaaggtcgacaatcccaagtactttatgagccctgagcggattaaggctggaatgatttggtggacgaacggcttcgtggaataccagttcccgaactacttagaagaaaaggacaaactggaaatgttggatttgtccatggaactcgggtcggaattccctttctccaacaatgtctggccttctgacattacgttttacatcaatgatgttgaaattggtacgtggaccagtccaggtgacttttccgatattcggggtaagtacacgcccgcgtgggttcccgacaacgttaaccaatatggtcagcttaaagtggttcgcatcaccgatcatggtagttatctggacggtcaaccctttaccgacatttccattgatgacattgattggaagaagccaacgttcacggttagatttgcgattaaagatagtgcgaagcacaaaggtggctgcaccatttttggtcaaggatttggcaattatgatcaagatattcaaatgaagctatttcacagttaataatatatagaatggatggcgagatttaatggaatttgaggatcgaatgcgggaatttatcttaagctttttagacacgcagcctaaccatgttgatctaaagacagtccagaaactgatcgattatggtaagaacaacaaatatactgcgccaatgctattaactcagctcaatcaaatggacgatgctcacgaaaaagtcctgacagtcacctttgacgttgattttattgatggtgtcaagctcttcaataatcatgcaaccaagtggttgacggacaaaggaaaagcctatattcaggaattaaaacgtgcccaaaacaaagccgaaacaattgattttccaaaggacgatacccaaactgaaagtaccgaatttgatggttatttatctcaactgatgtcggtcggaaaatcaatgaaaagccagtcggaacgcctgaccctgcaagaatttgctttagagttgaggcatttattaactgacacgaaaaagctggacaaaggtgccctcaacaaattcaaacccttcgtcgatcgcaactggaacgagctttcaaccccaatgacgccgatcttggtcgaattatcaaggcgctttctgatcgaaaatagttatgatgattaaataggactaactaaaacgagcaccaaactcaaccaatcgctgagtttgatgctcgtttaatatctacttaaggtagaaaatctattataaagactgaagccattcaagacacaatgggaaccacttggcaaagtgttcatcggtccggtcgcgattaacgacgccgacaaattggttggctaggctgaagccatgaccgccagtggcaaattcatggacttcaaagttaacattattcttaaacagtgcttcggtgtatggatagatgtggtcgatgtatggtgccaagccatcgcttctagcaccaaaaagaaatgttggtggtgtgtttttggtaacttgcttggtaacatcttcactgtgaatcccaattttttcatcaagggcctgtgttaatacagggtagcccaagatggcaaacttagctttggtatccttctgattggaatatgctgcggcaagttggccaccggcagagaagccgattacccctaatttgtcggtgtcgacattcaaatctttggcatggtctgtgatataatcaaaggccatggagatgctttgcttggcatcttgataatttttcttttcgttaactggatactccacaacgaatgcctggtaacctttggttaaaaaggtcagggcaacccgggcagcatcacgttctttaaatgttttgtaactaccaccggggattaccacgattccaggcagtgcaacgtcactatcagcatcgtaaatgtctaatttaatctctttgtctttatcaaatacaacttgtttaaaattcatacaatcacctcttcttctatgataagtggtgaccggcaaaattgctattgaaaaaacaatttattattggtgatttccttgatacacgtggggttgaccctcacattggaatattttatttgcttattgcaattttttataaccttcaaaagtattttgtcgtataattagaaagttaatagtaggtatattattataggtacggggaacggtacctataataattcgaatggttcgtaaatatcaattttctggggagaaaattcaatgattaatttctttaataaacacatcaagctgttctttgcggccttcgttgtggcatcaatttcgtttggaatttatagccaccccaccgcagacaaagcaagtgttcaagttgaatacacaacgcaaacgcatccgcatgcctttgcgctgaagaagaatgccaagctgtacacggatgttcatttggctaaatcagtcagcgccaagaagtttttgaagacggcctggtatcggagtcaagctgccaaattgatttgtggcggcaagagcaagatcgtctatcggatcagcagtgccaaccaaaagtacaaattctgggtattgaattcagctgttaccgatattacgtcgaaatcatataacgtcaaattggcttctgccggtaataaatacgctggcgaaaagatcggcgtctttggtgattcaattcctgcaggttgggacggctatcacttctatttaaacagttcttaccctgactggacagccaagtatctcggcaccaacaccgccgttgaaaacttcgcctgcccgagcggccgaattgttggcaatcggtatgcttatctgggaacaaccttggttccacaggatttgtcagctgcaatcaaggcccaccgaaatgacatcaagaagatgaacgtcatcttcgttcatatcgggaccaatgattacaccaactattccggttcgggaagtttgaagaatgtgatgcgccacctgcgctacaacattaagctgattcaaaagttgaatccgtccgccaagatttacggtatcctaccaatttcacggtttgacgccaatggcatgaatcgtgacaacatgagtgatatgtatggctacacctaccacgacttgcgggcagctgaagcaaggctctacaagtcaatgggcgccaaagtggtcaacttccaacagatcgcacccaacattatcaccgacagcaacaaggacatcactttgaaggatcatgagattcatccaactgcccaaacagctcagaagctggggtatgcgttggctaagtcgattgttaaataaataaacacaataagttccctgcttagcaaatactaggcggagaacttattttttgtggtggaagatgatccagaatgaatgatctgttgagaaaccatctctaaccttattgatttaacatccttctaaaacaattacgtggcatgacattcgtttagaaacgggtttaaccttattgatttaacatccttctaaaaccgtccacttgagaatcatccagcccgccgagggtttaaccttattgatttaacatccttctaaaacatgacggctggcaacctaagccaccttatggggtttaaccttattgatttaacatccttctaaaacgctgaaccagcaacatctgcaacaacgaatgggtttaaccttattgatttaacatccttctaaaactgtgatctcacgtgtttcgatcttgtaatagggtttaaccttattgatttaacatccttctaaaactcgtaatcttgccgacagctgtgccaatttgggtttaaccttattgatttaacatccttctaaaaccatgtggatgcaagatgtgtggtacattttgggtttaaccttattgatttaacatccttctaaaacaaagtaaagggttaatcaaatactcaagtggggtttaaccttattgatttaacatccttctaaaacccaacgttgatgagaacccgggcgaataccgggtttaaccttattgatttaacatccttctaaaacctaagcaactagagaaaattgatggcaggggggtttaaccttattgatttaacatccttctaaaacacggccccaacttgcttaacgccagaaagagggtttaaccttattgatttaacatccttctaaaacacctcgcagaggattatggcaacgggtaaagggtttaaccttattgatttaacatccttctaaaacttggctttagtttaggtgtcttttgatgaagggtttaaccttattgatttaacatccttctaaaacggagtaccccacgaattaatggtattaatagggtttaaccttattgatttaacatccttctaaaactactaaaccggttaaagcttcgtatattttgggtttaaccttattgatttaacatccttctaaaacggcgtgttatacgattagacaagtatgttagggtttaaccttattgatttaacatccttctaaaacccttgcacaaagcggccgccacctttttccgggtttaaccttattgatttaacatccttctaaaacattactttcgtaataagtccccacggtattgggtttaaccttattgatttaacatccttctaaaacagaacacggtgctcaaaagtttagcgaactgggtttaaccttattgatttaacatccttctaaaaccaccaccctcaattcaacatcaaccttatcgggtttaaccttattgatttaacatccttctaaaaccgtcttcatcgtcggtaatatcaattggtggggtttaaccttattgatttaacatccttctaaaacgaatatcatgtttgcttgcaccgctggcaagggtttaaccttattgatttaacatccttctaaaacgtagctacttttaagatcacgaaactcggtgggtttaaccttattgatttaacatccttctaaaactatcgaaaccgttattaacggccatcatgtgggtttaaccttattgatttaacatccttctaaaacctcctttatttagtagattcatttaagtgagggtttaaccttattgatttaacatccttctaaaaccgattttttataaccgaattttaatgcattataaatgccaatcaacaaagtcctcgtcgatgtagtaaaagtcgcaattggtataaagctcctgtgacttcatatctgtgaattctactaataatgtcgagattcccgtggaacttgcgaggttggatagatcaatgaattgctgctgattaagataatgagcgacattagttaaaccaacagccgacttcaatccgcactctaaatgaattttgataattgattcaattatagcataagggttctgcatggcatcggtgttaaagtgaattttacagtatttaaacagcctctttaaatcccaatcataggtgacttccagaggtaaatcgatcataaacaaacactgctggacgaccgtatacaattgattattaatatcagttatcgatttacgctgatcatcagtcaacacagcctctaattgcttaaaaatgccagaattatacttgtcactgacaccatcgctgagtccgacatctccctgccaatcaattacatctttaacttccactaactcaaaattgtcatcaaacacttttaccttgtcactaaaagaactcagtccaacaactagatcatgatagacggttgggttgttagtggcaataaccgtgggattctttgaattcagctcaatttcttgatggccggcatacgaaattttcatagaatgatcgtcctttcagaagaatttcgaacatcttccttgggtttgccggcaataaaatgcatgtcgttatattgcttctcagtcataattaacgattgaatcaacccttcaggaggggcaatggctgcaatccgcttctccataaaatcagcggacttcttgttaacgcagactcttacataaacagaaaactggatcatcaagaagccttcattgatcaaagccttgcgaaacttccgataattccgacgattctcactggtttcaaccggcaaatcaaacattaccattaatcgcattattcggtacctcatttttcaattccacctcaatttgaatttcgtcagtctcaccacttaaatatttcaaacaattccggacgtgttcggaaataatatttcgaaataacatttctttgccattaaatttcatctcaagatttaacaggtccaccaagccaaatttgacatctggcgtcaattctttgaaattttgatttgccagccagtaatcgataacgggccgaaagggctccatcaggtcagatcctaaattgaattgattatcattgctgtgatgatggattcctaagtatgtgaggtaaccattggaaacgatctcccgattaacgttggataacaaaattgaatagccataatttaaggcagcattcaccggcgaaaaatcacgccggctaaacttattatcaaacaacagcgggaaatatttccgtgcaactaccgcctcccgattggtgacgtcatcaatttccaatttatcaagttccgcaatcaaatcactgtttccaacgccataaatcgataaaacattaacctgattgacgattttgcttgcaacaatcctcgtccaaagaaactgctggcgtttctcatcccaacaaaactgtttcttgattaaatcaacgtcccgactatttggataatacccaaccgtttcacaaaccggctcattggcattatcggtaaaaatgattttgacctgacttttcaccagctcactaatcaaagcagtggtaatgactgcctgagtagttgataccaacaataaatcaatatcttcaattggcacttgattgatgccgtccatcgtttggacaatcatatttcgtgatgaatatgacatctttgcgtgctgcgatatgacaactgatcgccatcccataataaaatctcccttgcctcaattactgaattggggtatcattatttttgttgggtagctcccaacatgtttgaccttattgatttaacatcctgtgttaaaatcaagcaaagcgctttgcgcggagtttcaacttttgacccattatatgggcattacataagcgaaaggaaccattcttcagttggagaatggttccttttttgttacaagtccttcagactgacggttctttcgaataaacctgttggtgactgataacgaatctttgcctcatctgacagcagaattccattaggctgttgtaattgaccaaacggcgtggtgatgccgatatcctttaaatttccaaatgttggatttgcatgcaatccattcaatacttcttccaagatctcccgttttccagaagacgccttagtattcccatcaaagacattatgattaggaaatgagatgaatttgctgaaaccaagattcaacttgtgacgaaatttattcatatcatataaagaaaagtactgattaaccttgtctaaaatctcagtgtagacgttattgtaatccatactttcttgcaggggatctaatcttcctttgcttgcaagtgtcttgacagattgatcggagagtaccaactgcttggcgttatattgataggtcgagcttccaagcatgaacttcttatcaccatcaatcatcaattgtcggtacattacttttcctaaaacaatctcaaagtcttcaacgacttgggtgatctctcccgttttccgactcttcttagtcttcgtgagttgtggtgtcaatacatctttgagagcccggtcacagtccgcatcactgacttttttcgcggcgtctaaacgatcccgtgcccgcattggcacaccgacaaccctatatttatcgcccttcttattatgaattctgacaattgccatatacgcatccgcactgccgctatatccaccatagacattaatcggtcgatcagcttttatcggaatcaattttcgtttgccagcatctgatgcgggataaacggtttgattgaacattgcaccgcgaagcgtataaacttcgtgtgaaatcagcatgaatttataatggtaaacatcctttaactgctgaattgaattttcgcggtcccatattacttcaccagtctcggcatcagcgatcttttcttgagtgtcatcagtcagatcatggaggaaattaaaattccgcatggtgactttatcttctttaaacttcttgaaatcaccatagacgaagtatggacgtagcttgatgtatcgatggtacaaatatctacctaaaaaggctgttaagtaggcgtcaaacgcatgatgatagtcattgatctcacgattcttgataaacccaaactcatctctcatctgatggttcatccgggcagtaatttcaataatcttggtattatcattgcgatacttgtctcccaaaatgttcgcgaccagtttgataacttggctggtttcaaccaactgtcgacgaatgaatccatgcatcgcatacttactaatggtatcgggatctgtttgaaggttcttgagtttgcgcttactaatcaagcctgcttcagcaagctgtttccagaagtgccccatcttggcaccaaacaattgaacaggtacattatcagatttgccattgttaatcgccttcgataccaatacacggttgttgagtgaatcatctttgacgaacgcctgtggcaaaatatgatcaatatcataagtactaatttcatcgatgttgattggctttcctgtgtagatatccttcccaagttgcgtgaagtacaagtacaaccgatcagtcaggcccttcttagactttgctgcattgtccagttcagaaagtaactcgggattgattgatttagccaaagatttagcagtatcttttaaggtattttcaagttgccgttgtcgtgaaattgtccgacgtggattacggtcctctgaacgggtaaactcgatggaaatatacttaggcgcaactccgcccatggccttttggatatcatcaacgactttaaccacttggcggatggccttcttattttgtggagaagtgtatgcatctgccaacacatcttccacgtcgactgccttcatttggtcagcattcgcttcgtgaatccgtttggcaaaatcattgtcagactgaatttgcatgaaatttttattggtattccaaagttcgtcaatgattcgttcgccttggtcattgacaattccagttaacagtttcttggaaagccggccccaaccttggtaacgactggattctaaaacatctttttgctgatcagataaccacgtaatttcgttaagcttttcccggaggattcttttgtcctcaaatacagttgaccattcaacaatcttctcgaaatcatcttgaagatctggttcgtcaaccttattaccaaataatttcttgaaatcattgtaggtccccaaagaattgttgaaatactctgggtctgataaacctgaaatctccggatcactgggtaatccagtcttagacttaatgtagttttgcagcttcttgactgagatatgcttgtagttttcgaagagatcctggaatatggcctgtttatcagcaactttcaataatttgccgttaacccggaccatgttcaactcattgaggactttaaacttctcgtaaagtaaactttcgtccggaagaacatcttcaccgattaagtaagtatctttggtggtcattcgtttgatgaatctgttcgcggatgcgttccggtcaaccttttcatcaaaattccaaggggtaatctgcccagcttccttacccttacgctccatccaagaaaaaacagtctctgctgatttggcctggtcgtccggcgttatcattggcccaacataatatgggaccctaaaggcaaccaattcttcaatcttgtattttgcaaggtgaagatcatgcttgtttggattgatctcggcaagccatgggtaatatttgctttgatgttcaatgatttcatcaagttctctttgatgcagttgatgaggaatcacaccattttgtgatgttcgttgctttggcataaatttttctgcatcaatcagatccataatttgctttgaaagatctgaatcatccaaatttttcttgacgctcgaccagaagtcagcttgttcgatgactttaccatcgtcacccacgtattgactatatgccttctttaaggcggctttcttcttcggatcagcgagttgatcaattatctttttatacaacttcaagtggtcatgatgatcattgtacttttcgatcattgattctgataatgacatgccattaggaacaatttgattcaaagttacttgagaatataagttctgtaggatagcaataattgattgttggttttcgtccatttcaggtaaaatcttttgcagtttagcatcaatatcttcctcatcgaatttgagtgcccatgacttggaatctactggcgtacactgtacgacaacgtcgagttttgatttgtaacctaaaatggcattaataatttctgacgcaatttttccattaatcttatctgtagctttatcatccacagagacaggaacaatctttggaatttgctttttcttgtcaaatttacgaattgagggatcgaggaactgatggccaatatcttcgctatttgcgagattaatttgaaacgactcttcaggattaattgcggtatacaactcatttaactttttaaattggtcaacaaaattaactttggacgccttaaaggaatctactggtgttgagtttaagaagttgccacgatatttcacaatgtggtgaatggccaagtaaaccatccgaatatcaaatttttcatcttgcgtcattaatgcatgacgtaaatgataaatggtcggataatccttgtggtactgcatgtcggttaaatccgggaaaagcatggaacccttgaactctttgcgtgaatcttttggcgacaaattggattgcttcaacctggcgaaaaacgtggaatcgacaggtgtaatatatgggtcaaatatttcttctaataacttcaatcgccacttccgtcgactcagacgccgtcgagtggttcgaaacatcctgcggtcagcagcggggttgccttcctgaaacaaccgggcaccgattgcagtcttacctttgatccgcaatggttttccatcttcgccgattgcaacccaaccaattgatgaggtcccaatatcgagacctatatgataattattaactttcatgctcgtaaactccttggaatattgttgccctgtaaatcgccttggcacatcatctattatgcattaaccggcaattatccgaaacccttttggcatagattggttgggaatttttcgatccatttattgatcttgcatccagttaaggtcttataaagatcttcaatgtagaatgccgcatttttagaaccatcgatcctccttaagctcacaaaaaaactccttttgagcggaccagcaggtgagctggtccgctcaaaaggaattcattttatccatccatttcttcattacaacctgcctctaataaaatggatgtggcccttcgtttctgtgctcaaatattttgttctccagagcaattcggcttttttcaggcaacgttggtggaaccagtaacaaaactgggcagccatcatgttgggaaaatacttggtccttttcaacaccatcgattaagaattgaccatcgggcattcgataaacatcataaccgagttgagaagaattgtagccgatcgcatcactcatttcaacatctgacatgccttccgtattcgaagtgaggcccataactaccccatagtcaaaatcaaagaggcgaaggcgggggtcatttgttttgaaaattctagtttggagtttatgatgccctgactgtttatatcttttcttaactcgcttaagcttatcagcgttcatttacgactgtcctcctgctattttacgtgcttttaccaagcaattttgttataggaaaataagtatctatagcatacaaccccaatagaaacgagacaatgcactttaatgaatgttaatcaatatacactttgtccgaggttgagggagaaacggccaaccactggcgtttagtaaccactgaagatgcattttcttctaaaatccacggcgttatttccaccacaaaaaagaatgcactcacaaggctgtggctatttcacagcaaagggatccgccaaatgattcttagccttctcatcttgcacataggcaacttcccgatcaataattgcctgagaatttggatcagtatacacgttcagcttgtaatcaatttctttcagattgtctgccaacagccgctgttttgccaaaacctcttggcgatgctttaacaacagctgtttgcggtcatcaatcgaagcggctccctgcatacagtaaccaatgtatttcttaatgtccttaatcttcatatcagtgttcttcaaacagcaaatggtgtgaataaaattcaagtcagaatcggtaaactcacgatatccggcctcgtttcgggaaacaaacggcaagagcccctgcttgtcgtaataccgcagcgtgtaaatggaaaggccggtcttttcggcgacctctttaattgaataagtcatctcatcatcccttttaagtttaatgtcttgcactagagtatactctagcctttaggataaagatattaaattaacgaggagaatataaatgattaaaaaagtattagtaactggcgggaacggctttctgggcctccgaattatttcgcaattgttggctaaaggttatgacgtcagaaccacgctgcgttctctcgacaagcaatcactggtattggatacgttagccgccaacaacattgcaaatctcgaccagctggaatttgttcgagctgatttatcaaaagacgatggctggcaggaagcaatgaacggcatcacagatgtcatgagtgtcgcatcccccgtattctttggtaacaccaaagataaaaatgcggcaatgcgaccagcaatcgacggcatcacccgaaacgtccaagctgcacagaatgcgggagtaaagcgacttgtcatgaccgcgaattttggcggcgttggtttcagcaatctggacaaaaatagtatcaccgatgaaaatgactggaccaatccggatcaaaagggcctttccctatatgagaaatcaaaattactcgctgaaaaagaagcttggaagctggtgaatgagtctgacaattcaatggcgttgacaactatcaatccagttgccattctcggaccggcaatgaacgggcatatatcagggagtttcggtattttggaaaacttgatgaatggcagcatgaaacacattcccaacattccgctcaacattgttgacgtcagagacgttgccgatttgcacattcgcgccatggaaaatccaaatgccgccggggaacgttttatcgccaccgccgacggccagattaccatgccggaaatggcaacaattatccgacagcattacccccaactgaaaagcgaagttgccgataaaattttaccaaactgggtggtgagggtcggttccctattcaaccaacaggcaaaagaaggtcaactgttactggacgtgaatcggaatgtcagtaatcaaaaagcccgcgacctgctggggtggcagccagtcggcagtattgagaaaacaattctggatacgcttcagagcatggacaaatttgacctgttgaagtgaatgcaccatcaaaaaaggcattaacccacgtcacaaaacgtcactgaggttaatgcctttagtcgaccatgatttaattatcaactttaccgaggataaacacatagccatatcgacttgccaaatcaccagattcaccacttggcatgacaatgttattgacaatttgaatgccgagtttgtatccagataaggacgcccgcttactgtcggtgtagccttccgcattcagcaatttcttaacaccggcaattttggttgcgttggacgcattgtggttggtgtaaagccacttttgaattgccgggaacgtcttgatatcggtgtagccggttgtactgatcggactcggatcaccatcaatatcattatcaaagctgtcataattataggcagcgatctttgataaccccaaatccggctgagagttagggaataacttaataatttctctggcgagtttttgattcttaccggtttgaagatactggttaaaatcggtattattcacaaaataaccaatatcaacataattcattccggtatgatcgggattaagcccacccgtgatcgcagattctgcaacgtaccccctggtactcttggtggtaccgtttaaagtcccggacaggtagacgtacttggtatctttcccattgtgctgcatgacaactgtatgggttttctggaacacagcaccaggataatccttcaggttcgcccgtttcttagtatgggtataattccatacgtaaacattttttgctttgtacgaatcctttacgtggaaataatcgtacttgttataccactttgtgctgataatttgatacccatatgggctaaatccgggagtcaaagcatttgttcgaacatacccctgcatgttgccagtccggttggcaacgtaatagtaagtcgcactcttcaatttgtgatagatgcgaacctttttctcgacaaaccacgtggttgttttgtgattggcgagtttgtaaccctttttgtagaagacattcgacttgatatttttgtcaaattcctggttattccacacggacgccttggttttggccttcgcgtgaaaggcaacatcttcagtatagttgctgtaattttgataagtcttcagcgttttcacccgataattattgtgggctgcctgtgcgggctgtgggctggccaccacagcaaatacgacaaaggccagcatcacaccgacaagcttaacgagttttttcatgaatgaaccccctctttcaataacagaatatcatgattaagttaccactgtgttaaataatgtattcattttcatgatggattcagattggtgtgttgacgaaaggtagacaatcatttaaaattataggtattctatcacgaaaggaagattgctatgagttcacttgttaatcgcagttggcaaagccggtaacaagtcacatcgacacagatgcgacttgatcttaagcatgcgatcatgaacgcatctgtgccggcaatctttcggaaaacgaacggtctggccagatgatttcggcaggccgacttatcacgagtatttcggtcagaccggaatgctcgttttttgttcgcataactgatggcgttacatatttattcaaattgagggagacagctattatgaagaaaaaatatttaatttcaggtgtcgtgttaatttttgtcgtaatcttgggggttgcatttttccaaggacaacagaagcaaaagccccaggccaagccaaccgtggggattctccagttgatgtcccatccagctttggatgccatccataaaggaattatccacggtcttgaagaagagggctataaacctggtaagaacatcaaaattgactttcaaaatgcccaaaatgatcaaagtaatttgaagaccatgggcaccaagtttgccaacgaggacgccgatctttcaattgggatcgccaccccatctgctcaggcattggccaacaccattacccacaagcccgtcatcttgggggccatcactgatcctaaaggcgctggtttggtaaagaacaatgaaaaacccggcggcaacatcaccggtgtttccgatcaggcacctttaaaagagcagctgaatttgatcaagcaattcatgccaaaaatgaaaaccttgggaattatctacacttccagtgatgactccgctgttgcccaatacaagatgtttgtcaaattatgcaaacaggaaaacgtccgtctcaaagcatactcaatcgccaacaccaacgatttgacccaggttgctgaacaagcggttcgctcagtggatgccatttatgtcccaaccgacaacacgattgctggggccatgcagacactggttggcgctgccaataacgccaaagtccctgttttcccagctgttgatacgatggtcaagcaaggcggcgtagcaacttacggcatcgaccagtatcaattaggagttgcgaccggtaagatgagtgcccaaatattgaagggtaagaagaagccgtcaaccaccccaattaaattcttccgtcacggaaaattaattatcaatgaaaagcaggctaacaagttgggaatcaagattcctgccaacctcttaaaagaagcccaacaaaaaggagaattgatcaaatgagtattatcgtctcagccatcggccaaggtttgacctggggaattgtcggtatcggcttattcctgacttttagaattctggatttccccgacatgaccgttgaaggaaccttccccatgggcgcagctgcctgtgtcgccgccatttattcaggggcctcaccactagtcgcaactttgattgcctttgtggcaggcatgctggctggtttggtgactggtttgctgtataccaaaggtaaaattccggtattacttgccggaattctggtgatgaccgctgcttactcagtcaacctgagaatcatgggcagagccaatttatcgctcttcgacaaacccaccatgttaaagaaccactttttggaatccttaccaccctattttgacagtgtcgttcttgggatcgtcgtggttgccatcgtcacagcacttattgtttactttctccagaccaacctcggccaagcatttattgccaccggtgataatcccaacatggcccgctcacttggcatcagcacagatgccatgcagattatgggcttgggtgtttctaacggtttaattggccttggtggcgccttggttgctcaaaataatggttttgccgacgtcaatatgggaatcggtgtcatcgtggttgccctggcttccatcattattggtgaagtcgtctttggcgatttgacgatgaaccagcggctgatcgcagtgaccatcgggagtatcttgtaccgatttgttattttgctggttctcaagctcggcttcaacgccaacgatttgaacctaatttcagctatcgtcttggcattattcatgatgttcccggttttggaaaaacgcttccgaatccgccatactttagcaaaggggatgaccaaacatgactgaaccaatcttcgaattaaatgacattgtggtcaccgtcaaccacggcacacctgagcagattaacatcatggatcacgtgaatttatctgtcttccctggcgacttcattacgattctcggttctaacggggccggtaaatcgaccttgttcaacgtcattggcggcaatctccctgtgaccagcggccaaattctcctgaacggcaaggacatcaccagcatgtcggttgagaagcggacccggttcttaagccgagtattccaggatcccaaaatgggaactgcgccacggatgacggtggcagaaaatctgctgctgtccgaaaagcgtggccaacgtcgcggctttgcaccgcggcatctcaagacgcacatggataaattcaagcaaatcacctcagtgatgaataacggtttggaacatcggctgaacacggcaactggcaagctttccggtggccagcgacaggccttgagtttcttgatggccaccatcaagcgccccgacatcctgttattggatgagcacaccgcagcccttgatccgcaaacttcgcaagaattgatgactgccacgaacgatcaaattacccgcaaccatttaacctgtttgatgatcacccaccatttggatgatgccctgaaatacggaaatcgcttaattgtcttggataacggtcgaatcacttacgatatcgccggtgccgagaaggataatctcaccaaggaagagttgctgagtttctttaatgatattgaagagtaacgcacgattgcttttataattaaaatgtcaacttggtcggtgcatgcgaatccgcatgtaccggccttttttcttgcttccatttttgagagaaggttcaaatcctttaaaatctgagtaaaatgagacctaccattcggtttatgagaaattttaaagcgctttctttgtatattctatatcttcctatttataatgagggcgtacaaagtgtctataatcatttgtgattgtgaattttctatataattttaacttatgtaaataattcgatttttcttcacagaatctttatagattttttgtaaactatagtcagtaaaggaaaaggaagtgaacattatgcaaaatcaacaatcaactccaaagaaacgtcgatttaagatgccttcagcctacaccatcttatttctgatcattatttttgttgctattttaacttggatcatccctgccggacagtatagcaccgacaaagccggcaatatcattgcccacacttacaaagcggtggcttctaatccgcagggaatctgggacgtcttctccgccccgatttatggaatggtcggaaatgatacgacggaaggcgcgatctccgtttcactgttcatcctggtgattgggggcttcttgggagtcgtcaatcaaactaaggcgcttgatgatggaattgcgactgttgtgtcaaaatacaaaggcaaggaaaaagttttgattcccctgctgatgattttgtttgcacttggtgggtcaacttacggcatggccgaagaaaccattgccttttacccactgctaattccagtcatgattggggtcggcttcgattcactagtggccgtcgcaattgtcttggttggttcgcaggtcggatgtttggcatccacggttaacccatttgcgaccggggttgcctcacaaacgctgcacatttcacccggagatgggattatttcccgggcggtcctgtttgtcatcgtggtggcaatcagtatcctgtttgtttaccgatacgctgccaaaattgaaaatgatccttcaaggtcttacgtctttgaacagcgtgaagaagatttgaaacgatttgcgttgaaccatgaagaccaacccggcactaagatgaccggccgacaaaaagccgttctctggatgtttggtttgacattcctagtcatgatcatgggcttgattccatgggaccaaatcaacaagaactggaccttctttaccagtttcaccaaatgggttcaagatgtgccattcttaggtagtctggttggttccaacctggtaccatttggttcctggtacttcactgaaattacgaccctcttcttcttgatggcaatcgtggtgatgttcgtcttccatatgaaggaatccacatttatcgaatcattcttagccggaatgagtgacttcatgggtgtagcaattgttgttgctgttgcccgtggaattcaagttgtcatgaatgatggaaacatcaccgcaaccgttctccactggggtgaaatgggcttgtccaacctcgggtcggttgtcttcatcatcttggcatacatcttctacatcccaatgtccttcttgattccatcaacgtcaggcctggcagccgctacgatgggcatcatcggcccaatgggtaagttcgccggtgttgacccaagcttggttgtaacagcttaccagagtgcatccggctgggttaacctaatcacaccaacatcgggcgttgtgatgggagccttgacaattgcccacgtcaacatcacgacttggtggaaattcatgttcaaattgatggtttacttgttcttagcgactgcgattttcctgggggtaatggcactgctgtagagcgcgacgaggcccgggtgaccccggagtgtaagccgaaagctttgatgatggacgtttttggtccatcattaaagtttttggcttacacagtaggggtcagggccgtcggagcgcctttccactcggtaaaaagaacccacaaacacccatcaacctcaaacaaaagccaccaaccaaaaccactaacaacaaccaaaaaccaaaaaactcaacctaggaggcaccaacaaaaatgtctgaaaaattagtcacagaaacagaacaaaacgaagctgttgaaggcttaaaacgcctagtcagcaaaccttcagtcaatgatccagccaccgtttccaaaacgacgccatttggtcaaggaatcgacgacgcattaaccgaagtcttacagatcgctgaagaaaatggcttcaagacgtttaaagatcctgaaggccattatggctatgctgaaattggctccggcgataagatctttggcattattggccacatggacgttgtcccggccggtgatccaaatgattgggattccgatccatttaccgcaaccatcaaagatggctacatttacggccgtggcacccaagacgacaaaggtccttcgatggcagccatgttcgccgtcaaagccctagttgatcgtgggtacaagttcaactgccgcattcgatttatcttcggcaccgacgaagagaccctttggcgtgggattgctgtgtataaccaaaaggaatccccaactgattttggaatcgcacccgatgccgaattcccactgatttacgcagaaaaagggctggaacagtcctacctggttggtcccgggatggatgatctgtccctcgatttggaaaatgcttttaacgccgtccctgccaaagccccttacaacgggccaaagctggatgaagtcaaggcatccctggacaaacacggcttcaaatacgaagaccatggcactgatggcatcaccgtcgttggtaaagcggttcatgccatgaatgcccctcaaggtaccaatgcagtcttgcgtttggcaattgccttggacaacgtctttgacagccccgtactcgacttctttggcaagaaattccaggaggacgctaccggtaccaatctgcttggcgatgtcgaagatgaggcgtctggtcatttgaccatgaatatttccagtctcaaaattgatcaaaaagaaactcgcatgcaagtcgacatgcggattcccgtcaccgttaatcatgacgaattgattgaaaagctcaaggaggcggccgaaccatatgacctgcactacgaggcatttgactatgttgccccactgtatgtgccaactgacagtgatttagtcaagacgttaatgtcaacctacaaggatttgaccggcgatgacacccaaccgcaaatttccggcggtgccacatttgcccgaaccatgaacaactgcgtggcttatggtgccatgctgccaggaacccctgattttatgcatcaggtcaatgaaaattgggagcttaagagtatgtacaaggcaatggatatttacgctgaagcaattaaacgtctctgcacagactaaccgtgacgttcatgaaatataaaaaatgctcgggaaccaatcgttctcgagcatttttgtgtctctattaatctaagcgagtctatttgttttgagcagccgacttcaatgcggcattctttcgcatatccatttcaatttgttcaagcgtcttgccacgggtttctggcaccatgtagatgacgaagaagattgaaacgatcgcaaagaaggtaaagacggcaaatggtccaccaacattgttgttaaacatgtgaagtaattccaagaagaattgtgaaacgataaagtttccaatccagttggcagcggaaccaattgaagttccgactccacggacattcaatgggaagatttcaccgatcatcaaccagcaaattgggccccatgaaacggcgaaaccaaagatataaattccaatcaggatcatggttggaacagcagcgtcttgaacttttaaagtgaagttcaagattgagagaattccaattgacaatgccatgacgattgaaccaaatagcagaatggttcttcggttgaatcgatccatgatattgtatgccaagatcgtgcagaggaagttgacaatcccaatcccaacagaaatccaaatagcgttactctcagggaaaccaaagcctttaatgaagacttgcggcaggaaataaatcactgaattaattccaactaactgttgaagcagcatcagcaaaatcgcaacaatcactgctgggcgagcaaaggtaaacagctctttgagaccgcccttgggttggttggcaacttcttgaatcccagccaattccttgtcaggatcctcatctgtctttgcccggagttcatgaagaacgtcccgagcctcgtcaatccgacccttttcaaccaaataacgtggtgattcggggagaatgattgaaccgacaaacagcatcaaagctggaatcaaagcggatccaagcatccaacgccagtcacgtaatcccagcagattgtgatgtaagaatcctaagttggaaacgtatgctaacaggattcctaaagtaatcatcaactgaaacatcgtaccaagtgagccacggtgcggtgcatcagccaactctgccaaataggctggcgttaaagctgacgcagatccgacagcaaagcctaagatgattcgggcaatgaccattgatacaaatccttgggcaaacattgacagtcctgatccaattaagaataggatcgaggctaaaaccaacaggcgctttcgaccaaaccggtccgaaagtgaaccaatcgacaacgcaccaacagatgaaccaatcaaaacagacgagacaatgaacccagtctgttcagttcctaaattaaaattgctttcaatcaatggtgaggcacctgaaataataccagtatcaaatccaaatagaaggccacctaatgcaccaaagaagaaaataaagaacgtacttaaatgacgtgctttcacgattatccctccttaggggatcatttctgaatcaatcaaatcttgtaatccctttcatttgaaacaaaaatacattaaaacagttcagtattcatactccccctttagatactcaatttgtactatctttcagtataaaaacgttgaggctaaaattcaagaaattacatttttgacttactaatattcagttgataaccaatcagatttaaagctaatttgtaattcgttataatagttaggtaccgaaacactttgcttgtgttcaaaaaaattcagtgtatacttcttattgttaggtacctaagtataacaatttaaaggagaatgaatatggcagatattaataaaagagaactattaggcaagttcttcggcttccttcatggaacccaacgatttgcccgtcaccaagaacggccttaccatttgcggggccaaaacagagtcctggttatcctgtccaaggaaggcacactgattcaaagtcagttggctgaaatcatggacatccgaccatcatcaatgactgaattgttgtccaagttggaagagcgcggcttgatcacccggactcctgacgaaaacgacaaacgagttaccaatgtggccatcaccgacgaaggcaagaaagccatcgaagacgatgattccactgatgacatgctcgaccaaatttttgcggggctctctgatgaagaattggctcaattaaacgaactgttgagtaaattgaacacgtcactcaaagagaaactccctgaccacgacgacgaaccaggttggggacaccgtttccctcaccgcggatttggcggcggccctcatggccatcacggctttggtggtccccacggcgatcctcgcggtcatggaccaatgggattcgcgccaagagattaagttgtttcatcacagaaaggctgccgatttggcagcctttttgcatacatataatactctaacttttcacattctaactcttcacaaaattagcaatcacatcctgtttcttactcatcttaattttcgcctgagcagctgctaagcgagccaccggtacccggtaaggtgagcaggaaacataggaaacattgatcgactcgaagaactcgattgatttgggatccccaccaacttctccgcaaacgccgattggcaggttgggtttggtaaaccggcctttctcaacagccatcttcattaattcaccgacgccgtctacatcaaccgtttggaacggatctgctttgagaagccccttctcaatgtattctggcatgaacgaacccacatcatcccgggagaagccataggtcagctgggttaaatcgttggtgccaaagctgaagaagtcggatacttcggcaactttatcagcagttaagcaggcccgcggaatttccatcatcgttccaaccgtgtatttcaacctggttccttgctcgttaaacaagctttcgacctggttcacaacgatgtctcgaacccagctcatctcagccttggaaccggtgagtggaatcataatgtgtggctgaatttccagtccttgggtgtgcagctccaaagcagctccaatgattgcccgtacctgcatctcataaatgtctgggaaggttacagccaatcgatcgccacgatgaccgagcatcgggttgatttctttgagggcatccactcgacgaaccaggtattccgggtcaattcccaactgatcggaaacttgagcaatttctttggcgtcgtgcggtaaaaattcgtgtaatggtggatccagcaaacgaatcgtgaccgaacggccttccgataaacggaacaattcgtaaaagtctccctgctgcatctgcagtaactcggccaggggggcttttcgttcttcggcgtcttcagcgatgatcaaccgtctcatttccagcagtcgctccggtttgaagaacatgtgctccgttcgagtcaggccaattccgtcagcaccgaatttcagtgcttgggcaaaatcggcaggcgtgtcggcgttggcatacacgcccaggtctccttcctgcttggaccaatccaaaattgtcgacaggtcgtcattgacccttgaatcattggtctgaatctgcccgaaataaaggttaccgttagtgccgtcaactgacagccagtctccttcgtgcagctcagttccggcaatggtggcgaccccgttttgatagtcaacctgcagatcattcaccccaaccgtcgccggggttcccatgccacgcgccacaaccgccgcgtgggaagtcatcccaccacgggaagtgacaatcgcttcactaatgaccatcccttcaatgtcctctggtgacgtatcctgccgaaccaggataacctgctgttccaaatcatcatgggcagctttggcagactcagcggtgaaatagatctggccggaagcagctcctggtgaagccggcagaccactggcagccggctggctctgctgcagggcttcctcgtcgaattctgggtagagaatcgcgccaattgaatccggattaattctcagcaacgcttccgtccgagagatcaagccttcttcgactaaatcaaccgcaattttaactgccgcggtcggcgtacgtttgccgtttctggcttgcagcatgtacagtgttccgtgttcaatggtaaattccaaatcctgcatgtcgcggtaatgaatttccagtttcttggcagtggccacaaactcgttgtaaagatcgggcattgtgtcggctaatgtactgatcggctggggtgttcgaatccccgccacaacatcttccccttgggcgtttaagaggtactccccgaataatttgttctccccggttgctggattacgggtaaacgcaaccccagtccccgagtcttcgccagcattgccaaagaccatcatttgaacgttaacggcggttcccaaatcactggcaatatggttttcccggcgatagacctgggcgcgatgattgttccatgattcaaaaaccgcattcactgcagcaagcagttgaactttgggatcctgcgggaactctttgccggcttcggctatgtagagttctttaaacttaccgacaattgtgtgcaaatctgccaccgtcaagtccaggtcggagtcataatgattggtgattttaatatcttcgagaatctggtcaaaaatgtcctcggggatttcgtacaccacgttgccaaacatcgctaagagacggcggtaactatcgtaggcaaaccgttcattatcggtaatcgccgctaaagttttaacagtctggtcatttagaccaatgttcaagatggtgtccatcatcccgggcattgaaattgccgctccggaacgaacggaaaccagcaacggattatccgggctgttgaatcgtttccccactttagtgcttaattggtcgagtgcctgatcaatttgttcgagcgtgtcgtcattcaactgattaccgttgtcatagaatgcctggcaggcctcggtactaattgtaaatccacttggaaccgggaaccccagtgaggtcatttgtgccaaattagcccctttgcccccaagtaaacgacgcatatccttgttaccttcttcaaagcgataaatgtatttcatatcataacgtcctttctgaactaattagcgtgttacattggatgcatttatcatatatgatacgttttaataatgcaaattaaattttaaaaaacgttttatttaacggtaatgaaatgttgctcttaaaagggttggcacgttgaaaaagaattttactaccaatccgttttcttaaataagacgttttattggatacatatttgatcagatatgatagaattggactagtggtacggaccaacgactatcgaaagtgggagcgattaacttgaaactatccgaccggcaaaaccaaatcgtcgacattgttaaacagaaagaccccatcaccagccgccaaattgctgcagagttggggttgagtatgccgaccattcgatccgacctcagactcctgacggcattcaacattctggaagccaagcccaaagttggttacacctacaatgattctcaagccaagcctttaagctatcacaagctttatgcggaaccgatcgctaatattctgcagaaaccaactgagattcgtgaggatgccacattgaccgaggcggtcaacaccctgtttatcgaggatgtcggttccctttacgtcattggcgatcgtcaagaactggtcggcttaatttcccgcaaggatttgttacgggcaaccctgaataataccaatgcttcactgacacttgccagtacagtcatgacgcgaatgcccaatattttcaccgttaccccagatatgtcggtcctccaaaccgggcagctcttattggatcgcaaagtcgattctctgccagtggtggataaggaccagccaaccaaagtcgtcggcaaaattactaaaaatcgaatctttcaacatttcattaccagtgttgactaatcatcccactcaaaagagctcaggcatttgcctttgctcttatttaattggtgcaaaatgccagaccccagttttgatttaagtctgttttaaggtcaataatgtataagtaaactagattatttttactaaggacggtgactgcaaaacagctatgttgaaaaagagaattgaatggattgatatcgccaaagcatacggtattattgcggtggtgtttggccacgcgttagccagcggcacaaccaccaacattatttattggtggcacatgcccctgttcttcattgtcggcggattcttcttgaagccgattgacacaactaaattaactcattggaaaaagttctttaataaacgcatttaccgggatctgctgatctactttatcgcggggatcggcttgatcctgttgtatagcatcttgtatgacaaaaattgggattacttgattaaccacctctcaagactgttggtcgggggccggacattgaacctgtacacgtcaacgttctggtttgtgaacgtctacctgctgtcaattacggcggtgaccctgttgatttcgaccgttaaatccagaattggtcagctcacaattgtcgggttgggattatttatctctacctgctatgacaaaattgattgggtgaacttgtacaattatcaaacaatgccctggaacttggatatcgtcttgattgctgcattctttacctacgtcggttatctgtttttccacacaaattggcactggattgaaaagccattgccgattggattactggttggtgcttccttggcaatcattggcttgtatcttaatcagaaattcagctttgaattttcgatgaaatctcatctgattcaatcatcagagccgaaaatcttgatgctggccaccatcccactgattttttcatttggtgtgatggggctatcggcacttaccagcaagctgtcgattggcttgttgctgtcaaccattggtaagcacaccatgattattatgtatttacacggcgccctgctggacatcgcagaacagactggtattgaaaacgtggccgtcaaagtgatgattgcgttggttatcccaatgctgctggcactgctcaagcagccggttgttcgaaggaatagtatttatttacaaggataataaaagagagtgtgaaagcggacgtttagcaagggaaatttaagcaccgccaggcggaaaccgagtcaggttttcgagtggtggtgcttaaatttcccttgctgtccgctttcacacgtttgatccaaataacagtaaaacaccaggaaaccgagtcaggttttcggctggtggcgcttaaacctcgcttgctgtcctctttcacacgtttgatccaaataacagtgacactcaaaaaaggctgagattactaacaaattgttagatctcagcctcttctttcttggttctggaatcaacatcatgatcccatattcaattatttaaaatccaactctaaatactccgcgccatccaaggggttaaagcggtacgggtcgattggtttaaaaccggcggcgtgataaatttttaaagccccggtcattgatttcaaggtgtccaaacgaatcgcctgatagcccaaacgctcggcactggctaaaattctggcgaccagttcctgaccaatcccgagttttcggaagtcgtcacgaacgtaaagccgcttcatttcagcaatccccggttcaaattcatgaacagcgaccacaccagctaattgatcattcacatatgctaagatgagatctcctttgggctggttataccgggtcgctaattcatttaattcatcattgaagtcttggaatcccaggtcgaatccgagtgacttggaatactcaagaaaaatctgcttggcggcgttaaagtctgccgccgtactggcatgcttatacttcagttgtgctggttgagcttgttccatgtaaccatccctcctgacaattaggagtagtgtacaaaatttgagttatttatgcaaatggcgctggtgaagcaagcgctgcttttcttcttcggcagctttatcggccaactgctgttcatgttcccgttcactggcagctttttgcggcaaaaccaaattgagaacaattccaataatcgtggcaaatgccaagccggtaaactggaacttaccgagttggagataagcattaccaacaccgataaccatgaccgtggacgcaatcatcaagttgcgcttcaggcccatatcaactttattttcaaccatcacttgaatcccggcagttgcgatcgttccaaacaacaggaagctaattcctccgatgaccggcatcggcatctgcataatcaaaacattcaatttgttcacgaaggcaaacagaatcgcaaacatggcggcacccatcagcacataaacactgtggatcttggtaatcgccataacaccgatgttttcaccataactggtcatggcaggtgcaccaactaatccagcaaacagcgaagcagcaccatctccggccaacgtccggttcaagccgggatccttgaagaagtcccggccggtcaattcatccaagaccataatgtggcccatatgctcggtcatcgtcacgaaggcaattggcgtaatcgctaagatggcagcccaatcaatgtgaaatttgtaatcaattccaggaatatcaaaggccggaattttaaaccacggggcactggcaatcgcatttaaatcaacgatgccacagaagactgagatgagataaccacaaacaattgctaacaaaactggaatcaggccgatgaagcctttgaataacatgttaaaaataatagctaagaataaagttgccaaggcaatcacaaagtacaacaggctgtacttgccatttttcatcatcgcgtcttgagcggcgctaccagccagtgacagtccaatcaccatcacgatcggccccaccacaatcggcggtaaaatatggtcaacccagtccgagccaaccgcccagataatggccgccacgatcatatacacaattccgacaccaatgaccccttgagcgattccgggatacccagtggtcttcatgagcgccagcattggcgtgataaacgcaaaacttgatcccatgtatgcaggaattttgcgttgggtaatcatgatgtgtaacagtgtcccgacaccggatgcgaacaacgcgatgcttgggctcaatccaaccaacagtggaacaatgaccgttgacccaaacatggaaaacatgtgctgcaatgataatccaacccacgggaaaaatttgggcatgtcatggatgtcgagaatcgcacgatcatcatgaaattcattcttgtctgccataaatatttgccaccctcaaaagtatttgaatctttcaactccgcttcagggtgaccccttgatgaattgtgacaggctctcacttggaaagtcatgcaacaaaaaggtgtccaccccgcgttaggcaaggcagacaccaagtcgagcaattgctcgttcaatatcgtcctcttaccagcctcacgggaccagagttaaagattcattcgttgtgataattataatataccgtggttgcttgtcaatctaatcttgcaactgcatttccatatcaatatgggggatgccgtcttccagatagacatcactaacgttcttaaaaccaaacgatttgtaaaatccgttgaggtactcctgtccagctaagacaatttttccagtcttgggcatcaatgtcggaattcgatcaagagcagtttgcaccaactcgcgtcccagaccgtcgccgcgatgattggggtcaaccacgaccctgccaatccgggcaaccgtggcgttttcctcaggaataatccgcgcataggcggtgatgttgttttggtcgtccttaaacatcaaatgataagcggtcaaatcgtcatcatcgacttcttggtagtagcatttttgttcaaccacaaaaaccgccactcttaatttgtagatctgaaataattcttgagtggtcaattcaggaaatgttttaacttcatttctgtccatatttgccatccattaaggtttaaaaatacaagtttttcgctatctgttataatatattcaactagatcaacatgcaataagagaatctaaatgaggtattaatttgaataggcatgacgatgaaccacaatataaaaagtatgacttcaattctgaagaaaatcgacgtcgacaacgtcgcaaacaatacagcggctggtggtttgctctgctgattttgattattgggattgtcttggcgctttcaatcaattggtttgtgacatctggcaaccatcgacaaggaagttcaaccaattcgatcagcaagaccatcaaaaagtccgagaaagaattgtccggcaattctaagaagggatcgctgactacccaagttgagaagaatcgggtgaatgcgtttagcagtaagctcaaggatgctcagcaaaatggactcaatccaaaagaacgtcagcaattccagcaaaccatcaacgaagagcagaaccaatccgtcaagtcccaggagcaaaacctcttgaacggcgtcaaaagtgataaaccggctaagccacagaaagctcctgaccaattctcaagcacccacacatttgcctctgttcaggatgccaagaactgggcaaatgccaccaagcagcaatggctgaaggctggttacgtcaactacacgattacatcgaacggacagggatactatgtcttacggtttatcaaatagttggattcatattattttattctacgattaaaagacatatcattgagatggaggagggatcgatatggatatacaagttcctttaacaaagggtctcttagcagataagtacagtaagtatgccgccaaaaacgacatgcttgacggtaagccgatcgtttcatttccaattcaaattagcaacgttccaaagggcgcgcaatcattagcactcactttattggactgggacgcggttccggttagcgggtttccatggattcactggattgctgccaacattgcccctgacgtcacggaaatccctgaaaataacagtcagcaattaagggttccaatgattcaaggacgcaacagcactgccggcgggctaattggcaacaccaatcagacgactgcctggcactataatggtcccaacccacccgacaaagttcacaactatcatttatcagtctttgcactagacacccagttgcctttgaaagacggcttctggttaaatgaattacaggacgccatgcgcggtcatatccttgaaactgccgaattcattgttccaagtaaaccgtaattttctgaaaatgattctgtatttcagtttttaagcgccattcggtggaataattagtgatataatgaacttaaattaatttgtgggaggtttcttcatggaatccaattataaaaccatcttagtgccagtcgatggatccaatcaatcagaagatgcattggcgaaaggtgcacaatttgcaaaaaataatgatgcccatctcgatgttcttcacgttttgagcacacaacaatacggttataactatggtggaatggtcgatggggacgttattaacaaccttgttgaagataccactgattatctgaacaaactggtcgatcggattaagaaggaatctggccttgatgatatttcaatccatattcgttttggtaatcctaagaccgttatttcaatggaattcccacgagaccacaaatcagatttaattatcatcggtgctaccggtatgagtcgcctgcagcgagtcctcgaaggatcagtttcttcatttgttgaccgcaacgccaagtgtgatgtcatggttattcggaccaataccgaaaacaaaccttatataccattcccaaaagactaaacaaatgaaagcattcagcaatgaatgctttttttgttcttaaaaagaccctttcgttgacgttgccagtcaacacggtatgattaaattaacgaatgtaagcgctgtacttcgagaggagaatcaactatgaaagttcttgtaattggcggaattgccggcggaccctcgtttgcaacccgacttcgacgaatcaatgaggatgctgaaattatcatctttgaacgtggcgcggcaatctctgttgccagttgtgccctgccctattacctgggaggcttaattaaggaccgctcggcagtcattgaacggacgccggagatattaaagcagaaaaataacattgacatacggttatttaatgaagtcacccagattaatcccgatgacaagacggtggcagttaaaaatctgcaaaccggtgacacttataccgaggattacgacaagttagtcatcgcaaccggtgccagtcccacggttccagaaatttccggaatccatgatgccaataatgctttcgtattaagagcggtcacagatgcagataagatcaaatcatttattgatgaaaaacatcccaagacggtaacagtccttggagccggttcaattggcattgaagtctcagaagcctttgttgacaatcaaatggacgtcacgattattgaacaaaccggccacgttgctgcaccatttgatcctgagattaccgatatcgttgccgacgaactcaagaagcaaggggtccacgttattctcaatgaaagtgtcaaagagattcaggatcatgggcataccttaatcttagacgatggctcagtccatcaaaccgatatgttatttttaggtaccggagtcaaaccgaatagtgagatcgccggtgcagccggaatttcactttctgatgatcaccatattatcgtcgataatcatctgcagacaaacatttcagacatttatgcaattggtgacgtgattgaaacgaccagtttaatcactggcaagccaattccaagcctgctctcaagcgctgctaatcgccaaggccacttgctggcggacatgctaaacggcagtccgttggaatataaaggattcattagcgcaggtgtttccaaattctttgacttgactgccagtttcgtcggttttaccgagcaaacgcttcaacaaatggggatcactaactatcgaaccgtattcatcacgccatttgatcgggcttacttctaccccaatgccgaccgagtcaacttcaaattgatttatgaagatcagaccggtaaaatcctcggcggccaagcagttggccgaaacggcattgataaacgaatcgcagaattgtcggtcgcaattaccggtaacttgactgcgtttgaccttccatctctggaaattccctattcgccaccatattcttcaacccgtgatgtactgaatatcgcaggttatgtggccattaaccagttaaccaaccaatcagccacgatcaagattaacgacattcctgacgatgatcttaaaaacgccgtgttcctggacatcagggaagctggaaaaccagtaactggatcgatcaaaccaactttgaatattccactttcagaactccgagagcggattgacgaggttcctaaggataaaaaagtttatattaccttccgaaagggtctcggcccatacaacgccacccgtgtcttagctggaaaaggcattaatgcaactatgatcgaagaataatgaatcaataaaaggggattttttggacaaaatgttcatttagccccctttttctggagcatcaacgtataatatatgtagatgggagtgtgatgacatgccacgcaaactaagaccaaatgcagccgttaaaaaagtcttgaagatttatcaacaaaactttatgaggaaccaatttacggcacctcaaaacgatgcgctgcatttaatatttaacttaggatatacagttagtccggacgtcaacgaaagttcatacggctatgtcaaagttgtcaatatggacacgggaaaatcgctcgtcttgactaacctcagcggtaacaaggcgctattagatggtggaaccaccattatttctgaaccagatcttgacctggacacatttgattatgttgattatttgaattcgaaaggtgacaatccggattatctggcaccaaccgtcgcaaatctgaaaatgctgcgaaatcgattaaatcaattgaatgcggattttgatcgcttgaaaaaattgcgaaatgattatcaagaacatctgaccagtattgactcagaatacaataagaaagttagttctttcattactatcgtcaatcaagttgaacgaatgtccaacaagataactgaagaagatggcaaaagtaacaattcatccaagtaaaagtgggaattttcccgctttttttattttatcacaatggttatttatttggtacatattttatttaaagagggattattatatttattttattccaagctaatcagattgttattatttttatccctaattttcatattcactctataaacttaccctgttgcataattgtttgcaaacatattttttggagggaattatttcatgaaaatttcaagaatcgcattggcatcacttgtttcatttggtgtattaggaggagccagtctcaatgcttcagcaaatcacacccattatcaacgaatcctttggaacaagaccatggcacatcaaaaagtcgctttgaagaatggtaagggcattatttggaacaaaccatatagaactgccaaaaattctaaaattacttatcgtttgtcacacaagaaaggtcttgtgatgaccactcttcgccatatgaaggttaagaatggaagtatttactactttgttaaggccggtaagattagtggctggattaacaaaagtagtttgaagcttgttaagaacagctctccaaaggctgagaatcaaccttctggtacatccacagttactccggcacaaccaactggatccgttccaaattccgttcactatggagatacgacaaataatcaaaatccagctaagaatggtcaaagtacctcagcttctgttaataattacccatccgcctcttccgttaaccattacccaacggattcaagctcacaatcaaccgtcactccagcaacagacctgttcggtagttatacaaccggtcacattgtggctttaccagtcaagtccgataaaaaaacatccaaactttcaaaactcccacaaggagcagtcgtttatgaaaaggtttggcaggatggcaaactcgttgaaagtaacgtttcgtcaactatcgctgttggagcgcctgtaaaaattgcattgggcgatgaaaatccaacttcacaactcttagttcgtaccttagatggtaaagtttccggatacgttgaccgtaaccaagtttcaattggtgatctaacccaagcggaattgaatccaaccacaccaaagacaccagctaaaactgttacacagacgccagctgcatccagttcagccaagtaacaaatttgggagcataaccgctccctttacatacaccccaacaactaatcaccaacataaaactaagccatcttctaaatccatcaaattcccccaaccccctgttatgacaactaccactcgccactgcaagctttcattcatttgcaatcatttttatctttggtaaactagttgtcatcgttaacaggaggtatacatggattcaaaaaacacaacaaagattggactttttcaacttgtaatgctgacactgggatcactaatcggttctggctggcttttcggttcttgggaagccaccaaaatcgccggtccggccgcaatcatttcctgggttattggaggaattgtgattgctgcgatcgcatataactacgtcgaaattggcgcaatgtttcccgaagctggcggaatgagtcggtacgcccaatattctcacggcccgctgctaggattcattgcttcatgggcaaattggatttccctaatcactttgattcccattgaagcagttgctgctgttcagtacatgagttcctggccttgggcttgggcgaactggacgcattctttcttaaaggatggcacgattactacctcaggcttgatggtcgtattcatgttcatcctagtgttcacactgttaaatttctggtcagtaaaactattgaccagtttcaccagtttaatttcaattttgaaaattggggtccctgccctcacaattatcatgctgacaatctcaggattttacccacaaaattatggccattcaattcacgaatttatgccatacggctcggcaccgatcttcgctgccacctcagccgcaggaattattttctctttcaacgcattccaaacggttatcaacatgggaagcgaaattaaaaagtcccggaaaaatattggacgtggaattttcatttcactgctaattagtggtgtgatctatattttgctccaaagcacctacattactgccatgaagccctcaaccctagccgcaaccggctggagtgggtttgacttcaactcaccatttgctgatttagcaatcatgcttggcatccgctggttatctgttctactctacatggatgctttcgtctcacctgtcggcaccggcgtttcctttgccgcgtcaaccgggcgtgcgctttatgcaatggaaagtaaccaacatattccaagcttcattggtaaaatcaaccaaaagtatggcatcccacgagtagccatgatcgtcaacttggtattaagcatgttgatggtctcggtgtttagatcttggtccacattggcaaccgtcatttcgacttcgaccctgatcgcttatctgactgggccggtgacagccgttgccttccgtaaattggcccctaattttaaacgtccgattaaattgaagaaccttggttggatggcaccattgtcctttgttctggcctctctagccatctactgggcaatgtggccaacgaccgtcgaggtcatcttggtcattttggttgggctgccgttttatttctattacgaacaccgggccggctatgtcgacaccaggaaagctttctactcaagcatgtggatgattatctatctgatattcatctcgattatgtcctacattggtagtgaacagttcaacggaattaattggattcactacccttgggacttcgttgtcatcgccctagcctcacttgtgttctattattggggcatcaaaacggcgcacgtcttcccagacttttaccaagccaaggaactcaacgacaccgtcaaattggatgacgattaacatctgatacatcataaaaaagccgacaactgcatgaactgcagctgccggctttttgagcatcaagtgcccctgccaaggtaattccatcataccccaaatcatattgattggcgaagttaattcaaaaactgccaaaccgttttggcaaaaaagataactagcacaataataataatcggtctggcaatcgcactgccataccttttgtaatatgaggcgccaaggaaattacccaaaatactaaaggccccggcagtaagccctaaccaaaccaacaccttaccattcatcaaaaagactgctaaggcacaaacatttgtcgtcaggttgatcaccttggtgttaccagcagccaggttgattggcaagtgggcaatgccgaccaacgtcaaaatcaaaaaggttccggtccccggaccgtaaaagccatcccagacaccaagggatatggaaatcagaatcgttgcgacaaactgtgaccaagtcaatggcttggactcagccagtcgcgagttcagcgagtgtcgattcaataatagatacaacgccgttatcggcaaaacaaacaataaaatcagccgaaaataataatcagaaatatgtaaagccatgttggccccaaacgaagaacccaccatcgcagctaacacagagaagaaagccagtttgacgcggatatacccgctccgcataaattccaaggtagcgactgtcgtccccatggctgatgataacttgttggttccaaccgcaaaatgagccggaatcccaaccatcagataagctggtaatgaaatcagaccgccgccaccaccaatcgcgtccacaaagccagccagaaaaaccaacggacaaacaactaaaaattcgctgagcatcccctcatctcttttcttataataattcccagtttactgctaaataactgattataaaacgccaaatccaagtaagatgctgaaaactataagcaataaattaatttaaatttacatgcttggaatgattccgattgtggtataaatatatatgagggggatacatatcatgaaaacaatgaaatggttattactggcatttgccagttgtgcatgcttgttactattgactgaaaatccacgggttgacgcggccgggtcgattccacattggtacttgggcaactggcaggcagttaatggcaaagatgtttacgttggcattcgtcgaaacgaggtcatgctccaagtcaaaaacgacggtgtttactggaagcccgtcacttggaagaaagacacccaagaatccggcgtcgtttttggcaccggaatgggcgctaaaaattcgaagacctattttgtattagtcaaacaaaagatccaaaagaaatggtatatgattatgaccatgaaacaaagtaaaatcaaacctagtgatctgaggaagcacccgatgatcatgaaacgttattagacacaaaagtcacccatgtgagttcttgccatgagctgaagttcatccttcaaccttggaaaccccacagaggtgactttttctatatatctcgatttttctgccaataatcattaacggataaatatggccgtgaatcacccagcgactccgctacggccataatgcgcggtggtagtaatcccactcgctggacaagttcgtgatcgctgaacaattcccgtggactgccggcgaagccaaacttcccgtgctccatgacatacaccgactcaaactcggcggcgacccaatccatgtcatgggtgatggtcacaacttggtggcccgaatcagccaactgatggaaaattgcggtcaacttgcgccggctttcccagtcaagtgacatcatcggctcatcaaataaatagatcgccggatccactgccaaaactgtcgcaacgctcaacagcttgcgttcagacaacgacagatcatatggattttcagctgtttgatcatccaagccaactcttttcagagcttctaaagcccgcctcgtaatcgtgtcgtggtcatccatgacctgcgcgacactccactccacctctcgttgaaccgtcgggttgaaaagctgatcgtcaggattctgaaaagtaatcccaaccttttgtaacttttcgactggtttgagatcgttaaagtcttctccatcgatcttaatcacaccggtttgtggtgtcagtaatcccgtcaacaatttgaagagcgttgatttgccggcaccattttggccgacaattgccaccatcggatcggcgaagtgctcgtcttcaacatccaagctaaaggaccgttccggataggtgaacgtcaggtgattcagttcaattgtggacatatcgggcctcctttagctcagcgtcatttaccggataccggccgtcagccaagtgccaatccattttttgagcaagttgctgaattgtcggagctggaatctgccagtcagctgccaaatgattaaacacctcacccggcctgccctgagctaccagttgaccctcgttcaacacccacacaacgtcggcaacttcgcacaggtcgtcaatttcactggtgacaatgaagacagtcgtgtctttgacttggcccagccattggaaaaattgccggcggccaaagggatccatctcactggtcggatcatccataatcaaaacagccggattagcggcaatcgccgtggcaatcgccaaccgctggatctgaccgccggaaaggctctcgggagataaattcaactgttcaatcagccccatttgcgtggcaacttcttcaacccgtttttgaatcagtccttcagccattccctgattaatcaagtcaaaggcgatttcatcggcaaccgtgtctgccaacccacttagttggccagctggattttgcagcacaactccagtcatggcattatatgcgggccaattatcagacactcgctggccaaacatgtgccagtcgccctcaatatcggccgaaacaatcttgggaatgacccctgccagcacacggcacaaagtcgatttgccggagtggctgttcccaataatcccaaccacctggcccgaccgaacctgcgcgttaatctgacgcagttgtggttgctcagtacccggataacgggtggtcaaattttcaattacaatccgtttatcttcgtccatatcttccacccaatcaataaaattgccaatccagtcaaaacaatgtggaacgtccgtgacaggcgatacacgcgctgggaggttctgacagtccggttgggattatcaaaacctctgagctggagggaaatcgaccgtgccatcgattgatccaaggtcttaatcaccaatggaatcagcaccggcaggactgactttaatttctgaatcaacgttttttgcggattggttccgcgaactttttgagcctgctggattttccgcatattgcgcatcatttccggcaaaatataacacaccgacatcaaaacgtagacggttttataagacaatccagacagctccaaataggcagcgttttctgaaatactcgtggtcaccatgaaaaagccactggtcaaaataatcaccaatactcgacaaccgagagtggtagcgtaaattaagccttctttgtaaaaggacaccccaagcacagaaaacagcaccgtttgattccgactgtaaaacaacccttggatgatcagcatggtaccaatcaaaaacaggctgaatcccagtgccttaaatgtggtcgaactcaatttggaaaataacaatagcagtgttgcgacaagaatcagtccggcctgaagcaataaattcgtactggcaaaactcaacaacgtcatgtccaagatgaacaagagcttagtaatcggatcgatcacctggtaccacttgagcttgacccgtggtgctccagaaatcaatgtttgatcagtcatcatttatcatccctaaaaaagttcaccatccgctgcggcagctgacgatagataaagaatgccaggtaagccacgcagactttgtccaaaatatccaagacaaactcatcggtaaatgaggccaaccacactggtgcatgattggcgaccattaccgcaaataatgagtcaccccaagcgatcccggtctgaccaccccaaaagatgacattgagtggcgttgaaatgacagctgaaacaatggcaataataatagcagaaacaaatacccggcgtgctgacgagaaccacccattggcgtgcaaaactccgacagcaatcccaattccgatgctggtaatcgcatacacggttgaaattggcgataaggtcaacccatagatcacgttgttgatgaaaccactgatggcaccggcaaccggcccagccaacatgctggcaagaaaagttcccaaagaccccagccagacaggcagctttaacccctcagccaatgctttggcaacatagttaatccccacagcagcgggaatcaaagtcatggtggcagcacttaacttaaatttccacatactggtacgatgaatcggttctgttttcataatcttctcctttgattttgattatcataaaagtatcttctacttttaagtaaaagtaaaagatacttttaactcgacttggcacttattgtacaagtttcagctaaaatgtcaagaaagcgcctactcattttctggccaagttgtgctcaaaacggttaagaaacccataaactatcgactgattggcccatggacatttcaatatgcccataataaaattattaacaatcatcggggggaaattatgctacatcgtcatcgcaaattattgataactattagtctattagccgtgatcgcaattgtcggggtgatttttatcaaagccacccttagtccagataagacgccaaccgccgtcactgctgttaaggaagaagtctttcctaatcagatttttgaatcatacaaatatccttatgacctgcggattatccactcaaacgccaaactatactcggcgccagccggcactaaaggatcaaaatatctaggaaccgtcacatccaatcatctgactcggagaattgttggtcaaaaacgggccgatctgaatcaccggcgcgctgaaggttatatttctttcgcccaaaatggacatacttactgggtgagcgcacaaagcgtggtgtttcggaacctcaacaaactgaaaggcaacaaccccaaaattgaggccgcgatcgatgccggactcaaacttgtcggcaaatccaaatacgattacggtggcggtcgcaacttgagtgacatcaaaaatcacaagttcgattgttcatcatttgtccgctactgcttcagtaaggctggcgtcacccttggcaatctggatagcgtcacgacatacaccttggtcacaatggggcgtccggttaaatttcaaaatatgaaacgcggtgatctgttcttcttcaccaattcacgtggtcaggtcaactcgcacgttgccatttaccttggggaccatctattcttacacgaccacgggcaatcagatactggtggcgtggggatttcaaccttgaatgccccggggtggcggaatgaagccaatgggaccgttcggcggattgaatgagaaattaagggcgcttggcaaaatttgatgttttgctcaggggccctttttggtttctggagattacccttgccgaatcgtggaaaaatactttatccacttccgcaatatcccttcgcaacccctttgcctggcgatctcggtcatcataaaagtaccacacggcactcagtaaaaagaccaggacaccggcaatgatcaactccagtgagaaactgaaaatcaaataagcagtaaccaacaaggcgataatcggaatcaagttgccacctcgcagtcggaaccccagcggcagtttggtgtggttgcgcaatttaatcgccgctaaaatggttgggacatactgcataaatgacgtaaatacgatagctgaggctaagaacaaataatttcctgaaaatagcatcaatgcacaaagcccgcaggacagcaacaaggacacgattggcacaccgcgtttattctgcctgcccagcactcgcggcagcaattggtgttccgacgccagtgaactggcaatcgtcggcgtcgaaaatgagaccgacaaggcaacacccagaatggaaatcagcattccgaccagtgccaaatcatacccaactgtgccggccaagcggtaaaaagatgcggcaatcggcacgttgtcgttggctaaactactgccagacacgccaatcgccgtcaactggacaatcatgtacaaagttgccgacgtcaacagcacgctgatcagcgctttaggaagtgtcttttcgggatgatccatcttggaagcagcgatcggcaaaaatgaaaaaccagtgaacatataaaagaccattccaaagccggtattaattcgaccgaataatgacgaaccgtttgacatcccagcactcacattggcgtaatttgccggatgaataaagaacagccccatcccgacaaaaaggaccaaaacaccaatcttggcgaccgtcgagatattatcgacccaatccatcaaactgggtccaaacaagttaagaatcgtcaagactgccaaaattcccagtgccgccatcagataattgccatgctggttgaggctgggaaacacactgcgcaggctggttacaaatgctgagatttcagtggccatggtaataacacccaatagccacgtaaaaataccaatttcaaatccggcaaagcgaccaaaggccgtgtaagtgtacagccaagcaccaccatccccaggaattttgctggccaggttggcgaaacacagcgcaatcatgagcaccgagatgcctgccagcatcatcaatccggcgcttaagtcaccgactttggcgtacacccggctgggcatcaaaaagatccctgagccgacaattccgtcaacacccagtaaaaagacgctcaaaaaactcagtggtttgatctttgaacgtgccatgtgacagcctccccttctaagcagattccttagcagctgccggttttctgcgcgatccgaggtaacgaaccaaaacgatcactaatgccaccgcggaaatgacggttgctgtccaaaagacgttggcaaatgcatgaataaatggtaagccgacactggccgtgactcgtttaacccctggcagctggaagaacagcaaagatgacccaaagctaatcccaattgtcatccccaaggttcgggcaaacgaattcaatgatccggcaatcccggagagtgatttgtcaaccaatcccatcgttaaagcgttgttgggcgacaggaagatagccatgccaatcccgtttaagatgatcggtgggataattttccacatatccaagttattcgggaagaatgcgtaaccgacttgagaaatcatcaaaatcaacaacccgacaacggtcattaactcccggttgatccggtcggcaagatagccggcaaatggcgtcgtgcaaagcatcgtcaccgactgcaacatgataatcagcccgctgtaaaaggcactcatgccgttataactttgaaaataaaatggcagtaaaatgtttgaaactgaattaaccagcataaccagcgccaatgctgtaatcgacgtcatgaagccccggttatgaatgacttccggcgcaatccacggcaggttggccttatcatcttgaataaacgcatacagtgcaataaccccgccaacggcgaagaagataatccccgtcaatagtttggaacggccggcttgaaagaatgaaccgctcaagaagaagataatgattccaagggtaaataaattctgcccggtccagttggcgccctgagtgacccggcgaacatgcgcccaagattctttgggaatcggcaaaaacttgaaaccaagccatagaatgacaatccccaaaggaacgttaatccaatagatccaccgccagctggaagctgaaataatcaggccgccaatcccgggcccggaaattgagccaaccgaaatgaacatcgaaatgacggctaaagcttctgcccgccgtttatcaggaaaatactgagtgacaatccccattgagttggccataatcatcgccgatccaatcgcttgaatcacccggccaaataaaataatcggaaagttcggcgcaaagccggtaatcgccgacccgatcaagaagccaatccccccagctaaaaagaccacattttttgataagatgtcgccgatgtggccaaacatcaccaacagaatggctgtcgtaatcaaaccgatttgaacgatccacgtcgccatactactggaaatgtccatgtcaatcgcaattttagggatcgccaggttcgtactggagccggacaaggccgttagaaatgagaacatccctaacaccgcaataattgaataattctttcccctgcttgtcgtgttatcagccataatacccctcctctagctttcagtatcatttataacactatgcaggaaaaattttggctctgacgactttttttgttgaggatcggagagttcaaaacaattgcattcaacgtgtcactggggtcattaaaaacacccattatcactttcacctcaatgaatcagttatactgatactaacagcagtcattcggaggtgaacccatgctcacaacgattatgaccagcatcctctcatttattgggaccaacatcgacgatacctttgtcctggcagtctggttttcacaagttgatgcttctttgaggcgccgagatatcgttatcggccaattcattggatttgaaattttagtgctggtcagcgtgttggcggcatatgggctcagttttctgccaacagaacaagtcggctggctcggagtggtcccaattgttttagggatccgcaaatggcttcagtatcgacatcaattgatcgaaactcatgagacagctcacgttaaaaccaagctcaaccaagagctgaaagttgaacggcacaaatctgggttgcgaaaactattcaagccagagattttagccgtttcattaataacaatctccaacggtgccgggaacctaaccgtctatattcccctcttcacggaatataccgtggccgagttgggaatcaccgttttggtcttctcgctgatgacaggcctttggtgttatatcggctatcaaatcgctaacctgccgatcatcaaggataaattggagcactcaaagcaaatcctgatcccgataattttcatcgcgattggggtttatgtgctcatagaaagtggggtccttgggtaaaacaggtgctaattgactaattaaaaatgggccttcatccgaatttcaaaattcaggtgaaggcccatttcttataaaatttaatgatttagctgatatcaatcatctgcgggtaccatcaaacttcggtcccaactttcggttcagcttgataattcaaaatcacgtccataaactgctcaccgtatttctccagcttgctctcgccaacacccttaacatccagcatctgtgagtcagtcgtcggcatcacggcactcatttcatgaagcgtcttatcagagaagatgacaaatggtggtactccctgcttctcagccaattcacggcggagttgtctcaaggcttcaaataaatcgtcattttcagcgacactcttagtggccttaaccgagatttttcgagtgaccttcgtctcaccttggagcacggcggcacctttggcagtcacctttaacacggggaattggccaccggaagccaccaggtaacccccggcggtcaggtagtcgattaatgaaaccacatttttctgcgaatcacccttcataatgccgtacgtggagagctgattgaaatgaaaagctttcaccttttgcactttggagccggtcagtacttgagccactaggcttttaccgaaccgttccttcatccgaagaacacacgataaaaccttctgggtgtccacggtaatatcctgggattcgcgggtatcaagacagttgctgcagcggccgcagggttggccgtccttctcaccaaaatagttcaaaataaactgctgcaggcattgctgagtattggcatactgcgtcataatctgaagttttttgtaggcttgatgcttactttgctcgtcacgttcagattgatcaataaagaaatgctgagtctgaacgtcttttaatttgaacagcaaaatcgcttcactgggcaatccgtctcgaccagcccgaccagcttcctggtaatattcttccaaactaccaggaaccgaatcatgaattacgaaccgaacgttgctcttgtcaatccccattccaaaggcgttggtagcgaccatcaccaaggcgcgatcataaagaaaatcgtcctgattttttcggcgttgctccttggtcatgccgccgtgatacatagtcaccgagaatttgtgcttggacaaaagcttcgtgacccgctcaacttcttttctggtgctggcatagatgatgccggattcagcggcgtttaatttcaaataatccagcatatatttgtcgctgtcttggttctgaatcactttaaaagccaagttgtctcgggcaaaacccgtcttgacttcttctttaatgtgcagacgctgcttaatgtcgtcggcaacttgcggtgttgccgtcgccgtcagcgcaacgatcgtcggcttggttggcaagtcatgaagccgttcggtcaatgccaaataacttggccgaaagtcgtgcccccattgagaaatacagtgggcttcgtcgaccgctaccaaatcaatcggcaggttggccaagcggttaaacgccccggaatccaagcgttcaggagaaacatacagcagcttaacctcaccgtctcgagcctgctgaaagcgctcgtcgatttcgtcaaaatccaggctactgttaataaacgttgccggaatgcccgtttcgttcagcgcgtctacttggtctttcatcaaggcaatcagtggcgaaaccacgagggtcaggccatcttctaacattgccggaatctgataacacagcgatttcccgccgccggtcggcatgatggtcaagacgttttgatgggccaaaatgtcgttaatgacggtctgctgtccagggcgaaagctgtcatagccaaatttagtttttaatagtttttcgggcgtcaacctgttcagtcctcttttcgaattagtcacatactatagtatacgaaaaaatcagccccatgtcttcaaccatccggggatcgaagttaacaaccggcgacaaaatccatgagagaagcgtttgcttatgctattctaaaaaaggaatactaatagaaatgggtgatgattatgcagcaaatttccacaaaaactttaaatatgaatgtccaaaaagatttgaattttacctggtcaacgcaagcaatccttttctgtgccatcatcattgcctgtatcggcctcaacgttgattccgcgcccgtcgtcatcggagcgatgctgatctcgccattaatggcgccaattgtcgggatcggctacggcttgggaaatagcaatccaaagctattatcaaaagcggcgagactctttttgatccaggtaaccatcgggatcatcggtgcaaccatttactttttcatttcgccattaaataccgccagtgcccaactgctcgcccgaaccgaacccactctctgggacgttttaattgctttttttggcggttttgccggcgtcatcagttctgctaaaaaagatggtggcaacgtcgtccccggggttgccattgccacggccttaatgccgccgctatgtacggttgggtatgggattagtcatctcaacgcttcatttattttgggagcgggctacttatttttgattaacgactttttcatcgccctggcaacggcagccgggaccatctttttccgcatccgtagcggtgaacggctgaatgtatcattgcgccaacaagttctgatcgtcatcatttcgattatcattgtcattcccagctcaatctcagcttacacgatcgtccacaattcatttgtcgacacgcaattatcacaatttatcaacgagaagctcagcaatcaatacattgccaaacaaaacgttgacggcaaaaatattcaaatctcggtcatcggccaacgcttgtctgccagccaagtcgagcaactacagcagtcactgaagcagtatcatctcggtgattaccagttatcgttgacacagctcaccaaaggaaattacatcacacccaaagaatttcaagattatatgaagcaatcagacactaatgacacaattcaaaccaacaccaattcagccgacaatgcctcattgaccaatgtccaaaatgacatcgtcaaaaaatatcccaaacaaatcagcaatatttttgttggccaagttcaagacaaagccaatcacacgatttccctgattgccattcagctctcggataacggcaaaggaaaagcgactgagattgagaaggctgccacaaagactgccgctaataacaatgttaatgccgtcgttcgcatgatgactccttcccaacagggtgattaaagtcacaatgtatgattctttgattatcaacttggcttgtgcataaaataataagttatcttccttgtacgcgcataaaattcgtagtattcttcgcttgtggaagggcttacacgaattgattagagacggtcgagttattttcgaaaggagtttttgttatgtcacgacaaattactggtgcggtgatcgaagaattaaatgcaccgttcaagttggaaacacttgaagtcgacgatcagccaaaagcacatgaagtattggtgcatattgttgcaagtgggatttgtcactctgatgaagcggttcgtaatgggtctgccggcgactacgcataccctggggttgtgggtcatgaaggtgccggaattgtcgaaaaagttggttcgtcagttaccaccgttaaagaaggcgaccacgtcattctctcatacgattacgatgggacttgtcgtcactgcttaaccggtcacccatcttcatgtattaactgggggaagctgaattttgcgggcgttcgtcccgatggatcagtcgcctttacccgtgaagatggttcaccaattcataatttctttaaccaatcctcatttaccaccgaaacattggttcaagaacgaaacattacggtgatcgataaagatattgacttacgtaaagtgggccctctcggctgtggctttgtaaccggatctgggaccgtatttaacggcttaaaccctaaagaaggcacaacgattgcgattgtcggaaccggtgctgtgggttccgctgctttgatggctgccaagattaagggctgctcaaagatcatctgtgtcgatatccacgattcacgtttggaaatggctaaagaacttggcgctaccgatacaatcaacagtctgaacgaagactgggttgataaagtgcatgaaatcaccaatggtgaaggtgttgactttgcaattgataccactggaatttcagctattatgcaccaagccatcactgctttggcatccggcggtcatctggctccaatcgccgttactgccaagacattggaattcatgccatggaatgaaatcactgcgctgcaaaaacacgttgacggcgtgctgatgggcgatgcgattccacaaatcgggattcagactttaatcgatttctggcaggcaggcgaattcccatttgataagctggaaaaattctacacctttgatcaagtcaacgaagccaaccaagcttcaaatgacggctcggttatcaaaccggtcatggtgattgaccaggactacgtaccgggtgaataaattgatttgtattattaacgacattttgacatccaaatgagaaaggcggttctcaacagctaactagctgtgggaatcgcctttattgattcatttgatttaatttttgagcttacgttggataaatttgccaattccaactaatccattgagtaggctgacaacaattaatatcgctttggcctaccaaccgtcaccgccagtctgaggtagtcctggtaactggcgggcaactgtccgcggaaggattcgaagttgccagtccatagccttattcagtaaccgtttctttggcaaatcccttgatctcagcctgctgatgctgattaatattgcccatcttcggcatcaagccatgaaggtacaaatgatccttggcaactttgatgtgcttttgatccaaaatcttggtcaattgcttgcccactgtgaatagactgccagatgtgccaaacaaaaagacctctttgacctgctttggatccagattgcgggcaaattgtttcaagcgttcatcgacgttcaggttataaattcccccacctaaatacagtcggtcaaccgttccggtcagcggtgtatcaatcgatttcgcctcgatcttcaattgattgcctaacatgttcgcaagtttttcagtattccccgttcgtgaataatatctaattgcatccatattgtgcatctcctcacattttcgattatagttctgtatccgctttctttcaaataagaatcgcgttctatccgcatttattctctaaaatgaaataattataaagttcaatttaaagcgtttacatttgattaaggacgcactgtactcgagtaagtgaggaaaaaatatgaatcaaaaatttttaagggggttatttatttatggttgaaacaattagtggttcagatgctgttcttaaggtgctcgaacaatggggtgttaagaacatctacggcctgccaggtggctcatttgactcgaccatgaatgcgattcacaaccaaaagaaacagattaattatgtacaggttcgtcatgaagaagctggcgcaatcgctgctgccgcaactgccaagttgactggcaaagtcggcgtttgtttcggatcagctggtccaggcgctgttcatctgctcaacggcctgtatgacgcaaaaagtgacggcgttcccgttgttgctttagttgcgcaagtaccaaccggcagcatgaacatggacttcttccaagcaatggatgaagagccgatttttgatgatgttgctgtttggaaccgcactgccatgactgcagatgcattgccgcgaatgactgacgaagccatccgtcaagcctacatgaaacacggtgttgcagtcttaacgattccaaaggaccttggctgggctcaaattaacaatacgtatcaaccaaacgtcaagtcgcatcaaacacctgtctatccaagccctcgtccagaagacgttgaagaagccgttaaattaattaaagaagctaaatcaccaatgatttacttcgggattggtgccaaggatgctgccgacgaattgaaggaagcttccgaaaaattcaagatgccattggtttcatcattcttagccaaaggaattctcccagacgactatccagcctatcttggatcaaccggccgggttgcgccaaaggccggttcagaggccggattcagcaccgacttgattctgtgggtcggcaacaacgtcccattcagcatcttcttgttcaacaaacacgctaaagtcattcaaattgatattcaaagtgaaaaactcggtgagcgtcggcacaacgatgtttcaatgttggccgattcaaaagttgccttggatgccattcttgaagccggcgaaacccgtcagccttcagcattctatcaggcttgccttgccgataaagaaaactggaacagctggttggacagcttcaaagattccgatcaaatgccggtccgtccagaaccaatcttcgatgtcttgaatcaaactgcctccaacaaagcagtcttcgctgttgatgtcggcaacgttgacatcaacttcgaccggctgatcaacatgcacgacgaccagaaatgggcaacctcaggcatttacgcaaccatgggctttgccctgccagcatcaatcgctgccaagcttgagtatccagaccgtgacgtctacagcctcagcggtgatggcggctttgcaatgctgatggaagaagtcatgacccaagtcaaatatggcctgcacatcgtcaacatcatcttcaccaacgaaacgcttggctttatcgaagcggagcagactgacgatactcatcagccattatccggtgttgatttgcctgacactaattgggctgaagtcaccaagggaatgggcgccgtcagttacaccgttcacaccaaggaagatatgcaaaaagccctcaaagatgctgaaaacactgataaaccagtggtcattgacgttaaattaacccacgagatgccattgacaactcagcacatgttcctggacacttcatggcaggataaggacaaagttgccgaatacgtcaagaagtaccaggcacaagatttgaaaccattgagctacttcttgaaagaagccgagaaccatcagcttcaaaccaactgataatcgttgtgaaagaagatcaaaggccggaaacaagcgcttttgtttccggcctttgcactacatagaaaagtaggtagtaaggagtgccagcgatgaaagtcgtttacttgaatcaacattctcaatcaaatatgtccagctcccccaccccaattgtcttggcgctaggcttttttgacggcgtacacaaaggtcaccagaaagtcatcgcaactgcgcgaaaaattgccagccaaaagggttatcaactagcggtcatgaccttcaatcgacatgcctccagagtgtttaatcatagtcaaaccgccagtttcagatatctaaccaccctgaaacagaaaattgaactggtgcgggccacccacgcggatattctgtacgtcatcgacttcaccaaacaattcgcggccttatcaccaaagcactttgtagaccaatacgtgattgggttaaatgccaaagtcgttgtcgccggctttgactacacatttggccgtggtgggacaacgaccatcgattcactggccaaaatcagtggcggtaaggtcaaaacggtcaccgtcaacgaattggccagtgaccaactaaaaatcagttcgacgcgaattcgccatttggtccgcgacagcaatattcaagaggcgacacgcttactgggtcatccctacgaaaccactgggaaattgattcatgcccaaactaatgggttatcgatcgttaatccatccagccgtttgcagcagttgccggaaagcgggcggtatttgtgtgaggttcgggtggcggattctatcgccaaggttcctgtgaacgttgtccattccggaaatggtgatcaaagcgtcatctacttaaaccgaaaacgatttgatcacctcccccacgtgaattccttgccagtgtggattcgctgggttaattaatcaatttcaaaaacatccccacaaagttgccttaagctctgtggggatgcttttgcaaatcaacatcattttgaaagactttagaagcaatcagctccaagccgataattccggatggttatcaatttttttgttcaacaggtcaatttagagatataattaatttgttaactattcttataaaagaattatagttaaatctaaaaggagaataaatgattagaaaacatatcgcattattacttgcaattttttcgtttagtacttcagctgcgtttctgcaggatcaatctgtacaagcagccaagtggcatcacggaacgcccactgccttacgcgggcattggcgaacgaatgtcttttggcaatacggcttccgtaattacaacaccatggcaattggaaagcatgaacttatttcaacaattcacgcaatcggtagtactgctgatgtcagtttgccgacaatttggtcaccaaagtacatatatcttggtcatcacctgtacaaattcaaaggaatgggacctggcggtttcaaaacccactgttggataaaatggaaaaatcatcgcttattaacagtgaaaacgccaaaaagtggattgccagaacattactaccgttaatctgcagtgaataaaggaagaattccattgaaatttactaaaatgatccttacgatggtatttgtctgcctatttgccatcggttatcaaacaagtacaaccagtgctgcgacctggcatgccggaacaccaactgcgctacaggggaaatggcaacaaaagtccagtaatcacgacggcaaccatgcttactacaataaggtttctattactaaggaatcattggaaacgacgtatttcggtggcatgcccgatttatttacccatatcaaatggcacaaagtaagccacaacacctacgtgctgcatgctcgacgttttatcgatggttatcaacacaagatccacagactcacgattaaacgcatttcccataatcggatgtacatgcatctggatggacacacatatttttcaagtaggcatcatttatttaatcggtattagcaatgaaaatatagttacgaaagaggagttactcagtgtcttgagcaactcctcttgttgtattcatcaatattcaaatcatcgtttaacagcctacttcaaatacgacaacggcttttgaacttcaaccttcgtaccatcatacttatccttaatatacttctgaatcgctggttcatgatacagcttcaccaacttttggtaatccttgttatgccggttcttcttggccgtcgccaacacgttaatgttgcttctggtgctgacgtcaattttttcatggaagatcgagtctttcaacacgttcaaatggccttcgagtgcaactgtgtttgagattaagacggcgtccaaattgtggagaacccgcggacccgtggtatcgtcaatttctttgaattttaaatgcttgggatttgaggcaatatcactggtatttcccaaagcaccaaaatttttgtcgagcttgatgaggccggcactttgcagcaacagcagcccccgagccgtgttcgccggattattggcaatcgcaattgtggcgccgtctggcagctcattcaccttcttatatttatcagaataaattccgagcggttccagatatgtcgtccccaaagcggccaactgggccttttgatgttcctgattgtatgcctgtaagtacgagtatgactgaaaggcgttgacgtcgatgctgccttgagcggtggcattgttaagctgaacaccatcggtaatttgtttgaccttaattttgaggcccaattttttagcctgcttactgtcagcaatatgattccaaatatcataatctgacccttgtgatccgaccgtaatcgtggcgctcttagaattggatgcgttgccagtcagggtgtgaatgccaaagacaatcccaaccaataccacaatgccaattaacgtataaataatgcctttactattcttcatgtgttttctcctcaaataatcatttttttataagtgaactgtcttttttgccagccagtcgccagcgaattggacaataaagaccatgatcaaaatgactaacattgctgccacggtgacatcattttgataacgggcgtaaccgatactgatggcaacatcacccagaccgccagaaccaatcgccccagccatagtcgtcaggccaatcaaactaatgacggtcacaatggaggctcgaatcagatcaggcaatccttcgcgtaaatagattcggaagatgatttccaagtttcccgaacccattgaacgcgcggcttcaatcacctgcggatcaatttccagcaaggcgttttgaacttggcgggcatagaaggggaaaattcccacaactaacggcactaaagccgccgtcgttccaaccgtggtgtgtacgataaagttggtaatcggaaacatcaccgccagcaaaatgataaacggaatcgatcgcaataaattgaccactttgtcaaccaggctgtacacatacccgtcttcagcgatacccccttcttgggtaatcaccagcaaaatgccgatcccaaggcccaaaattccggcaatcagagaagaccaaaatgtcatataaatggtctcccaaattgactgaacaaattgcggccaaatatgggccacattaggaaatatttgttttaacatctttctgctctcctctcttagccgttgccaataatttaacgttgacgccgtgttgattcaaaaaattaattccatcggccagatgtttggattgtcccgacaagacaatgatcaaataaccaattgacgttgaaccgatccgttcaatgttggcaaataaaatgtttgctttcagtttatacagttctgtcaggtcagaaatcaaagattcctttgtggcttgaccatgaaacttgagaaagagtagccgttcattggcggccaaattctgcaaactttgatcggctttgatctgtgccaacgcttcggtcacatttgcggaggagtcgacaaaagtctgggttaaagcctgcttgggattcgagaagacagatgcgacatccccgcgctcaataatctttcctgcgtccatgaccgcaacgtgttggcaaattgatttaataacctgcatctcatgggtgatcaagacaaccgtcagccccaaactttcattcaaccgcttcaacaatttcaaaatatcatcggtcgtcttgggatccaacgcactggtagcttcatcgctgaccaaaatgttgggatcatttgccaatgatctggcgatggcgactctttgcttttgacctccggaaagctgctccggataagcctggacatattcacttagaccgaccaaatcaagcagtttcttggctttcaagcgtcgatctgttttactgattcgttggctcaacaatggatactcgacgttgcccaataccgttctggaatttaataaattaaagtgctgaaaaatcatgccaatctttttcctggcttttcgcagttccggattggcaagttgatctaaccgttggccaccaacaaggacgttgccactcgttggtcgttgaagcagattaatcgttcgcaacaaggtacttttaccggcaccggaatatccgatgatgccatagatatcccccttttgaatctgtaagttaacccgatcgaccgcctgcagcgacttgccgcccgactgaaaagtcacactaacatcctgcagatcaatgatggtgttttgtaaatccgccatatttcatccctactttcaaaaaataaaaacgcccctgtactaaagtacagaagcgtttaatcgcgataccattctgagttcacttcgttagttgcctaagaagtctcttcaaccatctcaatttgaaatggcgtgtctaataacgaagacgaacccgtctgccattttcattctgtgatcatgacagccaatcatcggccattttcaccacccaacagcgatcgacttccacccaatgtcgactctcttgacgctgtcagataactactctccgattcattttgtttaaatctattcaacattccaaacacttttcgccgtcttgatgaccagggccaatttatgccactgatcgtcttccgttaagcgattgccctcttcagttgaggcgaacccgcattgaggagagatacagagattgtccagtggaacgtactggctggcatccctaattctggctttgagaaagtcctctttttccagttgagggcgcttgctggtcacaattccgatcacaattcgttgatcccgacggttatcagcaatcttcttgaggggttcaaagccacctgaacgctcatcgtcgtactccaggaaatagccatcaatgtggagctgagccaggtaatctgcgactggatcataagcgccggccccagcccatgttgagtcgtagttgcccttgcagacatgcatggtaatcgtcagatcatccggcttgttatcgacaatcgcgttaatcgctttcacagccgctttggccaatggcaccagttccggtcgcaaagtctgcttggaaaagctggcccacatcccccacgaagtatcatcaagctgcagatagcggcaaccaaggtcatagaaatgttggacggtctgctgataagctttgatttcatcatccaagaaggtgtcaaagtccccatcgtaatagttgtcgaatacctccgcatccttgtttgggaagaacacggatggactgggaatcgtctgcttagctgtaatgccagctggaacaatgctgttaaggtatttgaagccagcaaagaacgggtgatccgggttgtaggcaatcttgccggtaaatcgaatgccgccctttcgcgtttcctcgccatgaaaattgtagccgtgctcaggttcaaagaactcagcgccattcaatccggcgaagaaatcaagatgccaccagctccggcgaaactcaccgtcagtcacatccttgagtccaagggcaacctgcttgtccacaattcgacgaatctcttgattttcaacctgggttaaatccgcttgggtaattttttgggcatggtaatctgctcgtgcttgcttgagttttgccggtcgtaataaactcccgacttcatcatatcgatatggaaattttaattttgctgcaactgtcattttgaccactccttattttttcgaataaaaaagtcctcatacagaataactctgtacaaggacgatattaatcgtgttaccaccttaattttcacacagctcacaccatgtgactcacttggtactcaaccaacttgaataccgcaacgcgataaggtgcgttcgccatgtcatcttgctggtgctcgacgacattgtgctcaaagaccatcttcaccgatttttcgccatccactttcaccaaatgtggactctctaaagacgcttccacgactactcatcttttcactgcttttgtttatcaatttaactaatgagtttaagctaaattatgagaaagtcaagggcgtattttaatctgaatggttttgaaattagaacaatacctgttaaaacgctatttatcgcgattaaagtgtacgatattctaatgaaattttcaagattcacggaagattaccaaactttctcatcacttcagattgcatccctgaaataaatcatctatgattcaaactatatctgtgacactcatttaacaaatccaccaacatcaaggagaaatcatgcaaccaactcaactagccgtcaacttaatcaaacaaatgccggaacttcccaccggctgcgaaattaccgcagtcacaatgatgctccaatacgccggccaacctgtcgacaaagtgaccctggctcacgaaatgccctacgatgccagcgattggaataagggcttcgtcggtgacccatttaccgagaacggtgacagcatttatccaccggcactagtcggtctggtcaccaaatacgccggtcatgcggtggatctcagcggcaaatcaatcacccaattaaaacaattcctggtcgaaaagcaacacccaatcgttgtctgggtcggccaattcgatggctttgccactcatgcgctggtgatgaccggctttgacgaccaacaggtttattacactgactgctggactggtgagcggactttcatgccgacagaagattttgagcaaatccgctcaaagaaaatgaagctggcaattagttattagaagtcttcgcaagccttccctgaacgaatacctgcttcacgtccgcctctgaagcgtggtacatgattttttcaaaaatttgatccatgctttcatcttcgaaagacttcaacggtgacttgaccacttgcaagtcagccaaatagccgactttgatctggccggtcttcagatgcaaactcttggccccaccgacggttgccaaatagaacccatttttagcagaaatcggctgctgattggttccccgctgtgccggtgccagttcagaattcaccccatcatttaacatccgcgaagacatcactgcttggcggatattttgatagatgcttggcgagtaaccaccggaaatgtcggttcccaggccaattttgacgtggtgttgcaggagcttgctgacgggcaacaccgcattaccaaaatagacgttggagattggacagtgggcaaccgccacgccgcgggctttgaaggtatccaggtcggcttgattgagcagggtgccatgagccatcaccgatttatcagtcaaaagaccatactcgtccaagacttcggcatcccgtttgtggtagtgttccagtgcataaccgttctcccaatcgctttcgctgcagtgggattggaccggcaaatcatatttctttgccaattcccccaggcccttcaatgattcaggcgtacaactggggacaaatcttggcgtaatgactgccgtttgcttgattggggcactctggttgagctggtcaatttgttgaatgaaacgttctgtgtcatcgactgcactttgagccgaggcatcccgatagttctcaggcgtctgatcaggattatccatcgccaccttaccgataaagccccgctggttgtgattgacgcaagctttcgccaattccaggttggcggggttatctacactgccaaaatacaggacggtggtcgtcccatttgcgagcaattcaccgaccagatcgtcataaacccgcttggcgaacccgacgtctttgtacttggcttccatcggaaatgtatatgtatcaagccattcatttaacggccgatccagtgccaccccggcattgggccactggggtgcgtggacgtggaggtcgatgaagccgggcaataggtattcatttgacttcaacgtgagcaactgatcattttgctcggcgtcgcgcctaaccgctggaaaatcgtcatctgattcattgatcacgcgctcgatataaccggaatcgtcaatgcagaccaactggtgctgttggcagtcgacctcatcaggtgttgcagcagtcatggtcgggccttcaattacttttgtgattgtgataatagccacctcagttttcattattttttaaactaactattcaaattccctatacaaagtgattatatactgccaaatgtcccgactcaatgcatgccatttcaccaatacgaaatggcatggacttttcaacaagaaatgtcggataaatctgtaggaagtgccaaacatttccaccccgtcacgatttatactgcggacgaagtggtgttcagcagtcaggttaatcgttattgagggggttaaaatgatgactcaaaagaggtttattcaggaattgttcattagttcggtggttttgctagggctattggtgggcacaaccggctcggttaaggccgcaagcacccccaccatctcagagctcaccagtttcatctggcatcgtgcagcctttagcggccgtaccccatcagaccggcgaaattgggacagtgacataccaaattagtgatggcattctaagtttgagtggtgggaccatctcaagccaccccgaagaaacctatccatggaattttaatgaaacgatcaccaaagttgagatcaatggaccaattattctggagggaaatgcggcccgtagtttctttatggcgttaccaaatgcgaccgcaatcgaaggcatcggccacttagataccacccaagcgactgacatgagccacatgttcgctgatgataccaatttattggagctcgatttgtcaacgttaaatacagataacgttacccgattcaaccagatgtttgcgggagaccaatctttaaccactgtgaatgtttccaagtttgatacatctaaagcagaattaatgacgggcatgttttccggcgaaacttctttaaccagcttagatttatccaactttgatactcataagccgttgctttacggagcgcggaggctgtcaaatatgctggcatacctgaccagcttgaccactctcaaactaggtccaaacgtggggtttggccctgccgagagtatcggcgatccacacctgattgccccggctggcgcagacaactggcaggcagtcggcagtggtaccccagaggatcctgaaggcccagtatactcgcccgatggcattcgcgggttatatgaacctaccaatcctgaacacccaactgaagtggaaactttcgtaccggaaaagccgtttgttgatcaatcggctatctcggttcaaccaacatacagtatgacaaccggaaccaagtttgatgtcagcaaggtcttcaactcaattaccacaccagaaggcaaagtcggctacattaccgccaatgccaagtttgtcactaatctctactaccaatcattgcctaagaataaagagattacgctcattgcaacacgaggcattcaagcctacaagaataagaatttgacccgaaagacaaaggcttacaagcaaggcacccatcttcgagttaaagcgatcgttaagcataatctcacgacacgctaccagttgagtaacggttactttgtatccgccaataagaagttagtcattcagggaaaagcttaactgaaagcagttcatatttttagccaccagtatcctgctggtggcttttttggatgctattgagaatcagcagcacaaggaaaacctatcgtggactttctcacaacaatgcccctgcaatctttgtacaaaccaacaaacaaatctctccatcttttccctatactgaaggcaaattgaacctggttcaggttttgacagtttgtaaacgttgagggggcgttttctatgaaacagagaaaaattgtgatcaaagtggctgttgctatggccgcggccatgggtttgcttttagggacggctgccagcacgaatgttttgactgaagcagccgaaacaaataccgctgttcaagatgagaccgccagtgggcatttgggtggcccagatggtccagactggacccgtgacggcaataatttcaatttaacgggtggtgtcctgacggagagaattgacaatcaattgacttcaaatataggaacggcaaccgtgattaatattacaggtaagctgtatcttgagggcgaggcctcgcgtgagttgttttcctccctcaataatgtgaccacgattaacggcatggagaatgtggatacggcaaaagcaacgaatatggagttgatgtttgccgaagatcaagcactcacctccattgatgtgtcgtcctttgacacccgggaagtcaccgatatggcagcaatgtttgctaatgacagttcaatgaaaagcatcaatgttgccaactttaatactgataatgtgacgattatgcccaacatgttcgccgatatgcacgaggttgaaagcatcaacgggaccaatttcaatacccaaaaggtcacagaaatgacggcaatgttttggaatgatcctaacttaaagacggttgatgtgtcgtcttttcaaacaccaaacgtcaccagtttcagggcaatgtttgcggatgattcaagtttgaccagcctcgatttgtcagggtttgacacccaaaagctcctaggatattctaacggaaccctcggactcatgctccggggaacatccagcctcgccaaactgacactggggccaaatattcaatttgataaaaataagaccattaacggcgcgtctgctgggctcccatcactcggcgcccctgccggctctgaacgatggcaggcggtcgctgccgataaaggcggtaccgccgacaaccctaaaggagcgactgccttcctccccgatgaattgacttccctttatgatcagtcgaatgccaatcatccaaccaaggttgagacttgggttccctacttcaaagacactctggatgttaaatcaccaattaacctgacagtcggccaatcatttgatcccaaagcaggatttgtctccgcagccgatggaaatggtcaaccggttacttatgaccaagccgtcgccgaaggaaagcctggcggactggcagttgacaccagcggtctcgacacctccaagccgggaacctataacgtcacctacagctaccacatgcgaaaggccattgtgaaggttattgtgagcgcagtccctggggtgacaccaaatccgaccccgacaccaaaccccaatggcaataattccggcaacagcaatcccgtctggaatcccaccaatccaaagaatccaaacggtactggcctgcccaactttgccaatgtgaaaaacgatgcggtctacgcaaccaagaaaatttacctctaccaaaatccaactttcaaaaagtcacagcgaatagccgtttatccaaaagctaagcgaatcaaccgaccaatgtttgtcgtcgtcgattttgccaaatcaaatggcggtgccctccgaatcaaagtgcgtgacgtcaatcacggcaaaaagactgctggcaaggttgggtacatcaccgctaatccaaagtatgtaaccaacgtctactaccagaccatgccaaaatccaatcaggtcaaggtgatcgccaccaagggtgtttacgtctaccagaatgctaatttgtccggcaaggccaagcactacaagaaaggggctcgtctgaccgttaagaaattggttaaacacaatctgacgacccgttatcaattaagcaatgggcattttatcaccggcaataagaagctggtcattcatagccgttaagggcatcaattgtttcagaaagtctgcgcactctcaccatcaactgttacaatcaaagtaatgggcgtgatcgttgtgtgcgcatccgacaatttggctttaaccttcccgcccagaaaatcactcaaggaggaatttctatggcggtattttcagaagaacaacggctgcaaattttcaaagagctcgtcgcgattcaatcggtgaacactgatgaagaaaaggtcagcgcttatttaaaaaatctttttgagaaacatggcatttcggccacaattatcccggtcgatgaaaatcggacggatctaaaagcagaaatcggcactggcagcccagtcctgggagtctccgggcacatggatgtcgtttcaccgggggatacctctaagtggaccagcgacccgtttacattgaccgagcgcgacggcaagttatacggtcgtggtgctgctgatatgaaatccgggttggctgcaatggtgattgccatgattgagattcatgatcaaggattgctgaaaaagggtcggattcgtctcatggcaaccatgggcgaagaagttggcgaattaggttcacgaaccttcgctgacgatggctcaatggacgacgttgatgcactgatcatcggtgaaccatccggctaccgaattgcctatgcccacaaagggtcaatggatattcgcctaacctcaactgggaaagctgcccatagttcaatgccggagcagggctacaatgcgctggatccactgattgatctcctgcacgacgccaatcatcaatttagaacaacaaataaaaagagcgcaatgttgggaaatctggcatttaacacgacgatcttcaagggcggggatcaagtcaactcaattccagccaaagctgttgccgatatcaacgttcgcaccatcccagagttcgataatgatgtggtcgataagctactggatcaactcgttgaacagcaaaataccaacggggccaaaatcgtcaaggaaacttacatgtctcaaccatcagtcgaaacgaccggcgacaaaaagctgatcggcttggcacaggaaatcggcaaacaatatgccgaaaaagacattccgagcggtgccatcccagctgtcaccgacgcatcgaacatgctgcgggataagccgaaggaatttccatttatcatctttggtccaggaagtaacagtgtccaccaagttgatgagtttgtcgacaaacagatgtaccttaactttgtggagatttatcagaagttgtttacgcagtatttgaactaaagacgaatccaatcaaatagcagccgtcaaaccacttgcttgtgatttgacggctgctgttttgttctgatagatactaccaagccaactcataataagtgaaaaatgcggtgccagccccgacccacacgagcaccatgatcacaatcatgagactcttaacggccgcattaaaaattgtgtaatcagcgaaccgctggtcaatccgcttgggtgcagaaatcagtcccagcacgattaacgtaacaggtaagataaaaatggtcattttggtgcctggactgtctgcgacgccaaagccaaaatgagtcggaacaatttgaggtaatcgtggataaaagacgatggccgccattgcggtaattatggtcacacaccagtggacggcaaggattttagagtaaactttggaaatcagaattgagaaattcatgtgggtcgcttccttagtggctatgtactttttgttaatgctgtggtaatcatatcacggttaactggtaacacaatccttatttgggcatcggatcgaattcatttgaaagtgaatatccaaacgcctaacaactagcacaaagtccccgttgatgatacgataaaaccaaaattatctctatcaaacaagcataattattgcatcagtcaatcaggggaggaattattatgcagtctgtggatgaccagttaaagcagttatcaccagaagaactcattaaattaacgtctggcgccaatttttgggaatcggtgacactgccagaccaccagattcccagttttcgaatgagtgatggtcccaatggccttcgctatcaggcgggtgaaggcgatgcactaggaataaatgacagcgctatcagcacctgtttcccaacggccagtgcggttgcctgcacttgggatccggatttggtcgctcaaatgggccacgccatcggcttggaagcccgcagcttaaaggtggatatggtgttgggaccggggatcaacatcaagcgaaatccgctttgcggccggaactttgaatatttcagcgaagatccttatttagcaggcatgattggtgccggttggattaaaggcctacagtctgaaggtgcggcggcctgcttgaaacactttgccggcaacaatcaagaaaccgatcggctgttatcaaattccatgattgatccaactgccttgcacgaattgtatctggaagccttccgaattgccgttgaatctgcgcagcccgaaggcgtgatgtgttcatacaatcaggtcaacggcacttattccagtgataatacctatttgctaagcaaagttttgcgtcagcaatggggattcaaaggcgccgtcgttactgattggggcgcgctcaatgacaaagtcgccagtctgaatgccggcggcgacctggaaatgccatccagtcacaacatgttcgacccgcaggcgctcgaagctttgaatgccggccgactcaaacgaccagctcttgaccgagcagcgggaaacgttgttcgaattgctgagaagcagcggccagagttcactggcgatcgcaaggacctactgacaaaaaatggccaacttgcccaaaagattgccgaaaacgccgcggttttattaaaaaataatgatcacattctgccgattgacccatccactaagctcttggtaatcggccagatggcagccgaaacccgttatcaaggtgccggatcttcccacattaatcccccatctcagacctccattttgcaaggattaaccaatgccgggattgcctacgattatgcgcagggctaccaatttaccggtgaaaacaaccgtgaattggcgactgctgccaccgatgctgctaagaatgctcaaactgtcgtggtggttgcagggttgccagaaagtgccgaatcagagggctttgaccgtcctaacatgaagctgcctaataatcagaatgagctgattgaacaactggcggcggtgaacccgaacgtgattgtgttactggttgccggagcgccggtagaattgccgtggcgaactaaagttaaggggttgatcaacctctatttaggcggccagtttgtcggcgacgcagcggctaatttgttatccggtaaagtcaatccatccgggaagcttgccgaaagttacccgattacctatcaggacgttccgtcggctgaactatatgaccacaatccacgttcggctgcttacgccgagagcgtctatgtcggctaccggtactatgaaaaggccaaccaaccagtcgccttcccgtttggcttcggtctgagctataccagctttgaaatgagtcgtttacagttaaatcaacaccaaattgacgccggccaatcgattaatgtcaccgttgacgtggccaacaccggcagccgtgatggggccgaagtcgttgaggtttacgttggcaatccgtctgaccgcgccttgaaaccattgaaggaactgaaggcctttcaaaaaatctttttaaaggccggcgagaaacagacggttacccttaccttgcctgctcaagcctttagcgagtgggatgagcaacagcaagcctggcagctgcccgcagtttcgaagaccatcatcgtcaaaattggatcgcgccttgaggaactcaccgcaccagttgaagtaatcggccaagccatcaccccaactgattccatcccgagttggtacacccatccagtgggcaagccgacgatcgccgatttcaccgaactgactgggatgaccgttgcgccaccatcaacgccggaaccggggcactataccccattgaacacaccgcgggagctgagtacccactcggcgattattcgcagaatcgtttcagttttaaaagccaacatgaccaagggcatttcagatccaaatagttctgaagccaaattcatggatgccatcgtcatggacacgccactgattcggcttgctcaacagtccagtggaaaactctcactcagtttggtccacaaactagtcgcacttgccaatcggcattatattcaggcaatctttaaaaactaatcgttgtatgtaagggggaagtattatgacacgaggggcaagatggcggttggcatccgcacttttatcgatttcaattctcttaaccagcgccaatgcggtcgccggaaccattccgatcatggcggaacggttcccgtcgattccactgagccaaattgaaagtttgaccaccattcccagtttgagcgtcttgatttttgtggtcttgagtaatccgatcgccaaaaggttaggcaacaaagcaaccgtgttaattggggtcttcatcgtcctgattgccggactgattccgactgtcgccaattcattctggctgattttgggatcgcgattcctactgggtgccgggatcggcttatttaacgcgatggcctacagtttaatcagctattattacgagggaacgcaacgccagaccatgatgggctatgaaggctcggtgaactcactgggcaacattttgatgtttgtgttttcctcaattctgatcgggtttggctggcgccaagtctatttatactatctgattgccatcccggtcttcatcctgttttggtggggtgcgccaagtgaccgccaggaaaagcaaccgcaagccgatcaagaagcggccgcaccatcagttggcttgggggaactactgaaaggccggttaatgatttatgcattattagtattgttcagtatgatgattgcccagacggtgatcgttaaaatttccgggctaattttaaccggcggctacggcaaaattgccgatggcagcattgccctggccttcctgggggtcgccaacatgattggcgggactctttacggccagatattcaaactcattcatcaattgattttaccggttggcttgctgattgccgcggttgccctgtttgccctggcgcgatcccaatcactggcgcttacctacaccctcacggtggttgccggattaagtacgtcgctggttggaccctacttgtttgccagttctgccgaaatcgccggcaaaggcaacgaaaccttggcctcttcaattctgattgtgggaattaatatcggtgtattcttaacgccatacgccttgtcgggattgagccatctgatcggcagtgatcagccggcaccgattttaatcgccgtcagcgttgtcttggcggtgattggtgcgttaaccttcttcatgaaagaacccaatcagcagtctcaatgatcacgccatttctaggccatcttaatcagtccaacgccgatgagcatcagcaccattcccaatgcttgagcaggcaccatctgttgtttggtggaccgccaccagccgaattgctgaatcagaatcgagccgataatttggccgatcaaacccatcatgatcgttaggccagcgccaatttgtggaacggccaccacggtcacaaataaaaatgtgccaccaagaatgccacccaaccagttccaaggttgggtggttttgagttgactggcggtggggacacgtttatcaatcatcagcgcaacggcggcaatcaaaagcgtgccgatgaaaaacgaaatgaaggccgcttggctggtggaatgcagtaacgttcccaaatgaccattaattgcctgctgcatcgcggccaacaccccaacaatcaccgcccaagtttgccagccaatcacgcgtgtcggcccgtcttgtcgagtaacgttggcgtcaaatcggcggacatcgcgattggtgaggctgggtaaggcaactgccaccagaacgccgacaatcaaaatcaggatgccaaccagccgccaagcagtcatggcaactttagccgcaccgaaccaccccaaccaatcggtcacggttcccatcgtgatctgccccataatcggtagaatcgtcgtttgaatggcaccaattttgggaaacagtaggatatttgacgttagataaatcgagcccagcagaccgcccaaccaaatccaggctggctgcgcttggatgaatctgccgcttggaaacagtcgtccagtcattgacatggcgagaatcgctaaaaacaaggtgccgataatgaacgaaatcgtcccggcaataaacggcgatttcactagccggcttaaatcggcattaatgggactttgattagacaacaggaacccggcaactagggaaatagtcataaaaatcagcattgttttccaccttcaaatcatgaaatcagactatttgatacacgacatatagtcgaaagaaaagcagtcaactatttcaggttaactgcttgtgtgaatgattggtcacgtaagtaaagatcaccagtttggatgactgtattatacaccgcccatctttgaaatctgaagatgaaccgaaccactttcccgaatgcagcttaaacaacatgcgcaacgcaatctccataaatgtgattcatttaataaatgtaatcgctttcaagactccaactaaggtgctatcgttaaccacgaatcgtgttcctcatgagtttaaggaggtcatcaacatggcagagttggacggaaaagttgccatcatcactggtggtgccaatggaattggtctggaaacaacgaagctctttctccaggaaggcgcaaaagttgttttcacggatgttaatgcggatgcaggtaagcaggtggaagatgaattgaataaccagaacgccctattcatccaacaggacgtcggtgacgaagcagcttgggaaaaagttgtgaagacgacgcttgatcaatttgggacaatcgacattcttttcaataatgcgggaatttacattattggtaaaattgctgatttaacagtcgatacttggaataagttaatgcggatcaacgtcttgggaactttcttgggattgaagcacgtcctcccagtgatggcagagaaccatcacgggtcggtcatcaacgcatcatcaattgccggaattgccggttcagccggtcatattctctatggtgccagcaagggtgccgttagaacgatgaccaaggacgctgccgcggagtacgccagcaagaacgtcagagtcaactcaattcatcctggctacattaaaaccgggatggccgactacgcctcagcatcccttgggataccagagaatcaacttggcaagattttcccgctgggtcgtttgggtgaacgaatcgaagttgcccaaactgttgtctttctggcatcggataaagcatcatttattactggggttgagttgccgattgatggtgggttcttggcccagtaataagacgattatttgtcagaaagcgactgacgggtaaggtttgaatgctccggaatatcgtttcaaagaaagatgtttcctccattaggaacggctctcaaaaaaatgggagccgttttcattacgaacaagattcattttgcgatctgcttattaaggaatcgtcaaatcaccacaaatcttttatacttgagataaacaaaactgcactccaatgaaagcagaaagaggatgctgacaaatgacaaatccagaaatcgtgtcctaccccgccatcttcagtaaccaagacaacgacagctattatacggtgacattccccgatattccagacacagtgtcacaaggcagaaccttggaggaagcactccgcgaagccccagatgcaattgccgtcgcgttacccgattatgcggagtatcccaaaccgtctaatctccaacgagtacaggctgaaaatcctaacgcaatcgtccgcttggttcgcgtaaatatgaaagaaaagcttgaagcaatgagatcaaagccaaataatattcatcaattattcagtggctggtcagatgatggtataagagatactgaattagactggggagatcggcaaggacaagagtttaaataaggacttgatcaacagcttttaattgcctgaattctacatcggatcaggctttcaagatgcagaatattgattcgaaggagtttgaaaaatgaaaacaataaggcatctttttatcatcacaatcgcattctttgtattcatcgcgatctcaaccgtcatggttcgcggtgattctctcgatgaggacactgtgcctgttaatttgaccaaaaaatcgttggccaaaatagaaaaatcatattcagatgtttggaacaatgtaaagtattaccgtgtcaacaaaactgtcagactcaaagtaaagtttattgatcgagatacagagaaaacaaccaaagttgccagcatcagagtacccaaaaacaccatcttggcgggaagtaaggaccacgttgaggaaacaagagaaaagttcatcaacacgtttggcctcaactacgacaccttcagttatcgattcttgaagcccgtccttagttccagcatgaacttattcacatatgatgcgttcgtcaatgcaaaaaagatgtcatcaatcaacaagtatttctcaagagtcaagcgcccggcgtatatgcctgcctattcttcaggatcactctatatttatcccactaataagaaaaaattcagtccgttcagtccaacgacaaatcgtttgaaaataacctctgatggatacctggaattcaccaaaaataatagtcctgacgtcgaaactaataagtcatttaatctgactccagattcacatgtcaaaattaacaagacgatcctcaaaaataattcaaggtatttatactacgcacaccatttggcaggtgttactgataagcaggtcgcaaaagccggtaaaaatatgtatagattaacaattaccaacttgcatcgacctttctcaatgtttgacggtgatcaaggagccgtcttaatgagcagatacaaagttggggacactgtatattacacaagtagcggcggatatagtgcgtagggagcccttcactggcgattccacatcctaccttaagcgcaaaaaaaccctggcttgatcaccagggctacatatcactcaacctatccaaagatgtgttttctaaaccggctgagaaacattattaaaatagtcaaccaaaaattgtgaaccgttccacgtcactttagtaatactcccattgattgttggcacgtaaacgggcagattactccaatgcgcaactaagtttcgaatggcggttccatgagttgcaaccaaaatctgatcatggtcagcggcctgagaaataatttcttgaatgccgcttgagaagcgttcccagaattcagcgctggtttccgcatcctgataaggatccgcagaggcaacacggtcctcagcctcttcaattgagtgttttaaaatcatttgctcaaacgagtcaatgccttcttctccgcctaattcatgccacaactgattttcatcattgccttcaaaatacccgtagttcaattcacgtaatgcttgcattggcttcaattgcagttttggagagacttcctgattttcctgtaatatcagcttgccggtattaattgtccgcattgtatcgctggtataggcttgggtaaaatggattcggctcagccgactgccggctctttttgctgcggcaattccctgctgagttagcggagagtcacaatttccttgaatccgattatatttattcaagaacgtttgcccatgtctcacaaaatataaagtaattgacatcaattgtgcctccttcgatgactcaacttcgcagtaatactgactggtctctttgagcccaccaagttaatcgtgattagcgattactgaatgtcaataaacggtagttgaaataacgttgccaaatccttaatttgttgttctgaagcagtaaatgtcaaaacggtatggtgaccgccgccattttgaatccactcggttgcaccatgtttcagacccatctttggagtccaatattgtttggcaattggcagatatggtgtcttcttagtcggtttgtgggcagtcacgccataaccgatcattctaaattcggttccaaagtcagaaatggttacatccatggcatcgccatctattccgtcgaacacgaggcgggctggatcgtccttaccaccaataccaagtgggtgaacttcaacccgtggcttatcactggcaatcgttggatcaacttccagcatgtgcgagcccaagatggcttcgttgcctttggtcaattccaaagtgtaatcttccataaagacagtccgatcattatgggtcataaccttaagtaaacgatcaagcgcagcggtcttccaatctccttcgccggcaaatccatatccttctgccattaacaactgcacggccagacctgggagctgttccatcccgaaaaagtcttcaaagttggttgagaatgctgtatagccacccttgtcaagaagatgcttgatgccaaagtattcccggatctggtagcgaacggagtgctcgtattttgcagcatcattatcaccctgaacgaaggtatacttttgttggagttcttggtacttattgtcgatatcagtgtcagaaaccgaattgatttcttcaaccaaattgccaactggccagtaatcaacggtccagccgaattgaatttgaccctgaatcttgtcaccttctgtaacggcaacatttcgcatggtatcaccaaaacgggccactttgatgttgaaactttcattgtaagcaactgcaacatcttcccaatcggcaatttcttgttgaatttctgggtcagcccagtgaccataaatgaccttattgtgcttctgaagtcttgcgttgatgtagccgtactcacgatcgccatgggcactttggttcaagttcatgtaatcaaagttgatggtgtcatatggaatatgatccaaatattgggtagcaagatgcagcaatggcttttgcagcaacttagttccgtgaatccagtttttagctggggaataagtgtgcatccaagtaatcacaccagcgaccttatctgtataattggcttccttcatgactgctgtaatttcatcagcggtggtagcgacagctttaaatttaattgggtagggaagcttgccggaagcattcaatttgttgataatatcttccgtatcagaccgaacctcgcctagtatttcttcgccatagaggtgttggctgccaacaacgaaccaaaattcataatcagggaccttaagcattgatatttctccttccgcaactttcaaaatggggcgtttgaagttgacatttaatgaaaaatcattaaatttgattgtattattgaacgttgtttcgcctgtctgttctaatttccagaacttggttcataaacgtttcaacacagtcatcataagggaacactgactcgataaatgcacgatattgcatgaaaaaatatacatatttgatagtaaatgatcactatttcaatcttgaaaggaatctattatgagaatcgcatttagcaacctgaatgacaccatgcccatttcttgcgaatcaattggctatcactggcggcagtatccaatataccggcccaatggctaccgcttttttcactggttacaaaccgaaagcagctcgggaaccgtcaaaattgatggccagcaaatccatctactgccaaactccggcattctcattcgccacaccgttccgcattcttatagcgccgactcggatgccaaagaatgggatactgcctacatcaccttttacggtccacttgcgaactacctggtgaactatctggacgtcgaggactatcgggtgtttgaagatttacctgaaaacattaccaattttatccaaagcaactaccgggcatttatcaacaatacaattgccgaccaagccaaccaatcagtgctgatctatcgctatttgctgctgcttcaccaaatggatatcgtccatggccaacaaagcaaatccgatccgatccgatcgttaaccgtatcaccagctttttggaaagtaattatcaatttaacattaccaatcaaagcatcagtaacatcaccggcctgtcgattccttaccagacgaatattttccggcaaaaatacggcgtgaccccacttcaatatttgtttgactatcggatccggcaagctgcctatctactcgtcaccagaaaggatctgcaagtccaagaagtgtctgagcaagttggcttccccgacacatccagattcattaatgccttcaggaacttttatggggtgacgcctaagcagtatagtaagacggcgtatcagggtaataattgatgacgaaggctcaattaaaaagcaagaagtgacttataacggaatgccggttacttaacgatttgcaaaacaaaaagtgaaccgaaccccttgaattagatttctccaattcaaggggttcagttcacttaatcacaagatccgcttcacaaaaggatagtcgctacaaaaagattttgttaacaaaacacgccaaccgctatgcaactcggattgatcaattttatcagcaaaataacaaagaattaaggcatgttctcggtgacaagaatacagatactcttgtagaaaatctgcatcaaattcaaaaatattttgatgataagctgaattgacagacattatgatgatctctcaaagattaatagattaactggtagagcctactccgacaattttctacgccctgaacaaacatcagcagccctgaacagctgatgttcgttcagggctattttgtagtgttctgattattacatggcataaaacatttattaacgggagcgttaaagatgagcgaaccagactttcgtgaagttaatcgctcctgctttttgactgataaattggcaataaaacatcatcaactaacaattccaatttgcgctgcgttaacggctgattagtaaaaagttgaaatcttagccaatcgaatggtagcaatgcaatctcttcaggcagatctgtttttatgatctcgcctcttttttttgcccgtgtaagaatgtgatcaagagcattaagatcgatcgcatttccttcgctcattaattgttgaatcgtcgtattttcttctttagttgcttcccccagcagttctgtaatacggaagtccttaaatgtttgcatactaataatgaatcgttgaagcagctgcaataaatcctcgcgtaacgaatgaccagtcaaagtgaaatcatccgttcggccgtgattttctgacgttatcttgtcctgaattgcggcaactgccagagagaatggcgtctgccatcgacgataaataacagatttactggtgttagccaaatcggccacatcagcgaaattgaaacttaaaaatcccttagttttcagaagctgtaaagctgcctgataaatcgcttgttccagttcggcaccccgacgacgtttttgaaccataatgatgactctccttttttaagatactttaagtatcttattgcattttttatcttcatagtgtattatatcaattattgttttaagatactaatagtttcttatttaggaggaaaaatgtaatgaataaacaaatcccaaaatccacaatcatcatcgcttgggttgtcgtctttggtgcaatggccccattacttgattcaacaatgattaatattgctattaataagttagttaatagttttaatagttctgtcacaacagttcaatggaccattacctgttatgtcttggcaactggaattgctgttccgttttcaagttggttattaaataaatttgatggtaaacatgtctttatgctcagtgaaatcttattcggcatcggttccattttagccgcagtttcaccaaacattcaatttctaattggagcccgcctggttcaaggctttgctggtggcttaattatgccgttgctaaccacccttttagttcaaactgctggtgccgccgttatggggcaaatgatggcaacggtcggtttacccatgatcttgggtcctctgatcgggcctgtcatcggcgggattattattaaatttttgtcttggcaatggattttttggattaacgttcccgtaaccttgacgtcactcggtttaattatttggaaaatgcctaattaccctgcacaaaataaatccgcaaaattagatctcatcggaacactgcttctgattggatccagcaccagtatcatttatgggatggttaaagctgcccacaaggccaattttagcaacccgtcaacactcacttttttggcaacgggcgtttcgctgctaattatctacgttatttggggcgccattcggggcgaaaaagcagttattccgcttaatttgtttagacatgggtccttcaatggatcagttattggcttgtttattgctggaactgttcttaatggtgccatgttattgttaccactctttttccagaacgtgcgtcatatgagtgtcttgatggcctcactggcgttgatcccccaaggattggggatgttgatttcccgcccactcaccggccgattgaccgattcaattggtgcaaaatatgtcgttcttgtcagtgtgtttattgcttttgttggtacgattcctttttactggatcacccaaagcacaccgtactggatcattgccgttgttctgctggttcgtggaattggggccggtggtattttgacgccattgatggctgactcttattccggaatgaggatcgaccaaatttcgagcgccacaatcggttcacggatcttgcaaaacatcggcagtgcctttggttcagcattagttacaactgtcgtaactgctttttcagcttcgcacgttaaaagctttcagcatcaattaaaaacgggtagcctcaaaccggcatcagggcaattggctgcttttatccaccaacatttagttgctattcgacttgacgcatttcaacagggatttttaatgatttccctggcagcactgttaatcattctgccgaccctactactttctaacaaaatgaaatcaaaagaataagcagatgcaggttgccaaactacgtgaagtattcaagagcctcgcctgaaggaaggttgattcgatcatgaaaaacgatatcttaacaatcattcatgggtggtacattgcccttggcgttgtcctatggcttacactcgttacaatttttgtttcgaaacgatacctcagcagctccccggttaattgggctaaattgtatttaactcctatactatttattgtatttggtattgagaaaatcgtccgctttcgacatttggccgccactttaacaattttcttagtgattattgtgttagccagtttctttggtgctcacttggcctacaaataccaatcttttttctggcgagaaaatcaaatcaaaatgattggcggcaaatacgcgattagtttaatgattatgaatgtcatcgtgatgctgctgattaatttccatggttgggtaaaccctgaaagttatgagacttggtcatatacattaacctatgcaatcacttcggcaattgttaaggggttattaattggccaatcggttaatatgtggtggcatttgaaggtattgcctaagaagctgtaaccgttagttgatcataattaacacaaaaatgagctgtgtcctcgaagataacagaaagaattcgaggacacaactcattttttgtttgataggcttcggatttggagacctatcttggtaaaagtcggcaatctcaagagggaaaagaaagtcagtcaaccaaaatctcattgaactgagaggtacttcttgaaagacatttcatctttacgcagacattcaacatgtctacaaagactacactccaagcatcgcaattggtaatacatgtacccgatcctgccgtgtatatgcaaactgactagtattcaaaagaaccttggtcacgtcaaattcactcttgaccaaatcttcaaaccaattcaagtgacgaacatagtcgtctttggcttccggatccgccttaacttcaaataaaatgagggatttacctttctgcaaaatgaagtcaacttctcgagtcccttggtgatttctaaattgagataagttagcatcattagcgtccgcgtatactactaaactttggtaaaccaaagattccaataattggccaagtaacgtttgattgaatttgccaacatattttggaacctgataagtttctaactgctcacgatttactcccaacaatttaagagcgatagcaggatcgagcatatagtgctttggcgcctttgctaaattagaatagattttaccgacagctaaaaatggaggtacttcgtcaataatatatagaatttccaaggcttctcgatagttcattgccgttggcttactcggagcttcaccactatttgccattgctgcgttaataattgtctgaaactttgtcgttgttccgattgaggctgagtaagctttcaaccacgccagcaaactttcaggtttttgtattttaaacccattttcttcaaagtcatgctcagcaatattatcaatgtagctttgtaataataagtctcgggcatgtggtgctttcaagcgaataccaggaaaacctgatttgaatatttcatccaagtaatcgttaatattattctgagtttgcccagaaatcttgccttctttggacaactcaaacaaacgctgaatggaaatatattgtttagacatcccccgttcttcaatcgtatacggccgtaacttcattcttatgattcggcctgcaccactatggattcgtgaattaacacgaatactacttcctgtgaaaagaacactaccatttggtaatccactgtcaacttgatgacgaacaaaggaccaaagctctggggcaagctgccactcatctaataagactggcttttcatccctcaatataacatctggatctccctttaacatcaatctcattgtttcattgtctagactgtagattgtttttgctaattgtaaacaagtttcagtttttccaactgctttggctccctctactaaaattgcaggaagctccatcagatttcgctttaatggttcatcaataattcttttttcatacaccactaatcacccaccttggcatttagaaggattatattttatcttttttgaacgctatattttaccaaaatcatatcttatattttaccattttgcaaccatccgttttacttttttgagagatatatttgactattttgcaagcaaatttttcagtgttggattttataagattttttcgcttgtattgacgctcagctatgtacataaagacaacaaaaagccgcctctcagcgactttctttgatagactcaattcttgacttcagaagaataaccaagtgaaaagggatgccggaaattggacatgcttttcttcattttgtaattaatgcttgtacaaccaagtataacttttaaatgagtatgagaacgcattcttcatcccactgccccaatggtaaacatccactggagattaagtcgttctcctctggtaaaatggccgacatcctactgagtacagaacttctaaatcctactacagggatcaatccttttttctggagtaggcatattctgctgtaatatggcacaacaatttaaaactcagataagccgattacacaagtcaccatatgcttgtacaataactcccggagcctccgagaccacttgagtgttaattctcaaattaaataaagcctggttttcaccgatactatttgctaaaacattgattgctttcccagtggctttatcgacatcacctagcggattgacaacgttccaggtactgccagaaccataaatcatagtttcatattcgtagcccgccggtattggactcatgctgataattgttttccccgctggataagtcaatttagtgatccccacttgaccaattccttgtttatcaccactagaattattcatcgactgaaatagtgcattcctttctttaagttgctgctgcttttttaaggccttagcatctgcggtcttaatacgctgttcgatctcttccctggctgcctgtcgttcttgttcttcttggtgcgcttccagtaatttataaaattgttcataatgacttatcgtctcattcaacaagggcaagaattcattagtgataaatgtgacatcttctgcggtattagcatacatttttaaatcagatttaagtcctgtaacgtcaacctgaacataggtttctttggaattcgtttgaagtaaagtgtgggcgtcaacatacttaaaccaatcatatggcttgccttcgtatgctgaaaacgcaaagaagttggtaatcacatatgtatcgtcacgtaataaccgatgatgctgatttacatagactcccaaaacacggtactgatcatagaaattatcaatcttttgaaatgtttcaaattcagcattactataatccaatatgtttttcttctttgcaatgaccttattcatcagtgtcctagctattcccaaagctttattttcatcttccatattagtcacaatcgccatcatatccatctccattctgtccaaaacatccacttaactaacgattaactggacgcttaatcaaaattggtgaccattttcaatacacaaacttatcaacctgtgagccccagtcccctgttacgtacttcattttggtaaagtaacaccaagtccgaaatggtggaattctgtctatgccaccccgatgatttgtgtggtcaaagtattccaatccccaataccgtttatgattagctagaacgaagtgtcggggcctgactgtctcaactttaagcaggtcagcttctccttgtggtccgaaagtatatgcgcccttcacatttgccggtcggatgaaataaccatcattcacaaaatcttgccgataccagtatcgactgccaaccctacggctgtattcgtaaaccgaatgcatcgtaaaatgtaatttataatagtactcaccgccaaatgggccagtgtgggttgaataccaattgtgagcccgcaatattttaggattggtgtaaattttcgcagccgcaggaatggttttgccgacacttcccattaggctaattcctgtggaaatgcataatagtgtacaaagctttttaaaatccattgttaccctccattttcattgaaagttatcttgttttcgtgcgcccctagcaaatctgactacctcgctaaaaccgtcatcggctcatattttttttcaaaagacagatgctctttaaattgaaatcgatgctgattcacataatatcttcctttatcacatccgccaaacctgccatgaagacttccactgtattgcatgcttcgtaaggcctactcctgtaatttagcaatatcctctgacaaagtatcaccaaaactcgacgccgcactcgttgcttcctcactaagttctaatcccccatcatactgatcatcgtcatcagaactaccgtcatccgccagcgatttattaagtgcagtttgataattgtcataaagcgaatctaacttctctcgatcaaaagtgctaaatcgggacttgaacaagtcataaaactttcctagggtttgatagtcatttagggtctcatctcctatggtttcgtaaccaggatcatccttaaggtcatttccaatttggtaaacaatgctgctaatatccgagctggaagaaggatcgttatatgctgttcgaacgtcgacatcattcagtttctccaaatactcccctctagatatgggattcatcgtattaataataccaatcatggcactaatatccgatttctcttgatcataagtcttggctttaaccaaattcccatgccaagtccaaccatataccgttttggatttgttgaagacgtagtagtaaacggatttaacaccataggattttttaacggtcgttgccttattggtataaaaagtcgtgtggacataatttttgccgttatgaagacgaacttttagctttggcgaactgtaaagatacccgtgagtaatgttgtagggttgcgcatcatccatcgtttttgatgagacaattttgatgtgactcgccgcttgagcgtttgagccattaggagacacaaacatcccaatccccattgatgcggctaatagtccgacgtacgtcatttttgaatgtattgattttgtcattttttacccctccgaaaattgattgtttagttgatgcctttttattttcttgaatttatgccatgccaaccacgatccaagtctttataaacattcaagcgttcacgttaatgactcgtttgtgccagaaagaagtcgttcacaatcccgtaatgctttgtgaatatgtacttggaataacgcttaccccaatagcaaatgtggggcaaagttcgttgaaactttacttaatttcattacatccccccaacaaattatttatagttcaataatctcattttaatcctagtcgttaaccctgacaatggtcgcttctaaattccatcaagcttccttaaggtcactcctgaggggaattttaatatcaaatgaaattagtgtctgagtttattgcagactcttggattgaagtcaaccagtcggaagttctctaattttttgaaccagatgggtatgtaaccacaaaaaacaggtagcccaatttggctacctgtttaaaactgagttgttaagtttcggactctccctatacttctccctgaaatggaagttgagatctgaagatgaacaccccagccagtcgttattgcgtcccccaagagtggaactcggagcatgagggccaaaatcttatctaagctttcaaataccaatcgcaaatgccgaaattattgatatccaagcagtaaaaggcaacgcaacattttgtactttgaagcaattttcaagaactcatcatgattgttaaaacacatgcggtctagctaagttattcagttagattaggaatctcattgagctgagcgatgtttcctgaaaaacatttcagctttacgcaggcattcaacatgtctacaaagactacactccaccatacatttgttacaattagagatgttttgtgtgataatgctagtagaaattggtatgggtctatgagggatatgataactgttaggaggggctagctatggggttaactacgaagtggctctataaaagaatgctttttgtattttgtattatatttggtcttatgtcacttttttctgtttccacaaatgccaataatacagtccagaaatctaaaatagaaaatagtgataatttacgaactgtaaacaatcaaagtgactttccatcttataccattaataatggtgttttaactttgtatactggcactattactgaacgtcctagtaatggttatgcctggaactttgattctagtataactaaggtacagatcatgggtgaaattaaacttgatggtaattccacgtcaggtttgttttggggtatgagtggattaaaaaacattgtaggacttgaaaaacttgatactcagaatgcgactgacatgggatctatgtttcgtgaagattcctctttaaccactttagatatttccagcttaaaaactagtaacgttactacaatgggcgccatgttctggaaagattcgtctttaacaaacgtagatctagatggaatagatacatctagcgtgagagatatgggttctatgtttcgagactgcacttctttaagtgacttaaatttaacaagtttcaatacatctaatgtcatcataatgggagctatgttttggaatgaccttgccttgactaatataaatctctcaagctttaagaccagtgatgttgctgatatgggttatatgtttgcaggatgcgctaatctgaatagtttaaatctttctacttttgatactcggaaagctataagtaataaccattttacagacgtacatggggtaacacagcataataccgttgacgggatgctcatgggcctttctaatcttacagctctaaccttaggcagtcttaatcaatttgctcctcaaagttcgtacggcaacccaaagttgggtcctgcatatggacctgcaaattggcaagcagttgcagccgataaaggtggaactgtttcggttccgcaaggcacaaaatatacacctgacgatctaatttctcactataccaatgtcggcgtgccaaaagagacctatgttccagcagtggacgttcttcctgctccaattaccatcaattatgtaaagcaaagtgatcctaataatgttctaaaacaagtaacaatcccatccgatggacaaaaagtaaatgatccagattatcaatatgatgcatcgcagcctgaatatattcagccatttactacctctgatggcaagaaatttgacgtgattacagatccactgccatcaaactacaaaggtgaatttactgcagatcctcaaacagttacctacaatgtcaaacaggcagacgcgaaagatgttacgattcactactatgaaaagggcaccacgactccagttcagcctgacaaggttcttccaggggcaggtaaatatggagattcattcagcgtggataccaaagacttaaaaccagctaccattggtaattatcaatacgattcaactagtgggacaaccagtggtcagtacaatgatgaagcacataccatcacattcttctatactcgccctgacgccaagacggtgacggttgaatacctcgatcaagatggcaaacctattcacgatccgcaaattattggtaaggatggcaaggttggcgatgaatatgatgcgactaccgacaaatataagctcaagacaatcactggttcggatggcgttgtttacagtttagacaccaacaaactaccaagtaatgcgaagggaacactgtccaaggacgcaattacggtcgtttatagatatgatacgaccaaggcagctccaatcaccatcaagtatgtggatgaaagtggcaatgtaatccacactggtaagacactgaatggtgttgttggcgaaaagtttgatgcacgttcagataaattgaacacgatcagctacggtggtaacacatacacgttagatactaagaaatcaactgctgatagtgctttacagggtagtttcagtgccgataaacagagcatcacctttgtttactcgaagaatgccacacctgttaatccaattaaccctgtaactccaataaatccaacgccgacaccgacacccaccccaactcctactcctcaaccacaaccaaacttgccaaattacgccgcaaccaaagggtctgccgtgtactccatcaatcatatttacctttacaagcatgccaatttcaataagcatgaccgtatcgcaaaatatgtcaagaaaccaagagtatatcgaccaatgtttgttgtgacgggttacgctcgatccaatgccggtaagttgcggtataaggtacgtgatgtcaatcatttgagcaaaacggctggcaagactggctacattactgccaactggaaatatgtccgtccggtttattatcaaagtaaccataagactgtgacggttattaatccgcgtggtgtgaatgcctacaagaaatccaatttggctggcaaggtcaagaactacaagcaagggacaattcttcatgttaccaagtttgttcatcataacttgaccactcggtatgttctcagtaatggccagtacatcactggcaatcgtaagttggtaaatatgggcaagcatcatcaggctcattacatcaagactaagaaagcaattaaccgttataagactgttggtttacatggaaagaataagcactttaagaagggcgccaaaattaagattaaaaactatgatttttcacacgcacacaatgtgacaaaatcaggtagcttgagataccgagtcgctggtggttacattactggtaattccaggtacgcacagattgttaagtaaatagttccatcaaaaaggatcctcggcagtagttgtcgtggatcctttttggttgataaaatcggagttttatttgttacatctatagtcgtttcaaaagctgcttggtgacaaatggatgctaattaatttcaattatttttggaatcccagtactgaatggatttaaagccatttcattatgtacaacaacagtgattcttatggcaaaagcaacacaaatcactgttgtttagtttatagactcttgcaagatactatctcaaaaatgtgttccaaaccgcctattcatcaactctgtcagcatcttcgtcttggactctggcatccagattggccacgcttcttccactttaacgggattagtactgaaactgggtagtacaagcccatcacctacatttttgtatcttcagaacataaaaatcttttgttttaccattttgtaaccatctattttacttttttgacagatatatttaactattttgtatgcagattgctaagctatagtttttataagattctttcgattgttctggcgcacaattatgtagataaacaataacaaaaagccgccaatccctcagcaactttctttaccaaactcgattcaattcacttatgcgtcccccgagagtcgaactcggatcatgaggaccgaaatctcatgtgctatccattacactaaggacgccttacatcatttaattatagcgttttctgaatattaatacaacctgaatgttcatgaaaatttgcgggcgactttatcggcttgatcttccaggtaccacatcaactggttgccgtccttttcaaaatcagcttcaaacgactcaccgattggctgaatcgttgtcagcaacttttcgccaatcccaatgacttgaatctcttttccaaccaatttgccagtatcatagtggccttcctcggcctcatccaagtagccttgaaaagcgtcttcaatcacttgcttcatcagtccgtccctggtggtttccgggtgacgggctttttcgattgcaaatttatcttcaaattcatgcatgttttctggataatctagggacatgattgtacctccacattttctcttacaaccattataaagcaccaaaagcagaaaaaacacggatcttgtttatagaaatccccaaccggcacattctacttgcaattgatgcgccaatagtcgaacatataaggtgtgaagtgcttacatcatcctaatgggaggtaatataatgacacaagcgatcacggttgaagaatcacgtgaattagatgataaaacgattaacaaaatcggcatcccttccctcgtcttgatggaacgggctggcctcaaaatttatgaaaatatgctcgataacaaagatctcgacttaagcaacgttttgattcttgccggaaccggcaacaatggcggcgacggcttggttgttgcccggcttttagccactcatggctatcaagtttccatcttaacggttggtaatccggatcatgccagcgaagatcatctggcccaagcgcggatctgtaactactatcagattcccaaggtcttcatgaacgccgattttaacaaattcaccaccttggttgacgccctatttggcagcggcctatcccgcaacgttggcggcgacttcgccacgattatcgataaggctaacgcttcaacggccaaaattcacgccatcgatattccatccggcttgaacggcgacaccggcgacgtgatgggaactgccatcaaagccatctcaacttcaacggtggcttatccaaaggtcggcatgctcaaagatcaagctaaaccatacactggcaagatctatgtcgatgatatcggcatttatcgtggcaacgcatttgaaaatgaataaatattaatataatattaacttaactagaatcttctcagaatacgtggaggtgccgagatggctgataagaaaacacaaggctatatcaatgttcacgacgttgatccagacatcattgttgacttgaagtacgcaaccagcgataattttactcaccaagtggtttatgactttgaccaggcaatttctcgaattgatacggtcaagaagttggcaaaggccagtcgagacctgaagaatcaaggttaccgcatcaagatttgggatgcttatcgcccaacatacgcccagaagcgtctgtttgaggtctatccggacccaatttgggtagccgagccggatcctaacttcagccaccaaaagggcgtgacatttgacttaactttaaccgatgaaaacggtaacgacattgagatgcccaccggctttgacgattttgacgggctggccaagcgcagcatgaaatcatcatggacaccggctgcccaaaagaactacgatatccttaatgaagcgatggagaaagccggctttgagggatacgaaaatgagtggtgggacttccgcgattcggacaaggatcaatttggcccacttgaggtcgatccaaaggattattaaattcaatattaggagtatgtaaaatgaaagttggaattattggggcaggtccaaggggaattttattaacctctcaattgtttaatcaatataaatatcatagtgaccagaaatcaccgctatcgatcactttgtttgacccgtacggtatcggcggccgcgtttggcgaaccgaccaatcggatgaattaatcatgaacagttcagctgatcaaatcacgttatttaccgacgcttctgtaacgatgtccagcaaggtgtatgacggcccttctttgtttgaatgggccaagagcgttgaggccaaccgttatttggatagcaacggctattcatcagacgtgattgccgcggccgctcaactgcagatcaacggctatgcacctcgcgttttatttggtgcctatatcaaatggttctaccaagatttgattaaacaacagcctaccgaagtttcaacatcattaatgaagtcacaggtcatggatctcatttatgacgccgaccatcacccggtgatcaagaccaacgacggcacctttacctttgacaaggtcatcatgagtctcggccagcaagacaactacctcagcgatgaggaacaaaagttggccagctatgcccaacaaaacgccctgacttatattgcccccactcaccccggtgacgctgatcttagtgacattccagctggtgaacccgccattatccgcggcttggggctgagttttatcgattacatttctgaattgaccctggggcgtggcggccactacatgcaaaatgaagacggcagcctgttctaccaaccgtccggcagagagccgcgaatcattgccggctccggccgtgggattccatactaccccaagccaatcaacgaaaagggttacggcgagtgtgaagtacccaagtttttgaccaaggaaaatatccaaaaaaattcaactgatggtaaaattcccttcgataagttcatggaacttttactgttagatttaaagctggtcttctacaagttgaccatcaatgataaatacccatacaagagtgcctcgaagtttgaaaccgaatttttagccaacgacgataaacaagccgttctcaaacaatttggtttcgctgaagaagatgcctttgattgggattacatcatcaaccccttcaaggacgttcaagcagttgggaccgaagactatcagtcagtattgattaactggctaaacggcgaaattgacgactcactgaagggctcgaaaaccggtccgctggccgctgccagagacttactacgggacttccggccagcttttcgccaaatgctcgtcgatcactgcttcagtaatcaagacttggttgagaaattctggggtcaactcgactcaaccatcaacttcttaattatgggaccacctgtggttcgcagtaaggaattgtcggctctcatccggagtggcgtggtcacgattttggcacccggtatgcaggttaaaggacaagacggttggtttgtgaccgctgcccctaagcgcaacaccgatactttccgttcagctaccttaattgaggcccgggttcctaaagccgacctcgatatcaccgccaacccagtgctggaaagcctggttgacgccaagttggcaagaacccaccaggttaagattaatgatcaatctgtcggcctcaatgcggtcgacgtggatccaagtaccgaccagttgttggatgccaacggtgccggtcaacccgacatttacgtctggggcgtgccgttggatggcctacgctatgttaccaacgctgcgccacgaccaggcgtcaacgacactaatttgcagacggcagatcgtttggcagcagaagtgttggggcttccggcagctgggaatgttgaaatggcttaattgaaataaatgagattgtaaaacggacgccgtcagtggcgtccgtttttgtttaacgattaaaaagtctaataccaaataaacgagcagtatcaccgccagcactacgaaagaccaacttgatgttggggcgctggttaataagaataactgaaatcggaatcctgacgtgataaaaaccctttgaatcggttgactgattctgatcaacggtgaggacttgatcgaatttatgatcgtcgttaaagccaaccacaatggaatgccctgcgtcttcaacattcaaggtaagttccaaggacaaacctggttgagctttagctaacgaaaattggtagctgaaccaaccatcttggtgagcaactctgaagcgtcggcctttggcattgctggcctcggaacgatgctgctcgagatgtttatcaaattcaaaattgttctgatcaaaattatccagttgaccgactgtttttcgccgatattcgcttaacgcttgcaattgttcttcgcgacgctgagcctctttggagccggcctgctgccactggaagtaaaccccatatcgaatttcaaaggtttgataataaggcacaaaagtgattgtttcactcgtattcggtagcttcaactcgaatagtgtattcgtcgtctcggtatcgacaacggcttgactgttcaatgactgctgccagtcgtgccaatccataccggtggtcaatgttgatgggaccgcctgatcatgggtgctgatccgcaccaacacaccatttgggcgatcatcattgatatgatgcttccccagctggcccgcaagaacataaggaccatacttgaaggctacataatgcgggttatcctttgtctgcaccattttcaaactcatcggaatctccaagtcaacggttgttcctgggccggcgttatcgatttcccaaaaatcagcattttgatccacctgctgagaaatgccatcgactgccaattttgccgactggaccaaccaggcagggtttctcaacttcaaattgattgccccagcactatcttgtgagcgtaatttggcgaccgttaagtgaaccttgccggtttttcgatcgacctgttcagtcatctggaggttatttgaatcaagccgtaaaacatttgagaagtacaaactcagatacagctgatctccggacatgaagtcataactgtcgcccaacttagtgaagttttcgatgccagtacccgtacagcaccaaaattcatcgaatggccggttatacaccttggtatagcctgctgccatcggctggaaataggtcatcatcccagtgtttggattctgtgaacccaagatggcgttggtataggtctgctcataataatctaaatattttttatcgccggtgactcgaaataactcccggctcaatttcagcatattataagtattgcaggtttcacacgttgttgctccgtcctccaatactgcatcatgaaacagctggccgggttcgtggaaatgctcactttggctattcccgccagtcacataggtatgatcatcgaccacgatttgccagaagttaaccgctgctttcagatacatattgagtgaccctttttcttcaggacttaaatattggtcggcccgcttcacgtcatgaagggattcatagcggtgtaaagcgccaatcaacttgggaatcgtcgtgttggcgtgttttccagccaggacatcgtcaccctcagctagctgtttaaataatgcggtttcgtcaaagtaagtcgccgccgtcagcatgcgtttatcatcagtcaaatcaaacaattcatacagtgcatcgttcatcccaccatactcaatcttgagcatttgagtggggtcagccagttgattgaggcgcttaaagacataaatgccaaattgatgggcaattttcagggccttctcagacagaagtggatcaattccttgaaggttgaccttgaccgccaacagccctgccaggaccttatgcaggttgtaccatggcaccaacacattctctttctcatctttgggaacttccctgccctctacctcatccagggccacttctctgaacgctgagacatacccagcactatcaggatgactttttgcataggcggcttgggcagactggaggccatttacgcccaggcgaagtttgtcgagcaattgctgccggatgtcgttctcttctgtagcgagaatcgcttgggaaagtgccgacagataatggccgaaaaaatggccacgaaaattcaaaccatcggtgcgctcccaaccttggtagccggttacgccacctgagtcgatgccagcaacttcatcaaaagttaccaagaatctttttggatccaacgctaataaatacttaacagtcatctgctgggcatgctcaatttctggatcagttaatgtaagaaatctttgatcaatgctttgtttcatatctcaagccaccttagtttcttaattgttcagtcaatagaacatcgtgactaccaatttgaaccgatgctgctgccaactgtctgtcatgccacacatcacgggcgtcattttcaattccaatttgttccaactgcacttggctaaccataatcggcttggacgatatgttgaaaataccatagtaagcataacgatcactatgagcataccaaacaatcatttgatcggttctggttaattcaaatttttcggaaattgaattgtccattttcaaaagggttgaatttgtcaataaactctttgtccaatcatccagatccgttaactcgccacccataatgagtggtgactgcattaatgaccaaagactcatcatcgtccgctgttcggcgtgagtgaagcgggtttgacgattacctcccggtccatccactgaacggatgccaatatgtcccaaaggcagcatatcgcaatctggccaattgccaggacgggaaattggcgcccactcttccgcacggtcaaacatattatataaaagcggccattcatcccaaaaatcatttgtaatgcgccacatattggcgttccgctgaaagaacgaaccgtttttaattggtgccggtccgggcgataacgaaagaacgatttggcgtcccgtctgagcaattgcttttcttaaggcgacgacctcatctttgtgcgttttatcatagagctgtgagtcggcaatatcatcgcatttgacaaagtcaactccccaagaggcatataaatccatcaatgagttgtaataaagttgaccctcgggtatagccatattgaccccatacatatcagaattccaaggacaaatattattcctggcgatctccctggctgacttgtcggatcccttgatggcggttgcttgatggaccgcttgacgtggaatgccccgcataatatgaatgccgaattttaatccaagactgtgcacgtaatcggccagcggtttgaatcctcgaccgcccgatgcagatggaaaccggcccggatcaggcaataatctgggataatcgtccatgatcaaaggataaaaatcatgatagcgagacgaattggcggtcggttcataccactgaatgtcgacgacgatatactcccaccctaattgcttcaggtgcttactcatatactcagcattttttctgacctcttcttctctaaccgaggccccgtaaccatcccaactattccagccttttggtgggacaggcgcgaatgtacgatgatgattaattaacatgtgttgtttcctttctgctactgggttctaaattgctttgtgctcattaacacactaaccgaataaggcggcaaaatgaattgatgtccagaaaatggtacatttcgccgttcaatttgattagtcattccaaggtgattttctgcatctggcaggccggttaactgatacaaagacccgtcagcaaaaagatctgtatcaagtgtaatttcttgctgcttatcagtcacatttaccgccttgaagtaatattgactggcttttttatcgtatgtcagatttgtgtacattggttgaacgacaaagggtgggatctcaatttcgttcattttttcgccatcaatccatgtggtgatatgacgaccggaaaccttgatctgacagtgataggtttgattcttattcattgtccatgatgtctgggtccaatcagtgtccattccattggtcattgttctaatcatggaatcggtattgccccagcctccaagaacccaggtaaacgtgttatccaagtcttgttcaccaaaacagaaatgggcacctttgggttcatctcctaccttggtgacatcaaaggccacttcatagtcatctgcatccgtagagccaaccctaatggtctgtttctcacttagagattgacccttaaactgctttgtctgaccattggctgttagtctgatattttcaaacttaacatctgtgccatctgcttggggacttaggccatcgttgagcgggccgtcatcaatcacttttgcttccggaacgttagctaaatgataatcaacattgtttgttccctgatacttcatgaagagctgttgaacgtagtaattaactgacggtgaaacttcgctttgattaaagaaaataaggtctggtgtccagtccttataatcgacattgcagaacaaaggtgcataacaggctaatccaaccttatcagcatttcgttctaagcctgtcatatagctcgcttcaaccacggcattgtaccactggtttttctttgaagcatattcaccaataaatgcttttggccccttgggatcataagaatcgtaccgatgctgattggctaagaaccaggtcggcgcagtgtagtaatgttcatcaaccaaatcagaatgattctcccgagctgacttccagccgcgttcaaattcagcacccgcggcaaatggacctgaagtattaatcaatttaatattaggatatttggctttaatggctttatggaagtatggataacggtcaaagaaggcttggccgacttcttcatttccaatggccaagtatttcaagttaaagggttttggatgtccaagcgctactcgaactttgccccatttactattttcggaaccattagcaaactcgattaagtccagcgcatcgtcaatccaatcacctaattgagcaatcggtgcttcccgatcatgatgcggatcgtgagcgcctggtaaaacaggtagcggttcagccccgatatcctcactcagctcaaaatattcaaagtatccaaggccgagtgtctgattataaccccagttattccggcgagctgggcgttgctcaaccggtccgattgagttcttccaacgatacatcgcaccacggttgtcaggatccagttgaccgtcgtgaactaaacaaccgccaggaaatctcaaaaacttgggatgcagatccttaagggtttcacctaagtccccacgaacataatttggtcgatgattgaacgtattttttggaaataacgaaatcatgtcaaccaaaatccgcgtcccctctggaaatgttagcaccagtcggccagttgttgtggtctgctcggctgtgaactgagcggaatatttcaaccactggtgactttcaaccgtgattgactgaggggcggcgattttcttacctgagtcatcagttaactggacagtcacttcttgagtcccgtttaaggctttcacaaagaatgaaaaattatattgttctccttgttgatagaacatgcctgaattaaaaccagcattggtgatcgtggctgtctgcttagcatcgacagttagataatgaagatttttggtattcaaaggatccttatcggcaactcgtaaactttgcgggtcactgagttcccatgcagtggttgcctgatagtcggaattatcaatgggggcaaactcaaatgagcgattctgaaccatttcagcatatagtccaccatcagcagcatggttgatatcttcaaaaaagataccaaataaatcattcaaaggtgccgttagttcgttagtaacggttaattttgtgtctttcaaagaaattctccttccaattgcgtgatacagaaaaaggatgaacactcgtacatattcatccttttcaatgccacattttccttatttaacagatttaattctgaagattaagatggcaccaactaattcaatcaggaatgaagccgggaagattgccttataaccaccaagataggtaacaatcaacgaagcaacgacggttcctgaaatctgtgacaaggtatttgccaagttaatgaagcccatatctttacccgaagtctcggcattcggcaaaacagccaggttcaacgcaccatcaacggcattataaaccccattaccaatagcagccaagacagcgtatgtcaaaatggtccatggcttagcagcaaagaatgggaagaattgtgcaataccaattaacagtgttgaaagtgcaactggtgcctttagtcgacccactttatcagcgattggcccagaaatcgcggtgaagacaaccccaaagatcaggttgatagaagcaatttcagccaatgtcttaccggctgtctgctgacctaaatgcatatagtcagtcaaaatgtaaagcatgtaagccgtggcaattgtgccacccataaccatcattaacttaccagcaacagcataccagtaatcacgggcacctttagttggtaatgagaagtgaagccaaagtgaactccacgagaatttctcccgtggctcgtccaagttgctgccttcattggcgaaaagaacatggataatgcccattacaaaaccaattccggccatgacgtacataccttccttaggcttaccaagaaattgagcagcgatcatggcaaccaattgaatggcagtatagccaatgccataaagggttgaaattgttcctcgccatcggggtgcaattcggtcggcttcttgagcaaccattgcggcagcaacagcattttctgcggcagcaacaatcccccaaaggacaacaatcaaccaaatcgacttgatattggcaacaatacaaatcaaccctgattcaacaatcgttccgccaaggatccaaggtttacgttttccccaacgggtacgggtaatatctgataagccaccaaataaaatgttagcaaccgcggcaacaattgatgagactgatgctaatagtgcaactaaggcaaccttttcgtttggtgcaatttgactaaagtattgtggtaataacgtgttacgaacgttaccagctggtgccagccaaacaaacggcccgatcagcattgccaacccaaacagtttcgggaactttggctgttcagcgttggtcactttggcgttggttggttctggcgccggttcaactgcctttaaatctttgtcatctttctttgacatctttaaaccccctatgggaataaattttattttattgaagcgttttcatttcaagcgcaaaatagaatcattcaatcctatttcaatgtgacggtgaccacactctttgacggcaaagctaattgcaattgatgctcattcaaacgagcagccttaaaatcagcttcaaccacgttatctggattttcaaaggtattgtgagcatccagtgtaccagccgttagaatcttggctgacgtcacttctttcaagtcggccaaaccagtgaactcaacggtctggttctcatgggcatcatagttacaaatggaaatcgttaactcgccgttttttcgtgaagcggtgtaagtaacattttcaggcacatcaccaaccccttcaaccaattcagcattcatgtgcttttgatacatatcaaaaacataataggtcggcgtcttcagcatctgatcacccttggttaaaatcatggcttgtaacacattgaccatctgagcgatatttgccatataaacccgatccgcgtgcttttgaaaaatatttaaattaattgctgcaaccattgcgtcgcgaatcgtgttttgctgatgcagaaatcctgggttagtgcccttttcaacgttgaaccaggtgccccactcatcaacaattaagttgacccgtttatcaggatcataccgatccatgatggtggaatgcttggtgatcaattcatccatgtgtttggcacgggtcattgtcgaatcccattcagattctgggaaaccggtggcgtcacctttgctttgaccccaggtccccttcggcaaagtgtaataatgaagactaatgccatccaaatattgaccagcgtacttcatcaccgtatccgtccagttataatcgtcttcatttggaccgcaggcaactttgtaaattggatgatccttgtcatactgaggcaaaaacgtttggtactgacgataaacgtctgagtaatattcaggacgcatattgccgccgccaccccatgattcattaccaattccaaagaatttaactttccaaggatccttttgaccattttgtcggcggaggttggccatcggtgattcacccggcatggtcatatactcaacccactcagccatttcttgaaccgtcccgctgccaatattggcattgatataggcatcagcacctaattggttcagcagttcaaaatactcatgagtcccaaagtggttattttcagtgacatcaccccagttggtgttgacgatctttttacgatcatccataggtccaataccgtccatccagtgataggtgtcagcaaacaacccacctggccatctcaatacaggaacgtgaattttcttgagggcatccacgacgtcggtccgcataccgttgacgtttgcaacatcagaatttttgccaacatagagactgccatagatcccatttcctaaatgctcagaaaattggccataaatatatttgctgatttgtggaccagacttctgaggtagaagttcaattgtcatattgttcaacctttcatgatttgctacttcttattaacataaatgttaatattcaagtggtggaaattgttaatgtttaccggtaaaagttttaacgcttttaatatagcgcttacaaatcccaatgtaaacaagtttttactaaaatgttgaatattttttcctatttagtataatgattaagaacgagttgctaaggagcttcattgagcttaagatagtaatataaatgttaacaagaattagaggtaatcatatggaccttgatatttcaaataagtcgctgcccatttttgctgctttggacagtcaggtcagaatcaaaatcatccgtttactttcagaaaaaaagatgaacgtctcacaaatttctaaggcaattcgcttgagcagcccaattaccctcatgcacttgaagaagctggaagacgcccacatcatcaagacgcaaaagaagggcaaccaacggatttgcagtctccagatcgatacaatcaacgtcagctttccgcaacaactctatattccttatgagaattgggatattgagctgccaattgggcaattcaccaattttgatgttcagccctcttgtggcttggcgggtcaaaagggcttcatcggcaaagtcgataaccccagttatttcatggaccccaaacgttatgaagctgggatgctttggtttgccaagggatacgttgagtaccaggtgccaaactacttgaagcctgaccaggaactggaaatgatcgagttgtcgatggagttaagctctgaatttccattttcaaacaaccgctggccgtctgatattaccattagtctggatggcaaagagattggcacgtggaccagtcccggtgacttctctgatattcgtgggcgctacacgccggattgggtgtataacgacatgaatcaatatggcatgctcaagtccctgcgtgtttccaaacacggctcgtttatcgacggccagcattctgcggatacgacgattaatgaattagacaccaccaagaattcgtggacgctgcggattggggttaaagataacgccaagcatgctggtggttgtactatttttggcaatcaatttgggaatcatgatcaggggattaagggtcggttttattttagtgaaaattgacgatgatcgttatcacagcttttttcaattctctgaatttgttttgaggacggcgactgacccccagatccctccgcttaaaaaagtaatcgggtgcaatgcgcaaagtacgcgcattacacccgattacttccttaatgctcgggatctcccgggggtcagtcgcccactacatgcataaacgacttatccggaattctaattaaactaaatcgatcggcctgccggccagcatggagtccaattccattgaagaaattcttcttatacgtcgtcgtgaccgttgccacccacgcgtgctggtaacgcgtatcaaggtgatccaggtattccttattccacttgtaagtttctgcttggacattcagattactcttgccatacaccaccgtggcattcgtgctgttcaccaagtatttaccgccattgacataatacgtatagttttgaattggctttcgaccattgtcatttctaaccgtcacgtagtccgattgatcggagcgataacggatgatcagtggtttataggcataactggtggttgtccggttcgtgtccaattttttgacatcttggaaaaaggtcgtgtacgacatcccccacaaaaacagcaggaaaattgccacttcactacacgaaatccaaaagttacgccacgtaaagctctttttttcagtcacgatcaagcgaagccgacgcgcccgcatatcgtgaataatataagcaaagtaacagatgagaagcagccaaagggccatcccaactaaattccaggcggatttcataatcattcccctttttcttcttaattaatttaagtttacactagtttattggtgagtgcgagtatgagcaaagataagttgaataccattctattgcccagccagcgatgctttgtcataatttccattcaaaatcgtgttatatttaacttgtatgcgattccatcaaaactaatcaatgaggtgactaatcatgtgcaccagcttaaccctagaaacacttaatcaacatgtcctcctggcacggaccatggacttccccgtcaaagcggcttggaaaccggtcctgattaaccagccaaattatgtaaccgctttatcgggaacccgcccgatcaaatatccttacattggtggcggccgcactgaagaaaatgacaacatcttggttgcagacggcgtcaacacccaaggcctgagctgtgccgagttgatgtttcccctgaaagcccattatttggacaatgaagtggatgacaagctcaatttgacccctcaggatttcttaccctgggtgctgggcgaacacgcttcactcgaagaagtcaaagcagacttgaagaacatcgccctgattggcaaatactggatggccggcaaagaggtcttttcatttcactggattctgactgacaaatcaggtcagacactgatcctggagccaacggttgacggcctggaagtcattgaggactcaatcggcgtcatgaccaactcgcccacttatccggaacatatggcccgactggaaaagaagctgaaagtgaccaatcaacagtccctggccgcaaaagcacaacaaatcatcatgagccaagacctgcccaaagcaaccaacaccccaaccaccagatttctggtagctgcagtgaacaaactcggcacccagcccagccggacccagtacgaagccagaaatcgcctgttcaacgttttagatgaagtggcaattccctacaagccgtcaatggacgaccatcccaatttcaactatacccattatatttctgtgttggattcaaccgaccagacttattactttaggtatcacgattccagacagctgttgtccttctcgttagctgacctggtcgaggaatatcccaacaccagccgcttcttagcttaagtagtcagcgatttttcgttggacaccctgctcattattggaataagccgttacctgctcaactttttgaagcaaatcggcagcagaattcttcatggcgtatccctcaccggcagcgttgaccatttcaaaatcattgccgttatctccgaatgctgcaacatcgtccaaggtcaatccccaactttgcaggagcatttcaattccggttagtttgtcggtaccgtcaaccatgacgtccaagccgttcatcccagaagaaatggcgtttaactggccgctgaatttgtgattgaattcatcctgccgtttgagcacgccgccttcttcccaagtgatgtcgagcttataaattgagtcgaagaccagccgcaaatcagccatcgactgcatattttcgtagaaatatttggaagcctggaagcgatcggaattctcgggtaggttgcagtacgtgccgtttcgaccgactaggatcacttcggcgccggcaaaactgggttcacttaaaatccaatccagggctttcttcaagactaaatggtcaatgatctcttcgtggatgatcacccctcgttcgtcgatgactaatgcaccgttgttacaaacgtatgagatcgggccgtggacatttttgaacagtcccaacagatgctggtattggttactgctggcggagatgaagtgcatccccttatcccccaattgatccaattgctgttggaactgttgctcatcaaaagttccctgatcattcaaaaatgttccgtccatgtcgcttgcaatcactttcaccacaatgactcctccattcaaatttcgataattggttatactctcattttaagggattagtttggtttgtaaattatttttatatcttgtatactgaatttgatcatacaactatctggggtgccttattggctgagaaaaacccatcgaacctgatctggacaattccagcgaagggagcatgctccgttgtatttagatggataaattgcaattagatgaatttttgaggccagggcaaaacgaccagttttgtgcctggcctctttgtgtgctcagcaattggactttcagtgacttatttgatcaaaatcatatttggaggtcttgttatggataacaagagtcaagcaaccggcggcaaaaagcaaagccaatggacgcttagaaacattattttaattgccttaattgctatttttactggtattattttttggggagccggctttttatacaccggattgactgttgccctgaccccatttggaatggccccatttgccaatgacctgttgatgggcctgtggtgcatggctggtccattaaccggattcattattcgcacgttcggttcagccttcttgggtgaattcctgggggcttcggttgaagtcttccttggcggtcaatggggcgcaggcgcctttatttccggcttggtccagggaattgcttctgaactcggttttacactgaccggctacaaacgctatgactggttcggattgaatgcgtcaatcttcactacggttgttttgacatttgcctgggacatgattcgaaatggttatgacaaattcagtctgccactgctcttgggactattcgtcacccgttatatttcaacctttatcttcgccggtgtcttgaccaagatgattgttaaattattggatcgtagtaaagcaattaacttgtaattataggggatttgatcatgactgatgtttcaattaaccatttcacttttcactatccacaaagcgacgtcaaggtcttaaacgacattaatctgaccttcaagagtcatcatttctcactgctgtccggaccatccggcagcggcaagtccaccctgctgtactttattgccggcctatacccgcattttatcgggattgatgcagtcggtgagatcaaatttggcgacaccaacatcaaggatatcccccgggaaaaaatcagccagtcagtggcgatgatgttccaaaatcccaatcagcaattcgcgatggacactgtcgttcacgaaatgacgtttgtcttggagaacttgcggattgcgccggataaaatggataacatcatcaacgacgccctggaattctgtggtatcaagcggctgcgttcgcgggtgatcaacaccttgtccggtggtgaaaagcagcgagtggctttggcctgcatcgttgccatggatcctcaggtgatcgtgttggatgaaccgtttgccagcattgacccggggtcgagggaagatttgattaacaaattaaaattactccaacaagaacacggcaaaaccattattttagccgaccatgatttgaccagttatcggggcttggtggatgaattctactatttggatccggatacccatcaaatcagccttttggatgaccaacaagctgaacatttcttcaaaaacttcgaatccactcaacagatgcacaaacgagttgagattcccactggcgatgaccatgcgattatcaagctcagcgattttaaattggagccgcacgcctcactgctattgaccctgaaccactttgatttttataaagaaaaaaccactttgatcaccggcgccaatggcatcggcaaatccaccctgtttaacgcgttgaccaaactgctgccctataaagggaccatcgtctttgacggcaaggatatccaaaaaattcggccgttgccgtatgcgaagaaagtgacgctactgttccaagatgccgaaaaccaatttttgaacatcacggtcaaagaggagctcgatttgtcactcgccaatcgaacgaataccgactacacgcaagctgacgttgatgacatgctcagcaagcttgatatggcgggtaaagacgaccgcatcgtgtattcgttaagtgaaggtcagaagaagaagctgcaaatcattgaaatgttgatcatgaatccgccggtattgttaatggacgaaccattcaaaggcttggattatcattccctggaggtcgtggttggcttcttgaatcgggccaaaaacgatttccatcaaacccagattatcatttcgcatcagctgtccggattggataccctgattgattatcacgccgcctttgaagaccaaaatctgacttaccaggaggttatcaaatgaatcctggaatgaaattattattggtgatgctgattgcgttggaaatttcgtttacccaaagcttgattgtcaacatcatcctgatcaccatcagctttttatatattctcacccaacacgtcagtatgaaggccttgtttgggatcatcttttggccactatttcctgccgttggtctattcgtttctcaatggctgtacggaagtgccggcatccattttgcctggattctgtttacccggatctatgcctatgtattcctgggggcaaccttcacgttgaccagcagcatcaccgacctgtcgttgaccttggagcaggattttcatctgccctccaaatttgcctatggcgttttggccgcatttaacttaatgcctaaaattgccgaggaagttcgcattatcaagacttcggcattaatgcgcggcgaggcgctgcatttctggtcaccgaagctgtactttaaatcaattctctcgtcaatccaatggtcacagaacttggcagaagccatgacgtcccatgggtttgtcgaggattatgaacggacccactacaaggtcattcgcatcacggcaattgattgggcactgtttgttgtcctgctggccgccgttcaagttttgctattctttatcaaatactaaacgccaatattccaacatttccttttttgacttataattatgtaagagaaagatatattggaagaaggcgttttttatgcgggcaaatcaatttgcatttgcgtttggaatttttgcgttaatcgttggaattattgttgatatttatgggttggtcacccaatttggctcgctggacagcgcccaggtggtattgatcgggtcaatcattttggcaatcggcctggcattcttgtccctgccgaaccgctgggagcgatatgccggccagttggtcgttggccttggtttactgtactatttttacattcaaaccaacaaatggtgggtggcagtcatcatcgccattatcgccatggccctaatggaatatggactgaaacatcgttaaaatgtgtcaaaatttcaattattggtataatagatttatagagcaagttggatcacgaattttgatggaggagaatgacgatggcagaaaaatttagtaccttagcggaagaaattattaattatcaaaagaagaacgatatgcccgacacagcgttagcatttaacctgcacatatccgttgaacgcctccacaatatcaaatcaatggaatcggaccccacaccggacgagaagagaacgattgagcagtttgtcagatagagcgcgacgagcaacgggtgaggcggtttctaagggtattttgattgaagtccctgggtttgggactttaattaaagtgcacttagaagttagcctcagttgcgtcggagcgtattttgaaagccgaaggatcctcagaataacataagcgcaccagagcgcgacgagacccggttagggccctgaacataagtgtattttacaagaggaagagagacccaaaaatcccgacaaccgttcccccgagaaacaaaacaaaccacaaacgaaaaggaccgaagcagactcgcttcgatcctatttttgatgcttctcattcttctcggcccgataccggctcatcccttctttataaggattgccaaacaaccggctcaatcccgtccaccaggaattggtacttgccggttgattctcatcgactggcaacttcttgccacagttcggacagacaacgtcatccggcttcaacttcgccccacaatacggacaaaatgaaaatttttgctttgccatcttgcttacctcgattgctgttggcctttgttgcgattggcattgcgctgacgccgtttttcggcttcggcttgttccttggcagctccagcttggcgaatttgttcttcacgttgctttttagctttatcttcggcaataatttggttgtgcattacgttcatccggtgcgacagaaagttccagccgccgattaaaaacagcgcaccaaccactgagtacggaaatgtccaccatggaaagtaactaccatttttgaaaaccattgggccaagaaaattatagagtgccatcaatattgcgaccatcaaagtcacctgcagggtattgaccagccacttgggcatcttaaatccttttttctttgccaccatgcatcccccctaatcaatttcattttcagtcagaaaggccttgaaataatcaaaggccatctcgcgaatattctcgatgccaatttgtcgggttggcaaatcaccatcgtcatcgacgtctagcaattccacattcaaaactcccgtttgcagatcgattgaggttggatacccagcaaaattgtcctcatcggcagtctcaaaacgaatcactttttggtattgaatcgattgggtgatgatatgaatcaagatgttgtccgcgttatcaaatgcccgatcagaattcaaaaccggcaacgcaaaatgcttgttgtgtttattctcaatcacgaatttatcgatcacccgtaaataatccgagtccgtaataattctaccaatatcatcgtaacgaatccagacgtaaccgccaaatcggccgttcatatcgacaaccatcatgacaaattctttttcgttgctggaaataatcttgccaacgtaaaaatacttccggttatcattggtgtcaatcacgacccaatccccgctattacgcagttgttcaatctgatcacgaaagacacttggatcatcaatgatctcattttccacatgattttccggtttaatcatatccaaaacattttgcagcagctgtagttcagtcccaccaaactcaataccacgaatatcatcaaatcgaatgttgaacaccgactgctttgagaaatcaaacttattaatgttagtaaagaccattccgtcgtcttgaaagtccgaaatgagcccttcgttatatttcagcttgcctgcctgtgcggtaatcaccagaccgactttttgatcatcgtgcaatgtctgaatgacccggtcgaacaacgagtcgctcatcttgattggtaaatcaaaagagggctgggaattgaggtggtgcttctcgtcaaactcaattcgatcctgcatgtttgccaagtcgtaactgtcggtatcaatggatttaactgaagaaatcttcaaataaacttcaccatcctgaatgccgtaatcgttgtaggtcaacatgatgaaatctttatcgcttaaaaactgaatgacaccggtgtaaacgatatcggagtcattttgaaaagcgttaatcagctgctcgtcgatttgggcggtgcgcagcttgtcgtagagggttttcatggtgtcacttctttcttggttgggttggttgtttgtggtgctgatttgtggtgcttgcttgtggtcgattaaggttcaagctttaattttctctagtggaaatgtgctccgacgaccctggtccctactgcgtaagtcaaaaatttcaacgatgaacaaagaccgttcatcattaaaatttttgacttacactccgggaccacccaggtctcgtcgcgcactctacgaaattgcattccccataaattccctaagttcatcacccgacatattatcactcaatccaactaaaagcttgattcttgctttctggccgttcaatccttggcagagaatcgttcccatcttcattaattggatgccgccgccctcataatcatagatatcctgggcgacgccgttataacatcttgagaccaagacaattgggatatggttatccaataatcgttggatcgccggtaaagtttggggtgggacatttcccgctcccaatccttccagcaccaatcccttggtgttgtcgttgttgatggcgtcaaacaacgtgccgtccattcccgcatacgccttaatcagatagacgccttcgaccacctggttgatgtcacacacttcggtttgaattaattcctggaagtattttgccttgttttgcgttacaatgccaattggtccaaaagtcggcgttctaaacgtcgccacattggtcgtatgcgtcttggtcacgtatctggccgtgtgaatctcatcgttcatcaccaccacgacccctttgccgtaggattcatcggttgcggcgaccaggatggcatttctaaaattgtacaacccatccgagccaatttcattagatgatcgcatggcacctgttacgacaaccggaattgtgttgggcagcgtcagatccaagaagtaggcggtttcttccaacgtatcggtaccgtgggtaatcaccacgccgtcgacaccgtcatcaatcgccttcataatacgctgcttaatttttaacatcacctcaggagttacgtgaggggatggcaggttaaacatttcatcagtaattaagttaatctgaccctttaagatcacttgttcttcagcaatcgggttctcatcattggggacaacttcgcccttttcgttttgagacatcgaaattgtgccgccagtatgaatcgcaagaattgttttcatcaatttcatcctccatcaacctgttaatctataccattgtaccgtaaaatggaacatgaataactatcaatcaagaaagaagtctcagatatgccaaattccgaccgctactacacgccgcaaaattcgaaagatgcgatgcgccagatcgaaaaactatttaacaagtataaggacgccccactcacccaagaactcgtcgactaccatcagaatttggtgaatcgcttaaagactgacattctggcggctgccaagcaggaaaacgttcccgcccgaattgagtcaatcaacacgatgatcgccgccatggagcgttggttaaaggtccgcttggccggcaatccctataacggcaagatgaagaactttaaatttgtcagtgatgaatcactgcctaagttcaagcgccacgtccacaagatgaatggcggatcgacccaccgttcttcaagacattagcagtttctctttgtaatcacgactattacattgcagaaacgtgggaattgaagcagtttccggccatataagcaaaaaagccaaatatcccggcccgggatatccgactttcttgcttatattctggaaactaaccgcttcatttcccactctcaatcgttataattaatttatcaatcatattagggggaagaccgttgagcaaaaccattgttgaattaaagaacgtctacaaaaagtacgacgacggctttacagctctcaaaaatattagtttcaaattacaggaaggcgaattctacacccttcttggcccctccggctgtgggaagacaaccatcctccaatcaatcgccggctttacagaagtcacatccgggcaagtgctgtttgacggcaaagaaattaacgatattcctgccaacaaacgccagctcaataccgtttttcaagactacgccctatttccaaacatgaatgtatttgacaacgttgctttcggcctagtcgttcataacgccaaaaaagacgaaattcaaacccgggtgcacgacgcgctcaaaatggttcagcttgaacagtacgccactcgggaaatcagcgaactatcaggcggccagcaacagcgaattgcgattgccagagcgattgttaatcgaccaaaggtattgttactcgacgagccgttatcggccttagacgccaaattacgcaaggatatgcagtatgaattgcgtgagcttcagcaaaatcttggcattacctttttatttgtcactcacgaccaggaagaagccctggcaatgagcgatgaaatctttgtcatgaacaagggcgcaatcctccagaaaggttcaccggtcgatatttacgacgagccaatcaaccactttgtcgctgactttatcggcgaaagcaatatcattcccggtaaaatggtggccgattaccaagtcgcctttttagggcatcaatttgaatgtgccgacgctggcatgcggcccaacgaaccggtggaagtcgtgatccgtccggaagacctggtcatcactacgccggaaaaaggcaagttgcaggtcaaggtcgacactcagttattccgtggtgactactacgaaattcttgcctatgatgaggccggcaacgaatggctgatccattccaccaatgccagcacggatgatgcgattatcggcttggcgtttggcccagatgatatgcatatcatgcgttataacgaaactgaagccaagttcaatcaccggcttgaaagttatgaagagtagggggggcggaacatgaagcgaaattatcgggggctttttttcacgccttatattttgtggctggcaatgtttgtcatcgcgccagttgccctaatcatctattattccttttttaatattcacaatcatttcactttcgcgaactaccaggagttcttctcgtcaggaacgtatttgacgatgacggccaattcggttctctatgcctttttgattaccctgttcgcaatcttgatcagttatccaatggcgctggtgatcagcaaattaaagcaccgcgacttgtggattctgttggtgattttgccaacgtggattaacctattactgaaggcctatgcatttattggcctcctcagccacgatggcttagtgaatgatttgttccaattctttggcatccctgcccagcacatgctgttcactgacgccagcttcattctggtcgccgcctatattcaaattccgtttatgatcctgccaatctataactcgttgaccgatatcagcgattcctacatccgcgccagccgcgatttgggcgccaccaaatggcagacactgaccaaagttatcattcctatgaccatgccgggaattaagtccggtatccaaattgttttcattccatcgctgtcactcttcatgctgtcccgattaatcggtggtaacaaggtcatcaccttaggaacggcggttgaggaacacttcttgacgacgatgaactggggaatgggttccacgatcggcgtggtcctcattatctcgatggtcatcgtgatgctgttgaccaacaccaagcgtaaaaggaggcggacatcgtgaacgataaggcttccagaaccggtaaaatttatatcaccattgtctttttgctattgtatattccaatcgtctatttaattctgtactcattcagtaagggcactaccatgaccaatttccagggcttttcgctgaaacactatggtgaattgtttaacgataaacggatgctggcaatcttcttgaacacgatcctgattgctctgctgtcttcggtctgctcgacgattatcggcaccatgggggcactggccgtccataatgccaaacggcgccacgaaagagaaaccctcctatcactaaacagtatcctgttggtatcaccagatgttatcattggtgccagcttcttgatcttctttaccgccctcaagctgccgctgggattctggtcagtgctgctaagccacattgcctttgaaattccaattgtcctactgctggttttgccaaggttggacgaaatgagcccgtcgatgaccaatgccgcgatggatcttggcgccagcccggcccaaattttaagtaaaatcgtcctgccttacattcaaccggggattattgccggcttcttcatgacaatcacctattcgttggatgacttcgcggtcaccttcttcgtaacgggaaatggcttcaccaccctgtctgtggaaatctattcaagagcccgccaaggtatcagtttggaaatcaacgcgttggctggtatcatgttcatcttctcgctcatcttagttggcgtgtactattggattgagaccagaaacactgcctcgactggtaagaaaccaattgtggaggtgactgaccgatgaaaaaatttctcgcagcattgattgccattctggcgttgtgcgccggcttggcttatggcagtaatcagctcaccaaatcaaccggggataccggcaataaggtccttaacctctacaattggggcgattacatcgatcccagccttttgaccaaatttcaaaaggaaaccggctaccacgtcaacgtcgaaaccttcgacagcaacgaagcgatgtacaccaaaatcaagcaaggtgggaccagctatgatctcaccgttccaagtgagtatatggttgaaaaaatgaaggccgatcacatgctgattccactggacaaatcacgtctggttggcatgaatcattatggccgctcatttctcaacaaatcctttgacccgcagaacaaatactccatcccctacttttggggaacactggggattatttataacgatcaatatgtcaaaccgggatccttggagcattggaaccagctttggagtaagaaataccggaatgatattatgttgattgattcagcgcgggatattctgggtttttccctcatctcgatgggtcaatcagtcaacacaaccaattcagctgaactgatcaaggccaaggacaaactcaatcgtttgtcacccaacgtcaaagcagtggtggccgatgaaattaaaatgtatatggcagaaggtgaggcaccggtggccgttgactggtccggtgaagcatcggaaatgatgtcccagaattcgcatctgcactacgtcgtccccaccgaagggagtaacatgtggttcgacaatttggtgattccaaagacggctaaacatttcaaggcaatttacgccttcctgaactttatgaacaaaccggaaaatgccgcccaaaacgccgagtatatcggttattcaacaccaaacatgtcggcttttaaactgctgccaaaggccacccgcgacgataaacagttctacccaacccaaaatgtgattgaccgactgcaggtctacagtaacttgagtccgcagaaagtccaagaatataacgatttgtatttggaattcaagatgcaccattaacccggattaaattcttaattggtctttgaccgccaaatgcattaaactgataacgaggtgaaaataataatggcaaagaaaaacatgcgacaagaaatcatcattgatatggacgaatttatcgtcacatacgcagcaaccctcttggatccgaaccagaacctttccgagttggtgtataacacagcaaaagaagatattacaaagtgggacgacttattccacgaccaaggatttggccgcaaaaataaatttatcaacatcggccgaggctacttaagagatgcccaaaacttggacgctgaagaggcggaaaagcaaggcgaccagttagcccaagaagccatcgattacttgggaaagcacacggactttttcgagaagtggagaacagactagagcgcgacagagcgcgacgagacccggttagggcccagaacataagcgaagaataccaatgatgaacggtctttgttcatcgttggtattctttgtttatgtggccgggccctgggtcgtcggagcgtatttcaaaggccgaagggacttcgaaagaacataacaaacgcgacagagcgcgacaagacccgggttgaccccaccaagtaggctaggccgttttcatccggccgtcggaacattagcgaaaacatccaatgatgaacggtctttgttcatcgttggatgtttttgtttatgtggccgggccctgggtcgtcggagcgtattttaaaagccgaagggagcgcaaaagaacataacaaacgcgacagagcgcgacaagacccggttagggcccaccaagtaggctaggccgttttcatccggccgtcggaacattagcgaaaacatccaatgatgaacggtttatgttcatcgttggatgcttttgtttatgtggccggggtcagggtcgccggaacgtattttaaaagccgaagggagcgcaaaatgacctaacaaacgggccccacgttcccaaacataaagagtaagaaacccattgcaccccaaaagaacgcccacaagctttttccaccaaaacttcccaactttgcgtcataatagacctaatcaaaatatgagaattctggggggaagggctcaaaatgaatcacacacctgcacaatcaacgacacaaaaaaatggttggtggattttggtttccatcggcatgtttgcattcatgtcgaacctggattccagcatcgtcaacattgccatgcccatcatggccaaacagttgcatgtcccgatgaatcaaattgaatgggtggtttcgtcatacctgatcgtcttaactgcactcttgctatttttcggtaaactcggcgatatctatggcaaaatcaaagtctttcgaatcggaacagtcgtcttcttgcttgggtcatttctgtctggcctgcaaatcaattttccgttcctgctggtcggtcgctttattcagggaaccggagcagcgatgactttatccaacacttacggcatcaccacgtccacctttggtattaaggaacgtggccgggcaatgggctttgttggaaccttcgtggctttgggggcaatcgccgggcccggacttggtggcctgattctttcaaggttatcttggggctacattttctgggttaacctccccattggcattgttgccgtcattctgggcgccattgtcatgcccaaggcttatcaaacggtgccgggaaccatcgattggctaggtttcatcaatttctcactgatgattatcggcttgttcctcggtgtcttcatcggccaagaaattggctatgggtcgccaattgcactggcattatttgccttagggctcatcaccatgtggggctttttccacgccgaaaaacgggccaagaatccattgatgccgctgtctttgtttaaaatcaagccattcacctatggcctcggggccactgttttgatctttctttccaatttcttcactgtaatcatcgtgccgttttacctggaagatgctcggcacttgtcagctggcgaagccggcgcattgctgatcattttcccggtcgtcatggtgtttgccggcccgtttggcggttggttggctgatcacttctcgccagccgcaactgccaccggtggtctgttgatcgtcgctgtcgcccaagccatgtatttcttcttaaccctaaccagcccaatgtgggtctacgtcgtcatcacgatcattatggcttttggcaccggcttgtttcagtcgcccaacagcgatatcgtcatgtcggtggtcccaaaggattcattgggaagtgccgggagtttgaacgccctggcacggaatgttggcatgatctctggtactgccttatcaaccagtgccctatttatcgccatgagtgtcaaagccggattccatgtcaccaactatttaccaaaccagccggaagtctttattttcggcatgcacgttgcctttgcggtttcactggtgattatccttggcgcttgggtgctgtcaatcatgcaaggccgaaccgtcaaacctggtgatttgaaataaccatttggtcagttgaaagatcccttgattttgccggtaacgatgcgttttgattatcgtcatcaatctttgtaaatagtccataaataaaaagtgagacctggcgttaagccggatctcacttttttgcttacttaattttagttgcttgtcccttacgcttccggtactcaattcttcccagcttgataatttcggtcacaaccagcacgataaaccctgcgatggttggcacaacccagccatagaagaagtcgatgctaccagtgtggaagacgtcttgcataaacggaatgtagaacatggcagcttgaagggccaacagaattccgatgatgataaacgccatcttgttctcgaagaaatgcttggaaataattggataggagttgcgaatattgaacagatagaaaatcttaccgaagataatgatgttgaccgccatggtactacccagaacagctgtcaggacacccgaatcaacaaatcgatcgaaggtgaagatcccaagggcggaaattaaaatcgacacgtaggtaatttcgaaaacgtccatttttcctaaaatccctttggcaacatttcttgggccacggatcatgatcgactcttcagccggttcaaagataaacgcaaattgaatggtcaatgccgaaaccgtgttaatccacagcagttgcgttgggaacaacggcaactcttgtcccataatcatactgatcaggacaaccaggccttcagcaaaactggttggcagcaggaatcggattgtcttttgaatattatcaaagacatgccggccttcagcaaccgcatcaacgatggttgtgaagctatcgttaaccagcaccatatcggcagcttccttggcaacggcagttcctttaatccccatcgcaattccaatgttggcctgcttcagagcggcggcatcgttgaccccgtcaccggtcatggcaacgattttgctgttggcctgttgggccttgacaattcgcagtttgttggctggtgtggttcgggcaaaaacattgtaacggccgatgttcttaattaaatcttcgtcggacatttcatcaatctccggcccggtgatggcatgaatactttcatccaagtccagtttgcgggcaatcgctgatgcggtatccgggtggtctccggtaatcatattaaccttgacgccggcacggcgaaggctttgaatcgaaggaatcacttcttcacgaggtgggtcaataatcccgacgaccccacttaattgaatgccgtccgcaatcttgtcctggtcaatctcgtccacatctgtggaaacatttttgtatcccagggcaaccactcgcaaaccttgctcagttaatttggcaacccgttcataccaagtctggtcatcaaagttggggtcactttgtttgaccatgtcgaaaatggttcccggtgcgcctttaaccattaactcgtgatgatcattttccttgatcaagcgggcactgtatcggtacgccgaatcaaatggcagcgtatccacttcatcgacttccggctcacggccgattaatttgtgaaataaggtcgttaacgcaccatcagtcggctcaccgtttaattgccattcgccatcggtttgcaccaactcggcatcggtggttgtcccggcaatgtcgaccaagtcgcggaattgctggtcttgtttccagtcatatttttgaccatccaataagacgtccccatcaacgcctttatcaccggcaataaatccaaccccggtaacttgataatgatgttgatcggtaatcacgtcggtaaccgtcatttcgttcttggtcaacgttccagtcttatcagtgtcaacaatatccacagcacctaaggtttcgacggcgggcagcgttttgacaatcgccccttttttggtcatcacctgaacgcctcgagccaaaacaacggatgtcgaagccggcagtccttcaggaattgagcccaccaccattgtgataatcgctatggtcaaggttggcagactgtaaatcttggtgtagagaccgaggacaaacagcaaaatggcaatcgccacaataaagagtgacaggttaatccctaatttgttcaaattccgcatcaacggtgtcacctgggtcttcacctcggcaacactttgttgaatctgaccaatttgggtatccttaccagttgcaatcacaattccgaccccggatccctgagtcaccgctgttgaagcaaacgccatgttggagcgttctgccaacggaaccgaatccttgttaatcggatcttcggtcttttcaacggagttactttcaccggtcaaagtcgattcttgagcccgcatattgtctgcggaaatcaggcgcaaatcagccggaaccgcgtccccagcctcaaggttaaccagatctcccacaaccagttcccgggccggcacttcaatcttgtggccgtcacgaatcacatagttctggctcaccaacagttccttgattttgcttaacgcattgtcagcctgcatttcttggaagaatccaataaacgcgttggcaataataacgatcccaataaccgccgagtctgaatagtgatgcatgaacagcgtaatcacagccgcagcgatcaaaatgtagatgatgctgttgttaaattgcagtaagaactgcagcagcttgcttttcttcttggcggttaattcattgtaaccatctcgagccaggcgtttagccgcctcttgctcgctaataccgtcctcttcgttggtctgatactgttttaccaactcatcggtacttctctgccacaacttttcatcgggaggaacctcgttcatattgtctgccattaaatgtatcacctttccttttacaaaaataagattgttgttaagagtattataatatattactcactacttttggtatataaaaatcttaaaaatcgaccacaactcatgtgatcgattccaaatccctatttgacaactttggtccactcgtcaatcgtcttgccgttttcatctttcaaaaccagccaactgttgatgccggcaaaatagaggaagaggcccacttcattgaccgattttaaaacgatgtctttggtggtcacaaaattccggaaactatcggcatgttcagatctcagtttctgagcaaacttggccgaaaaccccagcgacccatcctgattcaaatcgggttcgactttcatcaccgcgccggccttaatcaacatttcgttacgcttctgccagtagacggttgctttggcaccctcatgatcaacataaaacggaatctcactcacctgtttggtgaatttgtggcgtggcttgcccttgaatttcttcttggaaacaaatacggattggaatccaagaccattcaggacggttaaaaccaaatttcgaaaggcttcaacggtttttcgctgattgctgggaatcttgaccgtttccaacagatctttcttaagaattccccgttcaacggcatactcggaaaagctcttggccaaatagccagcctccaagtcccaggctggttcgatctgaatcacaccgtcggccttgtcagttggttcggtctgaacgctgatcagcttcccgtctttaaggtacaggttaacgtcggcattgacctgatcgactgtctttgtgaccacaattgtcccttggccgtccggtaaggtcatcctggtcgaatcatcattgatttcaactgccaatttcatgctgcattccccatttcatttgttcttctcgttaatcataccattgaataacaaaaaagaagcccacaaccctttagtggtaaaggatcatgagcttacttttaatcgaagaagaagtttgtgatgcatagattattctgtggtcagtttgttggttaaattaccggaccatttccagttttgaacctctggaatatcggtaccgtattgacgaatgtaatcgtggtgcttttggagcatgtggtccatcttagcttcaaaattgtctgccgaagcggcgaacttggtccgagaaatagcatccttagccaagtggtaacgatccaattcattgaggacccgcatatcaaatggggttgtgatatccccattttcacggtaaccatggaaactaatattgtgattatgacggttatataccaggccacggaaggtattctcaaagccatggaaggcaaagataaccggtgtgtcagtggtaaagtacttgtcaaattcagcttgggttaggccacggctatcctgatcttcgttgcttggacgcagtctcaaaatgtcaacgacgttgatgaagcgaaccttcaattgagggaaagcctcgtgcagcatatcaatggccgccaaactctccatggtggcttcggtaccggcagtcgcgaagatcacatccggatcgccttgatcatttgaagcccatggaataatccccaaaccatcgttaaccagcttagtggcttcatccattgagaaccattgtggccgtgggtgtttggaagccacaatcaaattgatcttctcgcgggtctgcaaggcagtgttcataacggccagcagtgagttggcatcagctggaacatattcgttaaccaactcatgacctttttcagccagatgtcccaacatgccgggatcttgatgagtataaccattgtgatcctgctggaaagcgtgggaaacgttcatgatgttcagtgacggataatcatgacgccacgattgttcagaggcctttctgagccacttgtagtgctgagtgagcattgaatcaatgacacgggtaaatgcttcatatgaggcaaagaatccgtgacggccgcttaagacgtatccttcaagccaaccttctgcttggtgttctgaaagttgtgaatcaatgacgcggccttcaggagccatgttttcgtcattcggggtcttgattggttcttcccattgacgcttaccataatccagcattgagaagaacttattggatttggtttcatctgggccaaaggctctaaatgacttgccgtttcgcttcataatctcggtgtagaagttggataatacttcagtatcctgagcttctttgtcacctggtttgtcaatcttcaaagcgtaatcggctgggttaggcatgtccaacttcttggggttaataccaccattgacgattgggttcatcgccatccgctggtcaccgtctggggtggttgctttgatttcagctttaattgagccgttgttgttaaacaacttttcaggttcatatgatttcagccaattaattaacagatctttgtggtccatctgaccagcactgacaggaattggcacttggtgcgcacggaatgatccggcaattggattgccatccaagtcgaacttaggacctgtccagccctttggtgaacgcagtaccagcattggccagtgtggcaaagtatcatcattattgtcacgggcgtgcttttgaatggccttgatttcagtaatgattgcatccatcgttttggccatcgtctggtgaacccgggtatagtcttcggggtcacctttcgtttcaacgaagtatggcttccagcccatgccttcaaagtacttggttaagtcagcgtcactcatccgggaaagaatggttggattggaaatcttgaatccgttcaggttcagcattggcaaaatggcaccgtcatgaattgggttgatgaatttgttggagaaccatgaggcggctaatgggccggtttcagcttccccatcacctatttcaactgcggcaatgacgtcggggttgtctaaaattgccccggtaccgtgggcaatggaataacccaactcgccgccttcatgcattgaacctggtgtttcgggggcagcatgggaagcaactccgcctgggaaggagaattgtttgaataatcgttgcagaccagtttcattttgagcgatctttggataaatttcgctatagctgccgtcaaggtatgaattggaaaccatcacctgaccaccatgaccggaaccttcaatatagaacatattcaaattatatttcttgattacccggttcaagtgggcatacataaagttctgtgaggcaattgtgccccagtgaccaatcggcttaatcttaacgtcgtcagcgactagatctcgtttgagtaacggattgtctctgagaaacagttggccgactgataaataattagcagccttccagtacagattgactttttgcaggtattcatcggaatcgaagttcgtcatattagtaacctcctgaatttaacagtaacgttattaccaattcgattattggaccggtccaaatcaaattacaagtttattgtatgcctcagaggttgataattcaatggtttaagcatttgaataatttattttgatatagacgaaatttatactaattccatttagtataaggattagcgcagatttcatgaaatatattcagacaatcaggattagaaacactttccacaaataaggctgggacactttttacaaatgtcccagccgatttaattaccctttgatccagataggtcctgtcagacctactgatcagcctgtttgcgactaatagtgacgctgtcgatgaatgtgcaagtacttggctaagaaatacgccaaatcacaataccaggtttcaatttgtttcatgattcgtcctccaatacaaacatgacccgttttaattcacccagtgcatcccctggattctgccattgaaaatcatatcccagggaaagatttcgataccgaatgccattttccgtgactgcgttgggcatgtgggaatggccactcaatgacaagctgacgtggttgtgttcaaacaactgtcgataccggtcgctgcctaactgatacatgaaccgatcataaaacggaatcggcagctggtgagccaactttttcgtcggcagcatgtggctggccaccaagatctttttgccgctgacagccaatcgattgatttgatgctgccaagcaagaatctgctcgactacccatttacgatctcgccgataactgatttgattgccattaatatatagctgatcgggccagacatgtttggcaacaaagttattcgcgtatcggggaccgtctgcttcacaaaaatgtttggcaaacgtgtaatcgtaccatccattaatcccggtgatcagccagtgcctggtctcgattggatgccgagttaaagacgttggcagcctgtccagttcacgataagccgttcgggaagccgactgaatctgctgaactgatttttgccgggggtgatccacgtagagatcgtggttgccaatcaaggtgtgaaacggaactggcaaggcttctgccaattgttgatagaaccgcaagttgcgttgaagtccattcgccgagtcccccatgatcaccagctggtcaagattttcatcactgatcaattggcccaatacggacacaaaatcatactggcggttaaaatcaatgtgtaaatctgacacaaaaccaatccgcatggttatctctccaatctggttgttttctatattgtagcgcacgaaaaacggaccaaatcaaaaaatgagaatctttaggagttcgtaagtataagaaagctgctgacaagcaattagtgacttgattggcatcaaacgacactttgacaccagaaaataataaaagatccgcatcatcccaagcatcgggacggtgcggatcttttttaaggtaaaggattatcaaaaccttccagcttcgttctagccgagataaggattctccggaacccgtaccaaatcatcggcaaccagtcgttcagcaatctgaaccgcattccaggcagcacctttcaagaggttgtcggaaacgacccacatgttaaatgccccttcattttcaaagtcaggacgaacccggccgacaaatgtttcgcgcttgccttcagcttcgattgactgcggataaatttgatgggcggtatcatcttgtaagacaacgccatcggcaccatccaatgcagctttgatttgatcagcagtcgcattcttatcagcaacttcaaagtaaactgactcaccatgggcaattcggatcggaactcgaacacaggttgcagtcaccttgatgtctttagcgtccatgtcgtccaacataatcttcttggtttcgtgaatcatcttccactcttcatgagtgtagtagccgtctgattcgaaaacatcaatctgtggcaataaattaaatgccatctgataatgcttcttgtcacccttggtaggcaaaatctttggatcagttggttcgccgttcaatacctgttgggattcttccattaactcattcagtgcagattggccggcaccggaaaccgcttgataagttgagacgataacttgcttcaaaccatactttttgtaaatcggttcaaggcaaaccaccatttgaatcgttgaacagttggggttggcaataatgccgcggtgattataaagagccttttcgttaacttcagggatgaccaacggaacctctttttccattcggaaagcactggtgttgtccacacagacagcaccacgcttaaccgcttccggcaggaattttttggatgttgagccgccggcagatgacaataccagatcaattccgttaaatgagtctggggtggtttcttcaaccgtgatatcttgaccacggaattgaagaaccttcccggcagaacgtgatgaggccaatagtttgacactcttcaccggaatggttgactgctctaattgttggatcatgcgggtaccgacagcacccgtagcacctaaaattgcaacgttaaactctttcatcctaatgaatccccttttctctattttgttaactcaagtaaataactgttcatgcgatccattgccaatgtgatgtcttcatcagacgccgcatatgacatgcgaatccagccttcgccgccggggccaaatgcggaaccgggggtcacgccgactttggcgtcctttgccaaatgagtggcaaattcaaccgaggtttcgtctattgtatcaggaatcttggcaaaaatgtaaaatgcgccttggggcatgacaatctgcatccccattttttcgagccgatcagcgatatagtcacgccgtttgtgataggcagcccgcattggaatcggatcatcaaggccgttggtcaatgcttcggcagctgcgtattgcgcaggattggaaggagcggtgaccacgaaagcgtgcattttggatgcgttggtcacaaaatcctttggtgcaacaatgtagccgattcgatatccagtcatagcatgggatttggacaaaccgttaatcaaaatggtttgaccgggaatcatggccgcgattgagtgatgcttgacgccataggtcaactcactatagatctcgtcagccagcacatacatcttgtgttgagaaataatatcagccaacgcctttaattgagcctctgtgtattcaactccagttgggttggatggataattcaaaataattgctttgacactgtccccattttcatcaaggactttttgcagcttttcaggagttaagacaaacccatcatcagaagtgtcaatggtgatcagttcagctccggcaacttgaataattgggaaatacaaggcaaatgccggggtcggcacgataaccttgtcacccgggttcaagatagtggtcaacgctgaatagatcgcttcggtagcgccaacggttaccacgatttcagtggccggatcatagtaaacacccgtccggtccttgagataattgctgataccgtcgcgaagttcaggaattcccttttgtgctgagtagtgggatttgttttcctcaatactcttaatagcggcctgtttggcatgttccggaacatcgaagtccggttcgccaatcgtcaatttgacggtgccgggaattgaagaaatcgcctggtcaaattcacgaattcctgaaggtccaactgcatttacattttgattaacgacttctgaaagtttgctgtctaactgtggcatgttttcctcctgatttaattacataatattttctaagccgacgattaacttggtcgctttggcggccgccggcactgccagttcaaccccgctcatgaaagaggcgcggtcaaacgagtcttggcggatcgtcaaggcttcacctttgctgccgaaaagaacttgctcatgagcaacgtaaccgggcaggcgaacggaatggatcttaatcccgtcgtaatcgccgccacggacaccctttaaggcttcctcggttgcgggtgcatcgtgcttcccacgaacttcgtcaatcattttagcggtcgccagagcagtgcctgaaggagcgtccagcttatcgtcgtggtgcatctcaatgatttcaacgcccggcatgtatttggcggcttctttggcaaacttcattaaaagaaccgcggagatgccaaagttgggtgccaggattccaccgacgttggtttgttgagccaactttttgagctgatcaacttgctcatcgctcatcccggaagtcccaataaccggatggatgccgtgttcaatggcaaatttggcattgtcaaatgcagccgcaggaacggtgaagtcaatccaaacatcggcgtcggtgtcgatttcatccaaactggcaaacagcttaacgttatcatccattcccatacctttgagatgaacggtgtcgattccgggattgtaagccccaaccaattcaaagtcatcgtttttattgaccatttgaaccgtcttttgacccattgagcccatgaaaccagcgactaaaactttaatcattgaaaaaactcccttgtctatctttgtttgataatttccaaaccaatcggcttaactgcgtgccatttcagtgccgtcaactggaatatcttccaggcggctgacacctaatttacttgccagggttgctttttcttcatcgttcaatgaaagaattggcaagcggcaatcaccggccccaaagccttgaacattcaaaatggctttgacacatgacggtgatgggtacatgaataaggcttgcacttttggcgtcaagaaacgcatcatgtcgccggcagtctcaacatcgcctgattcaagggcgtcgtacatcttccgcatctcccggccgtaaatatggctggtaactgaaatgacaccgttggcaccaactgctttagcagacagggcctgggcatcttcaccggtgtagacattgaaatcatccggggtattttgaaccagatattccaagtcttccaatgaggtacactgcttaacgccggcgatgttggcgttatgtgataattcgaccaccgtatcgttagccatcgtgacgccggttcgacctgggatgttgtaaatgatcaatggcactggtgactgttcagcaactgccgtaaagtgggcgatcatgccacgttgatttggtttgttataatatggcacaaccacaagggcgtaatcaatcccgggaatgttacccacttcagctgttaaacgcacggtctcggcggtattgttactaccggttccggcaataatcgtcccacgcccgttcacaatttgagcaaatcgggtatacaattcaatcttttcgtcatgactcaaagttggcgtctcgccagtggtgccaccgattacaaatccgcggctgccggtatccagtaagtgattggttaatttttccaaaccgtcaaagttgatgctgccgtcttcaccaaacggagtcacaattgctgtcataatatctgcactaatcatcataaatccctactttcttttattgggttaattattcattctgtattcaagaaatctggtaattgacttaattccctttggaatcgatgattctttggggttcagggtagctgagtgaagctgtgaatcatcgtcgacgcccaaccaaaacatggtgccgggaatcttagataataggtaaccaaaatcttcgccggtcatcgccggttgagtttcaacaaagtcggtttccggatcctgcttggcaaattcaatcaatcgtcgagtcagttcgtcgttattttccaccggcaaatagccaccctgattaaagtgaatcttgacttctgcgccatagctggttgccactccattggcgaccatttttagccggtcaacaatgtgttcaatcatcttctgggttaagccacgaatggtaccttcgattctggcttgcccggcgatgacgtttcgaatggtgccggcgtccagcttgccaaaagtaatcacaccgccttcgatgggattgacacttctggatacaatcgtctggacttggccgatgaattcggctgcggcaaccaccatgtcgttggcgttctgcggataggcggcatgaccacttttaccaatcagatcgacattgacctcggtcgttccggcaaacaaggttcccattcgacagccaatcgcgccagccggtaaatccgggttgtcgtgcaggccataaaattcatcgggccgccactttccttcaaagacgcctaattcataagcaaccttgccgccgttttcgctttcctcagccggttggaagaagaaaaccatgttgtcagccggctgatgctcggaaaaccagttgaggactcccagtgcgacggtcatatgaatgtcatgaccgcaagcgtgcatcacaccggggttcttggatgaaaatggtaagccggtcttctcgctaaccgtcagggcatcgatatcggtgcggtaaccaatcgtccgtttagggttggatccgttcacgtacaccagcagagccgtcggtaatttggggatttctcttatttcaatgtattgttgattgaaagattgaatggttttcaacaggtaatcatgagtggctctttcgtgcatcgccagctcaggatattcatgtaaatgtctgcgaatcccaattaaatcttccttcgttagttgactcattgaatcacaactttcttaaatcgtcttccagaccagtttccgaggttgtcttttcatcaacgtccttgacctttcgcgctgggacgccggcaaccacagtgtgtggggcaacgtccttggtgacaatggatccggccgcaaccacggcgccttcaccaacatgaacgccttcgataaccacggcattcgcgccaactaagacgttatcgtcaatctggaccggtttggcagatgccggttcaacgacgcctgccaaaacggctcccgcaccaatgtgggaatgcttgccgacaattgctcggccgcccatgacaacgcccatgtcgatcattgtgtcatcaccgatttcggcaccaatgttaatgatggcgcccatcatgataactgcgttgtttcctattgtaacgtgatcacgaatgatggctcccggttcaatccgggcattgatctccttgatgtctagtaatggaactgcagagtttctggagtctgcttcaacctggtaatcatcgatggccgatttgtttttcttaaggaaccgtttgacgtcagcccaatcgccaaacaaagttgcggtgtgcttttcggcaaatgccttgattgattttggaaacttgatgtccttaatcgatcccttgagataaatcttgaccggggtcttcttcttggcattgccaataaaatcgatgatttctcttgcgcttagttgttccattgtgattctccttaatgtcgttattttgtatgaacttttaatgtaatttttatcgggaactggaaacgtctcaaccagcctgtggctaaaaacacgtttgttagattcttttgaggtagcttaagctttgaaaatacgctccgggagccagatgctaacttctaagacaatcatgattcaagcccaaaatcagggcttcaatcatgattgtcttagaaaccgcatctcccggctccctccgcgctctgctctagttgaattcctcatccaacgccaccaaatcttcaaaagtttctcttctgatggcaacctgcgacttgccgttttccacaaataccactgccgggcggggattacggttatagttggaggccattgcatagccatacgctccggtgtccagcatcgccaaaacatctcccggttgggtggctggtaaatcctgcttttgaatcaggatgtcaccggactcacagtacttaccggcaatccggaccgtttctttaatcggtgcacttgggtccttggccaagaccgcctcgtatttggcttgatacagcgcgggacggatattgtcacccattccaccgtcaaccgtgacgtatgagcgaatccccggcacatctttgcggctgccaaccgtatataaattgtatccagcgggaccggcgattgaccggcctggttcaatccaaacagcgggcattggcaggttgacttcttcggtacgtttcttgatggccttaacgattgcatcgacaaacatttccggagcaatcgggtcatcatcttccgtgtacttgatgccaaaaccaccaccgacgttgacaactttggcaacataaccaatttctttgttccagtctgccaaagtatcgatcagcttaacagcagccatttcaaatccattgacttcaaagatttgcgaaccaatgtggcagtgaatcccaagcatgttcatccgctcatcttcaaggaccaggcccaatgctttacgggcctgaccgctttgaatatcgaagccaaacttgctgtcgacttgaccggtctgatcatattcgtgggtgtgggcggaaacccccggtgttacccgcagcatcacgttgatgtgtgattgtttatcttccaaaacttcttttaacaggtcaatttcatggaagttgtccaaaatgatgaccccaatttgatgttcaactgccatttccagttcttcgcgagatttgtcgttgccgtggaaactgacccgttccattggaaagcccgctttaatggccgtgtataattcgccgccggaaacaacgtcgatatggcccttttcctggttaatcagttgaaacattgcaatgcaggcaaaggctttgctggcataactgaccgcaaaatcgacgccgttatcttggaacaccttttgaaaatggtgaatctggtcacggatggatttcacatcgtagaccaccagaggggttttatattgcttaaccagatccaatgaatctactcccccgatttccaagtgtcccgcttgattggttaataactggtcgatttgattgctcatgttttctcctccaaaatatctttttgtgaatgatggtgtggtgaggtgttggtgggttggtagaagctgtgtctgtcgaggcttgtcgcgcaggaagcacgtttgttatgattctttgagctccctgcagcttccaaaatacgctccgagggccagaggctaacttctaaggggacctttgattaaagttccaaaaccgggaacttcaatcaaagtccccttagaaaccgcctctaccagccctcgtcgcgctcttaataaaaaaatctcctcattcggcgttcgccaaacaaagagattcagaattttagttcaatatcattccgtatcatttgtcgttagcgccccgcagccgacttatccgccgcgacagtccatagcctcttaagctaagtcccagcgcgccaagtgctacctcacatggtgcttcggcaaccgcccctttcattagcttcaaagttcaggtaggaactccactaattactgatgttggttgcaacctctaatgatttaattgacataattctataatgattctcataaaatgtcaaccacttttatgagtccggatgcaaattcatgcaaaccaatcacgataaactgatgactcttgcaaattaattcaaaactgctaaaattcgttttaacaatctctaaccgaattgttaattaatgggaatatccagggagtgaatgaaagttatgaaagtcgttaagtttgggggcagttcgttagccgacgccgcccacgttcaaaaggtgattcgaatcgttcaaagcgatccggaacgaaaggtggtcgtgacttcggcgccgggcaaaagattcgccgatgatatcaaagtcactgatctcttgatcaaatatgccaatgcgatcatcgatggaacggatgccaaagccactgttgcaaccatttttgaccgttaccaggaaattggcaatggcttccatgtttcaaaaagcgtccttgatgatcttaaggccaaattaactgccctgcccgatcaatcatatccaaacgacgactacctgatggccgcctttaaagctcatggtgagcgattgaacgctgaattatttgccgcctgcctgactgaggccgggacccaagcgcgcttcgttgatcctagcgaagccggcatcctgttaagcgacaatcccaatggcgccaccgttcttgaacaaacctacgacaatctcgctgatttgacatatggtgaggaaacgttggtcttccctgggttctttggattcacccaagaaggcaacattgccactttcgctcggggcgggtccgatattaccggctccattttagctcgcggcctaaaggcggatctctacgaaaacttcaccgatgtcgatgcaatcttcgctgccaacccgaaaattgttccggatgcccgaccgattcataaaatgactttcagagaaatgcgtgaactttcatacgccggcttttcagttttcaacgatgaagcaatcattccagctattcaaggtcaagttccaattaacgttaagaacaccaacaatcccgatctcccagggacattgattgtccccgaaaaagattttacttcaaaaaaaccggtgaccggcattgccgcatccaaccgattctcagccctttatctccacagatacctgctgaacaaggaagttggctttaccctcaaaattctccaaattctgtataaatacgatgtttcctacgaacacatgccatcaggaattgacgacttgacgatcatatttgaccgcagtcagctggacagtgatacaattaaaaaaatgtgtcacgacattcaggttgaactgaatccagatacgttggattggatcgatgattacgccattatcatggtggtcggcgaagggatgcgggcaagagtcggcacgattgaaaatatcatccggccattggctgaacacgacatccccgtccatatgattaatcaaggggcgtctagaatttcaattatgctgggcactcgtcaatcagacgccgacgcagcagttaaatacatttaccaacatttttttaaagaagatccttccgttaaccaacttgaataccaggcggaagtgtagaggaggcgcgttatggttcaattactcaaagttcatggatcacaaaataagttctttatcttagatcaaacagctttacaaactaaattaagtcagcccgaattggtggccttggctaaacacattactgaacctgaaacggggctcctcgatggtgccgacggcctgttggtcattgacgattccgaccatccagacactttaggcagcatgcaggtcatcaacaccgatggcagcattgcgtcaatgtgtggcaacggactgcgcaccgtttcccgttatctgtcagacaaatttggcaaagatcaattcaaggtcgaaacgatggatagtgatctgcatgttcatcgtgaagcggacttggctgacaacgtgccaaccttcagcgttgaaatttctccggtgacattcgctaaggaaaccctgccttttgacaatttaggcaccgatacactcatcaacaaggccgttcccgaatttgcgcccggccttaaattcaccgcaattagcgttcccaatccccacttaatcagttttgtggacgaggaaaccatgcactcaaagaccttggggcaactgggcaagatgctcaacgaccccaatccttatttcccagatggtgttaacgtcagctttgcccagattctcgaccacaacacgctgttcgttcgaacttatgaacgtggtgtcggcttcaccaatgcctgtggaaccggtatgtcggcaaccagcttggcgttttgcctcaaccatccggaaatggccgactttgacgaactgatctcggtttataatcctggtggcatggttaagaccagggttcacagccgcgatgataccttctcaattgacttgatcggtaacgcgactttcactcacaagattgaaattccggaagccgatctccatgccaatgatttagagcatgcacaggtcacagaaacagatgaacaaccggcatacctgagatttgtggaaagtcttaaaaaccaactggttaaataaacaagagtcgaacacaaggcatcttgattgcagaatttaagtaaaaaagcgagttattcctgttttggaatgactcgcttttttacttgaatggccgggatcagccgatggttccacgtttaagctagctatcgcggcccagacatgatcaacaaattagtctgtcttagcctcatttttcagtgtgctcattgacccacacctcatggattaattgattggccaacaccttgcaaatcatttcaatcagctgatcctgcatgaaagtggtcgcgtcaaagtctgccggctgcccattaatggcggtaatccgcatccgatcagtttgaatttcaacgttatatttggcaaaagtatcaacaatcgcctgtaatttttgcgcatttaacatttactgacctcccagccgcagctttagtcgccattcgtcttggcggacttggttcggcttgatgcgtaaatccagatagggcgccaccaacagcaagaaatctttgacgtcttcataatgtgatttgcttgagaagtaatgattggctttgcgttgggacaacttgtcaattttaatctgcagcttgtttaaatagtcttccaccagctgaatggtattttcccgaatactggcaatctgggcaatcttttcgtcgtcaggatcctcaatctccaactcttcaaccaactggtaatggtttaattcctggtcatcaggattaatcagttccaagtcaccgtcatcaactgcggcagcaaaggattcgccatccgttcgcgccaaataagtgggcaattcttccccggtcattttaaccagcaaaacgacttttcgggcaatcccttggccaaatttgatgtgaatgacaaaattctttttgccgatataattgacgttgtctaaaattaattgtgggttatgggtaaccacttcaccaatcgcgaaataagtcgcccgttttgttcgataaatctcaccaaattgtggtgtcaattctacacgtcctttcgttgttgctcataagcatcataatacgttacttgaagattttttcaaagtcgggattttccaaacatatgttcaataattttgtataataggtattagataattcaaaacgaaatggaggggtcgtcatggccgtacaccaagtcggtattcgagaactagtggaatttttactgcggaccggtgacttaagccccgtcatcagcagtcagaatacggcacaagaaggcagtcggatccaccgcaaaattcaacgcagccgaccagcttcttatcaatcagaggtggcactgaaaacctcgatccagtatttggatgacgaatacgtcattagcggtcgagcagacggcatcgatgaccgtgacggcaaaccgttgatcgaagaaattaagacctccgacttggaattcagctcggtgccggactccacccttcaactttattggggccaagtcaaagtctatgcttacatcgtcatgcatcaagcagatattcgatcagttgatctacagttgacctacgttcagacacctgatgaaaaaatcaccaccaagacccagacgattaccaaaaccgactcggaactcttcttcaccgccttggtcaccgaatttgagcaatggatcaaactccggcatgaactggacgaaaaccgaatcagttcagcgaaaaaactccaatttccattttccgactaccgccccggccagcacaagttagcaaccaatgtctacaagaccattcttttggaaaagcacttgtttgttgaagcgccaactggaaccggcaagacgatttctaccctttttccggcaattaaatcaatgggtgaacagctgatcaaccgcattttttattttacggccaagcagagtacccgtcacgtggcggaaaacaccatttcgatgatggctgaacaagggctgaaattaaaaagcatcaccctcaccgccaaggacaagattacgttcccaactgaaaaagaactgccacctgagaacaacccctacatggtcggctactatgaccgcgtccggccggcaattaaagatattattcaacacgagaatcaaatcaccaaagccaccattcaagaatacgcagagaagcacaaagttgaccccttcgaattttcactcgacgtcagcctgttttgtgatgtcatcatttgcgactataactacttgtttgatccccaggttcacctgcagcgtttcttctcatttcccgatcccaccaactgctttttggtcgatgaagtccataatctggtgcagcgatcacgggaaatgtattcggcgacgttggaatcatcaccgattgatcccctcttagaacagttggtgaagaaaaaggcaagcaaccaaaaagtcattaaacggcttgaatccttgaagcgctcatttaaacgttatagcaaaccagcctcagaagtggttgataagcagattgctcaactggctccactggataatttcaataacactttggagaatctaatcgaaacgattcaccagtggctggcaacccaagccccgagtgataccgttgacgcggtagtcgactattatctgcaatgccgccgctattacctgatcagcaccttttatgacgaaacctaccgcacacggatcatcattggcgatcacaccatcatttttcgccagttctgcatggatcccagcaagcagctcaaagcctgcttgaaccttggccgggctgcaatcctattttcggccactttgagcccgatgtcatattaccgacaagtcttgggtaacgaggaagacagtttgggaatgatttcacactcgtcatttccaccccaaaattgccaggtgattatcgccaacaacatcaatacactatacgccaaccgggaaaatagtctggagccgatctgcgagaacatttacaccatgatcactcaaaaggttggccattacatgatgttcttcccttcaatggcgtacctgaacgccacattgagtaaatttgtcgagctgcatccagatattgacgttatcaaccagcagccggaaatggacaatgcggcccggaccgcctttttggatgcctttcgcacggaagatcatcaaaccaaagttggttttgctttactgggtggcattttttcggaaggcatcgatctgaaaaatgatcagctgattggcgtcggcattatcagtgtcggtcttcccggcatgaacaaagaatccgacctcatcagagactactttgactcattgaatggtcaaggattctcatttgcctatcagctgccaggctttaataacgtcagccaggccgccggacgggtaattcgcactgacgaagacaaaggtgtgatcgttttgatggatcaacgcttcaaccaaacccgttaccggcaaattttcccccagaattggaccaacattaaggtcaccaataatcccaatcagctaagaaatgtcctgcaaaacttttggcagcacggtaatcagtaagtgttctcgtgccaaaaaaagcgaatgggtgtatactaataacgctgttcgttaatcgaattaaagccaggaggggtaatcttgaaattagcaatgtatgatcatcagccaacatttgtggcgctccaaaacggtcagttctggggcgttccaattattggttacgactcaatcgacgatattttaaacgattggcagaactttttggctaacgtactcattaatattaacgacgataaaatcatcgacaatgacaatgccactcaacttgatccacaacattttgagcagcccgttcagcatccccgtcagctgccggctgttggcttcaactatctcgatcacatgaaggaaatggacattgtcaaacccaagcggcccaacatcttcaacaagtttgtcagctctttagccggccctcacaactcgattcatttgagtagcgacaccgtcgactgggaatccgagctcgtcgttgtgattggccgtggtggccgcaacattagccgtgaagacgctgaagacgccattgccggctacatggtcggccaggatatttccgatcgaaccgttcaatcaatcgatggtcccagtacgcagtttgaccttggaaaatcctacaaaaattattcgccggttggcccttacataaccaccatcgctgacgttgacgatattgtctccaagaccgttaccaccaaggttaacggcgaaatcatgcagcaggcgacaattgataagatgatttttgatattcaaacgctggtctcttacatctcgaacgttattgaactataccccggcgacctgatctttaccggaacgcctagtggaactggcgttggccgtgatccgcaagtcttcttaaagtccggggacctgtttaccagtgaaattgatggtctgggaaccatcgagacaaaggtcaactaatcaagtcatttatttttaaagaatttccaatcaaaaaagctggagctaaatcgttgtgatttggctccagctttgttagtttaagttttaattgcaatttaattctgactgatactcgtcaatgttacttcttgcgtaaaattgaaacaccttcgggcaccgtgaaatccttttgaatcatggttaatttgccagactcggggtcacgcgtgtacaatgtagcgttgtcagaattttggttcaaagcgatcacaaaggattgatcatcgcttaaattaaagtcgcgaggaaaatcgccttccgttgaaatccgctgaatcaatgacaaattaccggattcatctgaactgaagaccgcaatcgaattgttcccacggttggaaacatacacgaagcgcccatctttggaaacccggatggcagcggccccattatgttcggtccagtcatcaggaatagtcgagtgaatgtcccttaaggataagacgcctttgtcggcatcatagtccagtacggcaacattgctgctcaattcgccgactaaataagcgactttcttcttggcgtcaaagtaaatatgccgtggaccatagccatcttgcatttgaagttcgctaaccggcactaatttaccgttggcttccaaatcatagataaagactttgtcgacgcccaagtcaacggccacaactctaccttccggtgtcaaattgatatagtggggatgaggaccgtcctgttgctcttttcgaaagccgagggttcccttatccatgattcggtcggcctttgaaattgagccgtcatcggcaatccggtaggtgttaaccgttccggcatgataattggcggtaaagactaactgctgatcttcgtcaaccgcaatgtaagccggtgaagtttcctgatcgtgaaccgaagcaattggtttcagtggaaaatcatcgctggtaccatcccattcaacgaagccaccggtcacgtctcccttatcatctttgactttggtgatcgcgtagatccgtttttgattggattccgcaacgtaggttgggtcaatggcgctgccaacaaacgttaaattttgtaatttttgattttcagtatctaattctaactgataaacacctttactaattcttctggtataggttcctagcaagtatttttctatcaaaattttccctccaataaaagtttatgtcttcattatgccacagataaaacctaaccaaaacacatttgaaagctttttcacgaaaggaacaaattttatgacatcttttgaaaaatttcatcccgttctcaccgcccacttaacccttgattggctaacccaaacaccggtaaaatccattgacgatctgttttccaagccggcagttacaaccgcaaaggccgagaaaatgcccagccaaattctcgatactgttaaagagatcaatcacataatgcgccgggtaatgaacgacaaggaattgacttggggaattaccgactccaactcagacgcgtttgttggcatcatcagcctgcgtggctttgaagaagccaccccatcgggatcaattgaattcatcattgaccaggatcaccgtgagtatctggcagaagttgttgaaagagctatccgattttcccaggatcattttgaattcaatcagctttcaatcacgcttaatgatgtatcttcacaaaccgcaaaagaactgagtggaattggttttgtaggcgacggcgaacagcggtttaccatccaactttaaactaatttcaaagtaacaaaattattaacgacaatccaattcagaatcgttgcatatccagaccaagcatattagaattgttctaaagtaacgattggattataataacagtgaagaataacagaacgctcctcatggaggtgccaataatgacaaacacaactttaaaacgttccctgggtcaacttaaaaaacagggcgtccggattactcctcagcgagaagtgatcttggattatttgattacccaccataatcacccggatgtcgaaaccattcgcgacggcatcgaagacaagttgcccaacctcagcgtggcaacaatctataacaccctcaagatgctggtcgacaatggcttggtcattgaactgccaaataacgatggcggcatccgttatgactattttggcgtttcccattaccatgcaatctgtgaaaattgcggcaaaatcatcgacatttttgatgatgactatcccgaattagtcaaacacgttcaacaaaccaccagagaaaaaaccgactttctggtaaccggtacccaattagaggtcaccgggatttgcccggattgccagcgcaaactccacctggccaagcttgccaataaatgattattacagcgttaaactgttgatatatcagtcattagctcgataatttaagaattttgtcaagaactcttaatatgattgacaattagtaccgcaaagcccacgggtacgcgttaaatcgctatccgtgggctttttgtccggttgaattgtatcatgcaaatcgtatatattaatgaccgtagctaattaccactatgtaaaaataaaataaacatttaaaacgaaacttaaaaaaatctgcaataaacacttctgaagggaataattaatttgaaaaaaagagcgattgtaacagccctttgctcgctgacactggcggcaatcggcatgtttggactaagcagcactgcgggggctagcagtgtcaacgattatattgccaataacaatatcggccatgccagtgttacctcatcggtgtggagcggttttccaaagaacgcctaccgcaacggaaccggtaagcctgaaggggtcgtggttcatgaaactgccaaccccaactcaacgatttataacgaaattgcgtacatgaagaagaattataataacgcatttgtccattctttcgttgatgccagtcgaattatcaacatcgccaacaccaactacttggcttggggtgccggctatcctgccaatgcccgcttcgtccaatttgaacaggtcgaagtccacagcaagtcagcgtttgcccacgaaattgccaacgcagcttactacaccgcctacattttggataagtatggcttaaagcctaatgatgcagcgtatgatggcaagggaactgtttggtctcacgggggtgtctccaaatatctgggcggtactaatcacaccgatccagccggctactatgcatcagcaggtaagaaatacttcggtgccagctatacgtttgcccaattttatcaattggttaagacaacctacaataatttggcagacgatggtgcggcccatgggtcactaaccgcttcatcagcaaaaacagcgtatgacaaggtcacatacgccaaagcagatacaaaggcgtcattaggagacaactacaagtcatacagattatacaatcacgttaagaattcacgatcaggggtcaaatcctattcgtgggcctcagttgacgcttctgttggtaagaaggtctatattgatgacatcgggactaaatcaaacggtcacgactggtatcggattaccttctccaccgacagtggtgcgcaaaaatattgggtctacgaaaaagcccttgacctaatcaattgacatcatttatgaattaatatatgattatgacaatttagaagaccaagtagtgtgcgtacagagaaagtgccgtcggctgaaaggcatttaagaacacgaatcctatcttcaagacgattgccctaatccggcacggatttttccgttataaaacaaaaagtgtgaagcctggctttgaatgagaatggtaccgcccgttgtgggtgtctcaatttcaaagcaggctttttttatacaaaaatatggggtgagcagatggacaaacggattattaacgcaaatcgaatcgtggtcaaggttggtaccagcagcctgatccacccaaacggtgcggtcaacttgaagacttttgatgagctggcgtacactttgagcgcgctgaataaccaaggcaagcaacttgtcctggtttcctccggggcaattggggttggcttgaacaaaatgcacctcaagaaacggccaaccgaaattggtgcccagcaggctttggctgctattggtcagtcagagttgatgacgctgtttacgcaacgattcgaccactatctgacagacattgctcaggtgcttttgacccatgatatctttgattatcccaagagcaaccagttcgttatgaacaccttcaattgtctactgcgggacaatgtgatcccgattgtcaacgagaatgacacggtggccactgatgagttggaccacaaaaccacttttggcgataacgaccaactttcagcaatcgtggccagccacgtggatgcagatttgctgatcgtcttgtcagatgtcgacgggttctatgatcaaaatcctaataaagtcgctgatgccaatctcatcagaaccgtgagccacgttgatgaaaatgaatttggtgttgccggcgggaccggcagccgctttggaaccggcggcatgcagactaagctgctggccgccaaacgaatgctcgacgaagaccggatcatggttttggccaacggtgccgatccacgcattatttttaaaattttagccggcaaagatgtgggaacgatctttcaaaaggagagtgtagctcatgaatgacaaattaatcgaaattggcaaaaatgccaaagctgctgcttataaattgaacctgctggataccgcgaccaagaaccgaatcttaaacgaatttgcgatcgccttggggcaaaacgctgagctgattcttaccgctaatcaaaaagacttggccaacgccaccgacatgcccagcaaatttaccgaccgattaaagctgacttcccaacggattgctgacatggccgagggtctccgccaagtggctggactcgccgatcccatcggtgatatcgacaagggctgggagaatgacgccggcttaaacattgaaaaaaagcgggtaccgttaggcgtcatcgccatgatttttgaagcccgccccaacgtcactgtcgacgcctccgctttgacatttaagagtggcaacgccgtcatcttgcgtggtggcaaggaagccatcaacgccaatttggcgctggctgaggttctccgtcaggttctaagcgacaatcagctcgacgaaaatgccattcagattctgcatgataccagccacgatacggccaacgacttgatgcatttgaaccaatacgttgatgttttgattccacgaggcggggccggcttaatcaatgccgttgtgaaaaactcgacggtccctgtcattgagacgggtgccggcaactgtcacgtttacgttgacaaggatgctgagttacaaatggccattgacatcgtcgttaatgccaaagtccaacgcccatctgtctgcaacgccgctgagaagctgttgatccaccgggatgtagctgaaagcatgctgccggcaatcgctgaggcgctggaggaccacggcgttgaacttcgtggtgatgaagccagccggcaaattgtctcctcaattaccccggcgactcaagaagactggtcaaccgaatacaacgatttgattatggctgttaaagtcgttgacgacgagcaggccgcaatcgaacacatcaatcaatactccaccggccactctgaagtaatcatttccgataactatcaaagcggtcaggaattcttgaataaaatcgactctgcctgcgtttacgtcaatgcctccacccgatttaccgatggcttcgagtttggcttcggtgcagaaattggcattagcacccaaaagctccacgccagaggacccatgggcttgaacgaattgactaccaccaaatatgtcattcggggcaatgggcaggttagaaaataacgagtttaataagcatattgatgagaccgggagactgggacaaaatgaaagattctgttccagcctctatttgcgtccgaatgttatctggcagaactgtgcgccaataagcagcttccggccgtataaggggattacccaaacatccaagccctggatatttgggtaatccccttatcctctggaagcaaaccgcttattggcccacgctgccgttttttattgaaaatacgctgtctttcacttcccttttctgaccagatgacgtatactgtatttagttagccggctaactaaatacagaaaggggggggaccaaccgtgagttattacaactttgtcgatcgacccagcaagcagcggattcaagagatggccgatcaattacacttggcagtatcacctgatgcggtgcatttattcttggattttcaactcgcctatcgggaagtcgaaaagaactatgaaagtctggtggcgagttttgacctaagcgaatccaggttcatcatcctgatgttcttgtattatgcagatgacaaacagctgctgccctctgagattgcacacaaattgggggttaccaagccaacgatcagtaagctgttgcgggggatggaacaacaaggccttgtcagcagtcaccagtcttcaactgacaagcgggttcgggatattcagttaacacctgcaggtgaaaagctgctgcgaacttttttgccctataactatcggtcaagttccctactatttgaagattttactgacgaagaaaaacaacaattcgcgcatttactacgaaaactgctcaaatccaaagacaagatccaacaactggaggaagactatcatgaacacagaaaaaattaatttactggaaacttatttaagtctgtacattaaccccatggacgttttgaaagccggtcaaaccggtcagtcgccctatgtgattttagatgttcgaaatgcccctgcccaggttaaaaaagaccagatcaaaggcgcagttgccctgcccgccaaagacttggcagctcatctgagtgaactggacaaagctaaaacctatgtggtttatgactggaatggcggcacaatcttgggtaaacaagctgttttgatcctgctcaaagccggatttgacgcattcgaacttgccggttccctggaaggctggaaaggcatgaacctgccactggaaaccattcaataattttggacgcatttcatttgaacaacggacaccaagaaggccgaaacattagagaatcctgatgtttcggcctttagtctgtctattttaatttacttcagtaaatggtgctgttgcagatattgcttagccacagccgcggccgaacgatgtttaacggtcacttggtaattcatctcctgcatgtcacgggttgtgattttgcctgctaatcgactgagtgcgcgaaccacttgtggatgcgtcttggcaaactggtcggtcatcaacggcgcgccttgatacggcgggaagaattgtttggaatccttgagcaccaccaaatgatactccctgatttgcggatcggtggtgtaagcgtcggtgacgtcgacccggccatctgccaaggcgacataccgtaaagagggctccattgtccgaactgattttaattggaaatgataggcttttcgcaatcctgggtaaccgtcggactgctggtaaaagtcgggatcaaaggcgccggttaattggctgccaacccgttgcaaatccgcaattgtgcgtaagtgatactttttagcggttgactgacggacggtaatcgcatagccgttttggtaggccattggcttcagataccgcatatggaatttttgactcaaggcatttttagcatccctgtaggccaattgaggctcgctattcacctttttgggggaatgaaccagggattggagaaccgtgccggtaaattcaggataaacgtcaatttggtcgctctgcagtgctttgaagagaaagctggtcccgccgaagttgggtttaagttgaacttttgtctgtgggctctcttgtttgaccaagtctttatacatattgatcaaaatttccggctcaccgcccatttttccagcaatcgtaaccgtttgggccggcttgttgaacaaggaccaccctaatcccgcgccaccgaggatcagtactactaagacgccgattcccagctttttgaaagaaaattgagataagactttgattaaccaactggcaaccagtgccaagatggctgataagactgcgccaacgattaaggcggcattgttgttagtctgaatgcctaacaggatatatgttccaagaccgccaccgccaattaaagcggccagggtggccgtcccgatcaccaggacagtcgcaattcggattcccgaaagaatcatcggcatcgctaatggcagctcgatccggaacaatttgaaccgtttggtcacgcccaaagcgtcggcagcttccaacaacacaggatcaatgtgggtcaggccggcataggtgttttgaaagattggcataattgcgtacagcaccaaggcgataattgccggtaccgtgccaatcccaacaaacgggattaaaattcctaaaactgcaaggctggggatcgtctgaatcacgccggcaatttgggaaatgatttcgccgatttttggccggttcaccaaacaaatcgctaaaggaatcgcaatcacgatggtaatcaagatcgcaatcaatgagatttcgatatgctgccaaagggcttggatgatggcagcggcatttttatcaacatatgccacgacttcgtcaatcatttgtcggctcctttcccaaatcggcgacataagaaatcaagtcactttgcgtcagaatggcaccatccaccaaaatcagctggccgggatttttttccaacagacccgcccattcatagactgtctggctgttctgcagcgtaatcgcctggtcatctttgccaactggacgccccaggccggcattaagcacttgttttaaaagtctggtgccggaattgtcgacgtcaaagaaccgtttgacaaactcatcggcaggattggccatcaaataatccggctcaccttcctgtaaaagaaccccattatgaataaccgccaatctatcagcgagtaaaaacgcttcgtgcatatcgtgagtcacgaatacaatcgtggtgtcaatttgttgatggagattcaaaataatcttctgcagttgcctacgggataccggatcaagggcactgaagggctcatccatcaacaccaacttggggcgggcagccagggcccggacaatgccgacccgctgagcttccccacccgataattcgtcgggcatccggttcaaaaattgatcagggtccaaattaactttgctcatcaattcaaccacccggtcatgctttttttgagccggccaacccaagttatcaagttgaatggtggcattttgttcaacggtcatattgggaaacagcgccccggtttgcagaacgtagccgatgtgtcgccgcaatttttgtaggtgactgtcggcgacgtcctcgccgtcaattttgaccgtgccgctggttggtaccactaaacgattaatcgtcttcagaagggtcgttttcccactcccggaaggtccgaccaacacaaaaagctcaccatcatcaatggtgaggttcaaatctttcaatgcaaattggccgtcaaacttttttgtgacattcgtaaactcaatcaatgtcgatcacctcgtaaaatccatggtgttttaaatatactcattttgacgatcgaacacaactcaatgctttaactgtgctttgtggagtcgcttcaacttgaaactcatcagccaagtcgtaacgggaatcgtcgtaacgaccccgattaaggaaaccacaatcgcgatcaattccgcagcaaacaccttgtcgttaagaatatcgccgaaggaataattcaagccatagaaccaaatgaataacgccaacgaactgccaaagaagccaaagaacagagtattaacggccgttcctatgatttgtttgccaatcacggtgccatccaagaagagctgttcacttttaatggcttgatgttgagttataatttcatccaagccagaggcaatcgcaattgcggcttccgcgaccgctcccaatgaactcagaatggcggttgcaatcgcaattttcgtgaaatcaatgccgacatacgttgaaaggccttcaagttcctcgctgtcttccaaaccaaaaccgccaacctgggcccaatattcaatcggaataataatgactacaatcaatatcaaaacaatcaccgaagcctgaaaggccgtggttgaggcgttgtcgctggcactgctccaaaaaatagtgattgacagtaaaatcacgctggcgacaatcgtgacgataattggcggcaggtgaaaggcaatcagcacaatcgtgaaaaagagaatgccaaaattaaccaccaggctgagaaatgaggtgataccctgtttgcccccaacaatgatcatcaagaccagcagaacaatccccaaggctgtaatagctcccattagcgttcatcccctttaatccagagtccggcaaaggcactcgataaaattaccgtcagaacgatcccaatgccgctaatcaggctggaagtcatccccaatgacatgttcatcgaaaacgaatagtgccaggtgttgccattttttaagtaaagtaaggtcatcgccagggtttcggccatgaagatgaagaacaaaacgttaatcaggggccccataatcgatttgccaatttgtctgcctgatttaaaaatcgccattcgagacagttccgggcgctcctgcttcaacgtcgccaaagaagcgacaatatcggtggcctcatccatgacggctcccagcaccccaatcaggacttcggcgataaacaacggcttgggcagctgagtaacgtactgcatcgactcataatagataccccgctcgttggtgaggccgaagacgatcagcgtaatcaagatcgttgccgccgtcgcgcacagcaccgccgacagcgtcaccagcattttcttgctccagcccataaccagcagtaaggtcacaaagcagaaaatgaccgccaaaacgctaaaaatccagataaccgcagccccgttattattgtggtcaagcttaacagctatccagaacagaatcgtgttgatcaggatgctggaaatcaccgtcacacctcgcaatttaagaatgacaaataacaggctgatggcaatcgcaaatagaaaggcaatcggtgcatcccgcttaatatctttaacagtcgcgtgtagtttaggctgagtatgtaacgtaataaagagcttttgtcccttggtatattgatggtccattgcatgcgaatctgagtaggcattcttaatgcttaatttttgaccagcatacttcccgttggtaatcgtgccgaaaagctgctgattgtggtaatgatcgacattttgaaactcatcggtcatcttgattgctttgccgttttgcacccggtctactcgataaatggtctgctggtacaggccatcattgtgctggcaaaaaaaggccgctaaaaaacaaaaggcgacgaccaggacaatctgaagccacgtcattttactcgttaatttagagttcatattgcacatcttttcagattaattttagaattattgtaacatctgtggaaatgaaagcgtggatttatttagaatcgttaggaaagcgaaagattcaccggattaaaaaagccggtgataaggacaacgccttgatcaccagctattcatcgggttattacgaaccctgttactcattattttttataatcaacaaccatcacgttaaccgttgaatgtcggacaacgtaagcagttgtggaccccaaaatcgctctggatatcccgttaaccccggactttccaatgacgatcaacgaagcgtcatacttttcgggtaattctttggcaatttgaatctttgggactccaacaacgaagtgggtttcgactttagcgcccttcttctcggcaatttctcgggcatcgtccaaaatttcttctgcccgctcacggaacgactccatcacgtcctggcccagcgtcacgccgtactgaacataacgttgatcactggcgaccgaaacaatctgcagggtggcatcaaatgacttggccaaatcagcagcttcttccaccgccctcattgcattgtcactaccatcaactggaaccaaaattgtgtcatacatctccaacacctccgaatctgactatctaagttaatcataccattgtgtgatggaataaacataaatcaagtccggataaatctactcaaagctcagatgcgaaataattgttttgttatccgccaactcggcatgccgttcttttaaccggtcatcataggtagcaagcagatatttttcttcggcagactcaccgaccaacttagggaaatggatctcactgatttcattggtgacgatcagcgtgcaaaaagccataaaggcaacctgaacgtctttggtcttggtatcggtggtcaaaaatttggtaaagacctccaccgcacgcttactgctgccggtgacataggagatgcacgttaaaatctcattgggccgggcaggtgataggaactggacatggtcatagcccgcggtcacaaatgatagatttcccggcagaaatttcaccccggccaatccggcattggcatccaaaattcgtaaggtttcgccgccaaattgaattcgattgttattcaactgggctggaaacacatagctttcatgaatcgccctggtgtctgagcacttgatcgtttcgatgataatcgcctccaaattcaacggattttcaatcacttgctaataaaatctacacattcaatgataaccttttcatgcctataatagcaagctttttaagtgttatacgaaaggattgtgaatgaaattttaaattattcagctgcttattgtaagcgatttcacataggtgtaaacttagggtgttgatggtaagaagtttttcattctaggaggtcataattatgaaagcagtacgtatttatggtgaaaaggatatcagagttgaagacgttgagattccagaaccaaaggatgatcaagttcaaattaaagttaaatattgtggaatttgcggaagtgatttgcacgcctatctcgaaggctggggcctgccaaccgttccttatccgttaaccggtaaaaacgtgccaattacgctggggcacgaattctcaggtgaaattgttaaagtcgggaaagacgttgacgacttacaagtcggtgaccacgttgccgttgaaccacttttagcttgcggcaaatgtgaaaactgtcgggcaggaaactataacttctgtaaccgtgccgtttcaactgatggcgccggcaacttcctgggcttctcagaagatggtgggatggctgaatttgccaacgttcaaggggtctttgcccacaagatgccaaaagacatggactttgaattaggtgctttggcagaaccaaccgccgttgtttacgaagctatcaagaagagtcatttgcgtgaaggccaaaacgttgctgtcatgggagccggcccaattggcttgctggaagctgttttagctaagatcgcaggtgccaaccacgtatacatcgttgatgtttctaaagttcgtttggacaaagccaaggaattaggcattgaacatgtccttgacccaagccaagacgacgttgaaaagatcatcaaacaagacttaccaaatggtgtggacattaccttcgaatgtgccggcgttcaagcaacctttgattcagcattgaaagttacgaagcgaaccggaattattcaagtagttgccctctatgcaaaaccagttaccatgaatatgactgacgacctgattatgcaaggtaaagacgttatcaccaccctctgctacaacaactcattcccgaatgtgttaggcattattgataaccacaaggatctgttcaagaaagttgtcactaagaaagttagcttggataatgcattggaagacggcattaaagctctctcaaccgataaatcacaagttaagattatgatcgatccatcactgtaagcatcaagtaagttaacgagaaagtaggaagactggtaacgatgaacatttttattcatcgttgccggtcttttctttgttagagaagttgctcattgggcttaaaaaataaccaacagatattcaatccatcggcaaaaacatatgttataatcttcatatgaaaggaatgacatatatgactgatgactccgtttcaatcaactcaatcgttcttattgataaccgacatttgtcggaatcggaacggatttttaaattactcagcaatcccaaccggctgcagatgctaaaagtcctcgcgcagcaggaactgaacgtcagtgaactgggaaatctgcttggtttggagcagtcctacgtttcccaccaattagcattattaaggaaacatcagctggtgtcatcccaccgcgaaggcaaagccaactattatcgactagatgatccccacatcctcgacgtcatcaatgagatgctcgagcatgctgatcacgttatcaggggtaaaaagcatggagagtaacactgattcacaaacactcgtcgaccgcagcctccacactgaatacttttcaacagcctggatggcgttcgaattcatggttgggttttattcaggtctcaaagccggctcaattctgttaatcgcatttgggctggacagttttttagagattatttctggaagcacgctcatttggcgactacgaaaagaaaatactggtgccggccctgaagcaatcgaacgggcagaaaagcgctcttcattaattgttggaatcgttttgctgttgctggctatttatgtcaccgccgtgtcactgtttaacctattcactcacgcaacggcagacaccagttattctggtatcgccattgggattgcctcggttttattaatgcctattttgataatccggaaacggtcactgggcaaagcgctccactcggatgccctcgtcgaagatggcatgtgcaacatcacctgtgcctacatggcagcgacagtcttaatcggcgcactgttaaccgcgctgctcaactggtggtgggctgactcagtcgccgctttgattttagtgtattttattgccagtgaaggatgggaatcgtttcaggaagggtataaaaagtaaagtccccacacaattaacgcaagtatggccaaagcatctccaattctattctcattttcatcattttgaatattacattgcggaaacgtgggacgtaaagcagtttccggccatataaacaggcaatccgaatatccaagttctggatattcggattgcctgcttatattctggaaactaaccgcttcacgtcccactctgaattacattcccataaccagccgaatcacaccaagcgagataacccccaccaccacaatcacgagcagattcttggaaatgactgctgccagcactgtcggcagtgaagcaaggaaattttcccagtcaatcgatggtaagtggccgatatgttgaacaaataaattttcaaaccataatgctgacataatcgcaattggaacaaaactcaagaattccacgacgcctttagacagctgaaactttttcagcacgacaaacggggtaattcgagacagccaagtgacgatgcccgtgccaatgattgtcagcagcacaaaattaaaagaaggcatgtttcatcaccaccccaaagctgcaggccacaagggtcaccagcaaaattaataaactgcttgggatgaagatcaagcccaagtaaattgcgaccaacacaaacccaaccacgatcagttgcaagttgaatttgattgatttgtcactaatcaattgcagatacagtaaaccaatgaacatcgctaccagggcaaagtccaagccgaatttttcaggattgctgatgaaattccctagaaccgcgccaaccaacgaagaaagaatccaagtcatgtaagaaatgacgttggcggtattgaaccaagcgaagttcagatgattgtcagaataattcagcttgttcatccctaaagcaaaactttcatccgtcagcagtgtcccaaccaaaatattcttaaacatgctgtcatgcttaaaataagaggccaaagttgtgctcatcagaatcatccgcgagttgaccaaaaaaacggaaaaaataattgaaaaaatgggactgtgggtcaccagcatgctgacaatgacgaactgtgccgacccagcatatgtaataatggacatcaacgtcaccaacagtgggcttaatcccgcggctttaccgacaatgccgaaagccacaccaattcctatgtatccaaataccgttggcaatgtatcctttgaagcggcagaaacagttaaatcaccattcatttaacacactccttctttgtttttattttatgtagctgaaaacgtgtgccaaaaggccgcttcctatgcataactacgaataactttccgagctttcagctcaaaaagccattctaggttatgctacgccggccatgaaatgccaagcctacgtggcggaagcaaaaccgccttttggcacactctgttattgcattagcaaaattttaatggtgttctaatttaaagtcaatgatatttagataagaaaatcctgaaattcagttattgagctgaacttcaggattttgttagttagccagtgctctttggtaggcatcatacgtcccagtatcaaaacacaccatcgtgacatcaagtggcgcgtcaaacgttcgaatggcgtcaatggcaatcttagcggccttatcaagtggaaagtcatagacccccgtgctaatcgagggaaaagcgaccgtttggcaatgattttcaactgcccgtttgaggctattcacatatgaatttcgcagcaattgtggttcattgttatgtccgccacgccaaattggcccgggggtgtgaatcacaaatttcgccggtaatctaaacccgggtgtgactttggcttctcctgttggacagccgttgagcttgcggcaggcctcgtcgaactctggaccagctgcgcgatggattgccccatcaacgccgccaccaccgctcaaagcggtattagcggcattcacgatcgcatcaacctgcatcgtggtaatatctcctttgatcaacttaaattgtgccatggtttcacatcactttctatgggctttttcccatgctttgatttgttccaaacgttttttgaagcggacttcattgccttgctcggtcggttcataatacgtgtggccaaccagagaatccggcattgtctgcatattagtcaacttatctttggcttcgtgagcatattgatagcccttgccataacccagcttggacatcaacgaggttggcgcattgcgcagttgcagcggcaccggctcgttaatcgagtgcttgacgtcggtttcagcacccagggtggccttataaaccgcattggacttgggggccaaggacaagtaaatcgcgcactccgtcaaatggacgttacattccggcatccccaaaaattggcaggcctgaaatacattaattgccacgttcaaggcgttagtatcagccaaaccaatgtcctcactggcaaaccggaccattcggcgggcgatatacaagggatcttcgccgccacttaacatccgcgtcagccaatatacggcggcgtccgggtcgctatttcgcattgatttatgcagcgcagaaataatgttgtagtgctcctcgccgtgtttatcgtacagaaatgacttggtattcatcaactggtggagattgtcggtcgacacggtcaccttgccatcctgcttgggactgttgttaacagccatttccaaggtgtttaaggcaactctggcatcgccattggcaaattcggcaacttctttaaccgcttgatcgtcaatctcaatcgtttcttttggaaaggctgctggatttttcagcgtctgatgaattagctgaacgatgtcatcggtctccaaaggttgcagcacgaatactttacaccgtgataacaaggcggaattgatctcaaacgatgggttttccgtcgttgccccgatcagagtaatgctgccccgctccacaaatggcaaaaaggcatcttgctgggctttattgaatcggtgaatttcatcaacgaaaacaattgtcttgccgcccatctcgcggttcgcctcggcgtctttcataatctctctgatttctttgatgccgctggtgacggcactgaaagtgacaaacttggcctgcgtttttttggcaatgatctccgccaaagttgtcttgccaacaccaggcggtccccagaaaataattgagggcaactggtcactttcaataatttctctcagaactttgcctttgccaaccagctgatgctgaccgacaaattggtccagtgtctttggccggacccggctggctaagggctgattgccgtcctggttgccggcaaataatgattcctgtttcatgaagacacctcctgacaaatgaaactgatatgtatatgcctattatacgaacacacgttctaaacgtcaactctacctttattttagcgcaatcagctttcattgaccgaatttcgcaacttatggcctggctgatcgtcttcctctctggtcacgtcaaaatcacccggattaataagacgctcaaacaacgcaatcaatcccagaacaaatcgtgaattgatgggtgataatttcccctcaacaataacaaacaggttataattaagctgaatttacgggctgtctgtttgtttttttgagggagatggcaaaatgtcatataacaataacttctatcgggagccggcattttggctgagcatctgtgcggctgccgtgggcttgatgtccctatttcttggtaatgcggtccagtacagcatcatctggtggctgcaattattgatcgtcgtcattgcactgattgggattttttatttcttttcgaaatattcaaaggatcaggacaataagaataaacatttataacactagaatcatcaaaggcgccccatctctaatcagaaatgaggcgcctttgatgatttaactatgacaaattaatccgttttcgatacttcctaaccagtccgaggcctaacaaccccagccagccaacaatcgacaaagcggtgaacaagccattgaatttaactccacggctttgaatgctgattttagcttgcttgacggtttgtggaatagtgagtttaaaggtcccccgatttgaagttgccggcttttggatggttttgccattgaatttgaccgtgtaattcatcccggcatagtggacaaatggtaagtccaatctggttccctctttcatcggcacggtcagctgataagcaagggaattgttgcctgggtgcagactggccgtggcgatttcaaaccgctgtccatttaaaatggtcaccttgttggcgagatcatcaatgtgttttccagccgtcaccggtaagtaatcggtccgcccggaaccgttatcggttgggaactgattctgataatcctggttgttcaccttgtaattttgcaggttcaggttggaacgtggaatttgatgcgttggcgttgctttgtaggttaactcaggctgactggtgcggttgaactgattatcatacgggttctgatcggtagctacgttcattgaatacatcgctgaataatcaaatgaattaatcagacaaaggcttgcaacaatcaccagtgcactgacgccaattgttctacgattgaactgggttgccaacagataactgccaaaagcggcaatgaacatcactaaaaccggaataatgcggtgcccactttgaatggcctcgattccattaagcaatggaatgtgatgaattaaattccatgggaacaagttggataacacaaacaacgttaccaaactactaaagtaggcatagcgaccaattggcggcacccgtttgatgaagaatcccccaaagatcaacaccagcaataaaatgaggccgatccctttgttggccagactctggttcagccaggtaaacaaactttgcggatctgcatacagtgtttgcggattcggtcgcatcaatttttggctcatcgccaacaccgcgatcggtccccaaacgatcaggctcaaaattaaactatagacggcggcgatgccaatcttcatcaagcgagctgcccgttctttaaccggctgcttggtgaaaaaggccaggtaaaacaccaataaggcgatgaccacaatcaacgtcgtcggtgccgtacatgatcccggtaatcccaatggtgagcaggtaccaacgattactgtcgtcaaacatcacttcgtaaagaccggcaaaggccagtgggatgaatgggtaggccagaaattcaccaaactgagtggtgataatttccatgaccaaataagtcgtcaatccatataagatggcaaaataaaatgaaattcggctggacttggaaaccaatttcatactgtaataagcaatcaccagtgtggcaaacacaaccaggacataggcaaaataaatcgcgctaatcggcgaaagtacgaaccgcagcccggcaaatatgtacagccaaatccatgggtagcaggccaccaccgcatccccaatttgattaaatgtccgggtggcaatgtggctgaatggcgctccgttttgaagattggccagcatttcctcaatccggctcaaatgaaactgtaagtccgggccggaatagacatgcattgtcagccaaaacggcaaaactgcaagcaaagatagacaaaaaaagccgaggttgatgaccagcccctgatgctggcgaaacttggaaagtaattgttgatacataaaaaatggacctcctaataaaaattagcggtcccccctgtcgctgttgtattttatgatacgagatatacggtcaaaattcaaatcttattctgacattagtgaatggtacaaaaaaacaactcttccaaattatgaaagagttgtcttaatggggaaaataacacgtgtaaaaagattaaacttaacggtcaatcgtatctgcagtcatgtggaatacgtcagaaagtgaagtggtcttgtcagcaaacttcttgttcaaaatcaactgacgaaaatcttcgactgagatattttcagtatctttgattgggaatgcctgaccggtgtatgaaccggttattaacgtgatcaccaaaccattcttgctgtccaaatgaacttggtaattctcaaagtagatcccatcatcataactaccggacaaaaacttgtgagttgcaaaatagtccgaaataaaatcattgaacttctcttttgaactcagtgcttctttaaattgtgtttgagttgcgactgtcatcgtaagactccctttctctcaaaattgtgtctaatcaaataacaacgcacatctatttttgtaaatggtctttatgaatcatctactaattttcattttagtccgtcagtcgcattgtgcaagtgaaaagctaatgaaaacgttgtcagaacgcaatttgtaacatttgcattctggcaacgtttccaattttatttattctttttcgacttttctggaaccttttccaattcagccagcgctttttccaattcggccttctctgattctggcaggtcagggtacttaagcggtaattctttcattcggcgatcaatgatgtcagaaacacaaagtctggagtaccatttatcgtctgaagggatgatgtaccaaggattggtcttgttggctgtgtgctcaatcgcatcctcataggctttctggtaatcgttgaagtaacggcgttccttaatgtcagctgaggcaaatttccaattgtgatccggcagttcaattcgccgcttgaagcgatcccgctgctcatcggcagacatgtggaggaagaacttcaagaccatgaagccgtttcgggtcaaatagtcctcaaagaaattgatatccttgaatcggccatcgaagaatttgttatccacttgatcaagcttggtgatcgagccaatcttggcattgacaatcatttccgggtgaacccgactgatcagcacatcttcgtagtacgaacggttaaaaataccgataatcccatgttccgggatgtgtcgatgaatccgccacaggtaatcatggcttaattcaattgaggttggcgacttaaagcttgtgacctcaattccctgaggattaaccccgctcaaaatgtgtctgatcatactgtccttgccagacccatccatgccttgaaagataaccaagacaccaaaatggttttgggcatacagtttcccctgcaaatcttgaagcgtcgcaatattattttcaattcgtgctttaatgtcatccttgttcaaatcttcaacggtggcggaagttggaatcttggcaatctttagatcccgatccccgttgtatcgaaaagatttctcacgatcaaaaattttcttttcgtccatagtgttgccccctaaggaatcattagtaacaactttataatagcttatcccttggaaaaataactaagagaatgtttattctccacatttatttctcatattgagtatactagattacatagaattagtttcatataacgctgttttagtgtcgcttgaaacatctatcaactctctttgaaggaggacttaatttgaatatcttaaaagcaaactcaacagctggtggccaatccgaccaaccagccgaggattcaatcgacaagtcgttattaaaggacgacctttacaaagccgttaacggccgttgggaaaagaccgccaagattccggccgaccattcgtcaacgggtggcttcatggatctcaatgacaacatcgacaaacaattaatgagtgacctcgatgacatcatcaaggaaaatcagccacacgaggcgccattctccgaattcttgaagttgtacgaactggcccgcaactataagaagcgggatgcagacggtggcgaaccactgaaaccgtatttggaaaaaatcgaaaacatcactaattttgatgatttgaacgaacttttgccggagctggttaaggaaggttacccactgccatttggcttttgggttgaacctgacatgaagaatacgcaggttaacgctttattcgcagcggttcccggcctatttcttcccgaccggacctattatgaaaacaataatccagcttacaagcaattgatgccggtcttcaccaagatggccagccaattactggtattagcggactacagcagcaatgaagcggatgaaattgtcgaatcagccaaacggtttgatgccaagattgcaccaaacgtcaaatcggctgaggaatctgccgattacagcaagatgtacaatcctcagaagtttgcctacttctcagaatcaagttctcatctcgattttgtcaatctggccgacgcgttgtttggcaaggcaccggagcagatcatcgtgaccgaaccgaagttttacgagcgctttgacggtctggttaacagtgacaccttcaaagacatgaagaactggatgctggtcaatatggtccgttcagcatccggctatctatcagaagaattccgtcagaccggttctgtcttcagccgtgcgctatccggtaagaaggaagcaacgccacagaagaaatcagccttctatctggcagaaggaacatttggccaaacaattggtgactattacgccaagaaatactttggcccgaaagccaaagctgacgttgaacacatggttaaaaacatgatcaacgtctacaagaaccgtttaagcaataacacctggctgggcaaagacacccgcgagaaagccattttgaaactggacaaactcgaactccaagtcggttatcctgaccacatcgatgaattggaatacaaattcaaagtgacccctgaaaatgaaggtgggaccctatttgacaacatgtccaagtttggtgcgattaccgtccaagacacctttgagaaattgggtaagccggtcgaccgaacaaaatgggaaatgagcgccgcaaccgtcaacgcttactacgaaccatttaagaacatcatcgtctttccagccgcaatcctccaagcaccgttctacagcttgaagcagacttccagccagaactatggtggaattggcgcagtcatcgcgcatgaaatttcgcacgcatttgataacaatggttctctgttcgatgaattaggtaatttgaataattggtggacgaaagaggaccatgaatacttctccaagctggccgacaagatgatcaaggaattcgatggcattccatttgcgggtggtaaggtaaatgggaagctgacggtttccgaaaacatcgccgatgccggtggtctgagctgtgccaatgaagcggccaagaatgaggccgactacaacttgtatgacttcttcatcaactgggctaaagtatggcggatgaaggccacggaacagtacaagcagctgctgttaaatatcgacgtacatgccccagctgaattgcgggccaatgttcaagtgaagaatttggatgatttctatacaacttttgatgttaaagacggcgatggaatgtatcttgaacctgataagagagtgaaaatttggtaggaagcagacctattgaaacgctttttatccaaataataatcgaataaacacaaaatggcacctaacctcaaaaaaagtttagtgccattttttatttttactatttgctattagaagtgatcaataaccagccaaaagtagcctttgccggcccttaggcaaaaaacacgcttcttaggttcttaagtgctcccttcagcctctcaaatgtgttccgacgggcctgaccctaaacccagccctcagccaaaaaacacgtttattagattcttaggtgctcccttcggcctttaaaatacgctccgacgggccaaaggctaacttctaagcgcactttaattaaagttccaaacccaggaacttcaatcaaagtacccttagaaaccgcatctcccggccctcgtcacactcttattttttgccccgcatacaccgccgcaccgaccattcctgcttcatcgcccagctgcgccatctccagcttgcaggcttcacgggccaccggcagtgaatgatgcgccaaggtttcgcgggtatatttgaacaatggctctccggcagccgagacaccgccacccaggattaacgtttccggattaaacaaattaatcacgttgcccaaaccaaatcccagcaactcgccagtttctttaaagacttcaatagctgttggatctccttttgccaccgcttccgagatcaatttggtggtcagttcctgcccttgtgacatccattcgccaaccaagctggtttcgccgtcagccagtttttcctgcatggttttgacgatcccgcgagcggaaacataccgtcccagacagccggtactgccgcaagcacatggccggccgtggcggtacatgttcttgtggccgatctcaccgacactattggaagcgccatataacacttggccgttaatcagaacagctgcgcccagcccagtaccaatcgtgaccaggacaacgtttcgatgacctcttccggccccgaacgccatttcgccgtacagattaactcggacatcgttgtcaatgaagaccggttggcccagcttctcatgcagccactcggcgaccgggacatccttccagtcggtaaaattcggtgaaaaaatcgaaatccccttttccacatccatttgcccgggaatgccaaagccggcagccaaaatatcatctgaggtaatcttttcctgagccattaattgctggcagcacgcccagatccgcttcagtacttcagtgggaccggcctcttcatgagtcggcttatgtaatttttggaccgtttgaaaatcctcatcgaacagtccggccttaatgttggtcccgccaagatcaacacccaaataatattttgtcatatcgtccacctcacaacagcgatcaattcaatcaaaaaacgcttacttactatgataataaccgattagactgcataaagcttccaaaaacattccaatcaccatcagatacatgacgaccatattcatgcccagataaagcagaatgcccatcaccaaatacaacagtacaaagaaccaacgtaaccaaatattattaaccatttcgatcccctccagatccattttaactcttacattagaatctttacaatctgtgaacaaataatttgtaaaaacgcggttttaatgtaaactaatgattattaggatataatatatgtaaagagtaattggagaggtgataccatgaacttaacagaatatcttcattcgcagctcaagtttttaaatgaccagatgagttccgctaagaaagataaagacgaaacgatgcaatatctggtagattcaaagattacagaagtcaaattaatcttggaagccctccaaaagggaatcatcgatggaataagttaaaatgtggccgattggccattttttatgttttaatagactagtgcgtaataaagattgattaaaaaaggaagtagaatattgattacattaaaatcaccacgagagattgagaagatggctgaatcaggtgctgttctggccggcgttcataaggaacttcgcaagatgattaagcccggtttggacacatgggacattgagttgtttgcccgccgctatatcaaagatcacgacgcctacccttcagaaatgggctttgacggctacaaatttgcgacatgtatttccattaacgatgaagtcgctcatggaattccccgtaaaggcttgaagttaaagaacggcgacatcctcaaagttgatatgtgtgtcaacaaggatggcttcgaaagtgattcttgctggacttatgctgtcggtgacgtcagcgatgacatcaaaaaattaatggaagttactcgcaaaggcttgtaccttggcattgaccaagctgttattggtaaccgtcttggtgacattggaaatgccattcaaacttacgtggaagaccaaaaccacatgggcgatgtccgtgaactgattggccacggcattcagccctccattcatgaagaacccaacgttcccgcatatggtgtcccaggccaaggccttcgtttgaaggaaggtatgacgatcaccatcgaaccgatggttaacaccggtacttgggaaattgccgaccgttacgacaagaaggatgactggacatactacgtttcagccgatggaactccttcagctcaatatgagcataccttggccattaccaaggatggtccaaagattttaacttcccaggatccagacattgacgcaaaatatctgctttaatttaaatcatcaacaaacggccgggacatttgttccggtcgtttgtttagatttgagaaccgcccctccaagcggactcctaaccgcttggatccgctcacttttacaggacagctcctccaagcaggagtctccttgtaagcacctcgcaagcaaatcccgaaaaaacgggaatttacttccgaggagacttacaatccgactcctaaccgcttggatccgctcacttttacaggaaggaatgattacatgaacaataagaactttaaatttcctgacactgctgcctacgaatttgttattcaagcactcaaagaccgcggggtgacctatgaagacatcgccgagatggcctataatcttcaaaagaaatttgtccccaacattcaaatggacgaagtcaaaaaagacaccatcgacgtgctccacaaacgagaggttctcaataacgccatggtcggcctggagctggatcgattggcaactgaaggcaaaatcaaagaaccccttgaaagcatcatcatgaatgattccggcgtttttggcgttgacgaaggtattgccttaaacattgccaacatctacggcacgattggaattaccaattatggctttgttgaccgggaaaaaactggcgtcacaaaaaaattggatgaagccaaagacggcacatccaatacgtttattgatgatattgtcggcgcgattgccagtgcggtctcagcgaagatcgcccaccggaacaactaacgccaaccatgtgatttttgatcataatcccgctttttaataccggaaacatagggattgcccttaacaaaataccgcagtggcttggtcgcccaagtcccttgattcgcaaccccgattcgattagattcttcaatctgaatggggatttttttgtcatcttgatgaatatttaacttgctgttaccaaagatttgcatattcatatctttatcggcaatcccaaaggcttccatcaatttccccggaccattggtgagctcaacgccatgccgggtacggttctgttccataacggctaacccaattgttggctcaattgcccggatcaaaatcccctgggggacatcttttgcttgagccgcaacatccaagaggtatcgcccatgaatcgaatagatgtacactgttcccggaggcccgtaaagcggttcgttggaagctgtccgccggcccttaaaagcatgggcagccgaatccttttgtcccatataggcttcggtttcaacaattcggccacccaccagacctttgggggaatcataggttaaaagcatccccaacaatttcttggagatttcgtcggtggtgccgttagaataaaatgggtcttggtccaaatcaaccatccctttcaacaaatggaggttatcacatgcaattaaaattagaacgaatttacgataagccgcaggatctttccggctaccgagtcctcgtcgaccgcctatggcctcgagggatttccaaagtcaatgccaagctggatgaatgggaaaaagaaatcgccccatccaaagagctgcgcacctggttttcacatgacccagaaaaatttcccgattttaaggaaaaatacgtcgctgaacttgacgccaacccacagaccaaagaattcctcaaactaattggtgatcagctcaagaatggcaatgtgatcctgctttatggtgccaaagatcgtgagcacaatcaagcagtcgtcttgaaacaatacttaaccgatcacttaggccagctttgacgaatattggccagggtcaattctttagtggactcaaagttaatatcggccattgttagaacttccggatcaccaacaccaattgagaccacgttagcagcgttaatcgactcgacgccgacaatcccgtcatcgatgccaatacattgatcaacgttcaggtggagcatctcagcggcctttaaatacacatcgggtgccggcttgttatgcttgatgtcggccaaattcacaatcaatggaaagtaatcttccaattcaagtttgtggatctctttaggcgcattagccgaggccgaagcaataatcatctggtagtggttcaaccggagctcagctagaaagtcgcgaatccccggtaagatatcatctggattcatgatctcaagcatttgctgataaatggcgttcttcttgtcagcaagtgcttctttttgctggtcagaatatttgccaaccaacccgccgacacgtaaaatctcgtttaacgaatcgatccgatcacggcccttgatcgcctcttccaggtcttgattccactgcacaccaatctcttcggcaatctgacgccaagattggctatggtaccgccaggaatcggtaatgatgccgttgagatcaaacaacacccctttgatattagtaaaatcagtcatttcaaacaccctttcttacaaaaaaagactgaaaacaagattgtgttttcagccccagcggcagcttgaattatttaacagcgttaaagatccaagtgatgccatacttgtcaacaatctggccgtatttgttgccagaagttttcttttcaaaagttacgattactttgacttcttctgattccaccactcgctcgtacaaatcctgcaacgaggaaagggcatcggaatcatgcagatcaacttcaaacatcagcgaaatcatcgaggaaatcaccggcttacctaaaaaactgtccgcacaaaaaatctgcttgcctaaaatgttgaaactggcttgcatcgtaaggtcgtcgagattgacatcgtcattaagcgacatgtcttgcgcctgcttttcagttggggattcacgttgaacatccgtggcaccaaaaacagtttgataataatccaaagcttctttggtgttttcgaacgtcaaatatggaattaaattaatattactcattaggtcagcaacccttacattttaatattattcaaagtttagaatacctttaaatacaatagttgtcaacgtcaaccgtctgccaatgcctattctgataggaaatggcgtcctttttggtaataatttttggaaaagtgatagacttaaattaaacggatcgggaggaactatttaatgaaacttgcaatcacaatttttgtattaaacgcgttatacatttcgattaataccttcagaacaatgctggttgtgaaaggccaccaatttttagcccccatcgtggccgtcggcgaagagtttgtctacgtgatggcgttagcgatcgctttgcagcatattgacagtccgttaaacatcgccgcatatgcggttgggttcggtgttggtatctacattggaattgtcatcgaagacaagatcgccttggggtacgtcaactttgaggtaaccgtccagattgacccgacaaatccgattcatgcccacaatgaagagttggccgaaaagttgcggaatctcggttacggtgttacggtcagccgtgctgaaggccgctcaggagcccgcctggttctcagcattctggctcccagaaaagccgaccgtcgtttgatggaacaaatcaaggaaatctcacctgacgctttcgtcatggttcaagaaccggttcaattatccggtggcttctggagtaaagaagttgaccggcgttatcattcaaccaatcatatgcactaatcgtcatcttcatcgaataagccgagctgtttgagactatttttaatatcttgaactgaagttggcgtcgttggtgccgcttttcgatgaatgggctttggctgccttggagttggctgttgtttggtcggttgaggtttaggaattggctgtggatccggcttatccggggtaacggcggggctggcctgcggatccagctgacccatttgatccatggtttggtttaacaggtggtcgacaaaaacatttccctcatcgcctgcgtgccccttggtccaataataccgaatgatcgggaaatctctcagattggcatcaactgcttgccaaagctgcttgttatgcagcttcgagccgtcgctcttgttccagccgcggcgtcgccaaccagccagccaacctttttgaatcgcatccaaaacatactgggaatccatgactacaccaatccgctcattttgcagaccctggcgtttcaaatacttcagggcctccaagaaggccattatttccattcgattattcgtagcaccaaattcgccaccggattcgaaatatttttgactaccagtttgaactaaaaatgcccaggctgctttatcgctggcttttacgtggccgccacgatggttgccgtggttgcgagaaccgccgtcggtgtagacgataatatcaccgtccggttggactgagcggcgacccgtcgaagcctttttgtgagatttgtggtgtggctgagtgggcggcgttgtttttttcgccccgttgagataggcattggcttcggcttcggtcttaaaacttttatattgggcaccggaaaatcctttaaccttcttttcggcctcgtcccaactggtaaagatgccggtctttcgaccttttttaactgcgtaatatttcatgaaaatcatggctcctcaatgtaaaaatttcagaaaaaatgttaattattaattataatgtttctatctactttgcaattagataaatctatgcgaaaatgttaataaaagggggcaaatttaatatgacccaaactaaagccacattgatctcggtcattgaagccaaagcacttctaaaagaccagtcagatcaaataaacgagcgttttccccgattaaaaaaacaaggtaagtatattctacctgattatcggttaacaagaaaacgtgaagctttcaagattcgaaagcatacatttttacagcaccacgcacgttcctacgttgcatttgattccgagaacggacagacgctttggatgcacaactttccaagcttgactgaagccttgttttggttggataccggtcttaaacctaccgataccgacactaacacatcgtataagtcatggaaagatctgcacgaagatgacattaacgccctcaaagacattttgaaggaacgttctcgtaaacgcaaggaagcggcggctgccaaaaaagctgcctcggttcccaaaaagaaaccggcagctgtcaaaaagttgacagtagttaagaaaaagaaagctaactaattcgttattcgatcctaaaaaaggtatgactgtgaataaaagatcattttgttcacggtcatgcctttttattgtccatttagttattgataatgaccagcaatgtcgtctggactaaaatccttagtgaattgacgatcataagccttttcataggcagcaactttttgttggtaatcaatttggcgcatcttttcagcagcttcgcgctgtgatgtggccgacttttcaaccgcatccggataaatcggcggtaacacatggaccgtatagttgatgccatgcggatccgatttggtcggggcgtcaaccatcgaaacaaagcaggacacgattggcacattcaatctaacggcgtagtagtatgctccccgctcaagcggccgcggtttgcgatagttgaaccacatttcccgttccggataaattagaattgattgtttgcgtgccaagctactttgcaaaagggcaataaaccccttgcccatgtaattgacgctgtcgctgacaggtatcgtatcagcgtatgtcatcaaaaatcccagcatcccgggcattttaaggttggtgagctcaacgacaatcgacaaatcaggttgattcagggctgatcgaaccagcaggctgtcaatcgggctaaagtggttacaggtaatgattgccggccattctaaagcctttaaattgtcagttccctcaacttttaaattgggattcatcatcctcgcagccatattcatgaccgaccgggcttcagctgcccgccaatggtaacgtttagttttgtgaagcttcaagaagtggtccaacacctcatgctgctcggtgagtgtcagcaccggatcatgtagttcgactttttgattaaattttccctgacggacgttttcagcaatgttttgaatcactttatcacgctcgccaagctttaccggtgtaaaagtcatagggcaatttttactccttgcttggcccttgcgtaaaatgtcgttggggtcttaataatatcaacggctaattgaatcaaatcggactgattcttctgatcacgggcaacttctttaggattcatatctgcgagctgctgttttaacatggtctcgtaatcggtttgtttggcataggtccaaaaatagctttgtcgaggggcatcatcatagcgccacggcttggcgaataagttatagtgaatcaaccaaggttcaacatcctgtggcgtagtgatttggatgttccatgacgggttcaaataataaattcgatttctcgcgatggcattcatgtagtcctgatccggggccaaactcttgaaatggtacttgttcaagagctgcaaaaagtgttcagcgaattttgaacggcgcatttcggcgaggttcatcaacaacacgccggaattaacgtatttctgtgaatcaatcccaacggcttgttcagcatagtcaatcgtttccggagtgtggccgatgaagtgatccggcactgcgccaaccaagttatcacccagctgggtatcaaataactcacccacatcctttaaaaccaccgtgtctgcatccagatagagtgccttatccaatttggggaacaattcagcaataaacagccggaaataaattgtaaaggtaaagtaatcgctgcgaagtttgttattcttatcggtaatttcttgcttcaagcggtcgttaattgaaacaaactgaattttgaggttgtccgtttcaaaggctttaagccgcccttgattatcgctattgagattatcacacaacacaatcacctggtaatacctgtccggtgatgtatgcgcgaccagtgaagccagtgaaactgccaaataaggtgcataattgtcatcgacagcgtaaaaaattggcacagtttgatttcccataatgaatcccccttaaatcaatgtgattgatgctggtaggtcataaatgacacgttgctttggtgactgcgggtcaccatttgggcatgaatctgatcatggagcttttgttggcgttgcttgcgcggaagtgacttgtccggcataaacggaccgtcaaagtataccacctgcttgggtcggctaaacagtcggcctttttgatatgtaatcgtcatgctgtaactgggcagatcggcagcgaccggataatggaaagcgccgactggaaacggacgaatcttggtgtaatacggccaaacatgggcttcgggatagataaacacccgttgatgctggtccaatcgagcattcatcgctcgctgaaattgaatcatttgtgataattttgcgggtaggatcaatgccccacccatcgtcaagagacggccgacgatgggaataccaaggttggcaggttccgcgatcggatacgcccgcctgggtactgccaccagcatcggcaaaagcgcatcccccagcggctgggtatgattggcataaatgaaggcgccccgtttgccttgggtgcgcagacaccgtttgttccgaaaagacgtccgcaaatacaggcgacaataaacgaagctgacaacaaccgccacccagtagacgaccgtcgccgttacgcggtaaaaccaattttgatgcagccaaatgtagccctcaggaatggtggcattttgattcttggtaaagaccacgtcatcatcaaaatcatgatacgtaaacacttttgatgcccgtttagtcattgccaatgtcaccctttcttccaacaagttaaaatcatgaacagaaccattctaccccaaatatgacattattttatcatacgggacgtttaaaaatggcaattcactaaaaatcgtcctttaaatgatgaaattggtgtaaaattaaggcttgctatgctaggatatttgggataacaatggatgtatacacatcattagaaggatttaggggataattttgatgcaagctcagtccaagaacaataccaagtttaactttaaaacatttataggcctaatcaaccgaattcacccccgttactggcaactgctgcttggtttttttctaggggttgtcgcaacggcgatgcaattgatggttcccggcatcgccaaggggatcatcaactcaatcggtcattcaatggatgtcggcctaattgttgccgtcattttactattcgttttcagtaccattatcggagccttttccggtagtattttaggcttcttcggtgaagacgtcgtctataagctgcgaacgacgctgtgggataagattttaaccctgccggtgggttattttgaccaaacccaatctggcgaaataacctccaggttggttaatgattccacacaggtcaaggaactgctggccaattcggttcccaaaaccgcaacttcgattctgcaattggttggcgcattggtcttaatgctcatcatggactggcggatgactatcattatgtttatcgccgttccactcgtcttgatctgcctgctgccaattgtccgccaatcccacaaagttgccagagcgagacaggacgcactggcagatctcaatggtaaagctggcgaaatgctgggcgaagtccgtctggttaaatcgtctacggcggaaaacttagaacgaacagccggcgacaaacggatgtatcgactttatcgcatcggactaaaagaagcgatctatgattcgattgccggacctgtcatgggcatggtcatgatggccatggtcctgggaattctgggctatggtgcgatccgggttcgggaaggtgccattgatattgggaccttattttcatttctgatgtacctggttcaaatgattagtccatttgcggttctcggccaattcatgtctgatgttgccaaggcaagtggctcaaccactcgaatccaggcattattgcaaacccatgaagaagatcatctgattggaacggatttggatattggcgatcaaacacttcagatgaaccacgtcagtttttcttatgatcagcatcaccccattttatctgacgtgtcgtttacggcagaacccaattcggtcattgcctttgccggtccatccggcggtggcaaatcaaccattttcagcttaattgaacgcttttatgaacctaacgagggcagcatcacgatcggcaataccaatattactgatattcaacttgccgattggcgccagcaaatcggcctggtcggccaagacgctgcgatcatgtctggaacgattcgttacaatttaacctatggtttgccgggacatttttccgatgatcagctttggcatgtcttggaaatggcttacgcaacgcaatttgtccaaaagatgccccagggcttggacacggaagtcggtgagcgtggcgtcaagggatcgggtggccaacgtcaacgattggcgattgcccgggccttcctgcgtaatccaaaaatcttaatgttggatgaagcaacggcgagcctggattccgagtccgaaatgatggtccaaaaagcgctggaccaattgatggccaatcgaacaacattggtgatcgcccacaggctaagcacaattaccaacgccgacgaaatttatttcatagaaaacggtaaggtaacgggccagggaacccaccagcagttggtgaaaacaactcctttgtatagggagtatgtgaacaatcagagcgcgacaagacccggttagggaccggagtacaaagagaatcaggccatgatgaacgttccttgttcatcgtggcctgattctttttgtacagtaggttcctgggtcgtcggagcgtattttaaaagctgaaggattctcaaaagagcataatcacaccacagcgcgacaagcaacgggtgaggcggtttctaagggtactttgattgaagtccctgggtttgggactttaattaaagtgcacttagaagttagcctcagttgcgtcggagcgtattttaaaggccggagggagctcaaaagagcataaccgcaccactgcgcgacaagacccggttaggacccaccaagtaggctaggccgttttcatccggccgtcggaacataagtgagaaaaatcaatgatgaacggtctttgttcatcgttgattttttttcgcttatgtggctgggtcctgggtcgtcggagcgtatttcaaaagcggcaggaatctcaaaatcccctaaccacgccaaccaattgataacacttccaccccctgcgcaccaatccaatcaagacaaaatataaaaagagccaatcattccaaaaacaggaataatcagctcgttcattaaaattctaagagcaacgcatctcgcatcgcaccctcactcagttttcaattccccttcagcatccaattcagccataatctcctgatactcggctaaaatatcatcatattcatgcaaatgaagttgctgatgcactttatcaacttcccaaggcttgaccgaaaccgtgtggacgatcggccataatttccaccgggtggagaaatgctgaaaaacggtgtcagattgaacatcctgctgctcattatatttttcaggggcaaaagccttgtgcttagccagcttattcattgcggactggtccggcataatcatcggccattttcgacagtactcccggcagcgggccagcaatttgtcttggcggatcatgtccagattcatcaggagcatccccgagttgatgtaatcaaatgctctaagttgatgatggaagaaccaacggccgtaatgatccaagacaccaacaaaatcagttccagccagtgattgatgataaaaatcttcaaacggccggcgacacacaacgtcagcgtccaaatacagaattcggtctgaaaattgcggcaccaaatcactatacagccgcaacatgctatagggcgtgaataacgtgttgatgttagccttgggcaaatccgcctcaaactgagcggtaatgtcaattttggtaacgccgctatcgacatcttcccgcttcaccagttgatccaaaaaggctgcgtgatcgtcagtcagcgcttgaaattgctgatgtcgattatacaattgtccagtcaaaatgtagatgttgagtggttcttgcgcgtgttttgtcagtgagaggattgaaataatcaaccccgaaaacatgtggtcgtctccacagtataaaatatccaaaccgcattcatcccccaattcgtgtctcatcaatcaaagtgtgtcatacttcctgataaatggcaactaatgaccttggaaattccccacaattcaaaaagagcacccagccgacgcagcaatgtgtgtcaaaaggctgagtgcttttaaattaatcttcgaaatagtttttgacctgtttgggctcagtttgaaccaagatcttaccattatgaatggagtagagaatttctgagcgttcatttaaggcgttgtagaaattatcattattcagaatgatacaattagccggtttaccgacctggatcccgtagtggccagtgatatgcatcgccttggcaccgttggtcgtaataaactggtaggaattcataatatcgtcgtaccccatcaaatgaccaacgtgaatccccatttcaactgggtcgagcatgttaccattgcccattggataccaaggatccttgatgtcgtcttcaccaaaggcaacgttgatgccatcctcagataactctttaacccgagtcatcccccgccgctttgggtaggtatcaaagcggccgccaaggttagtattaactaacggattggcaatgaaattgatgtgagacattttcaggaggcggaacaacttgtaagtataggcgtcgttatacgatcccatggcagtggtgtggctggcggtaactttgtcacccatgccgctttcaagtgccaaagttgccaagacttccaggtttcgtgaagccgggtcgtcaatctcatcgcaatgaacgtcgaccagtttgcccttgctttcggcaactttcatcaagaatttgagtgactcaacgccgtagtcgcgggtaaattcaaagtggggaatcccgccaatcacgtcggctcccatgtcggcagcggcaatcatcaattccttgccatttggataggataaaatgccttcttggggaaaggccaccagctggagttccacttgatcggcaacctcgtcacggacctcaattaaagcctttaaagccgtcaaatcgggatcggtcacgtcaacatggctgcggacaaattgaatcccgttggcaacctgaatcttaagagctttttttgctcgcgtcttgacatcatcaatcgtcagctttttctttcgctcactccaaattcgaatgccatcaaataaggtgccggattgattccattcaggatcaccggccgtttgggttgcatccaaatgaacatggggatccacaaacggcggcaacaacagcttgtcggtggcgtcaatcacctgttcaccgtcgccgggttgaattgaggcggcaattttgacgaacttgccatcctcaattttgacatctctggtttcttcagcgttttcaatatggacattttttatcagcatcagattatccctcacaatcaagtatttaataacattatagtctattttaacgccggagttgggcgcaatcggtggaatgtgcgataatacagatgacatcattattagaaattggcatttctgccaagtgaaaggtactgattctttgaacttaaaaaccaggttggcactcccgcagattttaacattgggatttctcatcatcattctggtgggaacttttctgctatcgctgccaattgccagcaaatccggtcacatgaccggctacattaacgctttctttacggcaacttcggccacctgcgtcactgggatgaccgtcgtcaataccgcgcttcattggagcgttttcggcaaaattgtcatcttgatgctcgtggaaatcggtggtctgggattcatgacctttgcggttctcctgtttgttttcatgcgccgaaaagttgatctgacaacccggttgttgacccagcaatcgctaaacctgcagtcatttgccaataccagttcggttgtgtttttggtggtccggatttctttggcgattcaagtgttgggaacggcactgatttttatcgatttttatccccggtacgggtttgccaaaggcttgggttacagcatttttcattcaatcagcgccttttgtaacgccgggtttgacttgtacgataacagtttggaacaatttcagaccgatccatacctgctctttgtcttgacgattttgattatttcgggctcactgggctttctagtctggaaggatatccttttctacaaagaagatcatcatttaagtctacataccaaattagcgttgacgacttatctgggactgatcggtctcagttttgtggtgtatatgctgacggaaggcaacttcggccaggaaagtcatttgaccatgttccagcgaatcatgaatacctggtttttggcggtcactccgcgaacggccggcttttacaccttgccggtcacccatatcacaatgggtgggatgttctttaccatgattttgatgctgattggcggaacccccggatcaactgccggtggtatcaaaacaaccacggtcggcatcctactgatcagagtgtggtcaacactacgcggcaaacgggacgcaactttttggggccgacggttcagtaacgacaacgttacccgttcattgtcactggtcttcttggtggcagtggtcttgtcgatagcaacgatgattctaacatttacggaaacgatcccgaaaactcagggattggaatacatcacatttgacgtcatctcggcattcggtaccaccggctttagcctgggcctggtggcgcacctgagtgtcgtcggtaaattaatttttgcggcgctgatgttcatgggcagagtgggtatctttacggtaatgtattcactgctcaactcaaagcgcccggaagatgctttccggtatccggaggagaatgtgatgattgggtaagagtgcggactagggcggttagcaaccgtagtctaaggtacttccaacggaaatcgagtttgattttcgttggaagtatcttaggcgcaggttgctgccctagggagcacgcctccactaggtaaaataaaagcactaacacctctaagtgcaatgagtgttatgaatcatattttcaagctaaacactattaaaaattaacccaacaaccaaaaggagcaaaacaatgaaacaaaactacgcagtcatcggcctaggcctcttcggttccagtatcgtcaacaccttgctggaacacgaccaggaggttctggtcattgataaaagtgaagctcgggtcaacgaatttcgtgaccgggcaaccgaagcaatcgtagccgatacgcaaaatgagttagccttaaaccaactgggcatcgggaactttgacaacgtctttgtcgccattggaaccgatctggaagccagtatcatgaccaccatgatttgtgaagaattaggcgtgaagaacctgatctgtaaggctgaaaatgcccgccatgcaaaagtcctggaaaaattaggtgctgatgaagtcatccagccggaacgagacatgggtcagcggattgccctgcacgtcatggagcctaagattctcaatgatttgaagctaaagggtgaattgtcggtgattgaatttgaactgaccaatccaaaactctttaacaagacgctcaaggaactcaacttaaccaatcgctacaaaatttctgtcatcgccctttcccacgcggacgagaacggtgcaattatcccgaatcaatcaacgattaccaaacccggtgacattgtcacgattattggaaccgagaaagatgtcgaagcatttgaagccgtggccacggcataaaaatagagtcagacagcttggttagctgactgactcctatttagtgtgtatcatgatgttaaacaaatacaaaaaattacttagcaggcttttgcttcaagaaatgttgcaagtctgataattctttgtttcgcttaatatcttttttacggttaactggacgacgtccttgtacgccgtgtggatgacaaattcgcataattagactctccttattttgtattatgatttcataattccaatagactaaattattataatacaagtttaggttggaacgcaaatcaatctgcggtttctctatgatttctaatgaaatgtggtattcttaataattaaatgaacagttgaggtgattaatttgacagaacaatatccacaggcactgacaattgcgggctctgacagcgatggcagtgccggcatgcaggctgatttacatacattttttagacggcacatctacggaacggccgttatgaccgccgcggtggcaggaaatagttacgggattcatgattcggtaaccctgccgacatcttttattgaccaggaatttaaagatttggccgacgattaccatgttcgggcaagcaaaaccgggatgctggccgacacagagttgattcgcaccgtcatcaagaactatcaaaaatacgatttcggcccattggtggttgatccggtgattaccaccaagcatggtaacatgctcttggaacaaagcgcctaccagacgcttcgcgatgagctgatcccgctggcaaccgtcatcactcccaacttctttgaagcccaaaaattggctgaaatggacatcgacactcaggatgacatggtcactgcagcccagaaactaaaggatctgggtgccgccaacatcatgatcaaaggcagccaccacaaacccggccaaaaagaagtgtccgattatgtcctcctcgaatccgggaaaagtttctggctgactggtgacttcttcgatactgaccgtaaaaacgggaccggcgacagtttgtccgcatgtatcgctgccgaattagcccgtggtaacgacgtcgaaactgctgttcgcattgctaaaaagtttgttgacgtggcaattgaaaataagatccaagttggccacaaatttgggccgattaaccactgggcaccgggatatcccgatcctgaacaatcaaacaattcctaatagcgacctccattatcggataggtcgcatcataaccagatcggcagaaaggcctgggcaaaactaacgattttgctcaggcctttttactatcttaatattacctagccgaatagtgggaagctaagcacttgttttaccacactgttctgttacccaatatgtctttcaaactttttgaatccaaataacttgtcgattcggccaaagtattcttctgggatttccaaatcaaccgccttcaaattattttcaagttggctgggcttgctggcaccagtaatcaagctactgattcgtggatcacgcattgtccaagctaaagcgaaggtcgccaaatcagtgtccaactcatttgccatcttaatcagttcttcaaccttatctaaattgtcatccgttaacagcgcttggatttgatcttgataagttgctcgtgatccggctggaatcttgtggcccttacgatacttgccagtcagcaacccttgggaaagcggcgaaaatgggacgatccccaagccaagtttttcgcagacatccatcagttcatgctcaatgtagcgatcaaacatgttatattgcggctgaaccacagacatcgggtgcaagcccaacttttgaatcactaattgtgcttccaaaatttgtattgggcgccactcactgacaccgtaatagagaatcttgccttggtcgacgagatcactcaaagcagttaaagtttctgccaatggtgtgttgggatcaaatcggtggcagaagtacagatccaggtaatcagtctggagattcgtcaacgactgatcaatcgattccataatatgtttgcgcgaaagcccacggtcgttgactccgggacctgtcggaaagtaaaccttacttgaaagaacgatttcttttcgtggaaattctttgagtgccttgcctaaaaaccgttcggctgccccaccactgtatgcgtcagcgcaatcaaaaaagttgatgcctttgctataagccagtttcaaactctgatcggccaaatcctgcttggctgaatcactcacgtcggtcatccagctgcctaaagccaattcactgactttgaggccttgtttacctaaattgcggtatttcattttgtttcctctcctcattttgatttgttagtttatatcttgagtttagcgcttcgagtgtacttgaagtaaaggacatttagtcaaaaaaatcgttttgggcgctgttactttgctgagttgtgctacccaggcaggcctggtcctgtaacttcgggggttgtttgactgttatctttagggattttcactgttactttgttgaattgtgctacgcaggccagactcctccgcttagataaataggaccctttgatgcaagaccagcatcaaagggtcctattcacctaatgctcggagtctaaccggcctggtgcgcacactgttttttgcaccgcgatcaacccgagtcttgtcgcacactaatccctgaacaactccatattctgcaaataagtcatctcatcagtcgaaatccgcgtttgcagcttttctgccaaagcggcatcaatttttccggtcgtcaaagagttttgaatcagctcatactcgctatggaacgcccgcatgaacatctggtagacaatgtccatatcaacatcctggccattaattcgccgatgcctggttcgatagaatcgcttgaccatgttggtctcgacaccattttcgccctgcttggtcttcaaaaagtccatgaccgcgttaaatccggcttcctcaattgggaggatattttcaccatgcttttcaaattgctcgcgccaatagacttcttccaaagccactggagcggttaaaaacgcctcttgagcacggttcagatccttatacagtctaccaacatgcagactaaacctaattctcaataagacatttttccaaatcttctcatccgcagaaaaattattcaagttcaaaaattttgtataatacgtcagctcatcctgagaaattttaccgtcatcaaacatcttctgaacggtcttcagctccacttggtggctctcactcatcaactgcctacgcaaatggaaattcggcgtgctgtccaagaccaactgctgctgaagcgaatcaatgaccacctgtgcctcggctgggtgctccttttctttcagcaggtcactaattgcggcttgaatcatccgtttaacccaacgataccgaggctgctgccgatcttgactcggtaaaatgattggaacaaaaatcgtcggcataataagactggttaagataaccaccgcagcgacaaaaatcatgatgccccggaactcaaacggctggccattaaccgtgttaggcatcgagaaagccagtgagagggtaattgtcccgttcgctccgctaagtgccatgacgaggctgtcacgccactcatggttcgatttaacacgacgcttgagcatatatctgctccaaaccagtctcaaggttccttttaccgcataaacgccaatcccaatcagaattaacttcaaaatattcagatcaggatttggagattggtgaagtgcctgaataacttccggcaacgacaggcccagcagcacgaacacaatcccggataatgctccggaaacgacttcccagacgttgctggtaaccagctgcatccgcgatgaagttaaccgtaatttgtcacgttcagatccctgaaccagcccggcggcgacaaccgccaagatgcctgacaatgctaatttttctgccagcaaatacactaaaaatggagacatcaattggatcaacaccatgataatcggcgtatcgtcgttataacgaatcaaaaacagccgggcactgacaatcgcaactccgatcaggctcccaaataacaagccgcctaaaaattcccagagaaacatcgcaacggccagttttaacgaaaaggtccccgagacaaaggcagtcagcgacaagtcaaacagcacaatgccggccgcgtcgttaaacagcgactcgtgctgcaagatccctgcctgctcttcagcaatcggattggcctcaaaaatcgaattaaccgctgaagcatcagttggcgtgacaatcgccagcaatgcaaagcatagcgttagcggcaggatggtcatgacggcgtgtaggcctgagccgaccaccaaaacggtgaccagtaccagcccaactgccagcgacaaaatgttggtgatcgaccggccaatccaaaaccgtgaactgttttgagcctcattaaacagcatcggcgcgataattgccaaggcaaacgtcgacgggtccaaatggaaattgcggtataccggcagaaccgccagcagaatccccagcaaaatcaggaaaaatggcagcggaataaacgagacgtgtcgcgcgagaatattagcaaatacgaccgcagccaaaatgatggtcagtagtagtaccatgtccattacattcacccctccgcttcaatatcgattctagtttatcactgattggacaaaaaaagccgtgtcgacacttggacacggcttacagatgaaaggcagatatatttctatttaacctaccacttatccgggctccaaatccgcccgtccaactcatcttgtgattgctgcgctcgcttttcctgctccttagccaacgcaatagctgcttgataaatcgatttattaacaaatgattggtcagcttcctttagttgggtcagctgttgaaccaaccaatccgttgtatcactcatccctattcctcctgatcgcgaatcattttcacgtcttgttttaaactttcaacattattttgttggtcttcaatggagttgatcaccaaatcaatggcctgctgaaggtccgctgacttatctgatttggtatcctgcagccgagcgaccagccactgttcgcggttggccaaactcaacggcatctcggcactcaagtattccagatagtcgaccagcaacttctctttttgggccggatccaaataaccaaattgattaacaacaaacggctttaggtaggtcatccctgctttattagcaaacgcctgaaatgggcgcagcagttcggaaacggtaaactgctccgggcccccggcttggaagtcggcctcggcatcccccaatgagacgacgattcccaattctttcgtctttaaggatcgtttggcaacgatatagtttctggtgaaaacatcgtccatgaatcgttttaagctcgccggggatgagtaccagtacattggaaattgaaaaacaatccggtcaaaatcccgcagtgcattttgttccttctcgatgtcgattgtcccggttgctgtatataattcatcaatcacctggtatttcacgtcgtccagggaataaaagctggttttaagaaattgttgcgttcccgaatcctcaaattgaggatgggaaattaagatcaatgttttcattgttatcctacgcctttcataagcctttttcatttcgtttccacttaaaatcatctatattaagattgtaaaccaaatcataatcaaaggagagttaaactatggcaatttataacgttcatactaccttaagagacattggagctcaaacaattaacactgcgggggtccatcagtttgtggctgacgagcccaccaaattccgtggcaccgatgccggccccaacccggttcaatacttgctgggcgctgtgggtgcctgtctgggtgccagcgccgcatcattggttcaccgccccggttccaatattaaagtggaagaatttgaagtcgaagttaccggcgaaacagaacgttttgccgacaagtcttcacgggtcaaaagtattcatgtgaaattgacctgccacaccaacttggataaggaaggcaacgatcgattcatcgaggataccattcatctgtgcaccgtccacaatactttgaaagattccgtggaatttacctttgagattacggattaatttcgatttaattgaagaataacattactgataccgttagcacttcatattatggagtgctaattttattttctacaatttagtaaattgtcttgcgaacattggtgtacaagcgtttctggcaattaaatttttatgctaattgtttgacctcattaccaatatatgatactatatagttgttcgaaaggggaatggatgttcgccctcgaacattttcaacaaatacaggaaatcatttagaatatgggggtattgcctatgaataacgatatttttggaactaatggttttgacgatattttcaacgacccgttctttaggaacgcaatgtcagattccaacggccgtcaacagtcacgtcaacaacccattcaagttcaagaacgcagacctcaacagaagaaaactttgttagatgaatatggaacagatttaaccaaaatggccaaagatggcaagttggacccagtcatcggccgtgataaagagattgaacaaatggaagaagttctcagccgtcgtaccaagaacaatccagttctgatcggagatgccggtgttggtaagactgcggttgtcgaaggtttggcacaaaagattgtcgccggcgatgtgtctgagaaactcctcaacaagaagatcatctcgattgatgttgtctcacttgttcaaggaactggaatccgtggccaatttgaggaacggatgaagaagttaatcgatgacgtttcaaaggataagaatgtaattctgtttatcgatgaaatccatcaaattattggagccggctcaactggtgaaggtgacaagatggatgccggaaacattttgaagccgaagttggcacgtggcgacttccagttaattggtgccacgaccagtaatgagtaccgggacattgaaaaagaccaggcccttgctcgtcgattccagccaatcatggtgaacgaaccaagtgaacaagatacgttaaccattatcaaaggcttggcaccgaaatatgagaagttccaccacgttcaatacactgctgatgctttgaaggccgctgtcagcttgagtaaccgctacattcaagaccgaatgaatcctgacaaggccatcgacttaattgaccaagccggagcaaaagttgccatgggctcatcgctcacgaaagacaagtccaccctgcagcaagaagcagaacagcttgaaaaggataaaaacgcagcttccaagaaagaagatttcgagcaggctgccaagttacgtgacaagctggacaaggttcaagatcaaatcaagaacatcgacagcggtaccaaagtcacaacaccaaaggttacccctgaagtgattcaatcagttgttgaacggatcactggagtcccggtaaccgacgtcaacaagaatgaagtcaaccagttgaacaatttggataaagacctgaagaaagaagtcatcggccaagacaaagccctggatgcaatttccgctgccattcgtcgtagccgggttggctttactgaaggtaaccgaccaattggcagtttcttgtttgtcggccctaccggagttggtaagacgcaaaccgctaaggcgctggccaaagaattgtttggcacgacaaaagccatgttcaggtatgatatgtcagaatacatggacaaaatcagtgccagcaagttaatcggttcagcccctggttatgttggctatgaagaaggcggccgtctgaccgagcaagttcgtcgtcatccatacagcctgattttgatggatgaaatcgaaaaggcacacccagacgtcttgaatctgttgttacaaattttggacgatggtcgtttgtcggacgcccaaggtcgaacagttgacttcagcaacaccgtgattatcatgaccagtaatgccggtcaaggtgaagccgataacaaacaaaatgtcatcgaccgattgaagccatacttcaagcttgagttcttgaaccgaattgatgatattattcaattcaactcattaaccaagcctgatctgttgaagattctcgatttgatgctcaacgatttgaaccaattagtcgacaagtcacgtgggatccacttcagcgtcactgccgacgccaagaacaagttggtcgacatgggttacagtaaagaacttggtgctcgtccaatgcacagagtgattaccaaagaaattacagataaattaaccaatagttatctgcagaatccagatgtcaaagacttcaaagtcgttgttgacaaggatgccatcaaggttgaaccagttgctgccaagcaagcaattgcttcataaccccgaaatgatcgtaaactaatttgacaaagaccagtgatgttggtatattatagtcaatgtgtttaagggttcgattttcaaaggtatttgttttatagtattatgaaataactccttggaatcactgcaacttgatacattaaaatataattatgcgctaaaagcgcaaggaggtttcatatattatgaaacaaggtactgttaaatggttcaacgctgataaaggttatggcttcattactactgacgatggtgacgtatttgttcacttctcagctatcaacaaagacggcttcaagtcattagacgaaggccaaaaagttacccttgacgttgaagacagcgaccgtggaccacaagctgctaacgttacaccaattgaagactaattcattagtttaaaatttgaaagaaccagcgatttcgatcgctggttctttttttatgcccaccttcatccaattgcctatatacatataaggtgctgaattatataatagaatggttctgaaaatattaagaaaggagaattcacacatgaacatttcaaagcacttcaatcactcgatgaagttaacggcttgcttgggtgtttgtttcggctttttgctgcttgccgaccctacatatgcggatacatcgcaagctcaaaccagcagtgagccaactgcgacggcaaccgctagttcatcaacgatagattcacctgtgccatcaagtgatagtgactcacaaacgactacggttgatcaaccaaatgaaaatgccaagtcgcaagctgttgaatcaagtaatgaacaaccgaccgtcccagagactgatgacagttctagcgagcaacccgttcctgcaaatcattcaaccgccgagacgacaaccaccagttcatcaactgacaatcaatcagatgcagatactgccaccagcaccactgacagcccagatgatagttcggacgatacgccagatgtccagccgaatgacagtcaagccacaccagctgagggtgctcagaccacaactaacaatccaactgatcagtcgtcaactactggtccatctgacaaggatcaaatcaccatcgacggcattaatcagtcaactgatcccgccatcaagcaatccagcaacaatccattgatcaatttcttgaccagcatcaccagtggcattgccgcctcagtgatttatccactagtcgccagtcgtcaaggggcacaattcatttcgcattttcgaacattgttgtccccaaaccgctgggatgtcagtcaaaattgggcggatttggatcagaaatataatccggattacgtcaaaacatactataccgacgctcaggactggtacgacaaccgtgtccaaaagcaaacttgggaggttccttttgcggacgggactggtactgccagggcaacttaccttaaaaatggtgactcgaagaagaccatcatttacggtcaaggctggacaaccgagccggagggcatggggcgaatttccaagatgttttatgacatgggctacaacgttttgatgccctacactcgcggccaaaactccagtgacggtgaatggttaaccttcggggataaagacaaacaggattgggtcaattggattaacaagattgaccaaaccaatggccaagacagccagattgttctctacggtcaatcacttggcgccgacactgcactacaatatgccggccaaggcaatttgccttcttccgtcaaagcaaccattgcggattgtggtttttcgaccatcccatctttgatctaccatttgtacactggtgcagctaacagtctcaatagcatcacttctaaaattggctggaacctcaacggctcaattccactggttccatttgatcagctcttaacggcgatgaacgggattaacaagcttgttcaaggctttagcctggatgacgtctccggcatcacagcagttaagaattcgaaattgccaactttattcatttcaactgaagatgacactttcatccctgatactgaaactgaaaccatgtacaacctgagtgcctcaactgataaaaaactgtgggtgcttgacggccacgttggcggtcatgcttcagcaagcaacgccgttcaggattacatgaagaacattgaagattttctggcttccgcaatgaatcaaagcagttcgtcttctgatgatcaactgaatgttccggcaaccaacaaagttgctgcatagcacttcaatatcaaccttggaaaaggctcagcgataactagtcgctgggcttttcttgatcaacaatcaagtttggggcagcttggcttacaaaggatttattaaaattgacccagatcaattttttaccatccaaaacgtgctaaagttaaaatgtaaaatgtttcgatgatatgtattgacatcagttttgccaatctgtattatgttaattattaactaataaaaagtaagtacactactggaggaattttaacccatgaaagaacaattattagatcttgccaagaagcgccgctctatttacgcattaggccgtaacatcaaccagagcgaagacgagattgctgacttaatcaagaagaatatcaagtgggccccaaccccatttaacaaccaaaccactcgtgccgtgatcttgtttggtgccaaccacgaaaagctgtgggacatcgttggcaaacgcttgaagtcagaagttcctactgaagaagcttaccaaaagactttggaaaagatcaacgccttcaaatcagcatttggtactgtcatgtactacactgacatggacgttgttcatcgctttgagaatgactttgcactgtacgccgacaactttgccgactgggcagaacaagctcaaggaaacgctcaatttgccgtttggacatcccttgccgaaaacggcatcggtgccaacctgcaacattacaatccactgatcgatgaccaagttaaagaagcatttggcatccctgacagctggaaattacgtgcccaaatggactttggttcaattgaagccccagctggcgaaaaagaattcatgaatgacgaagaccgcttcaaggttttgaagtaattaaattgcatgccaaaatggttcccaaccagatcacatctgattgagaaccatttttttgatacactcacttcttcaattgaactttcacaagctcatcgccatgactgacgacatcttctttggtgtaatcactttgagtaaccttgtcaccctgcgtcagcaagaccagcacggtatctttgtaaccagcctgttgaatcttgtctcggttaaattccagcagcaggtcacccttcttgaatgactggccagaatcaacgtggttaatgaagccttcaccgcgcatattcacggtgccaaggccgacgtgaatcaagatttccaacccatcgtcggaacgtaagccaatgacgtgcttcgtggtaaacaacagaaccacttggccatcaaacggcgcgtaaatctttccttccgtcggttgaatgccgatgccgtttccaggcaatcctttatgatcatgctcgtcaaccacatctgccaagttgactctcacaccacttactggtgccgcaacagtgatcgtggcttcttcagaactggtagtcgcattctcagaactagttgcttgctcatccgagttatcactaatcccttcaacagctaacttgtgctgcagttcgtcaacgatttcagcatgtttcttttcagaaatcttaaccttgaagacatagatgaataatgccaaaacatgcaagataagtgcggcccagaatgcgaccagtttgaataatgaaatgccgcctggggtcattgaagccgcggtggcggttccagtcatcccagctgcaacggcaacccagccaacaatcgcatttgaaatggcaccggacatcttatccaacatcggccgaattgccaaggtaacggcttcattccgcgtgccatttttcaactgaccatattcaatcgtatcggttaaggtcaaaataaccgccataaaaatgaatccttgtggcacataatacagaatcatcgctgtgacaaccatcgctaaattatccgtggaaacaatcagtaggatgtatgccaagatcatgctgcacatgctgacggcataaattgtcttgcgggtcacccacttgttaataattgggtaaagcggcgaagtaaagaaaccggcaatcgttggaatcagtccggtaatccagaataatcccggtttatccatgacatacttgaataaatagaacatcaagccggcagtagccgcattcccaaaaccataaatcaggtatggaaaggcagtccacagcatctggtcgttatgtgccaacgcccagaacatttctttcagactggtctttttcttagtaactgcccgcaaagcattttgcttctcgtgggttccaagagcaaccaccagggagcaaataatgcccacaacggcaatcaaaattccaaaggcagtccagcctggttggccttcgttgtgtttgccggtaaagaagaaggtcacataagtaaccaccggcacgataatgatcgtaacaatgttttgaccaaaaccggcgaagttggcggcagccgtgaacagtgaccgctcgtgactatcttcagtaagtgcaggcaccatgccccaataagacacatctctgaatgagtagaaaatatcaaaggtgatgaagatcgggataaagagaatggtgaaccaagttgcactcacccgagacaagccaaagattccggaaaacagcagtgccagcagcaaacttgaaatcgttccggcaccgattaaccacggcttaaatttaccccagcgcgtattggtgttatcgacaatgttcccaataatcggatcgataaagatttcgaccaaccgaataatgaaaattaacccggtaatcatggcaattaacttgttggcctgggctttgggaacccctgtgaacattgcggaagtgacatagaccatgaagtaagttccaaaggtcatgtagaccgcagatccacctatgttagcaaacgcaaagttgaaaatcgaccagaaatttttccgccgatctttcttttgtacagcatccaatttataaaacgcctcccagcgtgccgattcgccattacaaatgggcggttcggtatgaaaattcgtagaaaatatttccttaccaatcgagtatataatgtaagagttttcatcaatgctatatttttaccgtaaaatacccaaatttaacccaattatagtaaaatatactaaaagggagtgcgaagatgcgaattgcgtttaataaacctgcagaaacgatgccgctgtattgtgacagtgtcggctatgattggaatcagccgccaattcaccgactgaacggctattacgcctaccattggctgcaaaccgaaagtggcgccggtgtgattaacattgaccaccagtcgatttccctgcaggccaaccagggaattctcctccgtcccagagtcgcccatgaatatcatccaaccggaaaagaaccttggaaagtatcgtttttaaccttcaacgggacactctgcgattcgctggctgattttctgaaactggcagatttcctggtaattgacacggtttcaccagaactaacatcgtttattcccgaagtcttgaatgaatttaacaacaatcatccaatcgccctgctggatcaatccgttcaaatctataaatttatcatgctgctgaagcaaaaccatttactgaacaatcaccgttatcaagatgccacaattaccacgccaattcttcaatacattgcggcccactatgccgaaccgattacgaatgacaaattgtcgaaagccaccagttattcagttacctaccaaaaccgggtttttaagcggctatatgatatgaccccgctggaatacctgaccgattatcggatgtgaaaggcgaaggaattgttgttaaccaacccaactctggaaattggcgagatcgcaccaaaagtcggctttcataatccgtcgcatttcattgaccagttcaagaaatactacaaagcaacgccgtctcatttccggaaattcatttagaaaatcttacagattcaaaacagtctcatttatgaaatcaactttaattagtggtaaactttgcctacaacaataattgaggagtgatcttatcgaatcaactgttaagcgtggttggggcatcaccaacttcgacatcaaagtacttggaattattctgatgttcatcgaccacgtgcatgaaatgtttaacggtatcggtgtgcccaactgggtggactggtttggccggtagcaacgatctttttcttcctgagcgttgaaggcttcattcatacccataatcaaaaacgctacttgtccaggctgctggttggcttttgggtcatgcagattgggaacctgattatccaacatttcttcaaactcggcagttttggcttgattaacaacatcttcggcgacctattcattggggtgctgacaatgtatggcctgcagaccatttctcagggtcatcagaatcatcaggcagccaagatctgggaaggaattctcattattgccctaccgttgatctttgccggcctgaccttgctgacaatgggccaaggcggcaacagcattgcctttcgaattgtgaccctgctgccaagtcccctgattgctgaaaacggctttatcctttacctgggaccattgatgtatctgttaaggaagaaccgcaactggcagatgctggccgtcgtggcagtggcaattttgtccaccggctttaatttcagcagtatgttcacgactaacttccagtggttgatgtttcttgccattatcccaatgtacctttacaacggtcagcttggccgcagcatgaaaggcttcttctacgccttttacccactgcacatttggctgctgtacattctggcttggttcatgggtgtgcgctattaatttagacaaacaaaaaatgagatgctggtttccattgagttggaaatcacatctcatttttaatttaagcattattttgtgataaatacatacaaggtactggtcgagtaccccaagctaaacaatagcccattggaatggaacttcggtgccgttgtcgagctggacttcttggccttggccgccttctggaatttgttcaaaacgtgcttggcgttagcgccgacactgtttgtcaaaatcgagaacgacatgataaacggcttgaggtcctttttatgcttcaagctgttaaccggcaccatcattgcgatgcctaagactttatcacccgataaattgacccgcaatgtcatcttgttggtatcaatcaaattgtggatgccatctttgggattggccggcagaagctgatctttgacactagccttggctttcttcattgccggggccagtttagcttgcgtttgcttcaattcagctgcctgcttttgaagggccgtcgccttttgcgccttagcctgcatggctgccatactggtagccttgccggctttcaactcggcagcttccttcttcagttgggcaccctgcttagccattgattgggccagctgttggtccttctttggcaatgcggcgccggttaatccttggttataagtcgtccgcatcttctggtaactgccaaccacgttggccttggcgaccgtgacggtttggtgcttgccatccgtgctcaatttgacagtttgttgataattcttagttggcacactaattacaaatgcaccgctgtttgttttaactgtttgcttcgtaccgccattcacagtgtaatcgacctgcttttgattactcttgcctttcagcgtcactgccaaagcattcgcgctcaaatggtgattagagaccgtcaacgttggtttaccacaaccgctcagaatgaccatcagagaagcggcagcgactactaaactcattaattttttcatcgtaagctcctccttaatcaaacgaaacgtcatctgagaattgactattataaagatcagcatagaagccgtttttagccaacaactcattatggattccggtttcaaccacggcaccatggttcatcacaataatgttgtcggcgttttgaatcgtggacagtctgtgggcaaccacaaagctggtccgattctccaacaactgactcatcgcatgctgaatctgaacttcggtccgggtatcaactgaactggtggcttcatccaaaatcagaatttccggatccgccacaaaggctcgggcaatcgtaattaattgacgctgaccttgagaaatattggaagccgattcattcaaaacagtatcgtaaccctttggcagtttgcggacaaattcgtccacatgggcagccttggcagcttcgataatgtcatccttgctggcgtcttctcggccatatttgatattgtcgtagattgagccggtgaacagccaagtatcctggagaaccatcgcaaagtgtgaacgcagatcttcacggtccagatcacgcgtgtcgacccccttgaggcgaatgctgccgcccttaacgtcatagaagcgctccaacaagttgatgatggtggttttaccagcaccggttggaccgacgatagcgacctgctgaccgcgtttaacggccaggttgtaatctttcatcaacaattcgtcatcggtgtagccaaattgaacgtgttccaattcaaccaggttatccgtgtcggtttccactggtcggttggctttggtattcttcatttcctcttcatcaatcacttcaaacacccgctcagctgacgcaatcgtcgactgaatggtgttcatcaagttggcaagttgagaaattggctgtgagaattggttggtatactgcaggaaggcctgaacgtttcccaaagttaccgttccgttggcaacctgaatcccaccaacaaccgccacgaacacatagccgatgttgttgaggaaaatcatcaacggcatgataatcccggaaataaactgcgctttccaagcagcttgatagtatttcttattttgaacttcgaactggtcaatcgtatcttgttccttgttaaaactcttcagaacaatttgaccggcataattttcttcaacctggttgtttaacaaccccaggctcttctgttgagccgcaaaatatttctgcgatcggggagcgacgatgccgacgattaccaaactcaatggaatggttaccagggcaattaaagtcaacttccagctaatcgtaaacatcatccagagagttccgacaaaggtcacgaaactggttacagcctgggtcaaactttgctgaagggtgctggcgatgttatccatatcgttcacggcccggctcatgatatccccattactatgagaatcataatacttgatcggaaccagccgcatcttgcccttcatctgccgccgtaatttgtagacggtgttttgagaaatccgggtcatgatgtactgctggaagaaactgaaaacagccgatgccaggtacatcacgataacgataagaataatttgaacaattttttcataattgattggcagcgaagccacgctaaagccggctttctgctgggcatttcccttcatcaatcctttaaaaatttcagtggttgcttcacccaaaatcttgggtgtccggatttggaagataacactgatgatcgcaaaggcgaacaccaaaatcaggccaatcagtcgatcctgcatgtaattcagcagccgcctggtggtgccccaaaagttatggggcttttcaacaacaccttggaagccgccacggccaccatggccacgattggaggtaggttgtggtgccttatctttatcagccattatttgtcatcctcctctcgtaattgtgagtgaataatttcttggtaaaccttgttgttagcccgcaactcgtcatgggtgcctttgccaaccagtttgccgttatcaagcaccaggatcagatcagcatcggcaactgtggcaattcgttgggccacaatcacagtaatactctgctggatgtgttgatcggcccgcaaagcagctcgtaaatcggcatcagtcttgaaatccagtgctgagaacgaatcatcaaagacgtaaacggcggcctgcctgactaaggatcgcgcaattgccaatcgttgcttttgaccaccggagaagttgtccccaccttgttcaacttggagatcaagtccagcgggatcttcttcgacaaaatccttggcccgggcgatttccagggcgtgccaaatctgatcgtcagtcgcttctgggttcccatatttcatattgtcacggatagttcccgtgaacaaagtggccttttgtgggacaaaggaaacttgatctctaaggtctttcatcgagaaatcattgatgttatgcccatccagctcaatctcacccttatcaacatcatagaatcgagggatcaaggaaaccaaagtcgtctttcctgaaccggtcccaccaataatagcaaccgtttggccgctatgcgcctcaaagtcaatatcacttaacgccggcaattcagcttggcgataacggtattcaacatgatcgaatttcaagtcgtgctgagtggctttaggatcaaggaccaccggatgctccggctgtttcatggttgatttcaatgccagcacagtctgaattcgcttagctgaggcctgtgcacgaggaatgaaaacgaacaccattgagagcatcataaagctcatcagaatctgcatggcataactcatgaacgcaatcagattaccaacctgcattgactgggcaccgattaacttggcaccaaaccagacaatcgcgacgttggttccactcatgattaaagtcatcacggggaaggccaaagcgacaatcgtgttgaccttgatggcattatcggtataatcccggttggcatcctcaaagcgatcctgttcaaattggtcctgccgaaatgcccggataacccggacaccagtcaaaccttcacggaaaattcggttaattttatccgtcttagtctgcattgctctaaataatgggactgagaagtagagtaggaggccaacaaagataatcatgatcggtaataccaccaagaagatggtggttaactgatggtccttggtgtaggccaaaaaactggcaccaatcagcataatcggcgccatcagcatcatccgcagcatgataattgccacgttttgaatttgaaccacatcgttagtggtccgcgtgatcaatgatgacgtctcaatttgatcatattcatctttggagaagttgatgactttacggtaaacgtcactccgcaaattttgccccaacttttgtgaggtccgggcagccagaaagacgttgcagaccgccgccagaatactaatgagtgaaaagccggccatttccagacccactttccaaatatagccaatgtctcctttggcaaccccgttattaacaatgtccgaggtcaggctgggaagattcaaggtcgcgatcacttgaatcgtcatgaacagcactgccccgagaactgccacgtacgagatccggtttttggcaattttcagcattttcctactccttccaggttcgttttaagattgttgtgcgcttaattaggtaccgaactatattactgctagtgcatttaaaatacaagtataagttggtaaataactaggtaaacagatacgtcctattatgaacttttctgcggtgagtttcattaatgttaactaaaattttgctttagggattgcaagggttagataaccgcaaaaatgacaccgggaccatcttgtctgatgatttcggtgccattctttctatattattatcgtgtgaaaatgagtggacttgaatttttaacaagcgatccaaattttctcacatcacttcgccaatccatccaaagtgaatttaagattgggcaacatgttcttcaggcgtcttaaccgcattctgcttatctcgttcaaggactgacttcatgtagctgtcgacgtcaaatgtcccggcaaattcggccaagtgaaccaggtttctcaagaagtcgtgggtcttggcttcgtaatgatactttaggccaaggtcgtagatgtagccgttgatgtagtccacttcggtttgacgattcttagaaatatcttgatacatcgacgggaagtgaagtgggttggaaacggtgctgacgtatttaacggtttcccactcttcttgacgggtattcaataacgtgatcccggcgcgttcacagacatcgaaagcttcatcgattaattgaacgcccaacttctcggcaactggtgattggatatactcacccattcggatcttaaacatcgtgcacaaggtgttgatgacggagttaaagacgactttggccatcaaagttccaaggaagttcttggtcaaattaggattaagccctgctttttggaattcagcgacaatcttgtgagtcatctcatcaggtttctcggtttcattggcaatgttcattgaaccggcacccttgggaccgatgaagtcgacgtcgccggctttgttcaacacagttccgatcagagcggttccgccgagtaaacgttccttggggaagtactggttaagtttttcaacgtgacccatcccattcatgcaagtgataacgtattgtttgtcgttgaagaatcgtgaacagcgttttaagaaatcagcgagttgatattgcttggtgaagacaatcaagacatccggatcacccttgtattcttctggatagtacacgttgaccgggaccagatgtttattttgaccgtcacgggaaacgtaaacgccaccctgttggcggaccgtttcaacttgtggttcccaagtatcgacaaagtcgacatcgaacccggcttcctgcaaaagaaccccatatctcaaacccattgcgcctgcacctaatactgtatatttcataaatataacttcctctccactataaagtatgtaatcaacaatctttatcaatcccactaaagcaacccgcgatacaaaaaaatcgcccttctgtcactaagacaaaaggacgacaattggccgcggtaccaccttcatagacacttttcgtatccactcgttacttgctttaacggacaagtccgaaaccggctaacttacgctcaccgatttatgggtaaagcatgaaagtcacaatctacaatttcactaccatctctcagccgccgaatggattttctgttagcgaagcttgtagaaaacttctttcaaattgatagttcgtattatgatagtcagattagaatatgtcaatactttttgagaaaataatgtgagcagctaacatcctgacatcacaaaaaggcgactagagcaatgtctagccaccttttaattgattatttaattatggttattttttgattgattcctcatttctcttgtttgcgcttggcgtagtaaatcgttgctgttcccagtaagccaaccagcatgaacattccaatcaccatcagcagtgtgttgttgtcttcgccggtttgcggtaaggcggacttgccggtatagccggatgacgggattcccattgggctgtcgagggtgcctgacttgccggaagttccggtggtgtcattgctgtcgagcgtaccagaggatgcatcgtcgccgtcttcgccgggtaatggtaattcgccttcatcgtcttccaaatcgttgtggtaaacgatgctgtcatcttctttagtcgccgttccggtaaccgttggactgttcacaaccgctgttcgcttggtaacagttgttacatagccatcagctgagtagtccttttcagacacttcatatttcgcaccaagcggaatgaagaacttgatggactggccatgaattaatgtgaagctgccgttaccaccgttgaattgaatggaaccttcaacaacttggccattggttgtgacctgggtcttaaacgtcccgttcagtgggttgttagccccatcggttgcttcaatgtggaattcaaacttgcgagctctgtcgcccagttcgttcacaaatttgctcacagagaggattcccagttccatttccccattcttggtgttggtaaattcaaccgtccctttttgatcttcaactaacttgaaggtttgagtggtcatcccttcttgaaccttggcgccgttcacctgataggttggtgcaaagccatcaacatattcttcgcccaccgcataagtgtaatcaatcggcaagccggtaactgtcaatgattcgctgtccttcaaggtaagcacgtcggattgaccgtcggcgaatttcacagtgatttcgtgtgagtctccgtgctggtcaaccttggtggccttgaattcgccagttacaccagagtagatgcggaagttgaagtcacggtcgtggtcgctggttgtcaaaccatcgccggcaatttccttgttaatcttcaagctggcaactttctcggtgtccttgctgttggtgaagtccacgttgacgcgatccttatcaaccagctgaaattctttggtcttaacgccgtcttccatccgggttccgttgagttggtactgcgtgtggaaaccggaaccgttggtttcagtaacagtgtaggtgttgtgttcacttggcaagccataaatcagaatattttcgtcagccttcatattgacagtggctttgccatcagtaaacgtcactttcactttgtcatgaccgtttacgagtgcgtcgtattcgccatcaacacttgcgttagcttcaatcacgaactggaaggtcttgttcttgtcagcgtcgatgatgccgccgccagcaaggtgcttgctgatcttcagctcggccgtttcggcttcaaatttggtgttggtgaaaatcacggtccccaatttaccttcctcagtcacaaactctggagcgacattgcctgacttctcggtgttttcgttgaccttgtaacttggatcgtagccttcactacttgccttggtttcagttacttggatgttggcaccaattggtaggccaaggagttgggccttttggtcatgcttgaggttgaaggcaatgatgttgttagcattaaacgaaacaggtgtgtcggtgtacttaccacttacttcgtatttgcgaagggtgaatgttccgtctaatctgccaccgttttcactggttccttcaactctaaatctaaactgcttgttgaaatcttcatccccaacggtttcgccctttactgtcttcttgacttcaatgccagtcttaagcgaatggttattgaagattaaatcagccatatccttgtcagtcgtcaattcatgagtatcaccgtcttcggtatggttaccaaatttgtggctaacttcaaatccgtgagttttagtttcttgagcttcaagcaacaagccctttgaaatatagatggtaatcccctgatcagctttcaatttgatgatttcagatttgtacacgtcattgtctttagtgaacgtaatcttgccatccgcgttgtccgccttaaattctttagtctttgcgtcaccccaatttgcgggtggattcttgatagtcaacacaaactcaaatgctttatccttgtctcccgctgctacggtgccactaaccgttttccgcaatgtgaatggaacaaggtcgggagaaatattttcgaactggattgagttcttgaagttttccctgttcagttcaatgtcagctgctttgctgtcattcttcttttcctcgccatcaacatgtgtgttggtgtcgtagtggccctcgcttagttcagtcactgtaaacttggttgcatcttttggcaatccaagaatcaccagcttttcattgtccttaagggtgatctccttaattccggttacaccatactcaatttctgttacggcaccttcatcgtcaaatgtgatctcaccactgttaataattctgtcagtagtagaatttttaacaactgctttgtatttctgccccttaatcgcattacgagtggcatcatcatttgccttcactttaaacttgaagtcaacgacgccctctggcatgtcaccagcaactgttttttcaaattcaaactggttcacaacttgtcggttaatgaatttcaacatagtattcgtagcattaattgaaccagttgccttccagccatcttcatccgaattgccggcttcattctcatccccatcgccaactttgtaatgaacttcggtatattgggtatcttgtttttcatataccttcacttttacattggctggcaattggatgttccgatagctttcaccagtcttcagcttaatcggtgccgtgctaccatctgtgtagatgatttctttggcaacaccaccggtaaatttaaacttgactggaatgtctccacctgagtgtttgattccttcaatcgtgccgttaaagctcttatccggctgattgtcgtcatccaataccttcagcatgaaatcaaattccttgttcttgtcagcattggcatttggaccttggattgttttggagaatccaaaatgcgtcgtctgaacatcattggtaaactgcacgattccagctggagcattcttaccgatcatcatttggaaagtatctgtttcattaccgccatttccatcaggttcaaccgtcgttaagttgtcaagtgagtgggttgtgctgtatgaaccattggctgattcgatcacccggtacgttttgtcctgtggtaatccgtgaatggtgatcacctgaccgtctttgatctcttgaagattagttgaaaccccttctttgaagttcacaacactttcgtcaccatcaatatcgtaggtgaaatcgtcattgaagtcggtatcgacatcaccctcgtcgttgatcacatataccttaaattcaaacttatcgtctttattggtattcagtgaattggtaaccgtctttttaatcttcaaagcattagttcggtgattcttagcagtgacgcaataagtgttctcattgccgtcttcagtttcttcttgggcatctttaatggtaaattcttttgaaacccatctatcatcataattctctaggccctgagtttcgataatccggtaggtcggtttatcgtaaaggccgtcgaatgatgcgaaaccgtctttgtcggttgctttaggttcaccaacatttttccaaatactatccagatctttcatttgaagttggaatttgacgccttcaagtggagcgccagtcgtggcatcaactttcttaacgttggcagcgaaagttgtgtactgcccggcaacttctgcacttgattggatttcttctttgtcttcaaaatctttagaagcaattgtcaacttgatctcattactataggttgtcccaaccgtcttggaagtaacggtatgatactcaaccaatagcggtgttttaaccttatatgagttattcacattaatcgtcatcgtattcaaggtatcggagtaaaccacatcataatcgtggccttcaattaaggctttatccgatatcttagtgtaatgaacttccttattgaccaaggatcgttttgcttcatagattttcagcttgtagcgatcatcgttggtcttcaagtggtagtgcccaccactaagcgtatcggttagtttaactggcgatctaagttcgtagccattcccgttaattgccaaattccatttaacggctccaacggatcgggtctgcccgtcaccctcgtctaattcaaggttgtgttcgagcaacttccctgacttgtcgagtaaatgaccgccatctgcgtaagatacactcgcctttgcttcaagggtatgacgagtctcatcgtcagcattcagtttccatccggcagtgactttgttattaaatgtccaagttttgagatgttcataggtcgcttcttcatcggccttaaagttcaagacttttgattgatatttcaactcgaacacttttttaccgagtacactctcaccatcggcattctcatgatccagatagatattgttgtaagcatcttcggataactttaagttaaaagttactttatgattttcatcaacatcaacccgaacttcatattgatcatcaactaacctttgactgtcagatacgccgcgaccatcagagttaatcctagccagggagatctggagggtatcttgtaaacgttgctgaatatcttgaagattacgtttagtaagctttccagtagcgtctttgatcacatccggtccaacttcatcagtgatatcaatcccatcagtgaccaaggcggcgtgctcatttgaacccaggtattgccggtagttgaaacgcgtcgtccaattaatgaggccattgttcaggaaatccttatccaattgcccatcctttgaaatgttgtttcggatgaggcctccctgattgacgcaagtctttacacttgcgtcatcagaccctgagtattctaacccagcatagttacaaattttttcaagttgggcataattagcatttaagattttttctttgtccaatggaacatcctttagataaatattaaatgatttttcaccagccggtaaattctcaacggtgatgataatctggttaccggaaagtttgacactgaatgctttgttgtccttgttcttgccccagtatgcttctccatcgatgatcgtgtaatcccatgtttgatcattttcatgcttggaaaatgaaattcgtttcttaacttcttcagtcaaaccatctgtatctgtaaaactgttataaaacttcttataatccaagaagttgagcgtctccccttcgattggttccgtgatcttgaatgaaccatcaatttgtcgattgatttggttgacgtggatgctccatgagctcatcatcttttgccaatccaagctcacgttgttcttactgttgatttggggaccaaagtgattacccttcttttggccgttcacctcaaccgtattgctgatactctggtaatctttgtcagtcacgtctgctgttggcttaatgatgtaactaaacttatatacctttgacccttcgttttccctgggaacaattacatcagcaaactcaaccgtcaacgtctgaccgtcaattttgggatcacctttcatccaaccggtaacggatggtattaatgtgtaatcatcaatattctcactaaacgtaaatctcttggaattcaaagtatccttcaacacaatatttgtttgaccaggatcgacggtgaattcaacggtatatttgatgctgccgtctttatccatctttgcagtcttcttcacctgaccattttcacgggtgatcgtcgccgtgacatccaacgttttggcagggtctttcacaccaacaatttcgacatccgtcgcacgaattgtatttttgaaatctcgattgttgaaattagttacgggggttatcattttcactttaatttcaattattccccgttcaagcccaagtcctttagcgttaaattggaaatttggaccggtggctaccaatttatcataatcatcatgatttttggtgatggacactgtctgcccgtcagcacctttcacttcaaactcatagctgactttatcattggcggttgcatagccgccaccgaatttatctctcagggtaaccttatttgcttctttaccgtcctgcaccttaaaggtagatgtccattcaagcatatcaagatccgttaccccattagatgtgtggaacacaccatctttttgaatagataccaaatcttcttcgactttaattggatattcacctttagtactttcaccaaaactaatttcttcggcgttcgcattgatttcggtcttgatttttgccttgtaatcaatgttagtcacaccttccaagtctccaggaaggaaaataatcttagcatgttgcgtgtcgcggtcctctgcatcacgggtcatgataaaccgaccaattgtccggcccccataggtgatgtattcgtcaaaggaacctgatggaccgtattaatacttcaatcccttaagatcaaattggtagtagtcgccatctttaatgtcaatcccggtattttccttaatgctatcaatatcccaaagataagtaatctcaatatttttatgctctcgaagaatagccggtagttgaagctcctgttcaagtacagatggcactttctgattttgagggttaccatccttgtcaatatagttaaaattgattgaggtgaagaattgagggtttgaggcagcgtggatagcatcggtaatatcagtttttccttcatcaccgaacacaccatttcccggtaattgccgagtcaattcgttacttgtcggctcctcagcatctgagtcatcgctggcaacggcttcttttgcacccttcagatcagaaacatctggtgtttgtggtgtttgagattccttgctctcaccattatctttgactgttctcggatcattttgtgtcccaacagctgcttgttcttctgccttacgattctcttcaatcgcctgacggctcttctcctcagccttcttctgatcagcctcacgcttctccttcagtaaagcttcagccttatcgctgttcgattgctttggctgctgaatgtcatcagcttgagaagagttctcattaatttcggtttctttctttggttctgcttggtcttcggtcttaacttcagcttcctttttagcctcagcctgcttagcttcttccgcctcgcgggcagcttgagcttcatcggatgccttttcgtcagccagcgcttgcttcaagatgtcatcatcttgcaggttgccgtctggctgatcggttgtctcttcttgtttgactttttcgtcttcatcaagcaccgtcaaagttggcagcttgatcttttcatcgtccaccacaaagtccaactcgcggtcattgacagtccgattgaatttcaccggcaaaatcacctcgaggtcggtcttatcaatggcgttggtccatgaaatggttgactcttcgccatcaatgtcgacgacgactttggtgtcaccatttgaaaatttgaattgtttcttcttcactttgaaataatcagcattatagtcaaagtgcacagtgccggcctgcgatagcccacccactgtcatatcaaatgccaagttggcggagtcgccaacttttgatttcgttactaatgcacgtttatcatcaatcaatttcgcgttatcgacgacaacttccttagtcgaaatcacgtcggctaaagcggttccggcagtaaagaaattccccagaaccagcgtcaacacgccaattgcttgtatccaaaagcttgtccttttcttcattgttgtcttcctccatatgattgattacatccctctcttatcaacatcataaggatacctgaataatatgcgtaatttttgaagaaattatgaagattccgtatcttttatatccggtggcaggcgtgggatttggaagatggtcgtgaagcggcatggcgttaagtattccggagaatgacattgttttcccattgattattcaatgaatccgaatagaatgattaccgatcaaatcttagtcataaaaagttccaaagctaaagttttcgctttaactttggaacttttatgtcgacaagtggttagccatttttgttgtagtagtaattactaggtgttactatatatttaataaaaaaggaggggattagtttgaaagcacgtaagcagggtaacactctggttttaagtattcccaagcagttcaaagtcgctgagggaactgaatttatgagtatgcaggcagctgatggcagcctcatctatacaccaaaagccccaaatatttaccaagatcccaaatatgctacgactgatcttagatttatccccaaggatactaacgaccaaccagtcggtcgggaggaaatctgatgtcaaatcacccaattacccattatgattatcatggttacactcctaagcaaggggatctggtttacattaattttgatccaagtattggtcgcgaaattaagaaacgtcgtccagccattgtagttagcagtgacgcttttaactcgcggactggttttgtaaccatctgtcctattaccagtactattagagacttaccatttttcatcaatttacacggtaacaaattacacggtcaaatcaatgcatcacaactgcgaacaattgatttcatggccaaagaacgccatattgaatttgtagaacgagccgccagcacagactttatgcaaactgccaaaatcattatggatgggcttggttttgagagcatcattaataatctttaacacattctatttcaattcgagcagcttaaataactttaaaacgggtttttaagggggaattccaatgtgtggacgttacatgtttgagccaaaacgtagccgtgaaatcgcgcggatctatgagctggcaacccaagctggctatgagccaacaacgggtgaagtcttcccatctgatcaaacggcgctggtcattgcccagcagcagaaaattcaagttgtggcgatgaagtggggattcccaggctttcacaaagggcaactcattatcaatgctcgatcagagtcggtcactgaaaagaaaatgtttgccaagtccttccaagcccgccgatgcgtttatccaaccagtggcttttttgaatggacaccagacaagcaaaagtattggttcaactacaaagaccaacccgaacccttatacattggcggtttctacaatatctttgaaggcacaccccaaagtattttgatgaccactgaacccaatgattccgtcagtgtcattcataatcgaatgccattgattttgaagaagtcggagattagagcttggttgatggatgatgaatttgcgaatcgctttttgactcggcagatgccgatgttgatgcgacagaaggttacttcggaataaacagcttcatttttttgaaattggcgtcgtgtattgactgcaagcaattcagctatgttataaaaaggtcctgccaattttattagcaagacctacttaacattattattgtgcggtataaccgccatctaccagaaattcgctgccggtagaataagatgattcatcagaagctaaatataaaatcaaatttgcaacttctgcagtttcaccaaagcgccccaatggaagcattggcaaatgctcgctaactaacttctgctctttaggatcattatctttttcaggcttatggattggccccggatgaactgaattcacacgaatattgtacttttgctgagcacaatataatgccgctgatttcgtcatcaaccggaccccaccttttgctgcagtgaaggcaaataaattcggatagccaattaagccttcaatagaggacatattaataatcgaaccaccattagttttcatattttgaatggcatgcttgattccaaatgcaactccgtctaaatcaacggccataatctgatgccattgctcagcagtgaaatgttccgcatcccccattgccgcaattccggcattattaaacaaaatatcaacttttccaaacacgtcaataaccttttcaaataccatggcccaatcagcttccttagaaacatcttgttggataaagatcgccccattgccaattttcttcagggctgtttcccgattggtatcgttaacatcagtaataacaacttttgccccttctgtagcaaaccgagtggctgtggctagcccaattccgttcgcgcctccagtgataactgcaactttattacttaaacgtcccataatgataatctcctttcagaacatgattaatgacctagaaatgttgctaaatcgtaagatataatgactgtgaattaaatcggaaagtatggtgaatccgcgatgaacttaaccagtttgcgatattttatcgaatcagctaaatacttgaattttacaaaagcagcggaacatctttatgtgacacaacccacactcagcagacaaataatggatcttgaagcagagcttggcgtccagttgtttgttcgtggaagacacacgctaactctgactagcgaaggcgatgcgctactggaacaagccattgatattgtgacgaaatttgataatatcaagaaaaccatccagccacatactaatgaattaaccggcaagctcacaatcggatatcaaagtttctttgatactacgctcatgtacgatgtcttaaagtcagtaactaagaaatatccaagagtcaccctgtcactttttcgtggtacgccacttcagttaagacgccagttaatcaataatcagtgtgatgctatctttggcttaaatacttacatagatagcattccaaatatcaagacaattgaacttcaaaaaaacaagttgcaaattgcggtacccagtacacatccactagccaacatgaaatctgttgatattaagcgattggcaaatgataatttcattatgctcaatcgcaagatctcaccattcattgttgactacgcgatcagtctttgcatgaaaaatggtttctcacctcacgcgttgtattacgtaaatgatgctgagcaggcattgcttcacgtgggttctggacaaggggttaccttcctacactcaatgaataaggtgaacaacccagttgaaagttacggcgtcaacctgcttgatattaatggtctggataatgatttgaacttcgttttaggttacaaagaaactaataccaatccaattacggaaatttttgtcagagaattaatgaaagttcaccagcaaaaagatggcagcaattaacagaaaagcttaaaggcgagaagtctttaagcttttttgcatcaatcacttcgcttcaacgtcttcaagttcaaaaccaactgatttgaatccaccgtttaactgaataaggtgcaccttagcctttaatggcaatttagtgatcaaatcatctttattttcttcagtgacaccatatagggccgcatcgaattgatgagaaccatttggccaatgtccgactgatacacaataaggatccttttcagtgaaaaattcatcggcttttctaaatgtgtaatcgccacccacactagagtcctcaaagcgaatttcatcgattatggcctcatcgcccatctcgatccagtccaggttatagctgccgcaatcttggcaagttgggagcggaggccagaccactttgccacaatcctggcacttcatccctaacaccttgccgtcttcgagactgtcataataggtttttaaaattggacgtaatagatacatattactcactcctcaattttgatcttccaaaataataccaactgttgtatggccgccacccatacctcgtacaaggcacttattaacaggcttgggaacttgcgagccaccagcttcaccgcgcatctgtaaaattgcttctccgagcatacatactccagcacacccaaaaccatgcccaaagctaatatcgcctccatgagggttaattggtttctcagcatcaaatcgcgtcttaccttccaactcatacttgtagccttcaccctcaggtagatacccgaacacttcggcactatccagttgttcaccagaggtcataacagtggtaatcatcaaatcaaagtcgctccctttaattccagggtgcttcttgtaaagattgtctctgacatcaacgttcatttgatggaagttaaaaggatacctagttgtgtttgagacagttgcatcgtcaatcacttgaatagggtgatctgaatatttcttagcaatgtcagcagagcacacaacaatcgctccggcttccatgttatggagaacactgccgctcttgcgaatatattgagtgattttaggattatgttctgatctcatatattccaatggatcgtcgtagccggccttcttagcgatgtcctcatatctttcatgcatcaaggcacgaggattgtgtgaggcattatatcgaagattcattgccattgagttataagtgtcatccagttcatcctcggtaattccatagtgtttaatgtaatatttgccttgttcttcagtaagcaaattatcactgacaccatcaaaacgcgtgtaggcagtatcaaacaatacccgacctggtgaccaccaaccattgtcatactctttaataggttttaatttatatgctggttgatttcgagaattgaaatgtttaggattctctaatccggcaactaaaacaatgtcatattgtcccgatgcaacactatttacagcttcagtaaaggcaatatatccgccagcacaggcctgctcgatatgcgtgattggtttacctgccaaccctgcccactcctctaagctgccgaccggagccatcacaccacccatggtgatgaagttagcgaactgggaataaaccactttgtcaatatcttttggtttaacatgcgcatcatccattgcttgatgacaagcatctgcccatagttcataaggcgaaagaccagccattttaggatcgtcaaaacttcgttgaggaagactacttgtcccgataaccgataccggtcgtgcaaattgttgtttcatcatgatttcctcttttctttaaatatgtggtgatagttaaaatgtttgcgcttacatttttggatggaaatatcattcaaagttttttagtaccatatccctttgacacttaaatcatatcttgaatgcaaacccctgtacaattggacttttacgaattaacgtaggcccatgttaaggtattcacaaaacgtataccattattctgtcacccttctttataattcaatggattgaagtcaatatttgagacagatttgaagggaattggacccatttcaaccctataagaagccataataaaagccctgtgaattgaattacaacgcttcaattcacagggttagctcatttataatgatgttctgacttccgttaagatcaacagccaactggaccggatcctgtgatcaaaacattgaatgtccactcacaagaacctattcactcttatcaaaactactcatcaaaaagtcagtcaactgctcctcatcaaccgtctcaatcccagccttcttaaccgcacgcttaacattccaccgactaggtttcttcccacttaaggcggcttcgatggcgttcagatcgccatcaaccttgaagaacgggttgaacttcagatgggaaagcttgccgtcgtcaatcgtccagttgattcccagcttgccctgatcaaattcagtatcagcgtaatcgtaatagccaggattatggccaaagttccaggcgtcggtcccataggtttctgccaggcgtttgtcagcaacttcccaatcctgatcagtcatatggtaggtttcaatgtcatccagggatttgacttcaaagatttctttgagcaggtattcgcggaaatcagccatcgtcatcccatccggaagaaagtccttcaggttaacaattgggctgcgcttggagcggactcccaagcccttttggatttccatctggtcttcagtgaggacttttctggcattttcaatgttcaaatcatacataatcgttccgccggccgccaagccttggccgcttttaaacatggtcatgccagaccacttcttaccgtccaaaatgaggtcactggaattctccctcattttgacgtcgatgtttaatttacgaagcgctttcaaaactggttctgcaaaatgcccataatcaccaaagtcgtcggcgttatccgtcaaaatgttttcaaagatgaggttccccatatcgtgatagacagccccgccgccagacgttcgccggaccaactcaatgtcgtgctcgtgcagatagtcgatatcgacttcagcccacacgttttgatttcggccaataatcaccgatggcttgttaatatagaacataaatccgtgtccaggaagtttgagatcattcacaaaataattgtccaatgattggttcacccgcgcgtcatagctgggcttgccattcctggaaatatcgattaggtacatctgacattccccctttgttcaaattctcgtacatctctaattatacggtataattgaggtaaataatatcgaggcggtgtcgttatggcaaaaatttcaatttggcaaaaaatcatcaatttctttactggcaaaaagcagtctgctcaggctccggcccaggttaaagatggaatctggtatcgaaaagaagctgacggtaactatctattgggcatcgacaaatcggtctatgatttgatgggtaagattactttcgctgattttcccaaccagttagacacgattgaagtcgatgacgatctgttggacatcgaaggtgacaaatcggtggaaacattgaaatcaccaatttcgggtcggattgtggcccggaacaaagaaatcggcaaagatattgaaaccctcaacaagcccgacccacaggtaaattggattgtaaaagttcagccggcagcttaatcatgcaaataaatcgaacaaattttgagccactttctcaaaaagaactataatgaagttagatcaaatagaaggaggtaattatttatggctgaagaaccaggtgcagaatctccattattgaacaaaatgatgtctgaggcattcgactggagcgatcaaaaattaccagtccgtgatgctatttgggactattacatggagaaaaacgaccacgacactctcaagactgaaaaagatgttgaaccttacatgaacatgtcaactgatgatcttaagagcaaagctgaggcattactcaagaagtaatttttcagtggttaatcaaatacccgcactagtttcgtgctaggcattcaaatgatcttcaagcttttggcttggaggtcatttttttagccacatcaaatttacgatttgagttatgatgggattaattaataaacgaggatggtaaatgatgaaaactgtgacaatctcagatgtggcaaaggccgctggtgtttcggtgacgacggtctccagatacctcaatggaaactttgccaaaatgagcaccaaaactcaagctaaaattgaaaccgtcattcaccggttaaattaccacccttcagcatcggccaggcgcctcaggaccaatcagtccaaggtcattggtgtcatcgtcggtgacatttccaacgtcttctcgtcactactcttcagtggcatctcagaggtcctccatccctacgattacagcgtattgcttttaaatgccaacaactcagccgacgatgagcaaaaggggattaaccgcctaatggagcagcgggtcgatggtttcatcattcaaccaagccaaacgacgatcgatgactatcagatgctgctgaaagaaaaagtcccactgatcaccgtcgaccgtgacttgggaaatgtgccagccagtgtcggtaaagtcatgaccaacaacttggccgccagtcagcaatttggcaccgaattgattgccgcggggtatcgccaaatcctgctaatcagcagcacgaccgtttcaatttctgcccaggccccgcgggtggttgggtttaaggctgccatcgacggcacccaaacgacagttacagaaattaacattgccggccacccagacaactggttgactgaacagattcaagaaaaagttgccaatttctcgggcaaaaccgtgattgtctcattgatggggccattattattcaaaaccctggcttcattgagatcccttaagttggccttcccagatcaagttggcctggccagctttgatgactggaattggtcgcaatttgtcggtaacgggattgatttgatggaacaggatcctaaagaaatcggccgtagtgcagccgccatgcttctgcaatcaattaaagatccggctttggtcctgaaaacaaaattagttccggcaatcagagtcgccggccattcattttaagttcagaacttaactatttgtcagttatgtcttggtctctcttgaccactgctatcgtgcttaagcatgcggcaatcggctgagccaagtcattaagcaaacaaacgagtcattcctaattttggaatgactcgtttgtttgcttaagttctgggatcgaaacacctcactcttttgttcgctacataaacatcgaaaccgctaagactgataacaggccggtcacagataacaccgacgtcagagtcgtccacgataagaaggtttctttcagtgtcaaaccaaagtattccttaatcatccagaagccagcgtcgttaacgtggtcagcgaacacggaaccggcaccgaccgctaacaccatcaatactgggctggccccagacgaagcaactaagggcgctaccagtccggctgcggtcagtgaggcaacggttgccgaccccaggctgacacgcagtaacgcggcaacaatccacgccgcaatcagtggtgacatattcatattggtgaagatgtcggaaatatatttggcaattccaccatccatcaaaacctgtttaaaagcgccaccaccaccgataatcagcagcatcatcgcaatctgtttaatggccgtgaccatcgattcactaatttcctgcatctttttatttcgggccaatcccatcgtgtaaatggcaaataccagggaaatgagcatggcggcgtccggtgcaccgacaaattgaatgccttcgttgattggattggttgccgggaggatgaatgacataatcgttgccaaggcaatcaagatgaccggcatcatggaagttaaagcactgatgccaaacccaggggtgtcttcaatctcaaattctttgaactttcctaaagtgctgatgtcaatatttcgtcggtagacctttggatagactttgtgcaaaaacatgttaaacaaaggcccagcgacaataatcgttggaattgaaacgacaattccaatcaagaggacttgccccagaggtgcgtgaagaattccggaaatggcagttggagctggatgtggcggcagaaaagcgtgtgttacgttcagcgtcgcagccatcggaattcctaaatacatcagcggcaagtcaagttctctggcgatcacgaagataattggcagtaaaacaaccaagccaacttcaaagaataatgccaaaccaacgatgaaagctgccagaacaacggcaatctggatgtggcgcttgccaaatttctcaatcaaggtgtgggcaattcgataacccccaccggaatcagaaaccaatttaccaagcatcgaaccaaacccaaagataattgccaaatgtcccagttgaccgccaattccagtttcaatactcagcggaatcttggcaacggggatctgcagcatcagggcaacaataaacgacgtaatgaccaacgacaggaatgtgttgagcttgaccactgtgattaagaagactaacagggcaaccccaatcgcaacaattaataatggcataatacatgcgtcctttcagatagtgcctgtccaactgaattcaaatcgattaatttctttaggtacgctattgaatttaatttatctgagcaaataacccccatccaccggcagcatgactccggtcacataatcagatgcctggctggccaaaaagaccattgggcccatcaattcttcaggaacgccccactcacctgatggaatatgttccttaatttctggaccgcgaaccggatcgtcttggagggccttggtcatgttggttttgatataccctggagcaagcccattaacctgaatgttgtagggtgccaatgcatccgcatatgctttggttaagcctaaaacggcgtgtttactggcggtgtacgggaaaataaatttgccggcccgataagactgcatcgatccaatgttgataatcttgccgctcttttgcttggtcatcaccttagcagcttcatgagacagatagtaaagggcatttaaattcaaattgatgaccttctgccagtcagcatcctcaaatgccagcacgtcattacgaatctgcatcccggtattattaaccaaaatatccaagtggccaaattgatcgatgacactttggacaatcttttccgccgcaccgacttccgtaatatccattttcaaaaagccggcttgttgaccattgtcggtgataatctggcggatctcgtcccaaccattttgcgtccggctgacgatgaagatatcagccccatacattgacagggcaattgaataattgcggcccaacccctctgcaccaccggtaattaaggcaaccttacctttaagtgaaaaactgtctttgtcaaaatttgtcatagtcatacgtcctttcaatgcttgttgacttaggtgtatcgatacaccatttgaggataatataaccgattaaattaatttagcaagcgtttacactccttcccgcaaaaaaagaagctgaatgatcagcttcccgtttgtctgcacttatagggtcattcccaactacagtatcggaaccacctgtttggcataatgaaacaccaaaacccgcttaaccgcaaattcgttcaccatgtatgaaccatcatcagagaggtaggcttgcttgtatggaatcagataatgaggatcccgatagcccttttccaactttggattacacttaactgccagtgccgggtgcccagcaaaggcaattctaactcgcactgattccttgggagacagtgacatgagcgcaatcagcacgacaacgcccacaataaagatgccaatatatttcaagattcgtttcagataaatcatattctcccccaattagtgccgccaacactatttttcgagtttctttttccccgcattcaaaacctcatcagacacatattcactggtaaaccgctgcagtggtgtgtactgatgccgatccttaaaagcaactgggatcgcttggataattccaaccatcaaattattctcggtgataaagatctggccgacctgcttgaactttcccttggtgtgtttgccggtccgccagctatgtagcttaaagtctccggattcgtcgcgtttgatgcgatactggccggagtcatcggtttccagtgggacgccgatgaattggttcacttcgtacttgcctttcatggaattccgccctttcatgactaatttgtgaataaagttagaattaaaatctaatctttttcaaaacacaacaattatagttattcatgctatacaataataatataataatttttcgaggaatggggtgaaatgatgaatcaaattaaacttgtgaccgactctgcggcccacttatcaaaaatcgaccttcaagcatacggaatttcggtcctgaatccaccaattattatggatggcaagctccttggttatgtcaacaaaattagcagcgagaagttcctgcaattatttgatcaatgttccaataagccgatcattggtgacgtctctgtcggtgaaatcactcgactatacaatgagttgggcgctgacggcagccagattctctcgattcatttaagtgataagctgtcgaatacttacgccaatgccaagaccgctgccagcaagtcgaccagccaagtcaccgtcgtcaacagccaggtgaccgccgccggactatcctatcaggtcttggaagctgccaaactcatcgcggcaggtaaatccatcccggacattttgccccaactcaccaaaatccgtaaccgcacccggatcttcttttcggtccgcaacaaccagcagatcgtcaacaatcgcatcatcggcaagcttcgcggcttcttgggcaaacacgccaacaccgcctacatgatcaaatttggcgataacgatttcgacctggttgcccatggttccaaagacgagtcgctcaacgaattctggcagacccaaatgcaagcgatgcacgacgaatgcattgttaaactaacgattctgcattccggcaccaacgcccgggcccagttcttgcgggaaatgctcaacgatgagttcccatttgtaccaatttccatcgtgccaaccaacccggagatgaccacctttattggtcgggagtcgaccggcgtcacctatttactcggataatctgctgttcaaaaaatgttatgtaaccaataatgaccgctaacgcaaattcaacgttagcggtcattttagatgttaatttacaagttaatctgcctcatgaattggctttcccttgcggacactctcccgttccactaatcgggtggcgacaacaactttttccggcgtgtgctcatcgttgtccaggttattgtccagcaagcccaacaagcgaaccgcaacggcgcccatcttgccagtattaaccttaactgccgtcagtgacgggatcacgtacttggcaaccgcggtgtcgttaaaactgactaaactaacatcgtccggcaccttcaccccattttcatggagcgccttcaaagcaccgactgccatggcgtcgttggaaacaaacagcgcgttggggaacgattccttcgaccgtttcagtgcttcgtcaacggtgtcataactggactggagggtgtaatcaccgacaaatacattggctggatcatacagggagcgcttttcgaggtagtttttgaaaacatcgaagcggtggtcggtaatcttcaactgatgatcactgctgtattcgacaccggagatcatcccaatgcgcttcaagccattctcaatgaagtatttcagtacagacttagtggagctgtcaaagtcagtgaccacacaatcatgtcccttggccaaagtgtcaaagtcaacaaagaccaggttgtcactgacttcctgcatctcctcaatctgggcatcactgaacttgccaatcgccacgatgccgctcacgtcgtcaatcgcagtcagcggatcgccggcaaaataacgtttgatcttataatgatcgcgttcggcctgcttttccacgcccatccgaatcgacaaatagtacaaatcatcgagttcctgctgctcggtgtaccattcaacaatcgcgatcgtatctcgagttgagctcgaccgcttcttttttgtataatccagcgcttcggccgcctcaaaaatcttcttgcgagtcaggtcactgacagataatgatttgtcataattcagcactcgcgaaacagtggtgattgaaacccccgccttgtgcgcgatgtctttaattgttgccatgatctcacccctccatacaaatactgcgaatttatgtatcgaatccttttagttaatttactaaaataaatatatgttctttaccttgatatgtcaaggatattccgttatattggcgtttttggctagtaaacttgttgacgtgtgcctggtaaatttctataattaggttgattttaaatataaggagggtcatgtcgtggacgacaaaattgaagacgcttaccaacaatggaccaatcaacctaatttaccagaaaatcttgtacttgatttaaataaaatgaaaaatgattcagatcaaaaaaaggatgcattcggaacggttctctcatttggaactgccggaatgcgtggcgtgctcggtgccggcaccaaccggatgaacatctacaccgttcgccaagctgctgaaggcctggcatcatttatggataccttggatgaagccacccgcaagcgcggcgttgccatcagctttgactcccgttactattcaaaagaatttgcccatgaatctgccaaagtcttaggttatcaccatatcccaagctttgtattcgacgacattcgccctacccctgagttgtcattcgctgttcgccatttgaacacctatgccgggatcatgattaccgcatcccacaacccgaagcaatacaacggctttaagatttacggccaagatggcggccagatgccaccgaaggaatcggatctgattacttcatatatccgcaagaacagcgacttgttcgctatcaatgttacgccagaacaagagctgcgtgaagctaaaatcatgaacctgatcggcgaagcagtcgatcaagcctacttggaaaaagtgcaaactgtcaacatcgaccacgacctgatcaaaaacgttggggccaacatgaaattcgtctactcaccacttcacggaaccggtaaaattatcgctcgccgggccttggaagccgctggtttcaagaattacgtcgtcgtgttggaacagactatcgccgaccccgaattcccaaccaccccatttcccaacccagagttcccgcaagcctttgatttggcccgcgaactcggtaagaaactctctgccgacgtgctgatcgcttctgatcccgacgccgaccgcttaggctgtgccgttcgtcagcctgatggcgactacaccctcttaagtgggaaccaaattgccagtgtcctcctgaactacattttggctgccaagaagaaagccggcgacctgccagccgatgggacgatcgttaaatcaatcgtttcaactgatttggcacccaagattgccgcttcgtacggggttgccaccaacaacgtgttgaccggcttcaaatttatcgccgaagccattcaccactacgaaaccgaacacgatcataccttcctgtttggctttgaagagagctttggttatctgatcaagccgttcgttcgtgacaaggatgccattcagaccgtattgttactggctgaagtggctgcctactacaagagtcagggcaagaccttgtacgacggcgttcaagaaatgttccagaagtacggttactatgctgaaaagaccatcgccaaggaatttgacggcctcgacggtaaagacaagatggcccacatcatgtctgaactccgtgacaatccactgactgaatttaacggccacaaagtcttgagtcacgcagattaccagtcatcaaaattgacggatcaagatggcaagcagacgaccattgacctgccgaagtccaacgtcttgaaatactggctggacgatgaaacctggctggctgttcggccttccggaactgaacctaaagtgaagttctacttggaagtcgatgacaagagccaggacgcagctgataagaaacttgccggctacgttgatgccgtggataagatgattgacaaattgatgaataactaaatttttaacttgaagctgcctgatctgaaaggattaggcagcttttttgccgtctaaaatgctacaataattttatagatcgtatctaaagtgccatccaagggggaatctacattgaaaccaaccactcaattgattgcgggggcgttattcatgctcggggcaacatttatccaggctcaaccagcccacgccaccgtggtcaaaaacagctttttgaaaacccagcgcaccatcagtacatacaatagcaacaagcacgccaaactcactttgcccaaaggaacggtggttcaagtcgccggcaccaagcaccttcatggcaataagtatgtcgacgtctatgtcgaccggttaagctataacattcgaaaaccgctgctctcagtaaaaaagccaaccatttacagccgctggattcgcgccaaaggctacaattttaagcaaatccacaaaccaacttatctgagctactacgctgcccagtccgacggtaagaagtcccaggggaaggtccgaaccgaaaccggcaatctatggaaagggacccgtttgccagttgactacgccacttcggctgccgctcgactacgggtgacgaccgacggctacctggaatacgatgccagttcgccatttgtcttcaaagtttcacccaaaccgaccgccagcctgaaagtcgaaaaggccagccacccaatggccagtggcgagacgattttgaccaccaaatcacgagtgaaacagcttccctttgttaaaaagtcaaaacaacattaccaattgaccatcaccaatgccgaggccggcaccatcaccgtcgttccgaatacctccaaggtcaagaagatcctcaccaattggattttcaaagttggtaaggagtcttggtatgaaaataacagcgtgaccacgtttaaataaagggggggaagcaccatgacaaaattcagattacaattcggactgtttgcgctgggggttctcttaacgatcggtgtaacagcgcccgcaaatgccagcacctatctatcgcatttttccaagaatcaatacctgatggccaagaagacgatccacaccaccaacagtcactataaaaacatcaaaatcaccattccaaaggggacggtcttcaaatccagcagcctgaccaagagccgcaaaaccaagcatccctacttaaccatcaatttgaaccgcctgcactggtcactgcgaaagggcgtcgtccagtcctaccacaacgtgacgaccaccagcggcatctgggccaagtccagcaccttcaaaaaagtccacgcaccggcttaccaaagttacttcaagcagccgtataccggcacgatcggtggtctgatctggcagggcaccaaggccttccccctgcgccagcagtacaaaatcgaaaactgcctgcgggtgaccgatgacggctacctggaatattttaccggctacgactactgggtcaaaaagatgccagagccgcattcggctgccaaagtggaaaagttggtgaagaagggtaacgcctattacttctacaccaagtcaaaaatcagcggtctgaccatgaagcacgttgccaagaagggcaatcaccgctaccgtttgaagatcaccaaaaccgaccagcacatggccaccgttaatccggcgcaagataaaaaatatgatgaaagtgtcaccatttcgatccgctattacgttggcggtaaaaagttctacgtcaatagtcaggtcattgaaccctaatcggccgtcaagatacttgcataccagccatagattgtgaataataaaaatatgtcagaatacttatttaacttttaggggaaatgattagattggaaaattcagtgacacatcgctattggcaggtcgccattcttgaagtgctggtatttggtctgttgatcgcgatttattcaaccgaattggcacttgggatgggcgaaatctcacagattgctgttcaggaaattttgttattagtgatcttttttgcgttaaattattattgggttaagcaacccgtcagattggcagccactgtcaactttggcaaaacgctattaatttcggtgccatttattctggttcttttatacttgctattaatttcactggccccgcacagcggtcataccatcgtgatggcggccgtttccggaatcggtgccggcgtttttgaagagtatttattccgtggattgattttaggcatcctcttgaaatcttttcctcatttttcaaaagccaaaacgatttggtacgcggtgaccatttccagcatcttatttgggatcgcccacggcagtaattttatgtcccaatccgtttcatcaacgctggttcaaattttcggcgccataagtatcggtttcctactcagtgccctttatctgcggtcgggatcaattatcgttccaatgctgtttcacgcggcttgggacgctactatcgtcttggtttcaggcagcaccttcgccaacgtcggctcgtcaaccttctcaccgctggcaaccgttggtgagttagtattgttcgtactgatcgcgatgttctattttcgaaattccaaactcaatgagattgatttaaaacattttgaataatggtctgtaaatcctggggtaaatcaaatgaaacaacgatcaaaagtgctgatgttatcaattggattaggcatggcgctctccgcgtgttcggcagggactcccgcttctaaaaaggattcggtcacggtctacgacgcgcataaccgccagatcttaactaccaccagccagtcaaaaatcaaacgcgtcaccaacttaaccagtcaaagtgaccgcagcacggtcaatggccagctaccgactggtctgcgggtcaaataccgctacttgctccaccagcgggcgcacgacgttaacatcaatctgtacgtctatgccaactcgcgaaatgtcaaaatgactcagatcccgattctgcatacgatcgtttatcagttgtccaagcaggattataagaagttaagtcagccggaggcgtatttaaagggattttgctggtggacaatgatagaagataacaaaaaactcacaactgccaatcgacagttgtgagtttttgatttggttattgttctaataggtggttaatgtgccgagaaataatttacggtataacttttgcttgtagggttgttaaagcggtagcagtcgtttttttgaatcgaggtgttgtgcatgcaacaaaaatccatccaagaaaggattgctctacaacattaccacgactctattatatcatgggtcgtggtaattttgtatccagttctaccggacaatgatccgagccgaacacatccgtcaaaatcttcgagtcctcaatctgatccgccaaccggttgctggccacaaagtagtcaatccgccagccggcattccgatcgcgggaatggaaccgataactccaccaggaatagatgtctgtctggtcagggtaaaaatgcctgaaagtatccatgaagccggcctttaaaagcttggtgaaatcttggcgttcctcatcggtaaagccagcgttgtggtgattagattgcgggttcttcaactcaatttctttgtgggccacattcagatcgccgcagagaatgaccggttttttggcatccaattcagttaagtattggtaaaaggccttgttccagcccatacgaaaatcgagtcgtttcagcccagccccagagttgggaacgtagctggtcaccagataaaagtcgggatattcaagggtgatcgcccgcccttcgtgatcgaactcgtcgctgttaatgccataggtcacatgcatcggtgcgtgcttggtaaaaatggccgtgccggagtaacccttccgttcagcataattgaagtattgctggtaaccaggcaaatccagctccaactgcccttcctgcatcttggtttcttgaatgcagaagaaatcagcatccaactgctgaaatgtctcggcaaagtcatgcttcacagcggcccgaagcccgttcacgttccaagaaatgaatttcatgtgatcccgtccttttttgttgttgggttaattataacgtaaatctggctgcagcgatttagcatcattactcagagcaatacttcatgtactaaaataatatatacattttaatattattctgatttttaggatcatttggtatactatggtgaatgccgttgtgctaatatggtaatggatgggttttcaaacctattacatataattattgagggacaattgaaaggggaatttttatgataaatatgaagcataatttgcgtcgtcatatcttacaagcagcctttacgcttgttggtgcagcaacgcttggtttagtggctgctggagggacagcatctgctgcggattcaaatcctgtcagcgcgaaaatctcgttctcagctacaattaatggaaacgaaaaggaacttgtatctgctgatcaatatagtaataatgagccagcagacccaagtctaagtgacgctacaccgattaatgtcgataaggcatccaacatcaaagaaaatgttgttgttacaaacacgggagccacaccccagaaagtatatgatgttcttcagctaccaagtctgggtgatatgtcttctgcgcctctaatcaacaattcaacggttggaaagccaactttctcccagccaactgatggtccattccacttaggatataaatatccatctgtcggtgatacttattcagtaacatatccagctaacgaaaacctctgggctgttcaaatcgggcaagatgtctccaatggatatattggtcctgaagagctaggtgccggccaaactctcaacttatcagttccgctaaaagtggacacttctaattctaatccttcacaacttgctatcgggcgaaattcgaaagatgtccaaggttatatggaggtaacatattcctctccaatcgcattaaagattgttcattcaatcactgcaaaagatttcaatgatgccaactataattcactatggtccagtacaaataaaggtgtcgttagtctttatgatgctgatggtaacgccgtaagtgatgtagcaaaagcaactgtcaagtcagttacgcctacaaataacccagctcagtaccaggtcatttacagctatgatggtgtggacagcattcccgttaccgcaactatcgccgacaaaacatttatcgatgctaaagattttacaattccttatggtagcaattgggattcacaaaagtttaatggtttaaccaaacatctcggatcagatggcaatgctgtaactccgttatcaaaagatgtgactgtatctaccaacaaagcagttgataccaccgccgctggtagtacgtatgatgttacttacacaattgacggcattaccaagattgtcaaggtaactgtaggtcaacgcagtgtcacaccaagcaacaactcaaacaataacaattcaaacactaacaacaacggcaactccggcaacagcgcctggaacccgtcaaacccaagcaacccaaacggaaccggcctaccaaactacgccgccgttaaaggttcagcggtttacgcaaccaagggtatctacatgtaccgcagtgctaatttcacgaagtcacaacgaactgccacttatcctaaggctaagcgggttaaccgcccaatgtttgttgttttaggctatgacaagtccaatggtggcgcccttcgttacaaggttcgtgacgttaaccacggtaagaagaccgctggcaagattggctacattaccgccaacccgaagtacgttgtcaacgtttactacaagacaatgcctaagagccaaagattaccgttattaacaagaaaggcattcacgcctacaagaacgcgaacttaaccggtcgcgctaagaccttcaagaaaggcactcatgtaaccgttaagagttttgaaaagcacaacctgaccacccgttacaagttaagcaatggcacttacatcactgctaacaagaaactggttattcaaggtaactactaatatgtaggaattaggaagtctcgaccttcgtcgaggcttcttttttgtggacttcctttgttttgaatcaaaataagggttaaaatacaattacaaccccgaaaagaggataatcgaaatgaaaacagccgtaattaccgacagtgccagccacctcgatccagtggtcgctgcccaatataacatcaccgttctgccgattaccatcatcttcggcatccaggaataccacgatggcgttgacatcacctcgcaagaattcctgaaaaaattggcggagactgacaaattgccgacaactgcgcaagtcaccatggcccaaatgcaggaagcctttgataccttggctgacaaaggctacgatgaagccatctgtgtcaacctatcatctggcatcaccaccttctacgagaacttagtggcctacagtcgccaagtcaccaacatcaaggtctacccgtttgactcgaaaatcgccagcgccggcgaagctgacttatgcttgttagcgggtaagatggccgaaaatggtgagaatgccgatgtgattatccccaagcttgaacagctgcgcgactcgattcatgtttccttagtcgtagacagcttggatcatctgcgcagaaccggccggatttccaacacctccgcattttttgggaacatgctgaaaatcaaaccaattctaacgtttgacgacgccggcaaaatcgttccagaggccaaggagaggaccatgaaacaagcgctccagcacatcatcaattccatcgaccagacgactttcgattcgccaatgcggatttcagtggttgacgccaacaacccggacttaagtaaagcctgggtgacagcctttcatgagcatttcccgaaggccagcgtcagcacctaccaaatcagcccggcgatcgctgtccataccggcgaaaaagccatgggcgttgtctgggatttggattggaatcaaatttaaagccaccagcaagtaacttgaaccggagtgagtgaattgccactcgcttttttattgccctggaatttgtctgagaagttttgagcatctgccattatttaaaagtccgatcagcttaactcctcgacttttgaagtatcggtattatttgcaaattcacttcagtatttgccatcgacttttaaaatatcggctatttttcaaaagtcagcatccaatcaagcgatgactttgcaaaaatcgccgttatttcaaaagtcgacattcaaagtatcaccaagaattcaaattaaattccatttttaactattgaatcagaaagagatgaaatcatgtccaacactaacgaaaaaatcagccggcaaacctaccttgccctgctggctgccgcactgctctcatttaccggaatcctgaccgaaacgtcaatgaacgtcacctttcccgaattaaccaaagtctttaacgtcaccctggacacggtccagtggattaccaccggctacctgttgatggtgacgattgtcatggcaacaacggcctttctgcttaagaaattcaaatcgcaaagcatccacttactggccgcgattgcctttgtggtcggcgacatcatgtgtgccacctcagcgaattttccaatcttaatgagcggacgcttaatccaggcgattgcgaccgggttgtcgacgccgttgatgttccacattatctttaacaaaattcccgcgggccaaatcggttcgatgaccggtctggctgggatggtgatttctttagcacctgcgcttgggccaacctatggcggaaccgtgtcatcgaccatgtcctggcggatgattttctggttgattctgccaatcatcgtcatcagctggtacctcggatcccgctatattcggattgatccagtcggcaccggcggctttgacgttatcagcctgatcttcctggctgccaccctgttctcatttgtcttcggcgtcagcaaagccggtaaatactcactgttgagcgggcaagtcttgatcccgtttgtcattggcttcattagtctggcaatcttcatctactccgacactcatggtaaaacccagctgctggacatccgaattttgaaatggctgtcgtcttcgctgtcggcgttcacctacttcgtcctgcaattcgtcaacattggcgtgtcgttcctgatccccgtctattgccaatacgttctccacagttcgccattcatcgcgggactggtcttgctgccaggatcactggttggtgcggcaatttcaccatatgccggtcacctcgccgacagcaagggatacgccttgccaattattctggggctcagttcaatgacgttgggcggcctgattttcttcggcatccaagccgtcttgacggcctggattgtcctgttgaactacaccttcctgcgttttggcttcaatatgggcttctcgaacaccatttccaatgccatgttaaacgtgccacggaagtataccgccgatgtcaactccttgttcagtatgattcagcaatttgccggctcaattggagttgggattatggctgcggtgatggccatcagtcagaacaatggtaccggaagcttggctgcccgttcgtttgtcggtggaaaatatgacttcctgttggcaaccttactgagtgcagccgcattgattgctgctgtgattaactttagactgcagaaacgaatgaaattgaatattgaagaatctgattaggtccttctaagctgaggtcgttgtgcaagtcgatttacttgcatggcggccttttttgagtgccattcatagttcaaattgccaagtctctttgattgaatttccccctcaatccgcttaaacttattttgatgattacaacaggttgtacacaaagtaattatcatgtcgactgtcgatcagaattgtaagggggatttcacttatggtaaagataggaattaatggtttcggtagaatcggtcggttaattttacgccggatcttggaaatcaacgatcctgatttggaagttgttgcgattaacgatttgaccagcccatccatgctggcttatctcttcaaatatgactcaactcacggtaccctgccatatgagatttcgtcaaccgatgactcactggtcgttgatggaaagaactaccgtgtttatgcagaaaaagacgcaagtaacatcccttgggtaaaggaaaatggcgttgatttagtccttgaatgtacaggtttctacacttccaaggaaaaatcccaagcccatttggacgccggggttaagaaagtcttgatctcagctcctgccggcccaatgaagaccatcgtgtttaacgttaacgacgatactttggatgccgacgatcaaatcatctcagcaggttcttgcaccaccaacgctttggcaccaatggcttacttcctgaacaaggaattcggcctcgaagttggtaccatgaccgcgatccacgcatttaccagttcacagatgattcttgacggccctaaaggtaagaagttccgtcctaaccgtactgcttcagccaacacgattcctcattcaaccggtgctgctaaagcaatcggcctggtaatcccagaacttgaaggccatttacagggccatgctcaacgggttgccgtggttgacggttcagtttgcgaattggtttcagttctcaacaccaaagttaccgctgaccaggtcaacgatgccatcaaaccgcacaccgttgataacccggcatttggctggaacgaagatgagattgtctcatctgacattatcggcgacacccacggggcggtctacgacccaactttgactgaagtaacctctaacggtgacttccaagttgttaagaccgctacctggttcgataacgaatatggcttcgtttccaacatggttcggactgccaagaaattcgccgaagtctccggcttgaactaatttaactaagcaatcaaaaaaatcgtcacaccatttattgagaaataaatagcgtgacgatttttattgtgcccgagttaagctgacagtcaaaacattatctttggtggtgctgtagctggccaagatgccgttaacgacgtcggcggccttgccatgactggaagttgagcgatggtaagtattaatccaagttcccagtgcttccatgccaaattcgaagccttcaaacacccgcatgtactccagtgactggggttttggtgtcacaatcgtgatcttttgtactctctggtcggcaatgaccatcgacaatttgatcacgtctgtgtcgaagaaaacctgagtcccatcagccacgctcgtcggcagtttgtaatccggcagctgaatgttttcgttgtacacccgtgaaacgtactcgtatgtccccaaatcggtggtgcctaattcttgtgtcacagaaaatcccccctagaagtgttacgtgacttattggtacttacactgattatatattggtttgggtatttattggcaaaattagcttgcagaaacgtactgttatggagggataatcgtgaaaaatccgggaccaaaagccagtaacttccttgctgacggcaaacaaaaacaccattgagattgacttctccaatggtgttatttgaactatttgatcactttgacatacttctgattagcagtcacataaccgcccttcacagcatagcgcatggttccggacttggtcagtgaagcttcatgactgaaggtataacgcttaatcacgagtttggtacctttcttgaagtgcccgtttcgcttggccaaatttggatcggcataccggttgatgaagtgggtggctttcaattggtgaggctgcttgattttacccatcttaaccagcttccggttaccggtaatgtagtggccgttgctcagaacgtaacgggtggtcaaattgtgtttgacgaaaccggttacgtgaagaaccgttccctgcttgatgttcttcactttgcccgtcaaattcttgttgaggtattcattaacaccgcggggattgatcaccgtcagtgtttgatgactgctgtggtagtagacgggtcgaacataatcaaagttggtggtaatatagccggtccagccgtcggtcttgctcaagtggttgacgtcgcggactttgtaacgcaaccggccagcattggacttagcgtaatcagtgaccacaaacatcggtcggaagacccgtggcttcttgacataaccaaattgacgatcggccttcttgaaggttttatctttgtaaagataaatcttcttcaaggagtaaaccacttcgcccttcttagcaatcttaccggattggttgtcagtagtcgttccgggagtcggttgtggactcggcgtcggcgttgggttgaccggtgttaccgggttaaccggattaattggtggattgaccggagtcactggggtttgtttttgcttgtagtagtaattcacatcaggtgtcttgtcgctgtacgtcccagtgatattattcggcagtctgtcagtatccaaagtgtaagtctgcccattaacggtgagtgtttgtggttgataggaaccgtcggctcggtatgaatcgttaattttaccgtagatctttttggattgaatcagggcgccggttgcttcattgatgtagttgacagtgactgtcgccgagttatcggttggggttaccggagtggcatcctttttgtagtaatagttgactgcaggtgcattttcggtaaacttcccgttaatattatcaggcagcttagccttatccaaagtgtagctgtcgccgttgacggtcagcttgtctggttgataagggccatcagcttggtaactgtcaccatttttgccatagattttcttggattgaatcaaatcgttattttcttcgttgatatagttgacggtcactgcggcagagttattggttggcgttaccggggtggcatctttcttgtagtagtagttcactgctggtgtttgatcggaaaattggcctttgatatttgccggcagtttgtctttatccaaagtatagctgtcaccgttaacggtcagcttatctggttgataagggccatcagcttgatagtcgccaccgattttaccgtagatctttttggattgaatcaagtctccggttgcttcgttgatgtagttcacgtcaactgtggccgagtcgttggttggggtcggcggtacgtcctttggggtgtagtagacattgatggtatcgtctttgcctaagacgcctttgactaccggctgatcggctgtgtagccagctatttccggagaatcaatttcgtaggttcccgcaccactggccttgtatggatcagccagcactttgttagtgcccttttcgaggtagttgatagtgagttgatagtgaggtggtattcagtgatgggttcgtagacaaacgttagtgggttaccgacgggtaatggcatcgatgccgtcgcataggtccgaatcatgccataactgaaatcagcagcgataaagccacccggcgtcgccttaacagtcacagtcttactttgagctttgccagtaaaactaaaatcgggaatcttcgagtaatcaaatatcatgtacatctgttgggtattttggtcgtcgattacttttctggcaatcgccacgtaccgattagattgctcaaattgccaatcacctggtgtcgtggccgtaatgttattgattaaaaattgatgggcgttattcatatagggaactctcacaagtcgatagccaggaatggtggggtaattaacatccacaaaagttcctgaataaccggagatattctgggttggcgccaattcgtttcctttggcatcaacaaattttgccggcacattatttaaataattaagcggattggcggaacttgacgcatacagatcattattctgtaaatccaactcaatatgaccattttgccaggaaaattgaacattaccggcattataggtccagttgggattgaaatcactcgccgttggccctggaacctcaatcgtattcgtcaattttccatcgctatcgacgttatgcagataaaatctcgagttgtccttggcccagccgatcatccaggcattagagccggtgtaataagcatagttgatcgtttcatctggattgggtgcttgaatataatcattagagttgatggttccctgtgtatcggaaattgtctgggagcccactttcgcattggtgcccatttggttggccaattttccggaaacgtagacgggtgcttgatgaaaaacacttcctttgtaaaaattagtcactggaatatccgagtgttctttaggatcaatcgttgggttgtcagtcttatcagccggatcgggcgccttcaccactttcatcggcgtcacaatcgtcccgtccggtaccgcatcatcagcaacttgcgtggtcgcggcatgggccacatcatttgaagtcatcgtcgaatctgcgttggcaaacgtcaggattccccctgtgctaatcacgagaagtgacattagcaagtatttattgactttcatattcgtattccactttggttattgttgctattagttatcttatatatccaaacccattataacgaacatatcccagaaatgacattaacttgcttgccgcaaaagacaaaaaaacgcccactttgagaagtctcaaagtgggcgttaaatcggcattttaatcgtataaatcacttaattttttctgaacgtctgggtgattaatgaactcatcgtaggttgtatccgccttatcgatcagaccgttgtttgatacttcgataatgtggttggcgatcgtctgaatgaactcgtgatcatgagatgtaaagatgatcgacccggggaagttcaccaaggcctcgttcaaagccgtgattgattccaaatccaagtgattggttggatcgtccatcagcaaggtgttgcctttttggagcatcatcttcgatagcacgcagcgaactttttcgcctccggaaaggacgttgacttccttgttcacatcatccccagagaacaacattctccccaggaatccgcgcagaaaggcgtcatcatcgctgcccttttcagcaaattgccgcagccagtcaatgatccgctgatcgttatctttgaactccgaagcaaaatccttcatcagagcagacatctcaaccgtttggccccatttgatctcaccactatcaggcgtgagttcaccagccaaaatctgcatcaaagtcgtcgttgccaaatcgttacggctgaccaaggcagtcttctcacctggacgcagagtgaaggtcacgttatcaaggatcttgacaccgtcaattgacttggagagcttgtcgactctcagcaagtcattccccagcggccggttctcctcgaacttgatgaaaggatactttctcgaagacggcttgatgtcttccagggaaatcttgtctagttgcttttttcgcgaagttgcctgcttggatttggaagcattggcactgaaccgggccacgaaggcttgcagttccttgatcttgtcttccttcttggcgttcgagtcagcccgcatcttggcagccaattgactggactgcagccaaaagtcgtagttgccgacatacatattgatctcaccaaaatcaacgtcacacatcatcgtacaagtctggttcaagaagtgacggtcatgagacacgatgattgtaatcttggggtagtcagccaagaagttctccagccattcgattgagtagacatccagtccattggtcggctcatcgagcaacaggatatccggttcgccaaataaggctcgggccagcaataccttaaccttttggccttcagtcaactcgctcatcaattgttggtgcagatcttcaggaatttccagtgactgcagcaattgtgaagcatctgattcagcgttccagccgtccatttcagcgaattcggcttccaaattggcggccttgatgccatcttcgtcggaaaaatcagctttggcatacaaagcatccttttccgccataacgtcagccaaatgttggtagccttgaatcaccgtctgcatgacggtctgatcttcaaagccataatggtcctggcttaagctggaaatccgctcgttcttatcaatgtggatttcaccgctgcttggggtcaattccccccgcaacagttttagaaaagttgatttaccggcaccgttcgcgccaatcacaccgtaacagttgcccggcgtgaattttaagttaacatcttcatagagttttctacctgagaattgtaatcccatgttttgaatcgtaatcattgatttacctcgttcaatagcctgcgcgcagtcgcgttcaaaaatacaccgacagcccacgtttcccataatcaaaaacaatggccagggcttgattcgtcctgaccaatacatgtcttacaaatatatcatattaatagaagagaaacaactagacctcgccgagattgttgaagtactcaacgtcaatgtcatcatcagtgatgatcaacttggtgacactgccgttcttggtggcgacacccagatccagtttcggcgcgtaacggtcaacaattgagcggatcgtcatcccgtgggagacgatcaggatatcctcgccgtcatgggtgttttggcgaattttatcgaatccgtggtcgaggcgctcccagaacatggcgttattttcagcattgttgtacaagtcggcccggtgaatcaagtctcgtgcccgctccaagccaaagttggtcaatacttctttctcggtggtctcttgaacttgggcgccgacgaactgccacatttgattgagatcgttgccttcgaaataaccgtgaaattgttctcgtaattcgggatattggtaactaacaatattcatgttatgcggattagctttcaaaataatttttccggtgtcgattgcccgaccggagtcactggtaaaggaagcggcaaaattaatctttgagagtcgtttcccagcacttttagcatcttgaattcccttttcagtcagcggagaatcaatccaaccttgaaccttgttgtacatgttcaagtatgtttgtccgtgacggaccatgtaagcagtaaccttcgtcaaaaaatcatcccatttctcaaaaatttgcttttacataccctaagtatagcggacttatcatggtttagcattaaaagtcactttgaatctgagaaatgtgaacctgccgccagactggctttcactgccagcttcttgttatacttatggtagaaactgaactttacttataaagcgaggtcgttatggacactttaatgaattttgctccctggcagcaggcactgttcgccacattattcacgtgggcagtcacggcactggggtcggcattggtatttgctttcaaaaccatccgcagtcacgctttggccttgatgtatgggttcgcagccggtgtgatgattgcggcatctttttggtcgctgttggatccagccatcaacttggctgagcagcaggaccggatcccctggctggtcgttggtattggttttgccgccggcggattctttttgtatctggcagataaaatcattcccggaatttatttaaaacgcgctcgaaccgagggtagttcccgagcgacggttaagcgggcgattctactggtcttttcaattaccctgcataacattcctgaaggtctggcagtcggggtggcctttggggctatcggtgctgccggtaatggcgaacaggcggcaatgctgctggcagccacgacggttgccattgggattggcctccagaacttcccagaaggcgcagcggtttcgattccactccgtcagggcggcatgagtcggttccgagcctttatgtatggtcaagccagtggtgcggttgagccgatcgccggggtgttaggcgccctgttggttgcttcggtcaactcgctattgccgtacgccctgtcgtttgcggccggtgcgatgatctacgtcgcctgcaaggagctcatcccggaagcccacgccaggactaaggaagaatctcactgggcgatctttgggattatggctgggtttacgttgatgatggtgctggatgtggcgcttgggtgatccatcagaaaactaatattttgcatttttgaatgtcacatcatttacagctcagtatatatcagttattttggtccgtatcggaaattttcaaataactttggattccagctgtaccttgatgccgtttacctttgctagataatagacagtatcgccagaaccttggttatttgaaagcaacttaatatggatccgcttcgtccgatagtaactttgacgtagcttaacattgattcttctttttacgctaatttgtatcgtggaattatgcccattatttttaaattccctagacaattgttcctgagattgtgattgaacaacggaatccaaggcaaaaaaataataacaattgtatacaagtataagtcctattgcgacatatactattgcaattaaaatcgctacttgtcgtcgtttcataattttcctttttttacaaagaatctaagttgttttatggtgataaggtcttaaaattagaattttaggtcaaatacatcttaacaaaggagaaatatatcaacaaggtaaaatgctttttcttagcacttgcaacacttgtaactctactcgttggatccgctccagccttaggagctacaccatcatcttcggaagacgattcatccccacaaattatacttgtagctacatattctgtttcggatttggacaacgataccttaagcaatatacaaagtttgccactagagtatcccaacatttcagtcagattactcaataatcaacttcgtgttgaaatgaccatgccacaaaatgattctgagcaaggaacacctgatttgctgagttcaaataaagatctcagttcaagcaccagcgttgcatcaagctctccgaatgtaagagtactagactattcagatgtcatacagaacatggatgaagcaaatggagattcaaatactcctaatggaacattattaggtgcatatccaggccaaaatgttggtgaccatgtttctactggaacccacgtgcattgcaatagatttaacggtccaaaatctgaccatcgatactggagtcactcaagtgctaaaggacttgctgactttgcaggcagtgactgttattggcatcttgccgaatatgggtgttatgagtattccatgggacgttgtgacggactcaatcataaaaataaaggagttcatgattgctcttcatggtcgggtggattattccattcaaactggcccaaaactgcctggtacagataatattgctttccctatcagtcaacagaagggcatcaaatgtgaggcccttttggtgtatcccctttgatcatttgtttcgatcccacaaatcaactgccccgattgcaatcgctagaaccagcagcacaacaatgatcggaaataaaaaataatttcctgagatcacctgctgaataccgggaatcaaattgacaacgaatagcactgccgcaagaattattaacacggaatggcgatatgtaaacaagcgaacaattccaccaactacgttcatcccaccggcaaatatcagccaataaacagcggccatgcccttggatattggtaacgggcccagcgaaaagatgttgagaaagatcgcaataccgccaattagaatgaacaataagccaatcaaaatctgtgataacttcctgctactcgtttccatgttattctcccccaacagataagtatgttgctagaactgcatctaactcataattcagttatatcgctaatctgtcaaaaaacaagctcgaggaacggaacatcacttttgaacttcaggtcgctttctacaatcccaatcaaaaagactttgttactgaacgctaatcagttcagtaacaaagcctttttagacttcatcattaatgatgcggatactgatgcccaatctcatacaccatctcaggctcttggctgatccgagtgttccggttcaacccatccacctgttttatttcatcttcgctcaactcaaaatcatagatgtcagcgttctgcttgatccgttcaggatgaactgacttgggaatgaatgaatcaccacgttgaaaatgccagcgcaaaatgacctgggcggctgatttaccatgctgattggcaattctgacaatcactggatcatcaaaaatccggccgcgacccaacggtgcccatgcttgagtgacaatgtgattttcacggtcgaaatcaatcatagcctgctgtgagaggtatgggtggacttccaattggttgacgactggcatctcattagctttggttgccaaatactgcagatgcagcatgccgtagttgctagtgccaatcgacttgaccaacccctgctctttaaggctttcaaatgcccgccaggtttcaaagaagtgggtgtgaattggccagtgaaccagtagtaggtccacgtaatccaactgcagtttcttcaatgattcttcgactgaagcaatggtctgatcgtatccttgattctcttcagcaaccttagtcgtgacaaaaatgtcctcccgggcaacatccaagtctttgatggctttgccaaccgcagcttcgttgccgtacatttgagcggtatcaaacaaccggtaaccatcatcatatgcggatttaaccgacttaattaattcatcttcatcagtcatccgataaacacccagtccttcttggggcatcgtatgaccgtctgctaatttgattctactgccaatattctctttactcatcaaaatcctccagtattaattaagatgttttaagattctggctggattgccgccaattaggacgttgtcaccaaacgattttgtaaccaccgctccggctgccaccacaacgttatctcctaatgtgactcccggaacgattgtcgtgttgccgccaacccagagattatctcctattgtaacattcccaggatattcataattggcgatccgttccttggctccaaggggatgattgacagaataaatcgaagtgttcggtcccagcatggcgttcttaccaattgtaatcttaccaacgtcgataaatgtacaaccgtaattggcaaaaaagttctccccgactgaaacagtgtagccataatcacattgaaagggggattgaatatccaccttttcaccagtttgatgaaaaatttgcttaatcaattggctcccttgctcaggatcttggcgggcaacccggttaaatttatctaccagcaatcggttacggtgccggtccgctgccaattcgtcatccgtattcaggtaccgttctccagctaacattttctctttttcactacacatcatcaatttcctcctatatataagcgctatgtacaaaacgaggtcgaggcaaacgcaaatttgtctcaacctcattttagttttatgaagtcccgtccgaagcctctcgggggctttgttgttggactttatgttgagtaatctctcggggttactcgggtggtcgttttaggctacctagtcgaaacgtgttccctggggcaacaacctacacctaagccggttgtcaaccccccagctcacactctgctgaaatgtgttccgtgagccagatgctaacttctaagtgcactttaattaaagtcccaaacccagggacttcaatcaaagtacccttagaaaacgcatctcccggctcacttcacactgtgctgaaacatgttccgagcaactgaggctaacttctaagtgcactttaattaaagccccaaacccggggacttcaatcaaagtacccttagaaaacgcctcacccgttgctcttcacactctgctacttgatatcgttaaacgtcaagccaaacatcgtagctaagtcttggaattgtgtctcagtagcattgaatgtcaagacagtgtggtgtccaccaccatcatggatccattgagtagcaccattcttcaagcccatctttggtgtccacatttgttttgcaactggcagatgtggagttggctttggagccttgtgaccttcaacagcgtaaccgatcatgcggtattcattaccaaagtctgagatggtaacatccattgcgtcaccttcacggccggtaaataccaaacgtgcaggatctgctttgccaccaatgtccaatgggtgaacttcgacacgtggcttgtcgctggaaatgccagggtcaacttcaagcatatgtgatccaaggatagcttcttgacccttttgtaattcaagagtgtagtcttccatgaatgcagtagcctgattatgagtcatgattttaactaagcggtcaagggcagctgtcttccagtcaccttcagcaccgaagccataaccatcagccatgagcaattgtgctgccaggccaggtaattgttccaaaccataaaggtcttcgaagttggttgtgaatgctgagtagttacctttgtctaagaagttcttgattccgaagtattcacggatttggtaacgaactgagtgctcgtacttgtccttgtcattgtcgccttgaacaaattcgtacttgtcttgtaattccttgtacttggcatcaatatcactttcagaaacagcgttaactgattctaccaagtcgccaagtgcgtagtaatcaacagtccagccaaattggatttgggcttcaactttgtcaccttcagtaacagcaacattacgcatgttatcaccgaagcgggcaaccttgatcttgaagctttcgtcataagcgacagcaatattttcccagtcagcaatttcgtcttgaacttctggatcaccccagtagccgtaaacaatcttgttgttcttacgaagacgagcattgataaagccgtattcacggtcaccatgagcactttggttaaggttcatgtagtcaaaatcaatggtgtcatatggaatgtgatccaagtattgagttgccaagtggagtaatggcttttgaagtaacttagtaccacggatccagttcttagctggtgagaatgtgtgcatccaagtgataattccggctactttatcattgtagttaacatctttcattaattgagtgatgctgtctgcagtggttgcaaccatcttgaacacgattgggtaaggtaatttgccagaagcatttaacttatcaaccatgtctcgtgcatctttttcaacggatttcagttgttcttctccgtaaagatgttgactaccagtaacaaaccaaaattcataatcaggtacttgtaacatagttttctctcctcttgatgatttattatttttagacaaaatgtctaaaattggttaactattttgtaacgtttgacgcaacgtcttctccggcagccttatgaaggtcaagttcgatctcttcaagtgacttaccacgagtttcaaggaacttgctgtggcatacccaaatggcaattccacagataactgcgtagaacaggaaagcattgtccaagccccatgagctaagcatcattgggaaggtcaatgaaacgatcatatcagctgcccagttggttgctgaacaaagtgatgttcccaacccacgaatgttcaatgggaagacttcaccaatcagaacccaggtaactggtgcccaagttgttgcataaaaggcaatgtaaacggtcagtgccaaggcactcacaatagcggcaacgtgtgatccattatcgaacttgaggacggcgtacataacgaccagtgaaaggcccattcctgcagcaccaaactcaagcatcttcttacgatcaactttatccatcagtaacatagcaacaacagttacgataacgttaacaacaccgattccgatatgggcaagtaatgcggcgataactccccagccaacatcagtaaagatggttggcgcatagaagataacactgttactaccaataacctgctggaagatggcaacgccaagtccagtaatcaatgcgggacgaacacccttaccaaataattctttccagccgccaactggtgctttggcagtttcttcaatttcagtaagagcaacatcaacggctttggcatcatgcttgttggtgtccatcaggacttcgcgagcttcgtcagtcttaccaaccttaactaagaatcgaggactttccggaaggaaaagggctccgaagaaaagaatgaaggcaggcaatgcagcgaatcctaacatccaacgccagccggtatacagatgagcaaatgagtagttcaagatgtatgccaacaagataccaatcataatcatcagctggaacattgtagcaaccgcaccatgcatgctctttggtgccaattcatgcaagtaagctggaatcaatgctgatgtaataccaacaccaatacctaataccacacgggtagaaacaagtacccagaagtcaggcgcaaatcctgatgttaaagctccaatgaagaagataaccgaagcccagatcaataatttacgacgtccataagtatccaagaacttacttgttgccaaagcaccgataatcgcaccgattaatacggaactaacaacccaaccttgttgccatggtcctaagtgaagttgcttttcaataaacagaatcgcaccagaaactgacgcaatatcgtaaccgaagagcaaaccacctaaggctccaaacgtatatataaagccattatttgtgacctttttcaaaacgagcaccccattcgtattttattaaaccaattattgcaaaaactttgtgcgcacctgtaaacggtttctgacatcgcttacaaaaagagtataaaatatttatacgcataaatcaagatatattttatttgttagcacaaaatttttctggaaaataaaacacggacgggaaatccgccgtgcatcacctcctttcaagcgaagtgatcttggaatttattttctaaaagccggattaaatgcttttagtggaggctcgaacaatcagatccgagtctaaaatttttgaactgccatccttgccatccaacatatctaataatagttgggcagccgtgtggcccatttttcgttttggatgatccatcgtggtcagcgttggatcaatatattgagaaatctgataatcatcaaatcccgcaaccgagatttgatccggaacttgaatgccttctttgcttaacatcccaatgacttcaatggccaattgatcgttatagcagacaatcgccgtcggcagggcattcatctcaacctgaacccgggtcttgatcttatccaagacgtcatgaatgtcatcgctggaacgatacatcatgatatcgcccgaagttgagacgttgggatgggtctggtaggacttgatgaaaccgttcattcgatggacgccttggagatcatctacttgaaagacccccaaaacccgttcatgaccatgatccaacaaatagtcgaccaaagtcttttcggcatccgtatcgttggtttcaacgtatgggaaatttaattgtggataatgggcgttaatgaacaccgccggcttgccggaatcgacaatcatctggtagacgtcgaggttcgggttgtccaaggtacttctggttggttcaataatgaagccaaccacatcattgtccagcatattcaataagttatgacgttctttttcatattcatcatgggtattcccaatgagaatcgacaagccttcatcagagatcacctgatcgatgccgctgatgatgcttgggaaaatataattggcaatgtgagttgtgaccacgccgacgttttgattggatcggtcagaagagaccttattgttgatccagtcgtttacatacataccgccgccttgaacccgataaatatagccttcatgctccaagtcgccaactgcacggcggaccgtgtagcggctgaccttatacattgccatcaactcggactcggtagggattttatcgttaatcttgtatttcccgttaatgatgtgtgatttaatgttcttcttgaccatgacgtactttgtttccatgatgagatccccccgcgttcaaattgataagtgttctacgttaacattaacaagccaaaagtaatgaagacacaaacgattgcccagataccaaaatggtgattgggcttcgtctgatcttttctggcgaattcatacattgccataaagataaaagcaataattaataaatcggtaatccccgataaaacatacaaaattgtcgtcataatataacctctcgaatttaaataaaatactccagtaataaaaatatcatactttgagtaaaatttatatagaattatacggataaattaaaaaattggtattgcatcaccgtacaaaaacatattataatacagataaaagcggtttcacaaccgtaatttattttcgtaaggagaaagatgctatgaataccaagaaagaattgttcgataagttagatggtcaagacattgaaaagttcaccattaccaacgatcacaacgtttctgtttcagcaattacctttggggcaaccctggaagaattcaacgttcccggacctgacggcaaaccaaccaatattttggtcagtgtgcccagcagtgaagaattgatgaagaatcaatacttctgccaagcaatcggtcgaaccgccggccgaatcaccaacggtactttcaagatcaagggtcaggaataccacgttgattcaaacgaaggcaccacgactttgcatggtggcccccacgggttcaacacccaaatctgggacggatcatttgatggtgacaccatcgtcttcaccaagcacatcgactcttctgaggattcattccccggcaacatcgacgtcaagattactttctcactcaataacgataatgaattaaccgctacttacagtgccaagagtgacgccgacactttgttcaacccaacccagcatatgtacttcaacttgagtgagggtgacagcatcaacggccaatcacttcaaatcaacgccgacaagtaccttgaattgaacaaggacaagacaccaaccggtaagaaagtcgccgtggatgacaccccatacgacttccgcgataaccaaaacctcaaagtcggtatcgccgacatgaaggccgaagttggtcacagttatgatgaagtctttgaaatcaatgaccatcaagacgacgaaccagtcgcaaccttatccgatcccgaaagtggccgcagcatttcgatcagttccaagcgcaatgcattggttgtcttcacaccggatgatttaaccggcaccaactatctccgcggaaaaggcggcccatacatggcaattgctttggaagcccaaaacttgccagacacccctaaccacgaagactttggtgatgtcaccttgccagctggtgaagaaaagacctacagcattaagtacaaggttgaattctagacccatcattaatcaaacatttctcaaacaactcaaagagctccagataagaacgaaaccgtccttatctggagctctttattgatggaaaaattcacttgttagccaattgtgctctgtgcttgctgcttctcatattcacgatcaaattttacgaggtaaatcacactagcgaccagaatgacaccaaagacgccgataatcaccaaccagttcgttgcatcaggtactgcgcccgaagcaatatcaggttgccaatcaatcaagaagtgcagggcaatcggccagatcaaagtattggtcgtcacgcgaatcacaaccaacaagaggcctagcacgactgtataaacgacttgctgaatcacgccttcgatgttgtcctgactcatattcatcatatgcaggccgccaaacaccagcgaggaatagatggcagctttggtgaatttcagggaacgccggtggttcttggcgttttgtaggaaggcggaaaacaccaatcctcggaccagactttcttcaaagaatccggctgtcagagcaatcagagtgttaaccacaacgtgtcgggtcgtcaaagtggtgacgacggtcgctggcaactcttccagtaacagcatcccgatcaccgtggcagcaaaaattgcgaaccacaccttcaaattagtggttaatttcaaccgggtggttgttaccttatacgttcccacctccacgtacacgaaggcaaagacgatcaaaccataaaccagttggatcaccgaaaaaacaattggtgccgtatgttgaaatgccagcatctcaatgacgtagacaatcaggaagaaaatcgccatcacgatttgttcaatccatgaccgacggcttttgataatcaataaaatcactactttctcaaaaaatgttgactacctgccgaaatgtttaaaagtatcagcaggcagcccggtgtaacagaatctgccaccgttgcgcatgctgagttccccctcgctttgcatgccataattagtaattacgcaattttctttcgtgatttttatttttttgatctgaaagccaaaaaatctcctcaggctaaaggacttcctttaacttgaggagaatttcatttgttttatttgaaacaatcgaccgatctatgagtcttaaagggctgcggccacatcccggaccattgccaactcttcattagctggaattaagaggattctggctgatgaatctttggtgcccaagtcgccgggcttttgctgctcgttaaggtcgccgtccaatttgatgccgaaaatttccagcttcttaacaacctgttcgcgaacccatttgtcatgctcaccaatcccaccagagaagacgatggcatcgacaccaccgagttcagtgatgtagctggcggcatacttaaccgttcggttgacaaacatatccaaggctaatttggcacggtcatcatcagagtcttccaaatcacgcatatcagaggaaacgccagagacgcctaataggccggaacgcttgttgaacatatcaatgacttcttcagcactggcacccattttcttcataaagaaaggtaccaaggctgggtcgacatccccggaacgagtccccatcacaagaccgttcatcggcgtgaaccccatcgaagtgtcataacacttgccgtctttttcagcagcaacagaagcccctgagcccaaatgaagggtcactaatttagcgtggtcattgcccaacgccttttcagcttcttgtgtaatgaaaccatggttaatcccatgttcaccatagcgacgaatggtaaatttcttggtcagttcatagggaatcccgtaaatcgaattgacttccggaacgtctttaaagaaggcactgtcaaaaatcgcatactgatcagtgtccggcaaaattctgcggataatttcaatgtattcagcttcgactggattatgaatcggcgcaatatcgcccaactcaacaatttgtgacaaactatcatcgtcgattttgacgactttatcaaagatgtcacttccagccacaactcggttaccgattgcgtcaatatcccgtaaatgatcgatgacgccaagatctttaagattgttcaacataatccccgccgaacgctcgtaatcaatcttatcttcttcggctttatagacttcaccgtcgccatacttgattttgactttggagccgggcatgttcaaccgctcaacctcaccgtcagcgagcaccttttcttggggcatttcaaacaatttgaattttaatgatgaacttcctgcgttgacaatcagaactttggacataatcagtacctccgttgtttttattggatatttccattcgaaatgaaaacgtaaccacaactaaaagtatactatttgttaggagtttgtgacaatattagctattttaattttccaaaatcactaccaaattgggtgaatcatcgcacaaccaaaaaagcgccaatccatttcgcgcaaccggcagaaacgaattggcgcctcaatccaattattcatcagtatctgaaaattcacgttgatactccgcaattccttcatattctttagaaagatcgcgactgagccgcagataaatcggcatcagggttcgataacgtttaaagacgtcctcgtttggttcatacacggtttccttgcccatatacttcttaatgtcttcaaggttgtcttccaatcccaaagccattttggcaagaaacatcgctgccaaactaccactctcgtaagattcaggaatgacaatattgtgctcgaagatatcggccatcatctgggtccaaagagttgaccgcgcgaatccgccggcagccagaacggccttgggttcgccggtaacttctttcagtgccaaggtaactgagtacagattgtacataatcccttccataaccgcacgaatcatgtgggcgcgggtatgcttgcgattaaggccgaagaacgacccgcgggcattggcatcccataatggggcacgttcaccgccaaggtatggatggaaaattaagccatcagacccagctggcaccgtggcagcaatctttgaaagcatgtcgtaagagtcgatgtgcagcagttttgctgcttcaacttcaccgccaaacagtgaatcatgggcccagttgaggacaatgccaccattgttgatcgggccgccaaccagatacttgcccttcatgactgggtagcagtacaaacgggctttgggatccacccgcggtttgtcgacgaaggtccgaacggcagccgaagtcccgatgttgattgccaggacgccggtttgaatcgcgccgacaccaatcgttgataatgcgccatcagtagcgcccatgacaaaatagacgtccttgtcaatgccaatcactttggcatactccggcttaattccttggaatttatcagtcgtatcaaccaactcaggcagttgtttttcagtgaggccggtttctttgagtgcttcctcgtcccattgggcagaattcatgttcaacaggccggttgcggcagccattgagacttcttctttgagcaccccggtatacttccagatgatatattctttgatgcccacccaataggcggcctggccaaagatttccggtcgttcatttttaaaataaagcaatttgtagaaaggtcccatcgggtggattggcaaaccggttcgtttgtacatttccatcccgcggccattctgtttgtattccgccgcatacttctgggaacggttgtcagcccacgtcaacgacctggtcagcggcttaaagtccttatccaaggcaatcaagctgtgctgttgggcagaccaggaaatggcaatcactttgccatccgttatgttggcttttgccaccacttcctgcatggcagaaaccgtcgcgttgaaaatctcatccggatcttcttcggccatatcaggggtgtcttgataaagcggatagcccttattggccttgccataaatattgccgtcggtatcataaatcagcgctttggtgctggtcgtcccaacgtcaattccaataatataatccatcatcacattctccgtttcaggttctcgggttgtcatttatataaccggaacgcgttaatcgtccaagttatgagtcaactcacgtcccggacgtttgccggcaacaattgccttaacatcgctgacacatttttcgcccatgccgtgaagacattcataagtataagcagaagtatgtggcgtaaccaggatccggtcgttcttcaagaatggatggtctgccttaaccggttcaacttccattgcatcggcagcgtagccggagagctgaccagacttgatggcggcgctgatggcgtcttcttcaaccagggcaccacgggcattattacaaatgtaagcacccttcttgaggctcttaatggtcttggagttaatcatatgaaggctggtgtcatccagagaagcattcaatgaaatataatcacagcggctaagcaaagtttcaaggtcaacgcgttcaacgttgttgttggtaaaccattccggttcagttgccggatgtggatcgttgactaagactggtccaccaaagatactgaacaattcagcaactcggctgccgatgttaccacagccaatcacaccaaatgtcttaccactgaattcgttacccatgaattgggcacggtcttcataacggccggcgcgttcgcgttctgatgaaggaacaacttggcgaaccaaggccatcaaattggcgagttcgttttcagcaacggaatttcgttcaaccttttgtgggacgatggcaacttgagtgccatgttctttggcagcgtgtaaatcaacgttgttaaagccgattccgtgacgggaaattaacaaaagttcatctttgttatcgaagaattctttgttaaagaacggggtcacactggcaataatgacgttaaagccgtgaagcttttcagctaaagatttaccgtcaatgtcggttggcagcatgaaccgcttaacagtcccaatgccttccaattccttccaatgctctgtgaagacctgaccaaaactatttgaattaacaactgcgatattgtattccatgatgttctctccttaattttaaatcataattgttggtgcactaacatactagttctgcgatttggttaatctcgatcaaagaaatggaactgatcgtgggcattattatatgaaatatcttcaacaattttgcccaagtaatcttcgtcatctggtgcttggccacgttcagcccattcaccaatgacattacataagacgcggcggaagtactcgtgacgtggatatgacaggaaactccgcgaatcggtcagcatgccgacgaagttaggcagaagactttcttcagccatgatcgtcaactgtttcttcatcccgctgaaggtgtcgttaaaccaccaggcagctcccaactgcagcttttgaacgccgtcttgctggaaatcacccattccggttgctaattccatccagtcatttggattcaatgagtaaatgatcatcttagggatttggtcctcttcctgcgcatccatcaagagtttcatgaattcctgggccaaatcaggctgggttcccatggagtcaaatccaccatcagtcccaaagctcttcagcatgggcttgttagcgtttcggatgacattcatgtggaactgcatcgtccagttgaattctttgttcagatgcatcagggcttcaaccagcatggtttgatactggtcgatttcagtcttggtgagttgcttattattgcgggctttgtcgatgatatcgttcatttcatcgtctgaagcttttacaaagtggaagaagttgagaccgtggtctgacaatcggccgcccaggctttcgaagtactggaaccgttgccgaagggcgccaaccaggctcttaaatgaagtaatctttttgccggaaacttttgcaagttggtcaagataatcgccgtaaccgtcatcagtcaagttgaacgccttgtccggacgcattgccggcaatactttgaagccattttggtcttcttcttttttgagcaacttgtggtacttcaaatcagaagcggggtcatcagtcgtgcagacaacttgaacatttgaacgcttaatcaaattgcgtggtttaaaatcatcggtggctaacagctgattggccttttcccaaatggcaggagcggtcttggtattaaagacatcattaatcccaaagaaacggcgcagttcgagatgagtccactcaaacagtgggttgccgagggctttttcaatcgtgccggcccatgcaagaaacttctggtaatcatcgccgtcgccggtaatcaaatcttctggcacaccatttgcgcgcatcaaccgccatttataatggtcgccaaagttgccttcgttaatccaaattcgactgatgttcttgtaatttttgttttcatagatttcctttggatccaaatgacaatggaaatcgatgatcggcattttttcagcatgatcatggaacagctttttggccattggcgtggtcaataagaaatcatcattcaataatgacatggtttgtctccttagttaatttgtttagcgtactttgataacgtgtcttcaagcgtcttgcgaactgcaccaaccccgctgatttgtgaggtaaagtagccttccacaacgtcgcccaggccaattccatataagtcatgaccgaagatcttctgattggataagatgtctttcaagtgggcatgaacgtcggtcttttcgccgagcttaatgtcttggacctttggttggagttctgccaagagtggatcgcggcttggttcaaatggtttgccttggtcgtcaatggccatcaggtaacggcaccaagttgcgagaacgagtggaatgaagtggaggtcttttggatcacgtttgggatcatcaatgtaatgctggatggtgacgccataacggattgacagcttctgtgacgtgtcggcagcgattcgctgcggcatatccggaatgtatgggttaggcagacgcttgttcaccaactggtcgataaaggtcttggggttgataaccttaggatccttaacaaccggcagcccctcaacgtaaccaatttgtttgatcaggttcagcatgtctggatcgctgacttctttggcaattgagtcaaagccaagcaggctgccgttcacagccaacgcggtgtgcaatggattcaaacaggtggtaaccttcatctcatcggcatcattgacggtgtcgcgatcagtcagggtgacgccagcgactttgtccaaggctggccggccatttggaaagtcgtcttcaatcaccagataatgaacttcttcagtgttggtgaaggcagcgatattggtgtggccaggcgtatggaaaatttgatagtcttcaaagccgtcagccttgagcttttctgaaacggcttctgaaggattaggcgtaattcggtcgatcattgacaatgggaagctaaccttgtggtcgtcttttaaataatcaacgaaggcttcaggcaccaacccgttttcctcccagccttcagcgatagtcaaaacacttttttcgagtttttcaccattttgagagaagttatcagtgctcagtaaggccattgggtatttgccggctttaaagcgggcaaacatcaaagcagtcagggaagccatgttattcttgggggcctctggaccgttcttgatatcatcttcgatggctggcaataagttacccttgctgtcccacaagttgtaccctttttcagtaattgagaaagtcgccaactgaagagcaggattttcaaaaatcttgaatagtttgttccaaccatcgggattgctttggtcaaagaacaaggcatcggcaactgaagcaaataattctttttcaaagttaccatcctcgtgggtaatcacccggagaattttatcgttaaattttttataggcgtcttggacaacgtccttgtcatgcgtttcagcaacgaccacgccggcatccaaatcaccggattcaagcaatcgatcggcaatagcagcgtggaaagctcggaataagttaccgccaccgaagtgaacccattttgtggcgcccgttttttgtttaatatcataagttggaaccttaattccagcgtcagcaaacccctgttgattgttcaggtaatcgtcagtaatttttaccattaattaaacctcctgtattgcgttgcgtgagccaaacatgaacgtatgccagctggcttaaaacaaaatagtacaccagtccgctgaatacgctttcggttttattatattctgatatatcagattgtcaataccccagttttttcaaggatcttcgttaactttttcaccaaaatatgctaatatgatgatatctaaaggagacttattatgttggataatatgcgcagtgacgcttacaatgaaattaaatatcgcatcatccacttcgactacgtaccgggacagaagatttccgagaagctgatttcccaagagttaaatcttggccgaaccccagtcagggaagccatcatccgtattgaacgtgaaggtttgatcgaagtgatacctcagagtggcacctacatcactaaaattgatatggcagatgccaaaaatgcccgctttgttcgtagctgcattgagcccaagattatggtggacgccgctgtcaatatttctgatgaggccatcgccactattcagaaaaatttagatcagcaacagcagaccgcccttaagaatgagccggataacttctttgatctggaccaggaatttcatcacgctttttataaggtcgtcgataaggatacggtttggaactggctgcagattaataacacccagctcaaccgattccgccgactacggttgaaggaaactgaattggattgggatacgttaaccaaccaacataccgcaatttttaatgccgttaagaataaggatatcgacgatttgagcttcctggttacccagcatttgcatttgatgctgctggaaaagcaaaaggttgtcgatgcgtatccggattatttcaaaaattagtgtgcgacgagcaacgggtgatgcggtttctaagagggctttgattaaaacccctgactttggggatttaatcaaagcccttttagaagttagcatcagttgcgtcggagcatagctcgaaagccgaaggaacctgtcaattccataactcctgcctacctatgacaggatattccttggaaaaagatcgacataaacatgattggaaaccaaagagaatcagaccatgatgaacgttttattcatcgtggtctgattcttttttgtacagtaggtccctgggtcgtcggagcatagctcaaaagcagaaaccccagtaacttccaccccaaaacagcctcccacagttcatttgcctcaacccttacgaatactataatgataatagcatcacaagggggggactcatcatcactaagaaacaaaaaccataccgaaaaacatcgtggtggctgctaatcaggtcactattactgtcaccgctcatcgttggttctgttggcgtctacggaataacttcgtcaggttgggctatgctgccggcattgttcttgaacgcagtctattggtatcgctacaatcgcaagaatcaatttgccaattatcatcgccaaatttgggcattgctggttgccttaatttactatttcggttcactgacggtcgttctggcagccgcccgttacagctacttagacacggccatctattatccagccgccatccttccatataacctttctgccctatttttagcatgggggctgttctaccacaatctcggctggatgtttgtcggtaccttttggtcggcagtcttggggattttcatttatcagtggcaagcaaaggagctgccaaagcttcatcgtggtcaaatcatgggattaatcatcatttttttaatcagcggtttgccgatctaccaaaattttgcaaatagtctgaaatatactgatacatacggttcaaactcgcttaacttgaacaaataccggccattccgcaatagcagatcgctggcaaagttgaaccacccaacgtcggtcaaaatcactgccaattatccgcggttaaacggtgcaaccgccctttatcccatgtattcagcgattgcccaaactctgtatccgaaggtgtcaactaaacaaggatcacagctggtaagagttgactcaacgcctaaagcctttgatagtctgttaaccaaaaaagctgatgtcattttcatggccagtccgtcaagggcccaattcagaaccgctaaacgacaccacgtttatttaagattgactaaaatcggtaccgaagcattcgtcttctttgtgaaccaaaaaaatccagtcaagacgctgtcaactggacaaattcaatcgatctatcagcgaaaaaccatcttctggtcaagtgtcggcgggcgatttgcttctatccaaccgtttcaacggccagaaggttctggcagccaaacggcgatggagcagatggtaatgaaaaagcacaaaatggtcaagcccttacgctatcaggaatttgacgccatggacggcgtgtttgatggggtcgctggttacaacaaccggaccaatgcgattggctactcatttagatttttcgcgacgcaaatgatgcacaacagacaagtgaaattattgaaagtcgatggcattgcgccaactgcaaagaacatccgcaatgggaaatatcccctcatcgcccatttctacgccatttcacgtgaccaaccatccaaaaattctcaacggctaatcagctggttgagaactgatgatggccaaactttgatcaatcgaaccggatatgtgggcctcaagtgagtgacacgctataatcaataattgaagggggattatcatgcacaagaaattcacgctggccatcctggctgcggggctgctgacagggtcaatcgtttcaattcagtcaacaccgtccgccagtgccaaaaccaaaattaccactaacaaaacatttaaaaagacatcatttctgaccaacactcgcaaatcagtctacgtttggaatgcgagttacaccaagaagctcgccaatctgaagaactacccacacactaatctttattcgacaaagcgggtcacaattcggacgagcagctattatggtagttattactatgtcaaaagtgccaaccataagatcaaaggttacgtttggcatgggagcttagttcccggctcctacattaaaggtggcggctatcgctatccaaccaaacatgtgttaatgtcgagtaccccatacaataagaaggactggtccacttccaacgacatccgtcaaaccgggcgggtatttggcgtcatgaatgcgacttcaatgaagccatacctcaaggtgccaaccactagtcaacaaaagcaggttatcaattttcttaaaaagaagaatccaaacgttcccaagatgattgaaaatcgcgtttctagaggggtccgcatctcaatgatgaaactatatatcagcggccaaactgttgaactgccgatgattgaaacgtatccttatcattattggatggacgttaattcattctatccagttctccaactctccaaactgccaaatcgagcaaagccgatcaggacttacagcgatgccaagacggtcacaacggtctttggttctcggacctacgactttgaagatccaaccgcccaatccacctcgaatatggaggaaggtcctatcaccaaggtatacggcaacggctatggcccgaaccatgatctttccctggtggattgtcgggatcgcctacgttatgtcacaaccaaaaatatcatcagtatttccaacaaccagccaactttacgcgatggcatttggtacgtggcaccgtcctaccaatttgtcagcattggcggccacgaacaaaagttaaggaacttaattgatacctcaaaatcgactgattatcggtatgtgactccgaacggtttcacccaatacaagtacgagaacaacagttggaatcccaaatttggtctcagcttcgattttcaaaagaacggtgatgtgaaagtcaccatccatcagctatctggaacacttaaccatccaaaaaccgttggtgatccacaaacgatagccacattaaccggggcaaatgccgacgctgagatgatgacttatttgaatcattcagctgggtggtatgatcagtacttacaatagaatccgatccaaaaacaagcgctcagaatttaatctgggcgcttgtttgctttcaattataaaaatgagttacttggcagcagctgtgttatctgcttctttagcagcggcagctttgcttgcttcatcaccattaatcatgttgtatttcttttcataatggatcattgcaaatccagccaggccgaagattgcaacgataccaacgaatccccacattgtcatcttgatagtacttggaaggaccaacaatggtgtgaacattgctaaaattccacaaaggaaacgtgaaaccccattgataaatccttggatacttgcacgaatttcttcagggaatgattcctgtgtccaaactttgtaaatagcttcacctgagagcatacttccaacaccccaaacgagcatgaaggcaacgatcaaggcaatcgaagtggctccaaagattgccagaccacccattgcgatcagtgcaaagataacgccaagggtgaaccaagtatttcgttttgcggaaccagcaatcgttacgtagaagcctaagataaacagcgcagcgatgtgcagtcccaaaccaataccagtcgataatgtctgtgaggcaccggctttaacgaacatgaaggttgtgaattgaccgaacgtgttggcaacaaagttccagaaaatgtagtagatagcaattgcagcaaataatcggatgtaaatcttgcttcgtgaacttctaaagagtacctgaataactgaagctttttcggttggcttttcgtccagttgtgcttctttggcagctaatcgttctgcagcttctttgtggagaacacgaattcctttggtgaatgtccgccatacccaaagaatcaaagcagtgatggcgaagaagccaaacacaattcgtccaccagtaacactcatcgtagaaacaacgaaggcagcaccagttgaaacaaattgaccaacttgccagaaaatttgagttgaagcaaccatttcagaagccatcttctggttaggtgcatccctggaaatcaccgtcaacgatactggcaggtcagttccagaagcaaccccacaaatcacaacccctgccagtaacatgagatacccgtttgcgaagacacaaataccggcaccaattgcataaaggaaattcacccaatcaaagattgccacaatcccaactttatcggcaaatcgactcccaaaaattgatccaaaagcaatggcaaaggttaacgcaccggaaataatcccgacttgaccgttggttaaattcagtcccatctgccagacggtaatcgtacttgccaaaccaacaataattcctgaaccaagcatcgatcccagaccagccgagacactcaagttccaatatcttcctagatttttcataatcctgttctccttatcgtccattccaaggacgcatcaaaatatttaacttacaacaatattagttggtacgatatgagatttgataattgccggatcctaaaacaatctgaccagtcttcgtaagcatcccctccaaatcagttccattacgatcttgaatcgtcattaaatgactaccatcaggcagtatcactgttccctttgcattcattggaacgtggacagtgacaatctgttcatcggttcccactgttagagtggccttaataatcccttttgctgatggcgtttcaacgctcacacggtggaggctgcccggccgaattttgacactaaagttttcgaatcccggcttggttgggttgattcccataatcccttgcacgatcgtcaatcctggggtcgctccccacggatgagacatcgtcatattaggtttatagtgattgctccaagcctcaggggcaatcgtcgccttcaaagtattcaagatggccgcaaacgtcttttgatctttacggtcgtctgggttagttaggagacgtaccgcgtcatcggcatgaccgctgtcgattaaacctttgagcataaagtaaatgaagtagatactgccaacaaatttgccatcattagcgacaaatcggctcatcttatcggccatctgctgatcggtataaacgccatagcacagtgcataagctgttgcgtgatgagatgtatgcttattaatcgaaaggtctttattcatcgagtcgtagaaacgaccagttttggggtcatacattcgattaattaattcctttttaatgcgggcagcccgacttcggtaatggtcggcatctgcgtgatgcccaacaacgtcagcaattttactcatgctcagataagcgccatagaaaattgcgttgaatggtgtattgtactcaccttcgacaaaaccatcgcgttcaggaatcggccaatcaatcaacccatcgttggtaacaaggccaacttcttcgtcaaagttgtcaacgcctttggtatttttcaaagatcctttaaagtcttgtgaagcgccgtcaaaactctcttcgtttttcccgcgattaagcttgtaagtcaaatcagtatatcgattcttcaagaactcatcattaccggtgtagagataatcctgccaagccatttcaatactgtagagcttgtaatcttcgggccacgttggattatcaattaagtaatccatactatggcgattgagcgagtatttagatgaaacaacgaaactggtattgccgttgactaacagatcaccttcgtacggccgtcgctcacgggcttgggaatcaacgtaaacatcctggttagttgctttgatcgtatacttggacatctcatattcgcggttgagtaggtcattatcactgtcaaaggcggattcttgagattcaaatggttgctcaatcgcccatccatcaatatcattttcatttaggttgccttggaagccaaccagttcaatatagcggaagtttttaacctgaagagtagtgaattgattctgtcccttcacaaacgtccagttttcaacataatcggggccagctgctagatgatgacgaacgtgtccatcatcttggagctgctcacccatcaaaatcgtgacccgttgattaagtagactttgaagattaaccttaagacttccaataatttcttttcccaagtcaaccaggtaatcctgatcacctaacttgatcacctttttacttggctcatgggtttcaaatcgccgggtattttcactacggtaaggaataaaaacttcctcatcggaaaccatcgattgtggattaacccatactgccggccagttgtcatcgttatattcgacctccgaccagccttgtgggtagtagcgcaaatcaacattttcagacaccatgccgaaatacaagctgcggatttttacaccataatcgccaaaggccgtgctaccgtctaaaacgtgccaatttttgtcggtcacgattatctgcttcttagtcccatctgttaggtagacttcgagtttgcaccagaaggcttttcgattcgacttggcagttgccatgacagaaatgacgttttcaccattgatcaattcttcagtgacatcgtatttgttatagtaaatcccagttttgtcagttccttgataatggacttgacggtgagccgatccaacaccaacgttggtaccattcaccagcaaatcaaagccttggataaacagtggctcattacccctggaaaatgcggtgataaccgccgtatcaacatctaccaggttaagatcaaagcgtggactacgaataaaaacaacgtttcctaatttgggcagttcattatccgacttaggcccacgatctgcccaaatcccatggatcggctctacttgaggcttatcagtactgatgaatttttcgggttgggaaaaatcactgatattgttgaaattatccttgatccgaacttgccaataatacagctccccagcatccaagacctgctcaatttgaggaattgcaacacccgtattttcggaggattgtacccagcccgtatcaaagatatattcttgattggccaattgatgaaggcgtttggaaatcaccacctgataggccgtttgttggctatttgaaatattgctgtgatcccaccagctgaatcttggggacttatcgacgttgtaaggaaaccgtaataagttcacgttcaggtgagtaggaattaataattcttgttgattgttagtcatcaattattttcctctctaaaacttcatttatcgtcgggccaaactttgtcataaggaacaccggttagatcagtaacagtctgggcaacctttggctcaacatctgcctttttaccaccatttcgaagcctggtaatctcttcaaggacaatttgatgtgtctgtttgttaagtttgaaggtcaaagcttccaacaatgccaggataatcagtccgccagtcccaaagagcaggatcgctgcaatggcgtgctgagcttgaggcgactggctggcggcattcttggcaaagccgttactgtccaaaataaatccaactgcaatcgttgcgacagcgacagttgatttacgagtgaaactcatgacagccgcaaagacaccggcacgtcgacgtttagtgacaatttcatccaagtcgggaatgaatggaaagacgttccacggtgtgaattccaaggttgcccgcccaatttgatagaacagtgaaatgaagaataaaatcaagatcacatggttggtgacgtgcagctggaatatcagatagtaacccacaagcatcaacagcattaacccgtaaccgacttcatacaagaacttcggtccgtatttgaccattccaaatccggcaacgattgtaacgaccaacccaattaatgacagtgatagcatgttggctgcaaccgtcgctgaaagtcccagacaataaatgcagaagtaagcaaacacagtgttgaaggtatcttttccagtaaacgagaataaatagatcaacagatgctttctgaagctcttaattcgaagcgttgacccatagtcacacaggagtccccagaagcgatgaagcaatgagccttcattgactgaatctttctcaagctctgcgcgcatttgaggagtaactggtttttcccaagtaaccgcgtaacaaacgtaaacgccaattgcaaaaataatcgcaaataacgttccgtttactaagaacgggatggggctatgctgacccatgatggcaaataattgtcccggaataaaggttgccaagaaagttgccccagccgagatgaacattctagcagatgataatttggttcgctgattataatcatccgtcatttcatttggtaatgtttcatagggaatcatcatcgcactggaaatgacttcaaaaatcatataagtggcgaagtaataccaataattcatccctgcgatccacagcgtaatgtagagcaacataagtggcgaaccgattagtaagaagaagtgccggcgaccaaatcgttgccccaacttcgtcttataaaaattatcggtcagactccccatcaataaactacagattgcgtcagctacccgggcggcaccaataattgaggccccttgaacggcagttaaattacaatatgatgtatagaaaaatagcatccacgcaccgatgatggtcatcgaaccaccaccgacaaaatcaacaatcccataaccaatcccacgccagacggtgatctttcgtggggtataaactttactttgttttgccattgcttaaatctcctattctgaattcgttaactaaacgaacctcgtaacctcctttgcaaaaacagttatctggtatatcaatctgatatatcaactgtattaaggttatcttgtgaacccagatcggtcaataaagcgtttacaatctctataataaaaatttggtatatcgggggtaagccttgatatgtagggaattattcgtgatttgagaaattattcagttagcaacagatatgtacatttgatacataaactaggcagaaagcgatacgacttcacaatctttttttgactcttgaacaatccgagctattttctgggtaaatgaaaaggcgtctgcttaacaccgttattagtttactaaaaactagtaaatattggtaaattagcggttaaacagacgtcttaattcgtaaaactatttagtttgaattttctttccgacttgatccaggtgccattttgtagtaactgatatatttcttatagaaaaaggtccggtttttaatccctacctccttgataatcttggaaactggtagagtagttgacttaattaggatattagcgttgatcagccgctgctttgtgagaacatttgagaatgtatcacccacctctttcttaaacaggttactcaagtagtttcggttgtagtcgtacttcgcagctaatttttcaagagaggtatccttataattaccgttaatttctttgagcatttggacagcaatctcctgagattttgacattggcttattcatatctactttgtagttacgtaccagctgagcaatcaaaatcgaaagataggagctgatgatggtatcggcaaagtctcgctgtaaatagtattcctcaatgattcgatccaaggtctcttgaacctcgctctcatcttcgtgcccaaagaccaagtaatgaatcggactgtcatcgccgattcgccgattcaataaaaattcgtacaaaacgcttttactacttcgcaggtcgcttaacaaatccaggttgatttccttgtcgcggaacaagacattaattaataggtcattggttcctagataaccaactgaatgtttgcaaccaacatcaaggagtaaaacatccccctgctccaagtgaatctgttgtccctcaacaacctcatcacaagaacctcggagcatatagttaatttccaaaaaagtatgagcatgagttgggtacggcgcataccgattatgcttactcacgtaaatgctcttattcttgaacaaagcatcactgatgatcggcgttttttcctgttcagataaggttgtatcatagacatctattggcagatcattatgaaattccaggcttttcaattgttctttttccagcttcgtcggcttcatgagtgtatttagaatggtatcaagcatattattcgttccccttcaggtgatattgctatcctatgataacgcattcaaaagaattaacatattgatattgtcaacgaacctctttcttatgtaagaagaaaatcgacatttattatataaatatcatatatacagcccggtctattaattatctgttttgaaaaggcaattgcaaaacgtgtcactttaattatgtatcatttgtacatctgtatttgaaaacaacattttttaatataatctattaaaaataacaaatgtttctcttgtctacatattggacgtgctattcaagccagtttttgaggatagctcctacagccctgactcccagctttactgttatctagcggaaacgtgcgcctgcagcccaacccctaacgtataagaaaagaaggccaacaatgaacgagttcatcattgaccttcttctcttatacacctgtatcttcactattatctagcggaaacgtgctattcaagccagctttctccgcttaaccaaataacgggtagtaatgtgcacaacccgcacattactacccgttattccgttaatgctttaatactgaattacctcagcctttgaggacagctcctacagccctgacccctaccgtgtaacacaaaaaagccaacgatggacaaagaacgtccatcattggcttttccgcgttacactccggggtcaacccgggcttagtcgctcacttattttttcatatccatcgcatggccaccgaatccgtgacgcaatgctgatacgactttacctgtgaatgtatcttgttccattgaacggttacgggcgaataatgcgtccgtgataactggaactgggatgccttgcttgagggcttcttgaacagtccacttaccttcacctgatgagaacatcttgccgctgatttggtccaagttagcatcgttagcgaatgcttcttgtgccaattccatgagccagccacggataactgatccgttaacccaaactttggcaacggcttcgttgtcatagtcatatgggctgtggtccaagacgtcgtatccttcaccgatggcttccatcataccgtattcgataccgttatgaaccatcttcaagtagtgacctgaacctggcttgccagtgtaaaggtagccgtctttttgtgaaataccgtcaaataatggcttgatgtgctcgaaggcttcggcactggtaccaccgatcatgaagttaccaccgttgagggcaccgttcttaccgcctgaagtaccacagtcgaagaagttaatgtctttgtcttcggcaatcttaccgtgacgaattgaatcttgatagaatgagttaccaccatcgatcaggtagtcgccctttgaaagaaggccaaccagttcagtaacagttgagtcagttggcttgcctgctggaaccatgatccaaacagtgcgtggtgcgtccaacttgctgacaaggtcagcgttgcttgatgcaggagttgcgcctgcttcttgagccaatttgatgtttgcttcgtccaaatcaaatgcaacaacttcgttaccgttacggatcatgttcttaaccaggttaagacccatttttccgagaccaatcataccaatttgcataagtattgtacctctttcgtcttatatattagttagttacttgtctacgatgcttattatatattttgaaaagaattttcgcaagcattattgataattattttcaaaaagtgcgatattctttgaaaatatcatgaaagccctttctaaatgccgacatgttggggttctatatgaaaatcatttttaacccggatgcccgttgaataacctcattattgaaaatgttttacatatttgatttcaaccgccgccagatggcagtcccagtcagccccagcagtccgacaatcgtcagcaatgctccggctagtagtcctctgatgtgatagttaaaggcaatttggtgcctaccaggcgtcacacggacacccaccaagccgccagcaacctttttaatcggccgctggtgcccatcaactttggcctgccaacctttatcaaatggaatggtcaacaccagtgtttgagctcgtttgccaaccgttacatgccccttgaaatgcgcaccatgttcattgagctggcttgggttttgcaatttaaatttatggttgtcctgatagttttcaacctgcctgagtttggcgagatcgattccgcccagatcgccggcaacgtgatgcagttccttggttgaatgaatcgtcagggttgaaatttgacccttttgcatatatcccatcgtaatcatttccgtccccaagccactatacaactgagaaagtttttggccattgatatagaacgacacgtttatcaatctgacccgtggaatgtataaataatgcggtccggtggtgttagcccagaacttgactttatattcaaaatagtcgcgatgaacgaacttggcactgctaatggttgttggcgcgtacacatactgacgttggttccccgccgttgcttgaacaaaatcattcaagttgtcaaaggcttggccccgtttcaacttgaggtcttcaatctgtcggttggccataaatcccagcccagacgttcgttttctaaccgttaaatgattcccataacgtcccaggacatcataatacttcagaccaaagaaatagttggtaatcgccgttccgcccagcatatcaatccggcgaatgttgcgggtcgaaaatcccaagtcgcctaaaacatggtgagtgtgggcattcaaagtggaactatacgaactgatgccatgatttcggtataggaatgaatcgttatacccgctatagggcaccttgaacaaatctcggaacggtttatcaataatcaagaaacgatagaagccatcatctgattgatatcgcttttcaacgctcccgattaatctggtggattgcgcgtaagtccgttcaaaagccttttggttgccaagtggggcttcatcggtggcaatcataaagttcaagctcaactcaaatgccaagacgacacccaaaaagattcgactggtccaccgctgcctgccaacgccaatcatggcaatcgtcgtcagaaaaatcaggccgaccacgaaggcaaagatgatgttgcggacagaaagttggggaatatcaaaacgaaattccattaatttttgcccttcaatattggcaaaaatatacccaatcaaaatcgctgctccaaggccgaccgccgaacgaatcaacaacttctcttcggcaaacatcccctgcagatagccctcataggtcaccatgatgatcgcaaagctgaacagaaagaccattctaaacggaaacccagccggctgctgcatcatgtgccaaatggtatttaacggtaaaaaccacatcccaacaaagataccgccaatcaagataccggcagcctgcttatcgcgctgactaaccagcttggtgaagaagtagacaatcgctccgatgataaacaacgagccggtgaagaaactgggattatgtaccagccggccggcgaaatcattgccaccgacgccgagattgaccggaaaactgaggccaaacgttcctttgaacagaaagttggcggccagtaagtccttcttcccagtagccatcatcgcgatggcagtggggatcagaatcacggcaacactcatcccagctaacaatgaataccaaataaaccaactaatcttttgccaattggccttcaggttttggaaaaatggcaatgaatagggttgattctttttaagtaagtaggccatatacagaacattgaagatgcagatgatgtatcccatgtagaagttggtgaaaataatcatgatcaaactaacaacatatagcgcagggttcccgtgataatagagtttttccaatccatagaccatcaccggcagccagatcaaggcatccagccacatcagatcataaaagtacatggccacaaaaccgcacaagccgtatgccaggccgccatagactgccatcaagtcatagttttgatattttttagccaagaaaacactcatggaaatggaacacaaaatcaatttgatccaaataatcaaatcaatggcgatcggcagctgagccgttccaaacagcatgatgattaaattaagtgggctcaacaaatagtaagcatagattggcaccaagctgtcgccaatcgacatcaaaaaggaatacccagagaagctgaagtgggccagctggtgctttaattcagcgaagaactgcaggtattgcgtcgacaggtcactgaccagtagattgtggctgccaaacggggcaattccaatcaccacaaataaggcactgaccaacaaaattggaatcagcaccgccaaaatataaaacgatcgttttgtctgacgaccacgttgtgacagcatatccgtccacctcaaatttgattttcgatgcgccgaaaatcgatttcgaacttgaattcagttccaattataactgtttgcttggataaatctttcattagagggattgattttaggaactattaaaaaacgtcaatcttttgttacacttgacccccttaacctgtaacaaggcagccgattgcactgaatttgtcctgtaatgcgggcaaattgacaaatatatccaataaattagccgcttttttcaaattagattaccgtaaccattgccgtcaccacgcgactcacacaaatacgaagaaagtgtgaaatttttcttaacatttatgaaacaatcctgatactggttggtagcattcatttcatataattgttcttgtaagtttttagaggaggactattcatgacattgaaatttaaaaaaatagccggcctattaatgggtgccctggcagcatttacttttgcgacaaacgcatcagctgccaagacaaaaattgctgatgtttctcagtatcaaggaagcatcaactggagcaaagcctccaagcaattaaaatttgcgatcatccgggtccaacacggtgacaccggcgatgcagatttcagaatcgatactcaaaaagatatcaacgctaacggcgcatataaatataaagtaccatttggtcaatatggttacgcagagttcagcagcgtggccgatgccaaaaaagaagccaaggacttttacaagcgatcaagttccaaagcacgtttctacgttttggacaacgaacatcgaaaaggtaagggttcggaacaatcctacgtcaacgcttggctggcacagatgagaaagttaaccaataagcctttggtttactactcatatcaaaactacgtcaacgttcacaaaatcaactattccaagtttgatggatcatggattgcaaattattccgctaagccaaacgtttcaaccgacctttggcaatacacttcaaagggaagcttaagcggaatcagcggcaacgttgatttgagcaaggtcgtcgacagctcaactgttaattcctggctcaagacttcatcagccgatgcggctaagccaacctacttcacatcactaccaagtgataaagaagtcacagcttccaaaaacatctatcaatatcacgatgctaatttcaaaactcgggtttcaaagattactgctggcaagaagctttcagttaaatcaatcactcgttcaaacggcggcgcttatcgcttccaactcactaatggaaattacatcacagctaataaagcatacgtaactgactaatttaactaaacgacgaaatataaaggagtactcatcttgtcacacagtattattaaatcagctttaaaaccattattgttgctcgcagccttattcgcattcgctgtatctgcttatacttcagctaatacagccagtgcaagctcttcagaccaatcatattcaaaggtcttgaaggttgccaagaaacatctcggtgccagctatgtttacggtgcagttggtcctactcactttgattgctcaggtttcaccaagtacgtttataagcactcaattcagaagtcaattccaagaactgcccaagcacaatacaacggtaccaagaaagtttcaaagagcaacatcaaaaaaggtgatttagtatacttcggcggcagcaagcacagcatctcacacgttggtatgtacattggtaacggtaagatgatcgattcacaaaaccgcggtgtgattactgaaaaagtttactcaccctggtggcatgtggttggcttttcacgcccagctactttgagttacgatgactaatctatttatatcaatcgttagataggaaaacggatgtccgggtgggcatccgtttttttagtttgtggtgtttggttgtgattgatgcttgaaagtaatttgcttttctatagtgaaaacgtgctcccagagccagctttctccgcttagtccgataacggcagtcaacgcaaaacgagcgttgactgccgttatcacactaatgctcaaaagctaaccggctcttgtcgcactcttagaagctgaatttgtcaaccacttcaaaagtaacattctcattagccttaagtaatttcgcaactgggcaggtatccagtgcttcgtcgaccatttgttgtgcctgttcgttatctaattcatggaacagaatttgacagcgcaccacaaatttataaccggtagtatccttcaagttatcgactgcagtatgaataactgtatccggtttgagattatgtccccgctccactaaaccgatggttgcgttaaagcaggtactcaacgcaaagccgataaattgctcagggttggttcctggactgttaatcaatgaactgcttacgccaagagctaatccttcgttgccccggacgaaactttcaccaactaatccatgttcattaacaacttcagtatgataaagtgatccgtcaacagccatatataattcctcctatttaacaaatccaatccttcatccaacaacttaatgatatgtgatttaaatcggtaagtccatccaacagcacttacaattgttaacgcttactatagtaatcatttccccattcaggtcacttttttgatacactggacgttggcgcaaaaattcgaatgaaagaaggtcaactacatgcccgcaaaagaaatgaatttaaaatggctgatcattggggccatgttcagtagtgtcgggatgagctttgtctggccgttaaccagtgtgtacctgcacgatcggcttggtgtttcactcaccctgatcggagttgtcctgttgtttaactcccttgccagtgtgcttggcagttaccttggcgggtacctatatgaccgcaagaacccctatcatctactgattggtggcgttgccgcaaccacgctgactttgattctgctggtctttttccatggttggccggcatttggaatcatcctatttttcaacgggatttccggtggctggaacgtggccgtggtcaactccattggaaccagtattcaatctcaagatagccgctatgtttttaacatgctatacttcgcccagaatttgggaatcgttatcgggacctctttggtcggcttcatctacagcatcagtgtaactttgatgttcgttgtcgccacggctttgttcgtcgttttcctgctcatcgttctggtcaaattcaaaccggctgccaacaaatcacgtaaaaaagtttccgacaccgaaaagaccacttggagctccaaaaatttgccaaagcccaatgccattatgctgtttgcttttttcctgtcattattcattatttggatcatgtaccagcaatgggtctccaacctgtcggtctatatgaccggtatcggcatcccgctgcgcaactacagcttcctgtggacgatcaacggtggcgtgattgtcatcagtcaaatcatcatcaattggatttcccgctaccatgaaaacatgatttttgaagtctttctcggcgttttcttgatgtcgatgtcgtttgtcgtgctgatttttgccaaaacctaccccttcttcgtgctggcaatggtcactttgacaattggcgaagcgactgccctgccgactattccagcgttggttaacacgctgaccccggttgaggccaaaggacgttaccagggactgattcaatcctgggcctccgcaggccgggcgttggggccgctgttcggtggtttgataattgagatgtcttcgtacaccgccctgtttatcatcgccaccagcgccgttttattagtcctgatggggttaattgtcttgtggaacaccctgcaccgaaatctggtcatgtatcgatgagttttgaccaataatctggatgtataaaaaagagcttgctgacaatatcttgtcgcaagctttttttgatgcaaatttttaattacttttacccagttggctatgacgaatcccataactgaagtaaagaaccagcccaaaggcgaaccagatgccagaagcaatccacgtctcagcctgcaattgtgacagcatcagcatgcacaacagaccggaaacgattggcaatactgggtaccatggcacttggtagccatggtggttttgaatttctttgttccgtcgtaatggaataatcccaaatgaaacgaacagaaaggcaatcaacgtcccaatgttaaccaggttggttagttgctccagcggcacgaaaccgcccatgaaggcaatgatgattgtaatggtaatcatactatttctgggactgccctttttatcaagcttgcccaggaattttggcaggagaccatcgcggccgatggaataaatcaaccgtgatgaactgtagatcatcgtgaccatcatggtgaacattccagctagggcaccaagggaaataatcccggcaacccagttcaaatgaacaaattgcaaggcaaaagcaaccggatcagaaacgtttaacttggtgtaagaaaccatcccggtcaaaacgattgacaccccgacataaaggatcgttgcaacaatcaatgtcccaataattccaatcggcatgttcttcttagggttcttcacttcagctgcggaactggaaaccgcgtcaaaaccaaggtaggcaaagaagacggcagcggctccgccaagcacaccaccgtgggcactatgccagccaaatggtaaaaatggatgccaatttgatggcttaatgtagaataggccaactacgatgaataacaggataataccaattttaacaaccacgatgatgttgttgagccgaaccgatgaacgcatcccttggttcaacatccacgaaatcagcaccacaatgatgatggcaatcagattcccatacgtcccctgacttgggacgaacggcccggagatcgcttttggaaagccgatgtgaaagcctgccaaaaacgactggaagtaggcgccccaagcactggaaaccgcagctacggctaagacatactccagaattaacgcccagccgaggatccagccaatgatttcaccaaagaccagattcccgtaagaataggcacttccggcaaccggcagggccgaagcaaattctgcgtaacacatggcggcagttgaacagacaattgcagcaacgatgaatgaaataataataccaggaccggctttggttgcggcaaccgtcccgggaagaataaaaataccagtaccaatcacggcaccaatccccagggcaatcagatcaaaggctgacatagtcttaatgaatttcttgtcagtctcaagataacgatctaattgctctcggcgaaaaatacgagctaataatgacataaacgtgcctccacagttaaatgaattcttgattaaaatacttattctattttaacttttcaacctgtataaagtcaatttcattcccttgatgtaaccgatttatcgaaaaataattgcatatttaatcgaagtcgccaaagaaccattcactgcgaaattattgtatccttgtattaaagagacttcgaggggggacgaatttgaaaaagaatcggctggaagcattcactgacgccattgtcccgattatcatgaccgttctggtcttggaattaaatccaccagaaaagctcagctggcatggattctggggaattcgcgaagagctgatgtcctatgcgatttcattcttcttactggcaatcgtctgggggaaccatcatcacatgttcttactggtcaaatcaattgacggctttgtgatctggtcaaacaccgttttactatttttcttatcgtttgtgccgtttacgactgcaattgttgacaatgatcccaacagcctgtttggctcccaactttacacgctgttattcatctgtattaatctttcgtggaacctgctgcgagtgagtttggtgcgggccaacaagtcagtcaagccgctggtcgcatcgcttaaacgagatccaaaaagtatttacacgctggtcgcattcatcgcggtctttctcatctcattttactggcacgagtttgggatgatcgggacatttatcgtcatgttgctttgggtgatgccttatcggaagattgaggatgccgctaagcggatttgaacttgaatgtgctcggtgactatttaaaacacagaaagagccaaggtaacgctgcttgttagcgataccttggcccttttttacacctcaaagctacctatccgaattgtggaataacaagcagcttccagagtataagcgcttgttattccaaactctgctttgttagatccttcaattcaatattactatccataatcccactctcaccactcaaaacaacttgattgttcttgtagtcgagtttcatatcttcatcgaggtaaatcttgctgtaacccttgaagtaccagtcgccggtattggctgataattttgcgtcataatccggtaccttggcgtcctggtcaacggcaatcacgtcatagctggtgtccaacgagcaaacgccaactttcgagaatggcccgacgccatcgtcaaagctgagcaacagcttgctattggcaggaaagactttcttgagttgtgttaatgctgcatctgtaattgttaatttcattttctcacctctcttccttatcctaaacttctgagccggaaagtcaattagattgtacacaatccttttgatttttcatcaacttcattacctgttatgatattgtcgaggtgattaaatgacaaatcaaatgaacgccgtcgtgattaacgattacggcgatcgagatcaactaactgaaaccaaaatgccaattcctaacattaatgatgatcaactcttagtaaaagttgtcagtatcggggtcaatccgattgactggaaaactcgtaaaggcctgaggaaagcacgctacccatttgattttcccattattttgggacaagaaatggctggtgtcgtctcaaaaatcggtgccaaggtgacgggtttcaaagtcggtgatgccgtgatcggctatggtacgcccagcaaccgcggaacctatgcggagttttatgcgattgacgcggatcaagccgcccacaaaccgattaccgtctcctttcaagaagctgctgggctgggacttgccggcacaactgcttggcaggctttatttgatgccgggcacctcaaagttggccaaactgtcttaatactggccggctcaggcggtgtcggttccatggcaattcaactcgccaaacacatcggcgctcacgtcatcacgaccacgagcgctgccaacgacaattatgttagaggacttggcgctgataaagtcattgattacaaaacacaggattttgccaaagtctcaccagaagttgatttagtctttgacacattaggcggtcaaaaccaactagatgctttcaaagtcgtcaagcctggtgggcgcatcatttcgattgttgaaaccactgatcaggcagaagaactcagtcaaaaatatggtgtgtcatttgaaaaaatcaacgcccatcccgataaagacgtgatcaccactctaagcaataagctcggcgccggcaaactcaaagtatcgattgcgactcagctcaagttcaatgccgagaatgtccgcgaaatgcataaactcagtgaaacagggcatatagttggaaaattaatcttgaatgtttagtcccaatcagtgcgaagtcaaaacgatcaagccatcagtataaacaattgatgttttgccgatttgttcataaaaattagcaaaaaaagaaggtcaaccggatttctccagtcgaccttctttattacggcacctaccaaagtagatggacttcttggattccacaatccgctaaagtcaaacaccagcaaatctgtgccttaaattgtgtcccgctcgaattcacattaatcgcttgcgcaacagcataaatgctgtgtgatttctcgactcatcgcatacaagtattatgccacgtttccatgaaaacatcaaggcatctttcattggcctacttttcttcaggctgcttttcaaggttttctttgaccatatccaaatgctcagccacccagttgttcatctgatccaagtagttggcgacgttgcccacgtagtcatcggcactggcgacctcatcaatccgcaaactggatttattgacccacggtgaactgatcaccaggtacacattcaccggcaatgtctcttgatcctgcatcattttactgataactttggcatcttggaatggtaaattgatcaagttggtttccaaacgaatcgcaacatcttcatcggatgccttgacctcgccatatgcaagcttacctaagttcagttgttcctcaacgtagtcatacaccggctgcatcactttggccggatctttcatgatgtcgtcgagcttcttggtgaaagatttgccttcaatcttttcattaaccaaatcatccacgaaacttgctgcatctttttccaaattagtcacctatcttcttaatcctttttgcttgttaatccgccgttgaaatgtatcgtgttgaagcactgctctcaatctgaacgccaagatataccaatagacgttgacgacaattccaaatgcggcaaccgccgacacaaacagcttgaccagaatcgtcgcgtcactattcaggaacatcgtcgaaatcatccccacgaagccaaccgaataaatggcgatcaccactgccagcagataatagctgattttaacccgtagtgcggccaaaatcaacgtggccgcgtaaaaggcgatcgcaatccaagtcacctgcaatgcttctccagtcgtggccggtgctttcagtgccatgaaaggcaatgtcatcaaccaagtcactgccaggaaaaccaccaacgagatgattgcccagaaaatggtctgcttttcttcttttttcatttaacgttttaccctccagaattccaacaaaaaaagataaattcgatgatggaatttatctttttattaccagttttagtgtaccttattaaagcggtttagaaaagcatatcaaagaaatcatcacgagaaattccggtgaagtactggttcaaatcaacgtctttcaaggcatcttcgaagtctttacgttcgaaacgaacaccctttaatttgtcggcaacttcagttgaatcttgtgggccaaagtaatccccaaagaatttaacgttggataccttgccgtcatcaacttgcagacgggcatcaatggttccgttagtgaagtgttgacgcttcttaacggtgaattctggtgaattgccatatacccaatcccagttgttgtagtaatcatcaaaaatcttatcgatgcccttttgatcgtcatcggttaaatgatattccttgtccttgatctggtcgaggtcatccacgtggaacaactctttcagtaaacgatcacggaattcaggagtggttaagtcttgatacttcggtgacaagtatggtttcaagttggtaacccgtgagctgactgacttgattccctttgacttgatcttgtcttcaggaacgtccaaagcctttggaatgactgacaaatcaacatccagcatcaatgtaccgtgggagaacgtcttgccgcccttggtgtacattgcattgccggagaatttcttgccgtcaaccaaaatgtcgttacggccactaacttcaacggacttagcgcccatgtcgtgaagcgcgtcaacgattggttgaacgaatgacttgaagtcaccaaactcttcactgtcactgtcaaccacgaagctgaagcaaaggttgcctaaatcttggtagacagccccaccgccggaaagacgacgggtaacaacaattccgtgttcatcaacatattttttattaatttcttcaagagtgttttgattacggccaacgatgatacatggtccttcaatgtagaataaaagtaacggttcatcaaattttatctcgttcatcaaatactgttcagtagccaaattgcgcctgatatcattggatttcatgacataatagtacataaaataacagcctcttttcatttagttgatcaacttgaatattagcacgttaggaaagcgattacaatcacaagcaaaaagttgaaaattttaattgattacaagcatccaagagaatggtatagtttaggtaaggacaatacgaatacggggtgattgacatgcaacagcaaaaatatgaaaatgtcttggtaccggtagatggctcaaaagcaaccgaaaaagtgctgaatcgagcaattgaggtagctcgggacaacgatgcccatttggatatcttaaacattttggaagtaaaccaatttaaccaaacttatggaagtgctgtaagtggggacgttgttttcaagttaactgaaaatacggacgatcagctaaagaaatatcaaaagaaggctgaggacgccggcgtcaaaagcgtcgacatccacatccgatttggcaacccgaaaccaatcattgcacgtgaatttcctaaagaccacaacaacgatgttatcgtgatcggctccaccggcctaagcgccgttgagcggttgattatcggctcggttaccagttatgtgacccgaaccgctaaatgcgatgttttgatcgttcgaccaaaagacaaagtaacaccaaacaaataacaaaaacagcgtgtgggcggcggcaattatgtcgacgcctttttgctatcaacgattaaggacaatgaagatgaaagatattcagtggtgttttaatgagactgtaccggaagccatgaacggccgtcccttaaaggcgcttttaagtaattattggcagctgcccaagcatctggtttacagtattcgccatgccgaacgagtgctggtagacggccattatcagccggtaaatttcccggttaaagccggcagccaagtccagctgacttttgtgccggctgattttgccagaccatttccaaatgtcacggctgattcagcggccacggtcgcgattctctatgaagatcaaaatttagtcgtcatggataagcggcgcggtgataaaacccatcccaaccaacctggtgaagttggggcgacgattaaccatttggcggcttatttggcaaccgaaaagaccgttccctacatgattcaccgattagatcaggagaccagtggggcgattattttcggcaaaaatccggtggtcgtgccaattttggtggccaacatcgccaacaaacaaattaagcggacttatttggcctgggttgagggaaccgacttacctgatgaaggcacaatcaatctgccaatcggccgtgacccagatgacaaacgtaaacgaaaaatcaatgggcctcacgcggctcctgcgttaacgcgttatcgcgtactgcgcaaacagtccgggtacgcactcgtccagatttcgctggaaaccgggagaactcatcagatccgggttcattttgccgcgcttggtcaccctttagttggggatccgctgtataattcaagtaatggtagccctttcttgatgctgcattcttggaaggttgatttattaatgccattcactaaacaacgaaaattaattgaggcacccattccggatcattttatcaagtttgagcaagaattatcccgtcattaaccgtgccttagagaggagtcgaatatgacagaaacacatttatccagttactcggcaactgaattatcagaattaatccgccaagggaagttggatcgggtagcactggtccaggaactaatcgataccgtggagcagaacaatccaaagctcaacgcagtcactaccttatggggcgatcgcgctaaaaagatggccagtcaatttaacgataccggccaaccatttgccggggtgcccattttattaaagggccttggccaatccttcaagggtgaacctgataccggcagctcaatgctgctcaaggattacaagtcaaacattaccaacaacttcgttcaagctttcttgaaggccggcctcatcccagtcggtgaaaccaatgcgccagaatttgggttcaagaacgtcaccgactcaagattatatggtgatgctcacaacccgtggaataccgattatcaacccggcggctcctcaggtggttcggcagctgcagtcggcgctgattggctgccaatcgctggtggaaatgatggcggcggttcaattcgaatcccatcatcattctccggcaccattggcctcaagccaactcgtggccgggtaccaaccggcccaggcgagtggcggggttggcaaggcgcatcaatcaactttgcgattacccgggatatgaatgacaccgcccgcttactggatgccatatcgactgtccagatggccgccccattccaagttccacttccagcagcctctttcactgaaaccttgaacagcctgcccaagactttgacaattgcttattccacagaatcgccagttgggacgccggtttccgacgaggccaaacaagcggttatggatgccgttcagtttttgacagatgaaggatacgatttgattccggcagacgcgcccatcgacggtgtcgggttaatgaaaagctactatttgatgaacgctggtgaaacagcaacgatgtttgccaacatgcacctcaaagatgacgtcattaaggaaaacgttgaaccgttgacctgggcgctcggttatgccgggcgagcagtgacggccgttcagtacagtcaagcactgactttttgggataatatcgtcagtgatatggatgccttccagcaggaatttgacctttacctaacgccaacaactgcccatcaagcaccccgaatcgatcaaccattagtctcagctgagaatttaactaaaatgaagcacattgaagaattaaatccagaagaacaaatgcagttgatttgggaccaatggctgcctgccctgaccttgtcgccgttcactcagctggcgaatatcagcggccaaccagccatcagcctgccaacctatgtcggagaaaatggtctaccgctgggaattcaattcatggccagaaaaggtcgtgaagatctactcctacagatgggcaaattcttcgaggataatcaaaaatttcatttacttaaggactaatcagtttcacaacatttgaggaggagatcgcatgattaatattcgcaaactaatcggcttactgacaattaccggggcactcggtgttgtttcaatcacatcctcaaatccagtcctcgccaaacataatccaaaaaccaccgcaattaaaaaagcaaccaaccagccggccaaccaaaacgccttaaccaagggaaatgttcccaagctttggtcgcaaggctatcaaggccagggaatggtggttgcggtcatcgatagcggcgtgcagaataatcaggaatttcaactatctagtaacaccacagccaaaatttctaaatcccaggcccaaaagtttatcgctcaaaggggttacggcaaatacatcagcccgaagattcccttcgcctacgattacgtcaacaataataacgatgacagttccgcagacagtgtttccggtttccatggtctaatggtcgccggcgttgccgcagcaaacggtgtcgcacgaaggagcaaagccaaatttgtccaaggagtggctccggaagcccagattctcaatctgaaagtctacggtggtttctctgatgaatcaccaaacgacgttgcgcgggcgatttatgatgcggttgatctcggggcagatgtgattaacatgtccctggggatcggcgtcggtaatgaatcactcaatgatcaggaacaagcggccgtgaaatatgcgaccgatcacggtgtttttgtggctgtcgccggcagcaactatgggcatgcgggcagtatcaccaccgattataatgagcaatccaattcaacgattacgacttatgaaccggctaactctggcaccatcagcgatcctgccatttcaccatttgccaccacggttggcgatgaaaacaccaagcagggtgacaagagcgagatggattctttctcggcttgggggccgacaccggattttaagttaaaaccggatgtcagtgcgcctgggcagcaaatcgccgttttggatcaaaataatcactttacgaccaacaccgggacctcatttgcctcgccgtacattgccggttcggtagctctactcatgcagaaatttaaaaaagatcagccaacgttaactggtgccaaactggttgaggcagtcaaagtagctctgatgaatgccgcccaaccaatggccaacgacaaattcaaaggagaactgatttcaccccggcttcaaggtgccggtcaggtgaatgtcaccaatgccgctaatctaaaggcatccgccgccgatccaagtggtaaccaaggatcaatttcattgaaaacaattggccaaaccaccaagttcaacgttgccctgaccaatcacagctcagagccgttaacctaccatatcaacacggcaaatgggccgtttacagaaagccgaaaaaccaacaatcataatgttgggccggttcatgacactgcgatccctggtgccacactgcaatccgccaatgataccgtcaccgttaaccccggcaaaacgcagctggttccttttaccctcgatttgggcagccaagctaatttgaatagcgtcgctgaaggttatctaacttttgaaaatgccgattcaaatcaaaatttgacggttccctatttcggctactatggggatccaactgatgagcaggttgtcgataaacccgccaatcaggctgacagtattttcaacggtggctacctaatggacactcaggatatgccgctgggattgagtgaccgaacctctctggccagttggttgaacaccttgaaggatccggacgaactgcgagacgatatgccggaaaaaatccaatccgacaaggtggccttctcacccaatggggacggccattccgatgccatcagtccatacgtgttcaccacccagaacctccaaaacgtcactgctgagattaccgatgccagtggcaaggtcatcagaaccgtcgacaatgaaaccaacacccagaaatcaattgaagaagccggttccggctacattgacgatttaaccctttcgccttcgatgcgcttgaaccccaaggcattgaattggaatgggatgacttataatcagtcaaccggtaagatgacggtggttccagatggtcagtaccactacgtcttacaaaccaccaatttcaacgatggcgccaagcagcagcaagaatacagtcttccggtcaaagtcgacacggttgcgccaaagattaccaaggcaacttatcggaacggccgactggcggtgaactactccgacgttggggttggctttacttcaatatcgacacttgccgtccaaattggtcatcagtctgcaggcgtcagcttgaacaattctggccaatcaaataccggcagcctggtctacaaactgtcggaggccaagcaacgcgcactcaagcaagctaaaggcaaactaaagatgacgttggccgacgttgccggtaaccaaaccaagcgttcgatcaaagtcagtccaaagatgtataaccacgttcaaacgtcatcaacccctggttccaagcttgtctggacattgaaaaccgatgacttggaatcaatgatgagtcacgataagtatgcggtgaccacccgtttctcaccaactaaggggattacatttaaagggttaaacgacaatgacttcaccttaatcaacgcagccagcaacgtgtatgatccgcagacccatcaactaacgattgctgggaaagcggctaacccgaagtcgaagttaaccattttacgcagccccaaccaaaatgcgaaaattaaccaagtgaaaatttcaaaaactgggtctttcaaatttgagatgccaattaatccaacgacccagcaagggatcggctacatcctaaaagtacccaagaagcatcagtggacaacggccaaaggtactctcgtggttattgccgacacaaccgcccctacgctgaatttatcgatgcctgacaatgtttccgaaacctcacagaaccactatcaattaacaacttcgaatgatcaattcaccatcagcggtactgtgaatgataacgttgatggctatcgcctcttgatcaatggcaacaatcttttccatgagcaaaataacgcgggttgggtgaaccaccaagatttgggtgccaatcccaatccccacagtcctcatcaattcactcagacctttaacctgaatcagggaacaaatatcttccaggtttctgccgttgatgagactggtaatcaaatcacaaaaacaattaccgttacccgcgagtaattctcaaatatatatgtatcaaaaaaggagctcgaaatcatttctgatttcgagctcctttaaggttttagtaagcattaagtcgtaatgaaattacttcttaaggccttcccacttccagtcaacaacttctggaagatcagtaccttcttgacggatgtaagcattgtgcttatcaaccatgtcgttcatacgttggatgaagtaaccacccttaacagtgtaagctggaatatcttgaacagcttcctttgcaaggtcgaaacgatccaattggttcaagacacgcatgtcgaatggtgtagtgatatcaccattttcacggtagccatgaacgtgaaggttatggttgtgacgatcgaagaagatatccttgataaggtcttcgaagccatggaatgcgaagataactggcttgtcagtagtgaacaagttgtcaaattcttcatcactcaaaccacgagggtcaaccttaggtgaacgaagcttcaagagatcaacaacgttgatgaaacgaatcttcatttctgggaattccttgttcaagattgagatagcagccaatgcttccaagttaggttctgagcctgcggcagcaaagacaacatctggttcttgaccttggtcagttgatgcccaatcgatgtagccaagaccattcttaacgaggttttgagcttcatccattgtgtaccattgacgacgtgggtgctttgaagtaacgattaagttaatcttctcgtaagttctaaatgcaacatcaccaacagctaacaattcgttagcatcagctggaagatactcacggatgaattcaggcttcttctcagctaagtgagttaacatacctggatcttggtgggtataaccattgtgatcttgctggaatactgttgaagtatcaacaaagttcaatgaaggatattgctttctccagtattgttctgaagctttacgtaaccacttgaagtgttgagtcaacattgagtcaactactcgtccgaatgattcgtaagtagcaaagaatccatgacgaccagtcaatacataaccttcaagccaaccttctgcttggtgttctgaaagttgtgaatcgataacacggccgtggtttgaaagatcttcatcaaatggttcgtgaatgtcttccatccattgacgcttagagtcatcaagcaagctgtaaagacggtttgacttagtttcgtcaggaccgaatccacggaagctggtagggttaagttctgcaaccttttccaaccagtttgaccattcaatcatatcttgcttctgagttacaccacgatcgaatttaacttcgaagttgcgaacatcagggagcttcaatggttctggtttgataccaccgttagtgattgggttaactgacatccgcttgtcgcccttaggtgcaactgcacggatttctggtttaacagtaccattttcatcaaataattcttcaggcttgtatgacttcaaccagtcattcagcaagtctttgtgttccattgaacctgcggcaacaggaattggaacttggtgagcacggaatgaaccttcgatagggttaccatcgagatccttcttaggaccagtccagcctttaggtgaacggaagataatcattggccagttaggtaacttaacgttatctggtgtttcgttttcacgagcattcttttgaattgacttaatctcttcaataacatggtcaagggtcttggcaaattcttcttcaaccttggcatggtctgtatcagcagttgcttcaacaaagtatggatcccagcccattcctttaaagtaactagttaagtcttcgtcactcatacgtgaaaggatagtagggtttgaaatcttgaaaccgttcatgttaatgataggaagaacagcaccatcagtaattgggttgatgaacttgtcagagaaccatgaagcagccaatgggccggtttctgattcaccatcaccaatttcaacagcagcgattacatctgggttgtctaagatagcaccggtaccatgtgaaagtgagtaaccaagttctccaccttcatggattgaacctggtgtttctggtgcggcatgagaagcaactccacctgggaatgagaattgcttgaataatttagccatacctttttcatcttggctgatgtttggatagatatctgagtagctaccgtcaagatatgagttggaaaccataacttggccaccatgacctgatccttcgatgtagaacatgttcaaatcgtatttgttgataacacggttcaattctgcatagataaggttttgtgatacgatagttccccagtgaccaataggcttaactttaacgtctttggcttcaagaggtcgcttaagtaatgggttgtcgcgcaagaacaactgacctactgaaaggtagttagcggcacgccagtacttgtcaacaagttccaaatattctttggaatcgtaatctactgtcattaattaacactccttcttcgatttagcaacaaacttctgtatagaatgtccgtaaaattcaccaattgtttcttgatcaatttacatcactaatactaaacgatattttcaaaaagtcaaccttttagaaaattgatacggtccaatatttagtgggcgaaaatcctatacttatgtgccattatggacgctaacaaatatttagtccactattattaatattttgtaacaaaattttcgaacattttactcacgtatttttccgtttgaaattgacggccacttggacgataaacaatagaacaaaaatcgccgttgtgatccaaaatgtgaatcgcattccaaaaatgaatgcttctggttgagcaactggataatcaatggttgagtggccgagattcatactgataccagtaaatagcaggatgtttgcgaaaatcgctccaactgtcatcccagtattccgcgagaaccccagcagtccactggcaacgcccagctgatcttttgataccgagttcataaccagcacgttggttggtgcttgaaacaggccgttgcccaagccaacaaaaccaagccagagacataagatcaatagaggtgttgtatggttaacgctcgccaaccccgcctgacttatgatgagcatcgccaaggaaatcgccgcaatccggtgtgatccgaatcggtcgctgagccacccggcaaacggtgagacgataatttgaatgatgggaaaactgatcaaaatcaagccggccaggtcggtggtgatgaatcgattctgctccaaatagattggttcgatgatgttgacgacaaaattaattccataaactaaaatcgtcgctaacaggctcagcgaaaaatcaatattgctgaataaatgaaaattcatgaccggatcggctgcccgtttttccaaacaaataaagataatcagtaaaatgattgtcgcaatcatcaagctgagaaaaatcaaactcatgaaaccaacttgttgacctaaaatgaggcccataaataaactgccggccataaaaatcaaaaccagcatcccccaagcgtcgattttaccagcagttgttgcttcagctttcggcagcacaatttggccaaggataattgccgcgatcccgaccggcacgttgacccaaaagatgtagttccagggaaggtaagttaggatgaggccgcccagacccggtccggcgatactcccaagggcgaccaccgaaccaaagctgccaagtgccagtccccgctgttctttagaaaaggtctcggtgataattccggcgttggtgctcaacgtcatgctggcacccaaagcttgaattccccgcatgatcaagatccagacaaaccccagattgatgccgcagaatagggaagcgatagtaaaaatcacggtgccaatcttaaaaacccgggctttgcccaacatgtcacccaacttgccaaatggcaataagaacatgcacgtcacaattaggtaacttgaggccacccacgtcacttgggcagtcggcaccgccattgctcgggacatgaccggcaatgcaatgttgacgatgctgctggtgagtgtcgacatgaatgacaataagacgacggcggtgaaaatccaccattgattttgctgattgacttgcctggccatgctgcgtgcctcctcccgaagattcaaaactttcatctataggataggctttttcagtggcgtggttggaaaatttgctcacaaaaatactgcaggaatcactgtgtgactcactgcagtagaataaagatttaatgaaacatatgtgacataacttcggtgcccattggcgtggcaacaatcgccgcaaagatcagtagtaagatgccgatgaccatgaatacgcctttaactgctgggcgatttttttgtctcagaccatagattaaaatgagtaggcctaggattgcgatgattagcatgatgtagaaccccgtgggatcaccttcttttggttgagtggttctgggtgttggctttttgctcttttgaaaatatcttttaccgagccgaaatgggctccgacgggccagatgctaacttctaaacccgctttggttcaaacccaaacccggggtttcaaccaaagcgggtttagaaaccgcatctcccggccctcgtcgccctctgctacttatcctcatccaaattcacaaaggtattataattcaaatacttataatgaatgcgcatatttgaaacttcaaacggcgtgccatcatccaagaagaaaataccttccatcacgccaactggttcgaccggcttcaagcccaacaactgctggtcttctttggtcgatggatccgctgtgatggtcataaatgacttggtaaccgagttgccggttgcgtcttcaaaatagttgaagattgagccctccactcgttcgctgttgagttccggcgccactcgaattgggatatagccgagttcaatcatgaatggtttgtcgtcaaacgatcgcagccgcttaatctcgtacacaaattcacccggatttaaaaacaattcggtttgaagctcttcgcttgcgggaacgaccttaaaatccaacaacttaattttaggcgtctgaccatcactcttaaagctgtcagtaacccccaggttggatccctcgtattgaaaaatcgtctgattcttctgatatagcgggttaataaaggttccagaaccccgctttttaaaaataatgccttggtttgccaaaacattcaacgcgcgtttaattgaactgcggctaacaccataggattcgctgaggcttcgttcatccggcagcttctttgaggcaaattcattggcctgaatgcgctccttcaaatccttcatgatattgcgatatactaaatcagccatttgtgctccttattaaatcgttaaattgatctattatcaataaagtataacagattatcatcttttgttcagacagaatcgttttgccaattgtgctaaaatatccctgaggtgttatcaaatgtcaaaaaagaagaaaaataaagttcataaaacattagtcgaacaaattctcgataagcacaaaattccttttgaacagatggaatttcccacccacaaagaaggcgacgtcgaacaaatcagcgtcgaccacgtggatactgacgagcaccagatttttaaaactctggtcttctccggcaaaaccactggcccggttgtcggtgtggttccggtcgacgaacacttggacgaaaaaaagctcgccaaagtttccggcaacaagaaagttaatcttgtaccgttgaaagacttgttgaagacgaccggctaccagcacggtgccaacacgccaatcgggatttgggaaaagttccattaccccatttatgtcgaccaggaagccaaggagatgggggaaatcatcgtctcatctggacaaatcggccgttcagttaaggttgactcccagcagatggtcgacctgatcggcggcaaattcgccgacataaaggaatgattgaatgctcaaagatattctaacaaatattggtttggtactcggattaatgatcggagtaccatttctttttatctatctattgtcatccatcaaccacggcaccaagcaacggattgccaatcaatttggtattggcggacaaatcggctttggctttctggggattatcattcatgaagccagccacttattggtagcgttagtctttggccaccatattgatcagtttcgcttgttgcgagtaccaacggcagacaataataccctgggatacgtccaccacacttggaacaaacgcaatctctaccaaaatatgggtaatctattcatcggcgtcgcgcccatctttggctgctgtttatctgtcctgctgctggcaaaatacttcatccccgaagtctaccaatcattgatgacgactgctgaacagccgctgagtcaactaatcgtggtgctgccgacttttaactggctttcgatgggcttatttctgataattgctgccaacatctgtattggtggttttgatttgagccccgccgacttcgacaattccaaacagggattctggcagggggtcatctgcttaacattactggccgtcatcatctcgctcaccccactccaagcgccgtttttcagcttactaatccgtttgacggtgattatcgtggtcatttcactatttaatttactgatttcaatcgtgatgaacctgatttttcggtttatttagtgccattccattcgtcgacaaattcgcccacaaagtcttgcatgacctgttggcggtgttcggcgatttttttggcggttggcgtgttcatctgatctttgagtttgaataatttctcgtaaaaatggttaatgaccgtcccgcgcttacggtattcagccttatccattcccgtccgcggcataatccgtggattatacataatttcaccgaagtggccgccaaaataaaaggtccgggcaatcccaatcgcgccaattgcgtcaagacggtcggcatcctgaacgatctgcccttcaatcgacaagtggtggtgggtcttcagattggcactgtaggacatgttatcaatgatttcgaatacttgcttaacaaacgcctcatcataaccaacgccaatcaattcatcagcaattgccttgcgtttggcagccggattggtggtgactttatcatcactcacgtcatgcaggtaagccgcaatgattaccaatgactcatcagcatcctcaccttttaaaatcaacttggccaaactgaccacccgctcaatgtgcgtgtaatcgtggccagtggtttcgtacccaagctccttttgaacaaacccgcggatttgtcttagtccattaatcatttgaaaaccccttttaaatatttatcaagatgctaaaaatcactcgaagaatcaaaatcccccagaataactgccaatagcgcagatatgtatgtttaagcgatgcgaaccaggtgacgaaaaacgtccaccagtggacccgactgcgattttggccataaaagtcgctcatttctgcaatcatcacgaaaagcaacaagtgcagcatcatcaacagaagcaagtcgatgacgtaggctgtcgccaaataccatcgagcaccacttgaagcaatctgaaatgatgaagcgaccagggaacccagtccggcaacatttagcgccccagccaaacttaaccaaacagatgagagaatgtaggtcggaatcagtgatagcaaaagcagcggcaggatcagccgggtatcactgaccagctcttgggcagttattgagggaatcgcaccgattaatgaccgaatagatggcataacctgaatttcactagcaccaaattgaaaccgcgtacccaaaaagaagacgactgccgcaactgcccaaacaatcacaaaaaagttcttccggtaggctgtcgcgatcgagaccagctgtgttttaagattggaacgagtattccccaatttgaaatccccctactttattcaaacaactattagtatacccttgcaccgtcaaagctgaaatagccgtgctagaaacggttattctctgctcaaccacaaaaagccgtcaatccgagaacgctcatggattgacggcttcattaagcatgtcactttattgaattgaatagactgactggcccttcaaggccgccttataagctgcaactgccaagttgacctggccgacgccatacaactgactagtggcatttttaatcgagccggttttgttcacatacgtcaacatagcatacaacggagttgccttttgtccagcgtgcatagctgtgctgttaacatattttttggtgcttgacccattcgccagggcaatgatcgcctcagccgttgaattggcatttggggtggtcttgccgttaaatgtgtatccgaaagcaccattactttgtgtcagaccgtacaagaactgctggcctttcttgatgcttgattcaaccggactggttgttgattgtcctcgtgataatccagtcaaaaccatactcgtcgtatcggcgtccttagctccttgtgcgttgttataggtccagccattattcttcagttgaacctttaccaaccgggaactcaagctggccttgctaaatttggcattgctgggacgtttgaaatgattgctcatcgatacggcaatcaaggtttcggcctgagaactggccgtctgcttggcaacgctgcttcgatacagtcgtgagaccaagttaatgcccgttttatggccatacggcttgtagttctgcgcgttcatccccatggcttggacggccatcacggcattggccaaagttgcggcggtgctattgctcttaatgaccaagtttttcctcaggagattcttttcgcctgtggtgaattgataatggttccctttcagacccagtaagaaatcagaataaccagaggaagccccggtttctgagtaaagtttccggctgaaaatcgagctggtcttaccagacaaacccgtcttgttttctttaagcatcttctttgcgtaggcgtatgtcagtgcagtccggcggtgaatcgttgacgtgctggccttatgaatggaagctgcaccggcattggccgtcaaggtgacggtcatgaccactgcactaatcgaagctaaaatatttttagttaattgattcattttgaatacccctcttatttattgtaattcagagaaatccggtcaccattggccaccacataggcaccaatcgatgtattgggctggttaccattaatcgagtaaagccagccggtcatcgtgccggcggggccggcgttatagccgttaatccctttcacataagccgtgatgccggagccgaccgttgtgatcgacatgttgtgctgagaagccagcgcattcaaagcatccagcgcggtggcgcctttggcaagggtaatgctgccactggccagcactgatccgttggcattgacacttaccgtgaccgtttcggtggtggcattcgtattcgtacctgaattgtcgttagtggtcccggaagtgttggtcgacgaagaactagcattgttggacccggttggcgtcgtagttggcacgctcggagtggtagttgtcgtggacgacgaactggacgttgaggtcgtcggtgatggcgccgtggcaaccggcgttccagctgcatcggtattctggccgctggtcttggcaatcttggttgccagaaccaaccgtttattggctgacacgtaccggccattggtgagttgcaatcgggacgtgtgcccatagtcgaccactttttcaacatttaacgaccgattctttttaacatgtttctttcgcccgcttagttgtcgattactgtattcattgatgccctttggattaagaaccttaacccgggtgactttggctgagtagtaggcaccagtcaaatatttcgcagccgaaagcatgtagccggtcttgccactcctcaaatctctaacccgataaatggcatgaccctgttggttagtcgtctgcttgaggaccaaaaacattggccgattaatgcgggcctgcttcttgtagattttagtcagctgacgcttattaaaatcggtactcttgtaaagcttaacggtcgttaaagcataaacaaccgatcccttggcactcttggccttcttggttgtggtcggtttagtgaccggtaccgcagatgatgaactggaagccactgaagaactcgatgaacttggggcgctgttaataattgtcgtgtagttattggtaatcgtcgtgccactgctggacgaagctgcacttgaatcaacgactttgacattgttaatttccgcaacaccaactgcccgatcggcaatcgccgcttcatcggttgtatcagcattaatcttggtaatgtagttctcaagcgtttggttaatcgtgctgatcgcagttgctttgtcggtagctgacgattgtgaatcattgttgattgcttgccgtttggtcgttgcagccgcattaagttttgccagttcccgcgctctaaaggttgggttttcgccaaaattaaagatccacccctggccgccgtctttggtaaatttcgcttgttccaacgtgtaagttgcctgctggagcagcatggagttactgtcagcactaatatctttctggtccaataaccgttgaaccggtgcttgataatcagatttaccgtttaatgatgtgtagacgtcaacgccggcagcggcaagggcgttaaccatcgtaatgttattgtactgatcttccttattggtctgattcccaaagccaccattttgttgataataatcattttcaatcacactaaccgctttttgaatggcagctggaactccaggctgatccatattcatagaaagagcttgaatagcacgggccgtcaggtcaacatttccccatgaggacgtccagattccagcagctggatcgcggtcggccaagatctgtttagtcaaagtagcccgcgccgtttcgctggctttaacataactgccggtactcaatgcttcaagatcgttaaccaaggtgtacaaactcggtttggcaattttggccaatggatcattgataacttgacccacaaggtccttcttttcaacattagctgggtctttgcccagtgctcttaagccaatgaccccggcaacatctgagacaccgctcggatcttgcacagttccgcttaagaatccattagtggtgatgatatcctgataagcattttgggcctgagcatcagtgatgccattatcactcgtcgccaaaatcatggcatcccaagcatccaaggtatccttttgagcggtcagcttaacgccggtcgtaatcgccgaatcaacatcagcggcggtatcagcttgggcgaaggcttcgccaccaacaaataccaggaacatcccgactaccagtgatacccaataaataaactgtttcttcttcatacctgcgcgctcctccaaatcatgaaatagtgatggtaccctcaacaaaaaatgaacacaacaaaaaagcctggctagttagactagccagggccgtttctcaatcactaataacctaaattcagatattgaatcagagcacacaaaaatatccgagaaatacgctattaattgacaaagccgaccctaagaagctttgcaatcggcataacaaacgtatcctgacttgatctcgtcctacaactgtcctctttccagggtgacccagtgagttgtgacagcttcgtcaatcttacagtagcgaaggggctgtaaaggatttgcacctttttccgttttactatgcttcttaacatgaaaattatagcatggaatttgggtggatttagagtaattgagaaatttattgataatggggctaattgtttcctggcttgagaaggtgacgctcctctttttttgctggagagatattggtttctgcgaggactgggctgtttttgtggacagctacgcaaaacagcagaatctaaattagagaagagccccagccacgcgagtaatcgcgcaactgggaatctggtccacggttaccaagtgatcgatactattcaattgattgcttctttaaggattttcccagtttgagtctgcttttgaggacagctacgcaaaacagcagaatctaaataagagaagagccccagccacgcgagtaatcgcgcaactgggagtgttttccgcggttaccaagttgagaatgctatttaattgtttgtttatttaaggattctcccagtttgagtctgcttttgaggacagctacacaaaccagcgatacctaaataagaaaagattcccagccacgcgagtaatcgcgcaactgggaatcttttcttatttaggtatcgctaagcggtttgcttcgctcactatttttccacattagtcccctcataatcgtcaatcatcaactgtttcaaatcggcaatcaaaggttcctttgggttagcagtcgtgcattggtcttcgtatgctaatactgcaagacggtcaactgctgcatcgaatttggctttatcaacgccccaagccttcaagcttaaggtaacgccaacttcgtgagccaacttgataattctttgaactaatccttcgattaactcatcgtcgttcttaccttggatcccaacgtatctggcaatttctgcgtagtccttgttggcacggaagtactcatacttaggccatacggcgatcttttccggtaatttggcattgtatctgataacgtgtggcatcgtgattgcaatggcaattccgtgggttaagccgaattccccacccagtttgtgggcgattgaatggttaattcccaggaacgcgttaccaaatgccattccggctaaggttgcggcgttatgcatttcttctttagcgtgcatgttgccattgtatgagtctgccaagttgtcaaataccagcttgatggcttgcagtgacaatggacgagtgtaatcagatgccatggttgaaacgaatgattcgattccgtggcataaagtatccaatccggaagcggcaatgttaccctttggaacagtttccacaaattgtgggtcaacaatcgctacatcaggtgtcaaagcatagtcagctaatgggtacttaacgtgggtctttgagtcagtgataacagcgaatggggttacttctgaaccagtaccggaagtcgttgggatagcgatcatttgcgccttcttaggcttgttgaaacggtatgcccgctttctgatatcgatgaacttctgcttggcgccgaagaaactcgtcttaggatcctcgtagaataaccacatgttcttggcagcatccaatggtgaaccaccacccaaggcgatgattgtgtcaggcttgaatgcgttcatttgacgaacacccttttcaactgtgtcagtggttggatctggctcaacacctgagaacagtgagtattcgattgggtttggacggcgtttcaattcatcaagcaccttgtcaacgtagccaaattcaaccatttctggactggtaacgatgaataccttgttaatgccaggcatgtccatgaggtaacgaactgaagtcttttcaaagtaaacccgaggtaacttaatccattgcatattatttcgtctctttgcgatagttttgatgttcaaaaggtcatagtcggtaacgttatgagaaattgagttggcaccccatgagccagttcccaatgtcaatgatggggtcatttcgttataaaggttaccaattccaccgaagccgcctggtgtgttaaccagaacccgggcagccttcatctgcttaccaaattccaaggccaagtcgtcgtccagagtttggatgccggcagtgtggcccattccaccaaagtgaagtaattcgtcacagagtttgaaaccttcttcatggttcttagctttgtaaatactgatcactgggctgagtttttcagctgacagtgggtacttaggaccaacgccagtaatttcagcagccagaactttggtgttgtcaggtactttaataccagccagtttggcaatccctttagctgatttgccggcgattggacccttaacactgccagtcttagggttgaacattgcttctgccaatttgtcatggtccttcttatcaacaaagaagacaccgttcttaactaattccttcttaacttcagcgtagatatcagaatcgataaccgcgctgttttcagtggcacagatcataccattatcaaaggtctttgagagcaccaggtcgttaacagcacgcaagatgttggcagtcttttcgatgtaaaccggaccgttaccaggaccaacacccaatgccggcttaccagttgagtaagcagctttaaccatgcctggaccaccagttgccagggtacttgcgacacctgggtggttgattaatttcgttgtggcttcgatacttggttcttcaatccattgaatgcagccttcgggagcgccggcagcaatcgcagcgtcgcgaacaatcttagcggctgcaattgatgacttcaatgcttgtgggtggaaactgaagatgattgggtttcgagtcttcattgaaataattgatttgaataaggtggttgaagttgggttggtaactggtgtaattccggccaggacacccaaaggttcagcaacggtgattaattgacgttctttatcgtctttaatgacaccaactgttttgtgatcacgaatgctgtgccaaacttcttcagtggcgtacatattcttgatggccttgtcttcagcaactccacggccggtttcttcataagccatgagtgccaggtccatgtgtttgtcttggccggccattaccatttggtgagtgatgtggtcaactttttcttggtcaaatgaatccataatttcaagtgctttttgcgcttttgataccaagccgttgatgacagtgtcaacatcagttgtgttcgtcttagctgctttggtttcttttactttattatcaatcattgattttcctccaatgaaaagtttataggttgtttgtgctttgttatctttttcacaatattaataatatcacggatttttaaaatgtaaacagttttgttcaaaaaatcacaatttattttttgtaagtgcttgcacactgatataacaatatccaaaacaaaaaggacttgttcagcaagtcctttttttatgaaagcggttccattatttatatgtgaatgatttcacgactttggctatttggtcactttcgtgagtggcttttgaataatcgccaaaagtttctcggattggattcggtcaataatgacattgacagccacctgcattaatttgtcattcagattcttttcttccaatgcccggctgttacggctatccatgttcttgaatgagaacatgagccgtttgataaaagtgtcgtatgcctgctgcggataaatgttggccgtcacctgatcgattccgtgacgaatcgtttccagggaaaaggccggcttcaataagctgatcaaaatcagatcagcaacctgcatggtctgatacttccgcttgaccggtgccataatcgctttgttcttgacgtaattgttgatcattgccggagtgactttatcaattccgattggccccaacgtctcgttcaccagtgccacgagttgatccatgtacaattcaaatttgggtaaatctgcccacagcggcaattccacctgcttgagtttttgttcccactgctcgtattgttcttcattgtatgccatgttatcactccttcgagtttattataccacgttagctagtatgtgacactagatagtctaacttggagtggagtaagaggcgctttgatctcagaatttaagccggcaaaccaaatactcctgactttggaataattggtttgccggcttaaatggccgggatcagccgattgctgcacgtttccgctagataacagtggcgctcagcatctcagtcgtctcgcttttatttacttcccgcttgtttgcgcagtcgtctcttctcgcgtttgtccaagacagtggcaataaccccctgcatgaacatgtagagcggataggccgttgcgataagcggaatggcatacagccaaatgtctttattaaagaaggagaccaacgagaaaatattattaaagaagatgatgatcgttaaaaatgccaccagtaccaggatgtccatcccaatcttcagccggttcagtggccgtgataccatcactaatgccaaccagcaaattgccccggtcaacaggacacacagcgttgaggtgaactcgtattggagtccaaaaagctggccgatgatttcaattaacatcacgtagccaacaacacaaatcgctgctggcgttgagatgatcaacacctgcttcatgaactgattggtaatcttgttgaagttaggctccaaagccaagaagaacgatggaattcccaccattaacgatgtaatcggagtcaactgaataggttcaaaggggtaccccgtggcaaagaagacaaagataaatgacaacgcaacggagtacatcgtcttaatcaggtacatagaagcaacccgctcgatgttattaataacccggcggccttctttcaagacatcaatcatggcgtcaaaattggaattaatcagcacaaagtcagcaatactcttggtgctctcacttccggaagccatggcgatcccacagtcggcctgtcttaaagcaagtaaatcgttaaccccgtcgccagtcatggcaacggtatgttttttggactggagaccggcaatcagccgcttcttttggtcaggggttacccggccaaaaacggtattgttggcagcaatttccccaaagtcgtcttcatccttaaccgttgtcatatcaacgctgttggcagcatcctgaatgccggcctgttgagcaattgtggaaacggtggtcgggtcatccccggaaatcaccttgatattgacatcttgattgcggaaatattcgaaagtgttggcagcattgggccggatgacatcagaaatcaataccaggccaatcaactttggtgcgtcaagtggctttcgtggatccaaatcatccacttgggcaaccgccaggactcggtaccctttccgggcattttgagtaatcacggcttgaacctgttcatccaagtgttcaaaaataaactgcggtgccccaaacacatagtcgtggccatcactcaaaccaacgccactccactttcgatccgaggagaatgggatgatcttttcggtctttagctcaggatcatcaacagcatctttgatcgcgttggccgtttcattcgcgtcaccggtgccataggtaatcccggcaaccactttttcaacttccgcggcagaaacatccttcatcatgggaattgcctcgacaaattttagatcgccgctggtaatcgtcccggttttgtccaaacaaatcacgtcaacccgggccaaggtttcaatggctggcaggtcccgcaccagcgttttcttacgggccaaatgcatcgccgaaaccgccagtgtcattgaggttaacagcaccaagccttccggaatcatgccaatcatcgctgcagcagaacccagaatggcccgattgatgccggtgccgccatataatttggcaacaaataaaataattcccagtggaatgatgacgtacgtcaaaactttgataatccgattaatcgtatttaacagaatgctggaggcgtcctcgccctgcttggcttcgttggataaatggttaacaaaggtgtccgcaccaacagttgtcacctgcattttgccggaaccgccgaccagatacgtaccggaggttaatggatccccaatatttttggaaatggttaccgactcaccggtaatcggggattcatcgacttcaatcccccgtgaccggacgacgatgccgtcaaccgggatctggtcgcctcgtcccaactggataatatcgcccaggacaatatcgttggagtggacctgcagatcctcaccgtttctaatcacgttaatttttccttccgccaataagaccattttgtcgacttggcgtttggaacggatttcttggataatcccaatcgcggtgttaaagatagcaatccccagaaacagcagatttttgtagctgccggtgtagaaaaccagcgcccccaaaatcacgttaatcaagttaaaaagcgtgaacgtattgtcgcgcaaaatatccgaaacacttcgggtaagtgattcctcgccagtatttttgtggccgtctttaatgagttgctcaacttgagcgtcactcaatccaacttcggggtcgacctgttgactatttccgtctgccatcgcttaacacctcgctttaccataattgtacaaaattacggccgaaaatcacatttatttggacgcaacgaattaagtttatcggatttttatgattttcaggccaaaacgttgccaaacatcgactggcgggtatgctaaaatgaatctaactaactcgcaagggggaaatgaaatgtttcaaccagataaaagcacctatcaattagacgatggccatcaaatgccaaagcttggtttcggcacttataaaatcgacaatcccgaattaatggatcattcggtagccactgcctatgacagtggctaccgaatgtttgataccgcgcaactctaccgcaacgaaaaacagctcggcgacgccatcaaaaaagttgccagaagagaagatgtcttcattatcgacaaggtcatggaaatgaaccagggccatgatttgaccattaacagcaccgatttttcactccagcagctgggcaccgactacgttgatctcttattaattcactggccggtcgctgaacacttctttgaaacttggcaggcaatggaagaattgaagaagcagggcaaggccaaatcaatcggcgtcagcaatttcacccgttcccaattggaattactgaagacccaggccaacgaaatgccggtggtcaaccagattgaaacccacccatatctcactcagcagcctttgatcgatttcgacaagaagatgtcgatcgtgacccaggcgtggagtccgttgggaagaggcattgtcttggataatccgatgctcaataagatggccaagcatcatggcaaaacgccggcccaaattattttaagatgggacctccaacgcggaatctccatcatccccaagtcaaagacgccggcgagagtcaaagaaaataccgaattggactttgaactcagcccagacgagatgagcatgattgacgtcatgaataagaaccagcgaactggcaatgagcctgaattggtctatgaactgggccaccaatactaatttgggctcgcaaaaaggaggctttcaccatgtccacagaagaacaacggatgctgtccggtaaactctataacgtttacggtaaggacttggccaagaagtacgccaaaaaagatcatttgcttcatcagattaattttgccgaagaagggaccgacgttcaaaagctcttcagacaactgctgggtcgaaccggtaacaacgtctattttgaaccgccgtttttctgcgactttggcggaaacattaccgttggcgatgatgtctactgcaataccaacggcgtcttcttggactccggcaagattaccatcggcagtcgcgtcctgattgggccacgggtcaacttatttgctgccggccacccaattgatgccggtgtccgcaatcaatggctcgggttcgccaagccaattacaatcggcgatgatgtctggattggcggcaacgccaccctgaatcccggtgtgaccattggcaataatgtggtcatcggttccggatcggtggtgactcacgatatccctgccaattcggtggcggtgggaaatccctgccgggtcatttgaccaatcaccgcagatgataaaactgagtgggaaaatcaggaagctgaataccggaaatctttaaagtaatatttcaaatcttaataaggaagtgatggcatggcccttggacaactgacgaatcaaattgtgttgatgtttgtattgatgttaattggtgtcctcatcaacaaagtcgggtttatgcatacccagacttccaacgatctcactaacattctgctgtatatcgtttcgccctgcctgatcattggggcatttgaacaaacctattcggctgctcgcatgaagcaattgatgctggtatgtgtcggcatctgcttcttttacataattgaaatcctcatcgccaaattttcctttggccgcatcagcaacatcgacctacagcgaattaccaaatatgggagcatttactccaacgccgggtttatgggcattcccctgacctccgcattatttggcaacacgggggtcttcttcgccgtcgcgtcactggctggttttaacatttttagctggacccacggtgtttcattatttaaaacgaccaagaagcatcccgaccactggcagaactttcgcgaaatcatcatcaatcccaacatcattgcgatctttgttggcttggttattttcctactatcgtttcagctgccgacaccggtcgaccgcgtcattcactacgtcagctcgattaacacgccgttgtcaatgatcgtcattggtaacagcttgggaaatattcgcatcagccgtcaactgattgactggcacctatggttggcgatcttctttcgcaacctgttattcccaatcgtggcgatgttcattctccaagcattgaccgtttccggggttgccttggatacgactgtattgatggctgcctgcccaacggctggtttggtggttctgttcaccttacaggcatacggagatgccagcccggcagttgcgttgatgagtttatcgaccattttgagtttggcgaccattccgttagtgtttgctgtaatgatggcattttaaatttgataaacctgaataaaaagagggggaaacaaagcattgcgcttgtgtttccccctcttttagcattcattattattccaaaaaaaggattgaccctcatccccacttccagggaatcggcatcaatccctttagctttagtgaaattcgcaatcgtaactggattgttaaattcactaagcaactcaattaaaaattaacgaacgatcttttgacccattacgtcagctaatttctttaaagcatcgtcacgagtcttaatcacatccatgttccaaatgattgtgtcgatttcacctccggcatagtcaaacttttcataatagatgtaaggatccttgtcgctgtctttaaatacattatcgatcttgtcggcaaatccctttgaccagtcatcgtcatccatttctggaatatccttcttggtcacgtaaccttgctcgttaatcagatcaactgcttttttaatttgttcgtcggtgtatttgaggtctttatcattatctcgttcttcggcatcggctttcttttcggcagcactttcctttaccttttcagccatgataacatcccctttattttgatctatcttaatgctagcactgattgaagacaatagttaagaaaaacgaccatttccatcaataatatttcaaacacttttaaaaataccttgtgggggcgtataattagatgtaatctgtaggttacagattgatctaatttgaatatatcatttttgaaatgaggaattgaattttggacgatagccagatactgactaatctaattattgtgatagtaacgtttttgttcgctgctttcttcgtggcaagtgaatttgccctggttcaaacacgggcaagtgcgctggaagaacgcaagaaaaatctagaagaagccaaaggcaataaagccaaggggttaaagaagctcgaccgtgagattcacatggtcaccaacctgaatgaatatctttcgaccacccaagttggtgtcagcttggccggaattatcctaggttatctgggtgaatcatttgtggtcacaattttggttgatgtgatggaaatccacaactcgccaattgatccaaccgctgctcacgctgtgggcgctgtgctggggattatcatcttaacttatttggaagttgtgttaactgaaattgttcccaaaaacattagtattgatatgccaatgcaggtgctgtcctttatcagtacgccactgcattatttccatgtcatcttttatccgtttgtctggttgctcaacatttcagccaacggaatcgttaagatgctgggcttaaaagttgccaacgaaaacgacgagtcgttctcacaagcagaaatcttgaacctgtcgagaaatgccgttaagagcggtgcccttgaacagaacgattatctgtacatgcagcgggccttccagttaaatgataaggttgccaaagacatcatgattgaccggactcagttggtcgtcatcgacattacaaccacggttaaagaagccgttcaagtctatctgcagcaaaagttcagccgaattcctgtggttgccaatggcgataaggataagattctgggctatgtctacaactatgacctgattcgtcaatctcaagttgaccccaccatcaagatcgaccgcctgctcagagatatttcaaccacgccggaaatgacgccgatcactgatgttctccaccaaatgattcagaagcggacaccaattgtcgtcgttgttgacgaatacggtggaacttccggaatcattactgacaaggacatttacgaagagttgtttggaactgttcgggatgaaattgatccatcaattaccgactatatcttcaaacagccaaacggcacctatcaggtgaacggaaaattaaccactcatgactttgagcgatactttgatgctgatttcccagagtttaccaattcagacgccgttaccctggccggatacttcttggataactacccggatatcaaggccggcgacgtgatctcatttgagaacttcgatttcaaaattgttgactacgaaaactcatttatcaactggtttgaggtaaccaagcacaaggtcgtgccaaagcctgacgatgatgacgatcaccatgacaattaatggttaaagtttcaataagactgtgacaagacaattgttttgcgagcagtctttttacatattagagacgatttagacatcataacgtttaagggggatctaacaagtgaaaaagctatggcaaaaaacaccagcgtggatcacatacacggtgctgtttaccgcgctgatctgtgttttagtcggttgcttgttcttaacaggtcgatcaatgatttgggagctggacgggatggcccagcactatcccattttagtgcagctcaggcacatgatactgtcatttctgcacaatccaagtggcggctttactcattgggcctggaacatcagcttagggtccgatcagctgaccaatcttgcttattatgtgattggcgacccgttcaattacctaattgcactatttccaaagagtcagatcgaaaatgtctttgccttactggtctttctccgaatgtatttttccggtctgagctttatgttgtgggcttcatcgtatcaatttaagaagtccagccggatcatcgggtcgatcgcctatgcatttaacggttacgccttggcaactgctttgcaccacccattctttattctgcctttgattttcttcccactgctttgctacggcatcgatcgcgttttacataacaagtcatggctgcaattgatctttgcggtcttcctggtttttttaagcaatttctactttgcctggattctgggatttggttcaattgcttatgtcattctgagaatgctgagcctgagaaaatggcctgattttacgccactcaaatcctttggtaaattggtcctttcagcagcgattggccttgggatggcggccatcgtcttcttgccaacgattattttggcgacgggctccacccgactcaatgacaactttgccaatggcatgactttctttccgctccagtattacttagacattcctggggcaattctaccgactggtcgggcgatgaacttttggctggtcatcgggatttccgggttgtcatatctcggcctggtgtacatgctgaggcactttaaacgctatttatggcaaaatgtcgccctgattaccatgttcatcgggatcctattgccggctgtcggcgccattatgaacgcgatttcgacgccttccaaccgctgggtcttcctggtaaacatcctgtttgggtttgcaacgatggtctttattgaacatctcagcgattttacgaagcaggatatcgcctggttcggttgggcttcgattggcctgattgtcttagtctgggcatttggcggcttcttaatgaatctccagccccacgatttcatcgtctacgggttcttactgctgacagtgattgtggtgatgggctgtgtcgtctttgattggaaacgctcgactaaagtcatcctggtctcaaccgtcttcatgctgaacttatccgccaacatcattggcatttacagtccgcactccagcaaattagcgctgcagcagctaaaccgcggtctggcaacccgatttagcaacgattactttagtggggctcagaaatacctcaaaaaaatgcccggcttcttcagagtttccatgaatccgcggtatcactacaatacccacattcaaaatttagccaactattcgaataccaatacagatttcccaatcaacagtgggctcaacgacacatcagtctatctgaccctgcagaatggttatctgggtaaattctcacagtccgtcggcaacagccaattttcaatgaacacgccgattgcgcaaggtgattatcgaaccgcctttaacaacctgctgggcgtcaagtacatgtttgccaaagccaacaccaagaatccaccggttgtcccttatggctacaaaccagttcgtgacaagaatggccaaatcaaagtctttcctgctaaggcgcggacggatgccgtccaggcaatcgaaaatatgtatgggacgacaatttataaatccaataacgcactgccgctggtttatacgcagtacaacaccgtttcacccagtgcctatgacaaaatgagtgctgtcgatcgggagcgtgtcatgactcaaggggcggtggtgaatcaatcaaagtataatacccatcccctcaattaccaatcacccaagaaaaacattgattataccgtgaaaatggatacctccaagattgtctataacggccgtcaactcaccaagtatcgacttggcattatcaataaagccaactcggatcagctggtcgaccaaccccacgaacaggtcagcctgggtgccaacctgcaaaagaccaaggacctcttggcaaccaaccgctcgatcatcgagactaaccactacaagaacattaatggcctaaaagagatgacctcagacgttgttggtaatccaatcgactataccttgaaggttaagaaccccaaggccaccaagaacactgaattgttcctggttctctccgggattaagcaaaccgatggtacccctgccgaacacagacagtggatggctaaccagttcctgttggataacaaactctactcgcggatgggcaagatggacgagtatcgtcacagcattttgaagcccacctttggcggttacattttcaatgccttcgctaaagatcatcaaaatgggtataaccaatatgacaacaataatctatccaattaccgtcagatcagtaatatcgtccttaatctgggttactcaactcaccaacgcaagaacattgacctcaacttcaatcaggtcaagaacatcaagttcaagtcggccaagctggttgccatgccgttcaataagacttatgacactcaaatgcagaaactcaagcagactaagcctgccaatttgaaagtcaacggcaatcacgtcagcggcacggccaacaaccagcgctctggcacgatggttacctcgattccatactcaactggctggaaattaaccattgatgggaaaccgacgaagaccttcgttgttaataagggctttgtcggcgccaacctgcctgctggccagcaccagatcaagcttgactatacgacgccaggcattaaagtcggcaagttggtttcaggtatcagctggttggcatttatcatcctgctgggctttgcgatcatcggtaaattcttaccggaacgaaccggtcaacagcacaagccaaaacatggcaagagccagtcaaattgaggttgccaactggtggcccaatcgttaaagttaggataacaaacaaatttttcaaaaatcatttccatctaatctgaggaggtccattgtgagcccaataaaaattctattcatttcaattgagggaaatacgcgttcattcgttaaaaatttaaccagttatgcgactggcatgcacgaccaagatccagccaatccattggtggtctcaaaggaaatcagtgaacagacagattttgctgacgagacggaaccattctttgcttttgtcccaacgtatttggacggcggtaacggcattgacaacggcgttaaagagctgatgaccaatgccttaggggaatacatcgcctacgatgacaatgccaaattgtgtcacggaattgttggcagcggcaataaaaatttcaacgagcagtattgtctgaccgccaagcgttacgcctcacagtttaataaacctttccttgcggactacgaactccgcggaaccggccgggatgttgaacggatttataaattgttggcccaaagctaaacgggttccacaattaaattaacaggaatcaaatgattctgaattaatataaagcaactggttatcctcaccctgagaataatcagttgcttttttatatcatcgtcaaaaaaatccagttagcagctgaactaagccaattgctaactggattgatttctacattatttcgtttcagcgagctgttgccgcgtccgccgtcgattcatcgcccacaaaatgaccacaaagataatgatcaagccggctgctagtgagaacagctctttataggacgcaaagtccagcacaatgccgccaatcagcggtccaactgcccggccgcacgacatgaacaggttatacaagccttggaactttccccgttgttgaggcgtcgataagctgtcaatccacgctggaatcccaggaaagccaatcatctccccaattgtcgtcacgatcatcaccaaaacaaaggcagtataatcgcgggcaaagattaaccacacaaacgatgccgcaaagattgccacccctacgtaggtctgagtactcagtttgaagtgcgtcccaatccgattgacgaacggctgaccgatgacaatcatcaacccgtttaacgtccacagtaaactgtaattttcaaatggaatgtgcaggctggtcatgtgcaccggcaggacactttcccataaggcatacgccagatagactgacaggaccacgccacaaattgccagaatcatcccgccaactttggcttcaactggtgcgcctggcttgactggtttcccaggtgcccgccgatcaacgtgaacattgaattccaaaatcgtgatgaggaccagcgcggcataaaaggctgccgtcacggtaaacaccaaggtgaccccatgttttaacaggaagccaaccattaaagtcccaatcacaatcccgacgttttggccaatgtacaagatgttaaagatatcccgtgtcgaacgggtcttgatactggcggcatatgaattcagcagcgtcaaacaagcaccgtcaccaaagccaacgaacagcagcataatcccaaacatcggccagccatggaagaagaccaacgtgacaatggccgtcgttgaaatcagtgaaccgataatcgttgccttgtagggagaccagcgatcaaataaatagccgccaagatagttacccagcatcatacaacacgacatcgccagcaggaccattccggctagcgtcaacgacttatgtaggtagttatgcagatacaccgtcaccagcggccacatgaaagccgccccggcgtttaaaatcagtgaatacacaatgaccgaattaaatctaatttcactccgttgttttatcaattgctcagtcccctcttacactcatttttaaccacaaaatcttctacgtccattttcgcatattaatgacagaaactgtatttattactgaagattatttaaaataattcctttttcagcctaatatcgtcttgatcggtaatctttctcaccacgtgacaaggattgcccactgccagggaattggccggaatatctctggtgaccacactgcccgcgccaatcactgatccgttgccgatcgtcaccccaccgatcacggttacgttactggccaaccagcagttgtcctcaattgtgattggcttgctgtactccttgccgggtaaatcattattggcagcaaagtttcggtcctggtagcgcagtggatgcatcggtgtgaccaagctgatattcggcccaaataagacgttgtcgccgatggtaatcatgccggtatccaaaaatgtgatgttggtgttgccgtagaaatgatcaccaatcttgatgtgagtgccataatccacaaagatcggcccctgcagataaattcgttcagatgaattaggcagcagttgcttcaataaatcagcccgcttctcacgttcatcatcaaaggtgtcgttatattgtttgaccagccgatgggccaatcgctgacgcgccaataattcggggtcgcggggattgctcaatttgccggcaagcattcgttgatcttcattcatcattaaggcctccaaacctttgagttacagctatcatagcataggcagagtggaacacgaggcgttttgatcccagaatttaaggcacaaatcgagttattcctgttcttggaatgactcgatttgtgccttaaatggccgggatcagcctcgcgttccacgtttaatcaaggataacagtagaaactcaaaaagaggctggaacataacataaaagcagtcatgtcccagccccgaatcaaatagctggttaaaattatttaactaaagcaaatttgtagtagtgaagcggtgtgttgccatattgaaccttgatcgcatggttggctttgttgacaatgatgaaatgcgtattgtcagtgaatctcaagtagaacttgtggtaagtcttgctgccgcgttcacggtaagtaattccccagaaggtctttgagtaagtcgtaactttgtagttggcgaagttgatcagcttcttttgatacttgccattcttatacaagccttggttcaaaccacccttttggctgaagttggtgacaacgctgtagccattgttgttgcctgattgccaacgaccagttggttctgaaatgttgatcttactgctggttgatttggtgcttgaaccagtcgtggttgttgtcgtggcagtcttaggagtcttaacggtcataattcggtagaagtatgaggttgatgacttccgggcgtagacataaagcttctggttggctttaacactggtgtgcagctcggcgctgaacttgccagttgaactgtcagcagtggtgctggcaatggtggttttgttggtgtttcgaacaataatggcaacacctttggtggcagttccagtcactgcctttgaggtcgtgtaaatgttattgactttaagtgacggagaacttgcagaagcgttgacactgaacccaatcaaaaatgatgcgaggacagcaaagaacgcgataaacttaaatttcttcatttgatattgctccctaatctttattttgcatgactcattataaaggatatgggcaaaaaaagccgtcaagtcggccttcatttatccttttcttaagaaaaccgtcactgtttaggcatcgcttttagcgggctaattatgaaaagaatatgcttgtaaattttattcatttacattggcaattcgcttttgttggggtctcatgtgttatataatgttggggaactggtatagacatataccaaattacttagttaatattctgataggagtgaacattttgccaactgaaagacgttctttgattatgctcttcggagcaactggtgaccttgccactcgtaaactttatcccgcaatgttaaagcttttcgagaagggaaacattcgcgatcactttgctgtgattggaacttcccgttacaagttcgatgatgaaaaataccgtgaaatggtcatcaagtctgtttctaaagaatctactaataaaaaacaaattgctgatttcgccagccatttctattttgtgacccatgatgtgactgaccttgaacactattctgtattgaaaaacaaagccaacgagttggacaagaagtatgaattgaacgggaaccgcgtgttctacatttcaatggcacccaacttcttcggaaccgttgctaaaaaccttaaggctcaacaccttctctccgaaggaaacggctttaaccgcttggtcattgaaaagccatttggccgtgatttcgaatcagccaaacagttaaacgacgacctaagcaatgcctttgaagaagaccaaatcttccgaattgaccattacttaggtaaggaaatgatccaaaacatcgaagctattcgtttcggtaacaccattttcgaagccctctggaacaaccgttacatcgacaacattcaagtcacccttgctgagaagctgggtgttgaagagcgtgccggttactacgacaactccggtgcccttcgtgacatggttcaaaaccacatcatgcagattgtcagtttgcttgcgatggaacaaccggttgcgttcaaggatactgatatccgtgctgaaaaagtcaaagcattgcgtagcctgcgggtttacaacgttgcagaagcatcaagcaactttgtccgtggtcaatacgctgccgttggtaacgataaagaataccgtgaagaagacggtgttccaaaggattccaacactgaaacctttgttgccggcaagttgttattcgataactaccgttggtcaggcacaccgttctacattagaaccggtaagaaactcgctgacaagttcacccgagttgatgttgtcttcaagaagccattagttgacatcttcgccttcccacaaagcggcagtgcaccactgagtgccaacgttttgactatcttcatcgaaccaaaccaaggcttctcattgatggttaacgccaagaactccgaacaaggattccacactgaacccgttcagttgcaataccttgaagattcaaagcgcacccgcgaaacaccacaaccttacgaacgcttaatccacgacgttttgaagggcgacggtaccaacttcgccagctggccagaagttgccagtgcttggaagtttgttgatcaaatccgtcgagtttgggatattcaacaaccaatgttccctaactacattccaggatcaatgggcccagtttcagctgatgaattgcttgcccgcgatcaccgtgaatgggtatacaaattgaataagtaacatctaaccaatttagctgaccgaaaaccaattcgttttcggtcagctttttgtttgggttaacgtttgaaataaattgtaaatttttaccattttgctgaaagtccatggatccagatttacatttttcaagcaacaaaatccctcaatgattgaaaatcggtcattttgaattatgtaagcgctccccacaaaacgacttttcattttcacaatctctcatctaacaaattcggcatactgttccaacgcgtttttgtttcactttccacttgtgagatggtacactaattgtgtagtaattcttatatagaaaaggatggttttgaaatggctgatcaaaaagcaaacattggtgttgttggtatggctgttatgggtaagaacttagcccttaacatcgaaagccgcggttacactgttggcattttcaacagaaccggctccaagactgaagcagttatgaaggatcatggagacaagaaactagttccaagttacaagattgaagactttgttaaatcacttgaaacgcctcgtcgaattattttaatggttaaggctggtaaaccaaccgatgctgttattgatgaattactgccactcctcgataaaggcgatgtcctgatcgatggtggtaacacaaacttccacgatacgatggctcgaaatgcccgtcttgataaatcaggaatcaactttatcggcatgggtgtctcaggtggtgaacttggtgccttacaaggaccatcattgatgccaggcggccaaaaagaagcttatgatttggtagaaccaattctcaagcaaatcgctgccaaggcacctgctgacggcgaaccatgtgttacttacattggaccaaatggtgccggacactacgttaagatggtgcacaacggtatcgaatatggtgatgaagagttaattgatgaaagttacaacattttaagaaaccttgccggctactcagttgatgaattggctgacatctttaaagattggaacaaaggtgaactcgacagctacttaatcgaaattaccgccgacattttgactcataaggatgatattggtgctgacaagaccaagccaatcgttgacatgattcttgaccgtggtgccaacaaaggaactggtaagtggagctcacaagatgccctcgaagtcggtgttgaccaatcagtgatcaccgaagccgtttacgctcgttatatctcaatgatcaagaacgaacgtgtcgcagcatccaaagtcctccctaagccggaaggcaaagttgattttgataagaaagaaatcgttgaaaaagttcgtgaagccctctacttcggtaaagttatgagttatgcccagggctttgctcaattaaaggctgcttcagaacaatacaagtgggatatccaattaggcgaaatggccaagatttggagagccggctgcattattcgtgcccgattccttcaaaacattaccgacgcctacgacaagaacccagatttgcaaaacctgctgctggatccatacttcacggatatcgccaagaagtatcaagaatcagcacgtgacgtcgtagcattggcaaccaaggccggcgtcccagtaccatcattagccgccgctgtctcatactacgactcatatcgttcagaagttgtcccagcaaacttgctccaagcacaacgtgactacttcggtgcccacacctatgagcgtgtcgaccgtccagggagtttccattatacttggtatgaagaacaatagagtgccctttaagccggttagcttttgagcattaatggaataacaggtgttgatgcgctttttgcatcaatgcctgttattttattaatgctcaaaagctggcttaaatggcacgtttccactatgtagaagtcgagaacacactactcaacctgttggaagaacagtagtgagcgacgaaacccgggttgaccccggaacataagtcagaaaaatcatggatgaacgcttcttgttcatccatgatttttttggcttatgtggtaggggtcagggttgtcggagctgtcctcaaaggcagccaaatctgaaaaataaccataaatgccaatcaagcttttgagcattaatttaacaaggaccgttaacgctgtttttacgttaacggtccttattggactaagcgggaattccgactctttacaaaaagagctagcactaacacaccagctcttggtatttcacttaattggcagccacaatgtcgaccgccaaggtacataagcgtttacgaagtttatcaggaacttgaccaatgatcgcgccgttacgggcaacataatcataattgggtgtttgccaagtcacaatatagccattggtacgactacttgggtcaagaatcggttcgaatcccttttgaatttgactagtgccgtgcgtgataggcatcacgacaacaaatcctgtcaaccgattatattgggcgttcgataccaccactgctggtcgtcgcaggtggctagtcgtatgtccgcccatttcatgcccagtgtgggggtcaaaatctaaaacaataatatcgccttgttcaggaaaggatgtactcataattcccgacctttccttgactcgtttccaacattgaaaccaatctcgtcaatctggctacgaaaatcaacattgtcatatgcgcccgatatccacgggtttttatggctgtgggcgcgccggataatcaaagtatcttcatccactttttcaattaccaccggctcgttgctcgaaaatcctgtgcttttaggcaaggttacgctgaccgaattgccagttttatgcgtttttgtgtttgcaatttttaagttattcatgatcaattcctccctaaaatttgagctaagtatatcgtaattacaatgttattacaagtacttaccttggtaaatacccatcctttaagatgagctgatcttgatatttgagcatcaaatttgttcactcaagcactcagataacatacccactcaatcactgtcaaattaacaccaaatccctttccaggattcaaattcaaaatcccattaataaaaattgctcgcaatcatattaaaatactatatttattgttataataattatagataggaaaacagttatagagtgagggctcttgaattgactgtttccaagtagacatgatggccaacttggctcacaccattgacaaggatgccgtcagcaaagcacttcagtgtgctcaaatcaattttgaaaatagattatttcaatgcttcgacataatattcatgcctatatcgttatacataaccaacaggggggtgatgataacgcattactttttgacgtcgcagattgatgagaacacatctgcgatcgaaattgcggagattcaacgattacatttgttttcgaaactcaaggttcctgccaagattgtgacccgcaatcgcaatcgtggtagtaatcgggtgttacagcagctaatcgacaatcatcaaatcattaacctctaccaatactttactgagcttcccaaccaaaccgagccgatgcccaaagctgaagatgtgttgcacgatttcaccaacattccgattgaaaataatctgggatataaggacggcaagctccgggttcgggtcaatgaacagaatggctggatcaataacatcgattatttggacccgttcggcttcaccgaccgtcgcgacctgtacgacttcaatcagcgggtgtcttcagaatactttgacgatcatgcaaaattaatcacgcgggtattctatcaaaaagatgggcacatcgtcatgactgaatactatcggggtggccctggcaaccagccggtgctgacactgattcacttacggcataacggccggctctggcagttcgataatcaagatgagttaatgggctactttcttgactgcctggcaacagacgattccaacgccacgttttatagtgaccgcgaggacgttgccatccccgcatttaaattgatgaccaagcccgccaaacgctatcccattttgcattctatttttacgcaaaatgccaagcacgatggtgagctatttccatatttccagcaagcaattgaactaaaggacaagttatccggcatcatcgtttccactcagcaggaagccagtgacattcagtcgcggttcccgatggttcaaacgaccgttattccggtcagttaccttgacgaccagctgattcatcagtcggaatcatttagcgaccggattcccggcaaagtgattgctgtcgcgcggatcacgccgttaaaacagctgagccacattattcaagccattatcttagttcatcaacacctgcccttcgttactctggatatttatgggtacgaaaatgtcaatgattttcaggaaggcaacaagctgcgccaactcgtcaaaacatctggggctgagagctatatcactttcaaaggctacgttcacgatttggcgtcagtctatcagcacgcggacttgttaaccctgaccagttcatatgaggggtttgcaatggcgatcttagaagcccttggttacgggtgcccggtccttagctacgatatcaattacgggccggcagaaatgattcaagacaagcataacggggaactaatcacagccggcgatgaacgcgaactttatcgccgactgctgcacctgttgacacaccgagagatccttcaacgatacggtcaaaatgcgccggcgtctgttgagaagtattcggcaagccatgtgcagcagatgtggcacaactttattcaaaatcaatgaatgacaaactaattgaacaattcaattaagttcatttctacaaaatacattattcgaggggaaataataccatgacaaaattaaatcgaaccaattcaaaggttcattacaaaatgtataaggccgggaaacattggctgtacgcttcactactcaccgttggcttgatggccggcggtgcgtttggtgccagcacagtcgaagccgataccagcgataatcaggcaccggcaccaactacgacagctgcgactactcaaccgagtgccgatacgcaaaccgctgcccaaaccagttcagctgacagctcgacagccacaacggataatagccagactccagctcagtcacagaacactgcagcgacgaccacttctgattctaaccaagcaagtggtgcaaccaccacgactcctgacgctaatcaaacaagtggtgcaaccactccagcaacgacggcagatgatcagggaactgatcaagcaccgactgcggatcctgcaacaacggagacgaataactcgacccagacgactgggactgatcaagagagtaatcaacccgcaacgactacgaatacgactaatgatccatctacaaccggcactgacaatgatgccaccacgactgacccatcgaaccagacaagcgaccaacctgatcaaaatgcggctgacgaccagaacaaagcctctgacccaaccacaaccgatgatcagaacacggccactactgaaaacactgatgcaactgctgattccgcaaagacagccactaccgcggaccccactgcttcatcggcaacagccgatcagactgcttcgttagccaagacacccattgatacccagtcactggcggacccaaattccagtgatttttgggaacaggtctttcaactagcgactattattccacaagccattgccggcgcagtcatttcggcacctgcaattcttggtggtgggacaatatccttgtatccgattaactcctcatcggaaccgatcgtgattcctggacgagttcttcagttcttaactggtggactgtggtcttccccttgggatatttggaatgccttgaaggatgggttggggcttaatagcagctcaaccactaccaccgcccctgtaactagtcctaatcaaagtgaaacgacaaacttagcgaccgcgagtgtttccggccaacctatagattttggtgatacgattggcgagtttattgattccatggtggccaccattcttggggaactgcagtacccaatactttctgacgtccctggaatcattctgtgggttactccatccacgcctaatcagccaactgaaccaaaccaaccaactcagccgaaccagccgacgcaaccgaaccagccaactcagccgaaccagccgacacaacctaaccaaccaactcagcctaatcagccaacgcaacctaatcaaccaacgcaacctaatcagccaacgcaaccaaataagccaaataagccaaataagccaaataagccaaataagccaaataaaccaaatcggcctaatcagccgaataagccaaataaaccaaatcgaccgaatcagccgaataagccaaataaaccgacacaacctaatcgaccaaatacgccgaataaaccaagtcggccaaatcagcctaaccagccaaccaagtcgactcactccaattggccgactaagccaaatcattcaacgggaaccactactaaccgcacatcgcggaattcccgagatataactggcaagacaccaattgaaaaagcatccgtcttaccacaaactggtgataagcgacaaaattggctcagtattctgggtgacgtttcattggccgtcattatcatttccggcgccatgattttcaaacggcgtaagcgtgattaattaattttgaataaatcacgtaagttctacatttcataaatcttcagatgcttaaaatggcccatggccaaattccgatcatgattgttctcacgaacatcatgttaccgggatttggccatgggccattctttgtctaaatggttatttaacgggtcaacaattaaccaaacgctagccctgctcgccagccttaatcttcttaccaaaagcagtttcatcaaaatgatcgatcacgttttgaagatccgccttggttaagctagcgccaaacagctcactgccgggctccgtcatgatgccgtcagcaatgttgtaataaaccacggtgtcaaagcccatgctgtcgacaaattcagccacttgatcaacggctgcttggttatcgccggtcacaaacaacgctttgcgattgtctgctccagctggtttggcctcttcctgcaggttgtgatagcccatgtggttaaatgttttcaccacggtactcttattgaaatactgctgaacctgttcactggaagtcgacgatggatccaaaacttcttctcgaatcccgtcagtttcccaccagtagttcatggcatcgatcaccaatttgccctttaagagcttggatttgatgttcttgtagcggctcagtggaatcgctaagataatcagatcacttttggcaacaaccccttgattggtcgccggaactgcacccggtaccaaagtctcgatggtcatggcaattttttcgaccgatccggaaccggaaattcgcacgtggtagccagcctttaacgctaactgagctaatacgatacctactttgccggcacccaggatgcccacatttttaatttcagccatgcttagccctcctcagacaaaatttctttgacgcgaggaatcaccttagtcgcgtacagctcaatcatgcgttcacgctgggcagccgtctggttgccggcaccgtaaaccaagtcaaatcgacccaggttcatcaggttgatggtgcgggccattcgttgggcgacgtgttccggattaccgacgtaaaatgagccgaccttggtttcaccgtcaaattgttcccgactcatcggggcccagccgcgagttaaaccgatgcggtcgaagttggccttgatattcttccaagcaacttcaacggcctgatcctcatcgtcagcaataaagccatgagagtgaacggcaacgggttgaaccggcatattgtatttttcggcagctttcttgtacaaattcaaatacggcacaaaacgatccgcctggccgccgataatcgccaagatgaccttgtaaccataccgggcagtccgaataattgattcgggtgagccgccgataccgatgtaagtttcaatgccgttataatcggtctttggatagacatcctgatccttcaaggattgggtaaatttgccatcccaagtaatcggcttttccttaatcagttggctgtacatctctaatttttcattgaataaatcatcatagtcggttaaatcataaccaaagagtggaaatgattccgtgaaggatccccggccaagcatcacttgagcgcggccttgagataagccttcaagcgtggcaaaccgttcatagactctgaccggatcatcagagcttagcacagtcaccgcggtcgccagcttgatgcggtcagtcactgaagcaagtgcgcccaggacaatttcaggacttgagacactgtaatcgggccggtgatgttcgccgatcccaaagacatcgacgcccagcttgtcagccagctcgccttctttcacgatttggcgaatggattggccagccgtcaacagctcgccgtcttctccccgaacgatatcgccaaacgtttcgaggccaaattgtaatttgtctacatcaaccatgctcatgctttttcctcccgttgcttactttttgtaagtatgataatagattatagtaatttgggggaaattgcaactaaaatagctggggaattggcttcaaaagtctaaaggcagaaattaggactcgcacaataacaggcaaggctgaaagttagttcaaatcatattcaaactgttggaaaaaggattgaagccgccattgaataaattaattcatacgtaaagtccccctaaaaccccagaaaatgggcacatttacagttaaagacagttggggttcacgactttcaaataacgtgttaacagcggtcaattttttgacccactaaatcgaatttatcccattttaagtagccaactgccgatctttaagataaaataatatgaagatccagagataaccacaattttaactgaaagaaccgagaggcagaataagacagagggacatcaaatgactataaagccttggaaaagccgatatgagcttgccaaaacactgattgatgaacgactcctacaaaatactaatgttgaagagattgaatccacattaaaaaagatgaattattttcaactgatcaatggattagaaaatgatctcttatctcaaaaggtcccgaaatgttttcgtacggaaacttttgatgattttaaacgtttatacaaattcaataagcaacttgaaagtgcaatatttatcctgattgaagattttgaagatcagctaaaaacatcccttgcacataatttcagcgcaaatcattgccgaactctgaatgatacaatgcaatacaccaataagaacaattattacaacatcaagaatgactatcagtatccctttactcgttatcaatacaaatatacgtatgaaaattttgacaagtttgaactatttaagccaaacttcattgataaattaatccgaaacaatgactttatagatcccaaattttatcaagatccaaactatgtgcaaccaccaggagttaccccctatcataagaataaccaagttgccgtccctctatgggttacagtgcaaacactcgatttcggcacattaataaaaatgactcactatttaaaaccggctgatatgaccggtattctaagtgattttaacttcaaaccgagctcgagatttgcgtttttaagtgcacttgacgtaatcaaggagcttcgaaataagtgtgcacatggcttccttattgaaagattttcaacaccagaatatattaagctcaaccgtaatttagtgactaaattatcactcgatccctatcacaaaggcggtaatagcgtctttccgtcaaggctaaaattgttcgattctttaaaagtcctaggaatgtttgttgatttaaggcctttgggaaagattttcaagagtttgatataccaaaacaataaaaacttctcgaaaaatagttatgatttaaattccagaatactgcaggatattggcgccccatcatataaagcgttaaaagccgcctgcgttgacagtgttagtaatagatggtaaattaaatgtacagagaaataaatagggccttaaggccacaaggcggcagttcctttggtgccttcgataaaacggttcttcgtcaactgttgttggtgaacaaaatattggagttctaatcacttggtgattagggctctttttgtatgaactcgaaaagcgaacagcactcttagccggaatctgaagaagtttcggtaaccaaatccagtgcgcttaatgactttaatcttgttgtttgaaccttctaatggcccgttggtgtagtggtgggtgaaagtgttgccaatttcatcatgatgagccgccaaggtttggagggctgccaacatctcttccgagcacccctgcaggtggtgaaaggcttgattatagttgggccagtcgcggtttttgatggtttcacgtaaccgattcatcacgtcgtaagtttgcttgagctcgggatcaatgtccagtaaagcatcaaccacatccgtggcagttgccggataagggaagtttgtccacttacggaaagcctcgtagttaaggtgattggccggcgttaataatagtttccaatagcgtttcaaggcgtgatactggcgtgaggaagtggccagggttttcatgagacgcactcgcgtcttattaaaagcccggtttaaagcgttaaccaggtggaagggatcgatgacaacgatggcgttcgggaagatctgcccaaccaatttgggataggtatagttcatatcggtgacgataattttcacattttctcgcgcggcttggtcataatgttggaagtacttttgaagctgatagatggttctaaagggcaacaggtcaatcaattcgtgggtttccgcgtccataaattcaaagctcatcgcgtcggtggcgctcttagtacttttaacttcgtccatgaggagaactttgggtaagtagtgccagttggtttgaaagtcgtgttcagcgcgcaagagctgccgaccaacgaatgaatccgaagtggacaattcattggcaatgtgtttgaggctcactggttccgttaacttctctaaacattgtttccgggttgtatttgaaatcgtgcagtgcttcggcactgcactcgtctgcgccaggaagttggtatgacaagccttacagtgaaagtttcgccgattgaggcataggataaccgtgctgcccaatattttagcgaatctaatggtggtcttccgccaaccatagccaatgatctggtgatcattaataaccccacaattgcggcaggccttgggagaatagttcagtgatccatttaatctgattaccccatcatcacctattttgccattctcaatttttaagtgttcatcatctattcctaacaacattttcgtagtatcatttgacatagggcatttccttctttctctaaaatcttcgtggttgttggttttgatgaacggacaggaaatgtccgctttttttattctaatgaaaaacaaaaaatctgtcatcagtaatagataaaaatctattaccaacaacagatattgtagagccgataaaacagctactcattacgagtagctgtttttggtttcttaagctggaatttaaattctaaatgaggccaattgtagctgtcacttatgatcctgcaagaaatacattttaagtcaacaatgaaccaaaagattgtttagattccttctgcagtatttgctgaatgtatgttgcttctggaacactattcgtggcccgatataatttacccaatagcttcctcaaccgcatcccgcaactcccgggtagcactcgccggatcggcagccttcataatcgcagaaaccacagccaccccatcaacgtgggcaccatcaattgcctcgacattatcggccttcaagccgccaatcgcatacacgggaatatccaccaatcgtttgatcttaccaagggtttctaccgtcgtatgaacggtcttaacgtgtgtcgtggttgggaaaatggctccggttcccaggtaatcggcgcccatctcttcagctgctttagcctgcttcaatgtcttggccgttgcaccgataatcttcttgggtcctaagattcggcgagcgatgtctaccggcaaatcactttgaccaagatgaacaccggcggcatcaaccgcttgagcaatgtccaatcggtcatcaataatcaggggaatcttgtaccgatcggtaatggcctttacctttagagcaagttcaaaaatttcgcggctactgccctctttttgcctaagttggaccaagccaaccccattttgcacacccgcttcaatcgcgccaaagaattgttcatcagtcaatccggtgtggtccgtcaccaaatagagtggtcgatttgttagtttcacaatcatttcctccaatattttctcatttgccatcagtgtaaatgaacctcggcaaaaagtatagaagtatttctcacttgactttcagattgtaagcggttataaatagattatgagcttgagcaaagtttcaagcctaattgaatatttcgtctggggtgcctgaaacggctgagattacacccatcgaacctgatgtagtttgtactgccgaaggaagagcgaatttaatgttgaatttattttgaccttaaaccttctttttgcagaaaagaaggtttttcttttctgtgaatcgaacttaatgttgaaaagacatccactgacctctttcttcggaatctgaagaaaggggtctttttgtatggtgatggttaacggtgaacaagaatccggtatggttggtcaaacaatcaccgagttcttgaaacaaagagaagcaccaattgaaaacatcgtcgtcgaacagaacggcaagattgtccaccgctctgaatttgacacaactaaaattgccgacaacgacaaactggagttaatctcgtttgttggtggcggttaggatggtggttccaagcaggagtctccttgtaagcacctcggaagcaaatccccaaaaccagggaatttacttccgaggagacttacaatccgacggccgtgaaacgcctagcctacttggcgactcctaaccgcttggatccgctcactgattaggacagctcctccaagcaggagtctgcctgtaagcaccttcaagataaattccaaaaccgggaatttctcttgaaggagacttacactccgactcctaaccgcttggatccgctcactgatataaaaggagtcgattgacaacatgcaagaaccagaaattcaaggaatgagttacgatgacgtttatctcggcatgaaagaacgcaatgttaaggggtcaactgacaaattagctgccgctcacgtcacgattgccggggccggtggtttagggtccaatatcgcgattgcgctgacccggattggcgtcggccacttgacgttgattgactttgacacagttgagctcagtaacctcaaccgtcagcaatttaaactcagtcaggtggacatgccaaaagttgtggccttaaagcaaaacctgcaggaatttaatccgttcgtggaaattcaaattcaccaaactaaagtgactcatgacaacgtcaaagaattgttcgaagacgctgacatcatcactgaagcgttcgataaccctgctgccaaggcgatgctgctggatgccgcatccgagttctatcccgacaagccaattgtgatgggcaccgggatggccggcattcacagttccaacacgattaccaccaagcatctccgcaagaatttatacatcgctggtgacggtgaatccatgggggctgagggcttgatggcaccgcgggtcatgattgcggccggtcacgaagccaatatgattacccggttaattttaggagatacagaaatctgaggaggatttattcatggcaaacgaaaaagatgagttaatgattggcggacacgccttcacatctcgatttattttaggttcaggaaaatattcatacgatttgattgattcagccattaataacgccaaggcacaaatcatcacgatggccctgcgccgcaacaagaccggcaaggaaaacatcttaaactacattcctgaaggcatcaccattttgcccaacacgtcaggctcgaccaacgctgaagaagccattcggactgcgcgaattgcccgtgaactaagcggcagcaatttcatcaaattggaagtcgttcccgacaagaaatatttgatgccggacaactacgaaaccctcaaggcaaccgaagttttggctaacgaaggcttcatcgtcatgccgtacatgctgccggacttgaatgtcgctcaccagttggtcgatgccggagctgccaccgtcatgcctttgggcgcaccaatcggtaccaacaaaggattgtccaccaaagacttaatccaaattttgattgacgaaattgacctgccaattatcgttgacgccggcattggtcgaccaagtcaagctgccgaagccatggaaatgggtgccgcagctgtcatggccaacacctcaatggcgaccgccggcaacattccgttaatggccgaagccttcaagctggccgttgaagcaggccgcaaagcttacttagcaaaaccaggccgggtcatcgaacacggggcggttgcctcatcgccacttactggtgtcagcgcggtaaaataggggcggtcatatgacaacaacccaattaactgaactcgcacatcgtttagcgacaatcaaccaatttaagaccaacgaagccggtcaaaaccggctggtctattcaccaacctgggttgaggctcaaagacaagtcatcaaatgggggcttgagcttggctttcaggtaagcgttgatgactttgggactgcctatctggatatgccgggaaccacagaaccggaagcagtcattgcgaccggctcacacattgatactgtcgcgcaaggcggtcaatatgacggcttgtacggggtacttggtggccttcaggcaattgaaaatctggtaacagaattcggccgtccgcagaaaacgcttcgactgatttcattcagcgaagaagagggcagccgctttccggatacctttaccggttcgaagcactataccggccaacaggtggatttgacgatgaaggatcctgccggcattcaatttgatgatgctcgaaaacaggcggttatcaagttgatgctcgctggcgttcaccaccaactgccggatttaccggacacctttaccgaactgcacatcgaacagggaccgcgattaattgaccagggtttacaaatcggcttggttaaaagcattgtcggccaacgccggtacaccgtcaccgttaaggggatcgccaatcacgccggcaccacgccgatgaatgaccgagcggatgccctgcagcacgctgtggatctcatcgtcgccctgcgagaacaggcccgtcgattgaatccggatttaactttcacggttggggaaatgcacatttcgcccaatacgtccaacgttatccccggcctggtcacgtttacggttgactgccggaatagtgatgaagccgttttggatcaatttgaacgactccttcagcaaaccgttacggctcctggcaaccaacggattaccagcacggccaatcgctgggcgaaaagcgacgttacccggctggatcgccaattgctcgagaataatcaggcaattgctaatcaactgggcttcaaatccattcagctggcctccggtgccggtcacgacagtcaaatcatggctaagcacactcggacgacaatgatttttgtcccaagcatcaacggcatcagccatgcgccagctgagaacaccagccaagaagatttacttcgcggcgttgagctgttagccgcaagcctccaccaacaagcctattaagtttgggggaaccattttgaaacacattagtataactgcacaaattggaatcggcatgattggcggggcacttcttggattggcatttggtccaaaaatcgccggcatccaattactgggaaatattttccttcgcctgattcaaatggcggtcgtcctgctcattttcggggcggtcatcgaagcactgggcagcttaaaatccgatcaactgggaagattgggtggcaaaactgccatgtggttcttgatcacaaccttaattgcagcagtcctcggcttggccattggctacgcagtcaatccgggcagcggcatcaagctggcttcggtcagcacatctgcaacggtcgccaaggcagggactagttttagccagactgtcttagatttctttccgacaaacatttttgacgccctcgccaaaggtaatgtgattcaggtgattattttcgcaattctgtttgggatcgttttgaaccgtgccaatactgacggcaaattcaatcaagtgttgagtttcgtcaaacagatgaaccagctaactgtcaagctggtcatgctggtgatgaagctcgcccccatcggaattgccgccttgatggcctgggtaaccgctaccagcgggattaaagtcatcctgcccctgctcaagttcctaaccgcatttgggctgggctcgatcgctttcttgattgtcctgtttagcttcatcagctggtacgccaaagtaccgctcagaggattggtccgcggcttttcaagaattattttggttgcttttacaacaacttcgtcagcaatttcacttccaattgaaatggaagatgctgaaaaccggttgggggtcgaaaaatcgattagccaactggtattaccgctggggatggcgttaaacagcaatggtttggcgatgtatttgtcactgtcatgcttgacgctcacccaactttacgggatgtctgtttcaccaatgtcgatggtcaaaattgtcctgctgtcagtgatcgcttgcttgggaacggttgtcgttcccggcggcggcctggttgcattgacaatcgttgtcccaactttgggactgccattgcaaagcattgccattttagccggcattgactggttctcaggaatgtttcgaaccgtcctcaacgtggttggagatacgacaaccgcgattgcagtggcatccgacgaaaaattgctcaaccgggacctttataaactgcatgtcgacaagatggcaccaaaaaacaacttgtgagatcacttcttcgatttaagtaccatagattcatgcaggaaaacctgcaacacttttctaccacaaaaaaagaccagcacctgagattactagacgtctcagcgtgctggtcttttgtgaaattcgttacccgacgtccatcagtcccagtcgaccagaccaggtaatgaacgcccgctgttttattcgtggtgactaatgccacctaatcgttcaatcgtttcttgcttgaggtagtaaggggtaatcccgtcatcaatggccttggttaacaacccctgagcttccttttgtgcaagaatcgtcggtaccttcaaagacatgactgatttgttgataaccatttgatggacatcaacgtcagtcttatattgcaatttcttggaactttgctttttctttgatttttcggtctttcctttagccatgaaaatccctccccactactctgtatagctcaataatagcaaattcacaattgaatgtatattcaaaagcctagtcgcgatcaggaactttttcaaactttgcctggtaccattgatcccaagaacctgccttcaggctcccgttctcatcatactctgggttgatcactgaaatcacgtgtttaaggtcgtttccgcgttgttccagtaaatcttttctcatctgttctggcgtgaaggacttgttttcgaaaatgtaatggttaatgtcagccaagtaatagtcaatcttgtactcagccaaaatttccaaatcatttttcttgaaccatcgaaggtaaaaatcgataaagtcttccactgcttgattggttgctgtctcatctaacttgtcgaaagatactacatctgccacagtgccacctcctcttgtatttccattatgccacaaatcctgtattggcgtctaatttagtagtattattaaattgaatccaatataaacaaaggatgcggataaaatgtcagaacgaaaagtttacacagattatttttttgacgaaccagcttacaatacccatgacggtggctttgttccccttgaggaacctaagacaccacagcagccgctgaagattccggaattgcttaagccggataaagagaccgatactgacatgtactacacggtcatcgcccaaaccggtgaagcacagctgatgcctggtaagaagaccaagacatggggctataatactgatttacttggtaaaaccattttgttcaaaaagggcaaaatgattcatattactttaaaaaatgaattacctgaactaaccacttttcattggcacggtttaaacgtccccggtcccatcacggatggtggctgccacgcgccggtttatccaggtgaaagcacccacattgattttaaatgcgaccaagttgcggcaaccttgtggcttcacgcgcacccatgcccagcaacggccgaacatgtttggaagggattagctacggctgtcgttgtcaaagatgacgttgaagccaagctaccattcccaagaaattatggggttgacgacattcccgtcattttgcaggatcgtcgctttcatgaagacaatcagtgggattacatggctgactatgaccctgacggcgtgcaggggccgactgcgatgatcaacgggaccattaatccatactttgatgtaacaacccagcggcttagattacgctttctggacggtgctaaccgccgtgaatggcggctgcattttagtgatgatttgaaatttacccaaatcgcttcagatggtggcattctccctgaaccggttgattttacccacctgatgctcacgtgtgctgagcgggcggaagttatcgtcgactttggccaatacaagcccggcgatgaagtctccttgttctgtgacgacgtgccaatcatgcgctttagaatccatgaatttgcgccggacaataccaccttgcctgatcatctggtggacattcctgatccggatgtcaccccaggtgcaccagtccacaaggttgttatgtctggaatggatgaagaagtcatgatgaacgggaagaaatttgatatgcagcggatcgacgacaaacaaaagctcggcaacgtggaatattgggacatcagcaacaccaacgatatgagtaacgggatggtccacccctaccacatgcacgggacacagttcagggtggtttccagaaacggccatgcgccttatccaaatgaaaatggcttgaaagatacggtcggcgtcaaccctggcgaaaccgttcggctgaaagtttggttcaatcatctaggcgtcttcatgaaccactgccacattattgaacacgaagatggtggcatgatggcacaatttgaggtttatgatccggatcatccaaagcaatacaagctaatggatatggatactttgatgaatgcctttgctaaagagcgtggtgttaaggttgaagatctgaatattcctggaatggatatgtaagcctaattgttgcgcataattggttgacgtgatattataacttgtggaatgaaaaatgaataaagctgttaggtgaggctcctatgtggaaaatgctactgctcagaaacgtcgaaaaacgccaatgagtcagctgtccaggtcaaagtaaggcttggactaacgtagctgttaatttttaactacatcacatagtgctaaagctcaacgactggcgagaagtatttttgatgtgtccagtcgttgaacggctggacacttttcattaccaaataaaactttgaagaggtgagagttatgacagcagaatttatagacccaggagcgacgaagcatcagtctaccaagggaagcccggttgtgataactctctcacgacttaatcgttaacgagaaattgttgtaaccgatcttcccgaattgaataattgtttgacgactctaaacgttttgtttcttgcttactagctttacagctaagcgcatcacaagaaatttcccgacttcgtttgtttagatgagtcaacttttgggaattcggttaatgcaatttctcggtggtctcgaacacgttggtactggcgtacttgtgtccggtcgactactcatagtcgaaaaacgcttcaccttttaggaaactaattggggagaaatcaattaatcgtgttaaattgccacacataaagcgataataatagtaattatgaggaccatacctccaagaatccggtggaaactgattcttgaaagatgactgctatcttatcgaccaataacattataaagccgtcaacgtaaattcgttggcggcttttaatttgggttcttcgtcaactgttgttggtgaacaaaatattggagttctaatcacttggtgattagagctctttttgtatgaactcgaaaagcgaacagcactcttagccggaatctgaagaagtttcggtaaccaaatccagtgcgtttaatgactttaatcttgttgtttgaaccttctaagggcccgttggtgtaatggtgagtaaaggtattgccaatttcatcatgatgagtcgctagggtctggagggttgccaacatctcttccgagcagccctctaagtgatggaatacttgattatagttgggccaatcacggtttttgatggtttcacgtaaccgattcatcacgttgtaagtttgcttgagctcgggatcaatgtccaataaagcatcaaccacatcagtggcagtcgctggataagggaagtttgtccacttacggaaagcttcgtagttgaggtgattttccggcgttaataatagcttccaatagcgtttcaaggcgtgatactcgcgtgatgaggtcgccagggttttcatgaggcgcacccgcgtcttattaaaagctcgatttaaagcgttaaccaagtggaacggatcgatgacaacgatggcgttcggaaagatctgccccaccaatttgggataggtatagttcatatcggtgacaataattttcacattttctcgcgcagcctggtcgtaatgctggaaatacttttgaagctgatagatggtcctaaagggtaacaggtcgatcaattcgtgggtttccgcgtccataaattcaaagctcatcgcgtcggtggcgctcttagtgcttttaacttcgtccatgaggagaactttgggtaaatagtgccagttggtttcaaagtcccgttcagcgcgcaagagctgccgaccaacgaatgaatccgaagtggataactcatcggcaatgtgtttgagcgaaaccggttcggtcagtttttctaagcattgtttgcgggtcgtatttgaaatcgtgcagtgtttcggcaccgcattcgtctgcgccaggaagttggtatgacaagccttacagtgaaagtttcgccgattgaggcagaggataacggtgctgcccaaggttttagcgaatctaatggtggtcttccgccaaccatagccaatgatctgatggtcattaataaccccacagttgtggcaggccttgggggaatagttcagcgatccatttaatcggatcaccccatcatcacctattttgccattctcaattattaagtgttcatcatctattcctaacaacattttcgtagtatcatttgacatagggcatttcctttcttgacttaattctgtggtgggagcaagttaacggacgggagatgtccgcttttttactctaatgataaacaaaaaactgtcatcagtaatagacaaaaatctattaccaacaacagatattgtagaaccttaatttgtcgttagaatacaaaaaggccggagcaaaacattcagttttgtcccggcctttatcttagtaacctatccagcttcttcgacaggttttttctttttaaatgatgcaatatatttcttggatttctcttcgtcaaactctttttcagatttagcaatgacaaccgtagcgagtgagttccccaccacgttcacggcagtccgacccatgtcgacaattcggtcaattccggcgataaaagtgagtccggtaactggtaccccgatggtcgaaatagtcgccagcaaaaccacaaatgaggcccctggaaccccggccattcctttagaagtaatcatcagcaccaccagcaaagtgatctgttggccgatcgagaggttaatatgataagcctgagcgaggaacaaggcagcaatcgattgatagattgccgacccatccaggttaaaagtatagcctgtgggaatgacaaacgagacgattccttgactactcccaaatttgtccattttctcaatcatcttaggcaaaacggcttcagaactagccgttgaaaatgccaaaacaatttcatccttaatgactagcaagagatcaaaaatactaaagccaaagatcttggcaacgatccccataataatgagaatgaacgcggccatcgtgacataagcaattgccacaaaataaccgagtgggattaaggcaccaatccccatttcagccaaggcaactccaatcaaggcacagactccgatgggagcggcatgcatgacccagttagtcactttaaacatgacttcggcaactgcattcaaaccgtcaattagaatctgtcccttttcaccaatggcggcaattcctaaaccaaagaaaactgagaagaaaatgactggcatcatatccccatttgctagggacttgaagatgttggttggaataattcccagcaatgtcccccagataccggtatgctgcgcagtcttggcggttgccatatattggctgatatcagatccgtgcagcgagtgaatatcaatcagtgtcccaggatgtaggacgtttgcgacaaccattccaagggcgatggcgatggttgtcatcaactcgaaatagatgatcgtcttgagaccaactcgaccgagtttcttaatatctcccatactggcaattccaactgttaaacatgaaacgacaatcggtaaaacaatcatttgaatcaagttgataaacatggttccaatattctgcatggccgttatcgcggtattgtttttgtagaaaatcacaccaaaaaagacaccaagtaatagaccaataagaatctgccagccgaggctcagccggtaagctctgtatcgtttcataatttcacccattttcccaaaaatatgtactatttcaatataaaacaaaagccttcaatagtaaataccattgaagactttctaaattgcgtggcaacgtcctaccctcgcagggggcgatcccccaactactcttggcgtgcagaagcttaacttctgtgttcggcatgggaacaggtgtatccttctggctatcgccaccacactatttttccttgaaagaacttcgttctctcaaaactagctaatattaattttctgcccttgaacaccatttctacttggttaagtcctcgaccgattagtattggtccgctccgtacatcactgcacttccacttccaacctatctacctgatcatctctcaggggtcttacttccatataggaatgggaaatctcatcttgaggtaagtttcacacttagatgctttcagcgtttatctcatccatacgtagctacccagcggtgcgcctggcggcgcaactggtacaccagcggtatgtccatcccggtcctctcgtactaaggacagctcctctcaaatttcctacgcccgcgacggatagggaccgaactgtctcacgacgttctgaacccagctcgcgtaccgctttaatgggcgaacagcccaacccttgggaccgactacagccccaggatgcgatgagccgacatcgaggtgccaaacctccccgtcgatgtggactcttgggggagataagcctgttatccccagggtagcttttatccgttgagcgatggcccttccatacggtaccaccggatcactaagcccgactttcgtccctgctcgacctgtctgtctcgcagtcaagctcccttctgcctttacactcgttgaatgatttccaaccattctgagggaacctttgggcgcctccgttactgtttgggaggcgaccgccccagtcaaactgcctacctgacactgtctcccgccacgctaagtggcgcgggttagagtgttcacacagcgagggtagtatcccaccaacgcctctgccgaaactagcgttccggcttcaatggctcctacctatcctgtacaagctgtgtcaacacccaatatcaagctacagtaaagctccatggggtctttccgtcctgtcgcgggtaacctgcttcttcacaggtatcttaatttcaccgagtctctcgttgagacagtgcccagatcgttacgcctttcgtgcgggtcggaacttacccgacaaggaatttcgctaccttaggaccgttatagttacggccgccgtttactggggcttcatttctgggcttcgccgaagctaactcatccacttaaccttccagcaccgggcaggcgtcagcccctatacgtcatcttacgattttgcagaaacctgtgtttttgataaacagtcgcctgggccttttcactgcggctgtgcttgcgcacagcaccccttctcccgaagttacggggtcattttgccgagttccttaacgagagttcactcgctcacctgaggattctctcctcgactacctgtgtcggtttgcggtacgggtagttgatgactcactagaagcttttctcggcagtgtgacgttggttgcttccctacttaaatttcggtcctcatcaccacttgtcaacccgccaaaaagcatttgactctttgactgacttgtggcttgaacatccctttccaactggatgcacaacttagcctcctgcgtccctccatcgctcaaacatcatcaactagtacaggaatctcaacctgttatccatcgcctacgcctttcggcctcggcttaggtcccgactaaccctgggaggacgagccttccccaggaaaccttagtcattcggtggatcagattctcactgatctttcgctactcataccggcattctcacttctaagcgctccaccagtccttacggtctagcttcattgcccttagaacgctctcctatcacttgaccaaaggtcaagtccacagtctcggtaatatgcttagccccggtaaattttcggcgcggaatcactcgactagtgagctattacgcactctttaaatgatggctgcttctgagccaacatcctagttgtctatgcaactccacatccttttccacttagcatatatttagggaccttaactggtggtctgggctgttccccttttgacgatggatcttatcactcaccgtctgactcccggataaaaatcaatggtattcggagtttatctgaacttagtaacccatgacgggcccctcatccaaacagtggctctacctccatgattctacgtccgaggctagccctaaagctatttcggagagaaccagctatctccaagttcgtttggaatttcaccgctacccacacctcatcccagcacttttcaacgtacacgggttcgggcctccagtgcgttttaccgcaccttcaccctggacatgggtagatcacctggtttcgggtctacagcaacatactaaaacgcccatttcagactcgctttcgctgcggctccggcttttaaaccttaacctggcatgtcaccgtaactcgccggttcattctacaagaggcacgctatcacccattaacgggctctaactgcttgtaggcacatggtttcaggaactatttcactccccttccggggtgcttttcacctttccctcacggtactggttcactatcggtcactagagagtatttagccttgggagatggtcctcccggattccgacgacgtttcacgtgtgtcgccgtactcaggatcctgaactgagggtcattgatttcacctacggggctatcaccctgtttcgccaaccttcccagattgttcgattatcaacaactttggtaactcaaatgttcagtcctacaaccccaatgagcaagctcattggtttgggctgttccccgttcgctcgccgctactgagggaatcgaaaatttctttctgctcctgtgggtactgagatgtttcagttccccacgtctacctctatacagctatgaattcactatatagtaacagtcgattaaaactgctgggtttccccattcggaaatctccggatcaaagcttacgtacagctccccgaagcatatcggtgttagtcccgtccttcatcggcttctagtgccaaggcatccaccatgcgccctttttaacttaacctgtacatcacgacgtgatgcaaagttaattgagtatttgcgattttttctagttaacaaactcaaaataacgcggtgttctcggttgaaattatataaatacaatttcaaaaaattattacagaaaattaatattatctagttttcaaagaacgaattgagagtagacctctcaaaactaaacaaaactttcgacaatgtgcaggattccgtttttccttagaaaggaggtgatccagccgcaggttctcctacggctaccttgttacgacttcaccctaatcatctgtcccaccttagacggctggtccccgaaggttacctcaccggctttgggtgttacaaactctcatggtgtgacgggcggtgtgtacaaggcccgggaacgtattcaccgtggcatgctgatccacgattactagcgattccaacttcatgtaggcgagttgcagcctacaatccgaactgagaacggctttaagagattagcttgacctcgcggtttcgcgactcgttgtaccgtccattgtagcacgtgtgtagcccaggtcataaggggcatgatgatttgacgtcatccccaccttcctccggtttgtcaccggcagtcttgctagagtgcccaactgaatgctggcaactaacaataagggttgcgctcgttgcgggacttaacccaacatctcacgacacgagctgacgacaaccatgcaccacctgtcattctgtccccgaagggaacgcctaatctcttaggttggcagaagatgtcaagacctggtaaggttcttcgcgtagcatcgaattaaaccacatgctccaccgcttgtgcgggcccccgtcaattcctttgagtttcaaccttgcggtcgtactccccaggcggagtgcttaatgcgttagctgcagcactgaagggcggaaaccctccaacacttagcactcatcgtttacggcatggactaccagggtatctaatcctgttcgctacccatgctttcgagcctcagcgtcagttacagaccagacagccgccttcgccactggtgttcttccatatatctacgcatttcaccgctacacatggagttccactgtcctcttctgcactcaagtctcccggtttccgatgcacttctccggttaagccgaaggctttcacatcagacctaaaaaaccgcctgcgctcgctttacgcccaataaatccggacaacgcttgccacctacgtattaccgcggctgctggcacgtagttagccgtggctttctggttggataccgtcaagatgtcaacagttactctgacacctgttcttctccaacaacagagttttacgagccgaaacccttcatcactcacgcggcgttgctccatcagactttcgtccattgtggaagattccctactgctgcctcccgtaggagtttgggccgtgtctcagtcccaatgtggccgattaccctctcaggtcggctacgtatcatcgccttggtaggccgttaccttaccaacaagctaatacgccgcgggtccatcctaaagtgacagccgaagccgtcttttaaaccaaaaccaggtggttttggttgttatacggtattagcacctgtttccaagtgttatcccctacttcaagggcaggttacccacgtgttactcaccagttcgccactcgtctcaatgttaaatctttcaagtgcaagcacttaaaatcattaacggagacgcgttcgacttgcatgtattaggcacgccgccagcgttcgtcctgagccaggatcaaactctcatcttaaattgtttaaaatgataagcctgtgatagctcatgatttaaatttattatttgttttacgaattgacttcgcaaatgtttggttccaattccgaagaattgaaacgtcctgcacatttgtttgtcgaaaattttgttcagttttcaaaggtctacatcagaacacaaacatttttggcgaataaattagaattgttcgtttattcaaatccttgtgtcccttgcctctaacagcaagaacaattatataacagccaatctttcaagtcaacaaaaactttttaattagcaattggtatatgtgttcatgtcattgaagcaacgagtaatatattatcagctatttcggccgaggtcaacaggtaatttcaaattaattcaataaatcgttgctgacaaagcttaaagattgttaataccgggaacaaatcctccccgcaaacaccatttagcctgtatactggcaattgaaatcttcgcgaaaggaactgtcatcatttgaagaaaattgtaattatcgatgccaaacgatcagccatcggcaaattaaacggctcattatcttcattaactgccgaacaacttggttcaaaagtcacgcgtgctttattaaaagatgctagtctttccggcagccaagttgatcaagttatctttggcaacgccatccaggccggaaatggccaaaacattgcccgacaaatcgaattgaacagtcaaattccagaaagcaaaacagctttcacagtcaaccaagtctgtggttcaggactgcaagcaatccatcaagcacaatccgccttgcttctcggggaagtggaaacggtcattgccggcggaaccgaaagcatgtccaacgttccttacttgaacatgtcacaacgaaaggcaaccaagtttgggccggtcacattatatgatgggctgcaacgagacggcctaagtgattccgcgacggatgaaccaatgggaatgactgctgaaaacgttgccgatcaatatcatgtctcacgtgaagaacaggatgcttttgcattgcgatcacatcaactggctgcgcgagctactgaacagcattattttgatgatgaaattattcccattgaactcaaccaacccaaatcacacgctccccacatcgtagcgcaagatgaatcgatccgggtcgacacaaatttggaaaaactggccgcccttcgtcccgcttttaaaccgaacggatccgtcactgccggcaacagtgcaccactaaacgacggcgcttctgctctgatcatgatgactgaagaccgggcaaaccagttgggactatctccaatggcagaggtgctgggttacgccgagcgcggaatcaacccggaagtcatggggtatgcgccctacttagccattaatcaattggtctcccagctcaacatgtcagtcaacgacatcgacctctatgaaatcaacgaggcctttgcttctcaatcagtggcagttgttcgtgatctgggcatttcagttgataaagttaacattaacggtggggcaatcgcactgggtcatccgctcggagattctggtgcccgcatcgtgacgacgttattgcataatctgcgccggaccgaccaagaatttggcgttgcctctctttgtatgggcggcgggatgggctccgcactggcaatcaaacttctttaatcacaaaaaataggaccgtaggctaaacgctgacaacgtttgacccacgatcctattttattttaattaagttttatctgttcatcttcaggtaagtggtctttaaacgaagattgatacagccaataataaacccgcttggtggcttttgtcatctcagcatacgcaggattgatcgatttaacttccggatagacccgcattaaatgactgaaggcactgaaacttccagcagcagacatcccgtcatcgtccttcttcccccgttcaaccaggccaattaattgatcaacctggaatcgcgccagggcgtccacataatcaaagagggttccggcagcttggaaactcggctcaatcacctgccgtgacgttgtgtactgtccggaggcaatttgggtcaacaactgatttctgctcatcgtatattgcaccatcaatggcgttaaaaaaacattctgtagaatctgatgagtggtttcaaaaatcccataggctaccttgaccgtttcaccgcgatcattcacctgtggccggtcattttccaacacccgactgtatcgcaattgatagttctgatgtttggcatttctggcactgccggcgttacttaaattcaatacagccaacttttctgccagatcagcacctgattggggtaagttcaaatatttcccaattgcctcaactgcggctttggtcttggcaagaaccgttgcctgatcagcggcactggtgatcggagcaccgactaaatcgggattattttgagtgaattttgcgtaaaccaacgcatataaaccgattgatcccagtgaattgaccatgccggccaacgtgttgttgacaaatagattaatatcttctgtcagcgaaactttgccgatcgcatcggtcatcatcttgggtaaatcgtgctcgtcactaaaatcgtcttcattataggaataatttccgagcagcgactgttcatcattaccgactggctggttgcttaaaaagccatcgctaatttccctggcaacgcccgtggcgatcgtctcatcgatggccgatggcttggtcgtttggttattaatcgctttaaatggtgaagcaccgttcatatagccgttgacgtggtcaaaccactgattaaccagggtccgctgttgattgagatccaggttctgcaaggcagagttaatccggaaaacaacgccaccggcgccggcaatcgcccggacaaattgaatcaccgctgtcttataaccaacaacgtacttttcaggagcctggctctgacttaagtattcagaaaattgagtgccggctgcccggttgacgactgaactgtcgtcatctccggtcgcccacagcgacatatagttaaattgatcaatgctgacatgttttaaatccttggcggctgccaaataccccatctgcattggtttggacattttaaactctgccaacgaaacacttggctgcagcggaccgggcaaaaacgaccgcaagccccgggtaattcgttcagaatagattgagctcttagcgtaagtattttctcccagcacttttgaagtcattaaccccaacatgctgagaattttttgttgtttcgaacgggtgtcggaatcatttaccgacgaactggccttattcatgtcgaaaccaccccctagtattatgactataatatcataaactatggcgaatcattgccaacaaatggggaattaaccattctgaaacaattttcaaatctgaggcgttatttttgtgattcattcaaaaagtctgtatgcttatggtagagataaggaaagggtgtgaaactaatgggaaatctgaaaaacaagtccgatgaagtcatcggcaaagtcaaagaaaccgttggcgacgtaaccggaaacgacaagttgaagctgaaaggcaaagctcaaaagacatctgggaaagccaaagataaggttgaagatgccaaggaaaaggcgtccaagaaagtgaatgatgccttggacgacaagaagtaaaatccagctgttaaataagaaacccgatacctgcgaatcgcatggtatcgggtttctttccccaaaaatgagaaagtaaaactttttacatgttttgtattgcatgccaaataatattgttctataattcactctcgtgttattttgatctaatcaattgaattagaaatatgaacagggatgtgaatcgaaatgtcagcaacttatttgcgtcaagcaaccaatgcagaccttccagaaatcaaaaaaattattgaagaagcaaaagcctaccttaaaaagcaaggcatcgaccaatggcaggatggctatccggccaccgaagacttggagtttgatgtcaacaacgggatcacctacgtgttaattattgacggccaaatcgccggaaccgcagctctccaccaaggattggacgtcaactacctcaacattcacgatggcgaatgggtcaacggcgtccacggccgctataccgccattcatcggatcgccatgtcgtcgaatttccgcggccagcacctatcccaaaagatgatcagcggcctaatcaccatttccggtgttctgggttacaaagatatccgaattgacacgcatcccgacaacttgggaatgcagcacgtgatcaccacgaatggttttaccaaacggggcacgatttacatggctgaaaaagacagcgaagcatccccacgctatgcctaccaactggttattgggtaagcgaacaagttggagtacaatatggttaatgaggtgataatatggcacaagatgatgctgccgtaaagaccgcactaatcattatgtacgttatcggcgtagtttgtctgggaatcacattcttcctactcgataaagtcaacggaaaatggtttaccaagttctcagtcggccttgtcggggtgattttagtaatgggaattatcttagtcaatgtgattaatctaaattaaagagtgggacataaggcgttttgatcccagaatttaagcaaataatccggttattcctgtctttggaatagccggattatttgcttaaatggccgggatcagccgactgccgcacgtttaaactagataacagaggaataaaaacaaacgggtgagacaacacaaattgtctcacccgtttgttttatttaaactaaatttgttggaatgcctgatccaaatcagcaatcaagtcgtcagcgtcttccaagccgactgacaggcggatcaattcgtcctgaatacccattttaagccgttctggcttgggaatctcgaagtgtgacatgaatgccggcacttcgaccaaactttcagcagcgcccaaactaacggccagaatgatgagctgaaggctgttgacaaacttggcagcgtccaatccgggttggacttcaaaggagagcaccccaccggcacctttagcttcatcactgatgatttggtaatcctgactggttttgtcaacagttgggtaataaatcttggcgactttgggattactttgcaaataagcgatgattttctcggcgttttgaatgtgccgatccatccggatgtttagggtttgaataccacggcgaagcaagttggcttcttgaggtgccaaaactgcgccaatggtattttgaatcgcataaatttgatcgctcaaatccttggttttggtgacaatcatccccgccgtaaagtcagaatgaccacccaagtatttagttgccgagtgcagcaccacatcggcgcccaagtctaatgggcgttggagataaggtgtcaaaaaggtattgtcgacaaccaccaaggcattgtgttgatgagcaatttgggaaatctgcttgacgcttgaaaccttgagtaacgggttggtcaccggctcgaagtagacgcctttggtattcggcttgaaagccgctgccaccgcatcggcatcttgggtatcaacttcggtgaattccaacccacgtggcttcaaaaaatcattcaccagtcggaaagtcccaccgtaaatgttatcgccgataatcagatgatcgccaggcttaaagagcgccaatgccgcatgaatggccgccatcccgcttgaaaaagcaaagccgcggtcaccgttttccaatttggcacacacgtcttcaacggcatctcgagttgggttgccggaacgttcatagtcccatttaacatccgcccccagcttggggtagcgaaaagttgatgagttgtagatcggcacgttcacagctccggtggagttgtcattgggacggccgccgcgaaccagtaatgtattaaatttaaccattaaaaaatctcctatctctccaaagtggtggtgctactgaacaggaaccaattgatctgatgataacagatacagatatttctttgtaaccggcctgccgagaatttgatccaaagcagtcgcgtacaggcggatctggccgtcataacgttcatgaaccgtatcaacagtggtcttcggggtcagtcggtcagtcttataatcgaacaacacgacgcccgcctccgactccacatagccgtcaataattccgtgaatcaagatcggttgatcatcatcttggtcaaaatccttgaaagcgtttttagccttcattaatagtgaaaacgggacttcgcggtaagttgtctctgggttagccaaaacaaccgcgcccagagatgacgcataaaatctcagaatcccgtcgacgttaatttctccggcaacattctcttctaaaatgccttcctttaccaggttggcgatcaactcaacgatagtggcctttgtcggctgttggtgtaaatcaatctgctgcagtaccaagtgggtcgccgttccaacctcagtaggtgcgggtttatgagttccattttctgaaataaattttggcgtagccagactgggctgcgtataacggccgggtttgatcagctgatcgctgtcaatcagcgaataattgcccagctggacgttatcgggatcatcgaacagccgcttaatttcggaaacggattggtaggctgtcgtgcgagttgctgcctggtgtgggtaacggaaattcatgatggccttaatttgtcggcgatcaacggctgaatcggattcgaccggctgctgctgatcgagccaactacgaggatcaaccgctacacggccagcctgcttctttccttcagccaccttggcattgtcataaaattccaggctcaaccggctggggtcatcggcgagcaggttgacaattcggctgtcgccatagtctttaaccacatccggatgacgggaaattgccggaccaatccagtccaaatagcttttggcgctgttgcgctccgccattggcaataagatggccgattcttcagtctgtgactgccagctttcaacgatcgactgcaaatctaacgttggtttgcgagacccgccttttcctgggtcgactttaccgaccaagaacagccgctgctcggcccgggttaaggcaacgtataacttccgcatttcttcagacaaaccggcatttttggtcacatccaagacggcctggcgttgcaaaggttcttgaatctcccgggttttggtatccaaataagaaatgccaattcccagatgatcattcaacacggcacgtcccatggtgtcctgctggttgaattgtttaccaatatcattcaaaaagacaatcgggaactggaggcccttactgccgtgaatcgtcatcacgtgaaccatgttgtcggaagtgttcggcaccgctgtggctaagtcgtcatccctggcctgcattcgctcgataaacaggacaaatctgaacaaacccttaaacccattcttctcgtaatcaaaggcccgctcatacaaagcatgcaggttcgtctggcgctgatagcccccgggcatcccgccaacataatccaaatagccggtttgattataaatttcccaaatcagggcaaccaagccgtcttgtttggcaacgtttttaaaatgatccagctgcttgaacaaggtgtcgattaacggatagattgcctgagcatatttgttgggttcagcgttgggatagtcccggtaaaatttcaataccgactcataataattccccgtcttttgattaatccgcaaataggccagctgattttcatccaaaccgacgatcggcgaccgcagcacggctaccaaggggatatcttggtaaggattgtcgataatcgacagcagggatagcatcacctgaatttccgtggttttcagataactcttggcaccggtaatttcggccggaatgccataatctttgaaaattgaagacatggtaatctggctgccccgagttggcgaaatgacagcaaagtcaccgtagtcaaccggtcgatcgccatcgccatccgcaatccattccttatcatcgaccatctggcgaatcttttgggcaatgatttcaacctgcccaacgtcagcatccataacttgctcggcaggaaggttctcaccttctgacagcggctttttagggctgtacagcagcaccgaaacgtcagcgtttacgtcttttggataatacttggcgccaaactgcagcttggcatctgaataatcaatttcgccaacttggcggtccatgatctgctcaaagattaagttaatgaaattatcgacgttctcagttgaccggaagttatcggccaaggtgattaattcatcgtcattatcagccagcgaataggtccgctgcttattaatgaacatctggggatcggccagccggaagcgataaatcgactgtttggaatcccccaccatgaatcggtttccgccgccttctttggccagtttattcaaaatggcgtcctgaagccggttattatcctgatattcgtcggtcataatttcataatactgatcccggagctttgcttgaacttggcgggcctgcgggctgtcgtcgttcaaaatccggtaagcagcctgctcaatatcgatgaattccatcaaatggcgctgatgcttggttgcctcgtaagcggttcgaaaggctttgaccgctgaaatcagtttggccacccgttgcttggcggctgccatcaggtcaacgttggcctgttcgtccataccgaaatatttattgcaaaaggcattgaagtcttttttggtttgttgattaattgcgcgaatttggccatgaaactgtttttgttcaccctgcggtttggttagccttggcaaatcggcaaattcaaaaccagtcagtgacttgcggacatcgtcaaatgatgtgcaatttgaaaccgctttttgaagggcttcaatggctgccagctggtcagtgaaagctttttcgtccttatccaaggcaccgctttgggccaatttaatcatgtactgatgattgattttaagtttggtgaatgcttcagcaatctttggggcaacgttttgttgatagaaatcactgtcatacaatggtttgccgccaagatcataaaaatcggcgaccgcattcagccaaccatccggatcgtcggtaacatttgcgaactcgtccaatcggtaaatcaggtcggctaagccgtcgtcactgcggtcgttggaaaagttctccgtcaatcgggcaaatgagccatcttcatcgttgccatataggtcttctcgaaccgctccccaaacttgatcttttagcagctgtttttcagtatcgtcggccaaaatgcggaagttgggatcgattcccaagagatagtagtatctgccgactaatttctgacaataagcgtccatcgtcgtaatgtcggccaccgcgactttttggatttgggtgagcagccggcccttttcggcttcagctgcctgattaaattcttctcggagggctgcctgtagtcgttggcgcatttctttggcagcggcgttggtaaacgtcaccaccaggagttggtcgatgtcgacgtgctgatttttgaccatgtcaataattcgatcgaccaacacccgggtcttcccggatcccgcagaggcggaaaccaggacattgcctgccgggcggtctttaattgcctttagttgatcaggcgtgtattcaaatgccatcggacttttcctcccctaattttttcttaatatcctcaatcgaatcactgttaaccggccgatactggttacccggcaaaattgggtcaaagttcatgattgatttgtacggggtaaactgcatcccggtggtttgaccctgcttaaacggccacagtcgaacgtcaccggcaaaaatcttttctgccgcatcgacaataagtttctcagtgtgggtgagaaacgcatctaactgcagtggattaatcagtgattttttacccgtgtagcctttggcggtctttctaattggataaatcggtgagtagccgctatccagctcctcatccaaatgatcaatcaagccggactcgtcaaccaaaatgccgttatagcgatgcttctttaacaaggcatcgtcaaaggttaccttttgaaggtcctcgggtttgaagacggcattataaatgtgcaggtacaacgcgccggccaaggcgacttccttatcatcgggattaagccgttccagattgtgctttaacacgtccagatacgtcaacagttgcatcgaagttccgtcataagctgcattgaaatcaaatttgcggtcagaggacttgtagtcaacgattccgaagtagcgtttgtccttggtggtcatcgaatcaattcggtcaattctgccccgcactttaacctgatgatcatcagccaaatcaaagcttagaccattgagggcctgcttttgattgggctggccaaaaatcagttcagtattttgcggccgcattggcgtcagtttctgttggtcacgcaaggctcggatcatctgctggatggttgcggctaactgcatggaaatataatgcatccgattggaactggtcagcacaacgtagtcaaagttttggggatcattgatgattcggtcgacggtttctttgacgaggtcgctcacatcttgatcagataagctggccaaatcaatgttttgggcatgaatctgcttaataatccggtccatggcgtcatgataaaaggtcccagtcgatgccgtcgacagctcaaacttcggtcgttcctggagttttagcccatatttgaggaaatattcataggggttcttatagaaggtttccagctgagaaatcgaaatatttagttctgaaccgtatagatccgtgatgatttcaggtgctaatgactgcggaacatttgtgtaattaatgcttttaagcagcttggacgtctgccggctgacttccggatcctgctgcaggtactgcaaaatcactgcccagccggcactcaagtcctgctgaacatcaaagttattttgaatgacctgaatcaaatggtgaagtgtcccgctcttggtgcccacgtatggcatcacgtcgtgctcatcatcggggatcgccgggttgttgacgattttgaggttaaagaaatgctgaatccgtgaaacataaggtgaaagtttcacagcagattcgtcgtttaatttgttggtgtaggtgaagataagcttgtccgaagcggtcatgaaggccaaatagttcaagtacggttcaaaagccatttggacttcggcgggatcatttaagtactgatcgtcactgaggttgctttggagttggttgatgtcgtcatcgccaaagagattttcattgactagccgatccggcatgttgtcatcgttagcgccgatcatgaacgtgactcgataatcattcatctgaaccatgccgctttcagagacgctcacctgatccagcgtggacggaatttgtgaatagtccgctccttcaaagccggcatagatgagtgaccaaaaatcgccgggcacaaacggtttgtcccccagaatttggacacattcgtccagcagggaacaaaatgtccgccaaacctgctcaatttggttggaacgattgatatcgccctcgtctgttgccgcatcccgccagtcctggagccggtcaacaacgccggcatccactagaaactggtagagaatttgagcagcttcctggttggttttagctttgaaaaattgtttgtaaaaattgggcaataaatctcgcaccatatggcggatgatattgatcttgcgggaaatttcccgatcttggtcggtgatctttgtggtcttctgttcttcgtcgctgtccggcagccaaacgtactgccaatcagccttttgcgtccagcgggtgtcggcgtaatcgtttttcagcaccaagttgtcggtcaaggacactgcttgacgataatcatcaatggccatcggcttgccatcaatcattggtaggactaattcagattttaagaaccgcatcacgtcatcatagcgataattgcgggttcgatttgggtcgtagatatcaaatagcgctgctaatagttccaccagtggatggtcagccattgactgctgaatatccttgaaatagggaatctgctgggtggtaaacaccggctctaaaatgttttgataggcgtccaaatggcgggtcaaaataagaaaatccgagtatcggtacttgccggtggcgaccatttgatgaatcttcgtggcaacttggtccagttcggagtaaaggttgtcagcttgataaatttgaaccgagtttggggaaatttggtcgggcagttggtggtttcccagactgctggacgtaatccaataggcctctaatttttgcatatcttcatcaacccgcggctgatcagccatgacggcctttaaataaggcacccggttgtcagcggcaaatcgatagagctgatggaacaatttagccggctgaaagaaaatattcggctgttccggcagttcagttgggtatggccggtccaacgtcaatgacaccgtcaccgaagcggattggttgatcaaggtttgcaccaagccgcattcctgggcggtgaattttgaaaaaccgtcaatatagaagtgataaccacttaaatcaatgtcctgcagtttgctgctcagcaggttcaaaacggtgtggctgtcaaaataattctcagaaatgcgtttgacatactgggaataaataatggcaaaatcgtggagtttatcacgcagatcattagtaatcgtgctgtcaggccgctgcagcatttccaaaagatcttcaggcaagacattgccggcctgcatctcggcaatttgggtagcaatctgatcaataaacccgggattatgaatttcgtggtcaaagagcaccaatcgatcggcgtcatcaacaataatttgatacagcagcatattgataccggcactgctgatccgctgcttttgatattccggtgtgttgcgcaaaaagaaccacgctaatcgggtgaaggataacacctgaacatcactttgagcagtggtcatttggttggcgtcgccaagttgttttaaaatactgacttctgattcaaacttaatgtggtttggaaccaagtagaaaaattggtcgtggggattgtctgatttttgctggcgcagaatgtcgatcattttcgattgatggtcgacacctgctcgacctaagacaaactgaagggtcactgctctcacctctttaaaattactttaattttaccatagtatattcctcatgtttgatgaagattgacgatgatttcttaagtggagggaaacgccaatcgcgcgcccagcaagggattggttgggtatcaaaatgatttgtgaatttccggaacattatcattgaacattaacaaaaagggtctattatgagggttggatgtatcttacatccatctatttgacctaaatgaaagctttatgcttgcattgatcttgttagagagcctaccagtgcattccacgattaagtatcggaagcaagaatttacgatctacccccaatatatctttcaagttcaaatactgataggccctactcctaataacgcccggtgaaaactgggtgtacataaagaacagagtgcgaaacaagccggttagcttcggagcattaatttgataaccagttttgatgcgtatttcgcatcgaaactggttatcgaattaagcggacgaagctggcttgtgtagcacatttccactaaataagagtaaagctccaaactttgatgcgctctttgcctcaagactcattattagataaagcgaaacaatctggcccgtcggaacacacctttgccaactaacagtcacacaccacaaaccaaaatacatcaaaggaggcagccaacacggttgcctcctttaataatggtatcgatgcaaagaacctaagcccgcaccttattttcttccatcaccttattggtataaaactccaaatcatcgactgcctgatcatcctgatctccctgagccgttacagcgtggagattctgctgggcaaccgcccaataaaccaggttggtggtaatcggcagaatgtcccgaatgacgtgaaagtcgaaattatcgccatttgtggatttcatattcaaaaagttattccagtcggtcaccatattgacgccactgtgttctttcttcgagaccgcagaaatgatgacgaagtgggaattgcgatttgcttcttccaactgattttttagctgttcaatttgttctgcttccagtttaattgccattttatcgccctcccatcggtgtttgatcaataattccaattgaatgattcattaatttttgcttgatcagcatttcataagccagcttagcaaccgcttttggagataccgttttagccggcatcggcgttccttcattaaacagttcatagtcgctggcctgctggtcctttaattgacccattctaattatagaatacgcaatttcggattcgtcgacaatcttgatggcatatctttgctgttttataaattcttgggggtctttcacgccagcataagtgaccgactcactcaactcgtcatcaacaccggcgtatgagagcatcacaatatcactgattggcggctgaacctcatcgaccgcctcaaagagcgcttccacataaaggtcggcgtcgttgggaccaacggcgatgaaaagcaggttggtattcggcaaggcttgagcatagtcacttgctgattccaaattacccgaatagacctcgacagaaatgtcggagcgttgcttaagtaacgcgtttagtggcggcaccacggggctattttgattaatgattaataattttttcaaatcggtggcttcctaatctaaatgtttttcaaattgtgcataatggaccataattaatgtgtaccataataacaatggaaaatcaaaggaggacgtaaaaatgtcccaaaaagttaaaattggtcaatcagacgttgtcagcaccccgttaggctttggaaccaacgctgtcggcggtcacaacctgtttcctaatttggacgaacaggccggcatgaattccgttcgggcggcattggatagtggcatcaccatgctggataccgcatttgcctatggcttcggccgctctgaagaattaatcggcaaggtgcttaaagactatgaccgctcaaaagtcgttgtggctaccaaaggcgcccaaattgtgaacggcgatcaggtcaccatcagtaaccgacccgctgatcttgagaaatttgtgaaggacagcctcaaacggttgaataccgattacctcgacatcttttacattcacttccccgatgatcaaacaccgaaagcagaagccatcggcaagttagccgagctgaaaaagcaaggactcatcaaagcgattggcgtttccaacttctcgctggaacaactcaaagaagctaaccagaatcacgatgttgatattgtggaagaccagtatagcctggttcatcgcgatgccgaaaaagagctgttcccgtatctggagcaagaacagatttcatttgtgccattcttcccgctggcatccggtctgctaactggtaaatacgatggtagtccggttaattttcctgaagatgaccttcgaagcggcgaccccaatttttctggcagccgcttccacgccatcacagagtcagtcaagaacctccaaccaattgcagacaaccacgatgccacgattgcccaggttgtcttagcttggtacatcaagaatcctgacatcagcgtcgtcatccccggtgccaaaacgccagagcaagtccgcagcaatgccaaagcaatgaacgttgccctgtcggatcaggaatacaatacgattgataacgcatttagattctaatccacatctaaacagacatcgaggccaccaatgtttagcgcaaatttctttgcaaaccgcttcaatggtcaggccttgatatagaatttttttaaaatgcatttgtgacccccgcttaacgacaaatggtatactcaagttggatcggagagcgcttacaattaagttatgagggggcctcctttatgaaccgtttagatggaaaagttgcaattattactggtggtgttagtggctttggtttggcagctgccaaattatttgtccaagaaggtgccaaggtaaccattgccgatgtcaatgattccaaggctgaacaagctttaaatgaaattggcaaggacaaggcgatttttgttcaacaagatgtttccaaagaagccgactgggatccggttttccaaaagacgattgaccagtttggcccagtcaatgttctgttgaacaacgccggtatcttaatttttgacgatgctgaaaacgtcgacatggatcaatggcacaagattttatcggttgacctggatggtgtcatgcttggagttaagtatggcatcaagtatatgaaggaaaaaggcggatcgatcatcaacctggcatcaattgccagcctgatcgagatcagcaacctttattcctacaatgcagccaaaggtggtgttcgactcatcacgaagtcggctgcgctatacgctgctgagaaggattatccaatccgggttaactcgattcacccagggtatgcccacacaccaatggttgattcctaccctgaactcagacaaaaactcgagagccttcacccgatgaaacgactggcagatccaaaggaaattgccaacatggccttgtatctggcttcggatgaatcatcattctcgactggttccgagttcgtcgttgacggtggttatacagcacaataattcatcatggcttgagaagtcctgactggggcgtgatgattggcactgcttaataatccaactcaaaatattgatttttattaactgctcacgatgaatgtcgcgagcagttttttactaggaaattggtgtaaccagttacataaacattcaggcataacggtaaacattttattgctttttattaatttaattcgtttattgaacccttttaatgataatgctaaaataaatatgtaattttttattcatacacgaacgatagaaggagctattatatgttaaattcaattgccaagtatttcgagtttgatgaacgaaatacgaatttccgtaaagaaattatcgccggaattacgacgtttgtttcaatggtttacatcttgttcgttaaccctaacgttcttggagtcagcgggatggacaaaggggccgtcttcaccgcgactgcccttgcttccgcatttggctgtttcatgatgggcttcattgccaactacccaattgcgatttctgccagtctggggatcaatgccttctttgcctactcagttgtgattggcatgaaggtttcatggcagactgctttagccggggtcttcgttgcctcagttattttcatgattttgaccgctttgaagctgcgtgaaaaaatcatcgattccattccagctgacttgaaagctgccatcggtggtgggattggtttattcattgcctttatcgggctgagcgacggtggcttggtcactgccaacaaagacaccttggtgagcctaggatcgttacacgtcgggacaacttggctgacgatcttcggtctgttaatcaccgtcgttttgatgagcatgcggattccaggtgccatcttcatcggaatggtattaaatgccattcttggaatggtgaccgggttgattccattaccacatcaatgggtttcttcgattcccagcttaaaaccaacttttggtgttgccttgtcacacattggtgatatcaactcggttcagttagtcgtggtcgtcttaacgttcctgctggtaaccttctttgataccgccggtacgttggttggcttggctgaacaagccggatttatcaagaataacaaaattcctcgaatcggtcacgcattaattgctgattcttcaaccatgttagttggatctgttctgggaacttccccaatgggcgcattcgttgaatcttcagccggaatcgccgttggtggtcgaactggatttactgccgtcatcgtgggaattctgttcattttaggtactttcttctcaccattattgaccgttatcaccagccaagtaacggcaccagccttgattatcgttggtattttgatggctcaagcactgaagagtgttcactgggaacaatttgaaattgccgccccagcattcatcacacttgtcggcatgccattaacctacagtatcgccgatgggattgcccttggatttattacctacccaatcacgatgatcgccgctcgtcgtggcaaagaagtcagcgccatgatgtatggattggcagttgtgtttgtgatcttcctttggatactcaacaattagagcgcgacaaggtctgaaagaaacacttaaagaatctgacaaacatattctcttgcgccaaattcaactcttcgggccaaacccattttgacctcacaccccaaaagcggtaaggtataaaggttgtttaacaactgaatatttaacaaggaaggaatttgttatgaattctaagactaatttgtttggcatcagcaacgttcgtgacctcacgaaagccgctgttgtatctgcactctacatcgtgatcacgatggtctttgcagccttgagttttggcccaattcaattccgcttttcagaaggtttgaataaccttgctgtcttcaataagcgttacgttgtggcgatcacgctgggatgcttcatttcgaatatgatgtcgtcactcggaccactggatatggttgtcggaactggtgaaacgctgattgcgctgttgaccatcaacatcgtcacccggttcatcaagtcactgccattgaagctggttgcatccgttttgatcggaaccttttacatgttcatcgtggctgcagaaattgcttatctcggaaacaccgccttttggccgaccttctggggtgcatatctgaccactgccatcggtgagtttgtgactatgacgattggtgctgtgttggtttacatcatcagtttgagatatgatttgaataagtaaatatgaaaaccgcaatcagaaattctggttgcggttttttagataaccgaatcgtttacctcctgtccaaaatatcttaaaatatagttgtgaatataatcacaatttttatttaggaggttccatcatgacagaattatttgcaagtcccaacacctatatccaaggtcccggcgagctgttcaagagcgccggatatattgaaaagtatggcaaaaaagttctcttgctgtctgatccgacagtgttaaaaattgttggtaacgactttaacgattatcttcaaaataatggcttcgacgtcacccttgcccagttcgagggtgaggcttccgaatccgaaattaatcgggtgactgagattggtaaatccaaccaagaccagatcatcattggtttaggcggtgggaagactgccgactcagccaaggcaattgccgacaacctcgacattgctgcgatgatcgccccaaccatcgcgtcaacagatgccccctgctcacgattgtcagttatctataccgatgatggggcgttcgaccattaccgcttttacaagaagaatcccgaaattgtcctcctcgacaccaaggtcatcgctggcggtccggttcacctactgatttccggaatcgccgatgcgttggccacaaacgttgaagccaccgacgttcgtgctgccaatgccgataacatgttgggcgccaagcaaaccatcgttgccggcgcgattggccaagcctgtgaggataatttgtttgaatacgccgacctagcgattgccgctaacaaggcccacgtcgccacgccagctttggaccacatcgttgaggccaacgcccttctcagtggtttgggcttcgaaagcggcggcctggcagctgctcacgccattcacaacggcttcaccgctttgaccggcgacatccatcacctcacccatggtgagaaggtggcatatggcacattggtcgaattgattttagacggcagtgatcacgcccggttcgagaaattcctgaaatttgacctcaaacttggcttgccgaccactctggccaatttgcatttagagtcggcttcagatgaggacctgatgaaggtagctacccaagcttgcgatgagaacgacacgatgaaatgcatgccaaccgacattacgccggaagacgtcttcgcggccatcaaggcagtcgacgagtatagtaaagactttcagaatcaataaccagttggttcaacccgatttttgaacttataatgtacgcaaagacagcggctatcccattctcggaatagccgctgtctttgtttaaatggcccagatgagccaatattaagatcgatttattttgtctcagtcgtcacaataatgcggccgtcatgctttttgctcaataactcgtgtccttggatgacaccggcgacggtaaatggcagttcataaccaattcgaattgagagcttcttctctgccatcaatttcaacagtgcggtcaaagcttcggcatccgaaattgcctttgtcggcataatcggcttgaactggaactgcttattggataacggctcatccccgccaaccgttgtgatgatgccattttctttcacaatccgggcatcgctgtcactatcggcaccattcaaggccgaattgatcaccacgtctgcccggttggcgagaaccagtgccgggtcctgcttgttatatgagacgtactcgtcaactcccagcgatttaacgtaggcttcgttcttgctggcaccgataccgatgacggttgcgcccaaattaagcgctaactgcgcagccagcgaaccgacgccgcctgaagcaccgcgaaccaccaccgtttggccggccttgacttcaccaaagtaataaactgctttgtaggcggtaatccctggggtgacaatcccggcagcttccgcaaacgaaaccccatcgggaatcttgacggttcgagcagcggtggcataagcgtattcagcgtaagccccatggccatgggcaactactcgatcaccaacttggaagccatccacattggcaccaagcttggcaaccgttccggcaacatcccgaccaggaattacctgatgagtagtcgccttatattccccagcccgcatcgatttttcaaaattattcaggttaaaggccttggtctgaatcaaaatctgatcgtcggaaatttccggggtcggcacctcgtattcttcaaaaacgtccgcagccccgttatgatcgtatccaaatgctttcatcactagcactcctatccctatatcccatattgtttaataaaattgtaagggttatcaatttggttatcaaacaaaaggctcttctgcgatcaaaacgcctcgtgccccactctcaaaaataggacccaaccaccctctaggtgatcagatcctatctgaaacatgttgtctgaaaggcattcgaaccaatcattgaccaattcatggtcggtattcgtatcatttaaatatcttctgcagggtggaacggcagactactcggatctaagctcgctggcttagtacctacattattttcggaaatccctcgtctgtcttgcaggtgattagttcattcacctttcaccattattatataatttataagttagcggtacaaccaatccgtcttcaaaattattcctgcaagtcgcggaagatttcctgcattttgctttcaatgtcgaataattcactggcatattccttgagattaccggtgtgctgttcaactttttcttccgggacatccgtcttataacgtaacttgtgttccaagctggcccacatatccatcccgatcgttcttaactgaacctcgattggaacatcaaacacaccgttggattgaaagaccggcaccgacaccaccaaatgcaggctgcgatagccactgggtttgggatccttgatgtagtccttgcgtttgatcaaggttacatcggattgctgagtcagggcgtcttcaacccgataaacgtcatcgatgtagttggtaatcacccgaatgccgccaacgtctaaaattttgtgatgaatggtatccatgttgagtggatagccttttcgctgaattttacccaccaaactgcggacacttttcatccgttcttccatatgatgaatcgggttatggtcataattcattgaatactcttcgtccaggttctccagcttagtgccaatctcgttaacccccgagtgccgcaattggtagatttgggctaattctttgagatcgccaatctcgcttttcatgggcaatttatccaactctttcataatctgcttaacatccatgaaattactacgttctagtatcatatttgattccaccttacactttcaaaatgttacaaaattggtgacagcagcctactaaacgtctgcttaaacttcagccacagcgactgttgctcaaatttttccggggtctgcaattcactaacatcaatatcatttaagaagatgtcacgcaaatcggccgagaacttctgatcataaataaacgcattgatctcaaagtttaatttaaagctgcgataatccaggttcgctgaaccaaccgaagaaatcttgtcgtcaatcaccatcgttttggcatgaatgaagccatcgccataatagtaaattttaacgccttcctcagccagttggcgggcataatactgagtcgcccggtagacaaatggatgatcgggcatgcttggcaccataatccgcacgtcaacgccggacatagccgcaatccgcagggcatccatcatactatcgtctggaatcaggtagggagattgaatccaacagtaatctttggccatggtaatcagcttaatataacccattttgatctgttgcaaatccgaatccggtccgctggagacaatctgcatattgacatttcctttagtagtcgtaaccgggaagtatttgggttcaacttgatcctcatcgatttgatcccggggactggtggcgttccaatccagaatgaaccgggcttgtagtccgaagacccccgacccaataatgcgaatgtgggtatcccgccaattgccgaattttttcttgcggcccaaatactggtcaccaatgttgaagccaccagtatagccaatagttccgtcaatgacaataatctttctgtgatcacggaagttaatccggaaatccaagagaactgagcgggtgttcaagaatggaaaggccttgccaccggcatcaaccagaggctggaagaacttccgggttgtgcccatcgagccccaggaatcataaatcacccggacttcaacgccttcatgggcttttttaactaacaggtttaaaatttcatttccgatctgatcattgtaaaaagtatagaattcaatatgaatactctttttggcagcttcaatgtcaccgatgactttatgaaataagctgttgccgtcagtaaaaatatgaactttattttgacgagacaaaaaagcgtgatcggttgtcatgaacatatcaacagcggtcttggcctcggtaacgacttcatcggccggtgtcttttcatcatggcccaattgttttcgctgttcgttaagtcgctcatctaactgcatctgaacgtgtttatgtaatttaaacaaccgattcttaggtaattttcgacccagaaaggcataagcaataaagccgaccagcggtaaaaagaccagcactaacagccaagcccaaatcgcggcaatatcgcgtttctccctaaataccgtgaagatcgccaaaattgcgttaatgacgacaattacattaaataccatcgaccaatcaatagtcattttttcctccccgcagccacttttaggctaaaataagaatgcatactgtaagtatactagaaagaagcggaaaaattatggatttattcaattttcttattgcgggcctccatggggtccactcaattcgttttattcacttcatcttcaatgaacaaccgctccttggcatcgggctgatcgtggccttggtgctgtatatgatttatcgttatatgaaccgataatacccatttggaaatccgattaagcaattgccttttagagaacggattccctaattcatttatgaaacacaaataggcctaagccacgaaggcttgggcctatttgacgcatacctgcttcagcacttggggtgtaaggcgaacgctggcacacagtgacttaatgcaataagggcgtaacaaaatactaagtgatcatgataacttttcaaattattttgaaagcggtaccatatctttaatataaacttctgggcaagcaaccacactgttaaaaccaatttggttttaatgacctacccctttttgccgatattcggccggcgtcactccaaaaattttcttgaagttcttgtaaaaatgactcacatcggtgtagccaaccttatcaataatttcttcaatactcatcttagttgagatcagtaactttgctgcctcacgcattttaatatctctgagaagctgagagaaggaatacccagtttcccgtttgataaatcgactgatatagccttcactcaaattgaaatgttgagcgagactttccaagttcacatctttgcggttgacacgaatatactgaataatgtttgaaaccggctgctcgtcaatgttgccttcaagaattgtggcatcgtcagcgtgattgcgaataatctgaccgaacaacaacaggacgtaactgttcaggatgatttgagatccatgcatggatgcttgagactccatgtacaagccaaaaatgatgtgttcaatctccttgtcattatcacaatgaaccaacaccaactgagagaactcccgacgatacagcattctcaaaaagaagttggaaatatcattttgctccattagcagaggagaaaatgcatcctcgaacgatgatcgccgcataataatgttaaccacaatatcgtcgtcagcattacagaaaaacgcctgtttgaggtttgggggaacaatgaccaggtctccctgttccaaatcataggttttaccgttcaggaaaaacttgcaatgcccattgaggacataggagatttttacgaactccaaagtatgttccataatcggcagataacgcaaatgcttaaaaacaacaatttcagaatttaaatggggtggatagatcagcttggaattggaattgccattttgctcaggatgaatcacagtctgtgaaaagaattcactctcgaagaaccgcggacgaatgtcagaaagtggttgatctggaaatttcacaggattcttcatctttgctcgatactgatccgcaaaagcttgccaagttgaaaccggcttaaaattgtcatatggattggcgacatacaacttcttatactcaatttcagcggtttcaagtttcattaatgaatttaaacttggagagttcaatactttcacttccttgaccagacaaacaatgaccggtgacaacagtccgtcgtcccagtcgatcgtttgcaactatttaagatgcttggtaatcaaaactattttcatagtgtccatccctgagttcaactgtgtcatagcctggaatgtcgacttttgcagtggcgccatacggaacgtcaacggaaaccgacagcttgccgtcagtgtaattccattcaaccttggctgttccaaatggggtttcgtgtgaagccttggcagacgttaagttaccacccggacgaggggcaacttcgaactggtgccaagccggggcagtcggcttaagaccaccaaccgttgcatgaatccaatccgcaactgagccaagtgaatagtggttaaacgacgtcattacaccagggttaaccgagccatcgggcagcattgagtcccaacgttcccaagtagtggtgccacccattttgacttgatacatccagcttgggcattcttcagacaggaacaattgataagcctcatccatatgacctgtctcagtcaatgcaggcaggatgtaaggggttccagcaaagcctgtgccaattttaccatgagcgcgacgaacaagtaatgccaacctgtgaccggcaaattctttaatctctggatcgtcatccaccaacccaaaggcaattgccagtgcataggcacattgcgtgtctgaagtcatgatacccttgtcgttaaagaatcgcttcttaaatccaagatgaacatgcttggctaatttggtatattcatcggcctcatcatccttaccaagttcgtgacccattttaacaaacatgtcacaactattggcataaaatgcggttgcgactagattcttttccgtcatggcttttactggatcatccgctggtgccgtgggatccagccagtcaccaagttgtcccagtgagtatgccggcttacggtcccaaacaccatcctctgaaaggtaacctttaacctcatcgatccaacctttagcagtttcatactgcttggcaagcatctctttatcaccacttgccatgtaaattgcccaaggaactcgaacagcagaatcaccccaaatggcaatgccttgcggttcagtccattcagcaaatggaataaatgggacataaaacggtactgttcccaatcgcttttgttcatgtgaaacatcttgaagccagctgctcaaggaaccttcaacgtcgtagaaatatgcggctgtggggctgaacagtgagatatcgccagtccaacctaaacgctcatcacgttgcgggcagtcagtcggcaaggaaacaaagtttgatcgcattgaccaaagcgcattgtcatcaagccggttcacattctcattagaggattcaaaagtcccggtttgcaacatatctgagaagtagactttacactgcatatcatcggcagtcagttcaccgcgccaaccacggatttcggcatatctaaatccgtgggtggcaaagcgggcttcaaagtgtgcatccgacccgtttgaaatgtattgatcaatttgttgacctcgacggagtggccgagtggaaagtgacccgtcactttccaatacttcggcgtgctggagttcaatcacatcgccatcctgcgcgttggtaatatgcagatcaatccgttgagtacagttttgaccaaagtcgacttgccaatcagccttgccatcatactcgcgaatttttttgattgaaatcggcttgttaaccatgttggcacggactggtggcaggattggaaactccatcttccgtcgatcaaacggaatttgggcaactggcagccaatcggcatcatcatatcctggttggtcaaaaccgtccttctcaagatgcgaatcataagtctcaccttcacacaagtcagactgggtgattggccccttggtcactttccataatccatcatgtgaattagagaaaatctgctcgctggtgccgtcaggataagtcacttccagctgcgcgaagacaccaatcttgtctccatagacgttcgccttaccgcctttgaaaccaatccggccgcgataccagccatcacccaagtaaaagccaaacgcattttgaccggctttcaagtcgcccaccaagtcgtaagtccagcattccagacgatcatcgtaggctgtccagcctggggttaagatgtctttgccaatttgtttgccattcacatgaccttcaaccagaccaagtgcagaaaggtaaagtcgtgcatatactggcgtgtctttaagcgtaaactcattgcgaaccagtggtaaatgacgatggtcagtttctgcttccggccagctcggaccaacaaagcttgattggagttcccagtattcaagaattccttcatcaaatttaagggtttgtgaccagtcccctttggtatcaccatcaaccagacgggactttacttcaacctgttctctagaaaccaatggatccaatggccaggcaaacaaaacgttgttaaccggttcggtaacaattgattcaactgtcccagcttgacctggcatatgccgggtaatttggagttcgacctcatctgaatcagccacatggccatcatacttccatgaaatccgcggagtagcggttctaatggctaatacatcgccgtgatagtgttcaacttgtaaatcatatggtgcttttgcattaacaatcacagacattctaaaaatccttctctcttatcagattctgttttgacattaactaactcaattatttttcaattccatacttgcgctgcagacgaatcataattgcaccagcaatgaagctgacaacgacgactccggcaaagcaccacatggtaattttgatgacccctggtaaaacgagggctggggtaacgaaagcaaatagtgcacaaacaacccgtgatgttccgttgataattccttgaattgaagaacgaacctcaaccgggaatgactcttgcgtccaaactttatacaaagcttcaccagccattggactaccaatgttgtagaaaccgatcgcaacgatgattgcgattaagctaccgccacccattgtcattccaaccatggcaaggaacataataacggcaccaattacaaaccccgtattacggtatttgcttccggcaatggatgagaagacagcactgacaactaacgcaatcacgtttagaacgattccggcaccggttgccaaactttgtgaggcattggccttgaccatcatgaaggtctggaattgaccccaggtatttgcaagcaggttccaaccaatgtagaagatcaaaattgcaatgaagaagtacaagaactttttgttttcgccaaacaaaatcttagtaactgatttagtcgcaacttctttactgttcttgcgattttcttcgtaacgagctgttccttcgtcatggagttctttgaatttgcttgacatcgtccgccacaaccaagtgatgattgcgaaaataaccaacagtccaaagacgattcgagccccggtggcaccggtcattttggaaacggcgaaggcaccaatatatgaaataaagatgccggcctgccaaaagatttgcgttgatgacaccaattttgctgaagttttagcatcaggcgaatctcttgaaactactgtcaaagaaatcggtaagtcggttcctgaggcaatccctgtaatgaagaccccaattaataacgtgatgtaattcggggcaaatacagcgattccagcaccgattgcgtagaacaaattgatccagttaaagactttaatcagaccaattgattcagcaatccggccgccaaacaacgatccaaaagcgatggtaaatgtcaacgcaccggaaatgatcccgacttgaccatttgtcaatcccaatccggattgccacaccgaaatggtagcagccaaccccacaataatgcctgaaccaagcatcgaaccaatcccggcggcatacgccaggggacggtaatatgaaatgtcttttgtttccatagttaatgagtctccttatttgctgctaaattttgattgtattttggatccagtttgcgagaactgtatactggatcgggaatatcatgatgggcaataaagcgcataacgagttctgcagataaccagcaaatccctagtgacccaaccaatagccaaattaataatgttggtgaataggccatgattgcgggtgtgacgaacgaaaagactgctgtaactgcgcgaacaattgaatagctaataccggttacgcttgcccgaacatgtactggatataatgactgactccagattttgaataagggttcaccatgaagcatgttggcacagcagtaaacaaaatatgaaatggtgaaaatccaccaaacaccaccgaacactgctgagagaacaaatgataagatacacagaattagaccgaccctagtcataatgtaacggtacttcgtgtcagcaaacttcatgtagatgccgtagaggacaaatgcccccaagatgttggcaaagaatgcacacaaagtggaaaattgctggctgcgaccatcgacggtcaccaaaaagtagttcagaaatgatccccaggtgttagccggaatattccaaaaaagatagaaaccagtcagcccaatcattggcacaaagtaccttggcatagcgatgagttttcggaaaggaattttttctgcggcaacttcttcctcagtagaagcccgtctttcaactgggacaaccatttgagtctccagattatgaaacttcggtgaaagggcacggattccccaagttactaacgcgaccactgccagccaggcaaacaggattctggaactcatatagcccatgtcagctgtcaagaagcccaatccttgagaaagaacaattccgcccaaccaataaatttcggttgaagcaatcaccttaccgtactgatcaggttctgttcgttccgaaataactgccaaggaagtcggtaagtcggcccctgaggcaaccccggcgataaacaaaccaaccacaatcattggcagatttggcgccaaggcgactaataatgttccaagggcaacgaataaaatatctagattgaagacggtgacccggccaaacttatcagagagataacccccaaccgccgaccccaaggcaacagacaatgttaccaatgtactaagtgcgccaacccaccacgcgttcaagccgaactgggttttccacattgccagcacaattccagtcgttaccaaaatgcttgcgtcaagatatgaggcaatacttgcgttcatcgtcaacatccatccagatcttgatcgagacttcataaaatacctccattcttataatcaataatatgtggaaccgctttcgtaaacgtttacaggtattaggatatgctcgggatgaccattcaacaacgtttcaacttattggctttttatgacatgcaaataaagccactcttcatccggatacatacatgtacgctggacctgcatccttgagacaaaaaaacggaaccagtcaacggcaaatgtttgtcgttaattagttccgtttttttaattgatatttatttgagtgtcgccgcaatcagcagcatcatcggccgccttaattcatcacgcatctcttggctctctgccaacattttatgagtgggagtcggttcaacgatttgatctaaattaaagcctcggttcagcaatgtgttcaagtaagtggttaacgtgcggtgatatttctcaactggatagccgagaaaatccgtggtccgtttggattcgtcaaagtagcgatccaccggccaataccttggccggccatcgtctccgaggatccattcctcgtgaccttctgcggtgaagatgggatgttcaacactgatgatcaatttaccgccgggagtcagcttatccttaatcaagtcaatcaatccggcataatccttgatataatgaatcgccagcgaactaatcaccacgtcaaaactgccggcaagctgattaatcgccatcatatccaatacttgataatgaatttgggcttggtcggtcattgatttggctttttgaatcattttggtggatgcatcgattccaacgacttcactggcgccatgatcagcggcgtatcgacagtgccaaccgtacccacagcccaagtcgagcacgcgtttgccatgaaaatccgggaatagttttctcagttcatgccactcgccggctgcattcaggccatcctttgaccggttcatctggctgtacgcttgaaaaaatgctgcatcatcataaatatctgacatcgtcaatctcctacttatcgataaagttccggccgccgatcctcaaataccggcataaatccgcgggcatcgtcagtttctttggtgtcaatcgtgaatacttttaattgaggatgatcgtctaaagtcacaatttcatcccccattggattataaatgcctgaatggccgccaaatggattgtccggatcactgccgacccgattaacagcaaccacaaagctttggttttcaattgcccgagctgccagtaatcggcgccactgcgggattcgtgaagtcggccactcggcaggcacgaacagaatgcgactatcgtcaagactcaaagtccgcagccattccgggaaccgaatgtcgtagcagatcacactggccgcatcgatccctttgatttgaaaatgattttcttcaaccccggatgccaaatactcatcctcatgcatcaaaccaaaaagatgaactttgtcgtaagttgtcagcagtttgccgtcaagtccaaagatataagttgtattgtagaacgcaccattcttttcagttgagaccgaaccgccatgaatggtcatttgatacttcttggccaatttccccaataaagcctgtgtccgctggccgttcttatcggccacctgacctagacgggtcaaatcgtacccggtattccacatttctggaaaaacaacaatatctgcgctttgttcggcagctttttgaacatttggttcgatttgggcgaaattttcgtctggatcaccgaatgtaatatcaagctgtgccaatgcaattttgatcttcatgtgaccgtctccctgcatttttgaaaattatacaacaaaaaagcacattcaccaatcactggcaatgcgctttgacgacgttacataattgcggtgattgcggcgatcaatccaaatatgacaccgggcacatctgccacaattaaaatccaatcccgctttggcttgacccaaccgtaggcaacccacaatgccgcgttaatcgaggcacagaaagactgaataaatgacgtcggttggccgttcaaattttgcaggatctctcctatgtatgagatatacataatcatattggcgatggttgcgatatcgccaatgactttctcctcactgaatacatggttactctcgtgtagttgatgaccaccagggtgactcaactggttttgcacactaatccctccaatttctcttggttcagtgataccatactcaccaagagaatgctagacgttgtcgagattaaattgaacaatttgcgtaatcagatcttctggcaagggctggtcgaccggcagttggatggcgccgatacttgtcttgtagccttccaactgatctttaaagacattgatggcctttgggccgggataaattccgatgtgattcttaaaatttgcgaagtgaataatgtttttgtggtaatgaaacgtcggcatcccatatgaaattttttcatcgtagcctgctggcatttgtttttggataatttcatacagttgcaaaagcttctcttgccttgctgttggctggttttcaatatattcccgtactaatttttccattgacctgacccccttgagaaaaattgttttgatctttttgattaaaatctgttgacatttacattataaggctctaatatacaaagcaacaattaattcgtccataaaaccgatgaagtggagatcaagatcattgtgcacgcaaagagagttgccgcagctgagagtgcaatcgaacgcagatgattaaatggaccactgagggttcttccgaaagttcgcgagtacggagaaacgtgttggtatacgtcagttgccggagggatgttagtcccttgctaagagtgattaattggggaacttaacagatgttttttatctaccctgattaattgaactaaggtggcaccgcggaataatccgtccttaacaatcaacttttgttatggacggattatttttttatctaaattgacggaggtcacacttatgaaaatggaaattaaacgatggcaaatcatagagtgaatttcaactacttatttcgaaactactatatgaaaatattcggaggaatttatcatgataaaacaagccattgaaaaagttgttaaccacgaagatcttacatttgacgaaagccaatccgttctcgatgaaattatgaacggtgaaacatccgaaattgaaactgccagcctcttaactgcattaacggctaagaatccgaccatcgacgaaattgccggggctgcatcatccatgcgaaatcacgctttgaagttccccgaagccggtaacgtcttggaaatcgttgggactggcggcgacaaagccaacaccttcaacatttccaccaccagcgcaattgtcgttgccgctgccggaaccaaagtcgccaaacatggtaaccgggccgcatcatccaagagcggggctgccgacgtcttcgaagcactgggcttagacatcaacgaagatccggccaccagtttccaaagcttgcaggacaacaacctctgcttcttatttgcccaggaataccacaaatcaatgaagtacgttgcgcccgtccgtaaacaattagggattcgcacgatcttcaacatcctcggaccgctggccaacccagctcacccaaccagccaactgttaggcgtctacgatgaagacctgcttgaaccactggccaatgttttaaagaaattaggcgtcaaaaacgccatggtgattcacggccgggatggtctcgatgagatgaccgtcgctgatgaaacggccgtcgttgaattacgggacggcaaattaaccaagtacgttttgacacctgaacaatttggcttcacacgagcagcccgaaaggacttggtcggtggtactcctgaagaaaatggccaaatcaccaaggatatcttagctggtaaaaaagggccgaagcgagacattgttttactcaacgccggatcggcactgcaccttgcccacccggaattgacgattcaagaaggcattaacctcgctgccaagaccatcgacgaaggtaaagcccaagcagagcttgaccgactgatcgccttctctgacaaacgcaaagacgtggttgcatgattttagatgatttagtaaccgcaacccacaaacgtttaaaaaagcacgaagctcaaaaaccactccaagaattaaaaaatgaagctgctcaaatgcctgccagtttgaagcctgattttctggacgttttgaatgaatctgggctgcatgtgatcgccgaggtgaagaaagcctccccatctaaaggaacgatcgtcactgatttcccgtatctccaaatcgccaaaagttatgacgcggcgggggctgatgccatttccgttctaaccgaaccggattacttcaatggtcgcctcaactacctgaaggaaattagccaggcagtttccgcgccaacgctccgaaaggatttcacgattgatccttacatgatttacgaagcgaaagccaacggtgcctcgatcatccttctgattgttgccatcgtcgatgaccagcaattaagagcctaccgagaattggcagagcgcctgggcatgcaggccatcgttgaagcctacacggccgatgaagtgacccgggcattgaaattcggtgccaaaatcatcggcatcaataaccggaatctcaaggatttccaagttgactttaaaaacagtttgaaattacgggcaatggttccagaaggcatccctgtgatcgccgaaagcggcatcaagacccaagcagatgttgaagccctggccgatgccggcttcaacggcatcctgatgggtgaaaccctcatgcgggccaacaacaagcaacaactgattaaagaattcaaagcagctaccgtcaaataaccttcaggaggtgtgtccatggttaaagtcaaaatttgcggtttgatggaaccggcagatattcaggccgtcaatgaagcgcaggctgatttcgcgggatttgtctttgcgaaaagccgccacgtcgtttccttaacaactgcgctggcactgcaggcccatttaaatccaaacatccaaaaaattggcgtcttcgttaatgaatcaatcgctgacatcttggccatttaccaagctggcgccatcgacattgcccagctccatggcaaaagcacccctgaagagattgccgaactgcagcgcgccggactcaaagtcattcaagtcttcgaacgccaagccatcgatccaaagtcgaccgccgactatttgatggtcaatagcggcaaaggatccggccaagttttgaattggcaggcagtcccccacgttgatcgaacaatgatcctggctggcggattgacgcctgacaacatcaatcaagcggttcaaatcgttcagccagatattgtcgacgtctcatcgggtgtcgaatccgacggcaaaaaagatcccaataaaataatgaatttcatcaaaaatgcgaaagaggaatatgtcctatgaaaaatttaactgaagctcaaacaaccaaacgaccaggaattttcgccgatacatacggcggccaatacatccctgaaaccttaatgactgaattggaaaaagtcgataaagcctttcacactttgaaagacgatcccgacttccaagccgaattacacgatttattaatcaactatgccaaccggccatcactgctctattacgccaagaacatgaccgaagacctcggcggcgccaaaatctatctcaagcgtgaggacctcaaccataccggtgcccataagatcaacaacgttatcggccaagcgttactcgccaaacatttgggcaagaagcgcctgatcgctgaaaccggtgccggccaacatggggttgccaccgcaaccatcgctgctttgttcgggatggactgtgaaattttcatgggtaaagaagataccgaccgccaaaaattaaacgtctaccgaatggaattgcttggtgcaaaggttcacccggtcaccaccggctcgatggtcctcaaggatgccatcaacgccacactccaggaatgggctagtcgttccgaagacaccttttacgtcacgggatcggctgttggcccctacccatttccagaaatggttaactatttccaaagcgtcatcagtaaggaatccaagcagcaactgaaagccaaggaaaacaccttgcctgacatggttgtcgcctgtgtcggcggcggcagtaacgctatcggcagtttcgccgattacatcgatgacccaagagtcaaattagtcggcgttgaggctgccggtaaaggcgttaacagtgatcagaccgcagccaccattgaacggggtaccgtcggcatcttccacggcatgaagtcattattcctgcaaaacgaagacggccagatcaacccagtctactcaatctctgccggtttggattatcctggtgtcggtccggaacacgctgccctggctaaagaaggccgagcgcaatatgtcggcatcaccgatgatgaagctgtccaggcgtttgaatacatcgcccgacaagaaggcatcgttgccgcaattgaaagctgtcacgcagttgcttacgtcgaaaagattgccccaaccatgtctaaagatcagattatcgtctgcaccctgtcaggacgcggcgacaaagacgttgccagcatcgccaaatacaaaggagtcgatattgatgagtaatttatccgcaattttcaaaaatcataaagcctttattccgtttgtcgtggctgacgatccggattttgataccacagttgccaatatcgtcgccttagcagaaggcggcgctgacatcgttgaagtcgggattcccttctccgacccaatcgctgacggcggcgtgattcaagcggccgacctgcgtgcttttgacgccggtgtccgcaccaagacggtctttgaaatcgttgaggcagcccgtaaacaaaccgatgtgccgattgtttttctcacttatttaaacatcgtcttcaagtatggttacgatgcattctgtaaaaagtgtcaggccctcggcgtttctggcttggtcattcccgacatgccctatgaaagccgtgatgacatcgttccaaccgctgataaatatggcatcgacatcatcccgctgattgcgccgacatctggccaccgagttgaaaagattgctaaggcagcgtccggattcatctacgtggtttcctcactgggcatcaccggtgaacgaaatgaattcttcaatggtttgaaggatctggttgccgaaatcaaatcgtatactgacgttcctacggcaatcggctttggcgtccacacgccggagcaggccaagacgatggccgagatcgcggacggcgtgattatcggtagtgcgattgttgacattgttgcgaagcagaaacaaaatgcccctgatgcggtaaaaaaatttactcaatcgattcgttcggctgttgatcaagctaaaactaaagaagccagtgtctaaaaaagtccccggtgcggataagcactcggggactttttttggatttatgaaccagtttacgtagttattaccaaataaatccagtatagttagaatctgtggagaagttaaggcggtggcgcttctaaatggagatgatgcctatggtgtaaaccatcaaataggaatttcagaaactctagtaaaaggagagcccttggtgtccgtttcggacgctctacaattaatggtgtcctttggtatctttaccattggactaatcaccttagttgtagagttaatcaaaaattggcaaaaaaaataaccgcccataactttagccagtttgcggttatttaataactaaaaatgcgctgccgtcttaaacggttccacaatgggaagtcctgttgaatcggggcttcctttttgtgatttcattataacatggatatgagactatcgacaaaacaaatctcctaggtcgaggtaaccttttacggatttctagtgggacattaaagcaatattttgcccctcttatataaattatttctataatttacgtttccggagaggatctgcaagtcaacctccacatgctatactaaaataaatgaactagtggaggatgatatattgataaaaatcgctgtaatcttaggatctatccgcagtaaacttggtgaatccattttcaaatatttacaggccagctttcctgactctgatcaagtgacctacgattggatccggctagaagacttcccgctggaaccctatcaccatgatgaaacgccattatccaatccgattaccggcttaaaagacaacgagcaaaagtggctcaaccgattgaaagccgatgatggcttcgtgatcatgacgcccgaatatgatcacgcaattcctggcgttttaaaaaacgcattggactatgtcggcccggaagtggatcacaaaccggtccaaattatttcgtattcctactatagtgacggcggcatgctggcagcggaatccttcgtggaaattttgcaaatgctcaaaatgatggtcctgccgacgccggttctgttgtggaatgccaatgataatttcacccaggcaggcgacctgatcaaagatgccgataacagtgaccattttgaagcgcgactgaaagaagcttttcacgagattgccttttacacccaattactgcacgagcacccatttaaataaatcagaggtcagtcatgcgagccattttacccaacaaaactgaattcatcccccacgcccctcaaaatgagcacgaaatcttcatggcgatgcgcacctatcccgacaacgtcaaagtctaccatccccatggcagtattgacgccacttcggtcttttggcataacaagctacacccaaatgccttgaacttcgctgtgtatgtcgatcccaaggccaccgaacaagatgtcttgtttcaacgtgtctatgaggatattaaaaaattagcctggaagttcgatgacgaccgcatgatcacacgcgactatgctcctcagcatcctttcaatcagtggttaacgacgaagcacttccggttggtacaaaccgcgttgaccgcaacagtggatttaggcggcctatcactaaacgcgccgactgcgtcaggggcgctcaagacgttcgctgaagtatcatcgcaggattcactctaccaatccgtgctggaacgtagcatgcgcgaatacgccggcaaaccaacttttaatccagcgataacgatgccattaccagattggtcagcactcatctcacatcgacaaatttcgacagccccattcgcgttaattcaagacgatcagctggccgccttcagtttcctatatgaccttggtgaacactcggttgaacttggccaaatgaatgcgactaatgctcaggcgctaaatgagttattgaaccgacagcttcagtggcttcaagacaactaccagaccctggctggtgaatttggaatggccaaccggctggagatgaaaatttttcaaagtttgccgtttaaagatgttaacaagtacgaaaattatatgcgtttaacgtaaaacagactaacccttgtagtgaaccccaatcccgtcggatctgaattcaccacaaaggttagtctgttttataatgctttaacaatgtatgagcggccaaacacggtcattgccttctgcaggagatttaaactgacttttaagctgccattttcaattttggcaagctggctttgttcaatgccaatctttttggccagctcaacttgagtcatccctgcttgacggcgttggtatttaatcgtgtaggcggcgtcagcttcagcaggaagctgaagaacttcattcaaaggcttattagcttgagctgctaaaattaagtcggcaagttctgaattcgtcaagcttcggccaattgcctgactgataaatgatagttctcggatgccaatcgtgccattgaccagttcagaaagcctcgaagcagcctgctgatagtcagcggagtcagcccgatcattttcaataacagtgttcaaatgatccaacgtattaatcagttctgtcttaatcatgtcagatacctctccacggacagtacttttcaacgactaattttctggcttgagtattgaaaactatattttgtgaagacaaaaagttgccacctaagtgcttataaaaggcctctgtcccatcggatttgctaattaattctacatagccttcaaatccatcttgcaagaaagaatcctgcattacaagtgacaatagcgcagctcccaaacccaagccacgattttctttttgaatttcaatcagaataactcgattaaataagctctgatagtcacgaacaaatccaattagcccgactaaatttgaattaagaaatgcaccaactaaaatttcattaggtactaactgatgccaattaaagataaatccattcgtatccagtgacaaaattttttcagtcacaacatcaaaagtaacatctttcattttcaattataacagaatattccaaatttgaatattaccaatcttattctgccttctcctcaccctttagatacgaagaaaagtaaaccactctctattgaaaatgcttatacctaaaatacttataaccaagcttatgatcaaacatcgtctccgataggcccgtccgattcgccataaaaatataaatcgcaagagccaccagaccaaagacgacgcagtaaaggaatgccggaatcaaacggcttggcatgatcaattgatgagttccccaagtcagtgccatcacaatcacaaagaacagcaggttaaccaggacactgaccttcaatcgtccaaatgggacatggaactcatacataatttcgccataacttaacagacaaatgaagccaaaaccgatggcggtggaaatgatcgctccaaatccttgaagcaaaatgaccaatggaatttggaacagcaatttggcaaccagtccgacaaccagataatacatggccttcttactgtagtgcagcgcttgaagtagggttaggccattaatggccagtcccaacattaaactttggagaatattggctgccagatatttcccgccaagcaggctgaatgagaagaagatcccattagtttcatacgacagcccacacagaatggtcacgatcggcagcaggacaaacatcagcatgttcacattttgaaagatcaaatctccgacgtcacctttcttggaggcctgactgtttgccagcagcggcagggtcgtctcggccacagccaatgccagtgaaacgaccaccgtggtaattttggttggattggcagaaaacagcgtgtagatgtactgggtatattcggccgaaaaatgctggacgccctgcataacctgtttgaagaataactgatcaatcaactgactgagggtaatcccggagccaacaatgacaaagggaatcgattcataggcaatcatcgtgaaaatcttcttgatactagtcaagtcaaacggcgcgctcttcttggccatttcagcgtaatgcgccgattgtttacgataatacagccccaggtaaaggtaactggccaaagcgccaacaaaggccgccatgacgcttaaatacaccgcctcgatataactgcggtgaaaaacgtcaatcaccagatacgttgacaccagaataaagacaatccgcacgaactgttcccagagctgagacacgccgtacggtttgaggtcttggttaccctggaaccagccacggacactgctcattgacggcaaaatcacaattgccggcaccagcacgcgaatcgaagtcacagcactttgagtggaaaccaccggactattcttggcgattagcggcgcaatcacccaaaggactgccccacaaacaactccggagagaagcatgacaaaagagccaactttggcaagttgacgtgaattcaaaaatttattttgaccgttataaatcgcaacccgccgggcaattgcggagggaaatccggctgttcccagtgcgataaagaggccgtatggattataagaggcgttaaataaagccatggcaacgttcttgtgctcgggtgacccaatcatatacaaccacggaatcaggtagaggatccccagaacccgggaaaagatactgccaaatgaaagccagaaggatcctgacataatttttttgttcatggcgacatgcacactttctatatttcaatcataaccaatattataatatctttcgcaaaagtttgctatcaaatcagaaacttggtttgcgttttttgagaacttgttggtcttaataaaaacagtgtccaaaacaaaaacaggaaaattttgttttgggcactgttggttttaatttgtttggttgcgaaatgtgctactcagcccagaccctaacgtataaggcaaaaagccgaatcaaccagcatagcccgctggtcaatccgccttttcgccttatacaccggggctaactgggctgatccgcactctagtcttccgatacctgcgcgttcttttggatatccggtgacagatcgtacatttttgctgcttctgttaacattgcatgatatgaataggcgccatccttatatggttcgatgacaacctcgtcagcaatctttgaaaatggcttcttgccgtcttttacctgtgctgaatccagatctgcgacaattttcttctccacgtcggaataactgcccacaatctgcttagtctctaaactgccttgtatcgaaattttactcattagcaattcctcacaatcatcagttatatttagtgtcatcataccgccaaaagagaagcgatatctctaggtacatcataccaatttattgacccttatttcaccaaaaatcgtaaagaaagtcaaatttaattttttaatgtcaaatgaggttaccccagcaaaaagcgcccaacacaagttaatcacttgtgtcaaacgcctaaatacaatttattgatgatagaagtagctggtctgggccttatgcgtatcacttgatttataatacatcttcaaagccgtcttgccgttatgcttcacgtgcttcaagtacacaggctgattctgtgacaacaaggtcaacttccagtaaccgtgactgttcgctttattggcaaccttgaacaagtaagacttgctcttagtttgtcgatattttttgatgttaacgtaataggttctggcatcggctttttcagatgccttcgatgagccctgacggaatgaatatttggtcagccggtacttaaccggaacgttgccaaacaggtcatcgtgatacttaccaaaccaagttccctgcagcgtcgtcggaacggcgtgggtcgtggtcttggcggcagccggctgcgcttcgatggcaatgatgccaactccaagcgtaacggcgaggaatgataaagttttgctaaatttcatcgaactgtcctttcatttgcaaaaaagcaattggaagtagtctaacagataattcaatttcatgcaaaattccaaactaggatacgacctattttgattatcctactaaattggcagttaccacggaatacaaaaagtcagctgaaattgatcatcatcaattccaactgacccacttttccatttggtccaacatcttcaactccttaaccgatattcaaaccataatcgatcttcgtatggtttgaggactttttccagctggttgcggacgatattcacccgaagatccgcggccaaaatcagcccacaaatcaccagaatcgaaatttcaatggccactaagccccaattctgcttggcgtaaattaccagggcttgctgaagggctagaatcgccaacatcgtcccggtcttattggccaaaaaataccaacgattaatcactcggaccttcttttcggtcaaagcccgcgcttcggctgataaattaggcgcgtttgccaatgccaatttgagccctttggcgtccttcttcagcagctcagaaatatatgtcgaggtcttcccaacattttgcttcgcaaagaaatccccaaaccataaactaatcagaaaaaaacacaagaaaaaatctgctaacttcaacgtgtccgtcatcgtaatccctccgttctggcagcgactgcggttaacccccttgacaagttcaacgatggataggtaacttatcgttcaatcactaatttacttatcctggtacgagcagtatataacgattagctgggctttggtaataatctgcttgtgagattcgggtcgtgtgtgaggtagccagatacaaataaatagacgatactctttgctggtttcacaaagaatatcgtctattggcttggcaggaagcgaaaatattggcaatcgctacctgcaacacctcatcctcaagcttccacaaagtcccgacccatcttccgatcacagaccatcgcggcaacggccaatccaaatgagcagatgccaaaaatcagccagctggcaaacacaccttgactccccaagttggcgacggttaggaaaaaaccactgccaattggtgcgccaatcaggagcaccatgttaatgaaccccattgatgcgcccagccggtcatcgggaatcagtttgatgaacatggccgagacccggggattgattttacctaagaggtagccggtaatcaccgagaccaccgcaatcaagatgatggatattcccgttaggaatgttgctgccaacaacaccagcatccaactgatgtaggctgccaatctgacaacggttgtgtttgccaaaaagtcatgctgaatgacggcgccaagaatcattcccaaggacatgctgatgctgaccaaggcaacactgttgccatagttgcccagccatagcgcctggttgtgcagcaacgacacattaatcaacccggtcatcccactggcgatcgtgttcatcacaaatgcgaaagctaaaataaccacaaccacctttttggacatcatgaaatgaccagtcacgatcaaacttttcagcaaggattgtttgggcgtggctgattttggctgattaacgctgagcttcggatcaattcccttaaaaattgaccgccgagtccaaatcacgattgccgcgattaggaaagtcgccgcattgatggcaccaaacagcccgtagttatggttcagccagacaatcgcaacggccccgacgccttgaaaaaccatctgcaaagtcgtttctgtcgccatttcaaatcccattgcatcgttcatttcttcattggggattaaaaaccggaagtacggtaattcaagactgccggaaaatgttcccagacaatcgctgatcacgttaatcgccaacaggcccccaaagaccagcgtcgatcccggaaggccaatcatcagggctaacccaataaacaaggtaaactggctgactcgggcaaggaccatccactcgtacttatgatgggtattatcggcataatagccaaggaccacgttaatcatctctggtatgtaggttatgaatgaggcaatactgacggcggccgttttgaatgacaagctgccagcataaatgataaacacaatattgaacaggctattgccaatcccgttgaaaatggcagcgttcatcaatgcccggtagcctttacttctaaaatatgagtgcatgtgatcccttctctctcaatgcttgcttatacattatctgagaattacacttagagtattaaaattccactatatgagaattaatttggggtgatcagatgcaagaaccgggatgtttatatcgtcagttacgaaaagaacgccatttaacacttcagcaggtagctgacagtgaaaacagcgtttcatttattagtaaatttgaaaagggtggctcacagattagcttcaatcgaatgattcatctgctgggcaaaattaatttttcagtcgaggagttcctctatcttcaaggacgcgacaccatccagccaatcaagtcgacgttcatgtcgcaccatccaatttatctgacagcgccgttcatgacgccgatggtcacgttactcaacagtctgacgggcgattcagagacttcagcgacgttgccccagtcgatcgaacaatacgacgctaaaatccaccagcttgaggatgccggtaacctgaattggcaacactacttggcgattctctaccaaattcagcaagtcttaattcaaaacgacgcctcaccagcaggggatccgaagaccgcctttgccaagctgcgccaactgagccggcccatcgtgacttacctctataacattgacaattggagtacgtttgagattttgctctttagtatcagccactttgccatgccgcttcaaaccgtccatcggttgagtaaaatcgccatcaagcgaaccaccagtacagaaaccttcccgatgatgccgcaaatgagattcgaactgctctttggcctattttcaacctacattaatttccgccaaatggcttgggcaaaggaagccctggactcaattgccaaattacttgaggaggatgccgatagcaactttgcgatcatgctgcggttttaccggggctggtacgattacatcgactcaaacggcagtgtcggtgaggaaatgatgaccgatgtcgctgccatgttcaagctattaaatctgcgccaaccagccgacctgattagcaaaatcattccacagattaaacgcaatcagcgtgatccggagaagtcgatgatctttctgttttgaatcaaaatcaatcttcccatttactcaaatccggtccaccaggaatgacccgatcaaacgaagtcaccggatcatcgctcacttgaaagaagtgctgcttaatagcggtgaaatcagtattttgcttaaatgccggaatctggtagcattccttcgcgtaacgccaaagattagggaaatcaaccaaccgttttttattcagcttgctcttgaaataaaacaccacatcaaagcgaatcaaactgaccaccagccaaaagtccggcagggtaatgtgatcgcccattaagaagcgcttgtcagcgagtcgccggtccaattgcgccaatcgatcaaaatactgattgaacaacatgtcgtattcggcttgcgagtcaacgtcgttaatcttgcccggaattgacgtgatgtcggtaataatgcgcgtgttcatggcgtcaatttcagcctttaaatcgtctggataaacgtctggcacattttgatcgaaatatcccctccaagatccgcccaattcaaacataatatctcgtgaagaatcattgaccacgccaccggtagttaaatcaatcaatgccggaaccgttggccgtgccgagaagttcgggacggcctttttgtaattctgcgacaaccgcgtggtatggagcatcggatcttcatcgtcagcgttcttgccaaagaaccagtcgtcatcaatgccaggatgacgcaagggataggtcgcaaatttggaaatcaccttgttcaaaccggtgtaatcgatcatcatcgctgccggggtggcccagggacagaatttcgcccagacatagtgataacggttaggttcaaccggcagttcaccagtggaaaatttcttagtaaaacccgcgtcattcttttgtgtcggcaatgcacaagcatccccgcgtttcacattttgactcatcaacatcgctccaatctctcatatttgcctctactgtacacggatcgaccttaaatgtcagtaagtaaaaacggaattactcgcaatgagcaattccgtttttgattaattattgataactatcataaagtttctcaaagttcacagtaccaagcccagtcgcctggttatacaatttgccaggttggccgacatagtacaggttcgagttgttcgaatcactatccagcaccgtaaatggtgtcttctccggatcttgtgccagtgcgtaaatttgtggattccagaagcccattcgagttcccttaccactgttaataaccgcagtcacaccgttaaattggggtgcaacagcactggtaccacccaccgtcttccaaccagttgccttggtgtagatctggtaaccagtgaagacgtcggcatcagctgagacatcaggatagttccggccatattgggtgccgctgaccagaaccgggttgggactcggctgcatcaaattcgaaaggtattgacgcgcgttaaaggtattaaccccggaaacaccctgctggtaggctggggtatcatacagcttactgatgccaccgccgccagcgctatataacatttgcagtgcactcaagttggtttggaataactttcggtgcttagcgtatgccttgtacatataatcggcaccccaggcccgttccttatcgacggaaatcttcacaccaccgccaagattcttagtaaacggcagcgtggtaccgccagtcgaagtaacccatggattgtctgatggaaaatcagcgtaagtgctgtaattaggaatgttgattgggccaaacgtgccgccaacgcccatcccgtaagctccggtatcaccagaagcaacgaaggttgaaatgccttggagagccccctgagccatcaacaagctcattgcctgaccatataccggtgtcagcagtttcttctgattcaagtagtgggtcacgtattcatttaagccccaactcattgaaagtgagctggccttattctcatcgaatgccgttgcgtaggcattggtcaacccgacgtcactccagttggcttggtagacgcggacgttggcttgtggtgcaatcgcacccgattgttcaacatccaaggtggtttcaagctgaccagtaggaccagttgagctgtagacgggtgaagcaatcttcttgacgctcaagcgatttggtttcacgtcaagcccctcacccttccagaaggtttcagcgtcactcttcttaaagccggcaaaagtaatgatcccaacagtttgaccttggccttgatagcccttgtcatacagtggttttagattgtagtgattgacaaatttgcttggagaatccttcgggttcatcttacccttgggtgtcttgctcttggctttgctggaaaccaggccgctgccgccctgattgaaggtggtaacccccaagaccgtcagcaccttgtcggccaagttggcaggcatcactggctttttggacgagaattgaaccggattggagtggtaggtcgccgtcttcaggttagttgagaacgccttgttgacatccttggccttgccagtgaccttgatgatcagtccatttgaaaaggtgcttgatttgagatgatatttgctcaaaaacggcttaaattgaccggtcacacttgctggctgaccaaattggtcacggaagtgctgcggcgtatagaaattcttgaagtcaggattacccggtgtgttgacggcgtatatctgattggtaatctgatcttcattctggggcttcaaaacaatgtccaactggacttgcttgttaggggacatggtcttcttggccatgagtttcttaaggatcttctgaatcccataaggatctttcccagccgctttcttctgtgaagctgcttgagtcattggtgctgcggacacaaataatgctaaactggccaaaccgaccagccaatgattgattttcttcattcttcccaacctctttctaactttcaatatgatagtggtcgaagtacaccggttctgaataatcccccaatcatcaggactgcataatatatgtaaaaaggcgcaatctgcgaggcgccgaaaaacatctccaactattgcgagagtacacgtttcaagtaaatatgtcaagaatgttacagaatcatttggattgggtatttatacacaaagaagcatcctgaaagtttagagactttcgggatgcttctatagaactatagaaagttggaaaattaactgctatggtagctttcaatctagctttgattaccaatgttatattgataaaacgtgcaacgacggccggctgaaagcctgtctagcctacttggcgatcggctgatcccggccatttaagcaaagaaacgagtcattccaaaaacaggaataactcgtttcttcacttaaattctgggatcaaaacgcctcgcgtcccactcttattttggatttgcagcagttaatgaaaggttgctccagaattcattgttggttggtgcaacactgtagcccttaacccgcttgttaactgggctccatgccaaactgaagctttcaggagcgtaagcagcttgactgttcatgtaacgttgccacttcttgtactgttgagcacgatactttggattccaagccttatcattgttcaagctcttcatcaaagcagtgttcttttttgttgcaaagtgacccatgttgaatggtgcgtcgacaccataaatttgagttggtgttggttccgttgaaagtgaccatgcagcaaggaagacatcaatggatgtttgctttggcttttgaagggttgcgtagaaactattcatttccattggcttaccaccggtcatcttgacgttcaaaccaagcttgtgccattgttgcagatagaattgatactcagcttcagtagcagctaagctttgcattgcacccaaatggataaccagctttttaccatttggatcagtccgccacttgccgctcttcttgtagcctgctttatcaagaagtgatttggctttcttcatgttgtacttgaagccagggttcttagcgtcatagacatccttgaatgcaggtggaatcaaggtatttgcttgccatgaaacaccgtttccaaatttcttctcaacggcattaatattcgcagcgtaaatcattgctcgacgaagatccttgttagccatcttggaattcttatccatgacattcaatccggtcttagtgtccatgtggccaacattaaagccaaagtagctgtatcccattgaaggagtaccggcaattccgtagtcactcaacttcttgaacttaggatattgactggatggcataactgagttagcaccaccggcaacgaagtcatatttcttagacttgaaagcagccagaatgttgttagatgaaacaacttgaatggtaatatgtttaacttgtggcttcttgccatagtagtatttgtttggtgaccaactagtggattcaccctgaacaactttgtccagtttatatggtccaacgaaaattgggtttttacgaactttacttgaagcagccaacttggaaattggaatgcctttgtagtattcgtatggttcaacagttgtccagacaaatgagtttccggcatacttcattgaaggtgacatcttactgtaatggataacagtggttcgaccattttgaccatcagggaatgtaatgcctgaaatagtcttggctttccctgcatggtaagcagccatccctttaatggcagcataatcagctgaatactgttgagacgtggtgctcttattaccgatgatttcatatggatattcgacatctttggcggttaccttagcaccatttgaccatttagcatccttacgaagggtaattgtaatggtcttggctttacgatcaatcttctggttggcaaggccgccattcacaatcttatagtccttcgttacattgaacatattgcccataccaccaggtgaaaagacatcttgatcttctgcgttacttgccaaagttggtgctgaaatcccggcaaatggggcatcattaacttcagcaaccttcaatgtactattatttcctgctgtagtcgccttaccagggccactatatgtagctgacattgaaacatgcttgccggcgcctgattcactgctcttaccattagagcaagcagcgagtgtcataactgacagcatcgcaattccggctgtgagccatttctttttgctcatgaaacatccctccaaatctatatttgaactacactaccaactaaacctcacctcaatatgcaaaaaccgcatcatctcctttaatgcccaatttttacttttgatcctgaccacgccgttgagcagcgttggtggttcgacgcatgacttggccaatataactgattgacagacacaaaacgataatctcaattgcggcgggcaaccaagtccaccagtactgagtgatattttcagggtcgttggcattggcgatcaaagttcctagtgatggggttcccattggcaggccaaagcccaagaatgacagtccagtttcaacaccaatgttttcagcgaatgacaaagtagtatcaacaatgatcaatgacgaaatgtttggcataatttctctaaaaatgatcttaaaattactggtaccggaagtcttggaagctgcgacgtaatccttttgcgattcagctaacgttcgcgaacggatgagtcgtgaagttcccatccaatagaagatcgacaggatcagcgtcaacgtgatggcattgtaatgtggaataatcgtcacaatcacaataattgtcatcagcattggaataatcatcatgaagtcataaacacgctgcatggccaaatcaaccaagccgccgtagtacccggaaaccagaccccagcagataccaaaagttgatgagatgatcgtcaaaccaatcgcaatcgaaattgagttacgtgagccaacgattaattctttggcaatggaacggccaccagcatcggcacccagccagtaatccggggtaaagggcttattgtagtagcccatgatgttggtttccatcattttgggaacatcaatgaattctgaagcgataatcacaaacagaataaagaatactaataagaagagggaaaccatcgccggtttatcagccttaaactcaccccacatgattttaagccgtgacggggtggcttcttcattggcttctttagttaatttagcgaggtcctctttggaaatggtcgttgcgtcttcaatatctcgtttcatcttcagcaccccctactcaacccgaactcgtgggtcaacgatgctcaagacaatgtctgaaagcaaagttcccagcaagttcaggaagccatatagcagcaccaacgcggtaatgacggtgtaatcccggaagttgatggcgttcaagaataagagccccataccaggataagagaagaccatttcagtaaagatcgacccaccaagcaggccagtgatggagtatccggcaaaagcggcgattggcaacagtgagttacggaagatatggtgacgataaatatccttcatcggcacccctttggaacgagcggtgcggacgtaatcggagtgcttggcatcaatgacttctgaacgcaggtactgaacgatgttgacagttccaaacaacgctcctaaaagcccgggtaaaatgatgtggtcgagccgggacaacaccgtcccgccaagtccgcttgcctgagcggaaactgatccactggttgggaaccagttcaatgcgtaaccaaaaatccaaattccgataactaaaacaacgaagaatggaatcgacattgtgacatatgtatatacacgtaccaaagtgtcttgcagtttgccttcatgatgggcagcgtacatcccaagcggcagaccgatcccgtaagtcaaaaccattgtgaataatgcgagccataaagtattggcaccccgctgttgaatcaaatcaacaactggttcctggtactcataactcatccccagatcgccgtggaacaaatgaacaacccagttccagtattgctggtaccagggatcgtacaatccatggatttccattaaatgatgaatttgagcaggatcagctcgggggttaattgacccggtaaatgggtcaccaggcatggccttggccagcaagaaaaccaaaatactcaagataattaattccggaatcataattaagacccggcgtaaaattgttttccacatcagacgtttacccccttgttctcagactgctgttcaaattccttagctaactcaggcggtaaagccaccgagtgagttggtgagactttgacgagtggaaacgccatgccgtcttgatcgtaataagttttctgctgttcttggtaaattttctcaatctctaaacgatgcttgcggtgctcctctcgatgattcacgttggtttcaggaatcgcagccagcaggcgtttggtataaatgtgcattggattattgtagatatcatcccgggtcccaacctcaacgattcggccgcgggtcatgatggcgatgttcttgcacatgtgacgaacaactcctaaatcatgggagatgaagagataggaaattccaaactgacgttgaattttcttcatgaagttcagcacctgggcttgaacggaaaggtccagggcagataccggttcgtctgcgataatcaattttggatgggtggcgactgctcttgcaacgccaattcgttgtcgctggccgcctgaaaattggtggggatatttgtatagggcatcagcgtccaagccgacaatatccaacaattgaagaacccggagcttttcttcttctttatcgagatgctcaaaattgcgcagtggttccgcgatgacatcttcgattcgtttacggggatttagactcgaaagcgaatcctggaaaatcatttgcacgtcgcggttataatcgagtttgcgccgattttcgcccttcgtgacgtcttttcctttgtacataacggttccggcggttgctttttccaagccgatgattgctttggcggttgttgatttaccggagccagactcaccaaccaggccataggtttcgccagcttcaatatcgaaggtgaccccgtcaaccgctttgacgttatcgacgacgcggttccagaagccgccgcgaatcggataatgaaccttaaggccgttaatttcaattagactcatgaccggcgccctcctttacttggtctgggaaataaaagtctttatagcaggtgcagcggactaagtgattgtcgccaatgtcgtgcatggctggatgggcttcgtgagccgaggctggaatccaaggaatccgcggtgcaaatcgatcgccatcctttggcatccgttgaagtgacggtaccatgcccttaatcacatagagctcatcattttcgttgtcccgctgcggcatcgatctaagcagtgagcgggtataagggtgcttgggctcattaaagatttgagcggcagttccctgttcgacaatttggccggcatacatgacagcaacccggtcggctgtttcggcgacaaccccgagatcatgggtaatcagaataatgccggcgtggttttctctttgaatatctcttaaaacatccaatatttgggcctgaatcgtgacatccaaagcggttgtcggttcgtccgcgatgattaagtcgggcttacaagcgattgcaatcgcaataataattcgttggcgcatcccaccggaaagttgatgtggaaactggtgcgcggtccgttcaggatcttcgatgccaacttggttcagcaattcaatcacccgggcatgacgctgtttttcggtcatcttggtgtgataaaccatcacttcttgaatctgatcttcaattcgttttaatgggttcagagctgacagtgggtcctggaaaatcatgccaattttggctccccgaacctggttatagcccttctcatcaagtttcaataaatcggttccctcaaaatcgatttccccggaaatttgagtttcttccggatcatgcagccccataatggtggttgccaaagtactcttcccacaaccggactcccccacaattgcgagaatttcatcatgctttacttcaaggttgacgtttgaaacggcatcatagtattgaccattaatcttgaatgcggtgctgacatttttgatgctcaagaattggtcagaatttgtatcaaccacgagaatatctccttttggcaatgtatttatgtataaacattaaaaattaatgaacggtatgattgtttaattagaaaacattatattctcattgtattctcatttcaaaccatgttaagtgttttttgtaaatatttgttatttggtagattgcaaatttaatccgaatttttggacaaatttgtcagcataacctgatacggtgtttgccagtcgagtattttaagcggtcgctggttaatttggagtaacgtcgtcgttaaatcttgagcactaatgtgctcaaaacgagtccctttaggataaaaataacgtaaattccgattaaagcgttcattactaccacgttcagctggagtataagcatggcagtaataggtcttaataccatattgtgattcaagtgatactagcccactaaactcagtgccacggtccacagtaaagctgtgcaccggaccattaaaagtggttaggaacttagttagtgcttcattaacagtcgctgtcgtccgatcttttaaccggtatgcccaaaggaaccgtgattttcgatcgattaaagttaataaaactgccttactatgcccacgaggaccaacgactgtatctagttcaaaatcgccgatgcgcttacgttgattaatcatcatgggacgctgttcaattgatcgccccaaagattgattatatttggatcgttggtcaacgttacgccgttggcgtacgccatgttcaggtagatcattcaaggagaaaccaattctcccctgatttagccaattataaatagatttagtagctagtttaaattcgtgagcaatcattcctggtgaccagcttagacgtaaatggttgagaattttttgctttaactcatcgctcagcttagttttccgaccacatcgtgatcgcttgtattcggcatctgtttgtgctaattcagcctgataaggttgacatcgagataattcataagaaattgttgacggtgatcggttcagccgaacgcccatttggatattggacagccctagttcacaaaaggtttcgattttaattcgttcggaataggttatactagacaaaagatcagctcctaaaagatgggtttgtggtaaacaccattttaaaggaagctgatcttttttgtccgaacagcgttcggattaattttacaatctaccatttaaggatgaacaaggtgatgagatatgtgtctgaaaccccatttgaaaggcgttaatcggttgttcgcgattctaaaatgattactggattcttttaaaattaagaatcaacggcaacgctcccgctagctgaaagaagagcgcaaaaaagccgagacaacccttaatccagttgtctcggcctacttcttaagactattaactttgtatgaatcccttgattggagaatgtgacagcttctttttaaatgagaggaccaaaactctgtcagtcatcgtctccctgatccctcttctgcaccgctggttttataggaacggccgtacaccattcgctttggaattgcacttcgaagtgattggctagctcttccatgagcagtcttcgcccagtcactgcgcttggtcaccaagcgataaaaagaaataaaggcaaccggtgtcagcatccatgagtaaatcaggttaccttcaaccatgacaaccgtatcccgataattaaagtgatcgctaggctgtctcatcaatcgattggccaaaaaaatcatcaaataagtaatcagcatccctattaagataaccgtgccaactaccatcatggtctttcgagggaacacgaccaaatgataggtcatcacaatggttgccagcaacgagctgaatgtaaacagcatcgagaaaaacggcagaatcataaagatgattaaatcagttttaagctttggtgggattttcttggagaagaaaacccgcttgccgtatcgtttgagacactgcatcccgccttgacaccagcggacacgctgcttgattaagggtttgtattgattgacgccttcttgaggcataaaggtgttggcaagaaacccaccattaaaaccatgcagcaaaccgttgatactaaattccaaatcgtcgagcagtgaattattccatttgatttgggtggccatttccaaggtcatgaattggccgttgccggacgcgatcgcactcccccagcccatgcggataatctgctgtaagaagttgggaacgccaaactcaaattcctgcatcaaagtcagaaagttatgaatgttgctgatcgagatgccggtttgtaataaatcataattggaatgggtaaaaccattgaaaatgttcaacaaaatcttgaagctgggttttgaatcgctgtcgattacgccgacaaccgtctgtttgaagtcgtgggtttgcgttgtaatccactttaggccatcgttgagagctttccccttaccttctctggcatggggcagtttgcgagtcaaaatgtgcacccggttattgcccacgaatctttgtaatttcacatccgtgccgtcgtctgaaccatcgttaatgataatcaaagtcgtcttacagggaagtggactcattgcccgcaacagccggctaacagtggcttcaatttcattcgcttcattgagtgccggcatcataatatacatatgcttaacttttcgctgaatatcaaccgaataatgggcctcagcatttttatggcaaaaaatattgaagagattgagaatgccaaatcccatggtactaaacaatgagatgaataagaagacccaaatgataacccatatgtccatgtaatcacctccgtgcaaactgatttggcgttgtcatgaatcaagacgaccgccagccgcttaagtaaatcaagcaatcatccccatcaatcaggaacaattgcttgatttacttaagctctgggattaatcacaccattctacaatctggtgttaccatccccagcacggaatgaagtgatgatgacgtttgttataaacgttgatcaagttgacattattattggcgtctggtgtttgctgacctggggtcttagtcttgtagccaaatgggacgtagtcttcagcgactgtgtacacaaactggtttccttgactgtcatactgcggcaagtaacgaaaagtcgttcggtaacaatcaaaatagcttaatgttctaaatcgatatggaaccccattttgatacaacgtcacatgaacccgtggagtgcacttccaaaatggcacgttcttccaggtctttatgacgtgaacataggtgaagcattgcggtttcttctgataaacattggtaagggtaactacgccattactatcgggtgcctgcggcttgttaccatccggatcactcttataaccctccggcactgaagcttcgttgaccgtgtaactgattgcgtgaccgtctttggcaaatttggccaagccgttaaactgagcctgatatgaattagcttcattgagggtaaccgtcttgccggtatccttgccgtccgcgtacaacttagcagtaacagctggtgtggtgacaccatcaggaacatcctgccagacctttttgacagtgagactcgtggtggcgtcggtgtgatcaccggttgcggaacctttacccattgtcagaaccaccgtcttggtgtttgaagtcgtaacgggtgttccggcggcagctgtcgtgatgtcactggccgtaattgaggccgtgtttggcaaatccaattcagtaccgtaaaggctgtattcattatcgttactgatgtcggaatgatacataatattaattgccttatccagtgtgccattccactggaaagtgaatccagaatcagttggggtgatggtgtaatggctggcagcgattgtttggccgccggcattgtcagtcaccgttactgatttaggatcaaaggtttgtgcggttgtattgcccaaagtatcttcaacttggacattgttcaactggcggttattggggttaaccaagacctgccagtttacttgcgccaaagtcccattcggacggacagtttcgttgatgccccaaccatttttggcaagaaaaacgttcactggatagctgggggtaaatgcgcgggtaccggtgactgagaattccaatgacccgtgccggttggtgttgtatttggcccaataagccgcgttactgaacgtaatttgcccagtcgtggcctttggattggcaacaaattggccaaccgtttcgttggtgttgcttgatttgatatcaaatttctctggtgttcgaaatgttgcaccagtcggtaacgtgactgtggcagtatcaccgttattaacagttgtcccgtcagcaatcttaaaatcataatccagtgtgtggaccggaccggcataccactgttgtgaaacagcaggtaacacggtcgcaccgtcttctttggcggacgtggcagacagtccggtaattgtcgaatcaatatcggcagcacttgcactgtcagaaacagcggctgccgaagcaaacgtgcaaagaaagattgcaatgatacttagcagcttaaaatgcgccacaacaaaattatgcagcttatgaaatgaacaactcatcatatattccccctaaatatgaaattttccgattaagtcggtattgcaccgtcattacacattaataatgcctcgcaacccgcgtattcccagtacgttatcggcatatttccccttgtgtaactgcggtatagttaagtcgtaacgctagaatcctatcgtgacaaggtattttgagaaatgaaattaatttctcagtaaaatgtcacaatttttcgatatattcaattagttatgtatatcctcataattttattaagtgactaaaaaggaccaacttttctagtggaaagttggtcctttattacattttgtttattttactatattcatgtgtttaggattgacaacacaactcatgatctttcatgctgatcatttttcgagccactgtcatttttaacttgaaaagtcggcatcagatgtcccattcccagaccacttaaaatggtccatggaacataaaatgcaatctgatatcggctttgcacctccaccagcagaaaaataatggtcaatccaatcatgatggtgtcactcaataggacgccgttacgttcacgattaactttggagtcaatccgataagcaacaaattgcgccagcaacccaatgataaccagcaataacatgaccacttggtttccggtgaccagatttgtcaggccgttaatcatgtgacgtggcatcacttgaaattgatcagtctttttcctggtatttgagtaaaacaagacaggtccatagtccggcttcatcagggtttcgtttttgtcatagaagaaatgtttccaagtgccatgggctttgataccagcgacattagcctttaattgttttgaaaggaccttttcaaatccagcaaaccgctgttcatttgtgagcttctgattatgattatatttttcaagttttagaatcatgttgtaattgtaaacgccgccagtcttggggttggttcccgtcgccagcgtgtattgttcaccaattttggcatctgcaatcggcaccccaaaatagaagcgatcaattcttggctggagttgatttaaagcaaagaaccccaacatgacggcgaggatgccgattcgtggaacccaaaagtcagctctattttctttggtggtctgttcacttaacctgaaccacacaaagcaaacatacccaatgacaaaaaccatcgataatggtcgaatggattgagcgaaaaacaacaggacaataatcaatccgattgtgacccaaggatgccaatcctttaacgaccgatatgccaacaatttgatcagaaaatacatactcaagaacagtgcgagcaaccacgcaggttcagcaccaatcaatgttgtgtaaagataccaggttggcaggaaaaagaacgtcagagcggcaaacatcccgattgtccgattaaagaaatacgtgacaatcgctaaaatcaaaaaagtcgtcaatacactacaggcgatattgaatacctgaacgacctttggcgaattgatcgaaattctaaacagcacgttatacaaattggcaatgtgcaagacatgtggaaaaatactgtccaagtccaggacgccaacatgatacatccacgcccaagaatcctgattagcggcggacccacctaaagcattgtaactatacatatcagatattggattaagtttgaaggcaaataccagaatcagttttggaatcgccatgatgctgataaaagccacaaaccatccggtaaatctgccggcaaaccacttgccaatgtaccacaacaaaacggccgcaatcatactcacaataacactgacagtaagaccgttaacactaggtgtaaaggtcttatagcttgcccgaaaataaccagtgactgttccagccattagccaaacaacgcaaataactgccaaaatggtgatactgaaataagccgctttaatcagcttggactgtttgatcatcatcgttcccccaccccatcttctgttttgccaacaatttgatgatacaccaaaacaaaagcgcgggttgaagaatccaaattcgcccaggccaaattggaaaatcgggttacttatctaccgccgtgaaccgttcattatgatgagccggatgctcaatctcatcattaatcactttggccattgtgccggcagtaatttccgacttgccttcagcgttggtcagcagatcattttgaccaagttcgtaggccgttgcatccccaggtttaaaagtggcacttggcgaaaccgccacccaattgacattgctggtattggtgagcagctgatactctttgaactgctgacggggaatctcaatgaatgattcactattaggcagtttctccaacttttccacaaatcgatgaccatttccggtttccaaactgccggcccccaaaataaagaacagccgcggcttgtcagtgtccttggcaaattcgatcagtcgagcggccaaatcaacgtgtcggtatgcatggctcatgtcgtgcgtggcgtaggcgtctaccaagacgtccaaatcttggacatccacccgttgaatgtcaaaggcatctttgacaaccagcttgactgcgtctggcagcaggtcctttgccttctcagcgttgcgaacaaatcccgttacctcaaacccgcggttgactgcttcttgggtaatcgcactaccggccatgccagtggcaccgatgataccaacttttaatgtcatgttaaaacctccaatgattttgcttctttcgattgtttcgaattaattatcggccggctgagagagtcggtcaaccatttggacggtgaacattgaacataaaagaaccgggcattccaacgataggaatacccggttcattaagttaaacgatgaaatcaacacagattgatttcctgattattttgtcaattcaaccgccttaccggcgacatcaatcgtaatcggctcgccatcaattaacttgaagtgggaaccatcctgatcaacgtcgacttcaattaaacgatcacggaagacttgtctaaatgaatagtgtgaccatttcttcggcaggaatggtgcgtaatgcaacttgccgtcgcgaacccgcatcccagcgaatccttggaccaccgcaatccagccgccggtcatcgccgtaatgtgcaggccatcaacggtatcgttgttgtagttgtccagatcaagtcgtgctgttcgttcataaagttcaacggctttttcttcatagtgaaggtcagcagccaacacggagtaaatggcaggtgacaagcttgactcatgcacggtgtattgctcatagaaatcaaagttggatttcttctgttccggtgtaaagtcatcaatgaagtcccagataccctgcagtacatccccctgcttaatgtaaggggagcgcaaaatcttgtcccatgaccagttctggttcaatggtaattgatctgcaggaatttctgaaactggcttgaggtctttgtcgagaaagccgtcgtgttggacaaagatgttgagatccttgtcataaggcagatacatattgtcgacaatgtcttgccaatgtttcttctcatcttcactgacattcaattgtttagcttgttcaggagaaactcctttgagaatttccaaggtgtattttaacgtccattgagccaacagattggtataccagttgttgtcaacgttgttctcatactcgtcgggaccagtcacaccatgaatcatgtaattcttgtttcgctggctgtagtgaacccgatcggcccagaaacgggaaatttcggtcaagacttttgaaccttcgtttagaacatacgaagtgtcgccggtgtaacgggtgtaattgtaaatggcaaaagcaatatcgccatttcggtgaatttcctcaaaagtaatttcccattcattatgacactcgattccgtcaaaagtgaccattgggaacagggcacccttgagtccctgctgtttggcgttatggtacgcaccgtccaactgcttgtaacgatacatcaagaggttgcgggttaccttaggatcggtaattcccaggtagacaggcaccgcaaaggcctcggtatcccagtaggtagcaccaccgtacttctcaccagtgaagcctttagggccgatgttcaagcgtgaatcctcaccatagtaggtggagaagagttcgaacaagttgaaacggattccctgttgggcttcggtgtcaccatcaatgacgatgtcagatttgttccagcgatcagcccagacctgctcatgagcagccagcagttcatcgtatgattggccggcaacctgatcacttaattgatgcatggcatcagtcaaagcggcttgagtgtcgtaatcccgtgaggtcacaacgatcacgcgcttttcaagttgagcggattcgttgggagccaagacaccggagaattcgttggtcacttctttttcactgggttgggccactttttcagcagacaagtcagtgacattgcgcatttccattcctgaagtgaaccgcggcgtcccaaatggattaggggtcgtttcagctaagacgttaccggaatcagttccctgctcagttgagagaacttcccagaaacgttcgtcgtagttggcatcctcgttcttaacgtcgccgtcgattgctgaatcaatcacgaggtccactttacttgaaccaacgttttggacagtcacccgctgaacggacagttcctgctgggcaacgctcaagaaacgttcaaatttgacagctactttggcatcacccttcgtaaccgtaaatgagcgggttaacaaagcctttttcatatcgagattgagttcgaaatcgctgaactggtctttcgccaggtcaatgacctcaccattaatcttaacgtgcattttaatgaaattaacggcgttgacaactttgccgaagtaatcaggataaccgttcttccaccagccaacccgggtcttgtccggataccagacaccaccgaggtaaatcccgttgagagtgtcaccgctgtaatcttcttcgaagaagccacgcatccccatgtatccattccccaagctggtcatggattcctggagtcgtttgtcttccgggtcaaagtcgtgggtcacaatattccaaggagcgacttcaaaagttcttttcataagttaacgtcctttctaagctttgtaagtttctttaatgaatccaactgaggctgcaccgagagccatgatgatcccggctaacaggaacatgttaggctgtgcgttacccaataatgggaacaagccaaagctggcgagtgaggcaacgatttgtggcaggcagattgaaccgttgaacaggccaaggtaagtccccatatgttcaccagacaaggcgttggtaaccatagttaatgggtaggtgttcatcgatgcccaagccattccaactaagatgaatgacagaatcaaaatgtattgagtgtgaatgaagaatacggagataaatccaactgcaccaagggccaaactgattgagtagcccaacttgtggtgattgtttggcattttagccaagacatacgaccagataaccgcagcgattgattgaacggcagctaagacaccgtaccagttaccggcagcttgatagcctgctgaagcggcattggtagtgttccaaacgttgctggcaatcgcaccggctgagtaggtccagagatattgaaaggcaatccagcagaagaattgaactaaggtaacggtccaaaagactttaggggcctttttcagcaatgaccaccagttaccaccggttgtgttggcttcttcagtaattccgtgatatttggcgtaagtcttaggatcatattcatgaaccttgaaaatcgtcagcaaacttgtcagtaacagaattgcggcaccaacatagaaggaaatgacaactgattgtggaacgacacccttttcagctgtgttggcaacaccaaatgcggtaaagatgaacggaaaaatagctgcgatcaccgcaccaccgtttgacaagaaactttgaatcccgtatgcgtaactcttttggtcatcattgaccatatcgccgaccatcatcttgaatggctgcatggcgatgttagacgaaacatccaacagggcaacggttactgccccgaataccagggccgtaatcgatgcgtacccgaaaccaaaactccccgagttaggcagcagacacatgacgatgatggcaattaacgttcccagagccaggtaaggcaggcggcggccgccaagcttaggtgcccaggttcgatctgaataataaccaataatcggttgaacgattaaaccggcaagcggcggcaaaataaagaaccaacccaacttgttgggatctgccccaatcgtttggaagatccggctcatctgtgagctctgcagggtaaaggcaatctgcacacccaagaagccaaagttaatcatccaaatggtactggcaggaagtttgggcaaaccagacttcttggttgccgctgcgctactttgttcatccatttcatattcctccaattcaaaatatcgtattaataatagcgtttacattttgtattattgcacgttttaatcaatgttgcaaacggttgcatgaaattaattgagcatttttaaaatcggatcggcgaaaatagactggtaccggttactttggcgagatgtcaatctcataaaaatttcttgtggcattttgatacctactacttttagatttgtatttatgagagaaaaaaagttttttgacttttttcactgatatataacggctgtggtctagacctcatgtgtaatatgaaaataagacgtgtaaaactgtgctaacctttcattgcacttcaatcaaaaatgttttatattgaacaagcattcacaagtaacttgatggacacaatttcataaggtggtgagatttacatgttgttaggtagtgttgaagccggtggtacaaagtttgtatgtgctgttggtaacgaagattatcgcatcttggatcggacacaatttccaacgactacgccaaaagagaccttgcaaaagactgttgattatttcaagcagttcaaggatctcaaggcaatctcaatttcttcctttggaccaattgagctccgtaagaactcgcctaagtatgggtacattacaaataccccgaaaaaaggctgggccaatacggattttgtaggtcgaattaaagaagattttgatatcccgattagttggacaaccgatgttaacgggtccgcttatggcgaatacgtcatggcaacgctgttcaacgaaaagatcaattcgctggtctattacacgattggtaccggggttggtgctggtgcaattatcaacggtaacttcgttagcgacatcggacatcctgaaatgggacatgttcgattgaaacgtcatccagacgacctgaatttcaaggggatctgtccttaccatggcgattgtttggaaggcttggtttccggaccaacgttcgaaccaagaaccggtaagaaaggccaagatgttccactttcagaccacacatgggatatcatggcattctacgtagcccaagccgcaattcaagtcactttgatgatgcgtccagccaagattgtctttggcggtggcgttgtcagcgaagaattcttgaagaaggttcgcgagcagtttaatgagttgatgaataactacgttgacgttggcgatctcgataaatacatcgtgatgccattggtcaaggataatggttcagcaaccgtcggggattttgctttagctttgaaagaatacaacaagtaacaacttatttttttgggaagttccacaaacgtttgcggaacgaatgaattttaaaaggagattttttatattatgaaagcactcgtatttactggaaaacaacacatggaaattcaagacattgacaagccagaagtaaagcctaacgaagttcgtgttgacactgcttatgctggtgtttgtggaaccgaccacgccctttataacggccttccaggttcagcagatgctgttcctccaatcgtctttggtcatgaaaactcaggtgtcatttcagaagttggctcagatgttgacggcttcaaagttggcgatcgagtaactgttgaccctaacatctattgtggcaaatgtttctactgccacactggtcgtccagaactttgtgacaacctctcagccgttggtgtaactcgtaatggtggccttgaagaatcctttactgctcctgccacaaacgtttaccctattcctgataacgtttcattgaaagatgcagccgttatcgaacccatctcatgtgccgttcatggtatcgacttgcttaagttaacaccataccaaaaagctttggttatcggtgatggcttcatgggtcaattattcgctcaaattcttcagtcttatggtgtccaccaagttgacttggccggaattatcgacgaaaaattggatttgaaccgtgaaaaattaggtgttaccaacacttacaacaccactcgtgaccagattccttcagattacgacgttgttattgaagccgttggattaccacaaactcaacaacaagctgttaaagctactcgtaagggtgctcaagtattgatgtttggtgttggtaagccagatgctcatttcgaaatgaacacttacgaaatttaccaaaagcaattaactgttcaaggttcattcatcaaccctaacgcattcgaagactcaatcgcccttctccaaagcggtgacttgaacgttgatgccatcatcagcaacgtcttcgacttggacgaagttgaaccattcttgcaaggaaagactaaaggcgtttcaaaggcagttgttaaagtaggtgactagtttgaaaaataatgaggaaaccgccagccaagttctaaatggccggacgatctcgatgtctaaatccattacgtttttcatcatttctttggtgattaactccgccggaaacgtgcttaccttggttaccagcgcccaaatccacccttcctacttgggatcggcttattggaccgccgctgaagccaacctggcagttgcgtttggctggaatctattttggacattcttaattcttggggtcgtgatcacaattttaaatgccatcctggttggacactgggattggcggcgcgcacttggaaatctgatcttcatggttcccttctcagcgttgattcaagtattcgaagacttcttccttggtaagtacccggcattgtttggtggttttccaccagccaagacgccattcatgattggattttatatcctcttgaacttcttgggtgtcgcaatgatcggaactgccatctccatttatcagcgggtcaacctggtactgcaccccgccgatgacttgatgcagattctgcgtttcaagtatttcaaaggaaatgccaacacagcgatgtgggcatcatacattccaccaacactgatggcaatcttggccttcgcaatcactcgtcaattcaccaacttgggaatcggaaccatctttgcgttcttattccaaggcggaattaccgggatcgcggatactaaggtcttccctcacctgaagcatcaagctttggacgtgggaaaagattagagcgcgacgaggcccgggagatgcggtttctaagggtcctttgattaaagtccctgactttgggactttaattaaagggcacttagaagttagcatctgggccgtcgccaagtaggctaggcagggcttcacccggccgtcggagcgtatttcggaagccgaaggaatctcaaaatcggctaacaaacatttgcccaaggtgctttattaaaaatcaaccctggtttttactggaagttccttgggcttgggtttcctcgtaaatgaacgcggttacacaattaatatgaaagaggcaattaaatatggcaattaaagatgatattacaggaattcaacacgttggaattccatccgttgatttggacaaaacaatcgcattttatgaatcacttggctttgaacaagccggcttattccataacggtgagaaccgctgcgcattcatgcgttttggcaacttaaccattgaaacttgggaaggcgatccaactgctcgtaaagctggtgcaatcaaccatatttcactgaatacaccagatgttgaaaaagctttcgctgatgccaaagctcagggattacgcatggtgaatgatgaaattcaatccattccttcattctgggataagggaattaaattcttcaacatccttggccctaacgaagaaacaatcgagttctgccaaatcctgtaggacagagtgtgacgagcaacgggtgatgcggtgtgtaagaccgaaaagatttaaatcctggtcttggatttaaagctttttggtcttacacgttagcattagttgcgtcggaacacgtttcagctagataacagtggttaacaaacggggctggggcaaatgctttttgtcctagccccatttgtgttttataattaaatcattgaatgattccaagaagggaagtactaataatatggctcatatttcttttgatggctcaaaattatcaaagttcgttcacgacaacgaactcggtgaaatgcaggcattagtgaatgctgcggacaatgaattacgcaaaggcactggtgccggcagcgatttccgtgactggctgactctgccaaaggattacgacaaagaagaatttgcccgcatccaggcagctgctaaaaagattcagtcagactccaaagtcttggttgtcatcgggatcggtggttcatacctcggtgccaagatggccgttgacttcttgaatgatactttcttcaattatttgccagatgaccagcgcaaattcccacaagtgatgtttgcaggtaactcattgagctcctcatacgtttatgatctgattaacttgatcggcgaccgtgacttctcagtgaacgtcatctctaaatcaggtacgaccactgaaccttcaattgcatttcgaatcttcaaggaacgtctcatcgccaaatatggtgaagaaggcgctaaagaacggatctacgctacaactgacaaagctcacggtgctttacgcaaagaagctgacgccagtggttatgaaacctttatcatccccgatggtatcggcggccgttactcagtcttgagcccagttggcctgctgccaatcgctgtttccggtgctgacattgaacagttgatgaaaggtgccgcagatgctgccgatgaatacagcgatcctgatttgaccaagaacgaggcttaccagtacgctgcctaccgaaacatcttgtaccgaaaaggcttcaccactgaattattggaaaactacgaaccaaacatgacctacttcgccgaatggtggaagcaattgatgggtgagtccgaaggtaaagaccaaaagggaatttacccatcatctgccaacttcacaaccgacctgcattccctaggtcaatacatccaagaaggcttgcgaaacctcatggaaacggttatcaagttggataagccaaaccacgacgttgacatccctaaagaaaaagacaacttggatggcttaggctatcttgaaggccgcacgatggactatgccaacaccgaagccttccatgcggtagtcctcgcccacacagatggtaacgtgccgaacatggccgttcacatcccggacgaaacaccatacacattgggatatttgatctacttcttcgaggttgcggttgccatttccggttacttaaacggtatcaacccattcaatcaaccaggtgttgaagcatacaagcagaatatgtttgcattacttggcaaacctgggtttgaagaaaagggtaaggaacttaagaagcgcatctaactttcaaaagtccaaaaaatagcagtcctcgacggtaatcgtccaggactgctatttaattacaacaaacaatgtacaactaaattaagtgcacatcatcctcacacgatacgaaacagttgctttgatgttgccacaactaatggtatcgtcatttattccaacgaaaacttgtgtttatcaaacggtgtaattttcacaacagtagataaacacttaacggacaagaatacacctctttcgacaacaacattactgattggagcctcaaaattggccgcactaacaaaatgctgattatccttttcagtcattattatcgcttcctttaatttgaattagttttgttctaattcatttttaatataatgtcaagctttttcttaattttgtattaacctcatcgctttttaatgttatagttattccaataaaaaaagaggatgatacttatggaaaaaacaaaaggtatttcaagacaactaataacggcaggatggacgtctttttttccgaaatcggttcatccacgtttatgttttctgtaagtttgcttttattacatacataccacaatgcaggagtatttaccttggttcaacttttagagccaggcatcattctgttgttcaatccctttattggagtttacgttgatcagcacaaaaagaaaaatattgcattaacaagccagttgggattagttattactttcgtcattctttccgcttggattaataaagcaataaagtcacctctgtttcttgtgtatttaaccatatgcctttttattattctcatatctactcaatcacgaaaagtaagttatcaggcagcagttatctctatgatgcccagaggctcagtaaataaaatggtgtcagtccaacaaacctgtaccctctcagcaacattgattgctccatttattggctcactgttatattcaactctcggttttaaatcctcagtattttttgagggagttacagaaattatcgtcttacttggaatatttttgataaagtttgagctttatgcaaccggtaatcacactttccaaggtacacaaaaaaacatactttctcaactagcctcagggctaacaataatcaaagttcaccggaacttgttattagtagtactactaagctcttttataaacttcttcttcgcagcgataaatatagggttgcccatcaccgtgattgaatctaaaaatatggggtcattctcacttgctgttattgaggttgggttatcaatcgggatgttgagtggtggaattacttcagggttcatgaaaagtgtgaatataaccgttattggctttcgcttagctataattggaatacttgttgttgccatgggcgtatttttccttagtaatgttcttataattatcttaattggaataactaccctttgtttttttgttggtttattgatagtacgtataaatattcctatgagtagttatgtgaaggaatctgttccgctagactatcagggaagagtaaattcaaccgttgacgctttgtcatccttaatgtccccctttggaattatcacgtttggattcctttttgctcatacatggaatcccactatttatctgctaagtggcttattcatattattcataagcataggattttcacacaaaatatcaaaaggagactagtaaccatggaatataaaaatatgtataatttaatttcgaggataaagtgaacccttaaaattggacaactttattaagctgctttctggacggtaagttcccggtattttaccggggacttgccgtccagttttgttttgatgcgccgatgattgtagaagtctatccattcgttcatagcttcgataagcgctgttttggtctcaaaatgttcatccataacctcgactttcataatgtgaaaaaacgactccatggcggcgttgtcgagacaagtggctttacgcgacatactctgaaatacatggtgctctttaagcgtgtcttgccagtggcgatgctgatactgaaacccttggtcagtatggacggttgtccgataatctaacaccggtattcgatttagggcttctttcaaaggttttaaagcaaattcaacggtcgggtggtcactgatattgaaagccagaacctctccattgaagaggtcgaggactggttctaaataaacccgttcattttgactttggttcccatatcggaattcactgacgtcggtgactaacttctggtaaggccgatctgttttgaatcgtcgcttaagtcgatttggggcgatgacgccaacagttcccttgtaagaattatactttcgtttctgccgattaaaggcgccacatagccagtcttgttcccgcataatccgtaagacccgcttatgattgattttaaagccataagcgtcatgtaaagcaccggttattcgtcggtacccgtatttccgagtatattttggatcttgttgacgaatctcatcaattgcctgaataatttgtgaatcatctaagttacgaccacgatgctccttagcataataatacgtgctacggggaatacgaacagccttaagaactagtttgatggaaacttgaaaattctgccttaactcgtctactagttcgatgagttcgtgtgttttgacttctttcgtgctaaggcatcgagtttttttaagaattcattttctatttttaacatttgattctcttgttttagctgcttcaattctgcggctggagtctgtggtttttcaggtttggggttgttctgcttgtgtttgaccatggtcttaggattccctcgtttgcgctcaagtcccgctattccagattcctggaagtgtttttcccactgccaaatcgtacttggcgacgacaagtcaaagtgtaaggcagtcactggaagcgaagcttgatttcgtttcttccagtttaatacatcgactttgaactgactagaatattcttgggacattgaccggtcttttagaccttcaatacctcgccgctcaaatcgatgaacccagtccagaatgattgaatgattgctaatgcgatacttcttagctagagacggtgaacctttaccagataagtattcagtaacgacctttattcgaagttctaaattaaattttgacatagtaaaacccccaaggttagatttggtgtccaaccttaggggttcactttaggaacatggatttctttaatgtattagatgttccagtcaactcaacaatgaatgtagagctaaaagcatatatggaacttataatcacagacattttcagtaaaaacaatctacgaaagcatttgcacgggttttcctcccttgttgcaaagctaaatcattatttctttgttccagatgtctgtgcgagatttccacaactttgtgagggagcactgctcagcctatctatctccaatacctcttcgtctaattcgttctttttgtcgaaggttgaagaggatttagaaccatggaaccccattcttttacaattgcaacactttgcaatcttagaatatgttaaaaatgatggtagcgaaattcaacatatttcaaaattaatttgtaaaagctcacttggtctccacacgccacttgaaataagcgattataacgatatctatagtgcaacccatgcggtaatctctggatcaatttatggtaggcgattattatgtaatctatttccaacgagaacaacctatgattactttaaatatttccaacatgcattctttttttcgctcttggatcatcattacgacttagcagtagaaacactgattgccagttgtctactgtttgaattgagtattagcgaccgaaaaactattgagaatgagatcgattatattgatacaaacatttttcaaaaccaaagaataaatcacataacgaggacaaattttaaggactattaccacctattacttgtacgtataatattagaggaagtgagataatgattgctgatcttcaatctgaaattaaggataaattggataaagattacaacttttgggaatatttaaacttaacttactctatttcgattggggtattaattaagcattttgtcaatcaacctgtaaatacggaagaatacttaattctaaccaagttctgcaaattgttctacaacagtggccttatccaacggcttcccaaatgctttctcaaagcaaataccatattcgcagtttatagcataataaattccgactttacgtacacttatccaatgaattcagaaagctttgttcttaatcgagtagaactggacgaactgcaacaacttcagtacagccttctgcaaactctaaatgaaaagccatgtgtttttgttgatccagtatcaatttatcatgagcacattatttcttgcaaggatgcctcgtcactcggtatagaatcatttgtaattagcctaattaattcacttttgaagataaaagttagtaacggtagactggatggaagagttgaaactgttggaatgtttgcattattatcaaaaaaataccggtttttcttttacctatcatttctgaatcgaaaccttgaaagtatcgcacaatcgaccaacttagattattctactctggacgtagttagcctaatatcattaaacactttgataaacaaatagaggtgaacccttttgaaacaacaaaaatcattgataccattgaatcaaatcatatcaacaatgagcagtcaggacaaactatactcaacactagtatcacttctcaaaaggactaatcaaattcctataaaatcgaagaacaataagatagcgtttgattgggaaaaatttatttcattctccccaaagcttcgtcttcaaaccctggtaaatgttataaataatcaagtggtttatggaagacggttagatagaaaaaattacaatttctttattggctttttaatatttagcattcagcagtatgatattaaggccatcactaccagttcgataatgctgctaacacaaagtgactctgtagaattgaaaaatacaattacacgatttgttaaggcccagcaacgggaaaacggatatttcggatatctgaatccattattatcggaaataaatcgtgagtccgtcaccgaatttgtaaatactacaactgcttacttaatgttgcttaacagttatttaaaaaagtagtttcacaactacatgatgaggtgaactgaaatgaattacactttcagttttttttactagtgtaaatgttattcacgccaattaccagaaggggtaaatagagatgccgataataccgttgagaatcggtagtggccaccagttatctttaaacatttcctgatatcctttggttattaactgctgaattgaatgcaaaacacacatttttgaagtatgaaatcaatcctcccaatctacagaatctcatgtccaacaatgatgtgatcaattacctgctcatcctctgctggtttatccagtaatagcttaactgccgactgccccatttcatctggatgaatatcaacagaatggaaatgctgatcggtgagttcacttggtagtgaattgttgtaaccaagaacttcaacgtttttattaggattaatcattttgaaacggtggtacatttgcaggccactgtaatcatcaatggcgacgattccatccatctgcggattgtcgcgaatgaactgatcttctaattcatcattctcttgagttgacagcacgacaggcgatttgccggcctgcttcatcgctgccaggtaacccttgcgccgatcaatttcatacggccaaccgttatgggtttggacaaaaattggattctggcactgatagtgatcaattaagtagttggtgccgtcaaatccggcctggacgttatcgttatcgacatacagccaatcttgtccggccgccggtttaccaattgtcacaaaatcaacgttttctttttgcagcatttcgatgactgggtcattttggtgggagtatagcaggataaaatgtttgatttgggcgcgggtaatcattgatttaacattctcgattacctgttcagtactgtctccaatcgcgattgataggacgtaattgcggctgttgagctgcgcgttaatcccccgcaaaataccaacgtaaaaaatattgtcgacaacccggttattaactgggaagacgacgccgacggtattggcttcacgattggtcagattcttagcgttatagttgggctgataccccatcaaatccgccgttttcttgacgctgcggcgagtcttgagactgatgcgtttattatcattgagtgcccgtgacacggtggaaaccgataagcccagccgtctggcaatgtctcggattgtaaccatttgaattgcctcccctctactaaattttaccctttttgaagttgcgatcttgttaaacttttgtatcaattattaatattgaacgctactactagattttgacagtattatgtgataatttcaacgtatgaggtgattatggaaatgaaaaagcacagatcattagctgccatcttggcggttgttgcaagctttgcactaattttggctggctgcagcagttcttcaaataagagttccaacaacaattctaataaggccagcatgcaaaacgagactcaagataaatccgctaagcaactgttaacatcaagcgataatctttggtacatgaatggttcgattaattacaacagtaaatcaggcatcgatgcctacaaattcaattctaagaaccataccgtgaccatttacagtgtcaacaagatgtacaagacctacagtgaagctaagcaggcaaatgatctggacaaacagggaactttgaagtacaccttcaagaatgactcggctgacaaaccggtgatttacatgaagggtaaactttcggatatcccaatgcatcagacaatttcagtgaaaaataccgttagcggcaagaaccaccagtctaagctggcagtgaccggctataaggtcgttcgaaacctggataacgatccggctccccaagtttgggtaacgcccaaagactaattaattttaccagaagagacaatggcagaatcacttttgccgttgtttttttgtatcctgcgtaagcctcaaaaggagcgcgttaccagcccacgggccttatttcgctgttaaacagtcagttatggtaggataaaaccattcaacttgatcaaagaaggtattcgaacatgaagggcaacaaactattacagcggtcaatcagaacgttttttcagaattggggggcttacgtcagtttagttattgtgattaatctactgttgggcatcgttgttgtgccaatcatgcagtatatgactggcctgattctccaagtgaaccggatcccctacttatcgtatacaaatgcggtctggcttttgacccaacgaccactggcggtggtggaactgttcattttgctgctggttatctttgcgatggtcttttggcagttcgcgtttctgctctctgggattaacaacatcgccctcaaacaaaatttgagtctctggggagtttttaaaattgccatccatgacatgcgtggattgcgactgggcagcttcctgttctttattggctattttattttagttctgccattttcagttgcctacctgaactcaccactgctttcaaaagcgaccatccccgtctttatcttggacgatttggaaaagaatccgttgattgcaatcctgctcacagtcctgggcgttgccgtcttttacttgggaattcgactgatccaagtcctgccgatgatgattattcaccatcaaaagggcctggaagccgccaagaacagctggcagttgaccagccacaatacctggcagtatctctggcggatcttcgtactgggaatcatcagcttcgcgtcaacgaccttggtatcgtatttactttaccttttccagacttacctggatgcccagtcaaaagtgattagctttgttggtgcggtcaccaacatgggcctgttgaccgtctggcaacgaattgtcgcctcgtttagtgtggttgtcttcatgctcatcttgttaatggtcttggatgagtccaaatggcattcaacggcggctgtggtccgtttaccccgaaagcgacggattggtcggcgggtcatgggagcccttctgattggcctgtttttggtcggagacgtggcctttaatgctgtctatcttcaaggagcactgctgaccaaacccatcacgatttcccaccgtggggtagatgacggtaacggtgttcaaaatacaattccggcgttgaacaaaaccagcaaagaaaagcctgattacgttgaaatggacctccacgaaacccgcgatcatcaatttgtggtcatgcacgatgaaaatctgtggaacctggccggggtgaataaagatccttatcaattgaccctctcccaaatgaccaagatgaaagttcatgagaacggccacacggcccacattgccagctttaatcagtatctgcgggctgctgaacatgatcaccaaaagctattggttgaaattaaaactactcgtcacgatagtcaaaacatgctgcagctatttattaaacgttacgaaaaccgcctgctgcgggatcacgatcggatccattcactggattatcatgtgatcagcggcttaaagaagcaggctcctaaattatttgtcagctatattttgccgtacaacttctcgttcccccaaaccaaggccaatgcttacaccatggaagaaaccacgttgaacgaaacgtttgtcaacgaggcgcatttccaccaccaacaagtgtatgcctggacggtcgatgacgaagacgacatgacccgaatgctattcttgaacgttgacgggattattactgacaacttaactgagcttcaatcaaccatcaattctacgtttgatcatccaagttatgctcagcggttgttgatttattcgaatgaattgcaggatgaagaaaattagttatccaagacatcaaaaagggaatcccagctgggattccctttttgataacctaatattcttctaaatcaatttaggcaacgtctaatttgcatcaagccattcagcttcaaccctacgccaaggagtcccacgccggcagctccactggtgcttgcttcaatagggccttttgatcatctgaaaggtattttttgtggaccacgacttcgtagacgtagtcgtccatccaatcgtcactcatggtgaagtagcccttctcaccattcttgtcaccccaggaattttcaactttccatttagtgggcgtctcaccatcaaggtcaaccccagtgaaagtcatcgcgtgcgacacttcggcttgatgatattgcagccgggctgccttgtccatctccaagtcgacatcgaacagtttcgtgtagcgatacaagtgactgtccagatagcctttcttgcggtccatttgttcaagcacatcgttgccaaaccagaccgtttcgccatccttgagttgggcaatggtagcggcctttaaaacgtccatcggcagatttaagaaggcaatctgcttgccgccgacaacgttattttgacttggcagtgaatataattggttgtaatctttttccggggaattagctaacaccacataatcatccaaatcgacaccgaagtattgatcatagaattgttgagggggtagaccggagacccgatgatactttttgtcatcgtcgcgataggcaaaatcaacggttgccggtggttcaccgaatgaataggccgtgattcggtagacttcactcagcatttgtttgcgagcgacactgatcgcctcatcgctcttttcatccttgaccatcgaccgcagtttggcagcgtcaatccgcagtttgcggttcataaccgtatcaaaagcaccggtattctcaacgttcgccgtttccggaaaatcactgaccggcatcacaccatatttttggaccaatgccgctgccatcgcccattggccgccatcgtcgccagggaagctcaaataattttcaacttcccggtcattagccggccgactggcggtcgctaaaattcggtcatagaagatgttggcgcgctcaattttatcccagaagaacaggtatttttgtgaaaggttgaaatccttcaccttatacttagcagcaaactgatgccgtaaagtgttcaccaatgaaaacagccagcagcgaccactttgcttctggttggtcaccgaaccggtctggaggtccactgaaaatactggattcaatcgcacttgggcatccggatcctgagctgcttggttgatgccgttttgttcgattatcttcgacagcacatcactcttaggtgcattcttgaaatcattgtggagtgctgaaaaatcttgctccgttaaaacactattcttatcagtcattcagacatccctcctatgtaattgtgtcatattgtaaatcttttcttggttggtcgcaatgtggcatctgttgcttatgcttacttgttcaacagaaatctattagatgtgctgattactgccgcagagtcgcaggccgccggctctgcctgctgtagtggcttggatttcgagcctgtagtctcgaaataccaagatgctgtaatcgcgactttcagtcgcttcaacagcatggacactactgctggcaatgccggcggcctgcgactcggctattttgaggatgaactttaaccgggcgaatttggtagctcaaacactgtttacccgcaacggcatcactgaattactacaatttcggcaagacaaaattcaaattctcttttccaacgccacttaaagctgtaaaacaaaaaagtctacaggataatctgcagacccaaatgacgattacctcatactagatgcgcttcttaagccgtggcgttaccaaataagcaattaaggcaccgactgctccttgaatcaagttggtgccaatcccaatatagccggcataaatgttatacagaaacgagtctgccacaaaatagccgattaccataatgacgatcccgactgaaacggcgatcagcttggtccacttgcgatcagtatttttaccagcgatcaagccgacaatcaagccttctgcgccgtggacaatcagtgaaaaccacatatattgaccataaccggagatcaggtccaacaagaaaccactggcaccaccgacaactccgccgactctcggtcccagcaacagcgcgctgataaagattccagcgtcacacagattgatattgccatgggtcattggaattgggatgataaaaaagcggctgatcgcaaccgtgacggcgataaacatcgccgttaaaacaaccttgaaaatatcactgctgaccttgccgcctacacttttacgatccattactgacttcctcccaatacataatcttctttatttgcttcagtaaaatcatacttggcccgacttccgccaatcaattttggccgtgaagaaaggcagaccacattcgccgcaccgacacggcgattggtcatgcggactggaatctgaacgtatttaacgtgcatcccaatctcggttcccccgatgtcgataccgccaaatgccgtgatgtgctccacttcaactgggtcatccattcgttcataagcagcgacttgcgtaccgccaccggcatgcattgccggaaccacggaaacaatttctaaattattgcgctcggcaaccttccgttcaaccaagagggcccggttgatgtgctcacagccctgaatggcaacatgaatattgcgtggaattaaaaattcttccaaagtcgacacaacggctcgaccaacgtccaatctggaattagtccccttccagtcaccagaaatttcactggtactgcagccaaccacaaaaatgccattttccgggaatgtcacccgctcaaaatattcagttaagacagccgacaaatcacgcttgattgtttgtaaatccatcttttacacttcttcccctgtttgtcctaacgtaaacttcgccacattgtacaatgacctggtcaaattcaacccaaatttccgttggtgctgtggtgcgcggctggtcagactcaccgcatcgtacaccccaataactgccttttgaaccgctgtatcaaaatccagcttaaagttcaaatacccaattaacagtgctgaaaatagatcaccggtgccataaaaatgaccgccgattaaaggcgagccggcccatttgagttggtcgccgttgacatagacacagccaatcccaccgtcacggtggactccggtgataattaccttggctttggagtgggtcgcttcacgataatcggtaacagcttgatgaattcggtcatcactggcattaactcggaggcgttctccactgagcagccccaattcggtaatgtttggggtaataatcgtggcaattgatgcgagtcgcttaatggcatccaagtagccaggttcaaagccggcatacattttaccctgatcacccaaaaccggatcaatcagcaggtcaggcaggctaactcccgagagatagtcgtacaaaaggttagccgtactaatcttaccaacgtaaccaacgattcctgaattaaattgaagatcatccaacccattccagtgaccagttgcccgcctgataaaagaatcagtattctgagtagtaggcgttccaaaaccttctgtttgagtcgaaagcagttctgtcggcaaggttgccgtttgcagtccaaacgctgaaaatacggcgatggcggcagtagccgaaagcctgccgaccgcggaaaaatcttctgcaattaatacactcggcttgataatgatcatccttccaatcatgtttgttacaaatattgtaccccattgccaatctaaaagttaataccttacacattaaatgtaacattctctcatcaaaagtattttaagtataccaagaatcccagaagaaacaatagacagtttgctgttaatgtcagtgactctggtatagtagagctgtaaatagtttggaatatagaaaagagtgatcaccatgaactttgccactaaaaccggcatcacaaccctggcgcaaacttttatcatgggctcaattgatgcctacacctttcaaaattttgacggttcatttgtgagtgcgcaaaccggaaacctggttgttttcgcttacgaactcgccaccaagggttggagtacggcttacattcgcgtaccggtattactaggattcctactcggagcattcatctcacaagcctttaaacacattcaactggcaagcgaccgccggttcaacgtcctcttgctgttcagtatcatcctattgggaattctggcagtggcggcagcattccacctggcgatgctcaacatgttattcagcctcggcctcttctcaggttatgaactgaccgtgttcaacaagattggcacgaccagtgtgaacaacggcatcatgactgggaatttgaaaaattttgcaaataattcctatgaagccatctttagccacgatcgtgaagctttgctcaaagccggccgctttttgagtgggattatcatgtttattctcggcattatcttcagtgcctacctgcttcatgctgccgggccaaaagtctttgtggccgccttgatgatcaatctggttttgttgatcatcccactatttggttggcgaaatcgtcaacgggatgaaacaataagttgacattcacttatatttgagttagattaaaaagcaattagaaaacttacgaattatcaagctatgaggagaagagtaaccactcagatcgatttcagaaagcctggcagatgagagcaggtatcgaaatgacggtgaagatgagctccaaagggcattaagccgttcacgcggattaatcggtaggaaccgttaacttcccgggtatcataggtaccgttgaggcgttgtttgcaaaggcaacgtgaataagggtggtaacacgagcattcgtcccttgattgtcaatttgacagtcaggggacgagtgctttttttcgtaagtaaaacttttacaattacaggaggattttcacatgacaaatacagcaattacaactaaatttccatatcggtacgacgttgtcggcagtttattaagaacacaggcgttaaaagacgcccacgccaagtatcatgccggccaaatcagtacagctgacctacaaaaagttcaacacgctgaaacaaagaagattgttgataaacaagttgagcttggcctcaaagacattaccgacggtgaatttaaccgcagctggtggcacctggactttctttggggattaaccggtgtccaaaaatacgactatcacaagagttacaagttccacggcagtaagacgcggactgataacgctgaattggccggcaaagtcgccttcaacccaaaccatcccttctttgacagcttcaagttccttcaatcaattaccccggatagtgtgacccccaagcaaaccatcccgtcgccaacgatgcttttccgcgacaatcgcagtgataattggtcaaagttctatgatacctgggatcaatatttgactgatgtcgccaaggcctaccatgaaacgattttgcacttctatgaactcggtgcccgctacgttcaattagatgacaccacttgggcatttctaatcagcaagttaaacgaaaccgttcacgacgcggatgcccatgcgaaatacgtcaaattagccgaagattctgtcaaagtcattaaccagctgctgactggtttgccgaacgacttgaccgtgacgactcacatttgtcgtggcaactttaaatccaccttcctattttccggcggttatgacgatgtagcagagtatctgggtcaactcaattacgatggcttgttcctggaatacgacagtgagcgagctggtgacttctcaccacttggcaagatttggaatggcgataaaaacaaacgaattgtccttggcttgatcacttccaaatcacctgaattagaagacaaagacgcggtcatcaaccggattcatcaagccagcggccaggtcccactggaaaacttggcgctctcgacgcaatgtggctttgcctcaactgaagagggtaacaagctcaccgaacagcagcaatgggacaaacttaaactggtcagagatatcgtccgagaagtttgggatgtcgactagctgttagccaatcgaaaagaggcgtcgttatggataaaagcagggaaaaatactcgcaagcaactgatcgccagcaaactcactggctgggattggccattggtttggttggtggtctcattatcgatgcactatttaattttcggaccgggacgtttttcacttttattggaattgttctgggaatgagcgggttgctggattttaaacagcgttaatcgtttcaaaccgtctgccaggtgccatctaactggcagatttttatgagttgcctcaggaacgaaaaacaggtacgcttttattaaaagtttctcataattatgtaaaggaatgatgaacatgctcgcctggatcagcctgcaacacagcatcgtagagaccgttgcacttcagtgatgaatgacacttggcacatccccaaacggacaggtttcaaataaaccgtttggctgtgcttatcttaactggagtgcatctaatgacaattaaatatccaagtactattttcaaaggctacgcgtacactttcttttcctttttcgggatcacttcactttgggtgatttacctgcagatgcaggggctaaatctagtagaaatcggtttatgtgaaagcatcttccacgttgccagttttgttttcgaagtgccatcgggcgtattggccgatcgcttttcctatcgtttctcacttttctggggccgaattgcctcaatcgtttccgccatcctcatactggtagcccacagtttctggctgtttgccctgagcttcgtgctgagtgcgctgtcgtataatctccaatcagggacaatcgacgcgctcatgtacgattcattggtggcccctcaacaaaccaaacgattccccaatgttatcagcaatctcaacgtggtgattgagttttcgcagacggcaggtgtcgtgattgccggatttttggtccactggcatttcgaattgacctacgtcgcggcaattctgatcggtattttcggcctgataaccgttttattaatgaaggaaccgactgtccccaagtcaattgatctgccaaaacagacagtcaaatcaatcatcgtcatggcctatcggacgttgaaaaataaccaacaactccgcggtttgatgattttccaagcggtctttgatgggatttgtaccagctattacttctatttccaatccttaatggaaacgcaccatttctctggcttcatgatctccttgttgatggtgatttctgctggaatgaacatcgtcggcatcaaattgaccccgtggattcagaaacgcttggcaaagccggcgttggtaagtggcgtaagtgcaacgttggtcgggctactgctgctcacatggattaactggattccaacgttaaccgtcctgtttttgttttcccaactactggcgtcattaattgagccgatcttcagcagctactacaatgaaatgattacttcacaacagcgggcaactttactgagtgttgccagcgttctgttttcagcttcaatgatctttttattcccactaatgggctggctggttcagattcaaacattctcgtttggctttggcgtgattggctgcttgatgttggtattactattgttaagtcaaaaatattttaaaaaagcaaaatgaaaaaagtttgaggctccactggtatcttgtttaaacgtggaactatcggctgatcccggccatttaagccaagaagcgagtcattccaaaacaggaataactcgcttcttggcttaaattctgggatcaaaacgcctcgtgtcccactctctttgatgtttaaagcaatgcttcacccttatcgtgatcaactagccgttcactttccggcatcatactgccgccggttgcccagacaatgtgggtggcattagcggtgttaaaggccggcacttcggtaattgcccgttcgattgcggtaaagccagccgcagctgatggttcgactgtgatattctcagtgtccatcagctgggcttcatatttgtaaatcattggatcttcgaaagtaacgctgccaaataatagtgtccgcatcatcttaccggcaatgcgtgatggccggccaactgccaaaccgtcagctgccgtcttaccgtccaagccgatatcaaagaccgaaatcgcattattcagcttcgtcatcatccccaacgtcacggatggaacgtgagttggctcacagaagatggcgtggatgtatggcccaataatggtcttgagtccaaacgtcacgccactgggactaccgccaacaccagcgggaagatagacaatcactggatgatcgcgatcaactttgattccctgctgtttaaattgttgctgcaggcgaacggccgcaactgcataaccaatgaataagtcagctgatccctcatcatcgataaaatgaatgctcggatcttccgctgctgcctgtcgagcttgtggaatgaccgaggaaaaatcagtatccaactcgaccacattaaccccattggcccgaagtttggcctttttccaggctttggcatcccgtgacatataaacggttgtcttgaagccaaatgttgaagcggcgatgcccacacttaacgccagattcccagtagaggcaaccatcacgccatattgggcaaacaattgcttatattccggcgatcttaaaatcgcatagttatcagtttctttaagatcgcctttggtcatggcgacatgttcggcgaattttaatacttcatagattccaccgcgtgatttgatcgatccggagataggtaattcactatcagttttcaagtagaggctgcctgccagcgcagtgggctgggcctgattccaagccgacttcattttggtcagctcgattaatggtgattcaatcaccccgtgcatccgagcagtctctggaaagcagcttcaataaacggtgcaaagcgatcccaacgggcaactgcgtcaaaaatatcagcttttgaaaacggtagctctgcaggctggccataatcaggatttttccaaaaaattggcgtttcattcatcaagtctttaacctgtgggtatttaacttccaatgattgtgtattgtccatatcgatgatcccctaaaaaatatttactgctattgtattctgaaattaaggcaacacaatgctgccacagcaacctttaccaagctttaatcatggttgcagacagatgtcacttctcaaagcgtttgtcggcgacatccccatggcagcttactcgttgacctgattggtacttggtgcattgtgcttaatagcatccggtaccttaaatttcttcacttggttcacatttgaataggtgctggtgacctcctcggtaatcgacttctttgatgatttatcctgatactgcatataaatataggtattggttggcagataagtcttcttattcaatgtatatttgtaaacaaatttggtaatcgtgacctttttcaagacattcttggtactctcgctgttatttgcttcagccaaaataagcttcttggcaaccatcgaccctagcttgccgtggccattatatgagaggacatcggttgtctggttcttttggagcttcagatgcttcttcaaatactgcatggctttaaccgcagcgcttccggagacctgtcgacgaacacttttaatcagtgggctctttttaggcaggcgttgtttggaccagctattatcagcatgaatgtagacagtccggccatcaatgaagtaatcataatttttaaccaaaccagtggcattattcagtttagcttgaacgatcattggatcaaggtggaacttggcagtaaatttgccagtggatgtttttttattttgcgtatttttattaaccaacacaacattgccactcttaatcccatgagcggccttctgtgcgtgattcacaatggtaacagtatcagagggtttattagtcgattgctttgatgaacagccagccaggacgatgcccatgaccgcaactgctgcaataattacttttttcatcagatactccttattcgcatttaagtcaggttaaacatagaccacaagaccacgtaggctccggtcacaaccagaagcgacagccagtgggccttcagcactcttttgacggatttgaaccactttgagaaatagtaaaccgagcggttcttctgaaccacattgataatctgaaaggcagtcattgtggcgcaatatatcaagacgatgtaagaaatcacaaataacagatccatggcaattcctcgccaatttccggttaacacaaccatcaagaactgccagagatacgatccaagcataccaaaataaaagaaactgggaatgacaatggcaattctggtgggaaaaattgtgatcaccacataagcggccaacaacaaaattccccgcagcagcccttgaagtaggcggtgatcattgatggaaaagctgacggctaacggctggaatttaaaaatcaccgatgctaaaaagaaggcaatcgctccccaaacaataaaaatcaggtaagtcgagcgccgcagcttcaggttttctagcaaataaccacctccttgtggattgaattaattagtcagtgacaattgtgagttggggtttccatgttttggccgttgtatcaggaacgatgtagacaccataatggccattaacggaattggtggtcaagctggtgacgtgactggcaaccacagcggcataatacttcaaggcattggttgtccgatatttggaccaataagaataatagccggtcattgttttgggatcgacctgtttaacggtaaaattagttgcttttgcatttgtcacgcctgctttggccgcggcatctctggtactgatatcctgagtggcaagcagcttggccattgcgtctaatttggtatcagcggcactttgggttaatttggcagccacttgatccatcaccaacttttgaaattgactttgcggcaaacttgccaaagttgtcaaattatcctcaaagaattgaagtgatcgctgagctgagagcgaaataacaccctttgcggcagaagcatgacgtgagggattaacgcccttagtcagatagttgcgccaaataaagccgtcagcgccattcccatagttgtaaacttcgtagtaaacatggcttgaattgccatgctgcatcacaacactatttttaacgtaccaagttgtgttcgggtaatttttgaggttatgcagccgtttggtgtgggtcgcattccacaaataaactgcacttttggatttagcgtgataggccacggccgtgctgcgactcaacacttttgtccatatgtaacttgaatcggtgttcgttgcggtcgaattggcagtagccgcggtggtgtttcctgaaactggaaagcttgtagcggtgaagacgccaaatgtcaccagggcaagcaataataactttttcatgatgttttcctcctatgtaccagccaattaattatatcagaaaaatggggtgaaatatcgcctttagtgaatatatacgcaagagagcgggggcgttgtcttttaatcccagaatttacgcaaataaacgagtcattcctgtgcttgggataactcgtttatttgcgtaaattctgggatcagccgattgccgcacgtttgttctggataataatggggctcaaagagtctagcattagatcctgatagaaaccgagatacaactagcaaacagtgttgtctcaaactacttttgttctaatttatttttggtatgacaaaccccgccgcagacgtttccaaaaactggtgtcgtcggtctgtaaaatcaagccttcatagatctgaccaatgtaccaagtcaaaaggccgatgctaatgaccagaatcgccagtgaaatgctaatttccaacccactcgcgttgtcattgataattctcatgggcatgaaatacgacgagaagaatggcacatacgacaaaatttttgaaatcagcgcgtctgaattgctttgaaacggcatcgtcaagaagaaggcaatcatactcagatagatggcaggctgagcagctttcggggcatcttctgctttggcaaccagtgcaccactaaatgccgagatgatcgtgtaaatgatcacgcctaagaagacaaatagcaggttgattcccagcatgtttttaatcacgtcattgaccagtgtctggttgtccgaaattagctgtttaatgttatccaggtgcatggcgatctggaaaaagccgtaaccaccaacaatatagacgatgatctgggtcaggataacgccaaagacaccaagaattttgccgacaaagtacttcgaggctttggtgctggagaaaataatctccatgactttagtgcccttctcggaagcaatttcttgggcggtcacagaagagtaagtgatcaaaatcatatagatcatgaagactaatacccaaaatgaaatgattttcgccaggttggcaccgccatggttggtttgaattttttgtttgaaagacggctgaactgccagtgatttggtttgtttggcactcaactttgcgttcgccaggttaagctgttgctgggactgggcaagaaagacgttgattttagttctcatcccgccgcctagagaatcacttgaatgatagacaccactgacttttgccttatccgccgataacaccaggtagccagctaaattattattgctgacacttttcttagcggctgcagtggtggtgatgctggccttcacgtcatcccgattggctttgataaattgccttcggagtgccggttgatcagaaatgacggcaattcgctgttgatctgaactggaagtcgcactggtgtagccgatgcctaaagaaattgccaacaaaatgaacggagacagcaccaagacgatgaagctccaagacttaacttggcggagataggtttccatggcaacaattagggttttattcatgagagatccccgctttcattctgaaaatttcatcaagtgttggtggctgctgactaaattcttcgatgtatttaccgtcagtgagcttctcaaagacttcgggtcccttactgggatcatccaatcgcaacaagaaccgagaaccgcgaatattctggactttaacaacatgtgggagctggttcagctgttcttcagtccaatcggtagtgacaaaaatttctgatttgccaaactgatcgcgaacttcgctgatggtgccgtttaagaccacttcacccgtccgtagcataaccagtcgatcgcaaactgcctcaacattcgccatatcatggctggagaagataattgctgccccctgatcccgtgcttccagaattgcctttttcaacaaatccgcatttaccgggtccaggccactaaagggctcatccaagataatcaatttgggatgatgaattagggtcacaatcagttgcactttctgctggtttccctttgagagatccttaatcttatcagttttcttacctttaaccgcaaactttttcagccagtcgtcaatttgtgggcgaatttcttttgcaggtttccccttcaatcgtgctaaatagacaatctgctgctcaatggttagtttgggcatcaagctgcgttcttcaggcaggtagccaattgcatcaaaatcagcctctttgatgggctgaccactccagcggatttgaccatcatacttgagaaagtttaggatgctgtgaaaggtggtcgattttccagagccgttttggccgattaatccggtgatctggttgtcgggaacatcaaaactaatgtcgtccaatgcagtcagactgccaaattgtttgtggagatgattgatcgtgagcatgcgaatacctcccatttcttttgagcttatcataccataatcgtctggcggattttacggaaaacatttgatgtcaatggatttgtacataaaaagcaggatcgcaaacttgcaatcctgctcagaatcattttaattatcgatactgtttcattggtttaacaaagtgccaactgcgttgatggtacgcttgatcccagaattcccattccagttcgcagctcttcaagaattcttctttgaccacatccagatgatgttgatcgtagtgttccgcttcacggtcaatcaaagcaaataactggggcaaaatgctgtcactgtcatcttccatgtcagcgtaaaaatcaatccatggtttaaaaacattgtcgtcggtattcttcccctgcttcacaaaccggtttgcgatttccaggtaagtccatggacacggggtcatggccgcaacaacatcaatcaagtcgccagttcgcgcagcacgatacatgtgttcgttgtacaggtatgtgccgggagcttgtggttcgtgctgcagggtttcgtattcgacccctgccacgttgcagaagttgtgatgcggatggatttcactattcaggataaagtcaatttgtttggcaaaaatagccatatcggctctggtttgcgatttttgaatggcatcggcgtacaccttgatgaacgcattcagatagttgtagtcctgaccaacataaaaggacaaggcttcttgggtaattctccattgccgattccttcgacaaacggatgttgatagatctcgtgtaaaattggctgtccagctgcgactaattcttcagaaaatttcatgggtcagtgctccttaaagcaaaattttcaaatagaacgcgaccggacttggcacttttcgaactcattattccacttccctacgttggtattaaccaaatcaggttcaaagggattggcaagtcaccatctcagcacaaggcacccctagtgatcttatttgaatacccaaagtttaccatattttgaagagtattttacgattttcttcgtatatgatacgctgaaagcaacaattttctgagggttgggggaatcttactacaaggagagttgtttcatgaaattcaattggaagatcacactgattagcttttccccatacatccctttgatcgccatttatttgttaatccatttatacataacaaatgatgtcatcgctttgctattcactttaggtgttttttcagccggatatatttttgttcattataagtatgccaagactttcttcagtaaccatcctgaacttgatctacaaaactttgaattcaacacagtggcaaacgttgtcttggcactgtggatcatcgtcatggttggcctcataattctcaggctttatccacaaagtccagaaggctatctattggcatttggtttattctactccgtcattaacggcttcaaatcctacaggagagctgcaaaatgatatttaactggaaatacgctctattcactaacgcaccaatgttcctcacattgatcgtctatattggtatgactgcattacacattgattcaatctggctaattcttgccgtcgttgtaatctggctcgcatggtatacctatgctggttggaaagtctactctcttcatcctgaatttaatttcccataactatcagcgcggcacaacttcaatgatcatcatcacagtttcgacgattggttttctgttcttactcttaaagcttcaactaatagccaacatcgccctctttatcacatggcttgccatctcaaacttcttgatcgatggattctccaagtataagaatctcccataatgacacgacaattccaaaaaccggcgccgtaaatctcaaacaagatttacggcgtcggtcagtttataatcatatgttaagcgttcttcaccgcaaacaccggcaaagtattcaagaatacacagtcatctcgactagttgcccgtccctcggctaaaatggaacagcgttgcacaacattggcacccactttcttcaacaagtgttctgccgaagccagtgagccgcctgtactgatcacatcatccacaatgatcacctgtttgcctcgaagctgttctgcgtcacacccatccaaaaccagctgttgatgataatcagtggtaatcgaacgcatcccaatcgcaattgggtttcgcatgtacgccttaacactctttcgcaagacgaaataacgtgggtgatgggtaatcatgctcagttcttgagccaatgggatccctttgctctccaatgtcaccagataatcaaacggaatgttaatccgcttggccaactcctgagcggcataacgggttaactcagcatcccccaataagacgaaggaggcaattgccgccgtgtctgtgatcgggataatcggtagtgtccgcttcagtttaccaattgttaattcatattccttctgcatcttgatcctccagattatataagatagaaagaaagtaccaaaaacgactaatatgtgtgaaaatcgaggcttttcacagccacaactgttaacgaaatttctacttttatgttttttgttcgtctatgtatatgataatactccattttatcctttttatccacatatgatagtccagacacgaattttacagcaaaaacgtcaaaatgtcactttcagctcacaatccgtcacctaagacgacacattatgtggtctattttgggaatcatccacaagatacccccatatatagccaaaatgggtctcaatcaatccaactatttgtcactcccaaaaccacccttagtgtgattcaaatttttttgaagctcaccaatccgcgagtccacgcgattatgcagggtacaagcaaatctaccgaatacacaatatattgattctgaaaccggttagatatactatatatagtatcagttcgagcaattcaaacgaaatgagaatataatgtacatatgggaggaatcattatgcaagcaatgaaactttcatcagtttcactatctgatgaatttataaaacaagttaaagaagaagttacacctcactggggagaattaggctgggttacctacaagcggacttatgcccgttggctgcctgaaaagggccgtactgaaaactgggacgaaaccgttaaacgggtggttgaaggcaacatcaaccttgaccctcgtctgcacgaagacaacgttgatccccaagttgttgatgacttaaccgaagaagccaagaagctctacaagctgatttatggtctttcagctaccccatcaggccgtaacctttggatctctggtaccagctatcaggaccgtaacggtgacgccttgaacaactgttggttcatcgctgttcgcccacaatcatatggccacagccacattttgccagagtatctccaaccggacaccccagccgtttcgatgccttattcattcatgtttgaccaattgatgaagggcggcggcgttggtttttctgtcactaaagataatattcataagattcctctagttgataaaaagatcgatttgaaagtaatcatcgacaaggatagcaagtcataccaggattcccttgatatgggtgcaactgacaaagatgaatggttgaagaatcattcaatcaaagacgttcgttactatcgtctgccagatacccgcgaaggttgggtggttgccaatgcgcacttgattgatatgcacttcaatggcactaacgccgatggtaagactgacttagttctggatatgagcgacatccgtgaaaagggtgctaagatcaagggctttggcggaactgcttcaggtccaatgccactgattgaaatgttaattgatattaacagtctgctcaattcacgcgttggccgccatttgtcatcggttgatgccactgatattggcaacttgatcggaaagactgtcgttgccggcaatgtccgtcgttcagccgaattggctttaggctcagctgacgatgaagattttattacgatgaagcaggataaagacaagctctaccatcaccgttgggcatcaaacaacagtgtggcagttgattcagaattcgacaactacgggccggttgctgattcaatccaacacaatggcgaaccaggaattgttaacttggagctttccaagaactacggccgtaagatcgatggtctgcaaaaagacatcgacgccaatgttgaaggaaccaacccctgtggtgaaatttctttagcaaatggtgagccatgtaacttgtttgaagtcttcccttacgttgccagtcaacaaggttgggatctcgatgaagcctttactttgggaactcgtttctcaaagcgggttactttcagcaattacgactgggaagtttcccggaacgtcattgaaaataaccgtcggatcggtatctcaatgtcaggaattcaggattggattttggctaaatttggtaaccgagttgttaccggttatgaagatgctaaagatcctgaaactggcgaagctatcaagaagccaatttacgatccacgagttgttaaagaagttgatggcttgtacaaagccgttgtccgcgctgataaagattactctgatacacttggatgcaaaccttccatcaagcacaccactgttaagccatcaggaacggttgccaaattagccggtgtctctgaaggcatgcacttccactatgctggttacttgatccaacggattcgtttccaagattcagatccactgctgccagctttgaaggcttgcggctatcacgttgaaccagatgtttacaccaagagcaccatggttgccgaattcccaatccgcgcatcacacgccgacagcgagaacttcgcttcagccggaaacgtttcgatcgcagaacaattcgcaactcaagccttcctgcagacttactggtcagacaacgccgttagttgtaccgttactttccaaccagatgaaggcgaccaaattgccccattgatgagacaataccgcttcaccaccaagtcaacttcattgctgccatacgttggtaatgagttcaaacaagctcctaaggaaccaattgacgagaagacttatgaagacaaagtaatggaaatccacggcgatgtcgcaacggtcttcgcaaagcaaaacgataaccatgataagaagggtatcgaactggttgaccaaaccgattgtgctggcggagcatgcccagtgaaatagagtgtggagcaaaccgtttagtttccgagcattaatttgatacacatctttaatgcggttttcgcattgaagatgtgtatcggattaagcggaggaagctggcttgcggaacacatttcaaccagagtgcgagtcgcagtgtcagttgcctccgagcacgtttcatctaggtaaaaacaactgctaaaataatgcgttcaaccttggccccctcggtcccccgccgatcggccaagccctaaaacagatcattcccacggagaggccagggcaattaacttgctgctggcctctttcattacatacatcatggaggtatcacaatgttaaagatctacaccaaagtcggcgatcatggcaaaaccaagcaggtaaccggaaaaatggtgccgaagtacgacctgcaaattgaggcattaggggcactggatgaactggattcatggcttggctatgtaatttcagtcctgtcccccaagagtgcttcactggcaccgaccatccaaacaatccagcgaaacctgtatgaattacaggcagatatcaccgttaaacgtcaccacaacattacctttgacgacaccaaaaagctggaagtacaaattgatgaaattatggccaaattgcctgccatcaaagccttcattctccctggcggcaatcaagccggggcgtcgctccaatatgcccgggctttggcacgacgagctgaaagaatggtcgttgaattaaacgacaagcagcaaccgctcaatgatgaaatctttgagtatctcaaccgtttgtcggattacttattcgcccttgcacgttatgccaattacctggaaggctatgacgagattaaaagtaaatgttagttgggaaaaggtgaatcggaaaccagttactgaattggtttgcgattcacctttttaatttgtcattagaggttctccattacacatggatcgtatggcccgtcgtctgaccagtaattagttttagcgtgtcatcaagagattgtttgaccatattcttgacagcaatgtcggtgtaaaaagccacatggggcgttaagaaaacattgtccatcgccttcaacttggtatattccttaagcggaatgtccccatcaaacgactgattaaaaatctccgtctcattttcaatgacatcgatgccggctccggcaatctgatgattttgcagagcatcaatcagtgcgtctgtattgatgatgggaccgcgggaacagttgatgaaaaacgcggatggtttcatttgcgtaaattgggctttgtcgatcatatggtaattctcatcactcatgtaggtatgcattgtgatgagatcggcgtttttaaaaatgtcttccttggaggtatatgtaaccagatctcgaaacgcgtcgttttcgtgaatgtcatttcccaatacccgggcgccaaaacgtttaaaaatcttggcaaccgtgctgccgatgcggccaaccccaatgatgccaatcgtcatttccgatagttcccgtgagcgcaggccctcaacaatatagtcatttttggccattcgtgattgaaattgtgggatatggcggatcaaattcagggcatgggtcaacgtcatttcagcgaccgcttctggtgaatatgagggaacattggaaatcgtcaacccatattctttggcccattttagattacaagaatcaacccctgccgacctcaaggaaagctgggtgatgccaaaatcacggagtttgcgatataaatccggtgtttcgctgagcatgctgcgctgacggtaatcaatgccgtcataccctttagcaagatcgacagtatcgtcgtgtaattccacgtcattgaaatcaacctgaacatctggatgctccgccgcccattcgagcacaaactctttttcgtatcctaaaatgttgtatgccaaaatctttttcatcacgccatcgtcctcattgtgttatattataaaatgattagaatttggatataatatacctcataaagccgttggtgtcaaaatcatttcaatggctggccgtcatctcacaatcccaaggcgtctctgatcatcgtcaaaatatgctgttggtcgtttacaaaaacggtcgattgtcgataggccaggccaatcttgaagactggctgggcctcatcggtcaatcttaaagcgaccacattgggattattaaccttaactgcttgagtcaacaggctgacaccaatgccgtcggcaaccatattgacgatgctttgtgcctcactggatctgaaaatcacctgcggccgaatgtgattttgttgagcaagggtgtgaaagacccgatcgtggacaaaattatttttaaataaaatgaacgattcgttctttaactggttgaaagaaacttcagtgagtttggccaaggggctgtccttggcaacgagaatcgaaaagtgctgctgatcaaattcatcaacgatcagctcagaatcagtcacatcatccacgtaccccaaaaatgaaacgtccaattgaccgcttttcagatcccggagcgcagacagcgacccttcttcgacagtttgaatgtgattaagatctgataccggcagctactttgcgaccatcggaaagtaattagtctcaataatcggcggcattccaatcaccaactgctggcggtaactattttcaatctcccggactgcgagtcggtaatgatacaaaatttcatttgcatgaactaacagttgctcccccgcagtcgtcagggtaattgcctggtgtgggtttcccctgactaagagttggctgccaaatgcggcttcaagtcgcttaatcgcggcggagatagtcggctggctgaccgaatagtcttgagcaaccctggaaaaattcttttcggttgatagagaaacgtaatattttaaatcgttgatattcacgtttatttcccctttcctaaaggatatttatgttaactattataaatcataatggtctatgtagatattgactatataaagttgaacagactattctaaaggaaatgatcaagaaagaggcatttaaatgacacaatcaattttgaatgatccatttaaaaacaagggaaccgcctttacagaaactgaacgtcaacatttaggtttggtcgggatgttgccgccaatggttcaaacactggatcagcaggccgaacaagtgtatcagcagtaccaatcaaaatcatctgctttagagaagcgggtgttcttaatgagtattttcaatgaaaaccgcgtcctattcttcaagacattctcacaacacgtcgctgaattcatgccgatcgtttacgacccgacaattgcgactacggttgaacattacagtgaactcttcgttcaacctcaaaatgcagcatttctatcaattgacgatccagactcaatcgaagaaagcctcaagaatgctgcaaatggtcgcgacattcggctgctttgtgtgactgacggcgaaggtatcctgggtatcggcgactggggcacccaaggtgttgatattaccgtcggcaaactgatggtctacacggcggccgcgggaatcgaccccagtcaagttctgccggtcgttatcgatgccggcaccaataatgagtcgttgctgaagaacccgatatacctgggccttaaacagcatcgggtgcgtggtcaacgatacgatcagttcattgatcgattcgtatctgcagtcgaaaaccagtttccagacgtttacctgcattttgaagactttggtcgttccaatgcagccaatattttgaatcgttataaagatgaccaactcgtctttaacgatgatattcaggggactggaattattgttcttgccggcctcattggtgccctcaatatttccaaacaaaagttaactgaccagacttatttgtgctttggtgccggaacagccggtgcagggattaccatgcgggtttataatgagatgttagcagccggcttatcaccggaagaagcgaaacagcatttctatatggttgataaacagggattgttattcactgatacccctgatttgacgccggaacaaaaaccgttcgcccgttcgcgaagtgagtttgcgaacccggacagcctgactgatttgctttccgttgtcaaagccgtgcacccgacggttatggttggaacttcaactcaaccgggaaccttcacaaaatccgttgtgaccgaaatggccgcccatacggaacggccgattatcttcccgatttccaatccaaccaagctgatggaagccagcgcagctgatttaattaaatggactgacggcaagggattgattgcgaccggaattccatctgataacgtagaatacaaaggcgttacctaccagattggccaggccaacaatgcgctcatctatcccggactgggacttggagcaattgccagcgccgcatcagtgcttaacgatgcaatgatctccgctgctgcccactcacttggcggtattgtcgatccgacacagccaggggctgccgttttaccacctgtcagcaagctcaaccagttctcagatacagtcgcaactgcggtcgcacagagcgcggttgatcagaaacttaaccagaaaccaattgaatcagttcgcgatgccattcatcaagctcagtggcaaccagaatattaacgggaggacatatgactgaatatcggattgaagaagatacccttggaaaagtcaaagtaccaaagaaggcactatgggggccacaaactgaacggagccgacacaactttccaaccggccctttgatgccggttgcggtgatccgggcactcatcaacattaagcttgctgcagccacagttaaccaagtgcaacagacactaacgcccgaaaaagcccggttgattgaaaaggccagtcgccagttgttatcgctcaacgatagccaactcatggctgactttccacttcacgtttaccaaaccgggtcgggaacgcaaaccaatatgaatgtcaatgaggtcatcgcaaacctctgcggtcaactggactcaaaactgacgattttgcctaacgacgatgttaatcactcccagagttcaaatgatactttcccgaccgcgatgaacattgctgctaccttggccgttctcaaactaaaaccacaggttgaacatttgattgcagttttaaccaaaaagcaagaacagtattgggacgttgtgaagattggtcgaacccatcttcaagatgcgaccccgatcacgtttggccaagaaattagtggctgggtcagtgcattgacccacgaccttcacttccttgacgaaaccagtcagaccttgctagaggtcccgattggcggtaccgccgttggaaccggcttaaacaccacgccgggctttgcttccgcaatggtggccgaactcagtactgcatatgggttgccattcaaaacccaaaatcagttctacggtctggccaaccattcaggcatcacggcaacccacggagccgtgcgaacactggcagctgatctactgaaaatagccaatgatatccgttttcttgccagtgggccacgggccggctacggtgagttgagcatcccggccaacgaacccggttcatccatcatgccaggtaaagtcaacccgactcaagcagaagccatggccatggcggcgacgcgggtaatgggcaatgatacgacaattgaaattgccgccagtcagggcaactttgagatgaacgtttataaaccagtgatcatatttagtttcttagagtcagtcgagttactaaccgggattatgacgaactttaccgataaaatggtcgctggcatcaccgtcaaccaagatcgaatgaagcagttagtcgacaactcactcatgaccgtcacggcattgtcaccgcacattggttaccacaaggcagcagagattgctcaaaaggcgcatgaggacgggacaaagctgaaagttgccgctttggcacttggctatgtgaccgctgatgactttgataaatggatgaagccgattgatatgacgaataatgatcgaaaataacagtgcggaaaaatgagcgttaagcttccagagtaaaaggggactatctaaacatccagaggttggatgtttagatagtccccttttacggccggaagctgctcatttttccactattcggctagataatattaaaaaatgtttttggggtcaaatcattcagcgttaccccagagcctttaaatgtaaggatcttgccacatttttaaatccaattctaagaatcgcaaactatctaccgagtcaccggcccctgccaagacagcatcccgccgctaacattaatcacttgataaccagccttgcgcaaaatccgggccgctcttagacttcgtcgcccagatcgacaaatcaaataccaaggctgtggggcagatacttgggcgatgttgccaggcaatccagataatggcacattctttgcagctggaatgtgaccggcttgatactcatcaacctcacgaacatcaagaattaccggcttatttggcagtaactgcttcagttcagatggggtaattgactttatttttgaaaataacaatgaataacgctcctttaaaaatgattgatatatcgagtataaaagaactctgccaaaagtgaaacccggtttctgattcaataaaaattccaggttgtgaaaagtcttaaaattttgtatggtaaacccaacagaaagtgagggattcattattcgaaaagcaatccacgccgcaaatgcatggctgctctttgccatcgtcatcggcgtcatttcaacaccattcgacttgtggctacatcatgaaagcaacttttttgatctgctcaaggcattttttgaaaatggcttactcggatttttaggatcgttcctactagtgctggtattgggttggctgccagtgtttctacttgttcgttttttcatttggttgaacagactggtttcaaaacgagactattttaaatagttatccagaaaaatattcaagaacagaaatcccaaataagcgctgattaactcaatccagtattcctgaactgacattttaaccgcaccaagccatctccccagatagtggtcacttttgatatacatattattatgaaccgtccgtaatgccaccagggaaaagaagtagatgctcgcaccaaacgccaaggtatgaagtaggaaaaaactgccactccaaaattgacccttgataaacaaaaagatgaccaccaatgcccaaattgcaaacatggcataataccaagcggttggaaacaggattgaccacttcgtgtggatcaatgaaaaaaataaaaaggttaatggcacccgccaagcaaaataggtcgtatctatgatagacacgtgagaaacaccaaggttttcggttgctgggagaagatcactaaaatgcggcaatacaatgagtaaggcaatcaaccagataaaaccgccatatattaaaagcgccttaaccactgtttgattgatccgaatttttcccatagatcaacaacttcctttaatcagatttcccccttaaaatattagctactaggttatcatgaaccgaaacaaaataaaactgccatcgacaatcccgatgacagttaattctacctcacaacctcttgaaatgtcccaatatccagtgccaaggtgatcgtcaacaccagaataatttggaaaaaatcggcttcctggaaccgtcgatacacaattgacatgaatggatcaactagaaagtaagccgctactacattcaaaataacaaaaataattgcaaacacaattcgttttgcactcatgaaaccgccccattccgctctccctaatgtgtcgaagttgttgtaagtgtacaaagtttgcggtggtaagtcaagcaacttgcatatggtattataaatataatctaatatataactttgatacaataaaaccccactgccaattgcgacagtggggactcttttaacgatgcgctttattcgctttagcttcatgaataatcttcagagcccgcttacggatcttgatacttgggctcttcaaacgacgataagcactcgcgagatcttgtttttccatatcgatcactcctttgccgctgttatcttaccagctggccttgtgaacaccagggatctgacccaagtgggcatacttgcggaagttgagacgtgacatgccaaacttacgcatataaccgcgaggacgaccgtccaattcgtcacggttccgcaatcggttagggttagagtcctttggcagcttggccaaggcctcatagttgccttcctttttcaattcacgtcggatgttggcgtacttttcaatcaaagcttcttgacgtttattctttgcaatcttagacttctttgccatatgagtcctccaaataagtgtatttttgatattgtgggttttaggttattttgtgtacactcaatagtaacggttactattatgccaagaaacgtcggacctgtcaagaataatcattaagaagcatgggaacgtcggtgaaaccgatacgttagctcaacgatgataatcccaagccataagccaattgccaccgcagatgcattgtcaccaaggtgtaaatgaaagacccaaccaaacacaacgacaatcgtcaaaaatattgcggaggaataaacaaccttcctcaaattcggccatcgtaaaatggctggtcgagcatttaactcatcctcaaaccgtttgacccgcaccatgacgagcatgttcagcagcgctactaaaagtaggaacacgcccgccgctccgccgtgccgaataaatatcatactgataataaataaaatatcgatggtgattgtaacctgcttaatgggccgaatccattccaaggcttcttttttctttaagtactccttcatcccaacatcctccttcaagaggacgtccaatgatatatggaatagatcgcttaactgaattaaactatcaatgtcaggataactgttttcagtctcccaactggaaatggtttgtcgggaaacattcattgtgtcagcaacctgcttttgcgtcaaacccaattcaatccgttcagttttcaatcgtgcaccaaatcgcattatcatcctcctttcttatgagaatagtgtataacgcaaacccatcagaaacctagcaaataatctaagcatactattatacaggtatttagatgaacagagtgacgccggaatcccacacacaatgtagaatcgtgctgggccaaagattcttggtgcgataaaacatccagccaaagatcaggccaagtggtaacacgttggcgatgttaatgagccaagcgcccaacgtcagaccttccagatagtaaagtggaaaatgactgatctgaaataagattgcttggataatattggcggtgacaatcccgtatcgcttcatcaagaagttcatgaggaacccgcgaaacaagaactcttcaatcaagccggcgcccaaagtcacactcaagaactcgccgcttttgaacggattgggttgaatgtaaaagccatggtgggcaccaaacatcaagaaaaacagataggcaatgaacattgccaacacgacccaaaatacggtcggaaagtttccgttataaagtttgcgtttgtcaatccataattgggcgttcgtccgactgatccagaacagtcccagaccaaccatgatcacggctttgatccccaaactaaccagatcgctcgccatccctgtcgtgtagtgatgctcaatgaaattgataagttcgcgaccgaaaaaccagagtacaatcagaaacacataactcaggtaaaaggtcgtcatcgaccaggttcttctcaaaatgttgccttccgtttcgtcatatttagggtttgattatatcactatccgagaacaaccagaagtgagcgacaaaccaaaaaggccggtacacaattcacaagaattgtgtgccgaccttctcaatggtcatgattaactatcagtttcaacccagtgctttaacaggtagacacttccaacagattccaacgccgtgaacccaagcaagtaaatggttgcgtaatagagactcatatcactgttcgtatcagaactaaagaagtgattcatcacgccatctacccgattttcaatgatcgagaatatatacaggaatgccacgatgacgacaatgtacaaaataaatctgaagaacttttgtctagaatctggcagaaacgcggttagagcgttcccagttaagtggatcaatgtgatcgacgcccacaaaagaagggtcatggcaattgccagtaaaatcgtaccaattgtcaaaagaatcatattctttacaaagtttggcctatccgaatgcatataggtgtagtgaaacatcttcttaaattgagcaccaaaatcgccccaaaacggaatcgcagcgatcacccacagaactacctgggtaatgccggcgtacaccatcccgatgaacgaagatagcaggttaacagagtatagcttggtgtcacttgccggaattaaccggtaggcgtcgctcacgaaaatgtgctcactgttccgagacatcaacacaaaggcaacgatggcgacaaataccgagtacgaaagtgtgatggcaagtggcgtatcggtctccagatctccgcgataaacttgataaatcagcgttaatacaatggcaatcacatcaattaagacaatccggttcatgatccgcaacttgggccgagtgagcgatttaagtaagtcatagaaactagtcatcgatatcattcccttcataaatactttcgtaatagtgttcgattccttcagcgtactttgaacgaatctcttcggcactcttctgtgcgtaaactgttcggtctttgatgatcacgacttcatccaagatactggcaatttcggaaacgtaatgatcggaaaccagaatcacggcgtcatcactcttccatttgatgatactctgaatgattttcttccgtgacatactatcaatcccgccaaatggttcatctaacagatagaccttggtatcacgtgacaacgtcaatccgataatcagtttctctttcatccctttagagagtgctgataaccgtaaaccttcatcaatctggaggaaaccagccatttcgttatactttttggttgagaaatccgggtagacgtcctcatagaaacggataatcttatcaattcgcatgctgggattaaatccattcaactgttcactgaagctaatggctgatttcttgtctggaacgccatccgtgccggccacggtaatgctgccggaagcgcctttggcaaccccggcaatcagccgcatcaatgtcgtcttaccagcaccgttttcaccgaggaggccaacgatcttgcccatctcaatgtttaaattaacatcttccaaaatacttcgataatttctccggtaattcaaattcttgatttcaatcgtgtttgtcatgattgcacctgctttctcttattgatataatcctgcaaataatcgacaatttcctcatcgctcacattaagtttgcggaggttttcatataaatcctggagttgttctgtaatgaggagctttttgagtttttcaatcgtttcccgatcctccgtcacaaagttacccttgccacgctgaggttcaataattttctctgaaatcagctcgcctaatgctcgttggacggtattgacattgacggtaaggtcaacggccaactgccggacagccggcagcttgtcaccaggggccaactcacccacgataatttggcgatagatataattcttaatctggtagtaaattgggatcttatcatcgaatttcattgtcccacctccctagtgttatattttactattacactataacaccattttggcaaaaggacaaggaaaaccattattattaatcatctatgcaaaaaaaccgctacacagctacgcgcaacggtcttgataaatcaatttttattaacaatcttgccaccatccatgtgaatcacttcgtcacttagatatgcaatatcttctttatcatggctagcaagaatcacggtactcccagcatcggcaatttctttgagtgtctttctcagaagccaagtgctttcttcgtccaagccattcgttggttcatctaacaaaagtagcttaggccgttcgaagatcgcttgagcaatgcttaacttctgcctcattgccagagagtagttagcaactttcatattccagtcatcttcagttaaaccaaccctttcaaatgcagatttgatatcctcaatcgttgcaacttggttaattttggacaatgttaccaagttctggagtcctgaaaggtctttgggaaaagtggtgttctcaatgatgagacccatcctctcagagaaatccagtgtttcatgaggaactccttcatccacaattacttgtcctgatgttggaattagcaccccagtaaccactcaaatcaacatagtcttctcggaacagtgaatacaattatggtatcattcgatgcatggtgataaaatgatgaatcttcgagataacttaaagaatttcacaattaccattttttatatccttgaattgtcaaattaagtgcaacacgacattaaagaatatttcataaggcgttttccatccgagacatttacggggacgattattcatttgttctgcatatgcttgtatccggcggtcagtaattgaatcaaggtcagttccttttggcaaatattcgcgaagcaagccgttagtattttcgttagttcctcgttgccaaggagagtgaggatcgggaaagtagaagggcgtaccaaacttatcagttaaacattgaactttggcaaactctttacccctatccggggtaatcgttaacgatctaccaggccatagcttcattaagtcgctcaaagtatccgtgactgcttctgaagttcttttagcagctttaccaataagcaggtaacgagattttcgatcaaccaatgtaacgacacaagcctttccgcttttgcctaacacggtatcaccttcccagtgaccaatttctacacggttgtcagcttctcgcggacgatcatgaatcttgtttgggattggaatcttgcctcgcttttcttgataagctttattgtggcgagacttgccgtgatgccttagatggcgcacggcactagagctgccagatttaaacaaattatcaaataagccattgaaaatcccacggtaaatagtcgtggtactgatctgcaccggatacttttcgactgccaagcgattcgatatttcctccggagaccaaaggtcttcgcagaagtgttctctcaccacttcaaacacctgaggattactcaagagagagactctgccacagttgcctttgcgctgtttgtacttctcctgagccttcgaaggtgaataggatttaccagtagaattacggcttaattctcgagaaatggttgagtaacttttcttgatatggctggcaatctcacgaagtgagtttccatgattcctcattaaaaagatagtttcccgttcatctatggtaatatgcttgtagtgatccatggttaaattcctttcatgattgttttcgcaaacatcattttacagaaatttggccatgggccattctttatttaattagtgttgcacttaaagtgtaaattcaagtcttaataaaaagaaaaccgctgcatcagtacctgcaacggtcatccaaaagccatcaaaatatggcgatctaagattagttgtcgctcaaaatcgactcaacctaattcctgactcgaactacccttactaaacacttaagtaaaaagtagaattcttaaaatgtactagtaatgaatgtcgagaacaacaaatgtaatatagattgctgctaatattaatataaccaatcccaacagaagaattatttgcataattgttggctttgttcgccttttccccaataattttatgaatacggatgttacccctattatcaaaaaaactatagcaattccaattagcattagttgtctccttaactcagtttttgattaatagtttttatgagtaaattacagtttactttgactggttgaagtcagagaagcaattggaaattcatccgtaagtgtgatccgacacccaccttttgattttccattattaatcattgttttcacatccgattgtgctgatcctgatcttactgacagaatacctcctgcccctgcaccaaagattgcgccaaataatcccgccgaaattacgcccacgacggctcctccggtcaccaactcatcttgaattaaaccataatacgtacgtaattttgctaatgcactggttgatcctgcaaaatcattgactccacccttgactatcttttcatgaacactcgcaggctttgtaatcgaacgcagccctacttcattagaagctgtctaaaatctcttaagtaatagtgctaaaaacgctaaaacgaccatttgcagactggtggttaattgacgctcacaatttttccaaagtcgccgacaattctctagccaactaaaagatcgttcgactacccaacgttggggcatgacttcgaatcgatgcaactcattgcgcttcgcaacctgcacggttgcgtttaaattactggctacatcgagctgaaaattaacgcctgaataaccaccatcaactaagacattttgaacctggcgtaaatgcatggcatgtaaagcgatcatggcactggccccgtctcgatcagagacgttcgctcgcgtcatgtgaatggcttgcggaaagccattgatatcaactgccagatggcgcttaatccccgagattttcttaccagcgtcgtaacctttgttttcagcagtagcggtgtttttgacgctctgagcgtcaacgataataaaggaagttaaagctgaacgtccttggtaagttcgccgagcaatgacaatttttttaaaacttgttccaataaagaatcagccgtaggctcagctttagttgaccaaattttgtaatagttgtaaactgaccgccattctgggaaatcaccggggacttgacgccattggcaaccggttttcaagacatataggaccgcacagaagacctcgtagaggtcatattttcgaggcttagttcgcttacgaaaattttctaaagctggtcgaattaattcaaattgttgccgagtaatattgctgggataatttttcatagcttaaactcgctttttacatagaagtatatcaaaaatcatagatcttggacagcttcttagtagcccctgcatcgttgaactgaatatctgcttcagcaccatcatatttatttaaggcaaattacaagtttaatccgaacaagcccggaatctttcaatggcagtctgttgatgatgtatttttaatggtcgttgattaattagttcaagtgctgctaggatctcatcagtcgttacttggctaaaattggtctttttcgggaagaaccagcgtaaccgtctattaaaatattcattggaacctcgctcccatggtgaatatggatggcaaaaataaactttgatctgataatcctgttctaaggcctgataattggcaaactctttaccatgatcaacagtaatggattttacttggggaccgaaggcccccataaacttgccaaaggcggtgtttagagccttagccgttctattaggggctttgatggcccatagaagtcgggtcttacgttctacgaatgtaaccagacatgatcgtgactcacttcgactagaaagcaccgtatctacttcccaatgaccaaaagctaaccgttgattaacagttgttggccgttgttcgatggaagtcccacttgtaaatttcccacgattttcgctcactcggtgctggcggacattccgattgggtagatcagtcaatttgaaggggagccagccacgattaagccaattataaattgacgcagtgctcaagttataagcggccgcaatggtttctggtgaccaggttaatcgtaagtgattggtaattaaagtcgctaatgctgccgtcagcatcgaacgacgaccgcaattccgccttttgcgatctgcatcttgctgagctaattctggatcataaggtttaacccggtccaactcatagctaatcgtagctttggcgacgcctaaggcgtcagccattacttggtaagatttattcccctcattgaccagttgtgctagtgcgccacgttgaaaacgtgataaagtagatgtacccaaagtaatcactccctatattggttggaattagctactaccattgtaagtgattgctttgggctttttaatttctgttcggattaattatagaatttgccttaataaatcttgcatttttgcgctcaattgatcctcgggcaagttttgctgagataataacttacattccttagaaaattctttccactgctcattagaattggctaccgtaacattttgatccgaagcctgatctgtatccgaaaattttgtggtgctgtcactagccaccaaggatcgggcagaactatctgcattgacggttgatatgtcttgaaccgccatggaagataacaacaccgctgacatcatggttacacctatacgaatacttttctttcttgtttaatactaaaaacctccaaaatatgagtagatttatttatatttcaaaacccattatttcggaaaagtacacacatcgcaagaaaggattgcttgcgcaagtattgcttgatattaactgagcttacaaaaagttcatccaatacttttgataatattcacaaagcttttaaacgacattcacacattattcacacgtatactgtcgaatgtatttatgatactatttgacaaatggaggtaaaatgataaatcttggaaataatttaaaagagtttcgccaatacaatgagctttcacaagaaattattgcatgcagattaggggttagtcgtcaagcaatctcccaatgggaacacaacctcacataccccgacatcgaaaatttggtaagattaacacaaatttttgattgcgatattaacgaattgctattctaaaaaggaaaaatgcagccaatcatttaaataaagctctcaaatttcactaaagaggttccacacattagatatgtcaggtgtggagcctcttttctaattgatttttctgaccagtacataaacaattattacaaagttcgccgtataggtgtcagtgaacaagtcgtcaattgatgattcgctatgagtagagtaacctgtttacggcattgttaattatggaccaaccccggcaactctttgccattggcatcgattgccaagcgaaccaaaacaagcttgctggaatccaccggcaggccgtcaatgtagatttcccgatgctcatttccgtgcagacgagtgaagccctgcttttggatcgtattgtccaaggtcttcagtgcttcactatccgaggttacagcaccggtattaatggtctgaatttcaatgccttcagccaaatgctcaaacttgatttctcccaaatcaaaatctgagaaatcaatctgagttaaggcagcgtcgaaatccttttcgttaatgaataacggctgcttaatccaaatcttaaagtcttcaccgtctccggtatcagtccaaaccgcttgaaccgggtatgggcggtattctttgaagccctcgaccggaatccccttctcagggccaccgctgattgtcttggcaacttctgcagccgcattggccagccgtatgaagtcagggtcgtccgtgtgctgggtcgcatgcccttcggcagttacataacttcgtgtggttagatcaacaaagctcggttctttatctcgactgtactcatctggttcgaatgtctcccaattaaacatatgaattccccctttgatttcgcggtcaatataagctaaatcggcggggaaagcaagcaaagggctcttattcggactgtaacgattatccaaaaatgacaattaccgcaacgaagatcaggacggcgacggggaggatgactgaactattataattcataaatccccaaaagttcatttgatcatgattacttccgatgacaatctttttctgcagccgctcgtcgcccttaatcaagctgtccaaactaaccccaaataaatcacttaactgaatcaaccgttcaatatccggatacgctgaaccaacttcccatttagaaatcgcttggcggctgacatgcagctcttcggccaatcgatcctgggtccagcccaacttttcacgttcttctttaatgcgttgtcccaacaccatgttaaccacttctcttcacaaatttgattgttattattatgccattattagtcgggtgatgcacgctcatcttaagggcgatggcgtgcaaccagtcgttgcggacgataataatttttaacaatgcttttgattgctttccatagccgaccacttataattaaggtgaatcacgtaaccgctttcatttattaagggggattttatcatgacaatcaaaaacgtaacggttgcaggtagtggggttttaggaagccaaattgctttccaaacagcttttaaaggattcaacgtcacagtttatgatattaacgaggatgccattaatgccgccaaggagcgaatcaaggggttgcgacacagttatcggcatgacattgcggccaccgatgccgatttcgaagctggtttatcacgaatcacctatacttgggatttggcagacgcagttaaaaatgctgacctggtcatcgaagccattccagagcgactagacatcaagaaaccgttctacaacaagattggtgagatggcacccaaagaggccatctttaccagtaattcatcaacgttggttccaagtgcactgatggaagataccggccggccgagccagttcttaaacatgcactttgccaaccaagtttggctgaacaacaccgctgaaataatgggatcgccaaaaacagatccaaaaatctacgatgaaattgtcgaatttgctcgaaacattggcatgattccaatcgagttaaagaaagaacaacccggctatattctgaactcactgttaattccactgttgagcgctggtgaagaactttgggtaaagggggttgccgatccagaaatgattgataagacctggatggcagccaccggtgcaccaatgggtccatttgccattctggatgtcgttggcatccggaccgcttacaacatcactgcgacccaagccaagagtggcgaagatccaaatgctcaagttctcgctgacaaactcaaggaattactggatgccggcaagctgggaatggaatccggcgaaggcttctaccactatccaaatccagcatataaagatccagactttttgaagatttaagaagcaacgtgccaatgaacaaaaacgcttcaggagaattttagttctcttgaagcgtttttgttcattggcaattaaattctgtggttaaagattgccctgattattttgtaaatgatccaaaggataccagccgtgatcgcaagactgattactccggcaacaatcgaaaagttcataagaatactcccatgttgagataatttaaagtcacatctttaggttatactaaaaagatattctgggtcaagaaagcatccctttccccaaacgaggtattgttcacagaatttttcccaaccacttacatcagaaataccagaatttttatacaaaacgataattaattattgtcttgcaataattaatttccgcgttacaataatatcaaaagggagtggttaccatgattaagaaacaaccaaatacgttcatcaactttttatacgtcatcagtctgctaagtgtggcttcattattaattgcaatgggaactttggcacttgtctttgtgattgctggaatcgtttatctactaattccatctgctcgtaccgggatttttcacgatatcattagtggaattggcggatcgacgaacatttgggtgatctgcttatcatttgcattattgctcattatattgggattaattacccttgtctcattttcagtcttcaagctgattgcaaatgtccgtcgaaacatctatttcaagccaattaatttaaaatacatccaaggtattctttgggggtatgggggtatcattttaaccaactactgtagcggagtcttagccgacacctataatattaactcatcgtcgatttcatccgaccaaggaggcgacggtacctcgctactcatttggtttgccctctacgtgatctatgtaatgttcaaatatggtatcgatcttcaagaagactcggacaaaattgtttaggcggtggtgtctttgatcaaagtaaatctagacagagtgttgttggataaacaaatcacttcaaagatgttggcagcagaaattaatattaccccagccaacctatcgattctaaaaacggggaaagccaaggggattcgctttgagactctggcaagaatttgtaaagttttggactgccagccaggagacattttggaatatgttccggagtagaatactgagcagacattaggaaatgtcagagcgagataatcgtcaagtcatcagctccacaaatataaagaccagtttctacatctaccactgtaggtgtaaggaactggtcttattcattcgtgtaaacatagcgaaatatttacttggatatatttaatcactattatggatgcgcattgctcgctattcgtttggttttccaataatcaagccataccaattaattctggaagtacttttagttgatgcggagtcttttacattattaagcatataaattcccagtcgatatccggacaactcatcacgtttttcctgtgtatacccggctttagcaagcaactttttgacaccagccagtttttgagcattagattcattccgatgactcattaagtagttaataaccggcttgaaggaaacaatgtcggaatatcctttgacaggatcaggatcaaaatcgtcaccatcccaccctgggtcacgcataataccataattgactgctgcataatatgaaagctgatagtcaacaggcgtgttggggaataacttaatgatagcccgaactaatttttggtgattattatccttaatatagcttaagtaatcgcttgtgttatcaaattcagaaggatacacaatcacattcccatgataattttttgaacgccctttagccatttgactagccttcacgtacccggaaattgtaccattcttggtatccacatctgtgtaataataccattgctggttaccattatggctaactagaatagaatgccttcgagaaaatgtttgattcgtataatgctttagatttgctcgtacctttgtgtgtgaccaattccaaaggtaaacgttcttttgtccgcttgcaacatgatactggcctcctgcatattgaggttggccataccgcttctgaagaatttgatagcctgttggattaaatcccgcttttaaatagcccttccaaatccatccccgttttgaattcatagtggaataattggtaacttgaatccagttattgttccctttgtaactgcccgtcgccgtcttaaaccaagtgtaagttggataattcttcaaattataaagcttcttagtgtgcgtatcgttccaaatgtatgcattcttcttaatattcttggcgtgaacagcgacattgctgaacttattgtaattgaagtcattaatgtatttgatattcttaaaggcagattgtggttgcttcacggcatcaaccgtttgggaaccaacaccaccaatcaaaaatgcaaaacttaaagttattaacatcaatactttcttcatcttcgacccctcaacttgttggtttatcacatcttattctgtgacagagtttgatccgttcaactgtttctcagccataattatcagacattgggctttctttgtcaaaattaccgtcactgaatattcagatatgacgcaagacaaaataaaaaagttaccttagatttacgtaaggtaactacttgcgcggatttatgttttgtctctccaagtaacaagaattactaggacaggaatagagatcacgtttcccattgcagaccgatagtgaccaaaatatgcagtgaggccggccaagataagcaaagcaatggtgattattagatttttagtcttgagtttcatgatttaaggatatcaaaaattacaggttgttacatccctacttgccgctcttaaacaacttcctaaacaggaaaaagttaaccagcccaagcaaagccaacatcccaaatgccaaccggctgccgacgacgatgttttgcacataagacagggtgtagatgtgtaccgaggtcatcatagtcgcaatgaccgttgttccaagcgatcccgccaacatatttccggtgccgtatatggcattggcatccttctgttcatcttttggcaaatgtttcaagccataggccatgctattgccaaacgccatcgaacggcccgttgcgtaaaccgtgtacagaatggtaatcaccaaaacggacatttgttgacccattaccatcataatcacaattggaacgagaaacagcgaattccccagataaagaggtagtttgccgccaaatcggtccaacatccatccataaatcggctgccccaatccatttaggacactcccgggcagcaaaatcagcccagcgataaaggcactggcgctgttcacaatctgcacataacttggcagcatgaagttcaggccgatgtttgaatactgcagaaaaacatagggtagaaaactaaacagaaataccggtcgtttgaagacggacagtttgaataatgctttgtgactggattttgacagccagccgaacaagcaaaatgaagcggcactgaccaccatgtagcagatgaatttaactaaaaacccacgctggcccacaatattaaagcccatgagcagggtaatcattgctaacgccagcacaccgaaccgcagccagtcaaactcatagtgttcggtcggcgtatactgcttgataatgaagatccccaacagcaacagaaccagggtaatcggcacggtgatccaaaaaatcatccgccagctggcaaatgacacgaccgccccgccgaacattggccccaacgctggtgcaaccaagacgatcaagttggccatccccatataggttcccaatttgtgggcgggaacgacgtctaaaataatgttattcattagtggtcccgtcaggccaacacatcccgcctggaccaagcgccccaccagtagcgtccaataatttggcgccaaaccgcacatcacatccccggcaatgaacagcagtgctgctgacacaaagagctgtttgttggtgaaccgccgtttcaaaaaggctgaggtaatcgtcaatagtgccaccatcagcagataccccgtggtgacccattgaacggtgggcagggaaatgttgaactggtccatcaaagttgggaaggtaacgttcatcgatgtttcagtcagcactcccataaaggtcatgaatgccacgacggtaatcaccaggaatggatgcttttgggcgttctcattttgttcattaacagtggaatccacggtgttgccccctcaaaaagtcgtatagtcgaattaactcgcaactaatatactaccatttatcggggagcatcgacaattaaatttgtggggtatcaatgacctcaaatacttcgcagacaacggggctttccagtgaaaacgacttgccacgaatcttggcttgcttccggaaaagctgtttgtggagttgccgccaatatttcagcgaacgattcccttcgccttccaaataggcgtgttcttgagatacccatttgaatgggacaacctcgacaacttttagctgaacaatgcaggccggatcgccattccgcttgagtaacatccgatagtcgccgacctttggcaccacctggtcggcatcataaaaatcaaaccaggagctggcagcggtcttctgtccacgaactaccatttcaaccaacatatcagttgaattgggccggttggtaaacgaccaagtttcaaaattagttttctgggtgcggctgcgacgcataaagtcttcccagtaatcggttgcatccattttcaaaatatccatatgcattcctccgttcatttatgattgatggacatagtttactgtggcgagcttaaatgaagcttatgtacaaaaaagttcccgcacgcctgcaggaacttccatttcatttcatcattattttcgatttcttctatactatgtgtcaggtttcccctggaagcatttctacttctcactatgtcatccaaatctctgagttggtctgattatttaatccaaatgctggtatcaacctccttaattgcttctaagttagtgctgagccacacgagtggtttgattttggtcaattgtttctttaatcgcactgcctaagcactcaatcccggtttgaatctgttcttcagacatgttggaatagtttaatctgaaggttccaggagtgaccttgtcaggataaaatggttcacctggtacaaaggcgacgttgtgcttaatgcaggtgttgaataatttaatggtatcaacatctcccggcacttcgacccaaatgaacaggccgccttgtgggtgactatagttgacgccggctgggaaatacttctcgatggctgccatcatcacattttcacgtttgcgataaactttgcgaatcttattgacatgctcgtcaatgttatattcagccataaatttagcaacaatgtgttgggttaaattatccgaatgaacatctgcggattgtttcatcacactatatttaggcattaagtctttgttcatcacgatccagcctaatcttaatccaggagctaagattttcgagaaggtacttaagtaaattacccgctcttcattatcataaaacttgaccggttcaatgtcgtcgccggcaaaccggatggccccataaggatcatcttccatgatcatgatgtcgtacttgttggcaatctcaatcatttgttcacgacgttcagccgacatggttcgaccagttggattttggaaattcgggatcgtgtaaataaatttggtgttgggattagcagcaacggccttttccagttgatccatccgcatgccgtcttcatccatttccacaccgacaatatgggcaccataactgcggaaaacatctaaggcacaaaggtaggtcggcttctcgacgatcactgtatcaccaggattgacaaacattttagcggtgatgtcgatcgactgttgcgaaccggttgtaatcattatattatccgcagtggctttgatgccctgcctgttcatgcgttgggcaatttgctcacgtaaggcaggataaccaatagcagaagaatactgtaatgcttcccgaccactctcatcgaacacctcattggtcactttctttaaggcctcaatgggaaataattcaggggcgggtaacccgccagcaaaggaaatcacatctgggctgccggcgacttttaatatatcgccgaccggatcgctatcgtttttgggaactcgttctgaaaatcggaaactcatacgcgaacacctgccttttgtgtgtcatcattttgatctgccacgttcgtttgcggtttgtggtatttccgcatcatttctgccatgtgaacttcttgaaccacaaactcgtgggttcggcaaacgtagtcgtgttcacgaccaattttggcaatgtagccgttaatgtaatcaacttcagttggtcggccctttgagaaatcttgatacattgatggataatgatatttgtattccttgctgacactaatgactgaatcaacctgttcctgacgagtggcgataagataaattccggcccgctcacaagcgtcataggcttcatcgaataattgctgcgacatctttcgaacacccggatactcgatgaactggcccatttgcatttcaaacattgtacataatgtgttcgtcacagcgttgaaaacaactttggacatgcacatgcccatccattcgtcggcgaagaccggtcctaatttggcattggtgaagtcgtcgaagatcgcttgagtcttggtgtccggcttttcgttgttgtaacgagccatgtgcatgacctcgtcaccttcagcccccatgaaatcaatatcagctgggccatccattcgagtggcaatcatcgcagtcccacagataatgttatctttagggaaatacttggcaatcttttcaaagtggcccattccattcattgcagaaaagacatattgatcatcatgaaagataccggccttattatcgcgctctaattcttcagctaactgcatctgcttcttgaaaacaatccaaacatccgggtgacctttatattcttctggatagtagatgttgattggaacaatgcgtcggttttcgtggtcacgagcgacagtgacaccgccttgttcgcggatcttctcaacgtttggctcccaagtgtcgatgaaatcaacgtcgaccccggcattctcttgtaacattacgccatacctaactcccattgctcctgcgccaataataccgtacttcataatgaccactccttttattttttatttaggacagctgcgtcaggcagaaacctacgcataagcaccttgcccaaaaattccaaaaccaggaattcttgtccaaggagacttatgctccggtttctaaccgcctgactccgctcactacaaacaaatccgactaaaaaaacgccccttggttatcaaaaccaaaggacgttaagttcaacgtggtaccaccttaatttgagttgtcttcacaaacaactcctcgaagcgtacgggaaaaatccgatacgccggcacgttaatgggtgctaccattccacctcgaaaagtgaacttattttgctcgatctttcaattcatagtcttaatgccctcacaccaaccaggcactctcttggtaaggctgtaaatctaatccatcggaccaaatcaattagtcgtatttagatgttgcatgaactatagctcatgaacggagaaactgtcaacaacttttttacacttttatgagagcagtctcatgaaaatgccattttatcaaggggttgagcggcttaaaaatttttgagaacttttgtaattggtggtcgatttcggtatactcgatgtatcagttagattgattggaggtgaattgaatgcgggcattaattggttttgccgggttaatttcgatggtgatgtgtatcgctgccgtgattttcttaatcatgggtaatcgaactgtcgctgtgccattggtgagtgttggattggttatcttgattgtctgttatgctgcagcaacatacatttctcatacggataacaaaaaatgagattattttaatacataagttgaaacggagggctgctgcatgctgatgattagaacaattcgtcaaagtgactattcaaacgtcagtaacttaattcgaacagcatttgccaacaccgccaatggctatcggaatgaagccgaattggttgataagattcggaaagagcccatttaccaaaaacgattggaagtcgtggccgaaaatgggattcacttggttggctatggcttgctgagtgaagtcaaggttgtcgatggtgccaaagcatccacagggttggtattagcacctttggctgttgaacccggatcgcaaaaatccggtgttggcagtttgattatggcgaactcgataatcgggcaatcaaccttggctatcaattcaccgttgtgaccggctggccggattactatcctcgctttggttatcagaaggccagcgattatggtatcaagtctcccacaccggttccagacgatgtcttcatggctaagccattggttgacggcggcttggatggtgttcatggaatggttcagtactcgaaagcttttaacatgtaaataaaagcggaaaccaattgcaaacatggtttccgtttttgtatcgattcaattatttaacggtggtttcattttcagacgcagctattttgttttccgtaactgcttgggtggcaagcttcaccaggaattggccatacttgatcaccacaaagacgaccataaaggttgccagggtgatttccaggtttgcgatcgtgccaatgattgagttgagaccgtttcccaagtggaaactgttattaaacagattcaatgcagtggcagaaatcaccaaggggaatgtaaaggccccgaaactggggtaaaaggctaaccgaacgtatttaaagatcttcgtcagggttccccaatacaacccttgagccaggatcaccattgctaaggcgaatccccacgatgggttggtattcatcgacagataaccggtcaggcacaatgatgccggagcagccataatcgtcaatagcggcaaggttgcttcaaacataaactcccgtcgaagcaagcgaatgcagacaattggcaatagaattgcgtagagcccaagagacagccacaataccggtgtcccaagtgccggaatgaaattatttgcggtaaccggaatcactccgattcccacaaaagttacgaaccaacttggataaacatgatcgagttcaactgtcggacgtagcaaatggcggtagataaaataacccataatgacaaattgcaaaatcactgcgaacgtccaaacggctgtgggtaatactggaagcccccatgatttcaggaatgtactgataatcatcaaagacatcgtgaaggttggggcaacggatgcaataatcgggtcgttcaagtcgttcagacttaatttaaaatgaacgccaatctttgcgatcaccagtaaaatcagaaccagggcaagaatcccccagacattgccaatcactggtaagccaattgccttaaacaggtttcctaacgaggcaatcccaagaattaatccacaaattggtaaaggtaacttcttcaaaaataacttcatacggtcgtctcctctcttagatgagcttaataatatcatttatggtagaataaataaaattgatagtattaatatttgttataaaccaaatttataaggagtgccaatatgtttaaattcctggaaaccttcatggttgtctacaaaacccgcagtttttccctggctgcccaacagctctttatcacgcaaccaacggtgtccaaccagattaaacaactggaattgcagctgcacaccgaattgtttgaacgaaaaagccgccgggaaattgtgcccaccgaagctgccaacctgttatataaacgagcaggcaagatccttaaaaactggcaggatgtcaacgatcaaatcacccgcttaggtgataaaggaaatgaaaaagtgatctttggcatatcgcaaaccgtttcgcgaatcttgtttgcgaaaattgccagtgctctggtaacggccgatcctaccctcgattttgatgtgactgtctccaactccgagggcgtcttaaaccagctagaaacctacaagattgatatcgggatcatcgaaaagccactggttaccgagaacatctcccgaatttcaatcggtaaagatcagctggtcaaagccggcgtggacaacggcaattggatcactcgagaaccaggatcgggaatcggctattataccgaacagtatttccgtgaagccgatgtccagcccgccaaactgatccatgtgaataatagtggcctcattcgtcgaatggtggcaaaaggtgtcggtcaagccctgttgtctgacaaggatctacctaccgctgttccgattgaatcacttggggaacatttttcccgtgatttttatttgttggtccgagaggaaagcagtcacgacaacacgttgaatgacattcaacaaattatccgcagagcaatgtcttcccccaatcaagattagttctcgtccaaagtacgcgtccgagttgctaatgatttgaaatgatcatacgtcatctttagtaattctttgggtgcagcatcttccaggattttaattttatccggatttgcggccggtcggtccttatagatctgactgttaacatgatgggatccctccagcaaaataaaagccaggtccgtatcagtattttcaattcttcgataaataaaatcgccactacgttcgttgggatccaaaacatcgatattaactccaaatggttcaaatacccgtttgtagctaatctgcttgaaccatgaaaccacttcaatattcttaccggtcaaaacatctttcacatcgggataatcgattgtaaaccgctcaacaaacccttttgccgataatttggcggcttttttcttaacttgatgtaattcagcggaacgatcgcgattttccgttgatgcagcgtaatgtttgttaatcacaaactgatcggtggttaaattatagttcccgcgatatacatcaccttgattgagctcaaatttatttcccttcacaaccggattcgggaacaccgatccatctaaagcaataaactcaggttggtcgtcttgaaagtggacgtagccatacatctgttggttatcttttagcaactctgatcgccgcagatgaatcttggtgttggtcatccccgtcttcaaataataatcaatcatgttaaaaagcggcagtaacgacaagaattcacccactcgttcctcgtcaattctggcaaataattcgttgattaactcttgggtagttgcttgtcggacgagttttcctttgcccggcaattcatagtgccggtattgatggagctgttcttgatacttggtatttcgtttttccgagctcttcaagtgagcacttgttttttcaagttggtccttgtaatattgcttatccgctttaacctgctgagctttctggtactgtgagcttttaataaaatggcggatgccggttcgcagacttcgattgcgcctgttgagtaattggatttgctgattaagttggtcaatcgtttgtttcaactgcatttgggtatgatagtcagttgcctttagttggtcggcttcttgaagtttaatctgggcattatggactttgccctcaagttgatcatttgcttggtttaatgcaaagttttttgctttgagccgttgcattatttgctcttgggcattcttctcactttgaatagcccgaacttttttctggagctttttattctcccgttttaacctgctcttctgtcgatcgttatcggtgtgctgcggagcttgatttgtttgctgaccacgatttgtggtggccttttttaattgggtttgctttttctttgcctcttccaaaattctgtggaatctttccttagcctgttgtttatccttatctttgattgctttgatattcattggcttaaccattagattacctctcacccgttccacattgtaaagttgataaattaattgtaccaaatttcacccctgatgactcgttaacataaacgaattgaacaaaaataagctgaaccacaaactcaccagatccaatgatcaaagagtctatagttcagcttatttgagtagataccttctttaaattaccatcttaagcctggtcgcacttacagcagcgctccggtagattttttcgatggttttttcgtaatcactattggcaacgccaaagacgactttaatatcgctgccttcctggaccaccaaatgaatcttaatctgactgttatccaaaaggtcgagaatcttaccagcgattgccgggcgtttactaagttgggaggaaaccgccgcaaccatagcgatgtttttctccaatttgacactgtctaaatcgcaggttgacttcagtgagttgacaatcgccatcaatttgccgtcaacatccgtccgcttcgccaaaaattgaactgaatcggttccggctgggacgtaatcaaatttgacgccaaacttttgaatcacggagaagactttggccatcacatcaaggcgtttgttcaattgatacttttggatggaaatcaccacataatccttcttaccggcaattccagttaccaactggtgagcgttactgttcgcagaatcgactaccagggtcccatcttcttcaggatgattagtgtttaaaatggcaattggaatctgcttttctttggcaggttgaatcgcctcttcctgaaagacgctgatgcccatataggacagttcttggagttcttcataagttagttcggtaatcttgcgggagttattgataatccgaggatcagccatcttaatgcctgacacgtcagtccagttctcatagagatcggcatccacaaagttggccaacagcgcaccggaaatgtcacttccaccgcgaggcatcaagtgagtcaaaccgtcttcatcaaccccatagaaaccgggaacgacgatgtggtcatcgtagcttaaaaagtcgcgcagacggttaatggattccccatagttgacgccgttttggtcaaataccagaaagcgggcagcgtcaatgaattggtagccaaggaaatcggccattaatttggcagttaaaaattcgcctcgtgataccaaataatcatgactgcagttaggaatctgcttggcaattttctgcaagtcggtttcaatgcccaccttcaaaccaagtgcatcccgaatgccgacaaatcggctttggatgtggttatacactggcatgtaatcttcaccggcatctcgaagtttctcaacttcaattaataaatcggtgactttaatcgcctcactatcactcttacctgcggcactcaccacgattacttttcgatctgcatttgcttctacgattgcccggacctttttaaattggccggcatccgcaactgaacttccaccaaatttagctactatcatttttctgctcctcctttcttagttggtaaacttgccataaacgcggtttcatcgcgttgtaacactcgtctcatcttttgatgcatctcaccgactggaatgtcatgaacgaccagatagtcaccccgaagttccggggcatagtcgccaaacagctgtgagcaatcaatctctgatcggacaatgtaattattccgggtcaggttcggctggaacttaaaggtactcttaaattcccgcttcaaatgttccttaccttggaaaatatccaagatatcttgaatcacggcgttggcagttggcagttggccagctccctgacccatgaacttcaaagtcccaatcgtctcgccaatcaatgaaatcaaattatagttgtcacgggtgtgggcttcgagggtgtcgccgtagtacaaggtcggctcaaccatgtagtcaaactcatggccccgctggtgactcttacccatcaatttgatggtcatccccaacttgtcaaagtgagtcatgtcatcttcggtaatgttacgaatcccaaagattggcaattcctcggttggcttgataaataggtcgtatgcaatatcgacgctgatacataatttgttggctacatcgaggccgtcgatatcggcacttggatcggcctcggcgtaacctaattgttgggcctccatcaacacttcgttgaatggtttgccggttcggtgcatctggtcgaggataaaattactcgttccattgaagattccttggatcttattcacatcatcgacccgtaaagcccgctccaagccttgaatccagggaatcccaccaccgacgctggattcaaaataaaattttgcgtcgttttgggcagccactctcgtgaattcatccatatactgagaaatcactgctttattagcggtaataacgtgcttatggtgcttcaaggcatcgactatgtattgatgcgccggttcaatgccaccgatgacttcaaccacaacatcgacatcttgatcgttcaaaatttcatcaatgctgtcagtcatttccggtaaatccggttttttattctttctgatcaaaatatgctttacatggaggttttgggcttggcgcttcgcattcttaataatcttgtaaacgccggaaccgactgttccgaatcctaatatcgcaatattcacagctgaaacctccaattttttcgtgttcacaaataataaacacttgtatttaacatgaaaacagattatcatataaatcatagaaatgcaaggagtaagttgatgaataaatattatacgagtaccagaaacggttcagttcaaatttcagccaagcaggccatcaagaagggcttcgctgatgacaagggtctcttcgtttatcctgacttggaaaagctccaagtaaacttcgaaaaattgttaaaattaaattatcaagatattgccagagcagtgctgacgattttattgccggacttttctgccgatgaaattgacgaaagtgtccgagcagcttatcagtcaagttttgacacccaaaagattaccccggttattcccgttgatgatttccatatcttggaacttttccatggaccaaccagtgcctttaaagatgttggcttgcagctattgcctcaattgatgaagcacgtgttagtcggcaataataaggtaatgatcctgacggctaccagtggcgacactggcaaagccgccttggaaggctttaagggcttggataacatgggcattattgtcttctatccagacggtggtgtcagcaagatccaaaagctgcagatgatcacaaccggtgggaacaacaccaaggtcgcagcaattgaaggaaattttgatgacgctcagacaaacgttaaacggattttcaatgatcaggcactgaaggaatcccttggtgacgatgtcagcttatcaagtgccaactcgatcaatatcggccgactgattccccaagtcgtttattattttgattcctataaacagttggtcaacgatagctcgattgaagtcggccaaaaggtcaacttcaccgttccaaccggtaactttggtgacgtcctggccggctactacgccaaaatgctgggccttcccgtgaacaaatttgtcgtcgcatgtaatgaaaataacgtgttggccaacttctttaatcacggggtctacgatcgcaaccggccatttttccagaccgttgctccaagtatggacatccaaatttccagcaactttgaacgactcctctactataagagtggtcaggacaccgaatacgttaaacaattgatggatgacttggaagacagcggcaagtatgaagtttccaaggaagttctggcaaatatccagcaggatttctactgcggctacagtaccgatgaagatattgaacgctcaatcgccgaagtctacgaacaaaacggctacttgatggatccccataccgcggccggctacaaagtcatgcgcaattatcaaaagctcgaccccgaaacaccaatgatcctgttaagtactgccagtccctataaattcgtgaatgcggttgccaatgccgtccttccagaaacttcagcggacgtccagcaggtgatgcgggacttacatgacgcaaccaacgcaccaattccagacaacctgagaaaagtctgggatctgcccgtccgtcacgaaagcgtcatccaaaaagatcaaatgaccgattacgtcaaacaaaaagtcgaggaggtattttatgatcaagatcaaagtgcccgcaactagtgccaacgtcggggttggttttgactgcctgggtttggcagtgtcctattattcaaccattacttttgacaagagctcggagcacttggtcatcaccggctccccgaaagaatttcaaaatgaagacaatttggtctaccaagcctttgtgaagggctgcagcttcttagacaagcccgttccaaatgttcaaatcgacattgaaaccaacgtccccgttgcccgtggacttggtagttcatcgatttgtgttgtggctggcctaaaagccgccagcgtctggtacgatgacgcaatttcggtcgaccaactgctggtcttggccaccgaaatggaaggccatccggataacgtcaccccggccattctgggtggactgtgcgtctcctttttagatgaccaaaatcagcctcaggttatccaatatcacgtcagtgacaagctgcactttgtggccatgattccggattacgaagtcagcacccatgctgctcgaaaagtgctgccgacatcaatgagctacgcagatgtgattcatcaagtcagccactgtgcggcaatgactaaagcactggaaatcggtgatagccatatgatccatgttgcctgcgatgaccggatgcacgaaccgtaccgggctcaattaatccccgattacagtcaggccaaaaacatcaccgaacaattgggtggtacgatgtacattagcggcagtggttcaactatgatggccatcaccgcagacgaaaaggatgccgatcaaatcgctgccaacgcaaaagcggccttcccaagatggaatgtccgcaaaatggcagtcgattcaaccggcgtagtgagtgaggtaagtgaacgtggaaaagtattacatcgttgatagctcgattctcccggaatcatttgataaagtgattcaagctcgtcaactattggagagcggcaaagtcaagcaggtcagtgaagccgtgaaagttgtcggcattagtcgaggaactttctataaatacaaggatttggtcttcttaccggaagaaaacatgatggacagaaaagccgttatctccctcatgctggaaaacaagcgagggatcttatccaaagtcctcacgaccatttctgaaaccagtgccagcgtgttgacgattaaccaaaacatccccatccacaatattgccagtatcgtcatctcattggacctgagtcattttaccggaaccatcgataacctgttgggaaaaatccgcttggtggatggggccagtaacgtccagttagtttcgatcgagtaagtatcggaactctgcgtatgtcaatcagatcattgtttcttaatccttgatagctgctatcaaggattttttatgtattcatgatagaaactttcaaactgtaagcccttaccagcttgaaagttgtttcacagtccgcatataatacaatattgtatgcatttactgatttaaaaagtattctggaggaaatcatggcaaacagccagcaaccaaacgcacccaaaaaattccatttatcacaaaatcatcatatgacgattccctggaaatcattcacgacggacgaatctgtccccgccaaagaagccggcttgagggaacgggcttctatcgttggtagggttgggattgtcatgctttcctgtggaaccggagcctggcgggttcgtgacgcaatgaacacggtggccagagtgttggggctgacttgttcggcggatatcggcctgagctcacttcagttcacctgttttatcaacgaccacagttattcgcaggtgctagcactgcctaatactggtgtgaacacagataagctcaactcactggaacactttgtcagccattttgaacgggattttggcaatgcgacggtcaaacaaattcacgccaacatcagcaaaatcgaacaacgacctgtccagtacagcccgctggtttctggtttggcggccgcattggcctgcagcggttttatttttttgctgggcggcggcatccctgaaatggtttgttctttcattggcgccggtgtcggacagtatttccgggggtcaatgggtaaacaacacattaccacaattgccagcatttccattgctgtggccattgcgtgcttgacttacatgttttcattcaaaatctttgaagccaatttccaaattctggctcaacatgaggctggctatattggtgccatgctgtttgtgattcccggctttccgtttattaccagtttcctggatatttccaaactggacatgcgatccggactggaacggatggcttacgcgatcatgatcaccgctgtagcagccttagtgggctggctggtagcactattatttgatttccgaccagaaaacttcttaccattgggactatcaccactggtattgatgttattgcgaatcccagccagtttctgtggggtctatggattctcaattatgtttaacagttctcagaaaatggccatgacggccggactaatcggcgcggtggctaacaccttaagactggaaatggttgatctgacgagcgtcccacctgcagccgcagctttcatagcggccctggttgcaggactgattgcttcactggttaaccggtataacggatacccaagaatttcactgacggtgccgtcaattgtcatcatggtcccgggattgtacatttatcgggctgtgtataacatcggcctcaaccaaattagtgtcggcgcattgtggctgacaaaggctgctttgatcatcgtcttcctgccaatgggcttgtttgtggcaagagcgttaatggatagggagtggagacactttgattagagtgcggagagcaacgttttgacacggagagctaaggtcgctttgattgaaatcctgggcttggatttgaatcaaagtggcttagatcgcagtgtcagttgctcgcagcacatttcaatcccagtgcggagcaagccggttagcttttgagcatttatgtaataataggtgttgatgcgcactttgcatcaatgcctattattggataaagcggagaaagctggcttgtgcagcacacctcaacaaaaagaaccggaccctaccaaagtggcgtccggtttttttgactcaaaatgtctacttaacaataatcatgcgtccatcatgcttttcctcaagcaactgatggcctttaacaaatccatctcgattaaatggcagcttgtagccgatattaatatcgagcttgccttcacgcatcaaatcgatcactgcctgcagagcctcgcgatcgctcatcgcatcagtcggatgaatgtgggcaaatttcaatggcttatctgtcattggtgagttatgggcaacactggcaatgacgccgtttggtttcaccatcgtaacgtcatcatcagttccggcaccattcattgcggtattcaaaacgacatcgccagtatccgccagctcagtggccgggtcagtctgatcataagcaacgaacttcgttgccccaatcgattcaacataatcttgattgtgactggaggcaatgccaattacattagcgccaatatcagtcgcaatctgaacggcaagtgatccgacaccaccagaggcccctttgacgatcactgtctgatcaggttgaacgttggcaaaatatttcacagctttataggcggtcagaccaggggtaatcagacctgctgcccgtgtcggcgtaatcccgtctggaaccacaaccgtggcgtctaaattaccaagtacaaactcagcgtagccccgctcagtgtgggtcatcaccagttcaccctcactgagatcggaaacccgcttaccgactttcacgatttcgccaaccacatctcgtccaggaatatacggtgacggcatgctgccaaagccgccggcacgttctgcacgctcacgattgtttaagccaacggcaattgttcgaatgagcacttggttggcagccggcgttggctctggaacttcatattcttgaaaaacttctggatccccatgtttctcatatccatatgccttcataatatcttcctcctcatttgtctaactagcgcaattgtaagcgcaatcacgagttcgagcaagtaagtcgaatcgaccccataatgtaaaaattgagtcgaaaaattgtaaacaataggtaaatacccacttttgtaggacattttatgtcatgcttaatgcataaatttatagggattggaagttggaatgatgttagatatcattaaagcaattattttaggaatcgttgagggaatcaccgaatttctgccaattagttccacgggacatttaatattagtcaacgaatttatcaaaatgagtcaaaccactcagttcactgacatgttcaacgtcgttattcagctgggggcaatcatggcagtcgttgtattgtatttccacaaactcaaccccctttcaccaaagaaaacccacgtcgaacaacatcagacatgggtactttggtttaaagtcattgtggcagtgctgccctctgttgtcatcgggttattattcaacgactggatggacgcacacttgatgaattggcaagttgtctcggcaatgcttctcatatatggggtattatttatcctcatcgaaaaccgaaatgcaaaccggcaaccgctattttccgatctcaatacgctctccaatcgaactgcctttattatcgggatgttccagctgctttccctggttcccggaacctctcgctcgggtgccaccatcttgggcggcattctaattggcacttcgcgatatgttgccaccgagttctcgtttttcttggcaatcccaaccatgtttggtgcatccctgctgaaagtctacaaatatttcagccatggcggcgcttttaccggtatgcagacagccgtcctgttgactggcatgctggtttcgttcgttgtggcctacttcgccattcgcttcttactgaactacattcaacataacaacttcaaaatctttggctggtaccgcattattttaagtctgattgtgattggttacttcggctttcttgcgcattaactctccaacggctgaccatccgccagattaaccttcaatagccaagtcaacatttccggtagcattcgctgccaatacagccaatcatggccgcctgcgccagtgtgataagcgattggtagctttaaatcgttgcgcatgtactgaacgaatcgatcattggttggctttagttcatcttggtcgccaatacagtagaagaagcgaagttgcctcagctgttcagatggcgacttttcagctaatgtttccaaatagtgctctggcgcgattctctcaagaatcccctgggcatccggcatcatcgctggcaattcgctcaaatcaactaccggtgacatcggcatcacggcactgaaccactcaggatgggtgaaagccaattttagtgctccaaacccgcccattgatgtgccgccaacgaagttatcctgtcggtcactggacaacgggagtagtttccgcatttccggcgtcacttgcttggtcaaataatcccagtacggcaggccattgtgcaaattcatgtagaagctacgattcatttcaggtgtgatgaccgctaaattcgtatatttggtcaatacttccaaattagttttacgaataaacccactgccattatcgcccaagccatgcagcagccaaagcacttggagttttcggtcactttgaatctcatttggcagaattacatgaatcgttgtctgttcctctaatcgggtccaagctcgggtcaaagtcaatattgccatctgcttctcctttgttggttattcaaacttcttgagttgatcgtcggcaatttttctcagtaactgtttatcagcatttttactcaactgatccgccaatttacgcagcctcatatagttcacatgggcatcggtgattgtgccggtgtcatcttgaatatctttggccaacttggcacttttattggccttgttgggcgcaaaatcggcaaagtaggttgacgcataccgtaaagttttcgagcgtttccgaacatgatgaacttccgggtagtccttaaaatcgagtttctcgaatagggcaactagtttgtgatttctacgattgagctccttgacaatatattggtgccatgcagtggtttgggtgaacttaagctgggttaactgctgctggacactttccaaatccttttttaaggttgcctgtgtcccctcggttaaggtttgtgccatttcatgttgccgattatcgcgtaaaatcttcagcaagccttgatagtcggccttcttatctggatgagcgtatgcgtaggtgcctgtctcttcaatcaagacgtcaagttcccgcaaatcgccaaacaaattggctgcctgactgagattgatatcgatagtggtataagttgcaggggtcagccgtcgcttcaagaatttaattaatccccgtaaggtacgaatcatgacccgcaaatcatgcgcccgctcgggatcgaacggattattcaaataacgaacccattcaacctcaatgtcagcatatctgttttgtaaaatcgtctgaattgacattggcttctcccccttttaaccgccagtcggcagactttctactacgtgagtaaattttaactttaatgtagcatattttaataatgatgagttaatgattagctgataaaatgggacgtaaaaaaccgggacataactaacaggtagttatgccccggctttctgtataatagctggtccattcggtcgataccgatatctccatgaatgatgaatcttattcaaaaaatgaattgaaaattctatctgccaaactgccaccagtgctttttcttgccggcttcttgaaatcgcgcattactcggctggtagctgtcaggaatcttatcaccttgaggctcttcttcatttactgattcgggaatggtttgcttaattgaagaagtgtttttgctttcaagctgcttaagcttattttgaacatccagctgcagccgctgtgattggtccaataattgatgcaattctgcgatttgtttgtctttggcatcaatttgtttgcgttggtcctcaagctgttcagccagcaatgcggtttgctgatcatcgctcttaactgctaactggttagcggttttcgttgactgcttgtcagcagtttcaacttggttcttgaattggcctttgagaacttcaacaccctcatctttgatcagaatcttgtttcccttttttatcgtatatgtatctctgaacttatcgtccatatgttttctaattgcagttttcgataccgataattcgtccgccaactctttgatagtcagttccataatgtcgcccccaacataaataatatagtttgcaaacagggtgtttgcagtcacacatcatcattatagtgattaacaagccgttcggcaaatgaattctgggtattccagctaatttattataacaaacatccttttaaaatgagattttaattagattttatgttgacaatctaataaaaaatgcggtaaactactcgcatgctgaatgcgaattcgccgatttatctacatatttgttgatcgaggaaggaaaccgcgatcgttttcgtatttacaaagtgtggtttccacaggacttggtttgtcattacgcaaagttttcgtttagcgcggatatttcatagagagattaggagtgattgtatgagtagtataaccgaaaaaatgtttcgaaaagaagatccgcttgtgtatcaagataaggattctcatttaattcgaagcttaaccactaaagatttcctggcacttggcgtcgggacgattgtttcaacttccatctttaccttgcccggcgttgttgccgctcaacatgctggtccagccgttgccctttcgttcttggcagctgcgatcgttgccgggattgtcgcctttgcttacgcggaaatggccgctgcaatgccatttgccggatctgcttattcatggattaacgttgttttcggagagttctggggctggattgccggctgggcactgctagccgagtatttcatcgccgtggccttcgtggcttccgggctttccgccaatttccaggggttgatttcgccattaggattcaacctaccaaaggcactctcaactgcttcaaccggaaacaacggcggcttgatggatttagtcgccatcatcgtcattatcttagttacctcattactctcgcgtggtgcttctcagaccgcccgagtagaaaatacgttggttattttaaaagtgattgccattttagtctttattttcgttggtgcgactgccatcaagtcagctaattacacgccatttattcctaagtaccatgtcaacgctgacggttctgcattcggtggctggcaaggaatctatgccggtgtttccgagatcttcctggcttacatcgggtttgattccatcgctgccaactcagctgaagcaaagaatcctcaaaagactatgccacgaggcattcttggttccctggttatcgcggttgtgttgttcatctctgttgctttggtccttgtcggcatgtttaaatactcagattacgcaaataacgccgaaccagttggctgggcacttcgtcaaagtggtcacgcactggttgccacagtcgtccaagcgatcgcggttgtcggtatgtttaccgccctcattggaatgatgcttgccggatcacgtttgatctattcatttggtcgtgacggcttgctgccgaagtggcttggcaaactggataacaatttgcctaaccgggcattgatcgttttgacgatcatcgccatcgcattgggcgccttcttcccattcactttcttggctcaactgatttcagccggaactctgattgccttcatgttcgtttcattaggtgtctactcacttcgcccacgtgaaggaaaagatattccaatgccaagtttcaagatgccgctatacccagtattaccggcactaggattcttaggcgctctgggtattttctggggcttggatattcaggcaaaaacgtacgcattgtgctggttcattttgggaatggtcatttacttcgcatatggaatgaatcactctactgcaacaattgataaaaaagctgaacacgaaaaagatttgtaaaggttggtgatttcatgggtaaattagacaaagcgtctaaattaattgatgaagaaaacaagtattatgcacgttcggcgcgcatcaattactacaatctggtaattgaccacgcacacggggcaaccttagtggatgtcgacggcaataaatacattgatttgctggcaagcgcatctgcaattaacgttggccacacccatgaaaaagtcgtcaaggcgatcgccgatcaagctcaaaaattaattcattacactcccgcttattttcaccatgttcctggaatggaactttccgaaaagttagcgaaaattgcgccgggaaattcaccgaaaatggttagtttcggtaactccggctcagacgcaaacgatgcaattatcaagtttgcgagagcctatactggccgtcaatacattgtttcctatatgggttcctatcatgggtcaacttatggttcgcaaaccttatcaggaagtagtcttaacatgacacgtaaaattgggccaatgcttccaagcgtggtgcacgttccgtatccagattcatatcgaacctatccgggagaaaccgagcacgacgtttcactaaggtattttaacgaattcaagaagccattcgaatcattcttacccgctgatgaaactgcgtgtgtcttgattgaaccaattcaaggcgatggcggcatcatcaaagcccctgaagaatatatgcagttagtttataaattctgtcatgaacacgggatcctgtttgcgattgatgaagtcaatcaaggactcggccggaccggtaagatgtgggcaatccaacaattcaaagacatcgaacctgatttaatgtctgtcggtaagtcgctggcgtctggaatgccccttagtgcagtgattggtaagaaagaggtcatgcagagtttggatgcacctgcgcacctgtttaccactgccggcaatccggtttgttccgcagcttcgctggctaccttggatgtgatcgaagatgaaggcttggttgaaaaatcggccaccgatggtgcatacgccaaacaacgtttcttagagatgcagcaacgccatcccatgattggtgatgtccgaatgtggggcctcaatggtggaatcgaattggtcaaggatcctaagaccaaggaacccgacagtgacgctgccaccaaagtgatctactatgcctttgcacacggcgtcgttatcatcactttggcaggcaatattctgcgtttccagccgccgttggtcattccaagagagcaactcgaccaagcgcttcaagtgcttgacgacgcgtttaccgcagttgaaaatggtgaggttaccattcccaaggatacaggtaaaattggctggtaaaatagcattattcaataaagcaaaaggcacgaatcccaatttgagattcgtgccttttttatatccattcttattgaccatgcctcataaaggctttatatgctttcaccccaaagtatactaggacgactgcgatcgcaatgacgatgataaaagtaatcacgacaaagataaaatcgccaacgtgaaaaatccctatattgattcccccaatcattaggattcaaaagtgccgtccgcacttaaattcattatgacatcaaatctgcagtattccatatctgattggttattttagtttaaaatccatgacttccggattatgatcagaatttttgaaccctaacgatttgacatgaacccgattaacctgcacgttgtctgaaacgatgaagccatcaattatcgacgtaaaggtctttcctggatgatacggtgtcccatttgcccgcactgaaggcacttttgcctgggctaatccctgcttggcaattctaaatccttttggcaattgatcagccgggaacgggtgcgtccaattcatcggtttactggtcgtttcaaagacggccgggctattacccaacatatcatggttatagtctccggcaacaatgacgtagttgcctgcctgctgctcagtagtcattttggcgaataacttattgatctgagcttttcttaccttggcattcttggtaaaggctgagagatgtaggttgataaccgccaactgatgcccattggccactgggatatgggtcaccgaaattgcccggtccaagtccatgaatttattaaaatcggtatcaattggcagctggtatcgggtactatctgcaatcttagcttgagcaagggtcaacaatcccgatttggctttcccgattggccgggtgagcggataaaacaggtaggccgaattatagttttgggcatagacgctcgaataaccattcatccgatcccttagccactggacttcattcacgtgaaatgaacggtcaccgtcggtatcgacttcttggaagaacatcaaggccggatcttcttgtttgacagcttgataaatgccgttgaggtcattcaagacagagaatttactaaatgcccgcgaatatttgccgccatccatgaagaaagaataattatccggataggcggcatagccaatattaaaggtcatcgccttgtaggggtgatttgtctgtaaaatttgcgagttccggttaaccggtttgagtttaacgttgtcgggcacccggtgatacgtcagataaacgtatgccacatatgcaccgacaacgagtaatagaccggaaccaatcagtaaaagtgttttccagaattttttcataagaccctccatacctaatatcatatcaaatctacagccgaacaatctaaaaatattttcaaatattggtatcgtttacaaggctttaatgataaaatttaggtatatttgttcatacttttaggaggggtcaatcatgaagaaatcacatttttggtttgcacttttatttgccggggcacttagtattggggtggggacatcttcgcaaactgtttccgccaagacagttaacatttatttaacccgtcatggtcagaccatgttcaacgtcaacggacggggacaaggctgggctgacagtccgctaacggataccggggtttccgttgcccatcaactgggttacggcctttatggcttgaagttcaaggctgcctattctgctgataacatgcggacattccggacagcaacctatgccttgcagtcatctggtaacggcaacctgaaagttaactggactgccaatttacgtgaaggcggctatggtagtttcgaggggcaaaaatacgatgacgtcaacaaaatcaccatgccgctgttgaaaccagccggtacttattcaggcccacaagactttggcaaagctcaacaagcgcttggtaaagacttctggccggcacttcaagatgcgtaccacgctgccgaaacggtcgactttggtaaatacagcgacccaactcttcctgaatcattgaaagcagaaagctcaactcaagtaatcgatcgaatgaacaccgagttgacttatatcgcccaaaaggctgaaaaaaccggcggtaacgtcttagtggttagttctggaatgtcaattccggagtggttgtccactcaaaagaactatacggttcctggtttcgttaattggggaaatgaagcaaccatgaaggtgacttataagaatggtcaattctatttcccatcaaatgtcaccgacaagaccatcctttataccatcaacaagggagcagctttgcagcaacttccaaagaacaccctcaaggtcaacaagttttatttgaacaagaacaaggtttccggttctacttccaccggggcgtcactggtcttgcaaaacacaaagggatcaaccttgaagaaaaccaacgcaaactcaaacggaaactttgtgtttaagttaagtaaagccactttgaacaaactcaaaaagggcatgaatcttaagttgacctcaacccctaagaatgcttccaagtctctgaatatgaactctgatcaaattagtcaaactgtctttggcaacaagacagccaccattaaagtattgaagtaaaaccacttaaaacaagttcatgaaatatttaaaataggagtccagaacaacactcttgttccgggctcctattttttgcgaacattctgtctttgaatttttaagttacacagcaagcgtgaatgaatcttaaaccacaatcttctttctcaaaaaggtcatcgacagcaacagcagcgaagcgcaaattaccccccatcacgatattaatccaggcaattgcggccactggcgtcgattcggccaaagacacaatcaccatgccaacactcccgaaaatggttccaccggcactgtacagggcagaggcggatccattatcgttttcctcttgtttcaataccaaataagttccgggtggccggaccgcactgctggccagggttgctggaaattgggttaaggcaaaggcgatcggtgacatccggccgaaaaccatgactaggatgccggcaacgatcgtgaacccaaaagctgtatagacaatcgtaaaccggtcaatatacttggaaagcggaatatagaccagtggccccagcagcatgccaattgcgttaaacgagaagaacaggctaaacatccggctgctgaggtggaacgtattttggaaaatgtaggaagatgaggaaatataggataatgacacaatcgacatgagtgaaaaagtgaccagaagtgccgtaaaaccgggattaatcagcagtgcacctaaccggccaaatgatttcatgacgctggtagtcccacgttctgaagcatgagtttccttaaaaataatcgaaccataaatcactgagagtcccagcaatgcctgggcgaaaaagatcccccgccaggaaataaacgtcaacagtaacgacccaatcaccggtgcgaccgcaggtgaaatgaccaccatcgactgaacgatggccaacgtcgtttcctgttttcgaccaacaaagacatctttgatgaccgccgtggcaaccgtcgtcgcaactccaccaccaatggcctgaagaatccggaagaaaatgatttcataggcattggtcgcaatgccacagaggatactagctaacatgtacaaggtcaagccaaccaataaaatcggtcgacgaccatatcgatcacttaacggcccccagaataaagtggcgatcgaataaaacacaaaaaatagaattaaagtcaggttcatcacaatttcgggaaccgcaaagaacttggtcatctccggaagtgcgggtaaatacaagtcggttgaaagcggcacgaaggcactgagcagggccaaaaagatgataaaaccggtatttcccattcttggttgaactttactgtctgccatctttgacacctccatcctttgtccatttcatattaaccgcaaactcatcggtaacctgatcgagttcgtggttttcttcttgaaaaccttctttaatgtaaaagtgataggcacgcgaatttttctcatagactgccagcgttaattcggagcgggtttgtttggcagcactaagtagatgtgacccaatcccctgaccgcggtactgcttggcgacaaacaatccggcgatgtagttcccttctattcccaagaaaccctgaatttgaccgtcctccgtgtaaataaacagttcggctttggcaagttctcgtttcaccccatcgtaatagttggtccagtaagttggattgataaacgaatgggcgtccagattggcatccaaccagatttgggcaatttgatttagtttttcgcctttcattccttgaacatgcccaatcattgttggtccactccctatcaaggttcttttaatctttattgtaaaacaaaaatggcattccaaggtggaataccatttttgatttcatgttatttgacaatcttcacatatttcgtatttccggtaatgtacccgccggcaacgtgatacctcaaagcgccatgattagagacactgtttgcatgtgagtaatcgtagttcttgatcttaatcttggtgcccttcttgaaggaagtgtgacgattgcgcttactcaagttcacatctcgataacggtagattgcttttttaactttgatataccggggttgtgcttgtttatccatggtgaccagtttccggttcgcggtaatgtattggccgtttgtcagtacgaatcgggttgtcaaattgtgcttaacaattttggtaacatgaagaaccgtgccttgtttgtagtttctggtcttggcagtcaaattcttgtacatataggcattgaccccgcgcggattaataaccgtcacggttgagtgcatcgtctgataataaactggacgaacgtatgcccactgtgcggtgatataacctgtcttgccacgattcttagttaagtggttcacatcgcgaacctggtaacgaaggcgaccatttgcggaatgaccgtatccagtgacaacaaacatcggccggtaaacgcgcggcttggaaacgtaacctgctcggcgttcatgagtactaaacgtcgtattttggtagagataaattttctttaacgcgtacacaacggtcccttttggtgcgggtgtcgggcttggtgcgggtgtcgggcttggcgtgggcgtcggtgttggagttggcgtcggggacggatttggatttggatttggtgttggggtgggcgtcggtttcggcgttggcgttggggtgggtgtcgtgtccttggcaacatagacagtcaatttttgcgcctgattcgtccaagtaaccgtattacttggctgggcttggccagattttaattcgctggcatttgcataatgataaccactaggaatgttacttatgatctgactcccaatatcactggttgagttcagtgtgtgagaattccccaacagtatgaaactatccaaactggtgcttggggcattgacatctacataggaaacattaatatttttagattcgcttgggttggcattattgataatgtggaatttggctggaattgttgctgattcattgccatctttgtttaccgcggtaatattcaaagtatagtcacccgccgcaggggactgtggatcaagtactggcgatccatttgcatatgccgccttgaatgtatagcctttagcgatatcttttgattgatcggccacattataataattatcataagcggcttgcacaaattggcgaatgaaggcctgcgacgtaacatccccagcaataaagccgtcttggtcagtcttcgccaggtcaaatgttttttcaggcttaacttttaactgtggggtgtaaccaacgctgtcagggttcaggtattttaagaatgccttgtgatcagcaatcactcctggattaccaccagtagtagcaacatgtgacaccagatgaaccgtgtctttggcaccattgaccccgtcacccgtcaaactatagacggtctttgtcgttccaatatagaacaacacgttgattgtccagccgggcttgaaatatttctgattaaggcgcgtcagttcaatccctttgccgtcagaagcttgtttgagcgtataatcacccgaaggaatttgataatattgtgcaggctgattggtctttgaataagaatcagcccaaacttgaacaccagaaggatcaatcttgtgattatcgccatcagccggtttaattacccaatcgattgaatcaggcatattatcagcaactggaaacttgacttgccccgtgacactcattgcatcctgatagtgataataattcagagtcgtttcatcagttccaaccgacaatccggcagcattgttgacccacccattgttagtgatattgttggtcaaattggcaaagccattgaatagcgcttgtgacattttaaactgtgggtttggtccacccccattgtctgaactactcgagatattgattgtggttggatcaaaattaattgggtgacccggatcactattcaacttaaaggaaggagttactttaacgccatttaaatctgtagacgtgttaataaccccattgaccacagcggtcatctgctgaattatgtttaacttggcagcatcatctgtgttgacctttaagataatttgattgcccgaatgactcaattcaaagtcatcttttgttagccatgacgttgcactggtatctgtcggtaactcgaacgtaacggcatcagaattggtactgaaaataggagctgaaaagttcaacacgaactcatcacccttctgcagtcgctgcttctgctgtcccggaacattcaacgataactgaaattggacactattgcctgaatataaggtatcgttatttgaaaagttttgcttgtactttagaacactgttgtcaacaggcgtataagtgtcacccgcagcagctttagcaacaccgttaaagccggcgattaaaccaaaagtcaagcacactagtccgacaatcacccatttcaaacgacgaactgttaaattatcatttctgtcttttaccatataaacattcccccaaaataatccgcatttccatatgttcattgtaatgttatggacgaaccatttcaattaacttcggaggattcaaaataccaaggagaatcagttaatccgctaaaccacaggatcttgcggacttttgtcccgttttcatgtacaattgacttaaaaataaggaggatttcccatgtcaacctacaaaaacaaagtctaccttgcatccccatttttcagtgatggtcaaaaagatcgcatcgcccaagtggttgccttactcaagcagaacccaaccatcgatgctgacggcatattcattccccaagaccaccaattcgaatccgaacccttcggcagcttcaaatggcaggacgccgtcttcgcatccgatatgcgccaagtacataaagcggatgtcgtcgttgctattttggattatcaactggaagaaggcttaacggaacctgattcaggcacaatctttgaaatcggctcagcccacgaggccaacattccagtcatcatggtccaatttggtgaaaatggtcaattaaacctaatgttggcccgcagctacaccgccttctttaacggcaaagacgatattcaaactctcaaggattacgatttcaacaacctcgagcaaaaatataccgagaaaaaagttctttaatgatatgtagaaagacaactcaaaaaggaagtgaaacatcaggaacatcctgatggctcacttccttattttagttaatattctttaaaatgaaaatgaatcaaatcagccaactaatgatcactcggcacaccattttctaccggcaacgacaaatcagctttgtcatcggcaggcaacagatgaattgcatgtttcaacaggaacggcgcgatcagcgttgacaaaataatgaccagaatcaaatctgaataatacgaatccgacagtagtccagaggagaaaccgatttgagcggtaatcaaccccatctcgcctcgagaaatcatccccgaaccaatcatgtaactactgttgaggttaaagccgttgataattgcgcccagcccgcagccaaatagtttactgatacaggccagaaaggtcaagacaccgacaaataacagtgagttgccgatatttgcgaacgacatgtttaacccgatactgacaaagaacattggcacgaataccgcgtagccaatcggttccatgtgattctcaatcgtctctcgataaggggtatgggcaacggcgatgccggcaaagaaagcaccaacggcaccgctcaggccaacggcttcagcgatatacgccattcccaaacaaatgaccatcgaggtaatcgtgacgctggaggccatgagcaggcgctcgccaatctgcatcagataaggaacaatccacttgaccatcaaataggttagggcaaaaaaggcaatttgctcgataaaaatcaaagcaagattggaggatgaatcaccggttttaacaccggcagtccccatcacgctaatcataatcgacaggagaatgacgccgataatgtcatcggcaaccgcagcaccaagaatcgtcgctccctctttggtatccaaggacttataatcccgcaatacttcaacggagattgagacgctcgtcgcgctgaagacgacgccgataaagatggcttcaagtggcgagaacgagaatgcccagcaggccccgccaatcatgatcacggggaagatgaccccaataatcgcaacgataattgccggtcgcaaatattttcgcagtaatttcagattactttccagcccaccgataaacatcaagataatgacaccaatctgggaaaacagattaatcaaattatccaaatgaatccagcccagcatggccggaccgacaacaattccaaccaggatctggccgataaccgacggaatcccaattcgattcgccaagtgcccagccagtgtcgtcaatatcagtaacagacacagggcaccgataaacgccatgtcatgacctcctttctcatgatacttatgtgtgtataatctattatatgtgttttaggttctatgtgaatatgtgtcgacaaattagtcgttttcgatctgagttgttttagcgcccatcatggcaccaatatagtgaatggctaagccaatgattagtccgatggcggctggcaacaaccagtccatcccaagtgaagcgccaggaagaaagtcatctaatttcaaaattgtgctagcaaatgcagacttggaaataattgccggagctgcggcgatcgcatccaaaatcgctgggataatggtaaagatggtcgtccagatgtatacccgacggtcatgattgaacaatggtgaggcaattgagagaataatcagggtaatggcaagtgggtagaggaacatcagcattggtgttgaccaggcaataattgtatcaaggccaaagttggcaattccaaacgacattccggtggcgatgattaaccaagttcgataagaaattgatgggaatttagcatgcaatgcttctgagaatgaagtcgagagtccaacagcagttgtcaaacatgtcaaggtggccatcattgccaagagaatttcaccggtgatacccatgaaatgattggcaatctggttaaaggcaatcccaccatcaatggataacttaaaactaccaaggctggtagcacccaaccagatcaacgcgatataaataatggcttcaagcccgatgcccaaggcaccagatttcatagtggtcattgaaatttctttggcactagtggcgcccaagctcttaatggcggtaacgatagcgatcccgaagagtaacccggcgatacaatccatcgtgttataaccttgcaggaaaccgttgaaaatcgaaccattttgataagcggcatccgtaattggggcctttgaagctgagctgattgggctcatgaatgcaaacgcgaaaatgatcgcaagtaatgctaagaatgccgggttcaaaatttttccaattgagttaataattccagtgggtttacgtgatgcccagaaggtgatcccaaagaaaatcagtgagtaaatcaacagccacattggttgttgtgttggattcaaatggctggcaaaggcaatttgaaatggggttgtcgccgtccggggtgtcgcaaataagggtccaagggtcgcacaaaccaataccatgaagaaagtcgcatagcggctgccgattggtttggcgagatcataaattccgttactgtgagtaactgcaatcgcaataatagcaagtaaaggcaataatgttccagttaacagaaacccgattccagcagacatccagtgagcactagctaattgtcccaagtgaattgggaaaatcaagttaccggcaccgaagaacatcccaaacaacattgaaccaataattagataatgtttaaatgataatttctttgtattattttccatattaagcgctcctcataatttatatacgctaaaattcccattattttatgctgattgttggtgactcgactgatgccgcctgacttgcttcgatttaacatgattctcattttgaagacctccttaattgcacttgaatttacactttaagtgcaacactaattaaataaagaatggcccatggccaaatttctgtaaaatgatgtttgcgaaaacaatcatgaaaggaatttaaccatggatcactacaagcatattaccatagatgaacgggaaactatctttttaatgaggaatcatggaaactcacttcgtgagattgccagccatatcaagaaaagttactcaaccatttctcgagaattaagccgtaattctactggtaaatcctattcaccttcgaaggctcaggagaagtacaaacagcgcaaaggcaactgtggcagagtctctctcttgagtaatcctcaggtgtttgaagtggtgagagaacacttctgcgaagacctttggtctccggaggaaatatcgaatcgcttggcagtcgaaaagtatccggtgcagatcagtaccacgactatttaccgtgggattttcaatggcttatttgataatttgtttaaatctggcagctctagtgccgtgcgccatctaaggcatcacggcaagtctcgccacaataaagcttatcaagaaaagcgaggcaagattccaatcccaaacaagattcatgatcgtccgcgagaagctgacaaccgtgtagaaattggtcactgggaaggtgataccgtgttaggcaaaagcggaaaggcttgtgttgttacattggttgatcgaaaatctcgttacctgcttattggtaaagctgctaaaagaacttcagaagcagtcacggatactttgagcgacttaatgaagctatggcctggtagatcgttaacgattaccccggataggggtaaagagtttgccaaagttcaatgtttaactgataagtttggtacgcccttctactttcccgatcctcactctccttggcaacgaggaactaacgaaaatactaacggcttgcttcgcgaatatttgccaaaaggaactgaccttgattcaattactgaccgccggatacaagcatatgcagaacaaatgaataatcgtccccgtaaatgtctcggatggaaaacgccttatgaaatattctttaatgtcgtgttgcacttaatttgacaattcaagcaaataaaaaacgtcccttaagatcgatacgatcttaagggacgtttgcacgtgttaccacccaaattctcgacagcttcacaactatcgactcaccatgtacggccgaacgaattcagcgatacactggcgctgtaatgggcgctcccaacaaacactcgcagactcgctcgcatttgtcgctcgaaggctactttcatcgcttaggcttttgaatcgttctcacttacccgattctccctgaaaaagttctaagagactactctccttgtcttagcaaattctaatgtttctgattgacacaaatactaatacgatttctgatcgatgtcaaccagttttatttaactaattttacgttatgggtggtataggctaaatgccaaccttttggtaatgattgatgggcaaatttaccggataatttgttggatttaagaataaccactccggatttaagacctttcacatctttcactaccagtttaccgcctagtttagcagtaccggatacggaaaccttgtcgccagagttgaggttcaagctgcctttgccactttgcgtgtaattacctttgaccacaacattcttggcagagagggttaagttaccacccgctaaagtcaaactgccgtcacccaaggcgttgtcattttcagctgccagggttcctgctttgacagtggtaccgcccttgtacgagttatttccaagcaagctcagggatcctgaaccttccttagtcaagccgcccttaccggaaatgttattcttccaagtgtcggctgcgttaaagccgcctttggaagcatccatgttcacggtgacgttgtccaagaaggatccaaaaccgttagcagcttcaaagaggttcaaacggccccaaccttcagtatcatcagtcattgggtaacctgatggaataccagtggtgtagaggacttcacgtctttgagtagcatttagatatggtaatctggtttgtaagaggacttcagcgccctttgggacaaccattggcttagtggtgtcaccaattggtgagaagccataggtcaatcgataggtgtaattcttcaggttggtttggtaatcgctaaagtcgtccttggctgatttatcctgagccttggccaaatctttttgcgtgtcctggtaggcttggctgatcagctgcttgttgtccggatcgtttaaggtcgcagctgtcattgctgttccgatcacccggccacccataacagctaacggtgagtgtcgtccggcaagtactcggtcatagccgacttccgaagaacgggtaatcaattgttgatagcgctctgggaacaggtaggccaaggtttcaccggtttcaaatgcggcggttgtatggccgcttgggaaatcataatcgttggcggcagcagaagccattacgttcttcaagtatgggttaactttgacttgatcgctttgacgataaggacgggtatatttgatgtaagcctttggcgtccctgtgccagaccatgctgaatcttctgcaatatcaaccagcttaaccgcggaaccgagagttgagttttcatctgcccactgcatcgagctgtagggtgaacctgcgggaagcggtgcatcgggaacggcattaaaatcagtctgagcgttggtatccttgataaatgccggagcgtagggaccaaaaccactaatcaggttatatcgcaggtcccgccggtcagttaagtatgaacggtcaatttctgcttgcgaagcaccgttggtaatttgaattgatttgtccaaattgtcttggagcactttttgattcgtctttgtaccgtcagttggattccaataacttaaaaaggtattgttgaacaacgcgatcgccggattggtgtccggagtcgagttggtcttcacattctccttatagtgatcgacgaaatacccatatgaagctggaaccggattcaactcgtttgagacactggtatccgacttggcgtttaccttcacatcattaccttgagcacccaaaattgcagctccggtcaacgtcagcacaaaggcgcttttcagaaccgttttcaagatcgtactgctatgtctacttcccatgcttaatcctcccaagatgaaataatttctatgaaacgattatcagaacaacaagtatcagcaaaaccacaaacgatatttcccaacccaacttgggggtatgtttgatttcgtataacattgttgacatgatcacatcatcctttagatagtccctgatagccatttctgattcaactttagtgtactgggatgacgtaaattacccgcaaaatatttgtaaaaagtgggtaaatgttgatgtttcacatgaaacattctgttagattggcggcctgcgtgcatctgctctataatgtcggcaaggggtgatgactttgaacaaacatctaacacttttaatcgcaaccggatctctactgacggccgccattgtttcaatgcaaataccgaccacagtggatgctaaagtaaaaatcacaaccaatcagtcttacaagaaaacatcatttttgatcaattccaaccgaaacgcctatgtttggaatgccaaatacaatcaaaagttacataatttaaaaaattacccgcggacaaatttctattcaaccaagcgggtcacgattcggaccaatcattattttggaagttattactacattcataatgccaacaataagatcaagggctatgtttggcacggctttctcatcaaaggaacctactacaagggtggcttttatcgctaccccaccttcaacgtactgctttccaaccagccgtatcgtcgtggcggtatgagtcggatcggcgaatgggatgcttctggtgtgtatgcatcttcgaatcgtattcatgggactgttaatcaaaatgagctaaaaccgtttgcgacaacccctgccctcaatgatcaaaaacaggccctgacatatctaaagcaaaactggtcttatctccctgagatgttgaactatggtcagcataatggcgcgcgaattgtgatgcggaaagtttactatggaaccaatcaatggctaaaggttcccatgatcgatattcttaacggcccagccatcagtggcaattgggaagaaatcaatccatttgcggcggttttggatttgtcaaaattgcccaacggcgccaagccaatcgccaattacgatgttagccaagtaaccgtcttaccgctggggagccgggcttttgattttcctgatccaagtgctcaagtcactaattacaacagtggcccaatcacgcgtatttacggcaacaacttgggccccaatcataatctctccctggttgatttgaaccgttggctgcattacgttccgaccaatgatatttttaagctttccaacactcagccaaccttgaaagacggtatctggtactttgctcccagctttgaaagtggagttggttcaggtacccatcttcagcaaatgctcaaccaaatcaatccaactcagtcaccttactatcggacaatgactggtgagggcttcatccaggcacactatgaaaatggtcactggcacgaacagtttgaactctcgacaaatttaccggccttcaataaagggaacgggatcaccctcacaatttccaaaatgatcaccaaatcatcaggatccagttcatacaccactgctgacaacgctaatgctaaaatcgtcaagcattttgacagtaatgatgccgatgtttcggattacttcttcaagccggcaaactactatgaaacatttttgaataatgactaacaatgagagtccgttagaaacgacaaacagttcaatatcaaacgaagcgttaggtcatttgatgaggttcccacaaccggaaggaaagtttcacaaagtatctgaaatcgttttcttttatttgcaagtgtttctaagcaaaaaaatcaaagtttgtgaaccaaatggttgcactcagtttcaaaaggcgttatatttttaaacatacttataaaaagtaagcattacactttagatttaggagtgattaatttatggcaaaaatgacagctggtcaagccttggccaaattactggtaagctgggatattgaccatttgtacgggatcaccgctgactcaatcaataacaccgttgacggtctctatcaggaacgtgacaaaattaaatacattcaggttcgccatgaggaagttggctccctcgccgcaaccgccgacgccaaattgactggtaaagtcggtgtcagctttggctctgctggtcctggggcaacgcatctcttcaacggattatatgatgccaagatggatcatgcacccgtggttgcaatcgtgggtcaatcagcaacgccaattatgaatacctatttcttccaagaaatggaccaggatccgttgtttgttgacttaactgattttcataaacaagtcaccaatccggaacaaattccctacgtgatggatgaggctattcgctatgcctatcggaccaagggcccggcagttgtaatcattccggataatctatcgggtgaagaaattgattttgaaccttataaaactgccaaagtcttaaaaccggccaccaccgtgaatgttgaccaaaacgctgtcgaccaagtctatgatttactcaaacaagcaaagcatcccgtcttatgggcaggccttggcttgaaagatgctcgagatgaagtcgttgccttctcagaacgattcagtgtgccggtgctcaccaccgctccggcaaccggggttatgccgaccgatcatcccaaatttatgggatcgcggggacgtctgggaaccaagccgggctttgaggtaactcaggcagccgacttaattatcctggcaggaaccaattacccattcagccgtttcctgcccaaggggatcaaatttgttcaaatcaacaataacgttgaagatttagggaaacagcatgacattgacctgactgttttagccgatgccaaaccgttcctggccaaattaaatgaaaaagaaccaatagccccaaccccattcctgaaggctgctcaaaaggataagcagaactgggatgcctggttgaataaagtcgctgacgatgaacatgatggtttagcaccggaagcagttatccgggccatcaaggaaaatagtgatgacaacgcggtgtttggcctcgacgttggtaacaacttaatgtggtctatccgccaattaccatttaaccaggaccaaaagttcagtatgtcagcttggtttggaacgatgggctacgccttaccagcaagtatcgccggtaaattgagttacccagatcgccaggttttcagcatttctggtgacagtggcttctcaatggtgatgcaggatctgctgactcaagtgcaatatcagctgccaatcatcaatgtcgttcttgaaaacggcgcattcggttacattcagcatgaaaagatcactgcaagccaggaaccatatggtatccacttcattggtgccaattgggccggctttgctgacgacatgggtgcgattggcatccaagtcaccgatcggcagtcgctgaaggccgcattcgaaaaaattaaggaactccaagcaaatggcaacaccaagccaatcttaatcgatgccaaggtcaagaaccaggatccagttgataccagcttcatgccaatcgatcccgaccaattcgatcaagcaaccattgacacttataccaagcaatcaaatttgtttgatcaaccagctctttcaaccttgctgaaagaagaaagcaacagttaaagatacttgaatgcagcaaaccataaaaagccaccaatggacgatcaatccactggtggctttaattagcgatgaatcattttcaataattaattagcccctgctcacctttgatcccagccgagatgaaccacgaacgattatacaatcgataccccgttaaattagcaagccagggctttgagaagtgaagtaaaatcggatgttgtaatgaggctcgttttgaatttttgtatatccgtctgaattgagggggcattattctacttattatgtgatgccgactactcgctcactcattagtcagccacaatcgcctcgccagcatccttgtcatccttacccagcaggtcgctcacttcttgacggcgaccataaacgtaagtcaatgagaaactaaccacaaaagcaatgaccatgctaatcaagaatgccgggatggcgttggtcgcaatactaatgaatcccaaaacactattagagcctagtgagactgccaaaacatgggtaagtcccaaataaactgaggcgacagccgaaccgatcattgaggcgatgaatgggaactttaacttaagattaatcccaaacattgccggttccgtgattcccagcaaagcggacatactagctgatgacgccagtccccgctgttgcttatccttagttaaaaagaaaaccgctagtgccgaagcaccctgagcaatatttgatactgacgcaatcggaaaaatgaaactgccaccggtttgtttcacgttagcaattagctgggtctcgattgctggaaaactctgatgcaggcctgtaatgaccaaaggtgcatagaacaagcctaagacgcctgttccaaaggcccccgaagtctggtacaaccacaataaaccgttggttaagccatcgctgacatcccgcataactgggccaacaatcataaaggtcaaaattccagtcaataaaatcgtaatgagtggtgcaaatgtataatcaagtgcttctggaagtcttttatggcactgtttctcaatgactgacagcagccaggccaccgccaacattggaatgacggatccctgatagcctgcttgggcgactggcatccccaaaatgtgccaataaccaagtgaatgattggcaaccgcattgctcacatcgtagccacttacaagggcgggcgacaccatcatcatccccatggcagctcctaagtatggattcccaccaaagcgcttggtggctgagaatccaattaagaccggtaaaaatgcgaacggtgcgttagccaagacattaataaacgccgcaaatcctttaaactgagggtatgcagcaactaaagaagcagtcataaataggtggggcgccactaaaacattgtgaagtgccattagcaaaccagccgccacgattgcgggaatgattggaacaaagatatcagccaataagttaatgaatccgagaaatcctttttgggtctttttaatcgttgtgataaacaaatgcatatcctcctcaaaatagtcacttcgaaccattctacaagttttcgtcacagatgcaagaagattgacagaatttcttgcctgaaagcacctctacaaacgttttcattaccatttccatggacagacaacatctatcaaaaaatctgtcttaacttgggattataaccacacactgtggttgcttgtgctatgatttgagaggaagtttcacatgaaacaatttgaccattggagggtctgcaagtgactaagtataaagttcaatcattagtattcatcctcgttgcctttatgttggggtgcaacgaattcattgttgtcgggattctgccggatttatcggcccaatttcacacgccaatctcaaccatgggttacttggtcaccatcttcgcgatggtttacgccgtcagtacaccatttgtcacaatcctaacaagtcggtacagtcgctataaaaccctgttaaccctaatgattgtctttttgattggtaacacactcagtgccctttcaattggctacctaaccatgatggcctccagaatcatcaccgcaacgacagccgggtcaatcatttcactgatcatgactttcgccagcacaattgcaccacgggacaaacgggcttcactggtttcttggatctttgctggcttcagcattgcgtcagtctttggggtgccaatcggcgttgccgtcagcacaagcttcggttggcgttacaccttctggggaatttcggttattagcattctgacctttatattgttaacacaaatcctgccaaagaaagttaagcagacaaccagcaccatcaaaaatcagctgacaattttattggatccccgaatctattacggtgtcttcctggtcttattcacggccgcaaccatgtacggctactacacatatattcgcccgctgctcaccacgtcgatgggcttcagtacccagagtttgaactggctgttgttcatcatcgggattatgagtatcatcagtaatcggctatcaggaatgctggccgaaaaaccaaacagcctgcaaaaggtaccgctcttttacgttgtcgatatcctcttactggcagtttttccatttgcattacacagtaaaattgtcggtctggccatcatgctgatcctgacattgattgtgacaatcatcaattcaccggttcaaattcatttcctaaatctggcagaatcagaatacccacagtcgctggtctttgcatcatccctgagttcaattttcttcaattttggtatttccctgggatccgcgacggcttcgagtttagtgggcattgttggcctggatagaatcagtattggatcggttgtttttgcagttctttcgcttggttcgctatttttgattaaccgggccattaaggcgcattcgtcgacgaaggcaggagactagtttggcgccttgcattcgcgatatgttaaatccatcacacacttaaacgccgttctgaatgtcccttaaaatctgtctcaaatattgacttcaatccaaataccatcagttaacgcgtgatattttatcactgtttcccaatagtaccgtttccaagccattaagtcggtatgcgttgtttcgtgaacctaaggataagattgttaataatgtagctactttcaaggcaatggatgactttttgaatgtcaaaaaccggttaaccaaccagcagcggttagcaaaaattaaggcaattctagtggctaacggctatactgctgctaaacgtcaaaaggaatacgtcatcggcatctacctgactaacttccagtggtccgatcaatatgacactggcaatatgcatcaagggtttgtgattggaaccaaataaggagatacttaaggacaacagttgcttcgtatggatgtttcattgacccaaatacgtaactttttttaatgcgtgtaatgattgttagggggcatttccccctgatatgatatagtcaaagtgccaaaaagtcctgataggatgaacacccaagccccaacagatacaaattgttgaggacttttcttattgatgataggagaaatgaagtatgcacaagaagatactatggttgattcaatttgcgattaattgcagtttcatgatttatttggcaagcttcccgtcaaatgcagtttattctggatcagggtggtccattttaattggtctatttcttgtaatcattgcggttgttgcagcgattattttgacaaatttggttacagaaagatgaatggcctttactggatgtaagctgatcccagagacaacttttaagagaggggataatgaataaatcatctctcaaaagaaaggaattttcccatgccaacccgtcacttgaccgacaaacaaaaaatgccctattaattacactaatgaggcgctgatgaaaagaactgccgaaccagacaactctcattcaaattaattgctttcacatgcatatgaattacactgagtttgtataaatacaaacaaaggagcgattttgatgaaagcattcggttacgaaaaaaatggcggtcccgaggtgtttcaggagtatgaagtcccaacccccgaaatcaaatccaatcagatcttaatcaaaacggaagccttcaacttaaataactttgaagcattacagcgagctggtcaattcaaaccagtcgaccaccgaatcatccccggaagagacgtggccggctttgttgaaaaagttggcgaagatgtcactggttttgatattggtgatcgggttgtcgctcacggccatcattcctacgctgaatattcaattggcgaggattccaataccgtcttaatccccagtggtgttccctatctagccgcagctgggattgtgactcccggtctggccgcttataaaggtgttcacctgtttggcaaagttcaagccggccaaaccgttgtcgtgaagggggcttctggcggggttggctcacttgccgcccaaattgccatggatgttggtgccaaagtcatcggcatcggttccagcgaaaatgaagaatatgtcaaatcattgggcgttgatcaatacgttgcttacgaccaggaagatccagcagaagttttggcagacacagctgatgtcgtgattgatgctgcattaaacggcaacggcgccgaaagtgacgtcaaaatcgttaaagatgacggaattgtcgccagtgttgccgacaacgatgcgccaaccgataaaacggttcatttcaatcacattcacccaacccaggaaatctcggatgatgatgctttgaatgccatgttaaaactgatggcggcaggcaaactcaaaattcgtatcggttacaagctaccatttaccctcgacggggtcattaagggccatcaactgctggactccaagcacgccggccgaattgtgattgccaagtaagattgtgataaacagaaatactgaaacgcaaaaaggtcagaacatcattcaccagaatgatgccctgaccttttaatttggatttatttcatctcaacttaaatcccttatttcgaagaatccttgcccttatctttatccttcacaattgcctcagagtatagtttgtcaaccagctcaggatttgatttgccaggattcagttcgacaatctggccggcagccgaataaacaatccactccgccaggttgacgatgtgatcaccaattcgttcaagaagtttaatcaccataaagtaactggagctggccgcgatcgttgcggtatctgattgcacggcctcggtaatttcatccctaattaacagatactgttcatcaactttgacgtcattgtcggataactttttagcggcgtcggcatcgctcttcacataagcatccaatgcactctccaacatatctcggacttcttcggtcatcttggcaatggccttttcaaccttgggaatccggggattaccttttacacgaatagtttcgcgagccatactaaccgcatgatcaccaattcgttccaaatcagaactggcttttaaaatactgatgattacccgaaagtcggtcgcaaccggctgttgtaaggcaatcaagctcaaagcctgtttttccaatttcatttcatccgaattggtttcctcgtcggcatcgatgacttcttgggcggcttttttatcatgctcaataaatgccgtagttgatttataaatttgttcactgatcgtcaggcccatttccacaaaccggccgtggagcttttttaactcgtcgtcaaataattctctcatcgtctctattcctcctagccaaactttccgttcaaataatcgctggtcttctcatcatcggggtgaataaacatcttctcggtcttgctgaattcgaccagatcgccgttcaagagaaaggcggtcttatctgaaattcgtgaggcctgctgcatgttatgggtcacgatgatgatggtgtattggttgcggatatttaacaaagtatcctcaattttggcacttgaaattggatccagagcggacgttggctcatccaacagcaccacttcgggctgaactgccagcactctggcaacacagattcgctgctgctgaccacctgaaaatgacagggcattatcgtaaaggtggtctttgacctcatcccagatcgctgcctgcttcaagctggtttcaacccgctcatccaaaacgtgcttatccttctcaccagccagccgcagtccataagcgacattttcatagacgctgaatgggaacggattgggctgttggaacaccatgccaacccgctttcgcaggtcaacaatgtctgttccgggggcgtaaatatcttcgtcttcaagcttcatcgatccggtaatcgtgacccctttaattaaatcgttcatccgattgagacaacgcagataagtcgacttcccacagccggatgggccgattaaagctgtgatatcgtgttcttcaaagtccaaactaatgccatggagcgcctctttgggtccataacttaaatggacatctttactcgtaatgatttttggcattgttcagcctcctaaccgaagttcccggagatataatcttcggttgcctttatttgtggtgtcgtaaatattttctcagtcacgtcgtattccagaacatggcccatgtggaagaatgcggtgtagtccgcgattcgtgacgcctgttgcatattatgggtcacaataataatggagtaattcttgcgaagttccattaaggtgtcctcaattttggcagtggaaattggatccagcgcacttgccggttcgtctaagaggaggatatccggcttcattgcaacacatctggcgatacaaagccgctgagcctgaccgcctgataaggccaaggcacttttatcaagatcatctttaacctcatcccaaagagcggcggccttcaggctttcctcaacgcgtttattaagctcttgcttgtccttgataccattgcgtttgagagcaaaggtgatattttcacgaatcgatttggcaaacggattgggacgctgaaacaccatactgatatgcttgcgaacttcatagacgttaatcttttttgaattaatatccatatcccgatacataatttttccttgaacggtcgcaatccggtcgttcatccggttcagacagcgtaaataggtcgatttaccggatccggaagccccaatcaaagcggtaatgcgatgtcggggaaattgtaaggtggcgtcgtgcatggcgtggttgtcaccataaaacacctgcaggttttcggtggtcatcgctttttctaacggaatatcgataatgtgcgttttattatagtcatattcttgcataataatctcctacttcgttgctgtcatgcgtttgtacaaccaacgtcccagcatgcgggccaataggttgaacagtaaaatcacaacgatcaatacggctgatgccccacttgaaatggaagccgcatcaggggtaaccccctcagtgttcaccttccaaatatgcaccgctaaggtttcggctgggcgcataaagttcagaaaactggcactgtccatcggattccagtcaccgtaattaaccgtcggcgcactttgtccagcggtataaatcaaggcagcggcttcaccgaatacccggccggcacttaaaataattccggtcaaaataccaggcaatgcggctggcaaaacaatcccggtgatggttttccaacgtgataaacccagtgatagccccgcctcacgctgtaattcggaaacatcctggagtgattcctcaatacttctggttaaaagcggtaagttgaagaatgtcagggcaatcgccccagctaaaattgagaagcccatgtggaaattaaccacaaacaataggaagccaaacaacccaacaacaactgatggcaatgagctcaatacttcaacggcagttcgaattacgccggttacccagttgtcaggggcgtattctgaaagataaatcccagaacccaaggcaattggaaacgaaatgatcaacgtgaggaccaacaggtacatcgagttgaacaattgatcccgaatgccgccgccagcagcgaacgattgtgctgccgacgttaggaagtgccatgatacatggggaatcccagtaatcaagatatagccgagcaggaagaccagaatcgccaaaacacaggcaaccagaaaataaattacaccagtggcaatgttattactcgttttagaattcattttttcaggctccctcgctttccgattactctgactaagatgttaaagactaatgacatcaatagcagaatcaaagctagtgaccataaagcgttatttggcagggtccccatcgtggtgtttccgattccggtcgttaattgactggttaaagttgacgatggtgttaataagccatgaggcatgagaacagcgttaccaataaccatttgaacggccagggcttcaccaaatgcccgtgacatcccgaagatgacggcggttaaaattcctggagtggctgatcgcagcaccactttataaatggtttgccatctggtagctcctaacgccaatgacgcagaccgataaaacatcggcacagctttaatactgtcaactgaaagtgacgtaatggttggtagcaccatgacgaacaggaccaaggttccggcaagaatcccaaaaccagtgccgccaaatgagtgacggatcagtggcacgataactgaaagcccgatgaacccgtagacaactgaaggaattcccactaacagttcgatgaccggttggagaattttggttccccgctccggcgcaatttcggtcatgaataaggccacccccagtgcaaatggggttgcaactactgcggcgagtaccgtgacactaaacgaagtgacgatcattgggagcgcaccgatctggggattaccgtgtttgtccagtagggccggattccagttggtgccagataagaatttccataaactgacatggttcgttgtgaaggtcgctaacccacgggtggtaatgaagtacagaattgagataaccagcaagctgacgaagccgatgcagagatacgtaatcccgcggccgaataagtcttcgtgcgtcgcttttgatgggttttgaagatcatgtttgatttcatccatgattaacctcctataatttagtcgaatgaattttaaatgagtaccttaacttgaggaaggctggaggcatttgatttgccttcagccttcgttggttttgtgtttagtttgtagagttaatggtgcgtgaagattacctagtgaaaacttggttcgagccatgagactgagttctaagtgcactttgattaaagtgtccttggaaaccgcctctccaggagcacgtttgttaggtgcttttgtgctcccttctgcctttaaaatacgctctgacgggccagaggctaacttctaagtgcactttaattaaagttccaaacccaggaacttcaatcaaagtactcttagaaaccgcctctcccggcccttgtcgcgctctatttttcagagacggcattacttgcattcttcgttactttcatatcatgaatactgatgtaaccaagtttttgaactaagctgtcttgaaccttgcttgaatccatgtagttcaggaacttcttagttgctttgtttggttgacccttagtgtacatatgttcatatgaccagatcttccatttgttggtggttacgttggcatcagttggctttacattgttaactgacaatgccttgagcttgctgttaacgtatgagaaggccaagtaactgatcgttcctggtgtgcttgaaacaatcttttgaacagttccgtttgaatcttgttcttgggccttaactgctttggcaccctcaaggacggctgattcaaatgtggcacgcgtacctgaaccttgcgcacggttcacaacggtaatcttttcgttcttgccgccaacctgcttccagttagtatacttaccagtgaaaatgccctttaattgtgccatggtcaaattgctgacattgacatctttgttaacaactggtgtcattccaacaacggcaacttgatgatcaactaatttttttgctttaatcccatcttgttgttcagcgaagatatctgagttaccaatttgtaccgcgccggtttgaacttgactcaaaccagttccagaaccgccaccctgaacagaaatgttaacccctttatttgctttttgataattgcttgctgcttgttcaactaatggctgcaaagcagttgaaccaaccgccgtgatcttgacattcgaatcagctgagcttttctttgacttagagctgctggacgaaccacaccccgcaagtaaaactccgacagctgctactgctacgatagttgaaaaaaaggatctttttttcataattcgatttcctcctaatgaaaacccaagtttttttagtactcatttaagtacattgttaatataacaacagcatgtaaatatcgagtttcgtttatgtaaaagtaacgtaaaaccggccatttttatcaaaaagtatggcataacttaagatgtaaacaatttaactaatatggaggaagaccggatgccattggaaatcttattgatcagccagaacttaaagctggcggataagcttgagaaactacttgccgcctttcaaattaataccagaatctcatttgaaccccttgatcatctgcttcaacaagtttccggagtcgtctgggacttagacacaactgaactgccggaaaacgattcggaactgcagattctccgcagtcaaattgccgggccaatcttgctgctggataaacagccacggtccgtggaaacgatttgttcctattttttggattatcatttggatgattacatttatgacgaatcaccaagtgaaattgtcgccagaattgttcaaaaaatttgggtctatcaaaataaagacaatctccagctgacacagcagagtcaggagtcggaaagtctggtggtcggtcacttgaagattgatttgagtaaatttgaagttaataacggccaccaaaagctcaatttaagtccaatcgaatataaattgcttctattctttgtcagcaattccaacaccgttctcagccgaacccagattgcctcggcagtatggggtaacaccaccggggcgaccttgcgaattattgacacccatatcagtaacctgcgcaaaaagatcgaaatcgaaccaaaaaatccccagatgctaacaaccatcaggggatttggatatttatttaagaataaaggcaaccagcaatctcacgtccagtaaccgttaatcggacatcaacaaccacttggccattcaaaggctaggtggttttcttatatattcttgcttgatgcttcaactcacgctgacataattcgacaaagtcctgcccatacgcggttctaacctcatcttcccattcaccatcatttccctgctcatcaagcattggctggatccattggttggtgggtaagagtttaagcaatgaatgtttggtaaattgtgagaataagagattttcgccaaaatatgtcgctaattgatgctgaaacgctgggacatcaactggtagtaacagattattcgcattgttccggtcgcccagcaatagttggcaatcgaggaagtcgctctttaaatcgaacaacttatctttgtgtgccttggcgatgtctggaaccattctaatgaaccaaatcaatttgtggtgttcaagagcgatcagcaagttcaacacagcaatgtccagcgaactcaaagtaaattttgcgttttggaccgccactgggtgaagactgttggacaccgcattaaataaatcaccaaaggtccccggctcttcccacaatacctcaatttggtgggcgttctgcagccaaagccgatgagtggcaatccgaagtgtcagccagaaaacttgatcatgatcgtcataccccttaatcagccagtatgaactggccgtggagcgggcataattgctggcggccagttccaagccatcgggcagcgccgctcgaacagtctcaatcagccattcacggtaggagggtttatcagtaaattcataggtttgttcacgtggacgtggcttagccattgagatccctccttttacatttaaaattcatctcaatactagtttacgcttttttgaaaaagggaacaaaaagagagtggaacgcgaggcgttttgatcccagaatttaagtgaagaagcgagctattcctgttttggaatggctcgcttcttcacttaaatggccgggatcagccgatcgttgcacgttttatcaatataacagtggcaatcaaagtggcaatgaaagccgccgtagcaattaatgtcccaacctcaattagaaataaatctgcatttaaattgtttcacatgaaacattatgctttaacagtcttaattgccaagaaatctttgacttggtcactcggaattgatttgataaccggtccaccaattgtgtgaatgtagatcaaacttaaatgaccgtcacgattcttcttgtcattcttaatcttttcaaatacttggtcagaatccaataaatctgaagtaaccggcaatccaaccgcttctaaacgttcccggagttcttgagtgatgccggtcaaggccaagcccttgtcttcaaaaatctgctgcatggcaatcatgccaatgctgacggcttccccgtggcgaaggccaccgtcagagagcgcttcaacagcatgcccaattgtatgaccgtaattaagcaattggcggaggccgccaccctctttttcatcacccatgacaatgtctgctttgtattgaatcgaatgaatactcaattcttcagcgttggccaaaatgtcttcaggtgagttgattgatttgactaagttccacaaatcaccatcggataacgccgccactttgacaatttcaccgtacccctcaaccaagtcgcgagtttttaaggttttcaaagtgtccggatcgataattaccaaatccggttggtaaaatgagccgatgatgttcttggtggtatccaagtcaacagccgttttaccgccgactgaactgtcaacctgggccaacaacgaggttggcatctgaatcaggctgatgccacgcatgtatgtcgctgccagaaaaccggctaggtcaccggtcacaccgccacccaaggcaatgacaccatcatcgcggttgaaactgtcagcggccatttgccgggcaaggtcagctaaaacgtctacggattttgattcttcaccagcgggaaattggtactcgtgaacagtgaagccaacagcttctagagcctcagcgacttgggcctggtaaaggggcgcaacgttgctgtcactcaccagggcaattttgcgcttgctccaaacactggacaccaactgaccggtgcacccaaggattccgcgggcaatttcgacattgtatgaacgatctggtaaatcaactttaatgattttcataatttaacctcacttttttcttcgacaggggtcgtgatcactttccggattgcaaatgcctgctgagccatcgcacggtattcatctggcttaagtgcttgggcgccgtctgagaatgcatgagcaggatcatcatgaatttcaacaactaaaccactggcaccaaccgcaactccggccaatgcctcgggagtcacaaattctgtgtggccggcggcatggcttgggtctacgatgactgggtagtgagtcagtttttgaagcactggaactgcgccaacgtctaaggtgttgcgggtgtatttgttatcaaatgtccgaatccctcgttcagtaatgatgatgttatggttgccaccagcggcgatgtactcagctgcatttaagatatcatcaatcgtagcagacattccccgttttagcattactggagtctgagtcttgccgactgccttcaaaagtgagaagttctgcatgtttcgggcgccaatttggaaaatatccgtgtattgttcaaccattgccacgtggtcttgatccatgacttcagttaacacgtccatgtcgtaagcgtcagcggcagctctaagaaatttcaaaccatcttcgccaagaccttggaatgagtaaggggaggttcgaggtttaaaagcaccgccccgaaggattgtggccccaccactcttggcaactttagccatcttcatgacatgttccgcagactcaactgagcaaggacctgccatcatcgtgaagttatcgccgccaatttgactgtgcggtgtcacaacaacggtgtcttccgggtgaaagaggcggctcccctgaacagcggcgggaacgttgtcgatgattaagtcaatggcattcttttcttcagcatttaagccatcttcacttacgccttggattgccacgcggttgttatgaacaaatacctcgttggtttcggtaaagcgactcttgatctcgtcaataatgtcttcgtgtccgtttttaagtacaataatcataatattatctccatttctgtgtttgacgtgtttttgaataaaataaaactcccacagtgtgtacaacactacgggagtcagaattttgggtaaaaaaattggtcccgcagtatatttggtaaataactgtgtgaccgaagtaagtaatcatgatgaaatactattggccgcacaagatgtgagtgagtgcccacatcctgtccggtgtgaacactaaacgaaccaatagtaataaaatcgattaatttttgaattaatttttatcatgattagaatctcctaagaaagttaaattttaattgcatagagcatataatgaattccaagatgtgtcaaccccaaagtttaaattatgaattttcttgacatcttctcataaagagcgtaattttaatggcgattaaataccgtcctaaataaaccattgaagtggagatcaagattgttgtgcacgtcaagagagtcgctattgctgagaatgcggccgaacgcaagcagttaaatggaccaccgagggttcttccgaaagtgatcgagtacgaagaaacgtgttggcatacgtcagttgtcggagggatgttggtcccttgctaagcgtagttgacggaaaagagtgactctactgaatggtggactgtctttttcgatcaattaaacaaaggtggcaccgcggaatgatccgtccttaatgtgaaaacatttggggcggattttttatttagagcgcgacgagggccgggagaggcggtttctaagggtactttgattgaagttcctgggtttggaactttaattaaagtgcacttagaagttagcctctggcccgtcgccaagtaggctaggcagggtttcacccggccgtcggagcgtattttcaaagcagaagggagcacacaaaggcttaacaaacgtgctcctcgacatgcgtgaaaaatatgtcaatcagaggatgacgcaatccagcaaatacccaaatatggaggaacatttcatgaaaacatcaagaaaacgatggcaaatccaactttagcatttagcaaaacacgctaaagtaatggaggacaccatcatgaatctagaccaacttaaacaatatacaaaggatttttcagctataccaatttcaattaatttttcaatgcaggactttgaccctatcgctgtgacgcaacgattcgatcaaccagatgcaccatgcttcttactaactggaaaaccgaagaagcaggaagacgggtattcatttatcggattgaatccgacgatgaccatcacttatcgaaacggcgtcttaacccgctcggatgagcaaggcaatgtttcacatgaaacaacggatttaaagcctgttctggaacggattttggcggacaatcgaatgccaaaactgaaacacatgccgccattttcaggcgggctcgtcggttacttcagttacgactacgctcgctatgcgactaccgcagatttaccagccgtcagtgacccaatgaaactcaatgatgtcgacctggtgctcattaatcgggtcattgcttataatcacacgaccaaaatggtcacgttaattcaagtgatccctgccgatcagctcacgacgcaatatgaatcggtaataagtggcttaaccaatctgaaggaggaaattctgcaagtccatgagcaacagccgctccccccatttacaatgacaccattcaaattgcagttctctttaagcgaattcgaggaaaaggtcgcagaagcaaaacatcacattgtcgatggcgacatcttccaagtccagctctccaatccgcaacattccaaaatgaccggttcgctgtttgctgccacgccaactttattcaaagaaagcccatcgccgtatcaattttattttcgccacaacgattttgaaacaatcggtgcttcaccggaaaccatgattaccaaacgaggccaaacattattcacgtatccgttggccggcaccagaaggagagggaaaaatcagattgaagacgacgcttttgccgacgaactacaacacaatccaaaagaattatcagaacataatatgctgattgatttaggaagaaatgatctgggaagcatcagtcaatttggatcggtcaaagtgaccgcgtatcggaacctgctgaagttctcgagcgtgatgcacatgggttttgtggttgcaagtaaagtcgatccggacgtttcgtcaattgatatcattcattcattactcccagcggggaccctttccggtgcgcccaaaatttctgcaatgcagattattggcaaactggaaaacaacaaacacggcctttatggtggttgccgaggctatctgggttttgatggtgacctcgatatgtgtattgggattcgattagcatatcggaaaggtgacgatttagtcgtccgcagtgcggccgggattgtcgccgacagcatccccaaacatgaataccaggagtttaacaacaaagccagagcaattgtgacggcactgcaggaaacagcagccaagggaggcgtttgcgatgcattatctaattgataactacgatagtttcacatacaacctataccaattgattggcacccagacctctgaagagatcaaagtggtgaaaaacgatgccatcaccgttgaaaatttaatgaaagcaaatcctgaaagcgtcattttctcccccggacccggccgcccagaagatgctggtaacatgccggcgatcttagacgcattcctcggcaaggtcccgatttttggcgtttgccttggacatcaagccatcgcagaagctttgggggccaaagtagtgcacgcccccaagttaatgcatgggaaaccctcaaatatccaagtttccttagacgatccactcttcgcggactgcccacgtcattttgaagcagccaggtatcattcactcatcgttgatccaacaacggttcccgatagcttggatgtcaccgcggtaactgatgacggagaaatcatggcgatcagcaatccagccaagatggtctatggcgttcaattccatccagaatcaatcatgactgatccagaagtgggaaaacagattatcaacaattttctaacaatcgtcaagatcgctaaagtatcgactacagctcgttaaaccgaaaaaagggattgcggcaaaactgatcattttgccgcaatccctttagttttcatatattctattgaacttgtctgagcacttgcgagcggctgagcatcttgaatattgctcggacacagacagccccgaagaagaacacggagatcagacggactgagaacaatgccaagatcattggcaggtgataatggacataacccagacggaacagttcatatccaaaggaaacgacggtggtcgtaaccgctgaggtagttagtaccggccaaccccagttcttgtatccccacagcgtgaacccaagctcacttccgattccttgcacaattccagaaataagtgcactagcaccaaaggttccgccaaaaatgacctctgcagcggcacctaatacttcaccaataattgccgctcccggcacccttaccaagtaaatcgacaatggtccggccataatccaaaggccaaacagtgcctcgtttgagaatggtccaatggcaactgccaggaaattatacagataatctgtcccgacaaagatggcaccaaaaacgattgcaacaatggctaacagaatcacatcctgtaagcgaaatttctttttcatgatttttctccttttgaatgacaccaatcataaatgaatgcggccataattttggtatacgttaataattgctgaaaactaagactttcattatcactatgagcttgttccatggttcccggtccaaaatcaaccgctggaatatggcagtaaccaaaccaaccgctatctgatacggacggtgacatccccaaggttggttgtttaccggccacttcggcaaaactgctctcaagtgccttcatccctggatggtcggggtctagctccagtgacgggaacacctcgcctttatcgactaatagcgaatcaccgccccaagtaaaggtgggcagattatcccgcagccaagggtcggcttttgccgcagcaaggacttgatcctcgatttcatgggttatatcatcaacattttcatttgggtaaaaatgcacggtgatccataatttcgtgacgctcggaatgtaagccggatgtaaccccccttcaatataagcggggttaattgtatcgattcccggggcaaacccaggataacgctttgtaatcccccagtactgttccaatttctccaaagcctgaatcacgaccatcattttctcgatcatattggccgctttcaggccaccgccagtggtaatcattgctgctcggttcccatcgtggtaaatgtggggactcttgagtgtaatccagccggtcacgacgcctccctgaccttgaaatttcaagttgctggtatcgccaaccactgcaaaatcagccgtttcaccatttttcagtaaggttttggttccggcttctccagcctcttcaccaacgacagattggaaccgcaaatctccaggcaggtcaatcccaagctgttggagcagtgaaaagatgtacacaaagcttgagataccacctttcatgtcactgacaccccgcccgtagagtagatcaccctcgtggactaatttgaacggatcggtgtgccaactctgacgatcaacggtagccacatcaacatgaccattcaacagcaaactatgatagttagctgcatcagtccccggtttctcagccgagagcagctcatcgccatcataaaaagtttcttgcttagtcttaaatccaattttggttaattcatcatcaagaaaacgttgaattgccactgtgttgcgggcaggtggtgacatcgtttcaaatgaaattagccggtccaataacgctaacagttgattttggtgcgcatcaactgcctgaagtaacgcttgtttatctgtcaacttcgactccctccaattatttgatcatctatggtttggaaacaaaaaatccccctttcttcaaagcctcgaagaaagagggaacagattaaaagttgaatcgactttatatctatttgctcacacaaaaaaatttcgttcttccttcgacagtcctaactgcatcaggttcaatgggtatttatctcagccgtttagggcaccccagactactttattcaattagccacaaattacttggctggttttatgatataacgaattgacgaaatgtcaaagttaattttttgatgttgtgaggtcaaggcctgtgagcctacttgctgatcggctgatcccggccatttaagcaaagaaacgggtcattcccaaaacaggaataactcgtttcttcacttaaactctgggatcaaaacgcctcgcgtcccactcccacaatcgtttcatttgaccaaaatgaaaactttattctcgaaaatccagttgattatgatgttgccagaccgcctgtccagtgactggcagcgctgctggtatataccttaattgagtaggttccggaaccgacccacaggctaccgctcaatgtgccagtggatgaactaatcattttgtatagttcaccatctttgtagatactgattgaaaatggatcagcactggaggcgccactatccgttgacgttttaacattgtagtgcaaagtattaatgaggttggttgccttgacggtcacattgtagccagaattgtcattggtatactgactgcctgtctcacgaggttgctgggacagatttttaccgccgacctgcttagcggccttggcattgtcttgtttgtggccttgttgttgtcgttgaggttgaactgcatcggcattggcaacgacgctgctcagaaatgttggggcaaccattgcggctgcagccccaaatgtgactaaatattttttaattttcatggatgataacttcctttcaatttaacgtttgttggtttgatctggaacctatttcagttgccctcccttcatacttgatgttgctagaatatcggggcaagcttaattgggacttaaattagttaaaattgggaaggaagccgcataatctttagaaatccttgggacttttgtaaaatttaggcagcaaaaaagggcaatcaatgaacgcaaaccgctcaccaattgaccttgcgaacttcttcaatgaatctgatcaaccctattcaaccttaaagttcgacttgaatataaacccgcagttagggcacctgttcaagccgtaactgatagacattggtcgatgacactttggacagttgccctgcatcggccggcgaatcttagttggcttcggttctttctcatctgcctgatcactcatattgacctccactaaaatatcattactgattgataatctttagaaacttagccggcattgaatccaccaaccaaatgccactttcggttggataaaataacagtcctgaagccgcggcttttcttgcttcaatttcaaaaatcataggatgaggatcacgccgtttccccacctgaatcgccatttggggatttgcggataaatgaacaaaatcccggtccatcttttttaatccttcgtcgacaatgaatctggcagccgcatgagtcgttccatggtacagcttctctggaggttcaacgggtggcgtcagtggatctacggggatgctgtggccgtatagcgccctaatcgtgtgaccttcaatcgcataacgttgtttgtcgctatctttcataatttctcgaatgattttctcactaattggtgtcccaaagtgctggttaaatttttggatgagggtttgtaagtccactcgtccatatcgatccaactggatgccaattttgtccggatggtgtctgaggacgtacgacagacgcttgctcaacctggttaattgatgatccattttactgactccaatcgtttcaatattatctttattataatcccaattgtgggcaaaccacaaaaaacgcccggtactaaggcccaggcgttgctacaaatcatattcatattagaggggatcttacttcttgggggagacgtaagataatcaagttttatactttggaggagtaaattcacttgtaaaccaatttatctttcaaaattgattgtctttatattatggttgccaacttaactcagccttaaataagtgtgacgaaattgtgaagttccagaaacgattagataggggtgttgtttatcaagatttcttatataattggatacagaaaacatttgaaaggattcaacatgaaaaccatttattttgtgcgccatggtcaaacgttactcaatcaatttcggcggatgcaaggctgggtggactcaccattgactcaaaagggcgagtcccaggcaaaggcaactggggaaaaacttgctgatgtccattttgatttggcaatcagttccgatatgatgcgggcgattcatactttagacattattctggcaaataatcatgcttcgggtggcgtttctcgagaagtgtccctggacgttcgcgaaatttactttggctcatttgagggaatcgacagtatccaaacatggaacatgattggcggaccgctgggacatcgtaatcaagaggacttgatcgaagaatatggcctcctcaaaatgcgtgatttcatgcatgccgccgatccatttcacgaagccgagacttctgctcacctcgagagtcgaatcaacagtgcagtcgaacatattcaatctgaactgacagacggtcagaacgccttggttgtttcacatggaacttttctgagaaacctggcgactttatatactgatgatgcaacagttgttaagcagccccgtaacggtagcattacccagctggacgtgaccgacacgccgcatattatttcctacaatgaataaaaaatctcacgaaaagattgcgtaattaatcttttagtgagatttttaagttatcgttaatagcctagactgttaacgttagttcgtttggtcttgttggtttcccagaagaaggtcttggctacgccggtaatcttcttctttggaacaaagccccaataacgaccgtcatttgagacgcttcgatggtcaccaaggacgaaatactcacccttgggaaccttggtggcattggtatttttgtcccagctcttggataatgatttcaaattccaattgccggttccagtcgtccgttcgctcatgctaatgaacttctggggaacagcttttccattcacgtagatattgccgttcttactggagacggtatcgccaggtaggccgatcacccgcttaacatagtcggttttaggcttggtagccgttggatcttcaccatgggcatcaaaaacgatgacgctcagatgcttaatcttggcatgccgccaaacaatcaagcgctctttattaacgagattgggttccatcgaaggaccatccacccgggcgaacgtgaagacaaactggcgaatcaatagggcaaccagcagcccaaccaagatggggattacccagctcataatttctttaaatactttcatcttaagctcctttgtgaacaacacaattagctatgcatactatccataacgattagcttacacaatcgatattaattttatcacatttacccgccagaacaactttttcgcgcttaattaacagaaccctaatttattgctcatattgcaatcaaactgtatcataatttgtatgactccgcttgtgaaatagaggtaacaacatgaacacaaacctaaaactaggaaataaaatttggctgatctttattctgggaacgatcagtgcaaccggaccgctgtcaatcgatctgtatttaccggcccttcccgaaatgacccgtgacctatccgcccagccttcactcattcagctgagcctaagtgcctgtctcatcgggttagccctggggcagctgatttctggaccattaagtgacaaatatgggcgcaagaagccgttgatgatcgggtttttcatctttggtctggtatccttgatgatcgcctacagcagttcagtttatctgctgatcggcttaaggttcattcagggtctggctggggcaagtgggcaggtgctctcccgggcaatcgcttcagatatgttctcagggcctctgctaaccaaattttactcgatgctatcagcggtcaatgggatcttcccggtcatctcaccagtcattggcggctttatgatccgctatgtcgagtggcagggaattttcatcctgttagcagtcattggatttgtcttagtcctggcactctggctgggaattaaggaaaccttacctcaagagaaacgaatttctggcagtccggggaaatcaattggccaaatgtttaagttattgaaaaactcgcgctttgtccgcctggtactggcaactggattggtctccggtggtctattcagctatatttctgcttcatcatttgtattccagaacttcttccacatgtcagttcaaaacttcagcctactctacgcattgaatggcatcgggatcgccattggctcagtcattccaggggccttggcgggacactttagtgaagctggtcaaaccaaagttattttgacatccacctttataacctctgttttactaacattgagcgccttattcttgaacaatctcctgctggtgatcatcttagtgttcttaacggttactcaatttggaatgttatttacattaaccacttcaattatcatgaacctgacattacataacaacggtggtctttcagcaatgttgggcttgtcgcaaaatgcaattggcgggatcatgtcaccgttggtcggattgatggggactgggacctatctgccaatgtcagtggcaattatgggatgtatggggttgagtttatttcttttcagtactattcataataggcaacgctcactcagttaataaaaacggctgggagcaaaatttgctctcagccgtttttattgtgctgttgactaaatgatcatatttaagaaccggcagccaaagtggtagagcggttcattagactttaaaactactcagccagcttactaatcttcccctgttgaatataaacgctcaaaatcgcgatatcggcagggttcacaccactaattcgggatgcttgggcaattgtctcaggatgaattttctgcagtttctgacgggcttcggtagcgatgccatcaattgcatcgtaatcaatccggtctggaatctttttagcttccatccgcttcatcttttcaacactttgctcggctttcttgatatagccggcatatttggtctgaatttcaatttgctcgatcacgtgacgatcaggctttgtctctgcttggggaatgaaccgcatcaatgtctggtaatcgacgtatggtcggcgcagaaagattgatgccagtaccccgtcttgcaacggtttgtcaccgtgttcctgaacaaactggttcacttcatctgacggcttaatccgaatggtgttcaaacgatcaaattcagcttcaatggcctttttcttagctaagaacttagcgtagcgctcgtcagaaattaagccaatctcgtggcctttttctgtcagacgcatgtcggcattgtcagtccgcaacaataaacgatattctgctcggctggttaacaaacggtatggttctttggtccctttggtaaccaaatcatcaatcatgacgccgatgtatgcttcgttccgttttaagacaaatggccctttgccaagtgcgcgacgaccagcgttgatgccggcaatcagcccttgaccggcagcttcttcatagcctgatgttccattggtttgaccggctgtaaagaggtttttgacaactttggtttccaaagtcggcttcagttgatagggtgcaacgacatcgtattcgattgcgtagccgggccgcatcatctgggcattttccatgccgacgattgaatgaatcattttttgctggacctcttcgggcatcgaagttgacaggccatcgacataccattcctcggtttttctgccttcaggctccaaaaatagttggtggcggctcttgtcagcgaaacgaaccactttatcctcaattgatgggcaataacggggaccgactccctcgataacaccagtaaacattggtgcccgatcaagattatcgcggataatcttgtgggtcgtttcattcgtgtaggtcaaccagcaggatagctggtctttgactgccaggtagttctcatcagaagattcaaaactaaagtggtgcggtttctcatcgccaggttgttcctctgtcttggagtagtcaatcgttgtcccgtcaactcgcggtggggttccagtcttgaaacgctccaaatcaaaaccgagcgcttccaagttgcctgaaagtttttcagccggttgtgagttgttaggtccagaagcgtacatcaactcgccaatgataatctttccacgagcagcggttccggcagcgatgacaactgccttggcataacactcagcgccagtattggtgataacccctttacaaacaccgtcttcaacaatcaaggaatcaacaattccctgacgcaaagtcaaattgggttctttttcaatcgtatgtttcatctcggcgtgataggcatgtttatcagcttgtgcacgcaacgcttgaactgctggtcctttaccggtgttcaacatccgcatttggatgtatgtcttatcaatattcttgcccatttcgccgcctaaagcatcaacttcgcggacaactgtccctttggcagggccaccaacggatggattacatggcataaatgccaccatatccaaattaatggtcagcaagagggtcttgttgcccattctggcggcagccaaagccgcttcacagcctgcatgaccggcgccgacgacaatgacatcataatcttggccgcgatatttttgtttaacatcgctaactcgtaaacttttcactgtttttcctccaaatgtttcacgtgaaacaggttattttcctaaacagaattgactgaataactgatcaattaactcatcttggtaactgtcgccggtaatctcacctaagaaatcccagcagcgagtcatgtcaatttgaaccaaatcaaccggcatgccatcatccaatcctttgacaacgtcttccaaagcctgtttggcttgatttaacagaccgatgtggcgggcattggtgaccataatgtcgttttgactgctttcaattccttcatcaaagaacatcttggcaatcaattcttccagctgcgtcaacccgtctgccttaatcgctgaagtcgaaataacgttctggccgtcagctagagacttaatttggtcttgatcaattttggttggtaaatcagtcttattgaggatgatgatccgctgtttgtcttgagtggcactcaataactttttgtcctcatcggttaatggctcactggcgttaagcaccagcagcaccaaatcggcactattaatggcttttctggaacgatcaacaccgattttttcaactttgtcagtcgtatcgcgaattccggccgtatcaaccaattttaatggcacgccgtggacattgacatattcttcaaggacatctctggtagtaccgggcacatcggtcacgattgccttgtcttcatgaagtaaattgttcaacaaactggacttaccgacgttgggccgaccaataatcgaagtggccaaaccttctcgtaagatcttgccttgtttggcagtcttcagcagttgcacaattcgcgcatggacatcggtcgccttttcccgcaacaatttactagtcatggtttcaacatcatcgtactcaggatagtcgatgttgacttctacttgggcaagcacgtcgagaatatcttggcgtaaatgtttaatcaaatgcgatagattaccatccaattgattaatcgccgctttcattgaacggtcagttttggcttcaatcagatccatgacggcttcagactgtgacaaatcaattcggccgttgagaaatgcccgtttggtaaactcaccaggctcggccattctggcaccgtgactcagtgccaactgaagaatccgattggtggcaacaatcccaccatgacagttaatttcaacaatatcctcttcagtataagtgtgaggggctctcatcacggagagcattacttcatcgacctcttcgttggtatccggatcaatgatgtggccataattaatggtgttgctggcaactttatcaaggtctttaccacgatagagcttttttgcaacatcaagtgcttcttcaccgctaatgcggataatcgaaatcccgccctcaccaggtggtgttgaaatcgctgcaatcgtatcaaattctgttgttgttaaaaccatgattaagcttccctccacgaataattgaatagtgttctaatttaaccacaaaacttatctaaaagcacaaaaaaagcgccactccatgccaaaaaagatagcatggataaagcactttgactactttacctagttaagataagaatgattacctacataatattttaaagcaatgcatttgtcaattgattttgagaactattttggtgcaacgacaatgacacgatgaggttctttgccggttgaatacgtcatcacgtgatcattgtcagccaaagcattatgaatttgtttgcgttcaaatgccggcattgggttcaagtagactggcttgccgttggcaatggcattccgagcagtcttatcggccagttgaaccagcgactcgcttcttctggaacggtagtttgcggtatccaactcaacggtaacgttgttggcacccagtcgattaataaaaatctgtgacaagttttggagcgcattaatcgtgcggccatgacggccgattaagcggctctcctggtcagtatcaatgtcaatatagattgaatgccgattctttaaatccagcttcaatttgaacgagaagcccattgcttctaaaacatcgttcaaatagttggcaagtttttgggaaacttcttcaatgtcaacggcgttttcagtttcttcctcatgatgttttgattctgaaaccggctgattagttgatttattaaggtttgtctgttgtttagtgttagttttactgacaagttcaacctgtgcaagtttgcgaccgaaacctaaaaatccattcttaggttgttgaataacggtaacttcaacttggtccgaagtgagtgatagtgcggttaaaccctgttctacggcgtcttggatggtttttccagagtaaattgtcataatgaactccctttatttgaattaactggttaataatagcataaaaacgcgcattattaaacggtttgttgcgaaaaacggaaactaaacgcaaactttaaatgatttgtcacatttcaaagcatcaaactaccatctcactacaaagtcgatataatggggtgtagtagcttttttaagaaagatggtttcgtctgaatcgacatcaatctatagtgacggctgctttaggttttcgatttgggaagtgataaaatggcaaacacaaatcaatatgacgccggccgaaacattcaaatcgaccgtcagcaccgacttagcaagcttcaggaagcctcgcagatcacctgggtcaacctgagtgcctactcggccatcatggttgccgaactgatcattgggtatttggcacaaattaccgttttgattgccgatgggctgaataacctcaccggtgtttgtggtgcagctattttaatcattggcctgaaaatgtccaagcgcccaccggactccaatcacgtgatgggccactggcagtatgaaaatattgccgcacttttatctgcgacaatcatgtttgcagtcagtatccaaatttttgttgacggcgtttttgctgtccagcgattcctggctggtcacaccattcgaccgaatgactggtcgctgggcgtcagcatcattgcagccatgatcattggcatcttggcccggttcaataaaaccaagggtattcagctgaaaaatcaagctctcaccgcctccggacaagaccttaaaagtgatgcctggaccagctttggaacatttctttccattggcggtgcctacctgggggcccaatggctggatggagtggcaactttgattgtcggctgcctgattctccactcatcaattagtatttttagaacaaccattatgagattgagtgaaggttttgatccaaaagatattcaacgttatagtgagaccattagtgccatccctggggtcctcggaattgaagggattgagccacggtggctcggagatcaaattgtcatgaaaatcggcatctatctggatgatgacaccgatttaaaaacagcctatgcaattggtgaaaaagttgaacacaatttgatggagaaatacgatattctcgatgccgatgtgatgagctatccggtcagtcaaaaagacaatccgcattcggcagattaatcaaaatggtttgacaaataaaaaaaacagcgctatattcaattttaattaaatgataatttgttaaacaaaatgaatcggtgagtagtttgaagttgtctatcagagagttggcgctgatggaagccaatattcaacttaaatgaagatggccgatgattggttgttgtgagtcaataacgagcagcagacggatgagtccccgttagcagacacaccatcgactttcgatggttatcaaggtttgacgagtaatcgtcaaataaatcagaatggtaaagtgttattcgcttctgcagcattggctgcagaagcattttttcatttaatgaataaaaaattataaatttggggtggcaatcatggcaaaattagcaattgtaactggcgcaggacaaggaatcggagaaggcatcgctcatcgactggcaaaagatgggttcgcgattgcagtcgcagatatcaatggggaaacagctgataaggtaaccgcagacttgactaacgacggctacactgccaaatcgtatcatatcgacgtggctgaccgcgaacgggtctttgaattagtgcaaaaagcggttgccgatcttggtgagcttgccgtgtacgtcaataatgccggggtggctttcatcaacgaaattgttgattccgcggaaaaagacatccggcgattattggatgtcaatttattaggaacttattggggaacccaggcggcggccgaacaattcaaaaaacagggtcacggtggtcgaatcgttaacgcggcctccctggccggtgttgaggcatctgctctgcaaagcgcttattcgatttcaaagtttggcgttcggggaattactcaagcagcttcgaaggaattggcaaaggaccaaatcaccgttaacgcttacgatccaggaattgtcagaacacctctaagagacggcatcgacaaacggaccgctgaaatcaaaggaatctctgtcgctgaacaacaaaaaaactgcctcagtgaaatctcactgggcagagaagcgacaccagaagacgttgccaaagtcgtttcgtggtttgcatcccctgatgccgcttatatcaccggccaatcaattctagtggatggtggcatgagatatcaataggataatcgaaaacgattgtaatttaaaaggacagccattaaagtgaacccctaaggttggacaccaaatctaaccttgggggttttactatgtcaaaatttaatttagaacttcgaataaaggtcgttactgaatacttatctggtaaaggttcaccgtctctagctaagaagtatcgcattagcaatcattcaatcattctggactgggttcatcgatttgagcggcgaggtattgaaggtctaaaagaccggtcaatgtcccaagaatattctagtcagttcaaagtcgatgtattaaactggaagaaacgaaatcaagcttcgcttccagtgactgccttacactttgacttgtcgtcgccaagtacgatttggcagtgggaaaaacacttccaggaatctggaatagcgggacttgagcgcaaacgagggaatcctaagaccatggtcaaacacaagcagaacaaccccaaacctgaaaaaccacagactccagccgcagaattgaagcagctaaaacaagagaatcaaatgttaaaaatagaaaatgaattcttaaaaaaactcgatgccttagcacgaaagaagtcaaaacacacgaactcatcgaactagtagacgagttaaggcagaattttcaagtttccatcaaactagttcttaaggctgttcgtattccccgtagcacgtattattatgctaaggagcatcgtggtcgtaacttagatgattcacaaattattcaggcaattgatgagattcgtcaacaagatccaaaatatactcggaaatacgggtaccgacgaataaccggtgctttacatgacgcttatggctttaaaatcaatcataagcgggtcttacggattatgcgggaacaagactggctatgtggcgcctttaatcggcagaaacgaaagtataattcttacaagggaactgttggcgtcatcgccccaaatcgacttaagcgacgattcaaaacagatcggccttaccagaagttagtcaccgacgtcagtgaattccgatatgggaaccaaagtcaaaatgaacgggtttatttagaaccagtcctcgacctcttcaatggagaggttctggctttcaatatcagtgaccacccgaccgttgaatttgctttaaaacctttgaaagaagccctaaatcgaataccggtgttagattatcggacaaccgtccatactgaccaagggtttcagtatcagcatcgccactggcaagacacgcttaaagagcaccatgtatttcagagtatgtcgcgtaaagccacttgtctcgacaacgccgccatggagtcgttttttcacattatgaaagtcgaggttatggatgaacattttgagaccaaaacagcgcttatcgaagctatgaacgaatggatagacttctacaatcatcggcgcatcaaaacaaaactggacggcaagtccccggtaaaataccgggaacttaccgtccagaaagcagcttaataaagttgtccaattttaagggttcactttaatgagcacaatctcatcgctgtctttttgtttgaactctacccgttaagccattttaataacaatctttccaacggaccggccggctgcggagtaatccatagcagattggatatcggaaaacggcaccacccgatcaatgaccggctgaagggtcccatgttcgaccattttggttatcttggacaattgggtcccactaggtttcatgaataaaaactcatagccaacctgaaattggcgctgcagtcgcctcatttttgctgtagccagggaaaacgccagttgtttccacattggcaggccagcctgctgggcgaatgcccgatttggcagacccgaaattgaaactactttgccgcggggtttcacgacttgaaacgcgttagctaattgtgaaccacccagtgtatcaaacacgccatcgtaatcaaacaagacatcttcaaatgccgtttgatgatagtcgatgacctgatcggcccccaactgcctgaccaaacccgtattctttgcgctggtggtcgttgccacaaaggctcccaatgacttggccagttgaatcgcaactgtcccaatcccaccggaccccgcctgaatcaagactttatctccaggcttaacgtgcatcaagtcaattaacgcttggtaactggtcagcgaaaccagcggcagtgctgcggattccaccagtgataagttggccggtttcagggcaatatcaccctgatccaccgccaaataatcggcaaaagttccgatccgattcttctgtacccgaccatatacctcatcaccaaccttgaagtccttcaccaatgttcccgtctgaacaactgtcccagaaaaatcactccctaatctcaatggcatcgaatacttcaacagcattttaagtttgccatcgcgggtctttaaatcaatcggattaatacttgccgcagcaactttcactaacacgtcatgatccctaattgttggaatcggcacgtccgcgatctctaattgctgctgcccaaaatgctggatctgggcagctttcatcatttttgtcatcattactagctccactttattggtttaaatttttgaacgaatggtgtccaaatcataaatcacaattcagcggacgtcaagtaagacggtttaatgccaattcgttgacggctgagaaataaaatggtttaatggtttaaaaatatgaaccgagaggaacttacgatggctgatttacaccaaattcaaactgaattcaccaatgtcagcagtttcttaactgctttaggggaccaaaaacggcaagcaattatcatttccctgttaaaaaccaattcttgtgaggggctgcaagttcctgaacttaccagtgtcactggcttatcgagaccggcagtttcccaccatttgaaaattttgaaagatgcccatttagtggccgtcagaagtgaaggaaccaagaacttctactacctgtcccatgacatcaaggaaattgatgaactaaaaacccttctggatcacgtcacagcaatcattcatcaaacggagaccaaatcatgaaaaaagtattgattgttttaacgaatgttacccgttatcaaggcacgaacgatcccaccggtttatggttgggggaagcaactgaatttgccgaaacaattcagaaggctgggattgacgtcgactatgtcagtccaaagggcggctttgtgccacttgatccacgcagtatgaaatacactaacgaatcgatcataaaattctatgaaactgaggattttcaaaaacgggcgttgaccaactcactgcggccaaatgaaattaatcccgacgattatttggcaatctactacactggcggccacggagtgatgtgggattttccaaatgaccgggctctccagcaaatcgccttgtcaatttacgacaacggtggatacattacctccgtttgtcacggagttgcagggttactcaacattaaggacgatgccggtcgctatttaattgccggcaagtcaatcactggtttcacaactgcagaggaaatcatcgccggcaaaaaatcagtggttccctttctgaataagcaagcagttgaaaagcgcggtggtaaattcaaaaagaagcgggcttacaaggagtatgccattcaagatggtcacttgattactggccaaaatccattctcaccacgggctgtcgctcggctattacttgaaaacgtgcaataaataaatatattaaagcggggccaaggcatcagtgtattcgactgataccttggccccgctttaagtttggacgctaaatcaaacgtccggatctcattagttgatgagctgaatcagcttcccaattcgaaaaccagtctgctcaatcaattgaggagcttggtgaatcgcttcttgaacggtcagcggacgggtcgtggtggaaacaatcaagtcaaatccttgatcgtataatggttggatatcggcggccaaactcccggcaacggcaattaccggaactttggccgaatcagccagtttggcaacccccattggcaatttgccgctgagggtttgtgagtcaatccgcccctcaccggtaatgacccaatcagcatcacaaagcatcgcctttaagtccaccaacttcatgatttcatcaattcctgacgttaacttgccttttagaaaggccaggacgccaaatcccaaaccgccagctgctccagctcctggtacctgtgaaaggtccttccccacagtagcagcagtcagtcgcgccagtcgttgcagccgggcatcaaaatccgcaatctgttcatcttgaatccctttttgtggcccaaatatccgtgtagcacccaattggccggtcagtggattctcgacatcagaaagaccgatcatttgaactgtggacatccggtgatcaatctgggtcaaatcaactttgtccaggtctttgagtccgccaattccacgggagatctcataaccgtttcgatcataaaaatgaccacccaaagcctgagccatgccaacgccaccatcgttggttgaactaccaccaagtcccagaaggattttgctgacgccgtgatccagtgccgcttcaatgagttcccctacaccataagtggaccgaacagcaacatctgtcgtttggccctgcgtgtatccagccgctgcagccatttcgatcactgccgtttgatcgtcaatctgaccccatttagcgtcgatttgactgccggtaggtccagacacccgcgtcgatattaagtggcccttagtcgcgttgacaatggctgttacggtgccttcacccccatcagccagcggtacttttttgattttaagactgggattggccgccgtaagtccccgttgcaaattctccgccacttcctgtgagctggcactgcctttaaatgaatcggtcgcaattacaattgttttcatcgtcaacttcctttaactaactgttgaccttagtgtacctgaatatggatcgttcaacaaaaaagcagcgtgatcaaatgatcacgctgcttgctaattatttacgtttactcttcttggcacgtttaatggcttttttaattgcccgttgtttctcacgctcttcgcgttgtttattttcacgttcgcgacggatcttccaaggattttggataaccagggtttgacctacttggaacgcgttggtgatcacccaataaagtgacagggctgatggcaggctaatagccataatcaaaatgaagaatggcattccgaccgtcatcatcgtggtcattgaattagattcaggctgacctttcattgccagccacgaagaaatgaaggtgaacagggcagctaggatcggcaagacaaagtatggatccggatgaccaagctgcagccagaagaacgttccacttctcaaaatgtgggttcgccaaattgcttggtacaaggcgaacagaattggcatctgaacgatcaatggcaggcagccggcaagcgggttaatgcctgcttcggcatacagcttcttttgctctgcttgaagcttctgaacagtttctgcatctcttgatgaatattttttctgcaatgccttcagctgcggttggacttcttgagtcttacgcatacttctggtttggtaaatcatcaatggcagaatcacgatccggacaagaatggtgaagataatgattcccattccgtagttgtcgctaaagaatttagacagccagatgatggcccgcgagaagttcaaaacaacccagccatcccaaatgcccgtactgtgattggttattggtgcgttactacatgcggaaagtactaccgtcaaacttactaatgatagtaatactagtaatttctttattctctttttcaacttttttcctcactatcatagttgggatcgattagtttagctaacttgagcacatgaattaaacttgccttgacatcactcatcgacatctggtcagcagccggacgggcaatgacaataaagtccacgtcctgacgaagataaggctttaattccaacaaggactgacgaattcttcgcttgacccaatttctatgtaccgcattaccgatcttcttaccaacagaaataccgacgcgaaaatgtaattgattgggtttatccaaagaatagacaacaaattgacgatttgcaacagagttatgagtctcaaagacttcttgaaattcactctctttttttactcgatacgattttcgcatgatccatctccacagacttttgaaaaataaatgaaaaagaccactgaatggtcagtggtctatgcagacaatgattttctacctttttgacgtcggcgagccaacactttacgaccattgctggtactcatacgtttacgaaagccatgaacgcgagcgcgatgacgtttctttggttgataagttctcttcataatgaattcctcctttaactgtaaaagtcgcgtttaagcatttaattacaattatgttcaaatgcatttcccaaatatattaacataatttgttcattaatggaatagtcttttgaatgatcgcacatttcaaaaaa

(The sequence listing continues in the following parts.)